European Patent Application EP 4 686 757 A1, published February 4, 2026. Title: INHIBITORS OF EXPRESSION AND/OR FUNCTION. Applicant: e-therapeutics PLC. The sequence listing filed with the application follows.

SEQUENCE LISTING (1391 sequences)

SEQ ID NO: 1 - RNA, 23 nt, Homo sapiens
  source 1..23: mol_type = mRNA
actatttactggttgaaaatggg

SEQ ID NO: 2 - RNA, 23 nt, Homo sapiens
  source 1..23: mol_type = mRNA
tacaaaggcattatagactgcgt

SEQ ID NO: 3 - RNA, 23 nt, Homo sapiens
  source 1..23: mol_type = mRNA
tatgatgaaatcaagaagtacac

SEQ ID NO: 4 - RNA, 23 nt, Homo sapiens
  source 1..23: mol_type = mRNA
atgatgatgggactcaattgtat

SEQ ID NO: 5 - RNA, 23 nt, Homo sapiens
  source 1..23: mol_type = mRNA
aggcattatagactgcgtggtcc

SEQ ID NO: 6 - RNA, 23 nt, Homo sapiens
  source 1..23: mol_type = mRNA
cagtcactcctgataaataacaa

SEQ ID NO: 7 - RNA, 23 nt, Homo sapiens
  source 1..23: mol_type = mRNA
caatacaaaggcattatagactg

SEQ ID NO: 8 - RNA, 23 nt, Homo sapiens
  source 1..23: mol_type = mRNA
gagccgcctacttcggtatctat

SEQ ID NO: 9 - RNA, 23 nt, Homo sapiens
  source 1..23: mol_type = mRNA
cgagccgcctacttcggtatcta

SEQ ID NO: 10 - RNA, 23 nt, Homo sapiens
  source 1..23: mol_type = mRNA
atagactgcgtggtccgtattcc

SEQ ID NO: 11 - RNA, 23 nt, Homo sapiens
  source 1..23: mol_type = mRNA
aacactcacatcgtcatcagctg

SEQ ID NO: 12 - RNA, 23 nt, Homo sapiens
  source 1..23: mol_type = mRNA
taacttcgccttcaaagataaat

SEQ ID NO: 13 - RNA, 23 nt, Homo sapiens
  source 1..23: mol_type = mRNA
gcctacttcggtatctatgacac

SEQ ID NO: 14 - RNA, 23 nt, Homo sapiens
  source 1..23: mol_type = mRNA
tatttactggttgaaaatgggaa

SEQ ID NO: 15 - RNA, 23 nt, Homo sapiens
  source 1..23: mol_type = mRNA
tttgcccgtacccgtctagcagc

SEQ ID NO: 16 - RNA, 23 nt, Homo sapiens
  source 1..23: mol_type = mRNA
gcagtcagggcgcaaaggaactg

SEQ ID NO: 17 - RNA, 23 nt, Homo sapiens
  source 1..23: mol_type = mRNA
atttactggttgaaaatgggaag

SEQ ID NO: 18 - RNA, 23 nt, Homo sapiens
  source 1..23: mol_type = mRNA
ccgagccgcctacttcggtatct

SEQ ID NO: 19 - RNA, 23 nt, Homo sapiens
  source 1..23: mol_type = mRNA
ggcctcggtgactgcctggttaa

SEQ ID NO: 20 - RNA, 23 nt, Homo sapiens
  source 1..23: mol_type = mRNA
cacatcgtcatcagctggatgat

SEQ ID NO: 21 - RNA, 23 nt, Homo sapiens
  source 1..23: mol_type = mRNA
tatttcagtcactcctgataaat

SEQ ID NO: 22 - RNA, 23 nt, Homo sapiens
  source 1..23: mol_type = mRNA
gctggatgatcgcacagactgtc

SEQ ID NO: 23 - RNA, 23 nt, Homo sapiens
  source 1..23: mol_type = mRNA
aagcaatacaaaggcattataga

SEQ ID NO: 24 - RNA, 23 nt, Homo sapiens
  source 1..23: mol_type = mRNA
aggcctcggtgactgcctggtta

SEQ ID NO: 25 - RNA, 23 nt, Homo sapiens
  source 1..23: mol_type = mRNA
ggctttaacgtgtctgtgcaggg

SEQ ID NO: 26 - RNA, 23 nt, Homo sapiens
  source 1..23: mol_type = mRNA
acaaaggcattatagactgcgtg

SEQ ID NO: 27 - RNA, 23 nt, Homo sapiens
  source 1..23: mol_type = mRNA
ctgtgaacaggcatgttgtatta

SEQ ID NO: 28 - RNA, 23 nt, Homo sapiens
  source 1..23: mol_type = mRNA
tcatctgaccagttttctcttaa

SEQ ID NO: 29 - RNA, 23 nt, Homo sapiens
  source 1..23: mol_type = mRNA
caaggctttaacgtgtctgtgca

SEQ ID NO: 30 - RNA, 23 nt, Homo sapiens
  source 1..23: mol_type = mRNA
atgcagtcagggcgcaaaggaac

SEQ ID NO: 31 - RNA, 23 nt, Homo sapiens
  source 1..23: mol_type = mRNA
tggatgatcgcacagactgtcac

SEQ ID NO: 32 - RNA, 23 nt, Homo sapiens
  source 1..23: mol_type = mRNA
aaaggcattatagactgcgtggt

SEQ ID NO: 33 - RNA, 23 nt, Homo sapiens
  source 1..23: mol_type = mRNA
gatgatcgcacagactgtcactg

SEQ ID NO: 34 - RNA, 23 nt, Homo sapiens
  source 1..23: mol_type = mRNA
gactgcgtggtccgtattcccaa

SEQ ID NO: 35 - RNA, 23 nt, Homo sapiens
  source 1..23: mol_type = mRNA
agcaatacaaaggcattatagac

SEQ ID NO: 36 - RNA, 23 nt, Homo sapiens
  source 1..23: mol_type = mRNA
gtcatcagctggatgatcgcaca

SEQ ID NO: 37 - RNA, 23 nt, Homo sapiens
  source 1..23: mol_type = mRNA
gcattatagactgcgtggtccgt

SEQ ID NO: 38 - RNA, 23 nt, Homo sapiens
  source 1..23: mol_type = mRNA
attttgcccgtacccgtctagca

SEQ ID NO: 39 - RNA, 23 nt, Homo sapiens
  source 1..23: mol_type = mRNA
tcacatcgtcatcagctggatga

SEQ ID NO: 40 - RNA, 23 nt, Homo sapiens
  source 1..23: mol_type = mRNA
cctcttgattttgcccgtacccg

SEQ ID NO: 41 - RNA, 23 nt, Homo sapiens
  source 1..23: mol_type = mRNA
ttatagactgcgtggtccgtatt

SEQ ID NO: 42 - RNA, 23 nt, Homo sapiens
  source 1..23: mol_type = mRNA
gccgcctacttcggtatctatga

SEQ ID NO: 43 - RNA, 23 nt, Homo sapiens
  source 1..23: mol_type = mRNA
tagactgcgtggtccgtattccc

SEQ ID NO: 44 - RNA, 23 nt, Homo sapiens
  source 1..23: mol_type = mRNA
cgtcatcagctggatgatcgcac

SEQ ID NO: 45 - RNA, 23 nt, Homo sapiens
  source 1..23: mol_type = mRNA
cattatagactgcgtggtccgta

SEQ ID NO: 46 - RNA, 23 nt, Homo sapiens
  source 1..23: mol_type = mRNA
cgcctacttcggtatctatgaca

SEQ ID NO: 47 - RNA, 23 nt, Homo sapiens
  source 1..23: mol_type = mRNA
ttttatttcagtcactcctgata

SEQ ID NO: 48 - RNA, 23 nt, Homo sapiens
  source 1..23: mol_type = mRNA
tcgtcatcagctggatgatcgca

SEQ ID NO: 49 - RNA, 23 nt, Homo sapiens
  source 1..23: mol_type = mRNA
tgattttgcccgtacccgtctag

SEQ ID NO: 50 - RNA, 23 nt, Homo sapiens
  source 1..23: mol_type = mRNA
tgcaaagggaatgcttccggatc

SEQ ID NO: 51 - RNA, 23 nt, Homo sapiens
  source 1..23: mol_type = mRNA
ccaaggctttaacgtgtctgtgc

SEQ ID NO: 52 - RNA, 23 nt, Homo sapiens
  source 1..23: mol_type = mRNA
caaaggcattatagactgcgtgg

SEQ ID NO: 53 - RNA, 23 nt, Homo sapiens
  source 1..23: mol_type = mRNA
tcttgattttgcccgtacccgtc

SEQ ID NO: 54 - RNA, 23 nt, Homo sapiens
  source 1..23: mol_type = mRNA
accgagccgcctacttcggtatc

SEQ ID NO: 55 - RNA, 23 nt, Homo sapiens
  source 1..23: mol_type = mRNA
ttatcatctaccgagccgcctac

SEQ ID NO: 56 - RNA, 23 nt, Homo sapiens
  source 1..23: mol_type = mRNA
cttgattttgcccgtacccgtct

SEQ ID NO: 57 - RNA, 23 nt, Homo sapiens
  source 1..23: mol_type = mRNA
attatcatctaccgagccgccta

SEQ ID NO: 58 - RNA, 23 nt, Homo sapiens
  source 1..23: mol_type = mRNA
atcatctaccgagccgcctactt

SEQ ID NO: 59 - RNA, 23 nt, Homo sapiens
  source 1..23: mol_type = mRNA
ggctcttaacttcgccttcaaag

SEQ ID NO: 60 - RNA, 23 nt, Homo sapiens
  source 1..23: mol_type = mRNA
ccccacccaggctcttaacttcg

SEQ ID NO: 61 - RNA, 23 nt, Homo sapiens
  source 1..23: mol_type = mRNA
gtccgtattcccaaggagcaggg

SEQ ID NO: 62 - RNA, 23 nt, Homo sapiens
  source 1..23: mol_type = mRNA
aggagcagggagttctgtccttc

SEQ ID NO: 63 - RNA, 23 nt, Homo sapiens
  source 1..23: mol_type = mRNA
attcccaaggagcagggagttct

SEQ ID NO: 64 - RNA, 23 nt, Homo sapiens
  source 1..23: mol_type = mRNA
ggtccgtattcccaaggagcagg

SEQ ID NO: 65 - RNA, 23 nt, Homo sapiens
  source 1..23: mol_type = mRNA
gagcagggagttctgtccttctg

SEQ ID NO: 66 - RNA, 23 nt, Homo sapiens
  source 1..23: mol_type = mRNA
tggtccgtattcccaaggagcag

SEQ ID NO: 67 - RNA, 23 nt, Homo sapiens
  source 1..23: mol_type = mRNA
ggagcagggagttctgtccttct

SEQ ID NO: 68 - RNA, 23 nt, Homo sapiens
  source 1..23: mol_type = mRNA
aaggagcagggagttctgtcctt

SEQ ID NO: 69 - RNA, 23 nt, Homo sapiens
  source 1..23: mol_type = mRNA
tattcccaaggagcagggagttc

SEQ ID NO: 70 - RNA, 23 nt, Homo sapiens
  source 1..23: mol_type = mRNA
caaggagcagggagttctgtcct

SEQ ID NO: 71 - RNA, 23 nt, Homo sapiens
  source 1..23: mol_type = mRNA
tccccacccaggctcttaacttc

SEQ ID NO: 72 - RNA, 23 nt, Homo sapiens
  source 1..23: mol_type = mRNA
gctcttaacttcgccttcaaaga

SEQ ID NO: 73 - RNA, 23 nt, Homo sapiens
  source 1..23: mol_type = mRNA
atttcagtcactcctgataaata

SEQ ID NO: 74 - RNA, 23 nt, Homo sapiens
  source 1..23: mol_type = mRNA
ttcagtcactcctgataaataac

SEQ ID NO: 75 - RNA, 23 nt, Homo sapiens
  source 1..23: mol_type = mRNA
tttcagtcactcctgataaataa

SEQ ID NO: 76 - RNA, 23 nt, Homo sapiens
  source 1..23: mol_type = mRNA
gatgatgggactcaattgtattt

SEQ ID NO: 77 - RNA, 23 nt, Homo sapiens
  source 1..23: mol_type = mRNA
atgatgggactcaattgtatttt

SEQ ID NO: 78 - RNA, 23 nt, Homo sapiens
  source 1..23: mol_type = mRNA
gtcactcctgataaataacaaat

SEQ ID NO: 79 - RNA, 23 nt, Homo sapiens
  source 1..23: mol_type = mRNA
atattcatctgaccagttttctc

SEQ ID NO: 80 - RNA, 23 nt, Homo sapiens
  source 1..23: mol_type = mRNA
tgaacaggcatgttgtattatat

SEQ ID NO: 81 - RNA, 23 nt, Homo sapiens
  source 1..23: mol_type = mRNA
aaagggaatgcttccggatccca

SEQ ID NO: 82 - RNA, 23 nt, Homo sapiens
  source 1..23: mol_type = mRNA
aagggaatgcttccggatcccaa

SEQ ID NO: 83 - RNA, 23 nt, Homo sapiens
  source 1..23: mol_type = mRNA
tccgaggcctcggtgactgcctg

SEQ ID NO: 84 - RNA, 23 nt, Homo sapiens
  source 1..23: mol_type = mRNA
gaacaggcatgttgtattatata

SEQ ID NO: 85 - RNA, 23 nt, Homo sapiens
  source 1..23: mol_type = mRNA
gcaatacaaaggcattatagact

SEQ ID NO: 86 - RNA, 23 nt, Homo sapiens
  source 1..23: mol_type = mRNA
ttatttcagtcactcctgataaa

SEQ ID NO: 87 - RNA, 23 nt, Homo sapiens
  source 1..23: mol_type = mRNA
tgatgatgggactcaattgtatt

SEQ ID NO: 88 - RNA, 23 nt, Homo sapiens
  source 1..23: mol_type = mRNA
atctgaccagttttctcttaaag

SEQ ID NO: 89 - RNA, 23 nt, Homo sapiens
  source 1..23: mol_type = mRNA
tctgaccagttttctcttaaagc

SEQ ID NO: 90 - RNA, 23 nt, Homo sapiens
  source 1..23: mol_type = mRNA
cagataagcaatacaaaggcatt

SEQ ID NO: 91 - RNA, 23 nt, Homo sapiens
  source 1..23: mol_type = mRNA
agataagcaatacaaaggcatta

SEQ ID NO: 92 - RNA, 23 nt, Homo sapiens
  source 1..23: mol_type = mRNA
ctttaacgtgtctgtgcagggta

SEQ ID NO: 93 - RNA, 23 nt, Homo sapiens
  source 1..23: mol_type = mRNA
tttaacgtgtctgtgcagggtat

SEQ ID NO: 94 - RNA, 23 nt, Homo sapiens
  source 1..23: mol_type = mRNA
actcacatcgtcatcagctggat

SEQ ID NO: 95 - RNA, 23 nt, Homo sapiens
  source 1..23: mol_type = mRNA
gatgatgatgggactcaattgta

SEQ ID NO: 96 - RNA, 23 nt, Homo sapiens
  source 1..23: mol_type = mRNA
agactgcgtggtccgtattccca

SEQ ID NO: 97 - RNA, 23 nt, Homo sapiens
  source 1..23: mol_type = mRNA
gtgaacaggcatgttgtattata

SEQ ID NO: 98 - RNA, 23 nt, Homo sapiens
  source 1..23: mol_type = mRNA
tttatttcagtcactcctgataa

SEQ ID NO: 99 - RNA, 23 nt, Homo sapiens
  source 1..23: mol_type = mRNA
gataagcaatacaaaggcattat

SEQ ID NO: 100 - RNA, 23 nt, Homo sapiens
  source 1..23: mol_type = mRNA
acactcacatcgtcatcagctgg

SEQ ID NO: 101 - RNA, 23 nt, Homo sapiens
  source 1..23: mol_type = mRNA
agccgcctacttcggtatctatg

SEQ ID NO: 102 - RNA, 23 nt, Homo sapiens
  source 1..23: mol_type = mRNA
ctcacatcgtcatcagctggatg

SEQ ID NO: 103 - RNA, 23 nt, Homo sapiens
  source 1..23: mol_type = mRNA
ccgcctacttcggtatctatgac

SEQ ID NO: 104 - RNA, 23 nt, Homo sapiens
  source 1..23: mol_type = mRNA
gctttaacgtgtctgtgcagggt

SEQ ID NO: 105 - RNA, 23 nt, Homo sapiens
  source 1..23: mol_type = mRNA
gttcgccgccgcatgatgatgca

SEQ ID NO: 106 - RNA, 23 nt, Homo sapiens
  source 1..23: mol_type = mRNA
ggcattatagactgcgtggtccg

SEQ ID NO: 107 - RNA, 23 nt, Homo sapiens
  source 1..23: mol_type = mRNA
actgcgtggtccgtattcccaag

SEQ ID NO: 108 - RNA, 23 nt, Homo sapiens
  source 1..23: mol_type = mRNA
tcatctaccgagccgcctacttc

SEQ ID NO: 109 - RNA, 23 nt, Homo sapiens
  source 1..23: mol_type = mRNA
ttttgcccgtacccgtctagcag

SEQ ID NO: 110 - RNA, 23 nt, Homo sapiens
  source 1..23: mol_type = mRNA
cactcacatcgtcatcagctgga

SEQ ID NO: 111 - RNA, 23 nt, Homo sapiens
  source 1..23: mol_type = mRNA
attatagactgcgtggtccgtat

SEQ ID NO: 112 - RNA, 23 nt, Homo sapiens
  source 1..23: mol_type = mRNA
gaggcctcggtgactgcctggtt

SEQ ID NO: 113 - RNA, 23 nt, Homo sapiens
  source 1..23: mol_type = mRNA
ctggatgatcgcacagactgtca

SEQ ID NO: 114 - RNA, 23 nt, Homo sapiens
  source 1..23: mol_type = mRNA
ttgattttgcccgtacccgtcta

SEQ ID NO: 115 - RNA, 23 nt, Homo sapiens
  source 1..23: mol_type = mRNA
atgatcgcacagactgtcactgc

SEQ ID NO: 116 - RNA, 23 nt, Homo sapiens
  source 1..23: mol_type = mRNA
ggatgatcgcacagactgtcact

SEQ ID NO: 117 - RNA, 23 nt, Homo sapiens
  source 1..23: mol_type = mRNA
gattttgcccgtacccgtctagc

SEQ ID NO: 118 - RNA, 23 nt, Homo sapiens
  source 1..23: mol_type = mRNA
tatcatctaccgagccgcctact

SEQ ID NO: 119 - RNA, 23 nt, Homo sapiens
  source 1..23: mol_type = mRNA
tatagactgcgtggtccgtattc

SEQ ID NO: 120 - RNA, 23 nt, Homo sapiens
  source 1..23: mol_type = mRNA
cactgcagataagcaatacaaag

SEQ ID NO: 121 - RNA, 23 nt, Homo sapiens
  source 1..23: mol_type = mRNA
tcactgcagataagcaatacaaa

SEQ ID NO: 122 - RNA, 23 nt, Homo sapiens
  source 1..23: mol_type = mRNA
atcactgcagataagcaatacaa

SEQ ID NO: 123 - RNA, 23 nt, Homo sapiens
  source 1..23: mol_type = mRNA
cagcaagcagatcactgcagata

SEQ ID NO: 124 - RNA, 23 nt, Homo sapiens
  source 1..23: mol_type = mRNA
agatcactgcagataagcaatac

SEQ ID NO: 125 - RNA, 23 nt, Homo sapiens
  source 1..23: mol_type = mRNA
gatcactgcagataagcaataca

SEQ ID NO: 126 - RNA, 23 nt, Homo sapiens
  source 1..23: mol_type = mRNA
aagcagatcactgcagataagca

SEQ ID NO: 127 - RNA, 23 nt, Homo sapiens
  source 1..23: mol_type = mRNA
agcagatcactgcagataagcaa

SEQ ID NO: 128 - RNA, 23 nt, Homo sapiens
  source 1..23: mol_type = mRNA
ccagcaagcagatcactgcagat

SEQ ID NO: 129 - RNA, 23 nt, Homo sapiens
  source 1..23: mol_type = mRNA
cagatcactgcagataagcaata

SEQ ID NO: 130 - RNA, 23 nt, Homo sapiens
  source 1..23: mol_type = mRNA
tgataaataacaaatttggagaa

SEQ ID NO: 131 - RNA, 23 nt, Homo sapiens
  source 1..23: mol_type = mRNA
actcctgataaataacaaatttg

SEQ ID NO: 132 - RNA, 23 nt, Homo sapiens
  source 1..23: mol_type = mRNA
ctgaaagggaattccgaggcctc

SEQ ID NO: 133 - RNA, 23 nt, Homo sapiens
  source 1..23: mol_type = mRNA
atgttgtattatataacatatct

SEQ ID NO: 134 - RNA, 23 nt, Homo sapiens
  source 1..23: mol_type = mRNA
aattccgaggcctcggtgactgc

SEQ ID NO: 135 - RNA, 23 nt, Homo sapiens
  source 1..23: mol_type = mRNA
tgaaagggaattccgaggcctcg

SEQ ID NO: 136 - RNA, 23 nt, Homo sapiens
  source 1..23: mol_type = mRNA
gttgtattatataacatatcttg

SEQ ID NO: 137 - RNA, 23 nt, Homo sapiens
  source 1..23: mol_type = mRNA
ggaattccgaggcctcggtgact

SEQ ID NO: 138 - RNA, 23 nt, Homo sapiens
  source 1..23: mol_type = mRNA
aagggaattccgaggcctcggtg

SEQ ID NO: 139 - RNA, 23 nt, Homo sapiens
  source 1..23: mol_type = mRNA
ggagctgaaagggaattccgagg

SEQ ID NO: 140 - RNA, 23 nt, Homo sapiens
  source 1..23: mol_type = mRNA
ctggagctgaaagggaattccga

SEQ ID NO: 141 - RNA, 23 nt, Homo sapiens
  source 1..23: mol_type = mRNA
agctgaaagggaattccgaggcc

SEQ ID NO: 142 - RNA, 23 nt, Homo sapiens
  source 1..23: mol_type = mRNA
tggagctgaaagggaattccgag

SEQ ID NO: 143 - RNA, 23 nt, Homo sapiens
  source 1..23: mol_type = mRNA
gagctgaaagggaattccgaggc

SEQ ID NO: 144 - RNA, 23 nt, Homo sapiens
  source 1..23: mol_type = mRNA
aggcatgttgtattatataacat

SEQ ID NO: 145 - RNA, 23 nt, Homo sapiens
  source 1..23: mol_type = mRNA
tgttgtattatataacatatctt

SEQ ID NO: 146 - RNA, 23 nt, Homo sapiens
  source 1..23: mol_type = mRNA
ttgtattatataacatatcttga

SEQ ID NO: 147 - RNA, 23 nt, Homo sapiens
  source 1..23: mol_type = mRNA
caggcatgttgtattatataaca

SEQ ID NO: 148 - RNA, 23 nt, Homo sapiens
  source 1..23: mol_type = mRNA
gaaagggaattccgaggcctcgg

SEQ ID NO: 149 - RNA, 23 nt, Homo sapiens
  source 1..23: mol_type = mRNA
gggaattccgaggcctcggtgac

SEQ ID NO: 150 - RNA, 23 nt, Homo sapiens
  source 1..23: mol_type = mRNA
aaagggaattccgaggcctcggt

SEQ ID NO: 151 - RNA, 23 nt, Homo sapiens
  source 1..23: mol_type = mRNA
agggaattccgaggcctcggtga

SEQ ID NO: 152 - RNA, 23 nt, Homo sapiens
  source 1..23: mol_type = mRNA
gtgcttgtcttgtatgatgaaat

SEQ ID NO: 153 - RNA, 23 nt, Homo sapiens
  source 1..23: mol_type = mRNA
cttcgccttcaaagataaataca

SEQ ID NO: 154 - RNA, 23 nt, Homo sapiens
  source 1..23: mol_type = mRNA
ctgcctggttaagatctacaaat

SEQ ID NO: 155 - RNA, 23 nt, Homo sapiens
  source 1..23: mol_type = mRNA
tatctatgacactgcaaagggaa

SEQ ID NO: 156 - RNA, 23 nt, Homo sapiens
  source 1..23: mol_type = mRNA
cttttgtgcttgtcttgtatgat

SEQ ID NO: 157 - RNA, 23 nt, Homo sapiens
  source 1..23: mol_type = mRNA
ggtgactgcctggttaagatcta

SEQ ID NO: 158 - RNA, 23 nt, Homo sapiens
  source 1..23: mol_type = mRNA
atgacactgcaaagggaatgctt

SEQ ID NO: 159 - RNA, 23 nt, Homo sapiens
  source 1..23: mol_type = mRNA
ttcggtatctatgacactgcaaa

SEQ ID NO: 160 - RNA, 23 nt, Homo sapiens
  source 1..23: mol_type = mRNA
tattcatctgaccagttttctct

SEQ ID NO: 161 - RNA, 23 nt, Homo sapiens
  source 1..23: mol_type = mRNA
acttcggtatctatgacactgca

SEQ ID NO: 162 - RNA, 23 nt, Homo sapiens
  source 1..23: mol_type = mRNA
ctggttaagatctacaaatctga

SEQ ID NO: 163 - RNA, 23 nt, Homo sapiens
  source 1..23: mol_type = mRNA
gtatctatgacactgcaaaggga

SEQ ID NO: 164 - RNA, 23 nt, Homo sapiens
  source 1..23: mol_type = mRNA
caagggtgcatggtccaatgttc

SEQ ID NO: 165 - RNA, 23 nt, Homo sapiens
  source 1..23: mol_type = mRNA
agatctacaaatctgatgggatt

SEQ ID NO: 166 - RNA, 23 nt, Homo sapiens
  source 1..23: mol_type = mRNA
tacttcggtatctatgacactgc

SEQ ID NO: 167 - RNA, 23 nt, Homo sapiens
  source 1..23: mol_type = mRNA
catgggtggtgcttttgtgcttg

SEQ ID NO: 168 - RNA, 23 nt, Homo sapiens
  source 1..23: mol_type = mRNA
ggtattatcatctaccgagccgc

SEQ ID NO: 169 - RNA, 23 nt, Homo sapiens
  source 1..23: mol_type = mRNA
gcgtggtccgtattcccaaggag

SEQ ID NO: 170 - RNA, 23 nt, Homo sapiens
  source 1..23: mol_type = mRNA
atctatgacactgcaaagggaat

SEQ ID NO: 171 - RNA, 23 nt, Homo sapiens
  source 1..23: mol_type = mRNA
tgcttttgtgcttgtcttgtatg

SEQ ID NO: 172 - RNA, 23 nt, Homo sapiens
  source 1..23: mol_type = mRNA
tgtaccaaggctttaacgtgtct

SEQ ID NO: 173 - RNA, 23 nt, Homo sapiens
  source 1..23: mol_type = mRNA
gggtgcatggtccaatgttctca

SEQ ID NO: 174 - RNA, 23 nt, Homo sapiens
  source 1..23: mol_type = mRNA
cgccttcaaagataaatacaagc

SEQ ID NO: 175 - RNA, 23 nt, Homo sapiens
  source 1..23: mol_type = mRNA
cagggtattatcatctaccgagc

SEQ ID NO: 176 - RNA, 23 nt, Homo sapiens
  source 1..23: mol_type = mRNA
cctacttcggtatctatgacact

SEQ ID NO: 177 - RNA, 23 nt, Homo sapiens
  source 1..23: mol_type = mRNA
tggttaagatctacaaatctgat

SEQ ID NO: 178 - RNA, 23 nt, Homo sapiens
  source 1..23: mol_type = mRNA
tgtgcagggtattatcatctacc

SEQ ID NO: 179 - RNA, 23 nt, Homo sapiens
  source 1..23: mol_type = mRNA
aatctgatgggattaagggcctg

SEQ ID NO: 180 - RNA, 23 nt, Homo sapiens
  source 1..23: mol_type = mRNA
gtctgtgcagggtattatcatct

SEQ ID NO: 181 - RNA, 23 nt, Homo sapiens
  source 1..23: mol_type = mRNA
tctgatgggattaagggcctgta

SEQ ID NO: 182 - RNA, 23 nt, Homo sapiens
  source 1..23: mol_type = mRNA
taccaaggctttaacgtgtctgt

SEQ ID NO: 183 - RNA, 23 nt, Homo sapiens
  source 1..23: mol_type = mRNA
aatattcatctgaccagttttct

SEQ ID NO: 184 - RNA, 23 nt, Homo sapiens
  source 1..23: mol_type = mRNA
tgactgcctggttaagatctaca

SEQ ID NO: 185 - RNA, 23 nt, Homo sapiens
  source 1..23: mol_type = mRNA
gggttgacttcctatccatttga

SEQ ID NO: 186 - RNA, 23 nt, Homo sapiens
  source 1..23: mol_type = mRNA
tctatgacactgcaaagggaatg

SEQ ID NO: 187 - RNA, 23 nt, Homo sapiens
  source 1..23: mol_type = mRNA
ggttaagatctacaaatctgatg

SEQ ID NO: 188 - RNA, 23 nt, Homo sapiens
  source 1..23: mol_type = mRNA
gcagggtattatcatctaccgag

SEQ ID NO: 189 - RNA, 23 nt, Homo sapiens
  source 1..23: mol_type = mRNA
actgcctggttaagatctacaaa

SEQ ID NO: 190 - RNA, 23 nt, Homo sapiens
  source 1..23: mol_type = mRNA
atctgatgggattaagggcctgt

SEQ ID NO: 191 - RNA, 23 nt, Homo sapiens
  source 1..23: mol_type = mRNA
tcggtatctatgacactgcaaag

SEQ ID NO: 192 - RNA, 23 nt, Homo sapiens
  source 1..23: mol_type = mRNA
gtacccgtctagcagctgatgtg

SEQ ID NO: 193 - RNA, 23 nt, Homo sapiens
  source 1..23: mol_type = mRNA
ggtatctatgacactgcaaaggg

SEQ ID NO: 194 - RNA, 23 nt, Homo sapiens
  source 1..23: mol_type = mRNA
agctgatgtgggtaaagctggag

SEQ ID NO: 195 - RNA, 23 nt, Homo sapiens
  source 1..23: mol_type = mRNA
cgtctagcagctgatgtgggtaa

SEQ ID NO: 196 - RNA, 23 nt, Homo sapiens
  source 1..23: mol_type = mRNA
aagggcctgtaccaaggctttaa

SEQ ID NO: 197 - RNA, 23 nt, Homo sapiens
  source 1..23: mol_type = mRNA
tgcccgtacccgtctagcagctg

SEQ ID NO: 198 - RNA, 23 nt, Homo sapiens
  source 1..23: mol_type = mRNA
agcagctgatgtgggtaaagctg

SEQ ID NO: 199 - RNA, 23 nt, Homo sapiens
  source 1..23: mol_type = mRNA
gcccgtacccgtctagcagctga

SEQ ID NO: 200 - RNA, 23 nt, Homo sapiens
  source 1..23: mol_type = mRNA
cagctgatgtgggtaaagctgga

SEQ ID NO: 201 - RNA, 23 nt, Homo sapiens
  source 1..23: mol_type = mRNA
agggtattatcatctaccgagcc

SEQ ID NO: 202 - RNA, 23 nt, Homo sapiens
  source 1..23: mol_type = mRNA
tattatcatctaccgagccgcct

SEQ ID NO: 203 - RNA, 23 nt, Homo sapiens
  source 1..23: mol_type = mRNA
ccgtacccgtctagcagctgatg

SEQ ID NO: 204 - RNA, 23 nt, Homo sapiens
  source 1..23: mol_type = mRNA
ctgatgggattaagggcctgtac

SEQ ID NO: 205 - RNA, 23 nt, Homo sapiens
  source 1..23: mol_type = mRNA
gtgtctgtgcagggtattatcat

SEQ ID NO: 206 - RNA, 23 nt, Homo sapiens
  source 1..23: mol_type = mRNA
ctgcgtggtccgtattcccaagg

SEQ ID NO: 207 - RNA, 23 nt, Homo sapiens
  source 1..23: mol_type = mRNA
tgcgtggtccgtattcccaagga

SEQ ID NO: 208 - RNA, 23 nt, Homo sapiens
  source 1..23: mol_type = mRNA
cctggttaagatctacaaatctg

SEQ ID NO: 209 - RNA, 23 nt, Homo sapiens
  source 1..23: mol_type = mRNA
gtatgatgaaatcaagaagtaca

SEQ ID NO: 210 - RNA, 23 nt, Homo sapiens
  source 1..23: mol_type = mRNA
aagatctacaaatctgatgggat

SEQ ID NO: 211 - RNA, 23 nt, Homo sapiens
  source 1..23: mol_type = mRNA
ctgtgcagggtattatcatctac

SEQ ID NO: 212 - RNA, 23 nt, Homo sapiens
  source 1..23: mol_type = mRNA
ctgtaccaaggctttaacgtgtc

SEQ ID NO: 213 - RNA, 23 nt, Homo sapiens
  source 1..23: mol_type = mRNA
tagcagctgatgtgggtaaagct

SEQ ID NO: 214 - RNA, 23 nt, Homo sapiens
  source 1..23: mol_type = mRNA
gcatgggtggtgcttttgtgctt

SEQ ID NO: 215 - RNA, 23 nt, Homo sapiens
  source 1..23: mol_type = mRNA
ctcggtgactgcctggttaagat

SEQ ID NO: 216 - RNA, 23 nt, Homo sapiens
  source 1..23: mol_type = mRNA
gtctagcagctgatgtgggtaaa

SEQ ID NO: 217 - RNA, 23 nt, Homo sapiens
  source 1..23: mol_type = mRNA
tctacaaatctgatgggattaag

SEQ ID NO: 218 - RNA, 23 nt, Homo sapiens
  source 1..23: mol_type = mRNA
ctacttcggtatctatgacactg

SEQ ID NO: 219 - RNA, 23 nt, Homo sapiens
  source 1..23: mol_type = mRNA
gcagctgatgtgggtaaagctgg

SEQ ID NO: 220 - RNA, 23 nt, Homo sapiens
  source 1..23: mol_type = mRNA
cccgtacccgtctagcagctgat

SEQ ID NO: 221 - RNA, 23 nt, Homo sapiens
  source 1..23: mol_type = mRNA
tgtctgtgcagggtattatcatc

SEQ ID NO: 222 - RNA, 23 nt, Homo sapiens
  source 1..23: mol_type = mRNA
tgtgcttgtcttgtatgatgaaa

SEQ ID NO: 223 - RNA, 23 nt, Homo sapiens
  source 1..23: mol_type = mRNA
gtaccaaggctttaacgtgtctg

SEQ ID NO: 224 - RNA, 23 nt, Homo sapiens
  source 1..23: mol_type = mRNA
aagggtgcatggtccaatgttct

SEQ ID NO: 225 - RNA, 23 nt, Homo sapiens
  source 1..23: mol_type = mRNA
gtgactgcctggttaagatctac

SEQ ID NO: 226 - RNA, 23 nt, Homo sapiens
  source 1..23: mol_type = mRNA
ctgatgtgggtaaagctggagct

SEQ ID NO: 227 - RNA, 23 nt, Homo sapiens
  source 1..23: mol_type = mRNA
cgtggtccgtattcccaaggagc

SEQ ID NO: 228 - RNA, 23 nt, Homo sapiens
  source 1..23: mol_type = mRNA
tgacactgcaaagggaatgcttc

SEQ ID NO: 229 - RNA, 23 nt, Homo sapiens
  source 1..23: mol_type = mRNA
gggattaagggcctgtaccaagg

SEQ ID NO: 230 - RNA, 23 nt, Homo sapiens
  source 1..23: mol_type = mRNA
tctgtgcagggtattatcatcta

SEQ ID NO: 231 - RNA, 23 nt, Homo sapiens
  source 1..23: mol_type = mRNA
ttaacgtgtctgtgcagggtatt

SEQ ID NO: 232 - RNA, 23 nt, Homo sapiens
  source 1..23: mol_type = mRNA
agggcctgtaccaaggctttaac

SEQ ID NO: 233 - RNA, 23 nt, Homo sapiens
  source 1..23: mol_type = mRNA
tatgacactgcaaagggaatgct

SEQ ID NO: 234 - RNA, 23 nt, Homo sapiens
  source 1..23: mol_type = mRNA
cctcggtgactgcctggttaaga

SEQ ID NO: 235 - RNA, 23 nt, Homo sapiens
  source 1..23: mol_type = mRNA
gtgcttttgtgcttgtcttgtat

SEQ ID NO: 236 - RNA, 23 nt, Homo sapiens
  source 1..23: mol_type = mRNA
tgggtggtgcttttgtgcttgtc

SEQ ID NO: 237 - RNA, 23 nt, Homo sapiens
  source 1..23: mol_type = mRNA
cccgtctagcagctgatgtgggt

SEQ ID NO: 238 - RNA, 23 nt, Homo sapiens
  source 1..23: mol_type = mRNA
taagggcctgtaccaaggcttta

SEQ ID NO: 239 - RNA, 23 nt, Homo sapiens
  source 1..23: mol_type = mRNA
ttgtgcttgtcttgtatgatgaa

SEQ ID NO: 240 - RNA, 23 nt, Homo sapiens
  source 1..23: mol_type = mRNA
acaaatctgatgggattaagggc

SEQ ID NO: 241 - RNA, 23 nt, Homo sapiens
  source 1..23: mol_type = mRNA
atctacaaatctgatgggattaa

SEQ ID NO: 242 - RNA, 23 nt, Homo sapiens
  source 1..23: mol_type = mRNA
tgcagggtattatcatctaccga

SEQ ID NO: 243 - RNA, 23 nt, Homo sapiens
  source 1..23: mol_type = mRNA
gcctgtaccaaggctttaacgtg

SEQ ID NO: 244 - RNA, 23 nt, Homo sapiens
  source 1..23: mol_type = mRNA
taagatctacaaatctgatggga

SEQ ID NO: 245 - RNA, 23 nt, Homo sapiens
  source 1..23: mol_type = mRNA
gcttttgtgcttgtcttgtatga

SEQ ID NO: 246 - RNA, 23 nt, Homo sapiens
  source 1..23: mol_type = mRNA
ctacaaatctgatgggattaagg

SEQ ID NO: 247 - RNA, 23 nt, Homo sapiens
  source 1..23: mol_type = mRNA
ttcaagggtgcatggtccaatgt

SEQ ID NO: 248 - RNA, 23 nt, Homo sapiens
  source 1..23: mol_type = mRNA
tgggattaagggcctgtaccaag

SEQ ID NO: 249 - RNA, 23 nt, Homo sapiens
  source 1..23: mol_type = mRNA
cttcggtatctatgacactgcaa

SEQ ID NO: 250 - RNA, 23 nt, Homo sapiens
  source 1..23: mol_type = mRNA
accaaggctttaacgtgtctgtg

SEQ ID NO: 251 - RNA, 23 nt, Homo sapiens
  source 1..23: mol_type = mRNA
ggcatgggtggtgcttttgtgct

SEQ ID NO: 252 - RNA, 23 nt, Homo sapiens
  source 1..23: mol_type = mRNA
gttaagatctacaaatctgatgg

SEQ ID NO: 253 - RNA, 23 nt, Homo sapiens
  source 1..23: mol_type = mRNA
tacccgtctagcagctgatgtgg

SEQ ID NO: 254 - RNA, 23 nt, Homo sapiens
  source 1..23: mol_type = mRNA
ctatgacactgcaaagggaatgc

SEQ ID NO: 255 - RNA, 23 nt, Homo sapiens
  source 1..23: mol_type = mRNA
tctagcagctgatgtgggtaaag

SEQ ID NO: 256 - RNA, 23 nt, Homo sapiens
  source 1..23: mol_type = mRNA
ctgcaaagggaatgcttccggat

SEQ ID NO: 257 - RNA, 23 nt, Homo sapiens
  source 1..23: mol_type = mRNA
ttgcccgtacccgtctagcagct

SEQ ID NO: 258 - RNA, 23 nt, Homo sapiens
  source 1..23: mol_type = mRNA
gggtattatcatctaccgagccg

SEQ ID NO: 259 - RNA, 23 nt, Homo sapiens
  source 1..23: mol_type = mRNA
ccctcttgattttgcccgtaccc

SEQ ID NO: 260 - RNA, 23 nt, Homo sapiens
  source 1..23: mol_type = mRNA
cgtacccgtctagcagctgatgt

SEQ ID NO: 261 - RNA, 23 nt, Homo sapiens
  source 1..23: mol_type = mRNA
tacaaatctgatgggattaaggg

SEQ ID NO: 262 - RNA, 23 nt, Homo sapiens
  source 1..23: mol_type = mRNA
gtgtaccctcttgattttgcccg

SEQ ID NO: 263 - RNA, 23 nt, Homo sapiens
  source 1..23: mol_type = mRNA
ggcctgtaccaaggctttaacgt

SEQ ID NO: 264 - RNA, 23 nt, Homo sapiens
  source 1..23: mol_type = mRNA
gatgggattaagggcctgtacca

SEQ ID NO: 265 - RNA, 23 nt, Homo sapiens
  source 1..23: mol_type = mRNA
gtattatcatctaccgagccgcc

SEQ ID NO: 266 - RNA, 23 nt, Homo sapiens
  source 1..23: mol_type = mRNA
gggcctgtaccaaggctttaacg

SEQ ID NO: 267 - RNA, 23 nt, Homo sapiens
  source 1..23: mol_type = mRNA
tgatgggattaagggcctgtacc

SEQ ID NO: 268 - RNA, 23 nt, Homo sapiens
  source 1..23: mol_type = mRNA
taacgtgtctgtgcagggtatta

SEQ ID NO: 269 - RNA, 23 nt, Homo sapiens
  source 1..23: mol_type = mRNA
aaggcattatagactgcgtggtc

SEQ ID NO: 270 - RNA, 23 nt, Homo sapiens
  source 1..23: mol_type = mRNA
acttccccacccaggctcttaac

SEQ ID NO: 271 - RNA, 23 nt, Homo sapiens
  source 1..23: mol_type = mRNA
caatgtcatcagatacttcccca

SEQ ID NO: 272 - RNA, 23 nt, Homo sapiens
  source 1..23: mol_type = mRNA
atgtcatcagatacttccccacc

SEQ ID NO: 273 - RNA, 23 nt, Homo sapiens
  source 1..23: mol_type = mRNA
aatgtcatcagatacttccccac

SEQ ID NO: 274 - RNA, 23 nt, Homo sapiens
  source 1..23: mol_type = mRNA
ccaatgtcatcagatacttcccc

SEQ ID NO: 275 - RNA, 23 nt, Homo sapiens
  source 1..23: mol_type = mRNA
tacttccccacccaggctcttaa

SEQ ID NO: 276 - RNA, 23 nt, Homo sapiens
  source 1..23: mol_type = mRNA
atctaccgagccgcctacttcgg

SEQ ID NO: 277 - RNA, 23 nt, synthetic construct
  source 1..23: mol_type = other RNA
cccattttcaaccagtaaatagt

SEQ ID NO: 278 - RNA, 23 nt, synthetic construct
  source 1..23: mol_type = other RNA
acgcagtctataatgcctttgta

SEQ ID NO: 279 - RNA, 23 nt, synthetic construct
  source 1..23: mol_type = other RNA
gtgtacttcttgatttcatcata

SEQ ID NO: 280 - RNA, 23 nt, synthetic construct
  source 1..23: mol_type = other RNA
atacaattgagtcccatcatcat

SEQ ID NO: 281 - RNA, 23 nt, synthetic construct
  source 1..23: mol_type = other RNA
ggaccacgcagtctataatgcct

SEQ ID NO: 282 - RNA, 23 nt, synthetic construct
  source 1..23: mol_type = other RNA
ttgttatttatcaggagtgactg

SEQ ID NO: 283 - RNA, 23 nt, synthetic construct
  source 1..23: mol_type = other RNA
cagtctataatgcctttgtattg

SEQ ID NO: 284 - RNA, 23 nt, synthetic construct
  source 1..23: mol_type = other RNA
atagataccgaagtaggcggctc

SEQ ID NO: 285 - RNA, 23 nt, synthetic construct
  source 1..23: mol_type = other RNA
tagataccgaagtaggcggctcg

SEQ ID NO: 286 - RNA, 23 nt, synthetic construct
  source 1..23: mol_type = other RNA
ggaatacggaccacgcagtctat

SEQ ID NO: 287 - RNA, 23 nt, synthetic construct
  source 1..23: mol_type = other RNA
cagctgatgacgatgtgagtgtt

SEQ ID NO: 288 - RNA, 23 nt, synthetic construct
  source 1..23: mol_type = other RNA
atttatctttgaaggcgaagtta

SEQ ID NO: 289 - RNA, 23 nt, synthetic construct
  source 1..23: mol_type = other RNA
gtgtcatagataccgaagtaggc

SEQ ID NO: 290 - RNA, 23 nt, synthetic construct
  source 1..23: mol_type = other RNA
ttcccattttcaaccagtaaata

SEQ ID NO: 291 - RNA, 23 nt, synthetic construct
  source 1..23: mol_type = other RNA
gctgctagacgggtacgggcaaa

SEQ ID NO: 292 - RNA, 23 nt, synthetic construct
  source 1..23: mol_type = other RNA
cagttcctttgcgccctgactgc

SEQ ID NO: 293 - RNA, 23 nt, synthetic construct
  source 1..23: mol_type = other RNA
cttcccattttcaaccagtaaat

SEQ ID NO: 294 - RNA, 23 nt, synthetic construct
  source 1..23: mol_type = other RNA
agataccgaagtaggcggctcgg

SEQ ID NO: 295 - RNA, 23 nt, synthetic construct
  source 1..23: mol_type = other RNA
ttaaccaggcagtcaccgaggcc

SEQ ID NO: 296 - RNA, 23 nt, synthetic construct
  source 1..23: mol_type = other RNA
atcatccagctgatgacgatgtg

SEQ ID NO: 297 - RNA, 23 nt, synthetic construct
  source 1..23: mol_type = other RNA
atttatcaggagtgactgaaata

SEQ ID NO: 298 - RNA, 23 nt, synthetic construct
  source 1..23: mol_type = other RNA
gacagtctgtgcgatcatccagc

SEQ ID NO: 299 - RNA, 23 nt, synthetic construct
  source 1..23: mol_type = other RNA
tctataatgcctttgtattgctt

SEQ ID NO: 300 - RNA, 23 nt, synthetic construct
  source 1..23: mol_type = other RNA
taaccaggcagtcaccgaggcct

SEQ ID NO: 301 - RNA, 23 nt, synthetic construct
  source 1..23: mol_type = other RNA
ccctgcacagacacgttaaagcc

SEQ ID NO: 302 - RNA, 23 nt, synthetic construct
  source 1..23: mol_type = other RNA
cacgcagtctataatgcctttgt

SEQ ID NO: 303 - RNA, 23 nt, synthetic construct
  source 1..23: mol_type = other RNA
taatacaacatgcctgttcacag

SEQ ID NO: 304 - RNA, 23 nt, synthetic construct
  source 1..23: mol_type = other RNA
ttaagagaaaactggtcagatga

SEQ ID NO: 305 - RNA, 23 nt, synthetic construct
  source 1..23: mol_type = other RNA
tgcacagacacgttaaagccttg

SEQ ID NO: 306 - RNA, 23 nt, synthetic construct
  source 1..23: mol_type = other RNA
gttcctttgcgccctgactgcat

SEQ ID NO: 307 - RNA, 23 nt, synthetic construct
  source 1..23: mol_type = other RNA
gtgacagtctgtgcgatcatcca

SEQ ID NO: 308 - RNA, 23 nt, synthetic construct
  source 1..23: mol_type = other RNA
accacgcagtctataatgccttt

SEQ ID NO: 309 - RNA, 23 nt, synthetic construct
  source 1..23: mol_type = other RNA
cagtgacagtctgtgcgatcatc

SEQ ID NO: 310 - RNA, 23 nt, synthetic construct
  source 1..23: mol_type = other RNA
ttgggaatacggaccacgcagtc

SEQ ID NO: 311 - RNA, 23 nt, synthetic construct
  source 1..23: mol_type = other RNA
gtctataatgcctttgtattgct

SEQ ID NO: 312 - RNA, 23 nt, synthetic construct
  source 1..23: mol_type = other RNA
tgtgcgatcatccagctgatgac

SEQ ID NO: 313 - RNA, 23 nt, synthetic construct
  source 1..23: mol_type = other RNA
acggaccacgcagtctataatgc

SEQ ID NO: 314 - RNA, 23 nt, synthetic construct
  source 1..23: mol_type = other RNA
tgctagacgggtacgggcaaaat

SEQ ID NO: 315 - RNA, 23 nt, synthetic construct
  source 1..23: mol_type = other RNA
tcatccagctgatgacgatgtga

SEQ ID NO: 316 - RNA, 23 nt, synthetic construct
  source 1..23: mol_type = other RNA
cgggtacgggcaaaatcaagagg

SEQ ID NO: 317 - RNA, 23 nt, synthetic construct
  source 1..23: mol_type = other RNA
aatacggaccacgcagtctataa

SEQ ID NO: 318 - RNA, 23 nt, synthetic construct
  source 1..23: mol_type = other RNA
tcatagataccgaagtaggcggc

SEQ ID NO: 319 - RNA, 23 nt, synthetic construct
  source 1..23: mol_type = other RNA
gggaatacggaccacgcagtcta

SEQ ID NO: 320 - RNA, 23 nt, synthetic construct
  source 1..23: mol_type = other RNA
gtgcgatcatccagctgatgacg

SEQ ID NO: 321 - RNA, 23 nt, synthetic construct
  source 1..23: mol_type = other RNA
tacggaccacgcagtctataatg

SEQ ID NO: 322 - RNA, 23 nt, synthetic construct
  source 1..23: mol_type = other RNA
tgtcatagataccgaagtaggcg

SEQ ID NO: 323 - RNA, 23 nt, synthetic construct
  source 1..23: mol_type = other RNA
tatcaggagtgactgaaataaaa

SEQ ID NO: 324 - RNA, 23 nt, synthetic construct
  source 1..23: mol_type = other RNA
tgcgatcatccagctgatgacga

SEQ ID NO: 325 - RNA, 23 nt, synthetic construct
  source 1..23: mol_type = other RNA
ctagacgggtacgggcaaaatca

SEQ ID NO: 326 - RNA, 23 nt, synthetic construct
  source 1..23: mol_type = other RNA
gatccggaagcattccctttgca

SEQ ID NO: 327 - RNA, 23 nt, synthetic construct
  source 1..23: mol_type = other RNA
gcacagacacgttaaagccttgg

SEQ ID NO: 328 - RNA, 23 nt, synthetic construct
  source 1..23: mol_type = other RNA
ccacgcagtctataatgcctttg

SEQ ID NO: 329 - RNA, 23 nt, synthetic construct
  source 1..23: mol_type = other RNA
gacgggtacgggcaaaatcaaga

SEQ ID NO: 330 - RNA, 23 nt, synthetic construct
  source 1..23: mol_type = other RNA
gataccgaagtaggcggctcggt

SEQ ID NO: 331 - RNA, 23 nt, synthetic construct
  source 1..23: mol_type = other RNA
gtaggcggctcggtagatgataa

SEQ ID NO: 332 - RNA, 23 nt, synthetic construct
  source 1..23: mol_type = other RNA
agacgggtacgggcaaaatcaag

SEQ ID NO: 333 - RNA, 23 nt, synthetic construct
  source 1..23: mol_type = other RNA
taggcggctcggtagatgataat

SEQ ID NO: 334 - RNA, 23 nt, synthetic construct
  source 1..23: mol_type = other RNA
aagtaggcggctcggtagatgat

SEQ ID NO: 335 - RNA, 23 nt, synthetic construct
  source 1..23: mol_type = other RNA
ctttgaaggcgaagttaagagcc

SEQ ID NO: 336 - RNA, 23 nt, synthetic construct
  source 1..23: mol_type = other RNA
cgaagttaagagcctgggtgggg

SEQ ID NO: 337 - RNA, 23 nt, synthetic construct
  source 1..23: mol_type = other RNA
ccctgctccttgggaatacggac

SEQ ID NO: 338 - RNA, 23 nt, synthetic construct
  source 1..23: mol_type = other RNA
gaaggacagaactccctgctcct

SEQ ID NO: 339 - RNA, 23 nt, synthetic construct
  source 1..23: mol_type = other RNA
agaactccctgctccttgggaat

SEQ ID NO: 340 - RNA, 23 nt, synthetic construct
  source 1..23: mol_type = other RNA
cctgctccttgggaatacggacc

SEQ ID NO: 341 - RNA, 23 nt, synthetic construct
  source 1..23: mol_type = other RNA
cagaaggacagaactccctgctc

SEQ ID NO: 342 - RNA, 23 nt, synthetic construct
  source 1..23: mol_type = other RNA
ctgctccttgggaatacggacca

SEQ ID NO: 343 - RNA, 23 nt, synthetic construct
  source 1..23: mol_type = other RNA
agaaggacagaactccctgctcc

SEQ ID NO: 344 - RNA, 23 nt, synthetic construct
  source 1..23: mol_type = other RNA
aaggacagaactccctgctcctt

SEQ ID NO: 345 - RNA, 23 nt, synthetic construct
  source 1..23: mol_type = other RNA
gaactccctgctccttgggaata

SEQ ID NO: 346 - RNA, 23 nt, synthetic construct
  source 1..23: mol_type = other RNA
aggacagaactccctgctccttg

SEQ ID NO: 347 - RNA, 23 nt, synthetic construct
  source 1..23: mol_type = other RNA
gaagttaagagcctgggtgggga

SEQ ID NO: 348 - RNA, 23 nt, synthetic construct
  source 1..23: mol_type = other RNA
tctttgaaggcgaagttaagagc

SEQ ID NO: 349 - RNA, 23 nt, synthetic construct
  source 1..23: mol_type = other RNA
tatttatcaggagtgactgaaat

SEQ ID NO: 350 - RNA, 23 nt, synthetic construct
  source 1..23: mol_type = other RNA
gttatttatcaggagtgactgaa

SEQ ID NO: 351 - RNA, 23 nt, synthetic construct
  source 1..23: mol_type = other RNA
ttatttatcaggagtgactgaaa

SEQ ID NO: 352 - RNA, 23 nt, synthetic construct
  source 1..23: mol_type = other RNA
aaatacaattgagtcccatcatc

SEQ ID NO: 353 - RNA, 23 nt, synthetic construct
  source 1..23: mol_type = other RNA
aaaatacaattgagtcccatcat

SEQ ID NO: 354 - RNA, 23 nt, synthetic construct
  source 1..23: mol_type = other RNA
atttgttatttatcaggagtgac

SEQ ID NO: 355 - RNA, 23 nt, synthetic construct
  source 1..23: mol_type = other RNA
gagaaaactggtcagatgaatat

SEQ ID NO: 356 - RNA, 23 nt, synthetic construct
  source 1..23: mol_type = other RNA
atataatacaacatgcctgttca

SEQ ID NO: 357 - RNA, 23 nt, synthetic construct
  source 1..23: mol_type = other RNA
tgggatccggaagcattcccttt

SEQ ID NO: 358 - RNA, 23 nt, synthetic construct
  source 1..23: mol_type = other RNA
ttgggatccggaagcattccctt

SEQ ID NO: 359 - RNA, 23 nt, synthetic construct
  source 1..23: mol_type = other RNA
caggcagtcaccgaggcctcgga

SEQ ID NO: 360 - RNA, 23 nt, synthetic construct
  source 1..23: mol_type = other RNA
tatataatacaacatgcctgttc

SEQ ID NO: 361 - RNA, 23 nt, synthetic construct
  source 1..23: mol_type = other RNA
agtctataatgcctttgtattgc

SEQ ID NO: 362 - RNA, 23 nt, synthetic construct
  source 1..23: mol_type = other RNA
tttatcaggagtgactgaaataa

SEQ ID NO: 363 - RNA, 23 nt, synthetic construct
  source 1..23: mol_type = other RNA
aatacaattgagtcccatcatca

SEQ ID NO: 364 - RNA, 23 nt, synthetic construct
  source 1..23: mol_type = other RNA
ctttaagagaaaactggtcagat

SEQ ID NO: 365 - RNA, 23 nt, synthetic construct
  source 1..23: mol_type = other RNA
gctttaagagaaaactggtcaga

SEQ ID NO: 366 - RNA, 23 nt, synthetic construct
  source 1..23: mol_type = other RNA
aatgcctttgtattgcttatctg

SEQ ID NO: 367 - RNA, 23 nt, synthetic construct
  source 1..23: mol_type = other RNA
taatgcctttgtattgcttatct

SEQ ID NO: 368 - RNA, 23 nt, synthetic construct
  source 1..23: mol_type = other RNA
taccctgcacagacacgttaaag

SEQ ID NO: 369 - RNA, 23 nt, synthetic construct
  source 1..23: mol_type = other RNA
ataccctgcacagacacgttaaa

SEQ ID NO: 370 - RNA, 23 nt, synthetic construct
  source 1..23: mol_type = other RNA
atccagctgatgacgatgtgagt

SEQ ID NO: 371 - RNA, 23 nt, synthetic construct
  source 1..23: mol_type = other RNA
tacaattgagtcccatcatcatc

SEQ ID NO: 372 - RNA, 23 nt, synthetic construct
  source 1..23: mol_type = other RNA
tgggaatacggaccacgcagtct

SEQ ID NO: 373 - RNA, 23 nt, synthetic construct
  source 1..23: mol_type = other RNA
tataatacaacatgcctgttcac

SEQ ID NO: 374 - RNA, 23 nt, synthetic construct
  source 1..23: mol_type = other RNA
ttatcaggagtgactgaaataaa

SEQ ID NO: 375 - RNA, 23 nt, synthetic construct
  source 1..23: mol_type = other RNA
ataatgcctttgtattgcttatc

SEQ ID NO: 376 - RNA, 23 nt, synthetic construct
  source 1..23: mol_type = other RNA
ccagctgatgacgatgtgagtgt

SEQ ID NO: 377 - RNA, 23 nt, synthetic construct
  source 1..23: mol_type = other RNA
catagataccgaagtaggcggct

SEQ ID NO: 378 - RNA, 23 nt, synthetic construct
  source 1..23: mol_type = other RNA
catccagctgatgacgatgtgag

SEQ ID NO: 379 - RNA, 23 nt, synthetic construct
  source 1..23: mol_type = other RNA
gtcatagataccgaagtaggcgg

SEQ ID NO: 380 - RNA, 23 nt, synthetic construct
  source 1..23: mol_type = other RNA
accctgcacagacacgttaaagc

SEQ ID NO: 381 - RNA, 23 nt, synthetic construct
  source 1..23: mol_type = other RNA
tgcatcatcatgcggcggcgaac

SEQ ID NO: 382 - RNA, 23 nt, synthetic construct
  source 1..23: mol_type = other RNA
cggaccacgcagtctataatgcc

SEQ ID NO: 383 - RNA, 23 nt, synthetic construct
  source 1..23: mol_type = other RNA
cttgggaatacggaccacgcagt

SEQ ID NO: 384 - RNA, 23 nt, synthetic construct
  source 1..23: mol_type = other RNA
gaagtaggcggctcggtagatga

SEQ ID NO: 385 - RNA, 23 nt, synthetic construct
  source 1..23: mol_type = other RNA
ctgctagacgggtacgggcaaaa

SEQ ID NO: 386 - RNA, 23 nt, synthetic construct
  source 1..23: mol_type = other RNA
tccagctgatgacgatgtgagtg

SEQ ID NO: 387 - RNA, 23 nt, synthetic construct
  source 1..23: mol_type = other RNA
atacggaccacgcagtctataat

SEQ ID NO: 388 - RNA, 23 nt, synthetic construct
  source 1..23: mol_type = other RNA
aaccaggcagtcaccgaggcctc

SEQ ID NO: 389 - RNA, 23 nt, synthetic construct
  source 1..23: mol_type = other RNA
tgacagtctgtgcgatcatccag

SEQ ID NO: 390 - RNA, 23 nt, synthetic construct
  source 1..23: mol_type = other RNA
tagacgggtacgggcaaaatcaa

SEQ ID NO: 391 - RNA, 23 nt, synthetic construct
  source 1..23: mol_type = other RNA
gcagtgacagtctgtgcgatcat

SEQ ID NO: 392 - RNA, 23 nt, synthetic construct
  source 1..23: mol_type = other RNA
agtgacagtctgtgcgatcatcc

SEQ ID NO: 393 - RNA, 23 nt, synthetic construct
  source 1..23: mol_type = other RNA
gctagacgggtacgggcaaaatc

SEQ ID NO: 394 - RNA, 23 nt, synthetic construct
  source 1..23: mol_type = other RNA
agtaggcggctcggtagatgata

SEQ ID NO: 395 - RNA, 23 nt, synthetic construct
  source 1..23: mol_type = other RNA
gaatacggaccacgcagtctata

SEQ ID NO: 396 - RNA, 23 nt, synthetic construct
  source 1..23: mol_type = other RNA
ctttgtattgcttatctgcagtg

SEQ ID NO: 397 - RNA, 23 nt, synthetic construct
  source 1..23: mol_type = other RNA
tttgtattgcttatctgcagtga

SEQ ID NO: 398 - RNA, 23 nt, synthetic construct
  source 1..23: mol_type = other RNA
ttgtattgcttatctgcagtgat

SEQ ID NO: 399 - RNA, 23 nt, synthetic construct
  source 1..23: mol_type = other RNA
tatctgcagtgatctgcttgctg

SEQ ID NO: 400 - RNA, 23 nt, synthetic construct
  source 1..23: mol_type = other RNA
gtattgcttatctgcagtgatct

SEQ ID NO: 401 - RNA, 23 nt, synthetic construct
  source 1..23: mol_type = other RNA
tgtattgcttatctgcagtgatc

SEQ ID NO: 402 - RNA, 23 nt, synthetic construct
  source 1..23: mol_type = other RNA
tgcttatctgcagtgatctgctt

SEQ ID NO: 403 - RNA, 23 nt, synthetic construct
  source 1..23: mol_type = other RNA
ttgcttatctgcagtgatctgct

SEQ ID NO: 404 - RNA, 23 nt, synthetic construct
  source 1..23: mol_type = other RNA
atctgcagtgatctgcttgctgg

SEQ ID NO: 405 - RNA, 23 nt, synthetic construct
  source 1..23: mol_type = other RNA
tattgcttatctgcagtgatctg

SEQ ID NO: 406 - RNA, 23 nt, synthetic construct
  source 1..23: mol_type = other RNA
ttctccaaatttgttatttatca

SEQ ID NO: 407 - RNA, 23 nt, synthetic construct
  source 1..23: mol_type = other RNA
caaatttgttatttatcaggagt

SEQ ID NO: 408 - RNA, 23 nt, synthetic construct
  source 1..23: mol_type = other RNA
gaggcctcggaattccctttcag

SEQ ID NO: 409 - RNA, 23 nt, synthetic construct
  source 1..23: mol_type = other RNA
agatatgttatataatacaacat

SEQ ID NO: 410 - RNA, 23 nt, synthetic construct
  source 1..23: mol_type = other RNA
gcagtcaccgaggcctcggaatt

SEQ ID NO: 411 - RNA, 23 nt, synthetic construct
  source 1..23: mol_type = other RNA
cgaggcctcggaattccctttca

SEQ ID NO: 412 - RNA, 23 nt, synthetic construct
  source 1..23: mol_type = other RNA
caagatatgttatataatacaac

SEQ ID NO: 413 - RNA, 23 nt, synthetic construct
  source 1..23: mol_type = other RNA
agtcaccgaggcctcggaattcc

SEQ ID NO: 414 - RNA, 23 nt, synthetic construct
  source 1..23: mol_type = other RNA
caccgaggcctcggaattccctt

SEQ ID NO: 415 - RNA, 23 nt, synthetic construct
  source 1..23: mol_type = other RNA
cctcggaattccctttcagctcc

SEQ ID NO: 416 - RNA, 23 nt, synthetic construct
  source 1..23: mol_type = other RNA
tcggaattccctttcagctccag

SEQ ID NO: 417 - RNA, 23 nt, synthetic construct
  source 1..23: mol_type = other RNA
ggcctcggaattccctttcagct

SEQ ID NO: 418 - RNA, 23 nt, synthetic construct
  source 1..23: mol_type = other RNA
ctcggaattccctttcagctcca

SEQ ID NO: 419 - RNA, 23 nt, synthetic construct
  source 1..23: mol_type = other RNA
gcctcggaattccctttcagctc

SEQ ID NO: 420 - RNA, 23 nt, synthetic construct
  source 1..23: mol_type = other RNA
atgttatataatacaacatgcct

SEQ ID NO: 421 - RNA, 23 nt, synthetic construct
  source 1..23: mol_type = other RNA
aagatatgttatataatacaaca

SEQ ID NO: 422 - RNA, 23 nt, synthetic construct
  source 1..23: mol_type = other RNA
tcaagatatgttatataatacaa

SEQ ID NO: 423 - RNA, 23 nt, synthetic construct
  source 1..23: mol_type = other RNA
tgttatataatacaacatgcctg

SEQ ID NO: 424 - RNA, 23 nt, synthetic construct
  source 1..23: mol_type = other RNA
ccgaggcctcggaattccctttc

SEQ ID NO: 425 - RNA, 23 nt, synthetic construct
  source 1..23: mol_type = other RNA
gtcaccgaggcctcggaattccc

SEQ ID NO: 426 - RNA, 23 nt, synthetic construct
  source 1..23: mol_type = other RNA
accgaggcctcggaattcccttt

SEQ ID NO: 427 - RNA, 23 nt, synthetic construct
  source 1..23: mol_type = other RNA
tcaccgaggcctcggaattccct

SEQ ID NO: 428 - RNA, 23 nt, synthetic construct
  source 1..23: mol_type = other RNA
atttcatcatacaagacaagcac

SEQ ID NO: 429 - RNA, 23 nt, synthetic construct
  source 1..23: mol_type = other RNA
tgtatttatctttgaaggcgaag

SEQ ID NO: 430 - RNA, 23 nt, synthetic construct
  source 1..23: mol_type = other RNA
atttgtagatcttaaccaggcag

SEQ ID NO: 431 - RNA, 23 nt, synthetic construct
  source 1..23: mol_type = other RNA
ttccctttgcagtgtcatagata

SEQ ID NO: 432 - RNA, 23 nt, synthetic construct
  source 1..23: mol_type = other RNA
atcatacaagacaagcacaaaag

SEQ ID NO: 433 - RNA, 23 nt, synthetic construct
  source 1..23: mol_type = other RNA
tagatcttaaccaggcagtcacc

SEQ ID NO: 434 - RNA, 23 nt, synthetic construct
  source 1..23: mol_type = other RNA
aagcattccctttgcagtgtcat

SEQ ID NO: 435 - RNA, 23 nt, synthetic construct
  source 1..23: mol_type = other RNA
tttgcagtgtcatagataccgaa

SEQ ID NO: 436 - RNA, 23 nt, synthetic construct
  source 1..23: mol_type = other RNA
agagaaaactggtcagatgaata

SEQ ID NO: 437 - RNA, 23 nt, synthetic construct
  source 1..23: mol_type = other RNA
tgcagtgtcatagataccgaagt

SEQ ID NO: 438 - RNA, 23 nt, synthetic construct
  source 1..23: mol_type = other RNA
tcagatttgtagatcttaaccag

SEQ ID NO: 439 - RNA, 23 nt, synthetic construct
  source 1..23: mol_type = other RNA
tccctttgcagtgtcatagatac

SEQ ID NO: 440 - RNA, 23 nt, synthetic construct
  source 1..23: mol_type = other RNA
gaacattggaccatgcacccttg

SEQ ID NO: 441 - RNA, 23 nt, synthetic construct
  source 1..23: mol_type = other RNA
aatcccatcagatttgtagatct

SEQ ID NO: 442 - RNA, 23 nt, synthetic construct
  source 1..23: mol_type = other RNA
gcagtgtcatagataccgaagta

SEQ ID NO: 443 - RNA, 23 nt, synthetic construct
  source 1..23: mol_type = other RNA
caagcacaaaagcaccacccatg

SEQ ID NO: 444 - RNA, 23 nt, synthetic construct
  source 1..23: mol_type = other RNA
gcggctcggtagatgataatacc

SEQ ID NO: 445 - RNA, 23 nt, synthetic construct
  source 1..23: mol_type = other RNA
ctccttgggaatacggaccacgc

SEQ ID NO: 446 - RNA, 23 nt, synthetic construct
  source 1..23: mol_type = other RNA
attccctttgcagtgtcatagat

SEQ ID NO: 447 - RNA, 23 nt, synthetic construct
  source 1..23: mol_type = other RNA
catacaagacaagcacaaaagca

SEQ ID NO: 448 - RNA, 23 nt, synthetic construct
  source 1..23: mol_type = other RNA
agacacgttaaagccttggtaca

SEQ ID NO: 449 - RNA, 23 nt, synthetic construct
  source 1..23: mol_type = other RNA
tgagaacattggaccatgcaccc

SEQ ID NO: 450 - RNA, 23 nt, synthetic construct
  source 1..23: mol_type = other RNA
gcttgtatttatctttgaaggcg

SEQ ID NO: 451 - RNA, 23 nt, synthetic construct
  source 1..23: mol_type = other RNA
gctcggtagatgataataccctg

SEQ ID NO: 452 - RNA, 23 nt, synthetic construct
  source 1..23: mol_type = other RNA
agtgtcatagataccgaagtagg

SEQ ID NO: 453 - RNA, 23 nt, synthetic construct
  source 1..23: mol_type = other RNA
atcagatttgtagatcttaacca

SEQ ID NO: 454 - RNA, 23 nt, synthetic construct
  source 1..23: mol_type = other RNA
ggtagatgataataccctgcaca

SEQ ID NO: 455 - RNA, 23 nt, synthetic construct
  source 1..23: mol_type = other RNA
caggcccttaatcccatcagatt

SEQ ID NO: 456 - RNA, 23 nt, synthetic construct
  source 1..23: mol_type = other RNA
agatgataataccctgcacagac

SEQ ID NO: 457 - RNA, 23 nt, synthetic construct
  source 1..23: mol_type = other RNA
tacaggcccttaatcccatcaga

SEQ ID NO: 458 - RNA, 23 nt, synthetic construct
  source 1..23: mol_type = other RNA
acagacacgttaaagccttggta

SEQ ID NO: 459 - RNA, 23 nt, synthetic construct
  source 1..23: mol_type = other RNA
agaaaactggtcagatgaatatt

SEQ ID NO: 460 - RNA, 23 nt, synthetic construct
  source 1..23: mol_type = other RNA
tgtagatcttaaccaggcagtca

SEQ ID NO: 461 - RNA, 23 nt, synthetic construct
  source 1..23: mol_type = other RNA
tcaaatggataggaagtcaaccc

SEQ ID NO: 462 - RNA, 23 nt, synthetic construct
  source 1..23: mol_type = other RNA
cattccctttgcagtgtcataga

SEQ ID NO: 463 - RNA, 23 nt, synthetic construct
  source 1..23: mol_type = other RNA
catcagatttgtagatcttaacc

SEQ ID NO: 464 - RNA, 23 nt, synthetic construct
  source 1..23: mol_type = other RNA
ctcggtagatgataataccctgc

SEQ ID NO: 465 - RNA, 23 nt, synthetic construct
  source 1..23: mol_type = other RNA
tttgtagatcttaaccaggcagt

SEQ ID NO: 466 - RNA, 23 nt, synthetic construct
  source 1..23: mol_type = other RNA
acaggcccttaatcccatcagat

SEQ ID NO: 467 - RNA, 23 nt, synthetic construct
  source 1..23: mol_type = other RNA
ctttgcagtgtcatagataccga

SEQ ID NO: 468 - RNA, 23 nt, synthetic construct
  source 1..23: mol_type = other RNA
cacatcagctgctagacgggtac

SEQ ID NO: 469 - RNA, 23 nt, synthetic construct
  source 1..23: mol_type = other RNA
ccctttgcagtgtcatagatacc

SEQ ID NO: 470 - RNA, 23 nt, synthetic construct
  source 1..23: mol_type = other RNA
ctccagctttacccacatcagct

SEQ ID NO: 471 - RNA, 23 nt, synthetic construct
  source 1..23: mol_type = other RNA
ttacccacatcagctgctagacg

SEQ ID NO: 472 - RNA, 23 nt, synthetic construct
  source 1..23: mol_type = other RNA
ttaaagccttggtacaggccctt

SEQ ID NO: 473 - RNA, 23 nt, synthetic construct
  source 1..23: mol_type = other RNA
cagctgctagacgggtacgggca

SEQ ID NO: 474 - RNA, 23 nt, synthetic construct
  source 1..23: mol_type = other RNA
cagctttacccacatcagctgct

SEQ ID NO: 475 - RNA, 23 nt, synthetic construct
  source 1..23: mol_type = other RNA
tcagctgctagacgggtacgggc

SEQ ID NO: 476 - RNA, 23 nt, synthetic construct
  source 1..23: mol_type = other RNA
tccagctttacccacatcagctg

SEQ ID NO: 477 - RNA, 23 nt, synthetic construct
  source 1..23: mol_type = other RNA
ggctcggtagatgataataccct

SEQ ID NO: 478 - RNA, 23 nt, synthetic construct
  source 1..23: mol_type = other RNA
aggcggctcggtagatgataata

SEQ ID NO: 479 - RNA, 23 nt, synthetic construct
  source 1..23: mol_type = other RNA
catcagctgctagacgggtacgg

SEQ ID NO: 480 - RNA, 23 nt, synthetic construct
  source 1..23: mol_type = other RNA
gtacaggcccttaatcccatcag

SEQ ID NO: 481 - RNA, 23 nt, synthetic construct
  source 1..23: mol_type = other RNA
atgataataccctgcacagacac

SEQ ID NO: 482 - RNA, 23 nt, synthetic construct
  source 1..23: mol_type = other RNA
ccttgggaatacggaccacgcag

SEQ ID NO: 483 - RNA, 23 nt, synthetic construct
  source 1..23: mol_type = other RNA
tccttgggaatacggaccacgca

SEQ ID NO: 484 - RNA, 23 nt, synthetic construct
  source 1..23: mol_type = other RNA
cagatttgtagatcttaaccagg

SEQ ID NO: 485 - RNA, 23 nt, synthetic construct
  source 1..23: mol_type = other RNA
tgtacttcttgatttcatcatac

SEQ ID NO: 486 - RNA, 23 nt, synthetic construct
  source 1..23: mol_type = other RNA
atcccatcagatttgtagatctt

SEQ ID NO: 487 - RNA, 23 nt, synthetic construct
  source 1..23: mol_type = other RNA
gtagatgataataccctgcacag

SEQ ID NO: 488 - RNA, 23 nt, synthetic construct
  source 1..23: mol_type = other RNA
gacacgttaaagccttggtacag

SEQ ID NO: 489 - RNA, 23 nt, synthetic construct
  source 1..23: mol_type = other RNA
agctttacccacatcagctgcta

SEQ ID NO: 490 - RNA, 23 nt, synthetic construct
  source 1..23: mol_type = other RNA
aagcacaaaagcaccacccatgc

SEQ ID NO: 491 - RNA, 23 nt, synthetic construct
  source 1..23: mol_type = other RNA
atcttaaccaggcagtcaccgag

SEQ ID NO: 492 - RNA, 23 nt, synthetic construct
  source 1..23: mol_type = other RNA
tttacccacatcagctgctagac

SEQ ID NO: 493 - RNA, 23 nt, synthetic construct
  source 1..23: mol_type = other RNA
cttaatcccatcagatttgtaga

SEQ ID NO: 494 - RNA, 23 nt, synthetic construct
  source 1..23: mol_type = other RNA
cagtgtcatagataccgaagtag

SEQ ID NO: 495 - RNA, 23 nt, synthetic construct
  source 1..23: mol_type = other RNA
ccagctttacccacatcagctgc

SEQ ID NO: 496 - RNA, 23 nt, synthetic construct
  source 1..23: mol_type = other RNA
atcagctgctagacgggtacggg

SEQ ID NO: 497 - RNA, 23 nt, synthetic construct
  source 1..23: mol_type = other RNA
gatgataataccctgcacagaca

SEQ ID NO: 498 - RNA, 23 nt, synthetic construct
  source 1..23: mol_type = other RNA
tttcatcatacaagacaagcaca

SEQ ID NO: 499 - RNA, 23 nt, synthetic construct
  source 1..23: mol_type = other RNA
cagacacgttaaagccttggtac

SEQ ID NO: 500 - RNA, 23 nt, synthetic construct
  source 1..23: mol_type = other RNA
agaacattggaccatgcaccctt

SEQ ID NO: 501 - RNA, 23 nt, synthetic construct
  source 1..23: mol_type = other RNA
gtagatcttaaccaggcagtcac

SEQ ID NO: 502 - RNA, 23 nt, synthetic construct
  source 1..23: mol_type = other RNA
agctccagctttacccacatcag

SEQ ID NO: 503 - RNA, 23 nt, synthetic construct
  source 1..23: mol_type = other RNA
gctccttgggaatacggaccacg

SEQ ID NO: 504 - RNA, 23 nt, synthetic construct
  source 1..23: mol_type = other RNA
gaagcattccctttgcagtgtca

SEQ ID NO: 505 - RNA, 23 nt, synthetic construct
  source 1..23: mol_type = other RNA
ccttggtacaggcccttaatccc

SEQ ID NO: 506 - RNA, 23 nt, synthetic construct
  source 1..23: mol_type = other RNA
tagatgataataccctgcacaga

SEQ ID NO: 507 - RNA, 23 nt, synthetic construct
  source 1..23: mol_type = other RNA
aataccctgcacagacacgttaa

SEQ ID NO: 508 - RNA, 23 nt, synthetic construct
  source 1..23: mol_type = other RNA
gttaaagccttggtacaggccct

SEQ ID NO: 509 - RNA, 23 nt, synthetic construct
  source 1..23: mol_type = other RNA
agcattccctttgcagtgtcata

SEQ ID NO: 510 - RNA, 23 nt, synthetic construct
  source 1..23: mol_type = other RNA
tcttaaccaggcagtcaccgagg

SEQ ID NO: 511 - RNA, 23 nt, synthetic construct
  source 1..23: mol_type = other RNA
atacaagacaagcacaaaagcac

SEQ ID NO: 512 - RNA, 23 nt, synthetic construct
  source 1..23: mol_type = other RNA
gacaagcacaaaagcaccaccca

SEQ ID NO: 513 - RNA, 23 nt, synthetic construct
  source 1..23: mol_type = other RNA
acccacatcagctgctagacggg

SEQ ID NO: 514 - RNA, 23 nt, synthetic construct
  source 1..23: mol_type = other RNA
taaagccttggtacaggccctta

SEQ ID NO: 515 - RNA, 23 nt, synthetic construct
  source 1..23: mol_type = other RNA
ttcatcatacaagacaagcacaa

SEQ ID NO: 516 - RNA, 23 nt, synthetic construct
  source 1..23: mol_type = other RNA
gcccttaatcccatcagatttgt

SEQ ID NO: 517 - RNA, 23 nt, synthetic construct
  source 1..23: mol_type = other RNA
ttaatcccatcagatttgtagat

SEQ ID NO: 518 - RNA, 23 nt, synthetic construct
  source 1..23: mol_type = other RNA
tcggtagatgataataccctgca

SEQ ID NO: 519 - RNA, 23 nt, synthetic construct
  source 1..23: mol_type = other RNA
cacgttaaagccttggtacaggc

SEQ ID NO: 520 - RNA, 23 nt, synthetic construct
  source 1..23: mol_type = other RNA
tcccatcagatttgtagatctta

SEQ ID NO: 521 - RNA, 23 nt, synthetic construct
  source 1..23: mol_type = other RNA
tcatacaagacaagcacaaaagc

SEQ ID NO: 522 - RNA, 23 nt, synthetic construct
  source 1..23: mol_type = other RNA
ccttaatcccatcagatttgtag

SEQ ID NO: 523 - RNA, 23 nt, synthetic construct
  source 1..23: mol_type = other RNA
acattggaccatgcacccttgaa

SEQ ID NO: 524 - RNA, 23 nt, synthetic construct
  source 1..23: mol_type = other RNA
cttggtacaggcccttaatccca

SEQ ID NO: 525 - RNA, 23 nt, synthetic construct
  source 1..23: mol_type = other RNA
ttgcagtgtcatagataccgaag

SEQ ID NO: 526 - RNA, 23 nt, synthetic construct
  source 1..23: mol_type = other RNA
cacagacacgttaaagccttggt

SEQ ID NO: 527 - RNA, 23 nt, synthetic construct
  source 1..23: mol_type = other RNA
agcacaaaagcaccacccatgcc

SEQ ID NO: 528 - RNA, 23 nt, synthetic construct
  source 1..23: mol_type = other RNA
ccatcagatttgtagatcttaac

SEQ ID NO: 529 - RNA, 23 nt, synthetic construct
  source 1..23: mol_type = other RNA
ccacatcagctgctagacgggta

SEQ ID NO: 530 - RNA, 23 nt, synthetic construct
  source 1..23: mol_type = other RNA
gcattccctttgcagtgtcatag

SEQ ID NO: 531 - RNA, 23 nt, synthetic construct
  source 1..23: mol_type = other RNA
ctttacccacatcagctgctaga

SEQ ID NO: 532 - RNA, 23 nt, synthetic construct
  source 1..23: mol_type = other RNA
atccggaagcattccctttgcag

SEQ ID NO: 533 - RNA, 23 nt, synthetic construct
  source 1..23: mol_type = other RNA
agctgctagacgggtacgggcaa

SEQ ID NO: 534 - RNA, 23 nt, synthetic construct
  source 1..23: mol_type = other RNA
cggctcggtagatgataataccc

SEQ ID NO: 535 - RNA, 23 nt, synthetic construct
  source 1..23: mol_type = other RNA
gggtacgggcaaaatcaagaggg

SEQ ID NO: 536 - RNA, 23 nt, synthetic construct
  source 1..23: mol_type = other RNA
acatcagctgctagacgggtacg

SEQ ID NO: 537 - RNA, 23 nt, synthetic construct
  source 1..23: mol_type = other RNA
cccttaatcccatcagatttgta

SEQ ID NO: 538 - RNA, 23 nt, synthetic construct
  source 1..23: mol_type = other RNA
cgggcaaaatcaagagggtacac

SEQ ID NO: 539 - RNA, 23 nt, synthetic construct
  source 1..23: mol_type = other RNA
acgttaaagccttggtacaggcc

SEQ ID NO: 540 - RNA, 23 nt, synthetic construct
  source 1..23: mol_type = other RNA
tggtacaggcccttaatcccatc

SEQ ID NO: 541 - RNA, 23 nt, synthetic construct
  source 1..23: mol_type = other RNA
ggcggctcggtagatgataatac

SEQ ID NO: 542 - RNA, 23 nt, synthetic construct
  source 1..23: mol_type = other RNA
cgttaaagccttggtacaggccc

SEQ ID NO: 543 - RNA, 23 nt, synthetic construct
  source 1..23: mol_type = other RNA
ggtacaggcccttaatcccatca

SEQ ID NO: 544 - RNA, 23 nt, synthetic construct
  source 1..23: mol_type = other RNA
taataccctgcacagacacgtta

SEQ ID NO: 545 - RNA, 23 nt, synthetic construct
  source 1..23: mol_type = other RNA
gaccacgcagtctataatgcctt

SEQ ID NO: 546 - RNA, 23 nt, synthetic construct
  source 1..23: mol_type = other RNA
gttaagagcctgggtggggaagt

SEQ ID NO: 547 - RNA, 23 nt, synthetic construct
  source 1..23: mol_type = other RNA
tggggaagtatctgatgacattg

SEQ ID NO: 548 - RNA, 23 nt, synthetic construct
  source 1..23: mol_type = other RNA
ggtggggaagtatctgatgacat

SEQ ID NO: 549 - RNA, 23 nt, synthetic construct
  source 1..23: mol_type = other RNA
gtggggaagtatctgatgacatt

SEQ ID NO: 550 - RNA, 23 nt, synthetic construct
  source 1..23: mol_type = other RNA
ggggaagtatctgatgacattgg

SEQ ID NO: 551 - RNA, 23 nt, synthetic construct
  source 1..23: mol_type = other RNA
ttaagagcctgggtggggaagta

SEQ ID NO: 552 - RNA, 23 nt, synthetic construct
  source 1..23: mol_type = other RNA
ccgaagtaggcggctcggtagat

SEQ ID NO: 553 - RNA, 21 nt, synthetic construct
  source 1..21: mol_type = other RNA
tatttactggttgaaaatggg

SEQ ID NO: 554 - RNA, 21 nt, synthetic construct
  source 1..21: mol_type = other RNA
caaaggcattatagactgcgt

SEQ ID NO: 555 - RNA, 21 nt, synthetic construct
  source 1..21: mol_type = other RNA
tgatgaaatcaagaagtacac

SEQ ID NO: 556 - RNA, 21 nt, synthetic construct
  source 1..21: mol_type = other RNA
gatgatgggactcaattgtat

SEQ ID NO: 557 - RNA, 21 nt, synthetic construct
  source 1..21: mol_type = other RNA
gcattatagactgcgtggtcc

SEQ ID NO: 558 - RNA, 21 nt, synthetic construct
  source 1..21: mol_type = other RNA
gtcactcctgataaataacaa

SEQ ID NO: 559 - RNA, 21 nt, synthetic construct
  source 1..21: mol_type = other RNA
atacaaaggcattatagactg

SEQ ID NO: 560 - RNA, 21 nt, synthetic construct
  source 1..21: mol_type = other RNA
gccgcctacttcggtatctat

SEQ ID NO: 561 - RNA, 21 nt, synthetic construct
  source 1..21: mol_type = other RNA
agccgcctacttcggtatcta

SEQ ID NO: 562 - RNA, 21 nt, synthetic construct
  source 1..21: mol_type = other RNA
agactgcgtggtccgtattcc

SEQ ID NO: 563 - RNA, 21 nt, synthetic construct
  source 1..21: mol_type = other RNA
cactcacatcgtcatcagctg

SEQ ID NO: 564 - RNA, 21 nt, synthetic construct
  source 1..21: mol_type = other RNA
acttcgccttcaaagataaat

SEQ ID NO: 565 - RNA, 21 nt, synthetic construct
  source 1..21: mol_type = other RNA
ctacttcggtatctatgacac

SEQ ID NO: 566 - RNA, 21 nt, synthetic construct
  source 1..21: mol_type = other RNA
tttactggttgaaaatgggaa

SEQ ID NO: 567 - RNA, 21 nt, synthetic construct
  source 1..21: mol_type = other RNA
tgcccgtacccgtctagcagc

SEQ ID NO: 568 - RNA, 21 nt, synthetic construct
  source 1..21: mol_type = other RNA
agtcagggcgcaaaggaactg

SEQ ID NO: 569 - RNA, 21 nt, synthetic construct
  source 1..21: mol_type = other RNA
ttactggttgaaaatgggaag

SEQ ID NO: 570 - RNA, 21 nt, synthetic construct
  source 1..21: mol_type = other RNA
gagccgcctacttcggtatct

SEQ ID NO: 571 - RNA, 21 nt, synthetic construct
  source 1..21: mol_type = other RNA
cctcggtgactgcctggttaa

SEQ ID NO: 572 - RNA, 21 nt, synthetic construct
  source 1..21: mol_type = other RNA
catcgtcatcagctggatgat

SEQ ID NO: 573 - RNA, 21 nt, synthetic construct
  source 1..21: mol_type = other RNA
tttcagtcactcctgataaat

SEQ ID NO: 574 - RNA, 21 nt, synthetic construct
  source 1..21: mol_type = other RNA
tggatgatcgcacagactgtc

SEQ ID NO: 575 - RNA, 21 nt, synthetic construct
  source 1..21: mol_type = other RNA
gcaatacaaaggcattataga

SEQ ID NO: 576 - RNA, 21 nt, synthetic construct
  source 1..21: mol_type = other RNA
gcctcggtgactgcctggtta

SEQ ID NO: 577 - RNA, 21 nt, synthetic construct
  source 1..21: mol_type = other RNA
ctttaacgtgtctgtgcaggg

SEQ ID NO: 578 - RNA, 21 nt, synthetic construct
  source 1..21: mol_type = other RNA
aaaggcattatagactgcgtg

SEQ ID NO: 579 - RNA, 21 nt, synthetic construct
  source 1..21: mol_type = other RNA
gtgaacaggcatgttgtatta

SEQ ID NO: 580 - RNA, 21 nt, synthetic construct
  source 1..21: mol_type = other RNA
atctgaccagttttctcttaa

SEQ ID NO: 581 - RNA, 21 nt, synthetic construct
  source 1..21: mol_type = other RNA
aggctttaacgtgtctgtgca

SEQ ID NO: 582 - RNA, 21 nt, synthetic construct
  source 1..21: mol_type = other RNA
gcagtcagggcgcaaaggaac

SEQ ID NO: 583 - RNA, 21 nt, synthetic construct
  source 1..21: mol_type = other RNA
gatgatcgcacagactgtcac

SEQ ID NO: 584 - RNA, 21 nt, synthetic construct
  source 1..21: mol_type = other RNA
aggcattatagactgcgtggt

SEQ ID NO: 585 - RNA, 21 nt, synthetic construct
  source 1..21: mol_type = other RNA
tgatcgcacagactgtcactg

SEQ ID NO: 586 - RNA, 21 nt, synthetic construct
  source 1..21: mol_type = other RNA
ctgcgtggtccgtattcccaa

SEQ ID NO: 587 - RNA, 21 nt, synthetic construct
  source 1..21: mol_type = other RNA
caatacaaaggcattatagac

SEQ ID NO: 588 - RNA, 21 nt, synthetic construct
  source 1..21: mol_type = other RNA
catcagctggatgatcgcaca

SEQ ID NO: 589 - RNA, 21 nt, synthetic construct
  source 1..21: mol_type = other RNA
attatagactgcgtggtccgt

SEQ ID NO: 590 - RNA, 21 nt, synthetic construct
  source 1..21: mol_type = other RNA
tttgcccgtacccgtctagca

SEQ ID NO: 591 - RNA, 21 nt, synthetic construct
  source 1..21: mol_type = other RNA
acatcgtcatcagctggatga

SEQ ID NO: 592 - RNA, 21 nt, synthetic construct
  source 1..21: mol_type = other RNA
tcttgattttgcccgtacccg

SEQ ID NO: 593 - RNA, 21 nt, synthetic construct
  source 1..21: mol_type = other RNA
atagactgcgtggtccgtatt

SEQ ID NO: 594 - RNA, 21 nt, synthetic construct
  source 1..21: mol_type = other RNA
cgcctacttcggtatctatga

SEQ ID NO: 595 - RNA, 21 nt, synthetic construct
  source 1..21: mol_type = other RNA
gactgcgtggtccgtattccc

SEQ ID NO: 596 - RNA, 21 nt, synthetic construct
  source 1..21: mol_type = other RNA
tcatcagctggatgatcgcac

SEQ ID NO: 597 - RNA, 21 nt, synthetic construct
  source 1..21: mol_type = other RNA
ttatagactgcgtggtccgta

SEQ ID NO: 598 - RNA, 21 nt, synthetic construct
  source 1..21: mol_type = other RNA
cctacttcggtatctatgaca

SEQ ID NO: 599 - RNA, 21 nt, synthetic construct
  source 1..21: mol_type = other RNA
ttatttcagtcactcctgata

SEQ ID NO: 600 - RNA, 21 nt, synthetic construct
  source 1..21: mol_type = other RNA
gtcatcagctggatgatcgca

SEQ ID NO: 601 - RNA, 21 nt, synthetic construct
  source 1..21: mol_type = other RNA
attttgcccgtacccgtctag

SEQ ID NO: 602 - RNA, 21 nt, synthetic construct
  source 1..21: mol_type = other RNA
caaagggaatgcttccggatc

SEQ ID NO: 603 - RNA, 21 nt, synthetic construct
  source 1..21: mol_type = other RNA
aaggctttaacgtgtctgtgc

SEQ ID NO: 604 - RNA, 21 nt, synthetic construct
  source 1..21: mol_type = other RNA
aaggcattatagactgcgtgg

SEQ ID NO: 605 - RNA, 21 nt, synthetic construct
  source 1..21: mol_type = other RNA
ttgattttgcccgtacccgtc

SEQ ID NO: 606 - RNA, 21 nt, synthetic construct
  source 1..21: mol_type = other RNA
cgagccgcctacttcggtatc

SEQ ID NO: 607 - RNA, 21 nt, synthetic construct
  source 1..21: mol_type = other RNA
atcatctaccgagccgcctac

SEQ ID NO: 608 - RNA, 21 nt, synthetic construct
  source 1..21: mol_type = other RNA
tgattttgcccgtacccgtct

SEQ ID NO: 609 - RNA, 21 nt, synthetic construct
  source 1..21: mol_type = other RNA
tatcatctaccgagccgccta

SEQ ID NO: 610 - RNA, 21 nt, synthetic construct
  source 1..21: mol_type = other RNA
catctaccgagccgcctactt

SEQ ID NO: 611 - RNA, 21 nt, synthetic construct
  source 1..21: mol_type = other RNA
ctcttaacttcgccttcaaag

SEQ ID NO: 612 - RNA, 21 nt, synthetic construct
  source 1..21: mol_type = other RNA
ccacccaggctcttaacttcg

SEQ ID NO: 613 - RNA, 21 nt, synthetic construct
  source 1..21: mol_type = other RNA
ccgtattcccaaggagcaggg

SEQ ID NO: 614 - RNA, 21 nt, synthetic construct
  source 1..21: mol_type = other RNA
gagcagggagttctgtccttc

SEQ ID NO: 615 - RNA, 21 nt, synthetic construct
  source 1..21: mol_type = other RNA
tcccaaggagcagggagttct

SEQ ID NO: 616 - RNA, 21 nt, synthetic construct
  source 1..21: mol_type = other RNA
tccgtattcccaaggagcagg

SEQ ID NO: 617 - RNA, 21 nt, synthetic construct
  source 1..21: mol_type = other RNA
gcagggagttctgtccttctg

SEQ ID NO: 618 - RNA, 21 nt, synthetic construct
  source 1..21: mol_type = other RNA
gtccgtattcccaaggagcag

SEQ ID NO: 619 - RNA, 21 nt, synthetic construct
  source 1..21: mol_type = other RNA
agcagggagttctgtccttct

SEQ ID NO: 620 - RNA, 21 nt, synthetic construct
  source 1..21: mol_type = other RNA
ggagcagggagttctgtcctt

SEQ ID NO: 621 - RNA, 21 nt, synthetic construct
  source 1..21: mol_type = other RNA
ttcccaaggagcagggagttc

SEQ ID NO: 622 - RNA, 21 nt, synthetic construct
  source 1..21: mol_type = other RNA
aggagcagggagttctgtcct

SEQ ID NO: 623 - RNA, 21 nt, synthetic construct
  source 1..21: mol_type = other RNA
cccacccaggctcttaacttc

SEQ ID NO: 624 - RNA, 21 nt, synthetic construct
  source 1..21: mol_type = other RNA
tcttaacttcgccttcaaaga

SEQ ID NO: 625 - RNA, 21 nt, synthetic construct
  source 1..21: mol_type = other RNA
ttcagtcactcctgataaata

SEQ ID NO: 626 - RNA, 21 nt, synthetic construct
  source 1..21: mol_type = other RNA
cagtcactcctgataaataac

SEQ ID NO: 627 - RNA, 21 nt, synthetic construct
  source 1..21: mol_type = other RNA
tcagtcactcctgataaataa

SEQ ID NO: 628 - RNA, 21 nt, synthetic construct
  source 1..21: mol_type = other RNA
tgatgggactcaattgtattt

SEQ ID NO: 629 - RNA, 21 nt, synthetic construct
  source 1..21: mol_type = other RNA
gatgggactcaattgtatttt

SEQ ID NO: 630 - RNA, 21 nt, synthetic construct
  source 1..21: mol_type = other RNA
cactcctgataaataacaaat

SEQ ID NO: 631 - RNA, 21 nt, synthetic construct
  source 1..21: mol_type = other RNA
attcatctgaccagttttctc

SEQ ID NO: 632 - RNA, 21 nt, synthetic construct
  source 1..21: mol_type = other RNA
aacaggcatgttgtattatat

SEQ ID NO: 633 - RNA, 21 nt, synthetic construct
  source 1..21: mol_type = other RNA
agggaatgcttccggatccca

SEQ ID NO: 634 - RNA, 21 nt, synthetic construct
  source 1..21: mol_type = other RNA
gggaatgcttccggatcccaa

SEQ ID NO: 635 - RNA, 21 nt, synthetic construct
  source 1..21: mol_type = other RNA
cgaggcctcggtgactgcctg

SEQ ID NO: 636 - RNA, 21 nt, synthetic construct
  source 1..21: mol_type = other RNA
acaggcatgttgtattatata

SEQ ID NO: 637 - RNA, 21 nt, synthetic construct
  source 1..21: mol_type = other RNA
aatacaaaggcattatagact

SEQ ID NO: 638 - RNA, 21 nt, synthetic construct
  source 1..21: mol_type = other RNA
atttcagtcactcctgataaa

SEQ ID NO: 639 - RNA, 21 nt, synthetic construct
  source 1..21: mol_type = other RNA
atgatgggactcaattgtatt

SEQ ID NO: 640 - RNA, 21 nt, synthetic construct
  source 1..21: mol_type = other RNA
ctgaccagttttctcttaaag

SEQ ID NO: 641 - RNA, 21 nt, synthetic construct
  source 1..21: mol_type = other RNA
tgaccagttttctcttaaagc

SEQ ID NO: 642 - RNA, 21 nt, synthetic construct
  source 1..21: mol_type = other RNA
gataagcaatacaaaggcatt

SEQ ID NO: 643 - RNA, 21 nt, synthetic construct
  source 1..21: mol_type = other RNA
ataagcaatacaaaggcatta

SEQ ID NO: 644 - RNA, 21 nt, synthetic construct
  source 1..21: mol_type = other RNA
ttaacgtgtctgtgcagggta

SEQ ID NO: 645 - RNA, 21 nt, synthetic construct
  source 1..21: mol_type = other RNA
taacgtgtctgtgcagggtat

SEQ ID NO: 646 - RNA, 21 nt, synthetic construct
  source 1..21: mol_type = other RNA
tcacatcgtcatcagctggat

SEQ ID NO: 647 - RNA, 21 nt, synthetic construct
  source 1..21: mol_type = other RNA
tgatgatgggactcaattgta

SEQ ID NO: 648 - RNA, 21 nt, synthetic construct
  source 1..21: mol_type = other RNA
actgcgtggtccgtattccca

SEQ ID NO: 649 - RNA, 21 nt, synthetic construct
  source 1..21: mol_type = other RNA
gaacaggcatgttgtattata

SEQ ID NO: 650 - RNA, 21 nt, synthetic construct
  source 1..21: mol_type = other RNA
tatttcagtcactcctgataa

SEQ ID NO: 651 - RNA, 21 nt, synthetic construct
  source 1..21: mol_type = other RNA
taagcaatacaaaggcattat

SEQ ID NO: 652 - RNA, 21 nt, synthetic construct
  source 1..21: mol_type = other RNA
actcacatcgtcatcagctgg

SEQ ID NO: 653 - RNA, 21 nt, synthetic construct
  source 1..21: mol_type = other RNA
ccgcctacttcggtatctatg

SEQ ID NO: 654 - RNA, 21 nt, synthetic construct
  source 1..21: mol_type = other RNA
cacatcgtcatcagctggatg

SEQ ID NO: 655 - RNA, 21 nt, synthetic construct
  source 1..21: mol_type = other RNA
gcctacttcggtatctatgac

SEQ ID NO: 656 - RNA, 21 nt, synthetic construct
  source 1..21: mol_type = other RNA
tttaacgtgtctgtgcagggt

SEQ ID NO: 657 - RNA, 21 nt, synthetic construct
  source 1..21: mol_type = other RNA
tcgccgccgcatgatgatgca

SEQ ID NO: 658 - RNA, 21 nt, synthetic construct
  source 1..21: mol_type = other RNA
cattatagactgcgtggtccg

SEQ ID NO: 659 - RNA, 21 nt, synthetic construct
  source 1..21: mol_type = other RNA
tgcgtggtccgtattcccaag

SEQ ID NO: 660 - RNA, 21 nt, synthetic construct
  source 1..21: mol_type = other RNA
atctaccgagccgcctacttc

SEQ ID NO: 661 - RNA, 21 nt, synthetic construct
  source 1..21: mol_type = other RNA
ttgcccgtacccgtctagcag

SEQ ID NO: 662 - RNA, 21 nt, synthetic construct
  source 1..21: mol_type = other RNA
ctcacatcgtcatcagctgga

SEQ ID NO: 663 - RNA, 21 nt, synthetic construct
  source 1..21: mol_type = other RNA
tatagactgcgtggtccgtat

SEQ ID NO: 664 - RNA, 21 nt, synthetic construct
  source 1..21: mol_type = other RNA
ggcctcggtgactgcctggtt

SEQ ID NO: 665 - RNA, 21 nt, synthetic construct
  source 1..21: mol_type = other RNA
ggatgatcgcacagactgtca

SEQ ID NO: 666 - RNA, 21 nt, synthetic construct
  source 1..21: mol_type = other RNA
gattttgcccgtacccgtcta

SEQ ID NO: 667 - RNA, 21 nt, synthetic construct
  source 1..21: mol_type = other RNA
gatcgcacagactgtcactgc

SEQ ID NO: 668 - RNA, 21 nt, synthetic construct
  source 1..21: mol_type = other RNA
atgatcgcacagactgtcact

SEQ ID NO: 669 - RNA, 21 nt, synthetic construct
  source 1..21: mol_type = other RNA
ttttgcccgtacccgtctagc

SEQ ID NO: 670 - RNA, 21 nt, synthetic construct
  source 1..21: mol_type = other RNA
tcatctaccgagccgcctact

SEQ ID NO: 671 - RNA, 21 nt, synthetic construct
  source 1..21: mol_type = other RNA
tagactgcgtggtccgtattc

SEQ ID NO: 672 - RNA, 21 nt, synthetic construct
  source 1..21: mol_type = other RNA
ctgcagataagcaatacaaag

SEQ ID NO: 673 - RNA, 21 nt, synthetic construct
  source 1..21: mol_type = other RNA
actgcagataagcaatacaaa

SEQ ID NO: 674 - RNA, 21 nt, synthetic construct
  source 1..21: mol_type = other RNA
cactgcagataagcaatacaa

SEQ ID NO: 675 - RNA, 21 nt, synthetic construct
  source 1..21: mol_type = other RNA
gcaagcagatcactgcagata

SEQ ID NO: 676 - RNA, 21 nt, synthetic construct
  source 1..21: mol_type = other RNA
atcactgcagataagcaatac

SEQ ID NO: 677 - RNA, 21 nt, synthetic construct
  source 1..21: mol_type = other RNA
tcactgcagataagcaataca

SEQ ID NO: 678 - RNA, 21 nt, synthetic construct
  source 1..21: mol_type = other RNA
gcagatcactgcagataagca

SEQ ID NO: 679 - RNA, 21 nt, synthetic construct
  source 1..21: mol_type = other RNA
cagatcactgcagataagcaa

SEQ ID NO: 680 - RNA, 21 nt, synthetic construct
  source 1..21: mol_type = other RNA
agcaagcagatcactgcagat

SEQ ID NO: 681 - RNA, 21 nt, synthetic construct
  source 1..21: mol_type = other RNA
gatcactgcagataagcaata

SEQ ID NO: 682 - RNA, 21 nt, synthetic construct
  source 1..21: mol_type = other RNA
ataaataacaaatttggagaa

SEQ ID NO: 683 - RNA, 21 nt, synthetic construct
  source 1..21: mol_type = other RNA
tcctgataaataacaaatttg

SEQ ID NO: 684 - RNA, 21 nt, synthetic construct
  source 1..21: mol_type = other RNA
gaaagggaattccgaggcctc

SEQ ID NO: 685 - RNA, 21 nt, synthetic construct
  source 1..21: mol_type = other RNA
gttgtattatataacatatct

SEQ ID NO: 686 - RNA, 21 nt, synthetic construct
  source 1..21: mol_type = other RNA
ttccgaggcctcggtgactgc

SEQ ID NO: 687 - RNA, 21 nt, synthetic construct
  source 1..21: mol_type = other RNA
aaagggaattccgaggcctcg

SEQ ID NO: 688 - RNA, 21 nt, synthetic construct
  source 1..21: mol_type = other RNA
tgtattatataacatatcttg

SEQ ID NO: 689 - RNA, 21 nt, synthetic construct
  source 1..21: mol_type = other RNA
aattccgaggcctcggtgact

SEQ ID NO: 690 - RNA, 21 nt, synthetic construct
  source 1..21: mol_type = other RNA
gggaattccgaggcctcggtg

SEQ ID NO: 691 - RNA, 21 nt, synthetic construct
  source 1..21: mol_type = other RNA
agctgaaagggaattccgagg

SEQ ID NO: 692 - RNA, 21 nt, synthetic construct
  source 1..21: mol_type = other RNA
ggagctgaaagggaattccga

SEQ ID NO: 693 - RNA, 21 nt, synthetic construct
  source 1..21: mol_type = other RNA
ctgaaagggaattccgaggcc

SEQ ID NO: 694 - RNA, 21 nt, synthetic construct
  source 1..21: mol_type = other RNA
gagctgaaagggaattccgag

SEQ ID NO: 695 - RNA, 21 nt, synthetic construct
  source 1..21: mol_type = other RNA
gctgaaagggaattccgaggc

SEQ ID NO: 696 - RNA, 21 nt, synthetic construct
  source 1..21: mol_type = other RNA
gcatgttgtattatataacat

SEQ ID NO: 697 - RNA, 21 nt, synthetic construct
  source 1..21: mol_type = other RNA
ttgtattatataacatatctt

SEQ ID NO: 698 - RNA, 21 nt, synthetic construct
  source 1..21: mol_type = other RNA
gtattatataacatatcttga

SEQ ID NO: 699 - RNA, 21 nt, synthetic construct
  source 1..21: mol_type = other RNA
ggcatgttgtattatataaca

SEQ ID NO: 700 - RNA, 21 nt, synthetic construct
  source 1..21: mol_type = other RNA
aagggaattccgaggcctcgg

SEQ ID NO: 701 - RNA, 21 nt, synthetic construct
  source 1..21: mol_type = other RNA
gaattccgaggcctcggtgac

SEQ ID NO: 702 - RNA, 21 nt, synthetic construct
  source 1..21: mol_type = other RNA
agggaattccgaggcctcggt

SEQ ID NO: 703 - RNA, 21 nt, synthetic construct
  source 1..21: mol_type = other RNA
ggaattccgaggcctcggtga

SEQ ID NO: 704 - RNA, 21 nt, synthetic construct
  source 1..21: mol_type = other RNA
gcttgtcttgtatgatgaaat

SEQ ID NO: 705 - RNA, 21 nt, synthetic construct
  source 1..21: mol_type = other RNA
tcgccttcaaagataaataca

SEQ ID NO: 706 - RNA, 21 nt, synthetic construct
  source 1..21: mol_type = other RNA
gcctggttaagatctacaaat

SEQ ID NO: 707 - RNA, 21 nt, synthetic construct
  source 1..21: mol_type = other RNA
tctatgacactgcaaagggaa

SEQ ID NO: 708 - RNA, 21 nt, synthetic construct
  source 1..21: mol_type = other RNA
tttgtgcttgtcttgtatgat

SEQ ID NO: 709 - RNA, 21 nt, synthetic construct
  source 1..21: mol_type = other RNA
tgactgcctggttaagatcta

SEQ ID NO: 710 - RNA, 21 nt, synthetic construct
  source 1..21: mol_type = other RNA
gacactgcaaagggaatgctt

SEQ ID NO: 711 - RNA, 21 nt, synthetic construct
  source 1..21: mol_type = other RNA
cggtatctatgacactgcaaa

SEQ ID NO: 712 - RNA, 21 nt, synthetic construct
  source 1..21: mol_type = other RNA
ttcatctgaccagttttctct

SEQ ID NO: 713 - RNA, 21 nt, synthetic construct
  source 1..21: mol_type = other RNA
ttcggtatctatgacactgca

SEQ ID NO: 714 - RNA, 21 nt, synthetic construct
  source 1..21: mol_type = other RNA
ggttaagatctacaaatctga

SEQ ID NO: 715 - RNA, 21 nt, synthetic construct
  source 1..21: mol_type = other RNA
atctatgacactgcaaaggga

SEQ ID NO: 716 - RNA, 21 nt, synthetic construct
  source 1..21: mol_type = other RNA
agggtgcatggtccaatgttc

SEQ ID NO: 717 - RNA, 21 nt, synthetic construct
  source 1..21: mol_type = other RNA
atctacaaatctgatgggatt

SEQ ID NO: 718 - RNA, 21 nt, synthetic construct
  source 1..21: mol_type = other RNA
cttcggtatctatgacactgc

SEQ ID NO: 719 - RNA, 21 nt, synthetic construct
  source 1..21: mol_type = other RNA
tgggtggtgcttttgtgcttg

SEQ ID NO: 720 - RNA, 21 nt, synthetic construct
  source 1..21: mol_type = other RNA
tattatcatctaccgagccgc

SEQ ID NO: 721 - RNA, 21 nt, synthetic construct
  source 1..21: mol_type = other RNA
gtggtccgtattcccaaggag

SEQ ID NO: 722 - RNA, 21 nt, synthetic construct
  source 1..21: mol_type = other RNA
ctatgacactgcaaagggaat

SEQ ID NO: 723 - RNA, 21 nt, synthetic construct
  source 1..21: mol_type = other RNA
cttttgtgcttgtcttgtatg

SEQ ID NO: 724 - RNA, 21 nt, synthetic construct
  source 1..21: mol_type = other RNA
taccaaggctttaacgtgtct

SEQ ID NO: 725 - RNA, 21 nt, synthetic construct
  source 1..21: mol_type = other RNA
gtgcatggtccaatgttctca

SEQ ID NO: 726 - RNA, 21 nt, synthetic construct
  source 1..21: mol_type = other RNA
ccttcaaagataaatacaagc

SEQ ID NO: 727 - RNA, 21 nt, synthetic construct
  source 1..21: mol_type = other RNA
gggtattatcatctaccgagc

SEQ ID NO: 728 - RNA, 21 nt, synthetic construct
  source 1..21: mol_type = other RNA
tacttcggtatctatgacact

SEQ ID NO: 729 - RNA, 21 nt, synthetic construct
  source 1..21: mol_type = other RNA
gttaagatctacaaatctgat

SEQ ID NO: 730 - RNA, 21 nt, synthetic construct
  source 1..21: mol_type = other RNA
tgcagggtattatcatctacc

SEQ ID NO: 731 - RNA, 21 nt, synthetic construct
  source 1..21: mol_type = other RNA
tctgatgggattaagggcctg

SEQ ID NO: 732 - RNA, 21 nt, synthetic construct
  source 1..21: mol_type = other RNA
ctgtgcagggtattatcatct

SEQ ID NO: 733 - RNA, 21 nt, synthetic construct
  source 1..21: mol_type = other RNA
tgatgggattaagggcctgta

SEQ ID NO: 734 - RNA, 21 nt, synthetic construct
  source 1..21: mol_type = other RNA
ccaaggctttaacgtgtctgt

SEQ ID NO: 735 - RNA, 21 nt, synthetic construct
  source 1..21: mol_type = other RNA
tattcatctgaccagttttct

SEQ ID NO: 736 - RNA, 21 nt, synthetic construct
  source 1..21: mol_type = other RNA
actgcctggttaagatctaca

SEQ ID NO: 737 - RNA, 21 nt, synthetic construct
  source 1..21: mol_type = other RNA
gttgacttcctatccatttga

SEQ ID NO: 738 - RNA, 21 nt, synthetic construct
  source 1..21: mol_type = other RNA
tatgacactgcaaagggaatg

SEQ ID NO: 739 - RNA, 21 nt, synthetic construct
  source 1..21: mol_type = other RNA
ttaagatctacaaatctgatg

SEQ ID NO: 740 - RNA, 21 nt, synthetic construct
  source 1..21: mol_type = other RNA
agggtattatcatctaccgag

SEQ ID NO: 741 - RNA, 21 nt, synthetic construct
  source 1..21: mol_type = other RNA
tgcctggttaagatctacaaa

SEQ ID NO: 742 - RNA, 21 nt, synthetic construct
  source 1..21: mol_type = other RNA
ctgatgggattaagggcctgt

SEQ ID NO: 743 - RNA, 21 nt, synthetic construct
  source 1..21: mol_type = other RNA
ggtatctatgacactgcaaag

SEQ ID NO: 744 - RNA, 21 nt, synthetic construct
  source 1..21: mol_type = other RNA
acccgtctagcagctgatgtg

SEQ ID NO: 745 - RNA, 21 nt, synthetic construct
  source 1..21: mol_type = other RNA
tatctatgacactgcaaaggg

SEQ ID NO: 746 - RNA, 21 nt, synthetic construct
  source 1..21: mol_type = other RNA
ctgatgtgggtaaagctggag

SEQ ID NO: 747 - RNA, 21 nt, synthetic construct
  source 1..21: mol_type = other RNA
tctagcagctgatgtgggtaa

SEQ ID NO: 748 - RNA, 21 nt, synthetic construct
  source 1..21: mol_type = other RNA
gggcctgtaccaaggctttaa

SEQ ID NO: 749 - RNA, 21 nt, synthetic construct
  source 1..21: mol_type = other RNA
cccgtacccgtctagcagctg

SEQ ID NO: 750 - RNA, 21 nt, synthetic construct
  source 1..21: mol_type = other RNA
cagctgatgtgggtaaagctg

SEQ ID NO: 751 - RNA, 21 nt, synthetic construct
  source 1..21: mol_type = other RNA
ccgtacccgtctagcagctga

SEQ ID NO: 752 - RNA, 21 nt, synthetic construct
  source 1..21: mol_type = other RNA
gctgatgtgggtaaagctgga

SEQ ID NO: 753 - RNA, 21 nt, synthetic construct
  source 1..21: mol_type = other RNA
ggtattatcatctaccgagcc

SEQ ID NO: 754 - RNA, 21 nt, synthetic construct
  source 1..21: mol_type = other RNA
ttatcatctaccgagccgcct

SEQ ID NO: 755 - RNA, 21 nt, synthetic construct
  source 1..21: mol_type = other RNA
gtacccgtctagcagctgatg

SEQ ID NO: 756 - RNA, 21 nt, synthetic construct
  source 1..21: mol_type = other RNA
gatgggattaagggcctgtac

SEQ ID NO: 757 - RNA, 21 nt, synthetic construct
  source 1..21: mol_type = other RNA
gtctgtgcagggtattatcat

SEQ ID NO: 758 - RNA, 21 nt, synthetic construct
  source 1..21: mol_type = other RNA
gcgtggtccgtattcccaagg

SEQ ID NO: 759 - RNA, 21 nt, synthetic construct
  source 1..21: mol_type = other RNA
cgtggtccgtattcccaagga

SEQ ID NO: 760 - RNA, 21 nt, synthetic construct
  source 1..21: mol_type = other RNA
tggttaagatctacaaatctg

SEQ ID NO: 761 - RNA, 21 nt, synthetic construct
  source 1..21: mol_type = other RNA
atgatgaaatcaagaagtaca

SEQ ID NO: 762 - RNA, 21 nt, synthetic construct
  source 1..21: mol_type = other RNA
gatctacaaatctgatgggat

SEQ ID NO: 763 - RNA, 21 nt, synthetic construct
  source 1..21: mol_type = other RNA
gtgcagggtattatcatctac

SEQ ID NO: 764 - RNA, 21 nt, synthetic construct
  source 1..21: mol_type = other RNA
gtaccaaggctttaacgtgtc

SEQ ID NO: 765 - RNA, 21 nt, synthetic construct
  source 1..21: mol_type = other RNA
gcagctgatgtgggtaaagct

SEQ ID NO: 766 - RNA, 21 nt, synthetic construct
  source 1..21: mol_type = other RNA
atgggtggtgcttttgtgctt

SEQ ID NO: 767 - RNA, 21 nt, synthetic construct
  source 1..21: mol_type = other RNA
cggtgactgcctggttaagat

SEQ ID NO: 768 - RNA, 21 nt, synthetic construct
  source 1..21: mol_type = other RNA
ctagcagctgatgtgggtaaa

SEQ ID NO: 769 - RNA, 21 nt, synthetic construct
  source 1..21: mol_type = other RNA
tacaaatctgatgggattaag

SEQ ID NO: 770 - RNA, 21 nt, synthetic construct
  source 1..21: mol_type = other RNA
acttcggtatctatgacactg

SEQ ID NO: 771 - RNA, 21 nt, synthetic construct
  source 1..21: mol_type = other RNA
agctgatgtgggtaaagctgg

SEQ ID NO: 772 - RNA, 21 nt, synthetic construct
  source 1..21: mol_type = other RNA
cgtacccgtctagcagctgat

SEQ ID NO: 773 - RNA, 21 nt, synthetic construct
  source 1..21: mol_type = other RNA
tctgtgcagggtattatcatc

SEQ ID NO: 774 - RNA, 21 nt, synthetic construct
  source 1..21: mol_type = other RNA
tgcttgtcttgtatgatgaaa

SEQ ID NO: 775 - RNA, 21 nt, synthetic construct
  source 1..21: mol_type = other RNA
accaaggctttaacgtgtctg

SEQ ID NO: 776 - RNA, 21 nt, synthetic construct
  source 1..21: mol_type = other RNA
gggtgcatggtccaatgttct

SEQ ID NO: 777 - RNA, 21 nt, synthetic construct
  source 1..21: mol_type = other RNA
gactgcctggttaagatctac

SEQ ID NO: 778 - RNA, 21 nt, synthetic construct
  source 1..21: mol_type = other RNA
gatgtgggtaaagctggagct

SEQ ID NO: 779 - RNA, 21 nt, synthetic construct
  source 1..21: mol_type = other RNA
tggtccgtattcccaaggagc

SEQ ID NO: 780 - RNA, 21 nt, synthetic construct
  source 1..21: mol_type = other RNA
acactgcaaagggaatgcttc

SEQ ID NO: 781 - RNA, 21 nt, synthetic construct
  source 1..21: mol_type = other RNA
gattaagggcctgtaccaagg

SEQ ID NO: 782 - RNA, 21 nt, synthetic construct
  source 1..21: mol_type = other RNA
tgtgcagggtattatcatcta

SEQ ID NO: 783 - RNA, 21 nt, synthetic construct
  source 1..21: mol_type = other RNA
aacgtgtctgtgcagggtatt

SEQ ID NO: 784 - RNA, 21 nt, synthetic construct
  source 1..21: mol_type = other RNA
ggcctgtaccaaggctttaac

SEQ ID NO: 785 - RNA, 21 nt, synthetic construct
  source 1..21: mol_type = other RNA
tgacactgcaaagggaatgct

SEQ ID NO: 786 - RNA, 21 nt, synthetic construct
  source 1..21: mol_type = other RNA
tcggtgactgcctggttaaga

SEQ ID NO: 787 - RNA, 21 nt, synthetic construct
  source 1..21: mol_type = other RNA
gcttttgtgcttgtcttgtat

SEQ ID NO: 788 - RNA, 21 nt, synthetic construct
  source 1..21: mol_type = other RNA
ggtggtgcttttgtgcttgtc

SEQ ID NO: 789 - RNA, 21 nt, synthetic construct
  source 1..21: mol_type = other RNA
cgtctagcagctgatgtgggt

SEQ ID NO: 790 - RNA, 21 nt, synthetic construct
  source 1..21: mol_type = other RNA
agggcctgtaccaaggcttta

SEQ ID NO: 791 - RNA, 21 nt, synthetic construct
  source 1..21: mol_type = other RNA
gtgcttgtcttgtatgatgaa

SEQ ID NO: 792 - RNA, 21 nt, synthetic construct
  source 1..21: mol_type = other RNA
aaatctgatgggattaagggc

SEQ ID NO: 793 - RNA, 21 nt, synthetic construct
  source 1..21: mol_type = other RNA
ctacaaatctgatgggattaa

SEQ ID NO: 794 - RNA, 21 nt, synthetic construct
  source 1..21: mol_type = other RNA
cagggtattatcatctaccga

SEQ ID NO: 795 - RNA, 21 nt, synthetic construct
  source 1..21: mol_type = other RNA
ctgtaccaaggctttaacgtg

SEQ ID NO: 796 - RNA, 21 nt, synthetic construct
  source 1..21: mol_type = other RNA
agatctacaaatctgatggga

SEQ ID NO: 797 - RNA, 21 nt, synthetic construct
  source 1..21: mol_type = other RNA
ttttgtgcttgtcttgtatga

SEQ ID NO: 798 - RNA, 21 nt, synthetic construct
  source 1..21: mol_type = other RNA
acaaatctgatgggattaagg

SEQ ID NO: 799 - RNA, 21 nt, synthetic construct
  source 1..21: mol_type = other RNA
caagggtgcatggtccaatgt

SEQ ID NO: 800 - RNA, 21 nt, synthetic construct
  source 1..21: mol_type = other RNA
ggattaagggcctgtaccaag

SEQ ID NO: 801 - RNA, 21 nt, synthetic construct
  source 1..21: mol_type = other RNA
tcggtatctatgacactgcaa

SEQ ID NO: 802 - RNA, 21 nt, synthetic construct
  source 1..21: mol_type = other RNA
caaggctttaacgtgtctgtg

SEQ ID NO: 803 - RNA, 21 nt, synthetic construct
  source 1..21: mol_type = other RNA
catgggtggtgcttttgtgct

SEQ ID NO: 804 - RNA, 21 nt, synthetic construct
  source 1..21: mol_type = other RNA
taagatctacaaatctgatgg

SEQ ID NO: 805 - RNA, 21 nt, synthetic construct
  source 1..21: mol_type = other RNA
cccgtctagcagctgatgtgg

SEQ ID NO: 806 - RNA, 21 nt, synthetic construct
  source 1..21: mol_type = other RNA
atgacactgcaaagggaatgc

SEQ ID NO: 807 - RNA, 21 nt, synthetic construct
  source 1..21: mol_type = other RNA
tagcagctgatgtgggtaaag

SEQ ID NO: 808 - RNA, 21 nt, synthetic construct
  source 1..21: mol_type = other RNA
gcaaagggaatgcttccggat

SEQ ID NO: 809 - RNA, 21 nt, synthetic construct
  source 1..21: mol_type = other RNA
gcccgtacccgtctagcagct

SEQ ID NO: 810 - RNA, 21 nt, synthetic construct
  source 1..21: mol_type = other RNA
gtattatcatctaccgagccg

SEQ ID NO: 811 - RNA, 21 nt, synthetic construct
  source 1..21: mol_type = other RNA
ctcttgattttgcccgtaccc

SEQ ID NO: 812 - RNA, 21 nt, synthetic construct
  source 1..21: mol_type = other RNA
tacccgtctagcagctgatgt

SEQ ID NO: 813 - RNA, 21 nt, synthetic construct
  source 1..21: mol_type = other RNA
caaatctgatgggattaaggg

SEQ ID NO: 814 - RNA, 21 nt, synthetic construct
  source 1..21: mol_type = other RNA
gtaccctcttgattttgcccg

SEQ ID NO: 815 - RNA, 21 nt, synthetic construct
  source 1..21: mol_type = other RNA
cctgtaccaaggctttaacgt

SEQ ID NO: 816 - RNA, 21 nt, synthetic construct
  source 1..21: mol_type = other RNA
tgggattaagggcctgtacca

SEQ ID NO: 817 - RNA, 21 nt, synthetic construct
  source 1..21: mol_type = other RNA
attatcatctaccgagccgcc

SEQ ID NO: 818 - RNA, 21 nt, synthetic construct
  source 1..21: mol_type = other RNA
gcctgtaccaaggctttaacg

SEQ ID NO: 819 - RNA, 21 nt, synthetic construct
  source 1..21: mol_type = other RNA
atgggattaagggcctgtacc

SEQ ID NO: 820 - RNA, 21 nt, synthetic construct
  source 1..21: mol_type = other RNA
acgtgtctgtgcagggtatta

SEQ ID NO: 821 - RNA, 21 nt, synthetic construct
  source 1..21: mol_type = other RNA
ggcattatagactgcgtggtc

SEQ ID NO: 822 - RNA, 21 nt, synthetic construct
  source 1..21: mol_type = other RNA
ttccccacccaggctcttaac

SEQ ID NO: 823 - RNA, 21 nt, synthetic construct
  source 1..21: mol_type = other RNA
atgtcatcagatacttcccca

SEQ ID NO: 824 - RNA, 21 nt, synthetic construct
  source 1..21: mol_type = other RNA
gtcatcagatacttccccacc

SEQ ID NO: 825 - RNA, 21 nt, synthetic construct
  source 1..21: mol_type = other RNA
tgtcatcagatacttccccac

SEQ ID NO: 826 - RNA, 21 nt, synthetic construct
  source 1..21: mol_type = other RNA
aatgtcatcagatacttcccc

SEQ ID NO: 827 - RNA, 21 nt, synthetic construct
  source 1..21: mol_type = other RNA
cttccccacccaggctcttaa

SEQ ID NO: 828 - RNA, 21 nt, synthetic construct
  source 1..21: mol_type = other RNA
ctaccgagccgcctacttcgg

SEQ ID NO: 829 - RNA, 23 nt, synthetic construct
  source 1..23: mol_type = other RNA
  modified_base 1: mod_base = cm
  misc_feature 1^2: note = Phosphorothioate bond
  modified_base 2: mod_base = OTHER; note = 2'-Fluoro-cytidine
  misc_feature 2^3: note = Phosphorothioate bond
  modified_base 3: mod_base = cm
  modified_base 4: mod_base = OTHER; note = 2'-O-methyl-adenosine
  modified_base 5: mod_base = um
  modified_base 6: mod_base = OTHER; note = 2'-Fluoro-uridine
  modified_base 7: mod_base = um
  modified_base 8: mod_base = um
  modified_base 9: mod_base = cm
  modified_base 10: mod_base = OTHER; note = 2'-O-methyl-adenosine
  modified_base 11: mod_base = OTHER; note = 2'-O-methyl-adenosine
  modified_base 12: mod_base = cm
  modified_base 13: mod_base = cm
  modified_base 14: mod_base = OTHER; note = 2'-Fluoro-adenosine
  modified_base 15: mod_base = gm
  modified_base 16: mod_base = OTHER; note = 2'-Fluoro-uridine
  modified_base 17: mod_base = OTHER; note = 2'-O-methyl-adenosine
  modified_base 18: mod_base = OTHER; note = 2'-Fluoro-adenosine
  modified_base 19: mod_base = OTHER; note = 2'-O-methyl-adenosine
  modified_base 20: mod_base = um
  modified_base 21: mod_base = OTHER; note = 2'-O-methyl-adenosine
  misc_feature 21^22: note = Phosphorothioate bond
  modified_base 22: mod_base = gm
  misc_feature 22^23: note = Phosphorothioate bond
  modified_base 23: mod_base = um
cccattttcaaccagtaaatagt

SEQ ID NO: 830 - RNA, 23 nt, synthetic construct
  source 1..23: mol_type = other RNA
  modified_base 1: mod_base = OTHER; note = 2'-O-methyl-adenosine
  misc_feature 1^2: note = Phosphorothioate bond
  modified_base 2: mod_base = OTHER; note = 2'-Fluoro-cytidine
  misc_feature 2^3: note = Phosphorothioate bond
  modified_base 3: mod_base = gm
  modified_base 4: mod_base = cm
  modified_base 5: mod_base = OTHER; note = 2'-O-methyl-adenosine
  modified_base 6: mod_base = OTHER; note = 2'-Fluoro-guanosine
  modified_base 7: mod_base = um
  modified_base 8: mod_base = cm
  modified_base 9: mod_base = um
  modified_base 10: mod_base = OTHER; note = 2'-O-methyl-adenosine
  modified_base 11: mod_base = um
  modified_base 12: mod_base = OTHER; note = 2'-O-methyl-adenosine
  modified_base 13: mod_base = OTHER; note = 2'-O-methyl-adenosine
  modified_base 14: mod_base = OTHER; note = 2'-Fluoro-uridine
  modified_base 15: mod_base = gm
  modified_base 16: mod_base = OTHER; note = 2'-Fluoro-cytidine
  modified_base 17: mod_base = cm
  modified_base 18: mod_base = OTHER; note = 2'-Fluoro-uridine
  modified_base 19: mod_base = um
  modified_base 20: mod_base = um
  modified_base 21: mod_base = gm
  misc_feature 21^22: note = Phosphorothioate bond
  modified_base 22: mod_base = um
  misc_feature 22^23: note = Phosphorothioate bond
  modified_base 23: mod_base = OTHER; note = 2'-O-methyl-adenosine
acgcagtctataatgcctttgta

SEQ ID NO: 831 - RNA, 23 nt, synthetic construct
  source 1..23: mol_type = other RNA
  modified_base 1: mod_base = gm
  misc_feature 1^2: note = Phosphorothioate bond
  modified_base 2: mod_base = OTHER; note = 2'-Fluoro-uridine
  misc_feature 2^3: note = Phosphorothioate bond
  modified_base 3: mod_base = gm
  modified_base 4: mod_base = um
  modified_base 5: mod_base = OTHER; note = 2'-O-methyl-adenosine
  modified_base 6: mod_base = OTHER; note = 2'-Fluoro-cytidine
  modified_base 7: mod_base = um
  modified_base 8: mod_base = um
  modified_base 9: mod_base = cm
  modified_base 10: mod_base = um
  modified_base 11: mod_base = um
  modified_base 12: mod_base = gm
  modified_base 13: mod_base = OTHER; note = 2'-O-methyl-adenosine
  modified_base 14: mod_base = OTHER; note = 2'-Fluoro-uridine
  modified_base 15: mod_base = um
  modified_base 16: mod_base = OTHER; note = 2'-Fluoro-uridine
  modified_base 17: mod_base = cm
  modified_base 18: mod_base = OTHER; note = 2'-Fluoro-adenosine
  modified_base 19: mod_base = um
  modified_base 20: mod_base = cm
  modified_base 21: mod_base = OTHER; note = 2'-O-methyl-adenosine
  misc_feature 21^22: note = Phosphorothioate bond
  modified_base 22: mod_base = um
  misc_feature 22^23: note = Phosphorothioate bond
  modified_base 23: mod_base = OTHER; note = 2'-O-methyl-adenosine
gtgtacttcttgatttcatcata

SEQ ID NO: 832 - RNA, 23 nt, synthetic construct
  source 1..23: mol_type = other RNA
  modified_base 1: mod_base = OTHER; note = 2'-O-methyl-adenosine
  misc_feature 1^2: note = Phosphorothioate bond
  modified_base 2: mod_base = OTHER; note = 2'-Fluoro-uridine
  misc_feature 2^3: note = Phosphorothioate bond
  modified_base 3: mod_base = OTHER; note = 2'-O-methyl-adenosine
  modified_base 4: mod_base = cm
  modified_base 5: mod_base = OTHER; note = 2'-O-methyl-adenosine
  modified_base 6: mod_base = OTHER; note = 2'-Fluoro-adenosine
  modified_base 7: mod_base = um
  modified_base 8: mod_base = um
  modified_base 9: mod_base = gm
  modified_base 10: mod_base = OTHER; note = 2'-O-methyl-adenosine
  modified_base 11: mod_base = gm
  modified_base 12: mod_base = um
  modified_base 13: mod_base = cm
  modified_base 14: mod_base = OTHER; note = 2'-Fluoro-cytidine
  modified_base 15: mod_base = cm
  modified_base 16: mod_base = OTHER; note = 2'-Fluoro-adenosine
  modified_base 17: mod_base = um
  modified_base 18: mod_base = OTHER; note = 2'-Fluoro-cytidine
  modified_base 19: mod_base = OTHER; note = 2'-O-methyl-adenosine
  modified_base 20: mod_base = um
  modified_base 21: mod_base = cm
  misc_feature 21^22: note = Phosphorothioate bond
  modified_base 22: mod_base = OTHER; note = 2'-O-methyl-adenosine
  misc_feature 22^23: note = Phosphorothioate bond
  modified_base 23: mod_base = um
atacaattgagtcccatcatcat

SEQ ID NO: 833 - RNA, 23 nt, synthetic construct
  source 1..23: mol_type = other RNA
  modified_base 1: mod_base = gm
  misc_feature 1^2: note = Phosphorothioate bond
  modified_base 2: mod_base = OTHER; note = 2'-Fluoro-guanosine
  misc_feature 2^3: note = Phosphorothioate bond
  modified_base 3: mod_base = OTHER; note = 2'-O-methyl-adenosine
  modified_base 4: mod_base = cm
  modified_base 5: mod_base = cm
  modified_base 6: mod_base = OTHER; note = 2'-Fluoro-adenosine
  modified_base 7: mod_base = cm
  modified_base 8: mod_base = gm
  modified_base 9: mod_base = cm
  modified_base 10: mod_base = OTHER; note = 2'-O-methyl-adenosine
  modified_base 11: mod_base = gm
  modified_base 12: mod_base = um
  modified_base 13: mod_base = cm
  modified_base 14: mod_base = OTHER; note = 2'-Fluoro-uridine
  modified_base 15: mod_base = OTHER; note = 2'-O-methyl-adenosine
  modified_base 16: mod_base = OTHER; note = 2'-Fluoro-uridine
  modified_base 17: mod_base = OTHER; note = 2'-O-methyl-adenosine
  modified_base 18: mod_base = OTHER; note = 2'-Fluoro-adenosine
  modified_base 19: mod_base = um
  modified_base 20: mod_base = gm
  modified_base 21: mod_base = cm
  misc_feature 21^22: note = Phosphorothioate bond
  modified_base 22: mod_base = cm
  misc_feature 22^23: note = Phosphorothioate bond
  modified_base 23: mod_base = um
ggaccacgcagtctataatgcct

SEQ ID NO: 834 - RNA, 23 nt, synthetic construct
  source 1..23: mol_type = other RNA
  modified_base 1: mod_base = um
  misc_feature 1^2: note = Phosphorothioate bond
  modified_base 2: mod_base = OTHER; note = 2'-Fluoro-uridine
  misc_feature 2^3: note = Phosphorothioate bond
  modified_base 3: mod_base = gm
  modified_base 4: mod_base = um
  modified_base 5: mod_base = um
  modified_base 6: mod_base = OTHER; note = 2'-Fluoro-adenosine
  modified_base 7: mod_base = um
  modified_base 8: mod_base = um
  modified_base 9: mod_base = um
  modified_base 10: mod_base = OTHER; note = 2'-O-methyl-adenosine
  modified_base 11: mod_base = um
  modified_base 12: mod_base = cm
  modified_base 13: mod_base = OTHER; note = 2'-O-methyl-adenosine
  modified_base 14: mod_base = OTHER; note = 2'-Fluoro-guanosine
  modified_base 15: mod_base = gm
  modified_base 16: mod_base = OTHER; note = 2'-Fluoro-adenosine
  modified_base 17: mod_base = gm
  modified_base 18: mod_base = OTHER; note = 2'-Fluoro-uridine
  modified_base 19: mod_base = gm
  modified_base 20: mod_base = OTHER; note = 2'-O-methyl-adenosine
  modified_base 21: mod_base = cm
  misc_feature 21^22: note = Phosphorothioate bond
  modified_base 22: mod_base = um
  misc_feature 22^23: note = Phosphorothioate bond
  modified_base 23: mod_base = gm
ttgttatttatcaggagtgactg

SEQ ID NO: 835 - RNA, 23 nt, synthetic construct
  source 1..23: mol_type = other RNA
  modified_base 1: mod_base = cm
  misc_feature 1^2: note = Phosphorothioate bond
  modified_base 2: mod_base = OTHER; note = 2'-Fluoro-adenosine
  misc_feature 2^3: note = Phosphorothioate bond
  modified_base 3: mod_base = gm
  modified_base 4: mod_base = um
  modified_base 5: mod_base = cm
  modified_base 6: mod_base = OTHER; note = 2'-Fluoro-uridine
  modified_base 7: mod_base = OTHER; note = 2'-O-methyl-adenosine
  modified_base 8: mod_base = um
  modified_base 9: mod_base = OTHER; note = 2'-O-methyl-adenosine
  modified_base 10: mod_base = OTHER; note = 2'-O-methyl-adenosine
  modified_base 11: mod_base = um
  modified_base 12: mod_base = gm
  modified_base 13: mod_base = cm
  modified_base 14: mod_base = OTHER; note = 2'-Fluoro-cytidine
  modified_base 15: mod_base = um
  modified_base 16: mod_base = OTHER; note = 2'-Fluoro-uridine
  modified_base 17: mod_base = um
  modified_base 18: mod_base = OTHER; note = 2'-Fluoro-guanosine
  modified_base 19: mod_base = um
  modified_base 20: mod_base = OTHER; note = 2'-O-methyl-adenosine
  modified_base 21: mod_base = um
  misc_feature 21^22: note = Phosphorothioate bond
  modified_base 22: mod_base = um
  misc_feature 22^23: note = Phosphorothioate bond
  modified_base 23: mod_base = gm
cagtctataatgcctttgtattg

SEQ ID NO: 836 - RNA, 23 nt, synthetic construct
  source 1..23: mol_type = other RNA
  modified_base 1: mod_base = OTHER; note = 2'-O-methyl-adenosine
  misc_feature 1^2: note = Phosphorothioate bond
  modified_base 2: mod_base = OTHER; note = 2'-Fluoro-uridine
  misc_feature 2^3: note = Phosphorothioate bond
  modified_base 3: mod_base = OTHER; note = 2'-O-methyl-adenosine
  modified_base 4: mod_base = gm
  modified_base 5: mod_base = OTHER; note = 2'-O-methyl-adenosine
  modified_base 6: mod_base = OTHER; note = 2'-Fluoro-uridine
  modified_base 7: mod_base = OTHER; note = 2'-O-methyl-adenosine
  modified_base 8: mod_base = cm
  modified_base 9: mod_base = cm
  modified_base 10: mod_base = gm
  modified_base 11: mod_base = OTHER; note = 2'-O-methyl-adenosine
  modified_base 12: mod_base = OTHER; note = 2'-O-methyl-adenosine
  modified_base 13: mod_base = gm
  modified_base 14: mod_base = OTHER; note = 2'-Fluoro-uridine
  modified_base 15: mod_base = OTHER; note = 2'-O-methyl-adenosine
  modified_base 16: mod_base = OTHER; note = 2'-Fluoro-guanosine
  modified_base 17: mod_base = gm
  modified_base 18: mod_base = OTHER; note = 2'-Fluoro-cytidine
  modified_base 19: mod_base = gm
  modified_base 20: mod_base = gm
  modified_base 21: mod_base = cm
  misc_feature 21^22: note = Phosphorothioate bond
  modified_base 22: mod_base = um
  misc_feature 22^23: note = Phosphorothioate bond
  modified_base 23: mod_base = cm
atagataccgaagtaggcggctc

SEQ ID NO: 837 - RNA, 23 nt, synthetic construct
  source 1..23: mol_type = other RNA
  modified_base 1: mod_base = um
  misc_feature 1^2: note = Phosphorothioate bond
  modified_base 2: mod_base = OTHER; note = 2'-Fluoro-adenosine
  misc_feature 2^3: note = Phosphorothioate bond
  modified_base 3: mod_base = gm
  modified_base 4: mod_base = OTHER; note = 2'-O-methyl-adenosine
  modified_base 5: mod_base = um
  modified_base 6: mod_base = OTHER; note = 2'-Fluoro-adenosine
  modified_base 7: mod_base = cm
  modified_base 8: mod_base = cm
  modified_base 9: mod_base = gm
  modified_base 10: mod_base = OTHER; note = 2'-O-methyl-adenosine
  modified_base 11: mod_base = OTHER; note = 2'-O-methyl-adenosine
  modified_base 12: mod_base = gm
  modified_base 13: mod_base = um
  modified_base 14: mod_base = OTHER; note = 2'-Fluoro-adenosine
  modified_base 15: mod_base = gm
  modified_base 16: mod_base = OTHER; note = 2'-Fluoro-guanosine
  modified_base 17: mod_base = cm
  modified_base 18: mod_base = OTHER; note = 2'-Fluoro-guanosine
  modified_base 19: mod_base = gm
  modified_base 20: mod_base = cm
  modified_base 21: mod_base = um
  misc_feature 21^22: note = Phosphorothioate bond
  modified_base 22: mod_base = cm
  misc_feature 22^23: note = Phosphorothioate bond
  modified_base 23: mod_base = gm
tagataccgaagtaggcggctcg

SEQ ID NO: 838 - RNA, 23 nt, synthetic construct
  source 1..23: mol_type = other RNA
  modified_base 1: mod_base = gm
  misc_feature 1^2: note = Phosphorothioate bond
  modified_base 2: mod_base = OTHER; note = 2'-Fluoro-guanosine
  misc_feature 2^3: note = Phosphorothioate bond
  modified_base 3: mod_base = OTHER; note = 2'-O-methyl-adenosine
  modified_base 4: mod_base = OTHER; note = 2'-O-methyl-adenosine
  modified_base 5: mod_base = um
  modified_base 6: mod_base = OTHER; note = 2'-Fluoro-adenosine
  modified_base 7: mod_base = cm
  modified_base 8: mod_base = gm
  modified_base 9: mod_base = gm
  modified_base 10: mod_base = OTHER; note = 2'-O-methyl-adenosine
  modified_base 11: mod_base = cm
  modified_base 12: mod_base = cm
  modified_base 13: mod_base = OTHER; note = 2'-O-methyl-adenosine
  modified_base 14: mod_base = OTHER; note = 2'-Fluoro-cytidine
  modified_base 15: mod_base = gm
  modified_base 16: mod_base = OTHER; note = 2'-Fluoro-cytidine
  modified_base 17: mod_base = OTHER; note = 2'-O-methyl-adenosine
  modified_base 18: mod_base = OTHER; note = 2'-Fluoro-guanosine
  modified_base 19: mod_base = um
  modified_base 20: mod_base = cm
  modified_base 21: mod_base = um
  misc_feature 21^22: note = Phosphorothioate bond
  modified_base 22: mod_base = OTHER; note = 2'-O-methyl-adenosine
  misc_feature 22^23: note = Phosphorothioate bond
  modified_base 23: mod_base = um
ggaatacggaccacgcagtctat

SEQ ID NO: 839 - RNA, 23 nt, synthetic construct
  source 1..23: mol_type = other RNA
  modified_base 1: mod_base = cm
  misc_feature 1^2: note = Phosphorothioate bond
  modified_base 2: mod_base = OTHER; note = 2'-Fluoro-adenosine
  misc_feature 2^3: note = Phosphorothioate bond
  modified_base 3: mod_base = gm
  modified_base 4: mod_base = cm
  modified_base 5: mod_base = um
  modified_base 6: mod_base = OTHER; note = 2'-Fluoro-guanosine
  modified_base 7: mod_base = OTHER; note = 2'-O-methyl-adenosine
  modified_base 8: mod_base = um
  modified_base 9: mod_base = gm
  modified_base 10: mod_base = OTHER; note = 2'-O-methyl-adenosine
  modified_base 11: mod_base = cm
  modified_base 12: mod_base = gm
  modified_base 13: mod_base = OTHER; note = 2'-O-methyl-adenosine
  modified_base 14: mod_base = OTHER; note = 2'-Fluoro-uridine
  modified_base 15: mod_base = gm
  modified_base 16: mod_base = OTHER; note = 2'-Fluoro-uridine
  modified_base 17: mod_base = gm
  modified_base 18: mod_base = OTHER; note = 2'-Fluoro-adenosine
  modified_base 19: mod_base = gm
  modified_base 20: mod_base = um
  modified_base 21: mod_base = gm
  misc_feature 21^22: note = Phosphorothioate bond
  modified_base 22: mod_base = um
  misc_feature 22^23: note = Phosphorothioate bond
  modified_base 23: mod_base = um
cagctgatgacgatgtgagtgtt

SEQ ID NO: 840 - RNA, 23 nt, synthetic construct
  source 1..23: mol_type = other RNA
  modified_base 1: mod_base = OTHER; note = 2'-O-methyl-adenosine
  misc_feature 1^2: note = Phosphorothioate bond
  modified_base 2: mod_base = OTHER; note = 2'-Fluoro-uridine
  misc_feature 2^3: note = Phosphorothioate bond
  modified_base 3: mod_base = um
  modified_base 4: mod_base = um
  modified_base 5: mod_base = OTHER; note = 2'-O-methyl-adenosine
  modified_base 6: mod_base = OTHER; note = 2'-Fluoro-uridine
  modified_base 7: mod_base = cm
  modified_base 8: mod_base = um
  modified_base 9: mod_base = um
  modified_base 10: mod_base = um
  modified_base 11: mod_base = gm
  modified_base 12: mod_base = OTHER; note = 2'-O-methyl-adenosine
  modified_base 13: mod_base = OTHER; note = 2'-O-methyl-adenosine
  modified_base 14: mod_base = OTHER; note = 2'-Fluoro-guanosine
  modified_base 15: mod_base = gm
  modified_base 16: mod_base = OTHER; note = 2'-Fluoro-cytidine
  modified_base 17: mod_base = gm
  modified_base 18: mod_base = OTHER; note = 2'-Fluoro-adenosine
  modified_base 19: mod_base = OTHER; note = 2'-O-methyl-adenosine
  modified_base 20: mod_base = gm
  modified_base 21: mod_base = um
  misc_feature 21^22: note = Phosphorothioate bond
  modified_base 22: mod_base = um
  misc_feature 22^23: note = Phosphorothioate bond
  modified_base 23: mod_base = OTHER; note = 2'-O-methyl-adenosine
atttatctttgaaggcgaagtta

SEQ ID NO: 841 - RNA, 23 nt, synthetic construct
  source 1..23: mol_type = other RNA
  modified_base 1: mod_base = gm
  misc_feature 1^2: note = Phosphorothioate bond
  modified_base 2: mod_base = OTHER; note = 2'-Fluoro-uridine
  misc_feature 2^3: note = Phosphorothioate bond
  modified_base 3: mod_base = gm
  modified_base 4: mod_base = um
  modified_base 5: mod_base = cm
  modified_base 6: mod_base = OTHER; note = 2'-Fluoro-adenosine
  modified_base 7: mod_base = um
  modified_base 8: mod_base = OTHER; note = 2'-O-methyl-adenosine
  modified_base 9: mod_base = gm
  modified_base 10: mod_base = OTHER; note = 2'-O-methyl-adenosine
  modified_base 11: mod_base = um
  modified_base 12: mod_base = OTHER; note = 2'-O-methyl-adenosine
  modified_base 13: mod_base = cm
  modified_base 14: mod_base = OTHER; note = 2'-Fluoro-cytidine
  modified_base 15: mod_base = gm
  modified_base 16: mod_base = OTHER; note = 2'-Fluoro-adenosine
  modified_base 17: mod_base = OTHER; note = 2'-O-methyl-adenosine
  modified_base 18: mod_base = OTHER; note = 2'-Fluoro-guanosine
  modified_base 19: mod_base = um
  modified_base 20: mod_base = OTHER; note = 2'-O-methyl-adenosine
  modified_base 21: mod_base = gm
  misc_feature 21^22: note = Phosphorothioate bond
  modified_base 22: mod_base = gm
  misc_feature 22^23: note = Phosphorothioate bond
  modified_base 23: mod_base = cm
gtgtcatagataccgaagtaggc

SEQ ID NO: 842 - RNA, 23 nt, synthetic construct
  source 1..23: mol_type = other RNA
  modified_base 1: mod_base = um
  misc_feature 1^2: note = Phosphorothioate bond
  modified_base 2: mod_base = OTHER; note = 2'-Fluoro-uridine
  misc_feature 2^3: note = Phosphorothioate bond
  modified_base 3: mod_base = cm
  modified_base 4: mod_base = cm
  modified_base 5: mod_base = cm
  modified_base 6: mod_base = OTHER; note = 2'-Fluoro-adenosine
  modified_base 7: mod_base = um
  modified_base 8: mod_base = um
  modified_base 9: mod_base = um
  modified_base 10: mod_base = um
  modified_base 11: mod_base = cm
  modified_base 12: mod_base = OTHER; note = 2'-O-methyl-adenosine
  modified_base 13: mod_base = OTHER; note = 2'-O-methyl-adenosine
  modified_base 14: mod_base = OTHER; note = 2'-Fluoro-cytidine
  modified_base 15: mod_base = cm
  modified_base 16: mod_base = OTHER; note = 2'-Fluoro-adenosine
  modified_base 17: mod_base = gm
  modified_base 18: mod_base = OTHER; note = 2'-Fluoro-uridine
  modified_base 19: mod_base = OTHER; note = 2'-O-methyl-adenosine
  modified_base 20: mod_base = OTHER; note = 2'-O-methyl-adenosine
  modified_base 21: mod_base = OTHER; note = 2'-O-methyl-adenosine
  misc_feature 21^22: note = Phosphorothioate bond
  modified_base 22: mod_base = um
  misc_feature 22^23: note = Phosphorothioate bond
  modified_base 23: mod_base = OTHER; note = 2'-O-methyl-adenosine
ttcccattttcaaccagtaaata

SEQ ID NO: 843 - RNA, 23 nt, synthetic construct
  source 1..23: mol_type = other RNA
  modified_base 1: mod_base = gm
  misc_feature 1^2: note = Phosphorothioate bond
  modified_base 2: mod_base = OTHER; note = 2'-Fluoro-cytidine
  misc_feature 2^3: note = Phosphorothioate bond
  modified_base 3: mod_base = um
  modified_base 4: mod_base = gm
  modified_base 5: mod_base = cm
  modified_base 6: mod_base = OTHER; note = 2'-Fluoro-uridine
  modified_base 7: mod_base = OTHER; note = 2'-O-methyl-adenosine
  modified_base 8: mod_base = gm
  modified_base 9: mod_base = OTHER; note = 2'-O-methyl-adenosine
  modified_base 10: mod_base = cm
  modified_base 11: mod_base = gm
  modified_base 12: mod_base = gm
  modified_base 13: mod_base = gm
  modified_base 14: mod_base = OTHER; note = 2'-Fluoro-uridine
  modified_base 15: mod_base = OTHER; note = 2'-O-methyl-adenosine
  modified_base 16: mod_base = OTHER; note = 2'-Fluoro-cytidine
  modified_base 17: mod_base = gm
  modified_base 18: mod_base = OTHER; note = 2'-Fluoro-guanosine
  modified_base 19: mod_base = gm
  modified_base 20: mod_base = cm
  modified_base 21: mod_base = OTHER; note = 2'-O-methyl-adenosine
  misc_feature 21^22: note = Phosphorothioate bond
  modified_base 22: mod_base = OTHER; note = 2'-O-methyl-adenosine
  misc_feature 22^23: note = Phosphorothioate bond
  modified_base 23: mod_base = OTHER; note = 2'-O-methyl-adenosine
gctgctagacgggtacgggcaaa

SEQ ID NO: 844 - RNA, 23 nt, synthetic construct
  source 1..23: mol_type = other RNA
  modified_base 1: mod_base = cm
  misc_feature 1^2: note = Phosphorothioate bond
  modified_base 2: mod_base = OTHER; note = 2'-Fluoro-adenosine
  misc_feature 2^3: note = Phosphorothioate bond
  modified_base 3: mod_base = gm
  modified_base 4: mod_base = um
  modified_base 5: mod_base = um
  modified_base 6: mod_base = OTHER; note = 2'-Fluoro-cytidine
  modified_base 7: mod_base = cm
  modified_base 8: mod_base = um
  modified_base 9: mod_base = um
  modified_base 10: mod_base = um
  modified_base 11: mod_base = gm
  modified_base 12: mod_base = cm
  modified_base 13: mod_base = gm
  modified_base 14: mod_base = OTHER; note = 2'-Fluoro-cytidine
  modified_base 15: mod_base = cm
  modified_base 16: mod_base = OTHER; note = 2'-Fluoro-cytidine
  modified_base 17: mod_base = um
  modified_base 18: mod_base = OTHER; note = 2'-Fluoro-guanosine
  modified_base 19: mod_base = OTHER; note = 2'-O-methyl-adenosine
  modified_base 20: mod_base = cm
  modified_base 21: mod_base = um
  misc_feature 21^22: note = Phosphorothioate bond
  modified_base 22: mod_base = gm
  misc_feature 22^23: note = Phosphorothioate bond
  modified_base 23: mod_base = cm
cagttcctttgcgccctgactgc

SEQ ID NO: 845 - RNA, 23 nt, synthetic construct
  source 1..23: mol_type = other RNA
  modified_base 1: mod_base = cm
  misc_feature 1^2: note = Phosphorothioate bond
  modified_base 2: mod_base = OTHER; note = 2'-Fluoro-uridine
  misc_feature 2^3: note = Phosphorothioate bond
  modified_base 3: mod_base = um
  modified_base 4: mod_base = cm
  modified_base 5: mod_base = cm
  modified_base 6: mod_base = OTHER; note = 2'-Fluoro-cytidine
  modified_base 7: mod_base = OTHER; note = 2'-O-methyl-adenosine
  modified_base 8: mod_base = um
  modified_base 9: mod_base = um
  modified_base 10: mod_base = um
  modified_base 11: mod_base = um
  modified_base 12: mod_base = cm
  modified_base 13: mod_base = OTHER; note = 2'-O-methyl-adenosine
  modified_base 14: mod_base = OTHER; note = 2'-Fluoro-adenosine
  modified_base 15: mod_base = cm
  modified_base 16: mod_base = OTHER; note = 2'-Fluoro-cytidine
  modified_base 17: mod_base = OTHER; note = 2'-O-methyl-adenosine
  modified_base 18: mod_base = OTHER; note = 2'-Fluoro-guanosine
  modified_base 19: mod_base = um
  modified_base 20: mod_base = OTHER; note = 2'-O-methyl-adenosine
  modified_base 21: mod_base = OTHER; note = 2'-O-methyl-adenosine
  misc_feature 21^22: note = Phosphorothioate bond
  modified_base 22: mod_base = OTHER; note = 2'-O-methyl-adenosine
  misc_feature 22^23: note = Phosphorothioate bond
  modified_base 23: mod_base = um
cttcccattttcaaccagtaaat

SEQ ID NO: 846 - RNA, 23 nt, synthetic construct
  source 1..23: mol_type = other RNA
  modified_base 1: mod_base = OTHER; note = 2'-O-methyl-adenosine
  misc_feature 1^2: note = Phosphorothioate bond
  modified_base 2: mod_base = OTHER; note = 2'-Fluoro-guanosine
  misc_feature 2^3: note = Phosphorothioate bond
  modified_base 3: mod_base = OTHER; note = 2'-O-methyl-adenosine
  modified_base 4: mod_base = um
  modified_base 5: mod_base = OTHER; note = 2'-O-methyl-adenosine
  modified_base 6: mod_base = OTHER; note = 2'-Fluoro-cytidine
  modified_base 7: mod_base = cm
  modified_base 8: mod_base = gm
  modified_base 9: mod_base = OTHER; note = 2'-O-methyl-adenosine
  modified_base 10: mod_base = OTHER; note = 2'-O-methyl-adenosine
  modified_base 11: mod_base = gm
  modified_base 12: mod_base = um
  modified_base 13: mod_base = OTHER; note = 2'-O-methyl-adenosine
  modified_base 14: mod_base = OTHER; note = 2'-Fluoro-guanosine
  modified_base 15: mod_base = gm
  modified_base 16: mod_base = OTHER; note = 2'-Fluoro-cytidine
  modified_base 17: mod_base = gm
  modified_base 18: mod_base = OTHER; note = 2'-Fluoro-guanosine
  modified_base 19: mod_base = cm
  modified_base 20: mod_base = um
  modified_base 21: mod_base = cm
  misc_feature 21^22: note = Phosphorothioate bond
  modified_base 22: mod_base = gm
  misc_feature 22^23: note = Phosphorothioate bond
  modified_base 23: mod_base = gm
agataccgaagtaggcggctcgg

SEQ ID NO: 847 - RNA, 23 nt, synthetic construct
  source 1..23: mol_type = other RNA
  modified_base 1: mod_base = um
  misc_feature 1^2: note = Phosphorothioate bond
  modified_base 2: mod_base = OTHER; note = 2'-Fluoro-uridine
  misc_feature 2^3: note = Phosphorothioate bond
  modified_base 3: mod_base = OTHER; note = 2'-O-methyl-adenosine
  modified_base 4: mod_base = OTHER; note = 2'-O-methyl-adenosine
  modified_base 5: mod_base = cm
  modified_base 6: mod_base = OTHER; note = 2'-Fluoro-cytidine
  modified_base 7: mod_base = OTHER; note = 2'-O-methyl-adenosine
  modified_base 8: mod_base = gm
  modified_base 9: mod_base = gm
  modified_base 10: mod_base = cm
  modified_base 11: mod_base = OTHER; note = 2'-O-methyl-adenosine
  modified_base 12: mod_base = gm
  modified_base 13: mod_base = um
  modified_base 14: mod_base = OTHER; note = 2'-Fluoro-cytidine
  modified_base 15: mod_base = OTHER; note = 2'-O-methyl-adenosine
  modified_base 16: mod_base = OTHER; note = 2'-Fluoro-cytidine
  modified_base 17: mod_base = cm
  modified_base 18: mod_base = OTHER; note = 2'-Fluoro-guanosine
  modified_base 19: mod_base = OTHER; note = 2'-O-methyl-adenosine
  modified_base 20: mod_base = gm
  modified_base 21: mod_base = gm
  misc_feature 21^22: note = Phosphorothioate bond
  modified_base 22: mod_base = cm
  misc_feature 22^23: note = Phosphorothioate bond
  modified_base 23: mod_base = cm
ttaaccaggcagtcaccgaggcc

SEQ ID NO: 848 - RNA, 23 nt, synthetic construct
  source 1..23: mol_type = other RNA
  modified_base 1: mod_base = OTHER; note = 2'-O-methyl-adenosine
  misc_feature 1^2: note = Phosphorothioate bond
  modified_base 2: mod_base = OTHER; note = 2'-Fluoro-uridine
  misc_feature 2^3: note = Phosphorothioate bond
  modified_base 3: mod_base = cm
  modified_base 4: mod_base = OTHER; note = 2'-O-methyl-adenosine
  modified_base 5: mod_base = um
  modified_base 6: mod_base = OTHER; note = 2'-Fluoro-cytidine
  modified_base 7: mod_base = cm
  modified_base 8: mod_base = OTHER; note = 2'-O-methyl-adenosine
  modified_base 9: mod_base = gm
  modified_base 10: mod_base = cm
  modified_base 11: mod_base = um
  modified_base 12: mod_base = gm
  modified_base 13: mod_base = OTHER; note = 2'-O-methyl-adenosine
  modified_base 14: mod_base = OTHER; note = 2'-Fluoro-uridine
  modified_base 15: mod_base = gm
  modified_base 16: mod_base = OTHER; note = 2'-Fluoro-adenosine
  modified_base 17: mod_base = cm
  modified_base 18: mod_base = OTHER; note = 2'-Fluoro-guanosine
  modified_base 19: mod_base = OTHER; note = 2'-O-methyl-adenosine
  modified_base 20: mod_base = um
  modified_base 21: mod_base = gm
  misc_feature 21^22: note = Phosphorothioate bond
  modified_base 22: mod_base = um
  misc_feature 22^23: note = Phosphorothioate bond
  modified_base 23: mod_base = gm
atcatccagctgatgacgatgtg

SEQ ID NO: 849 - RNA, 23 nt, synthetic construct
  source 1..23: mol_type = other RNA
  modified_base 1: mod_base = OTHER; note = 2'-O-methyl-adenosine
  misc_feature 1^2: note = Phosphorothioate bond
  modified_base 2: mod_base = OTHER; note = 2'-Fluoro-uridine
  misc_feature 2^3: note = Phosphorothioate bond
  modified_base 3: mod_base = um
  modified_base 4: mod_base = um
  modified_base 5: mod_base = OTHER; note = 2'-O-methyl-adenosine
  modified_base 6: mod_base = OTHER; note = 2'-Fluoro-uridine
  modified_base 7: mod_base = cm
  modified_base 8: mod_base = OTHER; note = 2'-O-methyl-adenosine
  modified_base 9: mod_base = gm
  modified_base 10: mod_base = gm
  modified_base 11: mod_base = OTHER; note = 2'-O-methyl-adenosine
  modified_base 12: mod_base = gm
  modified_base 13: mod_base = um
  modified_base 14: mod_base = OTHER; note = 2'-Fluoro-guanosine
  modified_base 15: mod_base = OTHER; note = 2'-O-methyl-adenosine
  modified_base 16: mod_base = OTHER; note = 2'-Fluoro-cytidine
  modified_base 17: mod_base = um
  modified_base 18: mod_base = OTHER; note = 2'-Fluoro-guanosine
  modified_base 19: mod_base = OTHER; note = 2'-O-methyl-adenosine
  modified_base 20: mod_base = OTHER; note = 2'-O-methyl-adenosine
  modified_base 21: mod_base = OTHER; note = 2'-O-methyl-adenosine
  misc_feature 21^22: note = Phosphorothioate bond
  modified_base 22: mod_base = um
  misc_feature 22^23: note = Phosphorothioate bond
  modified_base 23: mod_base = OTHER; note = 2'-O-methyl-adenosine
atttatcaggagtgactgaaata

SEQ ID NO: 850 - RNA, 23 nt, synthetic construct
  source 1..23: mol_type = other RNA
  modified_base 1: mod_base = gm
  misc_feature 1^2: note = Phosphorothioate bond
  modified_base 2: mod_base = OTHER; note = 2'-Fluoro-adenosine
  misc_feature 2^3: note = Phosphorothioate bond
  modified_base 3: mod_base = cm
  modified_base 4: mod_base = OTHER; note = 2'-O-methyl-adenosine
  modified_base 5: mod_base = gm
  modified_base 6: mod_base = OTHER; note = 2'-Fluoro-uridine
  modified_base 7: mod_base = cm
  modified_base 8: mod_base = um
  modified_base 9: mod_base = gm
  modified_base 10: mod_base = um
  modified_base 11: mod_base = gm
  modified_base 12: mod_base = cm
  modified_base 13: mod_base = gm
  modified_base 14: mod_base = OTHER; note = 2'-Fluoro-adenosine
  modified_base 15: mod_base = um
  modified_base 16: mod_base = OTHER; note = 2'-Fluoro-cytidine
  modified_base 17: mod_base = OTHER; note = 2'-O-methyl-adenosine
  modified_base 18: mod_base = OTHER; note = 2'-Fluoro-uridine
  modified_base 19: mod_base = cm
  modified_base 20: mod_base = cm
  modified_base 21: mod_base = OTHER; note = 2'-O-methyl-adenosine
  misc_feature 21^22: note = Phosphorothioate bond
  modified_base 22: mod_base = gm
  misc_feature 22^23: note = Phosphorothioate bond
  modified_base 23: mod_base = cm
gacagtctgtgcgatcatccagc

SEQ ID NO: 851 - RNA, 23 nt, synthetic construct
  source 1..23: mol_type = other RNA
  modified_base 1: mod_base = um
  misc_feature 1^2: note = Phosphorothioate bond
  modified_base 2: mod_base = OTHER; note = 2'-Fluoro-cytidine
  misc_feature 2^3: note = Phosphorothioate bond
  modified_base 3: mod_base = um
  modified_base 4: mod_base = OTHER; note = 2'-O-methyl-adenosine
  modified_base 5: mod_base = um
  modified_base 6: mod_base = OTHER; note = 2'-Fluoro-adenosine
  modified_base 7: mod_base = OTHER; note = 2'-O-methyl-adenosine
  modified_base 8: mod_base = um
  modified_base 9: mod_base = gm
  modified_base 10: mod_base = cm
  modified_base 11: mod_base = cm
  modified_base 12: mod_base = um
  modified_base 13: mod_base = um
  modified_base 14: mod_base = OTHER; note = 2'-Fluoro-uridine
  modified_base 15: mod_base = gm
  modified_base 16: mod_base = OTHER; note = 2'-Fluoro-uridine
  modified_base 17: mod_base = OTHER; note = 2'-O-methyl-adenosine
  modified_base 18: mod_base = OTHER; note = 2'-Fluoro-uridine
  modified_base 19: mod_base = um
  modified_base 20: mod_base = gm
  modified_base 21: mod_base = cm
  misc_feature 21^22: note = Phosphorothioate bond
  modified_base 22: mod_base = um
  misc_feature 22^23: note = Phosphorothioate bond
  modified_base 23: mod_base = um
tctataatgcctttgtattgctt

SEQ ID NO: 852 - RNA, 23 nt, synthetic construct
  source 1..23: mol_type = other RNA
  modified_base 1: mod_base = um
  misc_feature 1^2: note = Phosphorothioate bond
  modified_base 2: mod_base = OTHER; note = 2'-Fluoro-adenosine
  misc_feature 2^3: note = Phosphorothioate bond
  modified_base 3: mod_base = OTHER; note = 2'-O-methyl-adenosine
  modified_base 4: mod_base = cm
  modified_base 5: mod_base = cm
  modified_base 6: mod_base = OTHER; note = 2'-Fluoro-adenosine
  modified_base 7: mod_base = gm
  modified_base 8: mod_base = gm
  modified_base 9: mod_base = cm
  modified_base 10: mod_base = OTHER; note = 2'-O-methyl-adenosine
  modified_base 11: mod_base = gm
  modified_base 12: mod_base = um
  modified_base 13: mod_base = cm
  modified_base 14: mod_base = OTHER; note = 2'-Fluoro-adenosine
  modified_base 15: mod_base = cm
  modified_base 16: mod_base = OTHER; note = 2'-Fluoro-cytidine
  modified_base 17: mod_base = gm
  modified_base 18: mod_base = OTHER; note = 2'-Fluoro-adenosine
  modified_base 19: mod_base = gm
  modified_base 20: mod_base = gm
  modified_base 21: mod_base = cm
  misc_feature 21^22: note = Phosphorothioate bond
  modified_base 22: mod_base = cm
  misc_feature 22^23: note = Phosphorothioate bond
  modified_base 23: mod_base = um
taaccaggcagtcaccgaggcct

SEQ ID NO: 853 - RNA, 23 nt, synthetic construct
  source 1..23: mol_type = other RNA
  modified_base 1: mod_base = cm
  misc_feature 1^2: note = Phosphorothioate bond
  modified_base 2: mod_base = OTHER; note = 2'-Fluoro-cytidine
  misc_feature 2^3: note = Phosphorothioate bond
  modified_base 3: mod_base = cm
  modified_base 4: mod_base = um
  modified_base 5: mod_base = gm
  modified_base 6: mod_base = OTHER; note = 2'-Fluoro-cytidine
  modified_base 7: mod_base = OTHER; note = 2'-O-methyl-adenosine
  modified_base 8: mod_base = cm
  modified_base 9: mod_base = OTHER; note = 2'-O-methyl-adenosine
  modified_base 10: mod_base = gm
  modified_base 11: mod_base = OTHER; note = 2'-O-methyl-adenosine
  modified_base 12: mod_base = cm
  modified_base 13: mod_base = OTHER; note = 2'-O-methyl-adenosine
  modified_base 14: mod_base = OTHER; note = 2'-Fluoro-cytidine
  modified_base 15: mod_base = gm
  modified_base 16: mod_base = OTHER; note = 2'-Fluoro-uridine
  modified_base 17: mod_base = um
  modified_base 18: mod_base = OTHER; note = 2'-Fluoro-adenosine
  modified_base 19: mod_base = OTHER; note = 2'-O-methyl-adenosine
  modified_base 20: mod_base = OTHER; note = 2'-O-methyl-adenosine
  modified_base 21: mod_base = gm
  misc_feature 21^22: note = Phosphorothioate bond
  modified_base 22: mod_base = cm
  misc_feature 22^23: note = Phosphorothioate bond
  modified_base 23: mod_base = cm
ccctgcacagacacgttaaagcc

SEQ ID NO: 854 - RNA, 23 nt, synthetic construct
  source 1..23: mol_type = other RNA
  modified_base 1: mod_base = cm
  misc_feature 1^2: note = Phosphorothioate bond
  modified_base 2: mod_base = OTHER; note = 2'-Fluoro-adenosine
  misc_feature 2^3: note = Phosphorothioate bond
  modified_base 3: mod_base = cm
  modified_base 4: mod_base = gm
  modified_base 5: mod_base = cm
  modified_base 6: mod_base = OTHER; note = 2'-Fluoro-adenosine
  modified_base 7: mod_base = gm
  modified_base 8: mod_base = um
  modified_base 9: mod_base = cm
  modified_base 10: mod_base = um
  modified_base 11: mod_base = OTHER; note = 2'-O-methyl-adenosine
  modified_base 12: mod_base = um
  modified_base 13: mod_base = OTHER; note = 2'-O-methyl-adenosine
  modified_base 14: mod_base = OTHER; note = 2'-Fluoro-adenosine
  modified_base 15: mod_base = um
  modified_base 16: mod_base = OTHER; note = 2'-Fluoro-guanosine
  modified_base 17: mod_base = cm
  modified_base 18: mod_base = OTHER; note = 2'-Fluoro-cytidine
  modified_base 19: mod_base = um
  modified_base 20: mod_base = um
  modified_base 21: mod_base = um
  misc_feature 21^22: note = Phosphorothioate bond
  modified_base 22: mod_base = gm
  misc_feature 22^23: note = Phosphorothioate bond
  modified_base 23: mod_base = um
cacgcagtctataatgcctttgt

SEQ ID NO: 855 - RNA, 23 nt, synthetic construct
  source 1..23: mol_type = other RNA
  modified_base 1: mod_base = um
  misc_feature 1^2: note = Phosphorothioate bond
  modified_base 2: mod_base = OTHER; note = 2'-Fluoro-adenosine
  misc_feature 2^3: note = Phosphorothioate bond
  modified_base 3: mod_base = OTHER; note = 2'-O-methyl-adenosine
  modified_base 4: mod_base = um
  modified_base 5: mod_base = OTHER; note = 2'-O-methyl-adenosine
  modified_base 6: mod_base = OTHER; note = 2'-Fluoro-cytidine
  modified_base 7: mod_base = OTHER; note = 2'-O-methyl-adenosine
  modified_base 8: mod_base = OTHER; note = 2'-O-methyl-adenosine
  modified_base 9: mod_base = cm
  modified_base 10: mod_base = OTHER; note = 2'-O-methyl-adenosine
  modified_base 11: mod_base = um
  modified_base 12: mod_base = gm
  modified_base 13: mod_base = cm
  modified_base 14: mod_base = OTHER; note = 2'-Fluoro-cytidine
  modified_base 15: mod_base = um
  modified_base 16: mod_base = OTHER; note = 2'-Fluoro-guanosine
  modified_base 17: mod_base = um
  modified_base 18: mod_base = OTHER; note = 2'-Fluoro-uridine
  modified_base 19: mod_base = cm
  modified_base 20: mod_base = OTHER; note = 2'-O-methyl-adenosine
  modified_base 21: mod_base = cm
  misc_feature 21^22: note = Phosphorothioate bond
  modified_base 22: mod_base = OTHER; note = 2'-O-methyl-adenosine
  misc_feature 22^23: note = Phosphorothioate bond
  modified_base 23: mod_base = gm
taatacaacatgcctgttcacag

SEQ ID NO: 856 - RNA, 23 nt, synthetic construct
  source 1..23: mol_type = other RNA
  modified_base 1: mod_base = um
  misc_feature 1^2: note = Phosphorothioate bond
  modified_base 2: mod_base = OTHER; note = 2'-Fluoro-uridine
  misc_feature 2^3: note = Phosphorothioate bond
  modified_base 3: mod_base = OTHER; note = 2'-O-methyl-adenosine
  modified_base 4: mod_base = OTHER; note = 2'-O-methyl-adenosine
  modified_base 5: mod_base = gm
  modified_base 6: mod_base = OTHER; note = 2'-Fluoro-adenosine
  modified_base 7: mod_base = gm
  modified_base 8: mod_base = OTHER; note = 2'-O-methyl-adenosine
  modified_base 9: mod_base = OTHER; note = 2'-O-methyl-adenosine
  modified_base 10: mod_base = OTHER; note = 2'-O-methyl-adenosine
  modified_base 11: mod_base = OTHER; note = 2'-O-methyl-adenosine
  modified_base 12: mod_base = cm
  modified_base 13: mod_base = um
  modified_base 14: mod_base = OTHER; note = 2'-Fluoro-guanosine
  modified_base 15: mod_base = gm
  modified_base 16: mod_base = OTHER; note = 2'-Fluoro-uridine
  modified_base 17: mod_base = cm
  modified_base 18: mod_base = OTHER; note = 2'-Fluoro-adenosine
  modified_base 19: mod_base = gm
  modified_base 20: mod_base = OTHER; note = 2'-O-methyl-adenosine
  modified_base 21: mod_base = um
  misc_feature 21^22: note = Phosphorothioate bond
  modified_base 22: mod_base = gm
  misc_feature 22^23: note = Phosphorothioate bond
  modified_base 23: mod_base = OTHER; note = 2'-O-methyl-adenosine
ttaagagaaaactggtcagatga

SEQ ID NO: 857 - RNA, 23 nt, synthetic construct
  source 1..23: mol_type = other RNA
  modified_base 1: mod_base = um
  misc_feature 1^2: note = Phosphorothioate bond
  modified_base 2: mod_base = OTHER; note = 2'-Fluoro-guanosine
  misc_feature 2^3: note = Phosphorothioate bond
  modified_base 3: mod_base = cm
  modified_base 4: mod_base = OTHER; note = 2'-O-methyl-adenosine
  modified_base 5: mod_base = cm
  modified_base 6: mod_base = OTHER; note = 2'-Fluoro-adenosine
  modified_base 7: mod_base = gm
  modified_base 8: mod_base = OTHER; note = 2'-O-methyl-adenosine
  modified_base 9: mod_base = cm
  modified_base 10: mod_base = OTHER; note = 2'-O-methyl-adenosine
  modified_base 11: mod_base = cm
  modified_base 12: mod_base = gm
  modified_base 13: mod_base = um
  modified_base 14: mod_base = OTHER; note = 2'-Fluoro-uridine
  modified_base 15: mod_base = OTHER; note = 2'-O-methyl-adenosine
  modified_base 16: mod_base = OTHER; note = 2'-Fluoro-adenosine
  modified_base 17: mod_base = OTHER; note = 2'-O-methyl-adenosine
  modified_base 18: mod_base = OTHER; note = 2'-Fluoro-guanosine
  modified_base 19: mod_base = cm
  modified_base 20: mod_base = cm
  modified_base 21: mod_base = um
  misc_feature 21^22: note = Phosphorothioate bond
  modified_base 22: mod_base = um
  misc_feature 22^23: note = Phosphorothioate bond
  modified_base 23: mod_base = gm
tgcacagacacgttaaagccttg

SEQ ID NO: 858 - RNA, 23 nt, synthetic construct
  source 1..23: mol_type = other RNA
  modified_base 1: mod_base = gm
  misc_feature 1^2: note = Phosphorothioate bond
  modified_base 2: mod_base = OTHER; note = 2'-Fluoro-uridine
  misc_feature 2^3: note = Phosphorothioate bond
  modified_base 3: mod_base = um
  modified_base 4: mod_base = cm
  modified_base 5: mod_base = cm
  modified_base 6: mod_base = OTHER; note = 2'-Fluoro-uridine
  modified_base 7: mod_base = um
  modified_base 8: mod_base = um
  modified_base 9: mod_base = gm
  modified_base 10: mod_base = cm
  modified_base 11: mod_base = gm
  modified_base 12: mod_base = cm
  modified_base 13: mod_base = cm
  modified_base 14: mod_base = OTHER; note = 2'-Fluoro-cytidine
  modified_base 15: mod_base = um
  modified_base 16: mod_base = OTHER; note = 2'-Fluoro-guanosine
  modified_base 17: mod_base = OTHER; note = 2'-O-methyl-adenosine
  modified_base 18: mod_base = OTHER; note = 2'-Fluoro-cytidine
  modified_base 19: mod_base = um
  modified_base 20: mod_base = gm
  modified_base 21: mod_base = cm
  misc_feature 21^22: note = Phosphorothioate bond
  modified_base 22: mod_base = OTHER; note = 2'-O-methyl-adenosine
  misc_feature 22^23: note = Phosphorothioate bond
  modified_base 23: mod_base = um
gttcctttgcgccctgactgcat

SEQ ID NO: 859 - RNA, 23 nt, synthetic construct
  source 1..23: mol_type = other RNA
  modified_base 1: mod_base = gm
  misc_feature 1^2: note = Phosphorothioate bond
  modified_base 2: mod_base = OTHER; note = 2'-Fluoro-uridine
  misc_feature 2^3: note = Phosphorothioate bond
  modified_base 3: mod_base = gm
  modified_base 4: mod_base = OTHER; note = 2'-O-methyl-adenosine
  modified_base 5: mod_base = cm
  modified_base 6: mod_base = OTHER; note = 2'-Fluoro-adenosine
  modified_base 7: mod_base = gm
  modified_base 8: mod_base = um
  modified_base 9: mod_base = cm
  modified_base 10: mod_base = um
  modified_base 11: mod_base = gm
  modified_base 12: mod_base = um
  modified_base 13: mod_base = gm
  modified_base 14: mod_base = OTHER; note = 2'-Fluoro-cytidine
  modified_base 15: mod_base = gm
  modified_base 16: mod_base = OTHER; note = 2'-Fluoro-adenosine
  modified_base 17: mod_base = um
  modified_base 18: mod_base = OTHER; note = 2'-Fluoro-cytidine
  modified_base 19: mod_base = OTHER; note = 2'-O-methyl-adenosine
  modified_base 20: mod_base = um
  modified_base 21: mod_base = cm
  misc_feature 21^22: note = Phosphorothioate bond
  modified_base 22: mod_base = cm
  misc_feature 22^23: note = Phosphorothioate bond
  modified_base 23: mod_base = OTHER; note = 2'-O-methyl-adenosine
gtgacagtctgtgcgatcatcca

SEQ ID NO: 860 - RNA, 23 nt, synthetic construct
  source 1..23: mol_type = other RNA
  modified_base 1: mod_base = OTHER; note = 2'-O-methyl-adenosine
  misc_feature 1^2: note = Phosphorothioate bond
  modified_base 2: mod_base = OTHER; note = 2'-Fluoro-cytidine
  misc_feature 2^3: note = Phosphorothioate bond
  modified_base 3: mod_base = cm
  modified_base 4: mod_base = OTHER; note = 2'-O-methyl-adenosine
  modified_base 5: mod_base = cm
  modified_base 6: mod_base = OTHER; note = 2'-Fluoro-guanosine
  modified_base 7: mod_base = cm
  modified_base 8: mod_base = OTHER; note = 2'-O-methyl-adenosine
  modified_base 9: mod_base = gm
  modified_base 10: mod_base = um
  modified_base 11: mod_base = cm
  modified_base 12: mod_base = um
  modified_base 13: mod_base = OTHER; note = 2'-O-methyl-adenosine
  modified_base 14: mod_base = OTHER; note = 2'-Fluoro-uridine
  modified_base 15: mod_base = OTHER; note = 2'-O-methyl-adenosine
  modified_base 16: mod_base = OTHER; note = 2'-Fluoro-adenosine
  modified_base 17: mod_base = um
  modified_base 18: mod_base = OTHER; note = 2'-Fluoro-guanosine
  modified_base 19: mod_base = cm
  modified_base 20: mod_base = cm
  modified_base 21: mod_base = um
  misc_feature 21^22: note = Phosphorothioate bond
  modified_base 22: mod_base = um
  misc_feature 22^23: note = Phosphorothioate bond
  modified_base 23: mod_base = um
accacgcagtctataatgccttt

SEQ ID NO: 861 - RNA, 23 nt, synthetic construct
  source 1..23: mol_type = other RNA
  modified_base 1: mod_base = cm
  misc_feature 1^2: note = Phosphorothioate bond
  modified_base 2: mod_base = OTHER; note = 2'-Fluoro-adenosine
  misc_feature 2^3: note = Phosphorothioate bond
  modified_base 3: mod_base = gm
  modified_base 4: mod_base = um
  modified_base 5: mod_base = gm
  modified_base 6: mod_base = OTHER; note = 2'-Fluoro-adenosine
  modified_base 7: mod_base = cm
  modified_base 8: mod_base = OTHER; note = 2'-O-methyl-adenosine
  modified_base 9: mod_base = gm
  modified_base 10: mod_base = um
  modified_base 11: mod_base = cm
  modified_base 12: mod_base = um
  modified_base 13: mod_base = gm
  modified_base 14: mod_base = OTHER; note = 2'-Fluoro-uridine
  modified_base 15: mod_base = gm
  modified_base 16: mod_base = OTHER; note = 2'-Fluoro-cytidine
  modified_base 17: mod_base = gm
  modified_base 18: mod_base = OTHER; note = 2'-Fluoro-adenosine
  modified_base 19: mod_base = um
  modified_base 20: mod_base = cm
  modified_base 21: mod_base = OTHER; note = 2'-O-methyl-adenosine
  misc_feature 21^22: note = Phosphorothioate bond
  modified_base 22: mod_base = um
  misc_feature 22^23: note = Phosphorothioate bond
  modified_base 23: mod_base = cm
cagtgacagtctgtgcgatcatc

SEQ ID NO: 862 - RNA, 23 nt, synthetic construct
  source 1..23: mol_type = other RNA
  modified_base 1: mod_base = um
  misc_feature 1^2: note = Phosphorothioate bond
  modified_base 2: mod_base = OTHER; note = 2'-Fluoro-uridine
  misc_feature 2^3: note = Phosphorothioate bond
  modified_base 3: mod_base = gm
  modified_base 4: mod_base = gm
  modified_base 5: mod_base = gm
  modified_base 6: mod_base = OTHER; note = 2'-Fluoro-adenosine
  modified_base 7: mod_base = OTHER; note = 2'-O-methyl-adenosine
  modified_base 8: mod_base = um
  modified_base 9: mod_base = OTHER; note = 2'-O-methyl-adenosine
  modified_base 10: mod_base = cm
  modified_base 11: mod_base = gm
  modified_base 12: mod_base = gm
  modified_base 13: mod_base = OTHER; note = 2'-O-methyl-adenosine
  modified_base 14: mod_base = OTHER; note = 2'-Fluoro-cytidine
  modified_base 15: mod_base = cm
  modified_base 16: mod_base = OTHER; note = 2'-Fluoro-adenosine
  modified_base 17: mod_base = cm
  modified_base 18: mod_base = OTHER; note = 2'-Fluoro-guanosine
  modified_base 19: mod_base = cm
  modified_base 20: mod_base = OTHER; note = 2'-O-methyl-adenosine
  modified_base 21: mod_base = gm
  misc_feature 21^22: note = Phosphorothioate bond
  modified_base 22: mod_base = um
  misc_feature 22^23: note = Phosphorothioate bond
  modified_base 23: mod_base = cm
ttgggaatacggaccacgcagtc

SEQ ID NO: 863 - RNA, 23 nt, synthetic construct
  source 1..23: mol_type = other RNA
  modified_base 1: mod_base = gm
  misc_feature 1^2: note = Phosphorothioate bond
  modified_base 2: mod_base = OTHER; note = 2'-Fluoro-uridine
  misc_feature 2^3: note = Phosphorothioate bond
  modified_base 3: mod_base = cm
  modified_base 4: mod_base = um
  modified_base 5: mod_base = OTHER; note = 2'-O-methyl-adenosine
  modified_base 6: mod_base = OTHER; note = 2'-Fluoro-uridine
  modified_base 7: mod_base = OTHER; note = 2'-O-methyl-adenosine
  modified_base 8: mod_base = OTHER; note = 2'-O-methyl-adenosine
  modified_base 9: mod_base = um
  modified_base 10: mod_base = gm
  modified_base 11: mod_base = cm
  modified_base 12: mod_base = cm
  modified_base 13: mod_base = um
  modified_base 14: mod_base = OTHER; note = 2'-Fluoro-uridine
  modified_base 15: mod_base = um
  modified_base 16: mod_base = OTHER; note = 2'-Fluoro-guanosine
  modified_base 17: mod_base = um
  modified_base 18: mod_base = OTHER; note = 2'-Fluoro-adenosine
  modified_base 19: mod_base = um
  modified_base 20: mod_base = um
  modified_base 21: mod_base = gm
  misc_feature 21^22: note = Phosphorothioate bond
  modified_base 22: mod_base = cm
  misc_feature 22^23: note = Phosphorothioate bond
  modified_base 23: mod_base = um
gtctataatgcctttgtattgct

SEQ ID NO: 864 - RNA, 23 nt, synthetic construct
  source 1..23: mol_type = other RNA
  modified_base 1: mod_base = um
  misc_feature 1^2: note = Phosphorothioate bond
  modified_base 2: mod_base = OTHER; note = 2'-Fluoro-guanosine
  misc_feature 2^3: note = Phosphorothioate bond
  modified_base 3: mod_base = um
  modified_base 4: mod_base = gm
  modified_base 5: mod_base = cm
  modified_base 6: mod_base = OTHER; note = 2'-Fluoro-guanosine
  modified_base 7: mod_base = OTHER; note = 2'-O-methyl-adenosine
  modified_base 8: mod_base = um
  modified_base 9: mod_base = cm
  modified_base 10: mod_base = OTHER; note = 2'-O-methyl-adenosine
  modified_base 11: mod_base = um
  modified_base 12: mod_base = cm
  modified_base 13: mod_base = cm
  modified_base 14: mod_base = OTHER; note = 2'-Fluoro-adenosine
  modified_base 15: mod_base = gm
  modified_base 16: mod_base = OTHER; note = 2'-Fluoro-cytidine
  modified_base 17: mod_base = um
  modified_base 18: mod_base = OTHER; note = 2'-Fluoro-guanosine
  modified_base 19: mod_base = OTHER; note = 2'-O-methyl-adenosine
  modified_base 20: mod_base = um
  modified_base 21: mod_base = gm
  misc_feature 21^22: note = Phosphorothioate bond
  modified_base 22: mod_base = OTHER; note = 2'-O-methyl-adenosine
  misc_feature 22^23: note = Phosphorothioate bond
  modified_base 23: mod_base = cm
tgtgcgatcatccagctgatgac

SEQ ID NO: 865 - RNA, 23 nt, synthetic construct
  source 1..23: mol_type = other RNA
  modified_base 1: mod_base = OTHER; note = 2'-O-methyl-adenosine
  misc_feature 1^2: note = Phosphorothioate bond
  modified_base 2: mod_base = OTHER; note = 2'-Fluoro-cytidine
  misc_feature 2^3: note = Phosphorothioate bond
  modified_base 3: mod_base = gm
  modified_base 4: mod_base = gm
  modified_base 5: mod_base = OTHER; note = 2'-O-methyl-adenosine
  modified_base 6: mod_base = OTHER; note = 2'-Fluoro-cytidine
  modified_base 7: mod_base = cm
  modified_base 8: mod_base = OTHER; note = 2'-O-methyl-adenosine
  modified_base 9: mod_base = cm
  modified_base 10: mod_base = gm
  modified_base 11: mod_base = cm
  modified_base 12: mod_base = OTHER; note = 2'-O-methyl-adenosine
  modified_base 13: mod_base = gm
  modified_base 14: mod_base = OTHER; note = 2'-Fluoro-uridine
  modified_base 15: mod_base = cm
  modified_base 16: mod_base = OTHER; note = 2'-Fluoro-uridine
  modified_base 17: mod_base = OTHER; note = 2'-O-methyl-adenosine
  modified_base 18: mod_base = OTHER; note = 2'-Fluoro-uridine
  modified_base 19: mod_base = OTHER; note = 2'-O-methyl-adenosine
  modified_base 20: mod_base = OTHER; note = 2'-O-methyl-adenosine
  modified_base 21: mod_base = um
  misc_feature 21^22: note = Phosphorothioate bond
  modified_base 22: mod_base = gm
  misc_feature 22^23: note = Phosphorothioate bond
  modified_base 23: mod_base = cm
acggaccacgcagtctataatgc

SEQ ID NO: 866 - RNA, 23 nt, synthetic construct
  source 1..23: mol_type = other RNA
  modified_base 1: mod_base = um
  misc_feature 1^2: note = Phosphorothioate bond
  modified_base 2: mod_base = OTHER; note = 2'-Fluoro-guanosine
  misc_feature 2^3: note = Phosphorothioate bond
  modified_base 3: mod_base = cm
  modified_base 4: mod_base = um
  modified_base 5: mod_base = OTHER; note = 2'-O-methyl-adenosine
  modified_base 6: mod_base = OTHER; note = 2'-Fluoro-guanosine
  modified_base 7: mod_base = OTHER; note = 2'-O-methyl-adenosine
  modified_base 8: mod_base = cm
  modified_base 9: mod_base = gm
  modified_base 10: mod_base = gm
  modified_base 11: mod_base = gm
  modified_base 12: mod_base = um
  modified_base 13: mod_base = OTHER; note = 2'-O-methyl-adenosine
  modified_base 14: mod_base = OTHER; note = 2'-Fluoro-cytidine
  modified_base 15: mod_base = gm
  modified_base 16: mod_base = OTHER; note = 2'-Fluoro-guanosine
  modified_base 17: mod_base = gm
  modified_base 18: mod_base = OTHER; note = 2'-Fluoro-cytidine
  modified_base 19: mod_base = OTHER; note = 2'-O-methyl-adenosine
  modified_base 20: mod_base = OTHER; note = 2'-O-methyl-adenosine
  modified_base 21: mod_base = OTHER; note = 2'-O-methyl-adenosine
  misc_feature 21^22: note = Phosphorothioate bond
  modified_base 22: mod_base = OTHER; note = 2'-O-methyl-adenosine
  misc_feature 22^23: note = Phosphorothioate bond
  modified_base 23: mod_base = um
tgctagacgggtacgggcaaaat

SEQ ID NO: 867 - RNA, 23 nt, synthetic construct
  source 1..23: mol_type = other RNA
  modified_base 1: mod_base = um
  misc_feature 1^2: note = Phosphorothioate bond
  modified_base 2: mod_base = OTHER; note = 2'-Fluoro-cytidine
  misc_feature 2^3: note = Phosphorothioate bond
  modified_base 3: mod_base = OTHER; note = 2'-O-methyl-adenosine
  modified_base 4: mod_base = um
  modified_base 5: mod_base = cm
  modified_base 6: mod_base = OTHER; note = 2'-Fluoro-cytidine
  modified_base 7: mod_base = OTHER; note = 2'-O-methyl-adenosine
  modified_base 8: mod_base = gm
  modified_base 9: mod_base = cm
  modified_base 10: mod_base = um
  modified_base 11: mod_base = gm
  modified_base 12: mod_base = OTHER; note = 2'-O-methyl-adenosine
  modified_base 13: mod_base = um
  modified_base 14: mod_base = OTHER; note = 2'-Fluoro-guanosine
  modified_base 15: mod_base = OTHER; note = 2'-O-methyl-adenosine
  modified_base 16: mod_base = OTHER; note = 2'-Fluoro-cytidine
  modified_base 17: mod_base = gm
  modified_base 18: mod_base = OTHER; note = 2'-Fluoro-adenosine
  modified_base 19: mod_base = um
  modified_base 20: mod_base = gm
  modified_base 21: mod_base = um
  misc_feature 21^22: note = Phosphorothioate bond
  modified_base 22: mod_base = gm
  misc_feature 22^23: note = Phosphorothioate bond
  modified_base 23: mod_base = OTHER; note = 2'-O-methyl-adenosine
tcatccagctgatgacgatgtga

SEQ ID NO: 868 - RNA, 23 nt, synthetic construct
  source 1..23: mol_type = other RNA
  modified_base 1: mod_base = cm
  misc_feature 1^2: note = Phosphorothioate bond
  modified_base 2: mod_base = OTHER; note = 2'-Fluoro-guanosine
  misc_feature 2^3: note = Phosphorothioate bond
  modified_base 3: mod_base = gm
  modified_base 4: mod_base = gm
  modified_base 5: mod_base = um
  modified_base 6: mod_base = OTHER; note = 2'-Fluoro-adenosine
  modified_base 7: mod_base = cm
  modified_base 8: mod_base = gm
  modified_base 9: mod_base = gm
  modified_base 10: mod_base = gm
  modified_base 11: mod_base = cm
  modified_base 12: mod_base = OTHER; note = 2'-O-methyl-adenosine
  modified_base 13: mod_base = OTHER; note = 2'-O-methyl-adenosine
  modified_base 14: mod_base = OTHER; note = 2'-Fluoro-adenosine
  modified_base 15: mod_base = OTHER; note = 2'-O-methyl-adenosine
  modified_base 16: mod_base = OTHER; note = 2'-Fluoro-uridine
  modified_base 17: mod_base = cm
  modified_base 18: mod_base = OTHER; note = 2'-Fluoro-adenosine
  modified_base 19: mod_base = OTHER; note = 2'-O-methyl-adenosine
  modified_base 20: mod_base = gm
  modified_base 21: mod_base = OTHER; note = 2'-O-methyl-adenosine
  misc_feature 21^22: note = Phosphorothioate bond
  modified_base 22: mod_base = gm
  misc_feature 22^23: note = Phosphorothioate bond
  modified_base 23: mod_base = gm
cgggtacgggcaaaatcaagagg

SEQ ID NO: 869 - RNA, 23 nt, synthetic construct
  source 1..23: mol_type = other RNA
  modified_base 1: mod_base = OTHER; note = 2'-O-methyl-adenosine
  misc_feature 1^2: note = Phosphorothioate bond
  modified_base 2: mod_base = OTHER; note = 2'-Fluoro-adenosine
  misc_feature 2^3: note = Phosphorothioate bond
  modified_base 3: mod_base = um
  modified_base 4: mod_base = OTHER; note = 2'-O-methyl-adenosine
  modified_base 5: mod_base = cm
  modified_base 6: mod_base = OTHER; note = 2'-Fluoro-guanosine
  modified_base 7: mod_base = gm
  modified_base 8: mod_base = OTHER; note = 2'-O-methyl-adenosine
  modified_base 9: mod_base = cm
  modified_base 10: mod_base = cm
  modified_base 11: mod_base = OTHER; note = 2'-O-methyl-adenosine
  modified_base 12: mod_base = cm
  modified_base 13: mod_base = gm
  modified_base 14: mod_base = OTHER; note = 2'-Fluoro-cytidine
  modified_base 15: mod_base = OTHER; note = 2'-O-methyl-adenosine
  modified_base 16: mod_base = OTHER; note = 2'-Fluoro-guanosine
  modified_base 17: mod_base = um
  modified_base 18: mod_base = OTHER; note = 2'-Fluoro-cytidine
  modified_base 19: mod_base = um
  modified_base 20: mod_base = OTHER; note = 2'-O-methyl-adenosine
  modified_base 21: mod_base = um
  misc_feature 21^22: note = Phosphorothioate bond
  modified_base 22: mod_base = OTHER; note = 2'-O-methyl-adenosine
  misc_feature 22^23: note = Phosphorothioate bond
  modified_base 23: mod_base = OTHER; note = 2'-O-methyl-adenosine
aatacggaccacgcagtctataa

SEQ ID NO: 870 - RNA, 23 nt, synthetic construct
  source 1..23: mol_type = other RNA
  modified_base 1: mod_base = um
  misc_feature 1^2: note = Phosphorothioate bond
  modified_base 2: mod_base = OTHER; note = 2'-Fluoro-cytidine
  misc_feature 2^3: note = Phosphorothioate bond
  modified_base 3: mod_base = OTHER; note = 2'-O-methyl-adenosine
  modified_base 4: mod_base = um
  modified_base 5: mod_base = OTHER; note = 2'-O-methyl-adenosine
  modified_base 6: mod_base = OTHER; note = 2'-Fluoro-guanosine
  modified_base 7: mod_base = OTHER; note = 2'-O-methyl-adenosine
  modified_base 8: mod_base = um
  modified_base 9: mod_base = OTHER; note = 2'-O-methyl-adenosine
  modified_base 10: mod_base = cm
  modified_base 11: mod_base = cm
  modified_base 12: mod_base = gm
  modified_base 13: mod_base = OTHER; note = 2'-O-methyl-adenosine
  modified_base 14: mod_base = OTHER; note = 2'-Fluoro-adenosine
  modified_base 15: mod_base = gm
  modified_base 16: mod_base = OTHER; note = 2'-Fluoro-uridine
  modified_base 17: mod_base = OTHER; note = 2'-O-methyl-adenosine
  modified_base 18: mod_base = OTHER; note = 2'-Fluoro-guanosine
  modified_base 19: mod_base = gm
  modified_base 20: mod_base = cm
  modified_base 21: mod_base = gm
  misc_feature 21^22: note = Phosphorothioate bond
  modified_base 22: mod_base = gm
  misc_feature 22^23: note = Phosphorothioate bond
  modified_base 23: mod_base = cm
tcatagataccgaagtaggcggc

SEQ ID NO: 871 - RNA, 23 nt, synthetic construct
  source 1..23: mol_type = other RNA
  modified_base 1: mod_base = gm
  misc_feature 1^2: note = Phosphorothioate bond
  modified_base 2: mod_base = OTHER; note = 2'-Fluoro-guanosine
  misc_feature 2^3: note = Phosphorothioate bond
  modified_base 3: mod_base = gm
  modified_base 4: mod_base = OTHER; note = 2'-O-methyl-adenosine
  modified_base 5: mod_base = OTHER; note = 2'-O-methyl-adenosine
  modified_base 6: mod_base = OTHER; note = 2'-Fluoro-uridine
  modified_base 7: mod_base = OTHER; note = 2'-O-methyl-adenosine
  modified_base 8: mod_base = cm
  modified_base 9: mod_base = gm
  modified_base 10: mod_base = gm
  modified_base 11: mod_base = OTHER; note = 2'-O-methyl-adenosine
  modified_base 12: mod_base = cm
  modified_base 13: mod_base = cm
  modified_base 14: mod_base = OTHER; note = 2'-Fluoro-adenosine
  modified_base 15: mod_base = cm
  modified_base 16: mod_base = OTHER; note = 2'-Fluoro-guanosine
  modified_base 17: mod_base = cm
  modified_base 18: mod_base = OTHER; note = 2'-Fluoro-adenosine
  modified_base 19: mod_base = gm
  modified_base 20: mod_base = um
  modified_base 21: mod_base = cm
  misc_feature 21^22: note = Phosphorothioate bond
  modified_base 22: mod_base = um
  misc_feature 22^23: note = Phosphorothioate bond
  modified_base 23: mod_base = OTHER; note = 2'-O-methyl-adenosine
gggaatacggaccacgcagtcta

SEQ ID NO: 872 - RNA, 23 nt, synthetic construct
  source 1..23: mol_type = other RNA
  modified_base 1: mod_base = gm
  misc_feature 1^2: note = Phosphorothioate bond
  modified_base 2: mod_base = OTHER; note = 2'-Fluoro-uridine
  misc_feature 2^3: note = Phosphorothioate bond
  modified_base 3: mod_base = gm
  modified_base 4: mod_base = cm
  modified_base 5: mod_base = gm
  modified_base 6: mod_base = OTHER; note = 2'-Fluoro-adenosine
  modified_base 7: mod_base = um
  modified_base 8: mod_base = cm
  modified_base 9: mod_base = OTHER; note = 2'-O-methyl-adenosine
  modified_base 10: mod_base = um
  modified_base 11: mod_base = cm
  modified_base 12: mod_base = cm
  modified_base 13: mod_base = OTHER; note = 2'-O-methyl-adenosine
  modified_base 14: mod_base = OTHER; note = 2'-Fluoro-guanosine
  modified_base 15: mod_base = cm
  modified_base 16: mod_base = OTHER; note = 2'-Fluoro-uridine
  modified_base 17: mod_base = gm
  modified_base 18: mod_base = OTHER; note = 2'-Fluoro-adenosine
  modified_base 19: mod_base = um
  modified_base 20: mod_base = gm
  modified_base 21: mod_base = OTHER; note = 2'-O-methyl-adenosine
  misc_feature 21^22: note = Phosphorothioate bond
  modified_base 22: mod_base = cm
  misc_feature 22^23: note = Phosphorothioate bond
  modified_base 23: mod_base = gm
gtgcgatcatccagctgatgacg

SEQ ID NO: 873 - RNA, 23 nt, synthetic construct
  source 1..23: mol_type = other RNA
  modified_base 1: mod_base = um
  misc_feature 1^2: note = Phosphorothioate bond
  modified_base 2: mod_base = OTHER; note = 2'-Fluoro-adenosine
  misc_feature 2^3: note = Phosphorothioate bond
  modified_base 3: mod_base = cm
  modified_base 4: mod_base = gm
  modified_base 5: mod_base = gm
  modified_base 6: mod_base = OTHER; note = 2'-Fluoro-adenosine
  modified_base 7: mod_base = cm
  modified_base 8: mod_base = cm
  modified_base 9: mod_base = OTHER; note = 2'-O-methyl-adenosine
  modified_base 10: mod_base = cm
  modified_base 11: mod_base = gm
  modified_base 12: mod_base = cm
  modified_base 13: mod_base = OTHER; note = 2'-O-methyl-adenosine
  modified_base 14: mod_base = OTHER; note = 2'-Fluoro-guanosine
  modified_base 15: mod_base = um
  modified_base 16: mod_base = OTHER; note = 2'-Fluoro-cytidine
  modified_base 17: mod_base = um
  modified_base 18: mod_base = OTHER; note = 2'-Fluoro-adenosine
  modified_base 19: mod_base = um
  modified_base 20: mod_base = OTHER; note = 2'-O-methyl-adenosine
  modified_base 21: mod_base = OTHER; note = 2'-O-methyl-adenosine
  misc_feature 21^22: note = Phosphorothioate bond
  modified_base 22: mod_base = um
  misc_feature 22^23: note = Phosphorothioate bond
  modified_base 23: mod_base = gm
tacggaccacgcagtctataatg

SEQ ID NO: 874 - RNA, 23 nt, synthetic construct
  source 1..23: mol_type = other RNA
  modified_base 1: mod_base = um
  misc_feature 1^2: note = Phosphorothioate bond
  modified_base 2: mod_base = OTHER; note = 2'-Fluoro-guanosine
  misc_feature 2^3: note = Phosphorothioate bond
  modified_base 3: mod_base = um
  modified_base 4: mod_base = cm
  modified_base 5: mod_base = OTHER; note = 2'-O-methyl-adenosine
  modified_base 6: mod_base = OTHER; note = 2'-Fluoro-uridine
  modified_base 7: mod_base = OTHER; note = 2'-O-methyl-adenosine
  modified_base 8: mod_base = gm
  modified_base 9: mod_base = OTHER; note = 2'-O-methyl-adenosine
  modified_base 10: mod_base = um
  modified_base 11: mod_base = OTHER; note = 2'-O-methyl-adenosine
  modified_base 12: mod_base = cm
  modified_base 13: mod_base = cm
  modified_base 14: mod_base = OTHER; note = 2'-Fluoro-guanosine
  modified_base 15: mod_base = OTHER; note = 2'-O-methyl-adenosine
  modified_base 16: mod_base = OTHER; note = 2'-Fluoro-adenosine
  modified_base 17: mod_base = gm
  modified_base 18: mod_base = OTHER; note = 2'-Fluoro-uridine
  modified_base 19: mod_base = OTHER; note = 2'-O-methyl-adenosine
  modified_base 20: mod_base = gm
  modified_base 21: mod_base = gm
  misc_feature 21^22: note = Phosphorothioate bond
  modified_base 22: mod_base = cm
  misc_feature 22^23: note = Phosphorothioate bond
  modified_base 23: mod_base = gm
tgtcatagataccgaagtaggcg

SEQ ID NO: 875 - RNA, 23 nt, synthetic construct
  source 1..23: mol_type = other RNA
  modified_base 1: mod_base = um
  misc_feature 1^2: note = Phosphorothioate bond
  modified_base 2: mod_base = OTHER; note = 2'-Fluoro-adenosine
  misc_feature 2^3: note = Phosphorothioate bond
  modified_base 3: mod_base = um
  modified_base 4: mod_base = cm
  modified_base 5: mod_base = OTHER; note = 2'-O-methyl-adenosine
  modified_base 6: mod_base = OTHER; note = 2'-Fluoro-guanosine
  modified_base 7: mod_base = gm
  modified_base 8: mod_base = OTHER; note = 2'-O-methyl-adenosine
  modified_base 9: mod_base = gm
  modified_base 10: mod_base = um
  modified_base 11: mod_base = gm
  modified_base 12: mod_base = OTHER; note = 2'-O-methyl-adenosine
  modified_base 13: mod_base = cm
  modified_base 14: mod_base = OTHER; note = 2'-Fluoro-uridine
  modified_base 15: mod_base = gm
  modified_base 16: mod_base = OTHER; note = 2'-Fluoro-adenosine
  modified_base 17: mod_base = OTHER; note = 2'-O-methyl-adenosine
  modified_base 18: mod_base = OTHER; note = 2'-Fluoro-adenosine
  modified_base 19: mod_base = um
  modified_base 20: mod_base = OTHER; note = 2'-O-methyl-adenosine
  modified_base 21: mod_base = OTHER; note = 2'-O-methyl-adenosine
  misc_feature 21^22: note = Phosphorothioate bond
  modified_base 22: mod_base = OTHER; note = 2'-O-methyl-adenosine
  misc_feature 22^23: note = Phosphorothioate bond
  modified_base 23: mod_base = OTHER; note = 2'-O-methyl-adenosine
tatcaggagtgactgaaataaaa

SEQ ID NO: 876 - RNA, 23 nt, synthetic construct
  source 1..23: mol_type = other RNA
  modified_base 1: mod_base = um
  misc_feature 1^2: note = Phosphorothioate bond
  modified_base 2: mod_base = OTHER; note = 2'-Fluoro-guanosine
  misc_feature 2^3: note = Phosphorothioate bond
  modified_base 3: mod_base = cm
  modified_base 4: mod_base = gm
  modified_base 5: mod_base = OTHER; note = 2'-O-methyl-adenosine
  modified_base 6: mod_base = OTHER; note = 2'-Fluoro-uridine
  modified_base 7: mod_base = cm
  modified_base 8: mod_base = OTHER; note = 2'-O-methyl-adenosine
  modified_base 9: mod_base = um
  modified_base 10: mod_base = cm
  modified_base 11: mod_base = cm
  modified_base 12: mod_base = OTHER; note = 2'-O-methyl-adenosine
  modified_base 13: mod_base = gm
  modified_base 14: mod_base = OTHER; note = 2'-Fluoro-cytidine
  modified_base 15: mod_base = um
  modified_base 16: mod_base = OTHER; note = 2'-Fluoro-guanosine
  modified_base 17: mod_base = OTHER; note = 2'-O-methyl-adenosine
  modified_base 18: mod_base = OTHER; note = 2'-Fluoro-uridine
  modified_base 19: mod_base = gm
  modified_base 20: mod_base = OTHER; note = 2'-O-methyl-adenosine
  modified_base 21: mod_base = cm
  misc_feature 21^22: note = Phosphorothioate bond
  modified_base 22: mod_base = gm
  misc_feature 22^23: note = Phosphorothioate bond
  modified_base 23: mod_base = OTHER; note = 2'-O-methyl-adenosine
tgcgatcatccagctgatgacga

SEQ ID NO: 877 - RNA, 23 nt, synthetic construct
  source 1..23: mol_type = other RNA
  modified_base 1: mod_base = cm
  misc_feature 1^2: note = Phosphorothioate bond
  modified_base 2: mod_base = OTHER; note = 2'-Fluoro-uridine
  misc_feature 2^3: note = Phosphorothioate bond
  modified_base 3: mod_base = OTHER; note = 2'-O-methyl-adenosine
  modified_base 4: mod_base = gm
  modified_base 5: mod_base = OTHER; note = 2'-O-methyl-adenosine
  modified_base 6: mod_base = OTHER; note = 2'-Fluoro-cytidine
  modified_base 7: mod_base = gm
  modified_base 8: mod_base = gm
  modified_base 9: mod_base = gm
  modified_base 10: mod_base = um
  modified_base 11: mod_base = OTHER; note = 2'-O-methyl-adenosine
  modified_base 12: mod_base = cm
  modified_base 13: mod_base = gm
  modified_base 14: mod_base = OTHER; note = 2'-Fluoro-guanosine
  modified_base 15: mod_base = gm
  modified_base 16: mod_base = OTHER; note = 2'-Fluoro-cytidine
  modified_base 17: mod_base = OTHER; note = 2'-O-methyl-adenosine
  modified_base 18: mod_base = OTHER; note = 2'-Fluoro-adenosine
  modified_base 19: mod_base = OTHER; note = 2'-O-methyl-adenosine
  modified_base 20: mod_base = OTHER; note = 2'-O-methyl-adenosine
  modified_base 21: mod_base = um
  misc_feature 21^22: note = Phosphorothioate bond
  modified_base 22: mod_base = cm
  misc_feature 22^23: note = Phosphorothioate bond
  modified_base 23: mod_base = OTHER; note = 2'-O-methyl-adenosine
ctagacgggtacgggcaaaatca

SEQ ID NO: 878 - RNA, 23 nt, synthetic construct
  source 1..23: mol_type = other RNA
  modified_base 1: mod_base = gm
  misc_feature 1^2: note = Phosphorothioate bond
  modified_base 2: mod_base = OTHER; note = 2'-Fluoro-adenosine
  misc_feature 2^3: note = Phosphorothioate bond
  modified_base 3: mod_base = um
  modified_base 4: mod_base = cm
  modified_base 5: mod_base = cm
  modified_base 6: mod_base = OTHER; note = 2'-Fluoro-guanosine
  modified_base 7: mod_base = gm
  modified_base 8: mod_base = OTHER; note = 2'-O-methyl-adenosine
  modified_base 9: mod_base = OTHER; note = 2'-O-methyl-adenosine
  modified_base 10: mod_base = gm
  modified_base 11: mod_base = cm
  modified_base 12: mod_base = OTHER; note = 2'-O-methyl-adenosine
  modified_base 13: mod_base = um
  modified_base 14: mod_base = OTHER; note = 2'-Fluoro-uridine
  modified_base 15: mod_base = cm
  modified_base 16: mod_base = OTHER; note = 2'-Fluoro-cytidine
  modified_base 17: mod_base = cm
  modified_base 18: mod_base = OTHER; note = 2'-Fluoro-uridine
  modified_base 19: mod_base = um
  modified_base 20: mod_base = um
  modified_base 21: mod_base = gm
  misc_feature 21^22: note = Phosphorothioate bond
  modified_base 22: mod_base = cm
  misc_feature 22^23: note = Phosphorothioate bond
  modified_base 23: mod_base = OTHER; note = 2'-O-methyl-adenosine
gatccggaagcattccctttgca

SEQ ID NO: 879 - RNA, 23 nt, synthetic construct
  source 1..23: mol_type = other RNA
  modified_base 1: mod_base = gm
  misc_feature 1^2: note = Phosphorothioate bond
  modified_base 2: mod_base = OTHER; note = 2'-Fluoro-cytidine
  misc_feature 2^3: note = Phosphorothioate bond
  modified_base 3: mod_base = OTHER; note = 2'-O-methyl-adenosine
  modified_base 4: mod_base = cm
  modified_base 5: mod_base = OTHER; note = 2'-O-methyl-adenosine
  modified_base 6: mod_base = OTHER; note = 2'-Fluoro-guanosine
  modified_base 7: mod_base = OTHER; note = 2'-O-methyl-adenosine
  modified_base 8: mod_base = cm
  modified_base 9: mod_base = OTHER; note = 2'-O-methyl-adenosine
  modified_base 10: mod_base = cm
  modified_base 11: mod_base = gm
  modified_base 12: mod_base = um
  modified_base 13: mod_base = um
  modified_base 14: mod_base = OTHER; note = 2'-Fluoro-adenosine
  modified_base 15: mod_base = OTHER; note = 2'-O-methyl-adenosine
  modified_base 16: mod_base = OTHER; note = 2'-Fluoro-adenosine
  modified_base 17: mod_base = gm
  modified_base 18: mod_base = OTHER; note = 2'-Fluoro-cytidine
  modified_base 19: mod_base = cm
  modified_base 20: mod_base = um
  modified_base 21: mod_base = um
  misc_feature 21^22: note = Phosphorothioate bond
  modified_base 22: mod_base = gm
  misc_feature 22^23: note = Phosphorothioate bond
  modified_base 23: mod_base = gm
gcacagacacgttaaagccttgg

SEQ ID NO: 880 - RNA, 23 nt, synthetic construct
  source 1..23: mol_type = other RNA
  modified_base 1: mod_base = cm
  misc_feature 1^2: note = Phosphorothioate bond
  modified_base 2: mod_base = OTHER; note = 2'-Fluoro-cytidine
  misc_feature 2^3: note = Phosphorothioate bond
  modified_base 3: mod_base = OTHER; note = 2'-O-methyl-adenosine
  modified_base 4: mod_base = cm
  modified_base 5: mod_base = gm
  modified_base 6: mod_base = OTHER; note = 2'-Fluoro-cytidine
  modified_base 7: mod_base = OTHER; note = 2'-O-methyl-adenosine
  modified_base 8: mod_base = gm
  modified_base 9: mod_base = um
  modified_base 10: mod_base = cm
  modified_base 11: mod_base = um
  modified_base 12: mod_base = OTHER; note = 2'-O-methyl-adenosine
  modified_base 13: mod_base = um
  modified_base 14: mod_base = OTHER; note = 2'-Fluoro-adenosine
  modified_base 15: mod_base = OTHER; note = 2'-O-methyl-adenosine
  modified_base 16: mod_base = OTHER; note = 2'-Fluoro-uridine
  modified_base 17: mod_base = gm
  modified_base 18: mod_base = OTHER; note = 2'-Fluoro-cytidine
  modified_base 19: mod_base = cm
  modified_base 20: mod_base = um
  modified_base 21: mod_base = um
  misc_feature 21^22: note = Phosphorothioate bond
  modified_base 22: mod_base = um
  misc_feature 22^23: note = Phosphorothioate bond
  modified_base 23: mod_base = gm
ccacgcagtctataatgcctttg

SEQ ID NO: 881 - RNA, 23 nt, synthetic construct
  source 1..23: mol_type = other RNA
  modified_base 1: mod_base = gm
  misc_feature 1^2: note = Phosphorothioate bond
  modified_base 2: mod_base = OTHER; note = 2'-Fluoro-adenosine
  misc_feature 2^3: note = Phosphorothioate bond
  modified_base 3: mod_base = cm
  modified_base 4: mod_base = gm
  modified_base 5: mod_base = gm
  modified_base 6: mod_base = OTHER; note = 2'-Fluoro-guanosine
  modified_base 7: mod_base = um
  modified_base 8: mod_base = OTHER; note = 2'-O-methyl-adenosine
  modified_base 9: mod_base = cm
  modified_base 10: mod_base = gm
  modified_base 11: mod_base = gm
  modified_base 12: mod_base = gm
  modified_base 13: mod_base = cm
  modified_base 14: mod_base = OTHER; note = 2'-Fluoro-adenosine
  modified_base 15: mod_base = OTHER; note = 2'-O-methyl-adenosine
  modified_base 16: mod_base = OTHER; note = 2'-Fluoro-adenosine
  modified_base 17: mod_base = OTHER; note = 2'-O-methyl-adenosine
  modified_base 18: mod_base = OTHER; note = 2'-Fluoro-uridine
  modified_base 19: mod_base = cm
  modified_base 20: mod_base = OTHER; note = 2'-O-methyl-adenosine
  modified_base 21: mod_base = OTHER; note = 2'-O-methyl-adenosine
  misc_feature 21^22: note = Phosphorothioate bond
  modified_base 22: mod_base = gm
  misc_feature 22^23: note = Phosphorothioate bond
  modified_base 23: mod_base = OTHER; note = 2'-O-methyl-adenosine
gacgggtacgggcaaaatcaaga

SEQ ID NO: 882 - RNA, 23 nt, synthetic construct
  source 1..23: mol_type = other RNA
  modified_base 1: mod_base = gm
  misc_feature 1^2: note = Phosphorothioate bond
  modified_base 2: mod_base = OTHER; note = 2'-Fluoro-adenosine
  misc_feature 2^3: note = Phosphorothioate bond
  modified_base 3: mod_base = um
  modified_base 4: mod_base = OTHER; note = 2'-O-methyl-adenosine
  modified_base 5: mod_base = cm
  modified_base 6: mod_base = OTHER; note = 2'-Fluoro-cytidine
  modified_base 7: mod_base = gm
  modified_base 8: mod_base = OTHER; note = 2'-O-methyl-adenosine
  modified_base 9: mod_base = OTHER; note = 2'-O-methyl-adenosine
  modified_base 10: mod_base = gm
  modified_base 11: mod_base = um
  modified_base 12: mod_base = OTHER; note = 2'-O-methyl-adenosine
  modified_base 13: mod_base = gm
  modified_base 14: mod_base = OTHER; note = 2'-Fluoro-guanosine
  modified_base 15: mod_base = cm
  modified_base 16: mod_base = OTHER; note = 2'-Fluoro-guanosine
  modified_base 17: mod_base = gm
  modified_base 18: mod_base = OTHER; note = 2'-Fluoro-cytidine
  modified_base 19: mod_base = um
  modified_base 20: mod_base = cm
  modified_base 21: mod_base = gm
  misc_feature 21^22: note = Phosphorothioate bond
  modified_base 22: mod_base = gm
  misc_feature 22^23: note = Phosphorothioate bond
  modified_base 23: mod_base = um
gataccgaagtaggcggctcggt

SEQ ID NO: 883 - RNA, 23 nt, synthetic construct
  source 1..23: mol_type = other RNA
  modified_base 1: mod_base = gm
  misc_feature 1^2: note = Phosphorothioate bond
  modified_base 2: mod_base = OTHER; note = 2'-Fluoro-uridine
  misc_feature 2^3: note = Phosphorothioate bond
  modified_base 3: mod_base = OTHER; note = 2'-O-methyl-adenosine
  modified_base 4: mod_base = gm
  modified_base 5: mod_base = gm
  modified_base 6: mod_base = OTHER; note = 2'-Fluoro-cytidine
  modified_base 7: mod_base = gm
  modified_base 8: mod_base = gm
  modified_base 9: mod_base = cm
  modified_base 10: mod_base = um
  modified_base 11: mod_base = cm
  modified_base 12: mod_base = gm
  modified_base 13: mod_base = gm
  modified_base 14: mod_base = OTHER; note = 2'-Fluoro-uridine
  modified_base 15: mod_base = OTHER; note = 2'-O-methyl-adenosine
  modified_base 16: mod_base = OTHER; note = 2'-Fluoro-guanosine
  modified_base 17: mod_base = OTHER; note = 2'-O-methyl-adenosine
  modified_base 18: mod_base = OTHER; note = 2'-Fluoro-uridine
  modified_base 19: mod_base = gm
  modified_base 20: mod_base = OTHER; note = 2'-O-methyl-adenosine
  modified_base 21: mod_base = um
  misc_feature 21^22: note = Phosphorothioate bond
  modified_base 22: mod_base = OTHER; note = 2'-O-methyl-adenosine
  misc_feature 22^23: note = Phosphorothioate bond
  modified_base 23: mod_base = OTHER; note = 2'-O-methyl-adenosine
gtaggcggctcggtagatgataa

SEQ ID NO: 884 - RNA, 23 nt, synthetic construct
  source 1..23: mol_type = other RNA
  modified_base 1: mod_base = OTHER; note = 2'-O-methyl-adenosine
  misc_feature 1^2: note = Phosphorothioate bond
  modified_base 2: mod_base = OTHER; note = 2'-Fluoro-guanosine
  misc_feature 2^3: note = Phosphorothioate bond
  modified_base 3: mod_base = OTHER; note = 2'-O-methyl-adenosine
  modified_base 4: mod_base = cm
  modified_base 5: mod_base = gm
  modified_base 6: mod_base = OTHER; note = 2'-Fluoro-guanosine
  modified_base 7: mod_base = gm
  modified_base 8: mod_base = um
  modified_base 9: mod_base = OTHER; note = 2'-O-methyl-adenosine
  modified_base 10: mod_base = cm
  modified_base 11: mod_base = gm
  modified_base 12: mod_base = gm
  modified_base 13: mod_base = gm
  modified_base 14: mod_base = OTHER; note = 2'-Fluoro-cytidine
  modified_base 15: mod_base = OTHER; note = 2'-O-methyl-adenosine
  modified_base 16: mod_base = OTHER; note = 2'-Fluoro-adenosine
  modified_base 17: mod_base = OTHER; note = 2'-O-methyl-adenosine
  modified_base 18: mod_base = OTHER; note = 2'-Fluoro-adenosine
  modified_base 19: mod_base = um
  modified_base 20: mod_base = cm
  modified_base 21: mod_base = OTHER; note = 2'-O-methyl-adenosine
  misc_feature 21^22: note = Phosphorothioate bond
  modified_base 22: mod_base = OTHER; note = 2'-O-methyl-adenosine
  misc_feature 22^23: note = Phosphorothioate bond
  modified_base 23: mod_base = gm
agacgggtacgggcaaaatcaag

SEQ ID NO: 885 - RNA, 23 nt, synthetic construct
  source 1..23: mol_type = other RNA
  modified_base 1: mod_base = um
  misc_feature 1^2: note = Phosphorothioate bond
  modified_base 2: mod_base = OTHER; note = 2'-Fluoro-adenosine
  misc_feature 2^3: note = Phosphorothioate bond
  modified_base 3: mod_base = gm
  modified_base 4: mod_base = gm
  modified_base 5: mod_base = cm
  modified_base 6: mod_base = OTHER; note = 2'-Fluoro-guanosine
  modified_base 7: mod_base = gm
  modified_base 8: mod_base = cm
  modified_base 9: mod_base = um
  modified_base 10: mod_base = cm
  modified_base 11: mod_base = gm
  modified_base 12: mod_base = gm
  modified_base 13: mod_base = um
  modified_base 14: mod_base = OTHER; note = 2'-Fluoro-adenosine
  modified_base 15: mod_base = gm
  modified_base 16: mod_base = OTHER; note = 2'-Fluoro-adenosine
  modified_base 17: mod_base = um
  modified_base 18: mod_base = OTHER; note = 2'-Fluoro-guanosine
  modified_base 19: mod_base = OTHER; note = 2'-O-methyl-adenosine
  modified_base 20: mod_base = um
  modified_base 21: mod_base = OTHER; note = 2'-O-methyl-adenosine
  misc_feature 21^22: note = Phosphorothioate bond
  modified_base 22: mod_base = OTHER; note = 2'-O-methyl-adenosine
  misc_feature 22^23: note = Phosphorothioate bond
  modified_base 23: mod_base = um
taggcggctcggtagatgataat

SEQ ID NO: 886 - RNA, 23 nt, synthetic construct
  source 1..23: mol_type = other RNA
  modified_base 1: mod_base = OTHER; note = 2'-O-methyl-adenosine
  misc_feature 1^2: note = Phosphorothioate bond
  modified_base 2: mod_base = OTHER; note = 2'-Fluoro-adenosine
  misc_feature 2^3: note = Phosphorothioate bond
  modified_base 3: mod_base = gm
  modified_base 4: mod_base = um
  modified_base 5: mod_base = OTHER; note = 2'-O-methyl-adenosine
  modified_base 6: mod_base = OTHER; note = 2'-Fluoro-guanosine
  modified_base 7: mod_base = gm
  modified_base 8: mod_base = cm
  modified_base 9: mod_base = gm
  modified_base 10: mod_base = gm
  modified_base 11: mod_base = cm
  modified_base 12: mod_base = um
  modified_base 13: mod_base = cm
  modified_base 14: mod_base = OTHER; note = 2'-Fluoro-guanosine
  modified_base 15: mod_base = gm
  modified_base 16: mod_base = OTHER; note = 2'-Fluoro-uridine
  modified_base 17: mod_base = OTHER; note = 2'-O-methyl-adenosine
  modified_base 18: mod_base = OTHER; note = 2'-Fluoro-guanosine
  modified_base 19: mod_base = OTHER; note = 2'-O-methyl-adenosine
  modified_base 20: mod_base = um
  modified_base 21: mod_base = gm
  misc_feature 21^22: note = Phosphorothioate bond
  modified_base 22: mod_base = OTHER; note = 2'-O-methyl-adenosine
  misc_feature 22^23: note = Phosphorothioate bond
  modified_base 23: mod_base = um
aagtaggcggctcggtagatgat

SEQ ID NO: 887 - RNA, 23 nt, synthetic construct
  source 1..23: mol_type = other RNA
  modified_base 1: mod_base = cm
  misc_feature 1^2: note = Phosphorothioate bond
  modified_base 2: mod_base = OTHER; note = 2'-Fluoro-uridine
  misc_feature 2^3: note = Phosphorothioate bond
  modified_base 3: mod_base = um
  modified_base 4: mod_base = um
  modified_base 5: mod_base = gm
  modified_base 6: mod_base = OTHER; note = 2'-Fluoro-adenosine
  modified_base 7: mod_base = OTHER; note = 2'-O-methyl-adenosine
  modified_base 8: mod_base = gm
  modified_base 9: mod_base = gm
  modified_base 10: mod_base = cm
  modified_base 11: mod_base = gm
  modified_base 12: mod_base = OTHER; note = 2'-O-methyl-adenosine
  modified_base 13: mod_base = OTHER; note = 2'-O-methyl-adenosine
  modified_base 14: mod_base = OTHER; note = 2'-Fluoro-guanosine
  modified_base 15: mod_base = um
  modified_base 16: mod_base = OTHER; note = 2'-Fluoro-uridine
  modified_base 17: mod_base = OTHER; note = 2'-O-methyl-adenosine
  modified_base 18: mod_base = OTHER; note = 2'-Fluoro-adenosine
  modified_base 19: mod_base = gm
  modified_base 20: mod_base = OTHER; note = 2'-O-methyl-adenosine
  modified_base 21: mod_base = gm
  misc_feature 21^22: note = Phosphorothioate bond
  modified_base 22: mod_base = cm
  misc_feature 22^23: note = Phosphorothioate bond
  modified_base 23: mod_base = cm
ctttgaaggcgaagttaagagcc

SEQ ID NO: 888 - RNA, 23 nt, synthetic construct
  source 1..23: mol_type = other RNA
  modified_base 1: mod_base = cm
  misc_feature 1^2: note = Phosphorothioate bond
  modified_base 2: mod_base = OTHER; note = 2'-Fluoro-guanosine
  misc_feature 2^3: note = Phosphorothioate bond
  modified_base 3: mod_base = OTHER; note = 2'-O-methyl-adenosine
  modified_base 4: mod_base = OTHER; note = 2'-O-methyl-adenosine
  modified_base 5: mod_base = gm
  modified_base 6: mod_base = OTHER; note = 2'-Fluoro-uridine
  modified_base 7: mod_base = um
  modified_base 8: mod_base = OTHER; note = 2'-O-methyl-adenosine
  modified_base 9: mod_base = OTHER; note = 2'-O-methyl-adenosine
  modified_base 10: mod_base = gm
  modified_base 11: mod_base = OTHER; note = 2'-O-methyl-adenosine
  modified_base 12: mod_base = gm
  modified_base 13: mod_base = cm
  modified_base 14: mod_base = OTHER; note = 2'-Fluoro-cytidine
  modified_base 15: mod_base = um
  modified_base 16: mod_base = OTHER; note = 2'-Fluoro-guanosine
  modified_base 17: mod_base = gm
  modified_base 18: mod_base = OTHER; note = 2'-Fluoro-guanosine
  modified_base 19: mod_base = um
  modified_base 20: mod_base = gm
  modified_base 21: mod_base = gm
  misc_feature 21^22: note = Phosphorothioate bond
  modified_base 22: mod_base = gm
  misc_feature 22^23: note = Phosphorothioate bond
  modified_base 23: mod_base = gm
cgaagttaagagcctgggtgggg

SEQ ID NO: 889 - RNA, 23 nt, synthetic construct
  source 1..23: mol_type = other RNA
  modified_base 1: mod_base = cm
  misc_feature 1^2: note = Phosphorothioate bond
  modified_base 2: mod_base = OTHER; note = 2'-Fluoro-cytidine
  misc_feature 2^3: note = Phosphorothioate bond
  modified_base 3: mod_base = cm
  modified_base 4: mod_base = um
  modified_base 5: mod_base = gm
  modified_base 6: mod_base = OTHER; note = 2'-Fluoro-cytidine
  modified_base 7: mod_base = um
  modified_base 8: mod_base = cm
  modified_base 9: mod_base = cm
  modified_base 10: mod_base = um
  modified_base 11: mod_base = um
  modified_base 12: mod_base = gm
  modified_base 13: mod_base = gm
  modified_base 14: mod_base = OTHER; note = 2'-Fluoro-guanosine
  modified_base 15: mod_base = OTHER; note = 2'-O-methyl-adenosine
  modified_base 16: mod_base = OTHER; note = 2'-Fluoro-adenosine
  modified_base 17: mod_base = um
  modified_base 18: mod_base = OTHER; note = 2'-Fluoro-adenosine
  modified_base 19: mod_base = cm
  modified_base 20: mod_base = gm
  modified_base 21: mod_base = gm
  misc_feature 21^22: note = Phosphorothioate bond
  modified_base 22: mod_base = OTHER; note = 2'-O-methyl-adenosine
  misc_feature 22^23: note = Phosphorothioate bond
  modified_base 23: mod_base = cm
ccctgctccttgggaatacggac

SEQ ID NO: 890 - RNA, 23 nt, synthetic construct
  source 1..23: mol_type = other RNA
  modified_base 1: mod_base = gm
  misc_feature 1^2: note = Phosphorothioate bond
  modified_base 2: mod_base = OTHER; note = 2'-Fluoro-adenosine
  misc_feature 2^3: note = Phosphorothioate bond
  modified_base 3: mod_base = OTHER; note = 2'-O-methyl-adenosine
  modified_base 4: mod_base = gm
  modified_base 5: mod_base = gm
  modified_base 6: mod_base = OTHER; note = 2'-Fluoro-adenosine
  modified_base 7: mod_base = cm
  modified_base 8: mod_base = OTHER; note = 2'-O-methyl-adenosine
  modified_base 9: mod_base = gm
  modified_base 10: mod_base = OTHER; note = 2'-O-methyl-adenosine
  modified_base 11: mod_base = OTHER; note = 2'-O-methyl-adenosine
  modified_base 12: mod_base = cm
  modified_base 13: mod_base = um
  modified_base 14: mod_base = OTHER; note = 2'-Fluoro-cytidine
  modified_base 15: mod_base = cm
  modified_base 16: mod_base = OTHER; note = 2'-Fluoro-cytidine
  modified_base 17: mod_base = um
  modified_base 18: mod_base = OTHER; note = 2'-Fluoro-guanosine
  modified_base 19: mod_base = cm
  modified_base 20: mod_base = um
  modified_base 21: mod_base = cm
  misc_feature 21^22: note = Phosphorothioate bond
  modified_base 22: mod_base = cm
  misc_feature 22^23: note = Phosphorothioate bond
  modified_base 23: mod_base = um
gaaggacagaactccctgctcct

SEQ ID NO: 891 - RNA, 23 nt, synthetic construct
  source 1..23: mol_type = other RNA
  modified_base 1: mod_base = OTHER; note = 2'-O-methyl-adenosine
  misc_feature 1^2: note = Phosphorothioate bond
  modified_base 2: mod_base = OTHER; note = 2'-Fluoro-guanosine
  misc_feature 2^3: note = Phosphorothioate bond
  modified_base 3: mod_base = OTHER; note = 2'-O-methyl-adenosine
  modified_base 4: mod_base = OTHER; note = 2'-O-methyl-adenosine
  modified_base 5: mod_base = cm
  modified_base 6: mod_base = OTHER; note = 2'-Fluoro-uridine
  modified_base 7: mod_base = cm
  modified_base 8: mod_base = cm
  modified_base 9: mod_base = cm
  modified_base 10: mod_base = um
  modified_base 11: mod_base = gm
  modified_base 12: mod_base = cm
  modified_base 13: mod_base = um
  modified_base 14: mod_base = OTHER; note = 2'-Fluoro-cytidine
  modified_base 15: mod_base = cm
  modified_base 16: mod_base = OTHER; note = 2'-Fluoro-uridine
  modified_base 17: mod_base = um
  modified_base 18: mod_base = OTHER; note = 2'-Fluoro-guanosine
  modified_base 19: mod_base = gm
  modified_base 20: mod_base = gm
  modified_base 21: mod_base = OTHER; note = 2'-O-methyl-adenosine
  misc_feature 21^22: note = Phosphorothioate bond
  modified_base 22: mod_base = OTHER; note = 2'-O-methyl-adenosine
  misc_feature 22^23: note = Phosphorothioate bond
  modified_base 23: mod_base = um
agaactccctgctccttgggaat

SEQ ID NO: 892 - RNA, 23 nt, synthetic construct
  source 1..23: mol_type = other RNA
  modified_base 1: mod_base = cm
  misc_feature 1^2: note = Phosphorothioate bond
  modified_base 2: mod_base = OTHER; note = 2'-Fluoro-cytidine
  misc_feature 2^3: note = Phosphorothioate bond
  modified_base 3: mod_base = um
  modified_base 4: mod_base = gm
  modified_base 5: mod_base = cm
  modified_base 6: mod_base = OTHER; note = 2'-Fluoro-uridine
  modified_base 7: mod_base = cm
  modified_base 8: mod_base = cm
  modified_base 9: mod_base = um
  modified_base 10: mod_base = um
  modified_base 11: mod_base = gm
  modified_base 12: mod_base = gm
  modified_base 13: mod_base = gm
  modified_base 14: mod_base = OTHER; note = 2'-Fluoro-adenosine
  modified_base 15: mod_base = OTHER; note = 2'-O-methyl-adenosine
  modified_base 16: mod_base = OTHER; note = 2'-Fluoro-uridine
  modified_base 17: mod_base = OTHER; note = 2'-O-methyl-adenosine
  modified_base 18: mod_base = OTHER; note = 2'-Fluoro-cytidine
  modified_base 19: mod_base = gm
  modified_base 20: mod_base = gm
  modified_base 21: mod_base = OTHER; note = 2'-O-methyl-adenosine
  misc_feature 21^22: note = Phosphorothioate bond
  modified_base 22: mod_base = cm
  misc_feature 22^23: note = Phosphorothioate bond
  modified_base 23: mod_base = cm
cctgctccttgggaatacggacc

SEQ ID NO: 893 - RNA, 23 nt, synthetic construct
  source 1..23: mol_type = other RNA
  modified_base 1: mod_base = cm
  misc_feature 1^2: note = Phosphorothioate bond
  modified_base 2: mod_base = OTHER; note = 2'-Fluoro-adenosine
  misc_feature 2^3: note = Phosphorothioate bond
  modified_base 3: mod_base = gm
  modified_base 4: mod_base = OTHER; note = 2'-O-methyl-adenosine
  modified_base 5: mod_base = OTHER; note = 2'-O-methyl-adenosine
  modified_base 6: mod_base = OTHER; note = 2'-Fluoro-guanosine
  modified_base 7: mod_base = gm
  modified_base 8: mod_base = OTHER; note = 2'-O-methyl-adenosine
  modified_base 9: mod_base = cm
  modified_base 10: mod_base = OTHER; note = 2'-O-methyl-adenosine
  modified_base 11: mod_base = gm
  modified_base 12: mod_base = OTHER; note = 2'-O-methyl-adenosine
  modified_base 13: mod_base = OTHER; note = 2'-O-methyl-adenosine
  modified_base 14: mod_base = OTHER; note = 2'-Fluoro-cytidine
  modified_base 15: mod_base = um
  modified_base 16: mod_base = OTHER; note = 2'-Fluoro-cytidine
  modified_base 17: mod_base = cm
  modified_base 18: mod_base = OTHER; note = 2'-Fluoro-cytidine
  modified_base 19: mod_base = um
  modified_base 20: mod_base = gm
  modified_base 21: mod_base = cm
  misc_feature 21^22: note = Phosphorothioate bond
  modified_base 22: mod_base = um
  misc_feature 22^23: note = Phosphorothioate bond
  modified_base 23: mod_base = cm
cagaaggacagaactccctgctc

SEQ ID NO: 894 - RNA, 23 nt, synthetic construct
  source 1..23: mol_type = other RNA
  modified_base 1: mod_base = cm
  misc_feature 1^2: note = Phosphorothioate bond
  modified_base 2: mod_base = OTHER; note = 2'-Fluoro-uridine
  misc_feature 2^3: note = Phosphorothioate bond
  modified_base 3: mod_base = gm
  modified_base 4: mod_base = cm
  modified_base 5: mod_base = um
  modified_base 6: mod_base = OTHER; note = 2'-Fluoro-cytidine
  modified_base 7: mod_base = cm
  modified_base 8: mod_base = um
  modified_base 9: mod_base = um
  modified_base 10: mod_base = gm
  modified_base 11: mod_base = gm
  modified_base 12: mod_base = gm
  modified_base 13: mod_base = OTHER; note = 2'-O-methyl-adenosine
  modified_base 14: mod_base = OTHER; note = 2'-Fluoro-adenosine
  modified_base 15: mod_base = um
  modified_base 16: mod_base = OTHER; note = 2'-Fluoro-adenosine
  modified_base 17: mod_base = cm
  modified_base 18: mod_base = OTHER; note = 2'-Fluoro-guanosine
  modified_base 19: mod_base = gm
  modified_base 20: mod_base = OTHER; note = 2'-O-methyl-adenosine
  modified_base 21: mod_base = cm
  misc_feature 21^22: note = Phosphorothioate bond
  modified_base 22: mod_base = cm
  misc_feature 22^23: note = Phosphorothioate bond
  modified_base 23: mod_base = OTHER; note = 2'-O-methyl-adenosine
ctgctccttgggaatacggacca

SEQ ID NO: 895 - RNA, 23 nt, synthetic construct
  source 1..23: mol_type = other RNA
  modified_base 1: mod_base = OTHER; note = 2'-O-methyl-adenosine
  misc_feature 1^2: note = Phosphorothioate bond
  modified_base 2: mod_base = OTHER; note = 2'-Fluoro-guanosine
  misc_feature 2^3: note = Phosphorothioate bond
  modified_base 3: mod_base = OTHER; note = 2'-O-methyl-adenosine
  modified_base 4: mod_base = OTHER; note = 2'-O-methyl-adenosine
  modified_base 5: mod_base = gm
  modified_base 6: mod_base = OTHER; note = 2'-Fluoro-guanosine
  modified_base 7: mod_base = OTHER; note = 2'-O-methyl-adenosine
  modified_base 8: mod_base = cm
  modified_base 9: mod_base = OTHER; note = 2'-O-methyl-adenosine
  modified_base 10: mod_base = gm
  modified_base 11: mod_base = OTHER; note = 2'-O-methyl-adenosine
  modified_base 12: mod_base = OTHER; note = 2'-O-methyl-adenosine
  modified_base 13: mod_base = cm
  modified_base 14: mod_base = OTHER; note = 2'-Fluoro-uridine
  modified_base 15: mod_base = cm
  modified_base 16: mod_base = OTHER; note = 2'-Fluoro-cytidine
  modified_base 17: mod_base = cm
  modified_base 18: mod_base = OTHER; note = 2'-Fluoro-uridine
  modified_base 19: mod_base = gm
  modified_base 20: mod_base = cm
  modified_base 21: mod_base = um
  misc_feature 21^22: note = Phosphorothioate bond
  modified_base 22: mod_base = cm
  misc_feature 22^23: note = Phosphorothioate bond
  modified_base 23: mod_base = cm
agaaggacagaactccctgctcc

SEQ ID NO: 896 - RNA, 23 nt, synthetic construct
  source 1..23: mol_type = other RNA
  modified_base 1: mod_base = OTHER; note = 2'-O-methyl-adenosine
  misc_feature 1^2: note = Phosphorothioate bond
  modified_base 2: mod_base = OTHER; note = 2'-Fluoro-adenosine
  misc_feature 2^3: note = Phosphorothioate bond
  modified_base 3: mod_base = gm
  modified_base 4: mod_base = gm
  modified_base 5: mod_base = OTHER; note = 2'-O-methyl-adenosine
  modified_base 6: mod_base = OTHER; note = 2'-Fluoro-cytidine
  modified_base 7: mod_base = OTHER; note = 2'-O-methyl-adenosine
  modified_base 8: mod_base = gm
  modified_base 9: mod_base = OTHER; note = 2'-O-methyl-adenosine
  modified_base 10: mod_base = OTHER; note = 2'-O-methyl-adenosine
  modified_base 11: mod_base = cm
  modified_base 12: mod_base = um
  modified_base 13: mod_base = cm
  modified_base 14: mod_base = OTHER; note = 2'-Fluoro-cytidine
  modified_base 15: mod_base = cm
  modified_base 16: mod_base = OTHER; note = 2'-Fluoro-uridine
  modified_base 17: mod_base = gm
  modified_base 18: mod_base = OTHER; note = 2'-Fluoro-cytidine
  modified_base 19: mod_base = um
  modified_base 20: mod_base = cm
  modified_base 21: mod_base = cm
  misc_feature 21^22: note = Phosphorothioate bond
  modified_base 22: mod_base = um
  misc_feature 22^23: note = Phosphorothioate bond
  modified_base 23: mod_base = um
aaggacagaactccctgctcctt

SEQ ID NO: 897 - RNA, 23 nt, synthetic construct
  source 1..23: mol_type = other RNA
  modified_base 1: mod_base = gm
  misc_feature 1^2: note = Phosphorothioate bond
  modified_base 2: mod_base = OTHER; note = 2'-Fluoro-adenosine
  misc_feature 2^3: note = Phosphorothioate bond
  modified_base 3: mod_base = OTHER; note = 2'-O-methyl-adenosine
  modified_base 4: mod_base = cm
  modified_base 5: mod_base = um
  modified_base 6: mod_base = OTHER; note = 2'-Fluoro-cytidine
  modified_base 7: mod_base = cm
  modified_base 8: mod_base = cm
  modified_base 9: mod_base = um
  modified_base 10: mod_base = gm
  modified_base 11: mod_base = cm
  modified_base 12: mod_base = um
  modified_base 13: mod_base = cm
  modified_base 14: mod_base = OTHER; note = 2'-Fluoro-cytidine
  modified_base 15: mod_base = um
  modified_base 16: mod_base = OTHER; note = 2'-Fluoro-uridine
  modified_base 17: mod_base = gm
  modified_base 18: mod_base = OTHER; note = 2'-Fluoro-guanosine
  modified_base 19: mod_base = gm
  modified_base 20: mod_base = OTHER; note = 2'-O-methyl-adenosine
  modified_base 21: mod_base = OTHER; note = 2'-O-methyl-adenosine
  misc_feature 21^22: note = Phosphorothioate bond
  modified_base 22: mod_base = um
  misc_feature 22^23: note = Phosphorothioate bond
  modified_base 23: mod_base = OTHER; note = 2'-O-methyl-adenosine
gaactccctgctccttgggaata

SEQ ID NO: 898 - RNA, 23 nt, synthetic construct
  source 1..23: mol_type = other RNA
  modified_base 1: mod_base = OTHER; note = 2'-O-methyl-adenosine
  misc_feature 1^2: note = Phosphorothioate bond
  modified_base 2: mod_base = OTHER; note = 2'-Fluoro-guanosine
  misc_feature 2^3: note = Phosphorothioate bond
  modified_base 3: mod_base = gm
  modified_base 4: mod_base = OTHER; note = 2'-O-methyl-adenosine
  modified_base 5: mod_base = cm
  modified_base 6: mod_base = OTHER; note = 2'-Fluoro-adenosine
  modified_base 7: mod_base = gm
  modified_base 8: mod_base = OTHER; note = 2'-O-methyl-adenosine
  modified_base 9: mod_base = OTHER; note = 2'-O-methyl-adenosine
  modified_base 10: mod_base = cm
  modified_base 11: mod_base = um
  modified_base 12: mod_base = cm
  modified_base 13: mod_base = cm
  modified_base 14: mod_base = OTHER; note = 2'-Fluoro-cytidine
  modified_base 15: mod_base = um
  modified_base 16: mod_base = OTHER; note = 2'-Fluoro-guanosine
  modified_base 17: mod_base = cm
  modified_base 18: mod_base = OTHER; note = 2'-Fluoro-uridine
  modified_base 19: mod_base = cm
  modified_base 20: mod_base = cm
  modified_base 21: mod_base = um
  misc_feature 21^22: note = Phosphorothioate bond
  modified_base 22: mod_base = um
  misc_feature 22^23: note = Phosphorothioate bond
  modified_base 23: mod_base = gm
aggacagaactccctgctccttg

SEQ ID NO: 899 - RNA, 23 nt, synthetic construct
  source 1..23: mol_type = other RNA
  modified_base 1: mod_base = gm
  misc_feature 1^2: note = Phosphorothioate bond
  modified_base 2: mod_base = OTHER; note = 2'-Fluoro-adenosine
  misc_feature 2^3: note = Phosphorothioate bond
  modified_base 3: mod_base = OTHER; note = 2'-O-methyl-adenosine
  modified_base 4: mod_base = gm
  modified_base 5: mod_base = um
  modified_base 6: mod_base = OTHER; note = 2'-Fluoro-uridine
  modified_base 7: mod_base = OTHER; note = 2'-O-methyl-adenosine
  modified_base 8: mod_base = OTHER; note = 2'-O-methyl-adenosine
  modified_base 9: mod_base = gm
  modified_base 10: mod_base = OTHER; note = 2'-O-methyl-adenosine
  modified_base 11: mod_base = gm
  modified_base 12: mod_base = cm
  modified_base 13: mod_base = cm
  modified_base 14: mod_base = OTHER; note = 2'-Fluoro-uridine
  modified_base 15: mod_base = gm
  modified_base 16: mod_base = OTHER; note = 2'-Fluoro-guanosine
  modified_base 17: mod_base = gm
  modified_base 18: mod_base = OTHER; note = 2'-Fluoro-uridine
  modified_base 19: mod_base = gm
  modified_base 20: mod_base = gm
  modified_base 21: mod_base = gm
  misc_feature 21^22: note = Phosphorothioate bond
  modified_base 22: mod_base = gm
  misc_feature 22^23: note = Phosphorothioate bond
  modified_base 23: mod_base = OTHER; note = 2'-O-methyl-adenosine
gaagttaagagcctgggtgggga

SEQ ID NO: 900 - RNA, 23 nt, synthetic construct
  source 1..23: mol_type = other RNA
  modified_base 1: mod_base = um
  misc_feature 1^2: note = Phosphorothioate bond
  modified_base 2: mod_base = OTHER; note = 2'-Fluoro-cytidine
  misc_feature 2^3: note = Phosphorothioate bond
  modified_base 3: mod_base = um
  modified_base 4: mod_base = um
  modified_base 5: mod_base = um
  modified_base 6: mod_base = OTHER; note = 2'-Fluoro-guanosine
  modified_base 7: mod_base = OTHER; note = 2'-O-methyl-adenosine
  modified_base 8: mod_base = OTHER; note = 2'-O-methyl-adenosine
  modified_base 9: mod_base = gm
  modified_base 10: mod_base = gm
  modified_base 11: mod_base = cm
  modified_base 12: mod_base = gm
  modified_base 13: mod_base = OTHER; note = 2'-O-methyl-adenosine
  modified_base 14: mod_base = OTHER; note = 2'-Fluoro-adenosine
  modified_base 15: mod_base = gm
  modified_base 16: mod_base = OTHER; note = 2'-Fluoro-uridine
  modified_base 17: mod_base = um
  modified_base 18: mod_base = OTHER; note = 2'-Fluoro-adenosine
  modified_base 19: mod_base = OTHER; note = 2'-O-methyl-adenosine
  modified_base 20: mod_base = gm
  modified_base 21: mod_base = OTHER; note = 2'-O-methyl-adenosine
  misc_feature 21^22: note = Phosphorothioate bond
  modified_base 22: mod_base = gm
  misc_feature 22^23: note = Phosphorothioate bond
  modified_base 23: mod_base = cm
tctttgaaggcgaagttaagagc

SEQ ID NO: 901 - RNA, 23 nt, synthetic construct
  source 1..23: mol_type = other RNA
  modified_base 1: mod_base = um
  misc_feature 1^2: note = Phosphorothioate bond
  modified_base 2: mod_base = OTHER; note = 2'-Fluoro-adenosine
  misc_feature 2^3: note = Phosphorothioate bond
  modified_base 3: mod_base = um
  modified_base 4: mod_base = um
  modified_base 5: mod_base = um
  modified_base 6: mod_base = OTHER; note = 2'-Fluoro-adenosine
  modified_base 7: mod_base = um
  modified_base 8: mod_base = cm
  modified_base 9: mod_base = OTHER; note = 2'-O-methyl-adenosine
  modified_base 10: mod_base = gm
  modified_base 11: mod_base = gm
  modified_base 12: mod_base = OTHER; note = 2'-O-methyl-adenosine
  modified_base 13: mod_base = gm
  modified_base 14: mod_base = OTHER; note = 2'-Fluoro-uridine
  modified_base 15: mod_base = gm
  modified_base 16: mod_base = OTHER; note = 2'-Fluoro-adenosine
  modified_base 17: mod_base = cm
  modified_base 18: mod_base = OTHER; note = 2'-Fluoro-uridine
  modified_base 19: mod_base = gm
  modified_base 20: mod_base = OTHER; note = 2'-O-methyl-adenosine
  modified_base 21: mod_base = OTHER; note = 2'-O-methyl-adenosine
  misc_feature 21^22: note = Phosphorothioate bond
  modified_base 22: mod_base = OTHER; note = 2'-O-methyl-adenosine
  misc_feature 22^23: note = Phosphorothioate bond
  modified_base 23: mod_base = um
tatttatcaggagtgactgaaat

SEQ ID NO: 902 - RNA, 23 nt, synthetic construct
  source 1..23: mol_type = other RNA
  modified_base 1: mod_base = gm
  misc_feature 1^2: note = Phosphorothioate bond
  modified_base 2: mod_base = OTHER; note = 2'-Fluoro-uridine
  misc_feature 2^3: note = Phosphorothioate bond
  modified_base 3: mod_base = um
  modified_base 4: mod_base = OTHER; note = 2'-O-methyl-adenosine
  modified_base 5: mod_base = um
  modified_base 6: mod_base = OTHER; note = 2'-Fluoro-uridine
  modified_base 7: mod_base = um
  modified_base 8: mod_base = OTHER; note = 2'-O-methyl-adenosine
  modified_base 9: mod_base = um
  modified_base 10: mod_base = cm
  modified_base 11: mod_base = OTHER; note = 2'-O-methyl-adenosine
  modified_base 12: mod_base = gm
  modified_base 13: mod_base = gm
  modified_base 14: mod_base = OTHER; note = 2'-Fluoro-adenosine
  modified_base 15: mod_base = gm
  modified_base 16: mod_base = OTHER; note = 2'-Fluoro-uridine
  modified_base 17: mod_base = gm
  modified_base 18: mod_base = OTHER; note = 2'-Fluoro-adenosine
  modified_base 19: mod_base = cm
  modified_base 20: mod_base = um
  modified_base 21: mod_base = gm
  misc_feature 21^22: note = Phosphorothioate bond
  modified_base 22: mod_base = OTHER; note = 2'-O-methyl-adenosine
  misc_feature 22^23: note = Phosphorothioate bond
  modified_base 23: mod_base = OTHER; note = 2'-O-methyl-adenosine
gttatttatcaggagtgactgaa

SEQ ID NO: 903 - RNA, 23 nt, synthetic construct
  source 1..23: mol_type = other RNA
  modified_base 1: mod_base = um
  misc_feature 1^2: note = Phosphorothioate bond
  modified_base 2: mod_base = OTHER; note = 2'-Fluoro-uridine
  misc_feature 2^3: note = Phosphorothioate bond
  modified_base 3: mod_base = OTHER; note = 2'-O-methyl-adenosine
  modified_base 4: mod_base = um
  modified_base 5: mod_base = um
  modified_base 6: mod_base = OTHER; note = 2'-Fluoro-uridine
  modified_base 7: mod_base = OTHER; note = 2'-O-methyl-adenosine
  modified_base 8: mod_base = um
  modified_base 9: mod_base = cm
  modified_base 10: mod_base = OTHER; note = 2'-O-methyl-adenosine
  modified_base 11: mod_base = gm
  modified_base 12: mod_base = gm
  modified_base 13: mod_base = OTHER; note = 2'-O-methyl-adenosine
  modified_base 14: mod_base = OTHER; note = 2'-Fluoro-guanosine
  modified_base 15: mod_base = um
  modified_base 16: mod_base = OTHER; note = 2'-Fluoro-guanosine
  modified_base 17: mod_base = OTHER; note = 2'-O-methyl-adenosine
  modified_base 18: mod_base = OTHER; note = 2'-Fluoro-cytidine
  modified_base 19: mod_base = um
  modified_base 20: mod_base = gm
  modified_base 21: mod_base = OTHER; note = 2'-O-methyl-adenosine
  misc_feature 21^22: note = Phosphorothioate bond
  modified_base 22: mod_base = OTHER; note = 2'-O-methyl-adenosine
  misc_feature 22^23: note = Phosphorothioate bond
  modified_base 23: mod_base = OTHER; note = 2'-O-methyl-adenosine
ttatttatcaggagtgactgaaa

SEQ ID NO: 904 - RNA, 23 nt, synthetic construct
  source 1..23: mol_type = other RNA
  modified_base 1: mod_base = OTHER; note = 2'-O-methyl-adenosine
  misc_feature 1^2: note = Phosphorothioate bond
  modified_base 2: mod_base = OTHER; note = 2'-Fluoro-adenosine
  misc_feature 2^3: note = Phosphorothioate bond
  modified_base 3: mod_base = OTHER; note = 2'-O-methyl-adenosine
  modified_base 4: mod_base = um
  modified_base 5: mod_base = OTHER; note = 2'-O-methyl-adenosine
  modified_base 6: mod_base = OTHER; note = 2'-Fluoro-cytidine
  modified_base 7: mod_base = OTHER; note = 2'-O-methyl-adenosine
  modified_base 8: mod_base = OTHER; note = 2'-O-methyl-adenosine
  modified_base 9: mod_base = um
  modified_base 10: mod_base = um
  modified_base 11: mod_base = gm
  modified_base 12: mod_base = OTHER; note = 2'-O-methyl-adenosine
  modified_base 13: mod_base = gm
  modified_base 14: mod_base = OTHER; note = 2'-Fluoro-uridine
  modified_base 15: mod_base = cm
  modified_base 16: mod_base = OTHER; note = 2'-Fluoro-cytidine
  modified_base 17: mod_base = cm
  modified_base 18: mod_base = OTHER; note = 2'-Fluoro-adenosine
  modified_base 19: mod_base = um
  modified_base 20: mod_base = cm
  modified_base 21: mod_base = OTHER; note = 2'-O-methyl-adenosine
  misc_feature 21^22: note = Phosphorothioate bond
  modified_base 22: mod_base = um
  misc_feature 22^23: note = Phosphorothioate bond
  modified_base 23: mod_base = cm
aaatacaattgagtcccatcatc

SEQ ID NO: 905 - RNA, 23 nt, synthetic construct
  source 1..23: mol_type = other RNA
  modified_base 1: mod_base = OTHER; note = 2'-O-methyl-adenosine
  misc_feature 1^2: note = Phosphorothioate bond
  modified_base 2: mod_base = OTHER; note = 2'-Fluoro-adenosine
  misc_feature 2^3: note = Phosphorothioate bond
  modified_base 3: mod_base = OTHER; note = 2'-O-methyl-adenosine
  modified_base 4: mod_base = OTHER; note = 2'-O-methyl-adenosine
  modified_base 5: mod_base = um
  modified_base 6: mod_base = OTHER; note = 2'-Fluoro-adenosine
  modified_base 7: mod_base = cm
  modified_base 8: mod_base = OTHER; note = 2'-O-methyl-adenosine
  modified_base 9: mod_base = OTHER; note = 2'-O-methyl-adenosine
  modified_base 10: mod_base = um
  modified_base 11: mod_base = um
  modified_base 12: mod_base = gm
  modified_base 13: mod_base = OTHER; note = 2'-O-methyl-adenosine
  modified_base 14: mod_base = OTHER; note = 2'-Fluoro-guanosine
  modified_base 15: mod_base = um
  modified_base 16: mod_base = OTHER; note = 2'-Fluoro-cytidine
  modified_base 17: mod_base = cm
  modified_base 18: mod_base = OTHER; note = 2'-Fluoro-cytidine
  modified_base 19: mod_base = OTHER; note = 2'-O-methyl-adenosine
  modified_base 20: mod_base = um
  modified_base 21: mod_base = cm
  misc_feature 21^22: note = Phosphorothioate bond
  modified_base 22: mod_base = OTHER; note = 2'-O-methyl-adenosine
  misc_feature 22^23: note = Phosphorothioate bond
  modified_base 23: mod_base = um
aaaatacaattgagtcccatcat

SEQ ID NO: 906 - RNA, 23 nt, synthetic construct
  source 1..23: mol_type = other RNA
  modified_base 1: mod_base = OTHER; note = 2'-O-methyl-adenosine
  misc_feature 1^2: note = Phosphorothioate bond
  modified_base 2: mod_base = OTHER; note = 2'-Fluoro-uridine
  misc_feature 2^3: note = Phosphorothioate bond
  modified_base 3: mod_base = um
  modified_base 4: mod_base = um
  modified_base 5: mod_base = gm
  modified_base 6: mod_base = OTHER; note = 2'-Fluoro-uridine
  modified_base 7: mod_base = um
  modified_base 8: mod_base = OTHER; note = 2'-O-methyl-adenosine
  modified_base 9: mod_base = um
  modified_base 10: mod_base = um
  modified_base 11: mod_base = um
  modified_base 12: mod_base = OTHER; note = 2'-O-methyl-adenosine
  modified_base 13: mod_base = um
  modified_base 14: mod_base = OTHER; note = 2'-Fluoro-cytidine
  modified_base 15: mod_base = OTHER; note = 2'-O-methyl-adenosine
  modified_base 16: mod_base = OTHER; note = 2'-Fluoro-guanosine
  modified_base 17: mod_base = gm
  modified_base 18: mod_base = OTHER; note = 2'-Fluoro-adenosine
  modified_base 19: mod_base = gm
  modified_base 20: mod_base = um
  modified_base 21: mod_base = gm
  misc_feature 21^22: note = Phosphorothioate bond
  modified_base 22: mod_base = OTHER; note = 2'-O-methyl-adenosine
  misc_feature 22^23: note = Phosphorothioate bond
  modified_base 23: mod_base = cm
atttgttatttatcaggagtgac

SEQ ID NO: 907 - RNA, 23 nt, synthetic construct
  source 1..23: mol_type = other RNA
  modified_base 1: mod_base = gm
  misc_feature 1^2: note = Phosphorothioate bond
  modified_base 2: mod_base = OTHER; note = 2'-Fluoro-adenosine
  misc_feature 2^3: note = Phosphorothioate bond
  modified_base 3: mod_base = gm
  modified_base 4: mod_base = OTHER; note = 2'-O-methyl-adenosine
  modified_base 5: mod_base = OTHER; note = 2'-O-methyl-adenosine
  modified_base 6: mod_base = OTHER; note = 2'-Fluoro-adenosine
  modified_base 7: mod_base = OTHER; note = 2'-O-methyl-adenosine
  modified_base 8: mod_base = cm
  modified_base 9: mod_base = um
  modified_base 10: mod_base = gm
  modified_base 11: mod_base = gm
  modified_base 12: mod_base = um
  modified_base 13: mod_base = cm
  modified_base 14: mod_base = OTHER; note = 2'-Fluoro-adenosine
  modified_base 15: mod_base = gm
  modified_base 16: mod_base = OTHER; note = 2'-Fluoro-adenosine
  modified_base 17: mod_base = um
  modified_base 18: mod_base = OTHER; note = 2'-Fluoro-guanosine
  modified_base 19: mod_base = OTHER; note = 2'-O-methyl-adenosine
  modified_base 20: mod_base = OTHER; note = 2'-O-methyl-adenosine
  modified_base 21: mod_base = um
  misc_feature 21^22: note = Phosphorothioate bond
  modified_base 22: mod_base = OTHER; note = 2'-O-methyl-adenosine
  misc_feature 22^23: note = Phosphorothioate bond
  modified_base 23: mod_base = um
gagaaaactggtcagatgaatat

SEQ ID NO: 908 - RNA, 23 nt, synthetic construct
  source 1..23: mol_type = other RNA
  modified_base 1: mod_base = OTHER; note = 2'-O-methyl-adenosine
  misc_feature 1^2: note = Phosphorothioate bond
  modified_base 2: mod_base = OTHER; note = 2'-Fluoro-uridine
  misc_feature 2^3: note = Phosphorothioate bond
  modified_base 3: mod_base = OTHER; note = 2'-O-methyl-adenosine
  modified_base 4: mod_base = um
  modified_base 5: mod_base = OTHER; note = 2'-O-methyl-adenosine
  modified_base 6: mod_base = OTHER; note = 2'-Fluoro-adenosine
  modified_base 7: mod_base = um
  modified_base 8: mod_base = OTHER; note = 2'-O-methyl-adenosine
  modified_base 9: mod_base = cm
  modified_base 10: mod_base = OTHER; note = 2'-O-methyl-adenosine
  modified_base 11: mod_base = OTHER; note = 2'-O-methyl-adenosine
  modified_base 12: mod_base = cm
  modified_base 13: mod_base = OTHER; note = 2'-O-methyl-adenosine
  modified_base 14: mod_base = OTHER; note = 2'-Fluoro-uridine
  modified_base 15: mod_base = gm
  modified_base 16: mod_base = OTHER; note = 2'-Fluoro-cytidine
  modified_base 17: mod_base = cm
  modified_base 18: mod_base = OTHER; note = 2'-Fluoro-uridine
  modified_base 19: mod_base = gm
  modified_base 20: mod_base = um
  modified_base 21: mod_base = um
  misc_feature 21^22: note = Phosphorothioate bond
  modified_base 22: mod_base = cm
  misc_feature 22^23: note = Phosphorothioate bond
  modified_base 23: mod_base = OTHER; note = 2'-O-methyl-adenosine
atataatacaacatgcctgttca

SEQ ID NO: 909 - RNA, 23 nt, synthetic construct
  source 1..23: mol_type = other RNA
  modified_base 1: mod_base = um
  misc_feature 1^2: note = Phosphorothioate bond
  modified_base 2: mod_base = OTHER; note = 2'-Fluoro-guanosine
  misc_feature 2^3: note = Phosphorothioate bond
  modified_base 3: mod_base = gm
  modified_base 4: mod_base = gm
  modified_base 5: mod_base = OTHER; note = 2'-O-methyl-adenosine
  modified_base 6: mod_base = OTHER; note = 2'-Fluoro-uridine
  modified_base 7: mod_base = cm
  modified_base 8: mod_base = cm
  modified_base 9: mod_base = gm
  modified_base 10: mod_base = gm
  modified_base 11: mod_base = OTHER; note = 2'-O-methyl-adenosine
  modified_base 12: mod_base = OTHER; note = 2'-O-methyl-adenosine
  modified_base 13: mod_base = gm
  modified_base 14: mod_base = OTHER; note = 2'-Fluoro-cytidine
  modified_base 15: mod_base = OTHER; note = 2'-O-methyl-adenosine
  modified_base 16: mod_base = OTHER; note = 2'-Fluoro-uridine
  modified_base 17: mod_base = um
  modified_base 18: mod_base = OTHER; note = 2'-Fluoro-cytidine
  modified_base 19: mod_base = cm
  modified_base 20: mod_base = cm
  modified_base 21: mod_base = um
  misc_feature 21^22: note = Phosphorothioate bond
  modified_base 22: mod_base = um
  misc_feature 22^23: note = Phosphorothioate bond
  modified_base 23: mod_base = um
tgggatccggaagcattcccttt

SEQ ID NO: 910 - RNA, 23 nt, synthetic construct
  source 1..23: mol_type = other RNA
  modified_base 1: mod_base = um
  misc_feature 1^2: note = Phosphorothioate bond
  modified_base 2: mod_base = OTHER; note = 2'-Fluoro-uridine
  misc_feature 2^3: note = Phosphorothioate bond
  modified_base 3: mod_base = gm
  modified_base 4: mod_base = gm
  modified_base 5: mod_base = gm
  modified_base 6: mod_base = OTHER; note = 2'-Fluoro-adenosine
  modified_base 7: mod_base = um
  modified_base 8: mod_base = cm
  modified_base 9: mod_base = cm
  modified_base 10: mod_base = gm
  modified_base 11: mod_base = gm
  modified_base 12: mod_base = OTHER; note = 2'-O-methyl-adenosine
  modified_base 13: mod_base = OTHER; note = 2'-O-methyl-adenosine
  modified_base 14: mod_base = OTHER; note = 2'-Fluoro-guanosine
  modified_base 15: mod_base = cm
  modified_base 16: mod_base = OTHER; note = 2'-Fluoro-adenosine
  modified_base 17: mod_base = um
  modified_base 18: mod_base = OTHER; note = 2'-Fluoro-uridine
  modified_base 19: mod_base = cm
  modified_base 20: mod_base = cm
  modified_base 21: mod_base = cm
  misc_feature 21^22: note = Phosphorothioate bond
  modified_base 22: mod_base = um
  misc_feature 22^23: note = Phosphorothioate bond
  modified_base 23: mod_base = um
ttgggatccggaagcattccctt

SEQ ID NO: 911 - RNA, 23 nt, synthetic construct
  source 1..23: mol_type = other RNA
  modified_base 1: mod_base = cm
  misc_feature 1^2: note = Phosphorothioate bond
  modified_base 2: mod_base = OTHER; note = 2'-Fluoro-adenosine
  misc_feature 2^3: note = Phosphorothioate bond
  modified_base 3: mod_base = gm
  modified_base 4: mod_base = gm
  modified_base 5: mod_base = cm
  modified_base 6: mod_base = OTHER; note = 2'-Fluoro-adenosine
  modified_base 7: mod_base = gm
  modified_base 8: mod_base = um
  modified_base 9: mod_base = cm
  modified_base 10: mod_base = OTHER; note = 2'-O-methyl-adenosine
  modified_base 11: mod_base = cm
  modified_base 12: mod_base = cm
  modified_base 13: mod_base = gm
  modified_base 14: mod_base = OTHER; note = 2'-Fluoro-adenosine
  modified_base 15: mod_base = gm
  modified_base 16: mod_base = OTHER; note = 2'-Fluoro-guanosine
  modified_base 17: mod_base = cm
  modified_base 18: mod_base = OTHER; note = 2'-Fluoro-cytidine
  modified_base 19: mod_base = um
  modified_base 20: mod_base = cm
  modified_base 21: mod_base = gm
  misc_feature 21^22: note = Phosphorothioate bond
  modified_base 22: mod_base = gm
  misc_feature 22^23: note = Phosphorothioate bond
  modified_base 23: mod_base = OTHER; note = 2'-O-methyl-adenosine
caggcagtcaccgaggcctcgga

SEQ ID NO: 912 - RNA, 23 nt, synthetic construct
  source 1..23: mol_type = other RNA
  modified_base 1: mod_base = um
  misc_feature 1^2: note = Phosphorothioate bond
  modified_base 2: mod_base = OTHER; note = 2'-Fluoro-adenosine
  misc_feature 2^3: note = Phosphorothioate bond
  modified_base 3: mod_base = um
  modified_base 4: mod_base = OTHER; note = 2'-O-methyl-adenosine
  modified_base 5: mod_base = um
  modified_base 6: mod_base = OTHER; note = 2'-Fluoro-adenosine
  modified_base 7: mod_base = OTHER; note = 2'-O-methyl-adenosine
  modified_base 8: mod_base = um
  modified_base 9: mod_base = OTHER; note = 2'-O-methyl-adenosine
  modified_base 10: mod_base = cm
  modified_base 11: mod_base = OTHER; note = 2'-O-methyl-adenosine
  modified_base 12: mod_base = OTHER; note = 2'-O-methyl-adenosine
  modified_base 13: mod_base = cm
  modified_base 14: mod_base = OTHER; note = 2'-Fluoro-adenosine
  modified_base 15: mod_base = um
  modified_base 16: mod_base = OTHER; note = 2'-Fluoro-guanosine
  modified_base 17: mod_base = cm
  modified_base 18: mod_base = OTHER; note = 2'-Fluoro-cytidine
  modified_base 19: mod_base = um
  modified_base 20: mod_base = gm
  modified_base 21: mod_base = um
  misc_feature 21^22: note = Phosphorothioate bond
  modified_base 22: mod_base = um
  misc_feature 22^23: note = Phosphorothioate bond
  modified_base 23: mod_base = cm
tatataatacaacatgcctgttc

SEQ ID NO: 913 - RNA, 23 nt, synthetic construct
  source 1..23: mol_type = other RNA
  modified_base 1: mod_base = OTHER; note = 2'-O-methyl-adenosine
  misc_feature 1^2: note = Phosphorothioate bond
  modified_base 2: mod_base = OTHER; note = 2'-Fluoro-guanosine
  misc_feature 2^3: note = Phosphorothioate bond
  modified_base 3: mod_base = um
  modified_base 4: mod_base = cm
  modified_base 5: mod_base = um
  modified_base 6: mod_base = OTHER; note = 2'-Fluoro-adenosine
  modified_base 7: mod_base = um
  modified_base 8: mod_base = OTHER; note = 2'-O-methyl-adenosine
  modified_base 9: mod_base = OTHER; note = 2'-O-methyl-adenosine
  modified_base 10: mod_base = um
  modified_base 11: mod_base = gm
  modified_base 12: mod_base = cm
  modified_base 13: mod_base = cm
  modified_base 14: mod_base = OTHER; note = 2'-Fluoro-uridine
  modified_base 15: mod_base = um
  modified_base 16: mod_base = OTHER; note = 2'-Fluoro-uridine
  modified_base 17: mod_base = gm
  modified_base 18: mod_base = OTHER; note = 2'-Fluoro-uridine
  modified_base 19: mod_base = OTHER; note = 2'-O-methyl-adenosine
  modified_base 20: mod_base = um
  modified_base 21: mod_base = um
  misc_feature 21^22: note = Phosphorothioate bond
  modified_base 22: mod_base = gm
  misc_feature 22^23: note = Phosphorothioate bond
  modified_base 23: mod_base = cm
agtctataatgcctttgtattgc

SEQ ID NO: 914 - RNA, 23 nt, synthetic construct
  source 1..23: mol_type = other RNA
  modified_base 1: mod_base = um
  misc_feature 1^2: note = Phosphorothioate bond
  modified_base 2: mod_base = OTHER; note = 2'-Fluoro-uridine
  misc_feature 2^3: note = Phosphorothioate bond
  modified_base 3: mod_base = um
  modified_base 4: mod_base = OTHER; note = 2'-O-methyl-adenosine
  modified_base 5: mod_base = um
  modified_base 6: mod_base = OTHER; note = 2'-Fluoro-cytidine
  modified_base 7: mod_base = OTHER; note = 2'-O-methyl-adenosine
  modified_base 8: mod_base = gm
  modified_base 9: mod_base = gm
  modified_base 10: mod_base = OTHER; note = 2'-O-methyl-adenosine
  modified_base 11: mod_base = gm
  modified_base 12: mod_base = um
  modified_base 13: mod_base = gm
  modified_base 14: mod_base = OTHER; note = 2'-Fluoro-adenosine
  modified_base 15: mod_base = cm
  modified_base 16: mod_base = OTHER; note = 2'-Fluoro-uridine
  modified_base 17: mod_base = gm
  modified_base 18: mod_base = OTHER; note = 2'-Fluoro-adenosine
  modified_base 19: mod_base = OTHER; note = 2'-O-methyl-adenosine
  modified_base 20: mod_base = OTHER; note = 2'-O-methyl-adenosine
  modified_base 21: mod_base = um
  misc_feature 21^22: note = Phosphorothioate bond
  modified_base 22: mod_base = OTHER; note = 2'-O-methyl-adenosine
  misc_feature 22^23: note = Phosphorothioate bond
  modified_base 23: mod_base = OTHER; note = 2'-O-methyl-adenosine
tttatcaggagtgactgaaataa

SEQ ID NO: 915 - RNA, 23 nt, synthetic construct
  source 1..23: mol_type = other RNA
  modified_base 1: mod_base = OTHER; note = 2'-O-methyl-adenosine
  misc_feature 1^2: note = Phosphorothioate bond
  modified_base 2: mod_base = OTHER; note = 2'-Fluoro-adenosine
  misc_feature 2^3: note = Phosphorothioate bond
  modified_base 3: mod_base = um
  modified_base 4: mod_base = OTHER; note = 2'-O-methyl-adenosine
  modified_base 5: mod_base = cm
  modified_base 6: mod_base = OTHER; note = 2'-Fluoro-adenosine
  modified_base 7: mod_base = OTHER; note = 2'-O-methyl-adenosine
  modified_base 8: mod_base = um
  modified_base 9: mod_base = um
  modified_base 10: mod_base = gm
  modified_base 11: mod_base = OTHER; note = 2'-O-methyl-adenosine
  modified_base 12: mod_base = gm
  modified_base 13: mod_base = um
  modified_base 14: mod_base = OTHER; note = 2'-Fluoro-cytidine
  modified_base 15: mod_base = cm
  modified_base 16: mod_base = OTHER; note = 2'-Fluoro-cytidine
  modified_base 17: mod_base = OTHER; note = 2'-O-methyl-adenosine
  modified_base 18: mod_base = OTHER; note = 2'-Fluoro-uridine
  modified_base 19: mod_base = cm
  modified_base 20: mod_base = OTHER; note = 2'-O-methyl-adenosine
  modified_base 21: mod_base = um
  misc_feature 21^22: note = Phosphorothioate bond
  modified_base 22: mod_base = cm
  misc_feature 22^23: note = Phosphorothioate bond
  modified_base 23: mod_base = OTHER; note = 2'-O-methyl-adenosine
aatacaattgagtcccatcatca

SEQ ID NO: 916 - RNA, 23 nt, synthetic construct
  source 1..23: mol_type = other RNA
  modified_base 1: mod_base = cm
  misc_feature 1^2: note = Phosphorothioate bond
  modified_base 2: mod_base = OTHER; note = 2'-Fluoro-uridine
  misc_feature 2^3: note = Phosphorothioate bond
  modified_base 3: mod_base = um
  modified_base 4: mod_base = um
  modified_base 5: mod_base = OTHER; note = 2'-O-methyl-adenosine
  modified_base 6: mod_base = OTHER; note = 2'-Fluoro-adenosine
  modified_base 7: mod_base = gm
  modified_base 8: mod_base = OTHER; note = 2'-O-methyl-adenosine
  modified_base 9: mod_base = gm
  modified_base 10: mod_base = OTHER; note = 2'-O-methyl-adenosine
  modified_base 11: mod_base = OTHER; note = 2'-O-methyl-adenosine
  modified_base 12: mod_base = OTHER; note = 2'-O-methyl-adenosine
  modified_base 13: mod_base = OTHER; note = 2'-O-methyl-adenosine
  modified_base 14: mod_base = OTHER; note = 2'-Fluoro-cytidine
  modified_base 15: mod_base = um
  modified_base 16: mod_base = OTHER; note = 2'-Fluoro-guanosine
  modified_base 17: mod_base = gm
  modified_base 18: mod_base = OTHER; note = 2'-Fluoro-uridine
  modified_base 19: mod_base = cm
  modified_base 20: mod_base = OTHER; note = 2'-O-methyl-adenosine
  modified_base 21: mod_base = gm
  misc_feature 21^22: note = Phosphorothioate bond
  modified_base 22: mod_base = OTHER; note = 2'-O-methyl-adenosine
  misc_feature 22^23: note = Phosphorothioate bond
  modified_base 23: mod_base = um
ctttaagagaaaactggtcagat

SEQ ID NO: 917 - RNA, 23 nt, synthetic construct
  source 1..23: mol_type = other RNA
  modified_base 1: mod_base = gm
  misc_feature 1^2: note = Phosphorothioate bond
  modified_base 2: mod_base = OTHER; note = 2'-Fluoro-cytidine
  misc_feature 2^3: note = Phosphorothioate bond
  modified_base 3: mod_base = um
  modified_base 4: mod_base = um
  modified_base 5: mod_base = um
  modified_base 6: mod_base = OTHER; note = 2'-Fluoro-adenosine
  modified_base 7: mod_base = OTHER; note = 2'-O-methyl-adenosine
  modified_base 8: mod_base = gm
  modified_base 9: mod_base = OTHER; note = 2'-O-methyl-adenosine
  modified_base 10: mod_base = gm
  modified_base 11: mod_base = OTHER; note = 2'-O-methyl-adenosine
  modified_base 12: mod_base = OTHER; note = 2'-O-methyl-adenosine
  modified_base 13: mod_base = OTHER; note = 2'-O-methyl-adenosine
  modified_base 14: mod_base = OTHER; note = 2'-Fluoro-adenosine
  modified_base 15: mod_base = cm
  modified_base 16: mod_base = OTHER; note = 2'-Fluoro-uridine
  modified_base 17: mod_base = gm
  modified_base 18: mod_base = OTHER; note = 2'-Fluoro-guanosine
  modified_base 19: mod_base = um
  modified_base 20: mod_base = cm
  modified_base 21: mod_base = OTHER; note = 2'-O-methyl-adenosine
  misc_feature 21^22: note = Phosphorothioate bond
  modified_base 22: mod_base = gm
  misc_feature 22^23: note = Phosphorothioate bond
  modified_base 23: mod_base = OTHER; note = 2'-O-methyl-adenosine
gctttaagagaaaactggtcaga

SEQ ID NO: 918 - RNA, 23 nt, synthetic construct
  source 1..23: mol_type = other RNA
  modified_base 1: mod_base = OTHER; note = 2'-O-methyl-adenosine
  misc_feature 1^2: note = Phosphorothioate bond
  modified_base 2: mod_base = OTHER; note = 2'-Fluoro-adenosine
  misc_feature 2^3: note = Phosphorothioate bond
  modified_base 3: mod_base = um
  modified_base 4: mod_base = gm
  modified_base 5: mod_base = cm
  modified_base 6: mod_base = OTHER; note = 2'-Fluoro-cytidine
  modified_base 7: mod_base = um
  modified_base 8: mod_base = um
  modified_base 9: mod_base = um
  modified_base 10: mod_base = gm
  modified_base 11: mod_base = um
  modified_base 12: mod_base = OTHER; note = 2'-O-methyl-adenosine
  modified_base 13: mod_base = um
  modified_base 14: mod_base = OTHER; note = 2'-Fluoro-uridine
  modified_base 15: mod_base = gm
  modified_base 16: mod_base = OTHER; note = 2'-Fluoro-cytidine
  modified_base 17: mod_base = um
  modified_base 18: mod_base = OTHER; note = 2'-Fluoro-uridine
  modified_base 19: mod_base = OTHER; note = 2'-O-methyl-adenosine
  modified_base 20: mod_base = um
  modified_base 21: mod_base = cm
  misc_feature 21^22: note = Phosphorothioate bond
  modified_base 22: mod_base = um
  misc_feature 22^23: note = Phosphorothioate bond
  modified_base 23: mod_base = gm
aatgcctttgtattgcttatctg

SEQ ID NO: 919 - RNA, 23 nt, synthetic construct
  source 1..23: mol_type = other RNA
  modified_base 1: mod_base = um
  misc_feature 1^2: note = Phosphorothioate bond
  modified_base 2: mod_base = OTHER; note = 2'-Fluoro-adenosine
  misc_feature 2^3: note = Phosphorothioate bond
  modified_base 3: mod_base = OTHER; note = 2'-O-methyl-adenosine
  modified_base 4: mod_base = um
  modified_base 5: mod_base = gm
  modified_base 6: mod_base = OTHER; note = 2'-Fluoro-cytidine
  modified_base 7: mod_base = cm
  modified_base 8: mod_base = um
  modified_base 9: mod_base = um
  modified_base 10: mod_base = um
  modified_base 11: mod_base = gm
  modified_base 12: mod_base = um
  modified_base 13: mod_base = OTHER; note = 2'-O-methyl-adenosine
  modified_base 14: mod_base = OTHER; note = 2'-Fluoro-uridine
  modified_base 15: mod_base = um
  modified_base 16: mod_base = OTHER; note = 2'-Fluoro-guanosine
  modified_base 17: mod_base = cm
  modified_base 18: mod_base = OTHER; note = 2'-Fluoro-uridine
  modified_base 19: mod_base = um
  modified_base 20: mod_base = OTHER; note = 2'-O-methyl-adenosine
  modified_base 21: mod_base = um
  misc_feature 21^22: note = Phosphorothioate bond
  modified_base 22: mod_base = cm
  misc_feature 22^23: note = Phosphorothioate bond
  modified_base 23: mod_base = um
taatgcctttgtattgcttatct

SEQ ID NO: 920 - RNA, 23 nt, synthetic construct
  source 1..23: mol_type = other RNA
  modified_base 1: mod_base = um
  misc_feature 1^2: note = Phosphorothioate bond
  modified_base 2: mod_base = OTHER; note = 2'-Fluoro-adenosine
  misc_feature 2^3: note = Phosphorothioate bond
  modified_base 3: mod_base = cm
  modified_base 4: mod_base = cm
  modified_base 5: mod_base = cm
  modified_base 6: mod_base = OTHER; note = 2'-Fluoro-uridine
  modified_base 7: mod_base = gm
  modified_base 8: mod_base = cm
  modified_base 9: mod_base = OTHER; note = 2'-O-methyl-adenosine
  modified_base 10: mod_base = cm
  modified_base 11: mod_base = OTHER; note = 2'-O-methyl-adenosine
  modified_base 12: mod_base = gm
  modified_base 13: mod_base = OTHER; note = 2'-O-methyl-adenosine
  modified_base 14: mod_base = OTHER; note = 2'-Fluoro-cytidine
  modified_base 15: mod_base = OTHER; note = 2'-O-methyl-adenosine
  modified_base 16: mod_base = OTHER; note = 2'-Fluoro-cytidine
  modified_base 17: mod_base = gm
  modified_base 18: mod_base = OTHER; note = 2'-Fluoro-uridine
  modified_base 19: mod_base = um
  modified_base 20: mod_base = OTHER; note = 2'-O-methyl-adenosine
  modified_base 21: mod_base = OTHER; note = 2'-O-methyl-adenosine
  misc_feature 21^22: note = Phosphorothioate bond
  modified_base 22: mod_base = OTHER; note = 2'-O-methyl-adenosine
  misc_feature 22^23: note = Phosphorothioate bond
  modified_base 23: mod_base = gm
taccctgcacagacacgttaaag

SEQ ID NO: 921 - RNA, 23 nt, synthetic construct
  source 1..23: mol_type = other RNA
  modified_base 1: mod_base = OTHER; note = 2'-O-methyl-adenosine
  misc_feature 1^2: note = Phosphorothioate bond
  modified_base 2: mod_base = OTHER; note = 2'-Fluoro-uridine
  misc_feature 2^3: note = Phosphorothioate bond
  modified_base 3: mod_base = OTHER; note = 2'-O-methyl-adenosine
  modified_base 4: mod_base = cm
  modified_base 5: mod_base = cm
  modified_base 6: mod_base = OTHER; note = 2'-Fluoro-cytidine
  modified_base 7: mod_base = um
  modified_base 8: mod_base = gm
  modified_base 9: mod_base = cm
  modified_base 10: mod_base = OTHER; note = 2'-O-methyl-adenosine
  modified_base 11: mod_base = cm
  modified_base 12: mod_base = OTHER; note = 2'-O-methyl-adenosine
  modified_base 13: mod_base = gm
  modified_base 14: mod_base = OTHER; note = 2'-Fluoro-adenosine
  modified_base 15: mod_base = cm
  modified_base 16: mod_base = OTHER; note = 2'-Fluoro-adenosine
  modified_base 17: mod_base = cm
  modified_base 18: mod_base = OTHER; note = 2'-Fluoro-guanosine
  modified_base 19: mod_base = um
  modified_base 20: mod_base = um
  modified_base 21: mod_base = OTHER; note = 2'-O-methyl-adenosine
  misc_feature 21^22: note = Phosphorothioate bond
  modified_base 22: mod_base = OTHER; note = 2'-O-methyl-adenosine
  misc_feature 22^23: note = Phosphorothioate bond
  modified_base 23: mod_base = OTHER; note = 2'-O-methyl-adenosine
ataccctgcacagacacgttaaa

SEQ ID NO: 922 - RNA, 23 nt, synthetic construct
  source 1..23: mol_type = other RNA
  modified_base 1: mod_base = OTHER; note = 2'-O-methyl-adenosine
  misc_feature 1^2: note = Phosphorothioate bond
  modified_base 2: mod_base = OTHER; note = 2'-Fluoro-uridine
  misc_feature 2^3: note = Phosphorothioate bond
  modified_base 3: mod_base = cm
  modified_base 4: mod_base = cm
  modified_base 5: mod_base = OTHER; note = 2'-O-methyl-adenosine
  modified_base 6: mod_base = OTHER; note = 2'-Fluoro-guanosine
  modified_base 7: mod_base = cm
  modified_base 8: mod_base = um
  modified_base 9: mod_base = gm
  modified_base 10: mod_base = OTHER; note = 2'-O-methyl-adenosine
  modified_base 11: mod_base = um
  modified_base 12: mod_base = gm
  modified_base 13: mod_base = OTHER; note = 2'-O-methyl-adenosine
  modified_base 14: mod_base = OTHER; note = 2'-Fluoro-cytidine
  modified_base 15: mod_base = gm
  modified_base 16: mod_base = OTHER; note = 2'-Fluoro-adenosine
  modified_base 17: mod_base = um
  modified_base 18: mod_base = OTHER; note = 2'-Fluoro-guanosine
  modified_base 19: mod_base = um
  modified_base 20: mod_base = gm
  modified_base 21: mod_base = OTHER; note = 2'-O-methyl-adenosine
  misc_feature 21^22: note = Phosphorothioate bond
  modified_base 22: mod_base = gm
  misc_feature 22^23: note = Phosphorothioate bond
  modified_base 23: mod_base = um
atccagctgatgacgatgtgagt

SEQ ID NO: 923 - RNA, 23 nt, synthetic construct
  source 1..23: mol_type = other RNA
  modified_base 1: mod_base = um
  misc_feature 1^2: note = Phosphorothioate bond
  modified_base 2: mod_base = OTHER; note = 2'-Fluoro-adenosine
  misc_feature 2^3: note = Phosphorothioate bond
  modified_base 3: mod_base = cm
  modified_base 4: mod_base = OTHER; note = 2'-O-methyl-adenosine
  modified_base 5: mod_base = OTHER; note = 2'-O-methyl-adenosine
  modified_base 6: mod_base = OTHER; note = 2'-Fluoro-uridine
  modified_base 7: mod_base = um
  modified_base 8: mod_base = gm
  modified_base 9: mod_base = OTHER; note = 2'-O-methyl-adenosine
  modified_base 10: mod_base = gm
  modified_base 11: mod_base = um
  modified_base 12: mod_base = cm
  modified_base 13: mod_base = cm
  modified_base 14: mod_base = OTHER; note = 2'-Fluoro-cytidine
  modified_base 15: mod_base = OTHER; note = 2'-O-methyl-adenosine
  modified_base 16: mod_base = OTHER; note = 2'-Fluoro-uridine
  modified_base 17: mod_base = cm
  modified_base 18: mod_base = OTHER; note = 2'-Fluoro-adenosine
  modified_base 19: mod_base = um
  modified_base 20: mod_base = cm
  modified_base 21: mod_base = OTHER; note = 2'-O-methyl-adenosine
  misc_feature 21^22: note = Phosphorothioate bond
  modified_base 22: mod_base = um
  misc_feature 22^23: note = Phosphorothioate bond
  modified_base 23: mod_base = cm
tacaattgagtcccatcatcatc

SEQ ID NO: 924 - RNA, 23 nt, synthetic construct
  source 1..23: mol_type = other RNA
  modified_base 1: mod_base = um
  misc_feature 1^2: note = Phosphorothioate bond
  modified_base 2: mod_base = OTHER; note = 2'-Fluoro-guanosine
  misc_feature 2^3: note = Phosphorothioate bond
  modified_base 3: mod_base = gm
  modified_base 4: mod_base = gm
  modified_base 5: mod_base = OTHER; note = 2'-O-methyl-adenosine
  modified_base 6: mod_base = OTHER; note = 2'-Fluoro-adenosine
  modified_base 7: mod_base = um
  modified_base 8: mod_base = OTHER; note = 2'-O-methyl-adenosine
  modified_base 9: mod_base = cm
  modified_base 10: mod_base = gm
  modified_base 11: mod_base = gm
  modified_base 12: mod_base = OTHER; note = 2'-O-methyl-adenosine
  modified_base 13: mod_base = cm
  modified_base 14: mod_base = OTHER; note = 2'-Fluoro-cytidine
  modified_base 15: mod_base = OTHER; note = 2'-O-methyl-adenosine
  modified_base 16: mod_base = OTHER; note = 2'-Fluoro-cytidine
  modified_base 17: mod_base = gm
  modified_base 18: mod_base = OTHER; note = 2'-Fluoro-cytidine
  modified_base 19: mod_base = OTHER; note = 2'-O-methyl-adenosine
  modified_base 20: mod_base = gm
  modified_base 21: mod_base = um
  misc_feature 21^22: note = Phosphorothioate bond
  modified_base 22: mod_base = cm
  misc_feature 22^23: note = Phosphorothioate bond
  modified_base 23: mod_base = um
tgggaatacggaccacgcagtct

SEQ ID NO: 925 - RNA, 23 nt, synthetic construct
  source 1..23: mol_type = other RNA
  modified_base 1: mod_base = um
  misc_feature 1^2: note = Phosphorothioate bond
  modified_base 2: mod_base = OTHER; note = 2'-Fluoro-adenosine
  misc_feature 2^3: note = Phosphorothioate bond
  modified_base 3: mod_base = um
  modified_base 4: mod_base = OTHER; note = 2'-O-methyl-adenosine
  modified_base 5: mod_base = OTHER; note = 2'-O-methyl-adenosine
  modified_base 6: mod_base = OTHER; note = 2'-Fluoro-uridine
  modified_base 7: mod_base = OTHER; note = 2'-O-methyl-adenosine
  modified_base 8: mod_base = cm
  modified_base 9: mod_base = OTHER; note = 2'-O-methyl-adenosine
  modified_base 10: mod_base = OTHER; note = 2'-O-methyl-adenosine
  modified_base 11: mod_base = cm
  modified_base 12: mod_base = OTHER; note = 2'-O-methyl-adenosine
  modified_base 13: mod_base = um
  modified_base 14: mod_base = OTHER; note = 2'-Fluoro-guanosine
  modified_base 15: mod_base = cm
  modified_base 16: mod_base = OTHER; note = 2'-Fluoro-cytidine
  modified_base 17: mod_base = um
  modified_base 18: mod_base = OTHER; note = 2'-Fluoro-guanosine
  modified_base 19: mod_base = um
  modified_base 20: mod_base = um
  modified_base 21: mod_base = cm
  misc_feature 21^22: note = Phosphorothioate bond
  modified_base 22: mod_base = OTHER; note = 2'-O-methyl-adenosine
  misc_feature 22^23: note = Phosphorothioate bond
  modified_base 23: mod_base = cm
tataatacaacatgcctgttcac

SEQ ID NO: 926 - RNA, 23 nt, synthetic construct
  source 1..23: mol_type = other RNA
  modified_base 1: mod_base = um
  misc_feature 1^2: note = Phosphorothioate bond
  modified_base 2: mod_base = OTHER; note = 2'-Fluoro-uridine
  misc_feature 2^3: note = Phosphorothioate bond
  modified_base 3: mod_base = OTHER; note = 2'-O-methyl-adenosine
  modified_base 4: mod_base = um
  modified_base 5: mod_base = cm
  modified_base 6: mod_base = OTHER; note = 2'-Fluoro-adenosine
  modified_base 7: mod_base = gm
  modified_base 8: mod_base = gm
  modified_base 9: mod_base = OTHER; note = 2'-O-methyl-adenosine
  modified_base 10: mod_base = gm
  modified_base 11: mod_base = um
  modified_base 12: mod_base = gm
  modified_base 13: mod_base = OTHER; note = 2'-O-methyl-adenosine
  modified_base 14: mod_base = OTHER; note = 2'-Fluoro-cytidine
  modified_base 15: mod_base = um
  modified_base 16: mod_base = OTHER; note = 2'-Fluoro-guanosine
  modified_base 17: mod_base = OTHER; note = 2'-O-methyl-adenosine
  modified_base 18: mod_base = OTHER; note = 2'-Fluoro-adenosine
  modified_base 19: mod_base = OTHER; note = 2'-O-methyl-adenosine
  modified_base 20: mod_base = um
  modified_base 21: mod_base = OTHER; note = 2'-O-methyl-adenosine
  misc_feature 21^22: note = Phosphorothioate bond
  modified_base 22: mod_base = OTHER; note = 2'-O-methyl-adenosine
  misc_feature 22^23: note = Phosphorothioate bond
  modified_base 23: mod_base = OTHER; note = 2'-O-methyl-adenosine
ttatcaggagtgactgaaataaa

SEQ ID NO: 927 - RNA, 23 nt, synthetic construct
  source 1..23: mol_type = other RNA
  modified_base 1: mod_base = OTHER; note = 2'-O-methyl-adenosine
  misc_feature 1^2: note = Phosphorothioate bond
  modified_base 2: mod_base = OTHER; note = 2'-Fluoro-uridine
  misc_feature 2^3: note = Phosphorothioate bond
  modified_base 3: mod_base = OTHER; note = 2'-O-methyl-adenosine
  modified_base 4: mod_base = OTHER; note = 2'-O-methyl-adenosine
  modified_base 5: mod_base = um
  modified_base 6: mod_base = OTHER; note = 2'-Fluoro-guanosine
  modified_base 7: mod_base = cm
  modified_base 8: mod_base = cm
  modified_base 9: mod_base = um
  modified_base 10: mod_base = um
  modified_base 11: mod_base = um
  modified_base 12: mod_base = gm
  modified_base 13: mod_base = um
  modified_base 14: mod_base = OTHER; note = 2'-Fluoro-adenosine
  modified_base 15: mod_base = um
  modified_base 16: mod_base = OTHER; note = 2'-Fluoro-uridine
  modified_base 17: mod_base = gm
  modified_base 18: mod_base = OTHER; note = 2'-Fluoro-cytidine
  modified_base 19: mod_base = um
  modified_base 20: mod_base = um
  modified_base 21: mod_base = OTHER; note = 2'-O-methyl-adenosine
  misc_feature 21^22: note = Phosphorothioate bond
  modified_base 22: mod_base = um
  misc_feature 22^23: note = Phosphorothioate bond
  modified_base 23: mod_base = cm
ataatgcctttgtattgcttatc

SEQ ID NO: 928 - RNA, 23 nt, synthetic construct
  source 1..23: mol_type = other RNA
  modified_base 1: mod_base = cm
  misc_feature 1^2: note = Phosphorothioate bond
  modified_base 2: mod_base = OTHER; note = 2'-Fluoro-cytidine
  misc_feature 2^3: note = Phosphorothioate bond
  modified_base 3: mod_base = OTHER; note = 2'-O-methyl-adenosine
  modified_base 4: mod_base = gm
  modified_base 5: mod_base = cm
  modified_base 6: mod_base = OTHER; note = 2'-Fluoro-uridine
  modified_base 7: mod_base = gm
  modified_base 8: mod_base = OTHER; note = 2'-O-methyl-adenosine
  modified_base 9: mod_base = um
  modified_base 10: mod_base = gm
  modified_base 11: mod_base = OTHER; note = 2'-O-methyl-adenosine
  modified_base 12: mod_base = cm
  modified_base 13: mod_base = gm
  modified_base 14: mod_base = OTHER; note = 2'-Fluoro-adenosine
  modified_base 15: mod_base = um
  modified_base 16: mod_base = OTHER; note = 2'-Fluoro-guanosine
  modified_base 17: mod_base = um
  modified_base 18: mod_base = OTHER; note = 2'-Fluoro-guanosine
  modified_base 19: mod_base = OTHER; note = 2'-O-methyl-adenosine
  modified_base 20: mod_base = gm
  modified_base 21: mod_base = um
  misc_feature 21^22: note = Phosphorothioate bond
  modified_base 22: mod_base = gm
  misc_feature 22^23: note = Phosphorothioate bond
  modified_base 23: mod_base = um
ccagctgatgacgatgtgagtgt

SEQ ID NO: 929 - RNA, 23 nt, synthetic construct
  source 1..23: mol_type = other RNA
  modified_base 1: mod_base = cm
  misc_feature 1^2: note = Phosphorothioate bond
  modified_base 2: mod_base = OTHER; note = 2'-Fluoro-adenosine
  misc_feature 2^3: note = Phosphorothioate bond
  modified_base 3: mod_base = um
  modified_base 4: mod_base = OTHER; note = 2'-O-methyl-adenosine
  modified_base 5: mod_base = gm
  modified_base 6: mod_base = OTHER; note = 2'-Fluoro-adenosine
  modified_base 7: mod_base = um
  modified_base 8: mod_base = OTHER; note = 2'-O-methyl-adenosine
  modified_base 9: mod_base = cm
  modified_base 10: mod_base = cm
  modified_base 11: mod_base = gm
  modified_base 12: mod_base = OTHER; note = 2'-O-methyl-adenosine
  modified_base 13: mod_base = OTHER; note = 2'-O-methyl-adenosine
  modified_base 14: mod_base = OTHER; note = 2'-Fluoro-guanosine
  modified_base 15: mod_base = um
  modified_base 16: mod_base = OTHER; note = 2'-Fluoro-adenosine
  modified_base 17: mod_base = gm
  modified_base 18: mod_base = OTHER; note = 2'-Fluoro-guanosine
  modified_base 19: mod_base = cm
  modified_base 20: mod_base = gm
  modified_base 21: mod_base = gm
  misc_feature 21^22: note = Phosphorothioate bond
  modified_base 22: mod_base = cm
  misc_feature 22^23: note = Phosphorothioate bond
  modified_base 23: mod_base = um
catagataccgaagtaggcggct

SEQ ID NO: 930 - RNA, 23 nt, synthetic construct
  source 1..23: mol_type = other RNA
  modified_base 1: mod_base = cm
  misc_feature 1^2: note = Phosphorothioate bond
  modified_base 2: mod_base = OTHER; note = 2'-Fluoro-adenosine
  misc_feature 2^3: note = Phosphorothioate bond
  modified_base 3: mod_base = um
  modified_base 4: mod_base = cm
  modified_base 5: mod_base = cm
  modified_base 6: mod_base = OTHER; note = 2'-Fluoro-adenosine
  modified_base 7: mod_base = gm
  modified_base 8: mod_base = cm
  modified_base 9: mod_base = um
  modified_base 10: mod_base = gm
  modified_base 11: mod_base = OTHER; note = 2'-O-methyl-adenosine
  modified_base 12: mod_base = um
  modified_base 13: mod_base = gm
  modified_base 14: mod_base = OTHER; note = 2'-Fluoro-adenosine
  modified_base 15: mod_base = cm
  modified_base 16: mod_base = OTHER; note = 2'-Fluoro-guanosine
  modified_base 17: mod_base = OTHER; note = 2'-O-methyl-adenosine
  modified_base 18: mod_base = OTHER; note = 2'-Fluoro-uridine
  modified_base 19: mod_base = gm
  modified_base 20: mod_base = um
  modified_base 21: mod_base = gm
  misc_feature 21^22: note = Phosphorothioate bond
  modified_base 22: mod_base = OTHER; note = 2'-O-methyl-adenosine
  misc_feature 22^23: note = Phosphorothioate bond
  modified_base 23: mod_base = gm
catccagctgatgacgatgtgag

SEQ ID NO: 931 - RNA, 23 nt, synthetic construct
  source 1..23: mol_type = other RNA
  modified_base 1: mod_base = gm
  misc_feature 1^2: note = Phosphorothioate bond
  modified_base 2: mod_base = OTHER; note = 2'-Fluoro-uridine
  misc_feature 2^3: note = Phosphorothioate bond
  modified_base 3: mod_base = cm
  modified_base 4: mod_base = OTHER; note = 2'-O-methyl-adenosine
  modified_base 5: mod_base = um
  modified_base 6: mod_base = OTHER; note = 2'-Fluoro-adenosine
  modified_base 7: mod_base = gm
  modified_base 8: mod_base = OTHER; note = 2'-O-methyl-adenosine
  modified_base 9: mod_base = um
  modified_base 10: mod_base = OTHER; note = 2'-O-methyl-adenosine
  modified_base 11: mod_base = cm
  modified_base 12: mod_base = cm
  modified_base 13: mod_base = gm
  modified_base 14: mod_base = OTHER; note = 2'-Fluoro-adenosine
  modified_base 15: mod_base = OTHER; note = 2'-O-methyl-adenosine
  modified_base 16: mod_base = OTHER; note = 2'-Fluoro-guanosine
  modified_base 17: mod_base = um
  modified_base 18: mod_base = OTHER; note = 2'-Fluoro-adenosine
  modified_base 19: mod_base = gm
  modified_base 20: mod_base = gm
  modified_base 21: mod_base = cm
  misc_feature 21^22: note = Phosphorothioate bond
  modified_base 22: mod_base = gm
  misc_feature 22^23: note = Phosphorothioate bond
  modified_base 23: mod_base = gm
gtcatagataccgaagtaggcgg

SEQ ID NO: 932 - RNA, 23 nt, synthetic construct
  source 1..23: mol_type = other RNA
  modified_base 1: mod_base = OTHER; note = 2'-O-methyl-adenosine
  misc_feature 1^2: note = Phosphorothioate bond
  modified_base 2: mod_base = OTHER; note = 2'-Fluoro-cytidine
  misc_feature 2^3: note = Phosphorothioate bond
  modified_base 3: mod_base = cm
  modified_base 4: mod_base = cm
  modified_base 5: mod_base = um
  modified_base 6: mod_base = OTHER; note = 2'-Fluoro-guanosine
  modified_base 7: mod_base = cm
  modified_base 8: mod_base = OTHER; note = 2'-O-methyl-adenosine
  modified_base 9: mod_base = cm
  modified_base 10: mod_base = OTHER; note = 2'-O-methyl-adenosine
  modified_base 11: mod_base = gm
  modified_base 12: mod_base = OTHER; note = 2'-O-methyl-adenosine
  modified_base 13: mod_base = cm
  modified_base 14: mod_base = OTHER; note = 2'-Fluoro-adenosine
  modified_base 15: mod_base = cm
  modified_base 16: mod_base = OTHER; note = 2'-Fluoro-guanosine
  modified_base 17: mod_base = um
  modified_base 18: mod_base = OTHER; note = 2'-Fluoro-uridine
  modified_base 19: mod_base = OTHER; note = 2'-O-methyl-adenosine
  modified_base 20: mod_base = OTHER; note = 2'-O-methyl-adenosine
  modified_base 21: mod_base = OTHER; note = 2'-O-methyl-adenosine
  misc_feature 21^22: note = Phosphorothioate bond
  modified_base 22: mod_base = gm
  misc_feature 22^23: note = Phosphorothioate bond
  modified_base 23: mod_base = cm
accctgcacagacacgttaaagc

SEQ ID NO: 933 - RNA, 23 nt, synthetic construct
  source 1..23: mol_type = other RNA
  modified_base 1: mod_base = um
  misc_feature 1^2: note = Phosphorothioate bond
  modified_base 2: mod_base = OTHER; note = 2'-Fluoro-guanosine
  misc_feature 2^3: note = Phosphorothioate bond
  modified_base 3: mod_base = cm
  modified_base 4: mod_base = OTHER; note = 2'-O-methyl-adenosine
  modified_base 5: mod_base = um
  modified_base 6: mod_base = OTHER; note = 2'-Fluoro-cytidine
  modified_base 7: mod_base = OTHER; note = 2'-O-methyl-adenosine
  modified_base 8: mod_base = um
  modified_base 9: mod_base = cm
  modified_base 10: mod_base = OTHER; note = 2'-O-methyl-adenosine
  modified_base 11: mod_base = um
  modified_base 12: mod_base = gm
  modified_base 13: mod_base = cm
  modified_base 14: mod_base = OTHER; note = 2'-Fluoro-guanosine
  modified_base 15: mod_base = gm
  modified_base 16: mod_base = OTHER; note = 2'-Fluoro-cytidine
  modified_base 17: mod_base = gm
  modified_base 18: mod_base = OTHER; note = 2'-Fluoro-guanosine
  modified_base 19: mod_base = cm
  modified_base 20: mod_base = gm
  modified_base 21: mod_base = OTHER; note = 2'-O-methyl-adenosine
  misc_feature 21^22: note = Phosphorothioate bond
  modified_base 22: mod_base = OTHER; note = 2'-O-methyl-adenosine
  misc_feature 22^23: note = Phosphorothioate bond
  modified_base 23: mod_base = cm
tgcatcatcatgcggcggcgaac

SEQ ID NO: 934 - RNA, 23 nt, synthetic construct
  source 1..23: mol_type = other RNA
  modified_base 1: mod_base = cm
  misc_feature 1^2: note = Phosphorothioate bond
  modified_base 2: mod_base = OTHER; note = 2'-Fluoro-guanosine
  misc_feature 2^3: note = Phosphorothioate bond
  modified_base 3: mod_base = gm
  modified_base 4: mod_base = OTHER; note = 2'-O-methyl-adenosine
  modified_base 5: mod_base = cm
  modified_base 6: mod_base = OTHER; note = 2'-Fluoro-cytidine
  modified_base 7: mod_base = OTHER; note = 2'-O-methyl-adenosine
  modified_base 8: mod_base = cm
  modified_base 9: mod_base = gm
  modified_base 10: mod_base = cm
  modified_base 11: mod_base = OTHER; note = 2'-O-methyl-adenosine
  modified_base 12: mod_base = gm
  modified_base 13: mod_base = um
  modified_base 14: mod_base = OTHER; note = 2'-Fluoro-cytidine
  modified_base 15: mod_base = um
  modified_base 16: mod_base = OTHER; note = 2'-Fluoro-adenosine
  modified_base 17: mod_base = um
  modified_base 18: mod_base = OTHER; note = 2'-Fluoro-adenosine
  modified_base 19: mod_base = OTHER; note = 2'-O-methyl-adenosine
  modified_base 20: mod_base = um
  modified_base 21: mod_base = gm
  misc_feature 21^22: note = Phosphorothioate bond
  modified_base 22: mod_base = cm
  misc_feature 22^23: note = Phosphorothioate bond
  modified_base 23: mod_base = cm
cggaccacgcagtctataatgcc

SEQ ID NO: 935 - RNA, 23 nt, synthetic construct
  source 1..23: mol_type = other RNA
  modified_base 1: mod_base = cm
  misc_feature 1^2: note = Phosphorothioate bond
  modified_base 2: mod_base = OTHER; note = 2'-Fluoro-uridine
  misc_feature 2^3: note = Phosphorothioate bond
  modified_base 3: mod_base = um
  modified_base 4: mod_base = gm
  modified_base 5: mod_base = gm
  modified_base 6: mod_base = OTHER; note = 2'-Fluoro-guanosine
  modified_base 7: mod_base = OTHER; note = 2'-O-methyl-adenosine
  modified_base 8: mod_base = OTHER; note = 2'-O-methyl-adenosine
  modified_base 9: mod_base = um
  modified_base 10: mod_base = OTHER; note = 2'-O-methyl-adenosine
  modified_base 11: mod_base = cm
  modified_base 12: mod_base = gm
  modified_base 13: mod_base = gm
  modified_base 14: mod_base = OTHER; note = 2'-Fluoro-adenosine
  modified_base 15: mod_base = cm
  modified_base 16: mod_base = OTHER; note = 2'-Fluoro-cytidine
  modified_base 17: mod_base = OTHER; note = 2'-O-methyl-adenosine
  modified_base 18: mod_base = OTHER; note = 2'-Fluoro-cytidine
  modified_base 19: mod_base = gm
  modified_base 20: mod_base = cm
  modified_base 21: mod_base = OTHER; note = 2'-O-methyl-adenosine
  misc_feature 21^22: note = Phosphorothioate bond
  modified_base 22: mod_base = gm
  misc_feature 22^23: note = Phosphorothioate bond
  modified_base 23: mod_base = um
cttgggaatacggaccacgcagt

SEQ ID NO: 936 - RNA, 23 nt, synthetic construct
  source 1..23: mol_type = other RNA
  modified_base 1: mod_base = gm
  misc_feature 1^2: note = Phosphorothioate bond
  modified_base 2: mod_base = OTHER; note = 2'-Fluoro-adenosine
  misc_feature 2^3: note = Phosphorothioate bond
  modified_base 3: mod_base = OTHER; note = 2'-O-methyl-adenosine
  modified_base 4: mod_base = gm
  modified_base 5: mod_base = um
  modified_base 6: mod_base = OTHER; note = 2'-Fluoro-adenosine
  modified_base 7: mod_base = gm
  modified_base 8: mod_base = gm
  modified_base 9: mod_base = cm
  modified_base 10: mod_base = gm
  modified_base 11: mod_base = gm
  modified_base 12: mod_base = cm
  modified_base 13: mod_base = um
  modified_base 14: mod_base = OTHER; note = 2'-Fluoro-cytidine
  modified_base 15: mod_base = gm
  modified_base 16: mod_base = OTHER; note = 2'-Fluoro-guanosine
  modified_base 17: mod_base = um
  modified_base 18: mod_base = OTHER; note = 2'-Fluoro-adenosine
  modified_base 19: mod_base = gm
  modified_base 20: mod_base = OTHER; note = 2'-O-methyl-adenosine
  modified_base 21: mod_base = um
  misc_feature 21^22: note = Phosphorothioate bond
  modified_base 22: mod_base = gm
  misc_feature 22^23: note = Phosphorothioate bond
  modified_base 23: mod_base = OTHER; note = 2'-O-methyl-adenosine
gaagtaggcggctcggtagatga

SEQ ID NO: 937 - RNA, 23 nt, synthetic construct
  source 1..23: mol_type = other RNA
  modified_base 1: mod_base = cm
  misc_feature 1^2: note = Phosphorothioate bond
  modified_base 2: mod_base = OTHER; note = 2'-Fluoro-uridine
  misc_feature 2^3: note = Phosphorothioate bond
  modified_base 3: mod_base = gm
  modified_base 4: mod_base = cm
  modified_base 5: mod_base = um
  modified_base 6: mod_base = OTHER; note = 2'-Fluoro-adenosine
  modified_base 7: mod_base = gm
  modified_base 8: mod_base = OTHER; note = 2'-O-methyl-adenosine
  modified_base 9: mod_base = cm
  modified_base 10: mod_base = gm
  modified_base 11: mod_base = gm
  modified_base 12: mod_base = gm
  modified_base 13: mod_base = um
  modified_base 14: mod_base = OTHER; note = 2'-Fluoro-adenosine
  modified_base 15: mod_base = cm
  modified_base 16: mod_base = OTHER; note = 2'-Fluoro-guanosine
  modified_base 17: mod_base = gm
  modified_base 18: mod_base = OTHER; note = 2'-Fluoro-guanosine
  modified_base 19: mod_base = cm
  modified_base 20: mod_base = OTHER; note = 2'-O-methyl-adenosine
  modified_base 21: mod_base = OTHER; note = 2'-O-methyl-adenosine
  misc_feature 21^22: note = Phosphorothioate bond
  modified_base 22: mod_base = OTHER; note = 2'-O-methyl-adenosine
  misc_feature 22^23: note = Phosphorothioate bond
  modified_base 23: mod_base = OTHER; note = 2'-O-methyl-adenosine
ctgctagacgggtacgggcaaaa

SEQ ID NO: 938 - RNA, 23 nt, synthetic construct
  source 1..23: mol_type = other RNA
  modified_base 1: mod_base = um
  misc_feature 1^2: note = Phosphorothioate bond
  modified_base 2: mod_base = OTHER; note = 2'-Fluoro-cytidine
  misc_feature 2^3: note = Phosphorothioate bond
  modified_base 3: mod_base = cm
  modified_base 4: mod_base = OTHER; note = 2'-O-methyl-adenosine
  modified_base 5: mod_base = gm
  modified_base 6: mod_base = OTHER; note = 2'-Fluoro-cytidine
  modified_base 7: mod_base = um
  modified_base 8: mod_base = gm
  modified_base 9: mod_base = OTHER; note = 2'-O-methyl-adenosine
  modified_base 10: mod_base = um
  modified_base 11: mod_base = gm
  modified_base 12: mod_base = OTHER; note = 2'-O-methyl-adenosine
  modified_base 13: mod_base = cm
  modified_base 14: mod_base = OTHER; note = 2'-Fluoro-guanosine
  modified_base 15: mod_base = OTHER; note = 2'-O-methyl-adenosine
  modified_base 16: mod_base = OTHER; note = 2'-Fluoro-uridine
  modified_base 17: mod_base = gm
  modified_base 18: mod_base = OTHER; note = 2'-Fluoro-uridine
  modified_base 19: mod_base = gm
  modified_base 20: mod_base = OTHER; note = 2'-O-methyl-adenosine
  modified_base 21: mod_base = gm
  misc_feature 21^22: note = Phosphorothioate bond
  modified_base 22: mod_base = um
  misc_feature 22^23: note = Phosphorothioate bond
  modified_base 23: mod_base = gm
tccagctgatgacgatgtgagtg

SEQ ID NO: 939 - RNA, 23 nt, synthetic construct
  source 1..23: mol_type = other RNA
  modified_base 1: mod_base = OTHER; note = 2'-O-methyl-adenosine
  misc_feature 1^2: note = Phosphorothioate bond
  modified_base 2: mod_base = OTHER; note = 2'-Fluoro-uridine
  misc_feature 2^3: note = Phosphorothioate bond
  modified_base 3: mod_base = OTHER; note = 2'-O-methyl-adenosine
  modified_base 4: mod_base = cm
  modified_base 5: mod_base = gm
  modified_base 6: mod_base = OTHER; note = 2'-Fluoro-guanosine
  modified_base 7: mod_base = OTHER; note = 2'-O-methyl-adenosine
  modified_base 8: mod_base = cm
  modified_base 9: mod_base = cm
  modified_base 10: mod_base = OTHER; note = 2'-O-methyl-adenosine
  modified_base 11: mod_base = cm
  modified_base 12: mod_base = gm
  modified_base 13: mod_base = cm
  modified_base 14: mod_base = OTHER; note = 2'-Fluoro-adenosine
  modified_base 15: mod_base = gm
  modified_base 16: mod_base = OTHER; note = 2'-Fluoro-uridine
  modified_base 17: mod_base = cm
  modified_base 18: mod_base = OTHER; note = 2'-Fluoro-uridine
  modified_base 19: mod_base = OTHER; note = 2'-O-methyl-adenosine
  modified_base 20: mod_base = um
  modified_base 21: mod_base = OTHER; note = 2'-O-methyl-adenosine
  misc_feature 21^22: note = Phosphorothioate bond
  modified_base 22: mod_base = OTHER; note = 2'-O-methyl-adenosine
  misc_feature 22^23: note = Phosphorothioate bond
  modified_base 23: mod_base = um
atacggaccacgcagtctataat

SEQ ID NO: 940 - RNA, 23 nt, synthetic construct
  source 1..23: mol_type = other RNA
  modified_base 1: mod_base = OTHER; note = 2'-O-methyl-adenosine
  misc_feature 1^2: note = Phosphorothioate bond
  modified_base 2: mod_base = OTHER; note = 2'-Fluoro-adenosine
  misc_feature 2^3: note = Phosphorothioate bond
  modified_base 3: mod_base = cm
  modified_base 4: mod_base = cm
  modified_base 5: mod_base = OTHER; note = 2'-O-methyl-adenosine
  modified_base 6: mod_base = OTHER; note = 2'-Fluoro-guanosine
  modified_base 7: mod_base = gm
  modified_base 8: mod_base = cm
  modified_base 9: mod_base = OTHER; note = 2'-O-methyl-adenosine
  modified_base 10: mod_base = gm
  modified_base 11: mod_base = um
  modified_base 12: mod_base = cm
  modified_base 13: mod_base = OTHER; note = 2'-O-methyl-adenosine
  modified_base 14: mod_base = OTHER; note = 2'-Fluoro-cytidine
  modified_base 15: mod_base = cm
  modified_base 16: mod_base = OTHER; note = 2'-Fluoro-guanosine
  modified_base 17: mod_base = OTHER; note = 2'-O-methyl-adenosine
  modified_base 18: mod_base = OTHER; note = 2'-Fluoro-guanosine
  modified_base 19: mod_base = gm
  modified_base 20: mod_base = cm
  modified_base 21: mod_base = cm
  misc_feature 21^22: note = Phosphorothioate bond
  modified_base 22: mod_base = um
  misc_feature 22^23: note = Phosphorothioate bond
  modified_base 23: mod_base = cm
aaccaggcagtcaccgaggcctc

SEQ ID NO: 941 - RNA, 23 nt, synthetic construct
  source 1..23: mol_type = other RNA
  modified_base 1: mod_base = um
  misc_feature 1^2: note = Phosphorothioate bond
  modified_base 2: mod_base = OTHER; note = 2'-Fluoro-guanosine
  misc_feature 2^3: note = Phosphorothioate bond
  modified_base 3: mod_base = OTHER; note = 2'-O-methyl-adenosine
  modified_base 4: mod_base = cm
  modified_base 5: mod_base = OTHER; note = 2'-O-methyl-adenosine
  modified_base 6: mod_base = OTHER; note = 2'-Fluoro-guanosine
  modified_base 7: mod_base = um
  modified_base 8: mod_base = cm
  modified_base 9: mod_base = um
  modified_base 10: mod_base = gm
  modified_base 11: mod_base = um
  modified_base 12: mod_base = gm
  modified_base 13: mod_base = cm
  modified_base 14: mod_base = OTHER; note = 2'-Fluoro-guanosine
  modified_base 15: mod_base = OTHER; note = 2'-O-methyl-adenosine
  modified_base 16: mod_base = OTHER; note = 2'-Fluoro-uridine
  modified_base 17: mod_base = cm
  modified_base 18: mod_base = OTHER; note = 2'-Fluoro-adenosine
  modified_base 19: mod_base = um
  modified_base 20: mod_base = cm
  modified_base 21: mod_base = cm
  misc_feature 21^22: note = Phosphorothioate bond
  modified_base 22: mod_base = OTHER; note = 2'-O-methyl-adenosine
  misc_feature 22^23: note = Phosphorothioate bond
  modified_base 23: mod_base = gm
tgacagtctgtgcgatcatccag

SEQ ID NO: 942 - RNA, 23 nt, synthetic construct
  source 1..23: mol_type = other RNA
  modified_base 1: mod_base = um
  misc_feature 1^2: note = Phosphorothioate bond
  modified_base 2: mod_base = OTHER; note = 2'-Fluoro-adenosine
  misc_feature 2^3: note = Phosphorothioate bond
  modified_base 3: mod_base = gm
  modified_base 4: mod_base = OTHER; note = 2'-O-methyl-adenosine
  modified_base 5: mod_base = cm
  modified_base 6: mod_base = OTHER; note = 2'-Fluoro-guanosine
  modified_base 7: mod_base = gm
  modified_base 8: mod_base = gm
  modified_base 9: mod_base = um
  modified_base 10: mod_base = OTHER; note = 2'-O-methyl-adenosine
  modified_base 11: mod_base = cm
  modified_base 12: mod_base = gm
  modified_base 13: mod_base = gm
  modified_base 14: mod_base = OTHER; note = 2'-Fluoro-guanosine
  modified_base 15: mod_base = cm
  modified_base 16: mod_base = OTHER; note = 2'-Fluoro-adenosine
  modified_base 17: mod_base = OTHER; note = 2'-O-methyl-adenosine
  modified_base 18: mod_base = OTHER; note = 2'-Fluoro-adenosine
  modified_base 19: mod_base = OTHER; note = 2'-O-methyl-adenosine
  modified_base 20: mod_base = um
  modified_base 21: mod_base = cm
  misc_feature 21^22: note = Phosphorothioate bond
  modified_base 22: mod_base = OTHER; note = 2'-O-methyl-adenosine
  misc_feature 22^23: note = Phosphorothioate bond
  modified_base 23: mod_base = OTHER; note = 2'-O-methyl-adenosine
tagacgggtacgggcaaaatcaa

SEQ ID NO: 943 - RNA, 23 nt, synthetic construct
  source 1..23: mol_type = other RNA
  modified_base 1: mod_base = gm
  misc_feature 1^2: note = Phosphorothioate bond
  modified_base 2: mod_base = OTHER; note = 2'-Fluoro-cytidine
  misc_feature 2^3: note = Phosphorothioate bond
  modified_base 3: mod_base = OTHER; note = 2'-O-methyl-adenosine
  modified_base 4: mod_base = gm
  modified_base 5: mod_base = um
  modified_base 6: mod_base = OTHER; note = 2'-Fluoro-guanosine
  modified_base 7: mod_base = OTHER; note = 2'-O-methyl-adenosine
  modified_base 8: mod_base = cm
  modified_base 9: mod_base = OTHER; note = 2'-O-methyl-adenosine
  modified_base 10: mod_base = gm
  modified_base 11: mod_base = um
  modified_base 12: mod_base = cm
  modified_base 13: mod_base = um
  modified_base 14: mod_base = OTHER; note = 2'-Fluoro-guanosine
  modified_base 15: mod_base = um
  modified_base 16: mod_base = OTHER; note = 2'-Fluoro-guanosine
  modified_base 17: mod_base = cm
  modified_base 18: mod_base = OTHER; note = 2'-Fluoro-guanosine
  modified_base 19: mod_base = OTHER; note = 2'-O-methyl-adenosine
  modified_base 20: mod_base = um
  modified_base 21: mod_base = cm
  misc_feature 21^22: note = Phosphorothioate bond
  modified_base 22: mod_base = OTHER; note = 2'-O-methyl-adenosine
  misc_feature 22^23: note = Phosphorothioate bond
  modified_base 23: mod_base = um
gcagtgacagtctgtgcgatcat

SEQ ID NO: 944 - RNA, 23 nt, synthetic construct
  source 1..23: mol_type = other RNA
  modified_base 1: mod_base = OTHER; note = 2'-O-methyl-adenosine
  misc_feature 1^2: note = Phosphorothioate bond
  modified_base 2: mod_base = OTHER; note = 2'-Fluoro-guanosine
  misc_feature 2^3: note = Phosphorothioate bond
  modified_base 3: mod_base = um
  modified_base 4: mod_base = gm
  modified_base 5: mod_base = OTHER; note = 2'-O-methyl-adenosine
  modified_base 6: mod_base = OTHER; note = 2'-Fluoro-cytidine
  modified_base 7: mod_base = OTHER; note = 2'-O-methyl-adenosine
  modified_base 8: mod_base = gm
  modified_base 9: mod_base = um
  modified_base 10: mod_base = cm
  modified_base 11: mod_base = um
  modified_base 12: mod_base = gm
  modified_base 13: mod_base = um
  modified_base 14: mod_base = OTHER; note = 2'-Fluoro-guanosine
  modified_base 15: mod_base = cm
  modified_base 16: mod_base = OTHER; note = 2'-Fluoro-guanosine
  modified_base 17: mod_base = OTHER; note = 2'-O-methyl-adenosine
  modified_base 18: mod_base = OTHER; note = 2'-Fluoro-uridine
  modified_base 19: mod_base = cm
  modified_base 20: mod_base = OTHER; note = 2'-O-methyl-adenosine
  modified_base 21: mod_base = um
  misc_feature 21^22: note = Phosphorothioate bond
  modified_base 22: mod_base = cm
  misc_feature 22^23: note = Phosphorothioate bond
  modified_base 23: mod_base = cm
agtgacagtctgtgcgatcatcc

SEQ ID NO: 945 - RNA, 23 nt, synthetic construct
  source 1..23: mol_type = other RNA
  modified_base 1: mod_base = gm
  misc_feature 1^2: note = Phosphorothioate bond
  modified_base 2: mod_base = OTHER; note = 2'-Fluoro-cytidine
  misc_feature 2^3: note = Phosphorothioate bond
  modified_base 3: mod_base = um
  modified_base 4: mod_base = OTHER; note = 2'-O-methyl-adenosine
  modified_base 5: mod_base = gm
  modified_base 6: mod_base = OTHER; note = 2'-Fluoro-adenosine
  modified_base 7: mod_base = cm
  modified_base 8: mod_base = gm
  modified_base 9: mod_base = gm
  modified_base 10: mod_base = gm
  modified_base 11: mod_base = um
  modified_base 12: mod_base = OTHER; note = 2'-O-methyl-adenosine
  modified_base 13: mod_base = cm
  modified_base 14: mod_base = OTHER; note = 2'-Fluoro-guanosine
  modified_base 15: mod_base = gm
  modified_base 16: mod_base = OTHER; note = 2'-Fluoro-guanosine
  modified_base 17: mod_base = cm
  modified_base 18: mod_base = OTHER; note = 2'-Fluoro-adenosine
  modified_base 19: mod_base = OTHER; note = 2'-O-methyl-adenosine
  modified_base 20: mod_base = OTHER; note = 2'-O-methyl-adenosine
  modified_base 21: mod_base = OTHER; note = 2'-O-methyl-adenosine
  misc_feature 21^22: note = Phosphorothioate bond
  modified_base 22: mod_base = um
  misc_feature 22^23: note = Phosphorothioate bond
  modified_base 23: mod_base = cm
gctagacgggtacgggcaaaatc

SEQ ID NO: 946 - RNA, 23 nt, synthetic construct
  source 1..23: mol_type = other RNA
  modified_base 1: mod_base = OTHER; note = 2'-O-methyl-adenosine
  misc_feature 1^2: note = Phosphorothioate bond
  modified_base 2: mod_base = OTHER; note = 2'-Fluoro-guanosine
  misc_feature 2^3: note = Phosphorothioate bond
  modified_base 3: mod_base = um
  modified_base 4: mod_base = OTHER; note = 2'-O-methyl-adenosine
  modified_base 5: mod_base = gm
  modified_base 6: mod_base = OTHER; note = 2'-Fluoro-guanosine
  modified_base 7: mod_base = cm
  modified_base 8: mod_base = gm
  modified_base 9: mod_base = gm
  modified_base 10: mod_base = cm
  modified_base 11: mod_base = um
  modified_base 12: mod_base = cm
  modified_base 13: mod_base = gm
  modified_base 14: mod_base = OTHER; note = 2'-Fluoro-guanosine
  modified_base 15: mod_base = um
  modified_base 16: mod_base = OTHER; note = 2'-Fluoro-adenosine
  modified_base 17: mod_base = gm
  modified_base 18: mod_base = OTHER; note = 2'-Fluoro-adenosine
  modified_base 19: mod_base = um
  modified_base 20: mod_base = gm
  modified_base 21: mod_base = OTHER; note = 2'-O-methyl-adenosine
  misc_feature 21^22: note = Phosphorothioate bond
  modified_base 22: mod_base = um
  misc_feature 22^23: note = Phosphorothioate bond
  modified_base 23: mod_base = OTHER; note = 2'-O-methyl-adenosine
agtaggcggctcggtagatgata

SEQ ID NO: 947 - RNA, 23 nt, synthetic construct
  source 1..23: mol_type = other RNA
  modified_base 1: mod_base = gm
  misc_feature 1^2: note = Phosphorothioate bond
  modified_base 2: mod_base = OTHER; note = 2'-Fluoro-adenosine
  misc_feature 2^3: note = Phosphorothioate bond
  modified_base 3: mod_base = OTHER; note = 2'-O-methyl-adenosine
  modified_base 4: mod_base = um
  modified_base 5: mod_base = OTHER; note = 2'-O-methyl-adenosine
  modified_base 6: mod_base = OTHER; note = 2'-Fluoro-cytidine
  modified_base 7: mod_base = gm
  modified_base 8: mod_base = gm
  modified_base 9: mod_base = OTHER; note = 2'-O-methyl-adenosine
  modified_base 10: mod_base = cm
  modified_base 11: mod_base = cm
  modified_base 12: mod_base = OTHER; note = 2'-O-methyl-adenosine
  modified_base 13: mod_base = cm
  modified_base 14: mod_base = OTHER; note = 2'-Fluoro-guanosine
  modified_base 15: mod_base = cm
  modified_base 16: mod_base = OTHER; note = 2'-Fluoro-adenosine
  modified_base 17: mod_base = gm
  modified_base 18: mod_base = OTHER; note = 2'-Fluoro-uridine
  modified_base 19: mod_base = cm
  modified_base 20: mod_base = um
  modified_base 21: mod_base = OTHER; note = 2'-O-methyl-adenosine
  misc_feature 21^22: note = Phosphorothioate bond
  modified_base 22: mod_base = um
  misc_feature 22^23: note = Phosphorothioate bond
  modified_base 23: mod_base = OTHER; note = 2'-O-methyl-adenosine
gaatacggaccacgcagtctata

SEQ ID NO: 948 - RNA, 23 nt, synthetic construct
  source 1..23: mol_type = other RNA
  modified_base 1: mod_base = cm
  misc_feature 1^2: note = Phosphorothioate bond
  modified_base 2: mod_base = OTHER; note = 2'-Fluoro-uridine
  misc_feature 2^3: note = Phosphorothioate bond
  modified_base 3: mod_base = um
  modified_base 4: mod_base = um
  modified_base 5: mod_base = gm
  modified_base 6: mod_base = OTHER; note = 2'-Fluoro-uridine
  modified_base 7: mod_base = OTHER; note = 2'-O-methyl-adenosine
  modified_base 8: mod_base = um
  modified_base 9: mod_base = um
  modified_base 10: mod_base = gm
  modified_base 11: mod_base = cm
  modified_base 12: mod_base = um
  modified_base 13: mod_base = um
  modified_base 14: mod_base = OTHER; note = 2'-Fluoro-adenosine
  modified_base 15: mod_base = um
  modified_base 16: mod_base = OTHER; note = 2'-Fluoro-cytidine
  modified_base 17: mod_base = um
  modified_base 18: mod_base = OTHER; note = 2'-Fluoro-guanosine
  modified_base 19: mod_base = cm
  modified_base 20: mod_base = OTHER; note = 2'-O-methyl-adenosine
  modified_base 21: mod_base = gm
  misc_feature 21^22: note = Phosphorothioate bond
  modified_base 22: mod_base = um
  misc_feature 22^23: note = Phosphorothioate bond
  modified_base 23: mod_base = gm
ctttgtattgcttatctgcagtg

SEQ ID NO: 949 - RNA, 23 nt, synthetic construct
  source 1..23: mol_type = other RNA
  modified_base 1: mod_base = um
  misc_feature 1^2: note = Phosphorothioate bond
  modified_base 2: mod_base = OTHER; note = 2'-Fluoro-uridine
  misc_feature 2^3: note = Phosphorothioate bond
  modified_base 3: mod_base = um
  modified_base 4: mod_base = gm
  modified_base 5: mod_base = um
  modified_base 6: mod_base = OTHER; note = 2'-Fluoro-adenosine
  modified_base 7: mod_base = um
  modified_base 8: mod_base = um
  modified_base 9: mod_base = gm
  modified_base 10: mod_base = cm
  modified_base 11: mod_base = um
  modified_base 12: mod_base = um
  modified_base 13: mod_base = OTHER; note = 2'-O-methyl-adenosine
  modified_base 14: mod_base = OTHER; note = 2'-Fluoro-uridine
  modified_base 15: mod_base = cm
  modified_base 16: mod_base = OTHER; note = 2'-Fluoro-uridine
  modified_base 17: mod_base = gm
  modified_base 18: mod_base = OTHER; note = 2'-Fluoro-cytidine
  modified_base 19: mod_base = OTHER; note = 2'-O-methyl-adenosine
  modified_base 20: mod_base = gm
  modified_base 21: mod_base = um
  misc_feature 21^22: note = Phosphorothioate bond
  modified_base 22: mod_base = gm
  misc_feature 22^23: note = Phosphorothioate bond
  modified_base 23: mod_base = OTHER; note = 2'-O-methyl-adenosine
tttgtattgcttatctgcagtga

SEQ ID NO: 950 - RNA, 23 nt, synthetic construct
  source 1..23: mol_type = other RNA
  modified_base 1: mod_base = um
  misc_feature 1^2: note = Phosphorothioate bond
  modified_base 2: mod_base = OTHER; note = 2'-Fluoro-uridine
  misc_feature 2^3: note = Phosphorothioate bond
  modified_base 3: mod_base = gm
  modified_base 4: mod_base = um
  modified_base 5: mod_base = OTHER; note = 2'-O-methyl-adenosine
  modified_base 6: mod_base = OTHER; note = 2'-Fluoro-uridine
  modified_base 7: mod_base = um
  modified_base 8: mod_base = gm
  modified_base 9: mod_base = cm
  modified_base 10: mod_base = um
  modified_base 11: mod_base = um
  modified_base 12: mod_base = OTHER; note = 2'-O-methyl-adenosine
  modified_base 13: mod_base = um
  modified_base 14: mod_base = OTHER; note = 2'-Fluoro-cytidine
  modified_base 15: mod_base = um
  modified_base 16: mod_base = OTHER; note = 2'-Fluoro-guanosine
  modified_base 17: mod_base = cm
  modified_base 18: mod_base = OTHER; note = 2'-Fluoro-adenosine
  modified_base 19: mod_base = gm
  modified_base 20: mod_base = um
  modified_base 21: mod_base = gm
  misc_feature 21^22: note = Phosphorothioate bond
  modified_base 22: mod_base = OTHER; note = 2'-O-methyl-adenosine
  misc_feature 22^23: note = Phosphorothioate bond
  modified_base 23: mod_base = um
ttgtattgcttatctgcagtgat

SEQ ID NO: 951 - RNA, 23 nt, synthetic construct
  source 1..23: mol_type = other RNA
  modified_base 1: mod_base = um
  misc_feature 1^2: note = Phosphorothioate bond
  modified_base 2: mod_base = OTHER; note = 2'-Fluoro-adenosine
  misc_feature 2^3: note = Phosphorothioate bond
  modified_base 3: mod_base = um
  modified_base 4: mod_base = cm
  modified_base 5: mod_base = um
  modified_base 6: mod_base = OTHER; note = 2'-Fluoro-guanosine
  modified_base 7: mod_base = cm
  modified_base 8: mod_base = OTHER; note = 2'-O-methyl-adenosine
  modified_base 9: mod_base = gm
  modified_base 10: mod_base = um
  modified_base 11: mod_base = gm
  modified_base 12: mod_base = OTHER; note = 2'-O-methyl-adenosine
  modified_base 13: mod_base = um
  modified_base 14: mod_base = OTHER; note = 2'-Fluoro-cytidine
  modified_base 15: mod_base = um
  modified_base 16: mod_base = OTHER; note = 2'-Fluoro-guanosine
  modified_base 17: mod_base = cm
  modified_base 18: mod_base = OTHER; note = 2'-Fluoro-uridine
  modified_base 19: mod_base = um
  modified_base 20: mod_base = gm
  modified_base 21: mod_base = cm
  misc_feature 21^22: note = Phosphorothioate bond
  modified_base 22: mod_base = um
  misc_feature 22^23: note = Phosphorothioate bond
  modified_base 23: mod_base = gm
tatctgcagtgatctgcttgctg

SEQ ID NO: 952 - RNA, 23 nt, synthetic construct
  source 1..23: mol_type = other RNA
  modified_base 1: mod_base = gm
  misc_feature 1^2: note = Phosphorothioate bond
  modified_base 2: mod_base = OTHER; note = 2'-Fluoro-uridine
  misc_feature 2^3: note = Phosphorothioate bond
  modified_base 3: mod_base = OTHER; note = 2'-O-methyl-adenosine
  modified_base 4: mod_base = um
  modified_base 5: mod_base = um
  modified_base 6: mod_base = OTHER; note = 2'-Fluoro-guanosine
  modified_base 7: mod_base = cm
  modified_base 8: mod_base = um
  modified_base 9: mod_base = um
  modified_base 10: mod_base = OTHER; note = 2'-O-methyl-adenosine
  modified_base 11: mod_base = um
  modified_base 12: mod_base = cm
  modified_base 13: mod_base = um
  modified_base 14: mod_base = OTHER; note = 2'-Fluoro-guanosine
  modified_base 15: mod_base = cm
  modified_base 16: mod_base = OTHER; note = 2'-Fluoro-adenosine
  modified_base 17: mod_base = gm
  modified_base 18: mod_base = OTHER; note = 2'-Fluoro-uridine
  modified_base 19: mod_base = gm
  modified_base 20: mod_base = OTHER; note = 2'-O-methyl-adenosine
  modified_base 21: mod_base = um
  misc_feature 21^22: note = Phosphorothioate bond
  modified_base 22: mod_base = cm
  misc_feature 22^23: note = Phosphorothioate bond
  modified_base 23: mod_base = um
gtattgcttatctgcagtgatct

SEQ ID NO: 953 - RNA, 23 nt, synthetic construct
  source 1..23: mol_type = other RNA
  modified_base 1: mod_base = um
  misc_feature 1^2: note = Phosphorothioate bond
  modified_base 2: mod_base = OTHER; note = 2'-Fluoro-guanosine
  misc_feature 2^3: note = Phosphorothioate bond
  modified_base 3: mod_base = um
  modified_base 4: mod_base = OTHER; note = 2'-O-methyl-adenosine
  modified_base 5: mod_base = um
  modified_base 6: mod_base = OTHER; note = 2'-Fluoro-uridine
  modified_base 7: mod_base = gm
  modified_base 8: mod_base = cm
  modified_base 9: mod_base = um
  modified_base 10: mod_base = um
  modified_base 11: mod_base = OTHER; note = 2'-O-methyl-adenosine
  modified_base 12: mod_base = um
  modified_base 13: mod_base = cm
  modified_base 14: mod_base = OTHER; note = 2'-Fluoro-uridine
  modified_base 15: mod_base = gm
  modified_base 16: mod_base = OTHER; note = 2'-Fluoro-cytidine
  modified_base 17: mod_base = OTHER; note = 2'-O-methyl-adenosine
  modified_base 18: mod_base = OTHER; note = 2'-Fluoro-guanosine
  modified_base 19: mod_base = um
  modified_base 20: mod_base = gm
  modified_base 21: mod_base = OTHER; note = 2'-O-methyl-adenosine
  misc_feature 21^22: note = Phosphorothioate bond
  modified_base 22: mod_base = um
  misc_feature 22^23: note = Phosphorothioate bond
  modified_base 23: mod_base = cm
tgtattgcttatctgcagtgatc

SEQ ID NO: 954 - RNA, 23 nt, synthetic construct
  source 1..23: mol_type = other RNA
  modified_base 1: mod_base = um
  misc_feature 1^2: note = Phosphorothioate bond
  modified_base 2: mod_base = OTHER; note = 2'-Fluoro-guanosine
  misc_feature 2^3: note = Phosphorothioate bond
  modified_base 3: mod_base = cm
  modified_base 4: mod_base = um
  modified_base 5: mod_base = um
  modified_base 6: mod_base = OTHER; note = 2'-Fluoro-adenosine
  modified_base 7: mod_base = um
  modified_base 8: mod_base = cm
  modified_base 9: mod_base = um
  modified_base 10: mod_base = gm
  modified_base 11: mod_base = cm
  modified_base 12: mod_base = OTHER; note = 2'-O-methyl-adenosine
  modified_base 13: mod_base = gm
  modified_base 14: mod_base = OTHER; note = 2'-Fluoro-uridine
  modified_base 15: mod_base = gm
  modified_base 16: mod_base = OTHER; note = 2'-Fluoro-adenosine
  modified_base 17: mod_base = um
  modified_base 18: mod_base = OTHER; note = 2'-Fluoro-cytidine
  modified_base 19: mod_base = um
  modified_base 20: mod_base = gm
  modified_base 21: mod_base = cm
  misc_feature 21^22: note = Phosphorothioate bond
  modified_base 22: mod_base = um
  misc_feature 22^23: note = Phosphorothioate bond
  modified_base 23: mod_base = um
tgcttatctgcagtgatctgctt

SEQ ID NO: 955 - RNA, 23 nt, synthetic construct
  source 1..23: mol_type = other RNA
  modified_base 1: mod_base = um
  misc_feature 1^2: note = Phosphorothioate bond
  modified_base 2: mod_base = OTHER; note = 2'-Fluoro-uridine
  misc_feature 2^3: note = Phosphorothioate bond
  modified_base 3: mod_base = gm
  modified_base 4: mod_base = cm
  modified_base 5: mod_base = um
  modified_base 6: mod_base = OTHER; note = 2'-Fluoro-uridine
  modified_base 7: mod_base = OTHER; note = 2'-O-methyl-adenosine
  modified_base 8: mod_base = um
  modified_base 9: mod_base = cm
  modified_base 10: mod_base = um
  modified_base 11: mod_base = gm
  modified_base 12: mod_base = cm
  modified_base 13: mod_base = OTHER; note = 2'-O-methyl-adenosine
  modified_base 14: mod_base = OTHER; note = 2'-Fluoro-guanosine
  modified_base 15: mod_base = um
  modified_base 16: mod_base = OTHER; note = 2'-Fluoro-guanosine
  modified_base 17: mod_base = OTHER; note = 2'-O-methyl-adenosine
  modified_base 18: mod_base = OTHER; note = 2'-Fluoro-uridine
  modified_base 19: mod_base = cm
  modified_base 20: mod_base = um
  modified_base 21: mod_base = gm
  misc_feature 21^22: note = Phosphorothioate bond
  modified_base 22: mod_base = cm
  misc_feature 22^23: note = Phosphorothioate bond
  modified_base 23: mod_base = um
ttgcttatctgcagtgatctgct

SEQ ID NO: 956 - RNA, 23 nt, synthetic construct
  source 1..23: mol_type = other RNA
  modified_base 1: mod_base = OTHER; note = 2'-O-methyl-adenosine
  misc_feature 1^2: note = Phosphorothioate bond
  modified_base 2: mod_base = OTHER; note = 2'-Fluoro-uridine
  misc_feature 2^3: note = Phosphorothioate bond
  modified_base 3: mod_base = cm
  modified_base 4: mod_base = um
  modified_base 5: mod_base = gm
  modified_base 6: mod_base = OTHER; note = 2'-Fluoro-cytidine
  modified_base 7: mod_base = OTHER; note = 2'-O-methyl-adenosine
  modified_base 8: mod_base = gm
  modified_base 9: mod_base = um
  modified_base 10: mod_base = gm
  modified_base 11: mod_base = OTHER; note = 2'-O-methyl-adenosine
  modified_base 12: mod_base = um
  modified_base 13: mod_base = cm
  modified_base 14: mod_base = OTHER; note = 2'-Fluoro-uridine
  modified_base 15: mod_base = gm
  modified_base 16: mod_base = OTHER; note = 2'-Fluoro-cytidine
  modified_base 17: mod_base = um
  modified_base 18: mod_base = OTHER; note = 2'-Fluoro-uridine
  modified_base 19: mod_base = gm
  modified_base 20: mod_base = cm
  modified_base 21: mod_base = um
  misc_feature 21^22: note = Phosphorothioate bond
  modified_base 22: mod_base = gm
  misc_feature 22^23: note = Phosphorothioate bond
  modified_base 23: mod_base = gm
atctgcagtgatctgcttgctgg

SEQ ID NO: 957 - RNA, 23 nt, synthetic construct
  source 1..23: mol_type = other RNA
  modified_base 1: mod_base = um
  misc_feature 1^2: note = Phosphorothioate bond
  modified_base 2: mod_base = OTHER; note = 2'-Fluoro-adenosine
  misc_feature 2^3: note = Phosphorothioate bond
  modified_base 3: mod_base = um
  modified_base 4: mod_base = um
  modified_base 5: mod_base = gm
  modified_base 6: mod_base = OTHER; note = 2'-Fluoro-cytidine
  modified_base 7: mod_base = um
  modified_base 8: mod_base = um
  modified_base 9: mod_base = OTHER; note = 2'-O-methyl-adenosine
  modified_base 10: mod_base = um
  modified_base 11: mod_base = cm
  modified_base 12: mod_base = um
  modified_base 13: mod_base = gm
  modified_base 14: mod_base = OTHER; note = 2'-Fluoro-cytidine
  modified_base 15: mod_base = OTHER; note = 2'-O-methyl-adenosine
  modified_base 16: mod_base = OTHER; note = 2'-Fluoro-guanosine
  modified_base 17: mod_base = um
  modified_base 18: mod_base = OTHER; note = 2'-Fluoro-guanosine
  modified_base 19: mod_base = OTHER; note = 2'-O-methyl-adenosine
  modified_base 20: mod_base = um
  modified_base 21: mod_base = cm
  misc_feature 21^22: note = Phosphorothioate bond
  modified_base 22: mod_base = um
  misc_feature 22^23: note = Phosphorothioate bond
  modified_base 23: mod_base = gm
tattgcttatctgcagtgatctg

SEQ ID NO: 958 - RNA, 23 nt, synthetic construct
  source 1..23: mol_type = other RNA
  modified_base 1: mod_base = um
  misc_feature 1^2: note = Phosphorothioate bond
  modified_base 2: mod_base = OTHER; note = 2'-Fluoro-uridine
  misc_feature 2^3: note = Phosphorothioate bond
  modified_base 3: mod_base = cm
  modified_base 4: mod_base = um
  modified_base 5: mod_base = cm
  modified_base 6: mod_base = OTHER; note = 2'-Fluoro-cytidine
  modified_base 7: mod_base = OTHER; note = 2'-O-methyl-adenosine
  modified_base 8: mod_base = OTHER; note = 2'-O-methyl-adenosine
  modified_base 9: mod_base = OTHER; note = 2'-O-methyl-adenosine
  modified_base 10: mod_base = um
  modified_base 11: mod_base = um
  modified_base 12: mod_base = um
  modified_base 13: mod_base = gm
  modified_base 14: mod_base = OTHER; note = 2'-Fluoro-uridine
  modified_base 15: mod_base = um
  modified_base 16: mod_base = OTHER; note = 2'-Fluoro-adenosine
  modified_base 17: mod_base = um
  modified_base 18: mod_base = OTHER; note = 2'-Fluoro-uridine
  modified_base 19: mod_base = um
  modified_base 20: mod_base = OTHER; note = 2'-O-methyl-adenosine
  modified_base 21: mod_base = um
  misc_feature 21^22: note = Phosphorothioate bond
  modified_base 22: mod_base = cm
  misc_feature 22^23: note = Phosphorothioate bond
  modified_base 23: mod_base = OTHER; note = 2'-O-methyl-adenosine
ttctccaaatttgttatttatca

SEQ ID NO: 959 - RNA, 23 nt, synthetic construct
  source 1..23: mol_type = other RNA
  modified_base 1: mod_base = cm
  misc_feature 1^2: note = Phosphorothioate bond
  modified_base 2: mod_base = OTHER; note = 2'-Fluoro-adenosine
  misc_feature 2^3: note = Phosphorothioate bond
  modified_base 3: mod_base = OTHER; note = 2'-O-methyl-adenosine
  modified_base 4: mod_base = OTHER; note = 2'-O-methyl-adenosine
  modified_base 5: mod_base = um
  modified_base 6: mod_base = OTHER; note = 2'-Fluoro-uridine
  modified_base 7: mod_base = um
  modified_base 8: mod_base = gm
  modified_base 9: mod_base = um
  modified_base 10: mod_base = um
  modified_base 11: mod_base = OTHER; note = 2'-O-methyl-adenosine
  modified_base 12: mod_base = um
  modified_base 13: mod_base = um
  modified_base 14: mod_base = OTHER; note = 2'-Fluoro-uridine
  modified_base 15: mod_base = OTHER; note = 2'-O-methyl-adenosine
  modified_base 16: mod_base = OTHER; note = 2'-Fluoro-uridine
  modified_base 17: mod_base = cm
  modified_base 18: mod_base = OTHER; note = 2'-Fluoro-adenosine
  modified_base 19: mod_base = gm
  modified_base 20: mod_base = gm
  modified_base 21: mod_base = OTHER; note = 2'-O-methyl-adenosine
  misc_feature 21^22: note = Phosphorothioate bond
  modified_base 22: mod_base = gm
  misc_feature 22^23: note = Phosphorothioate bond
  modified_base 23: mod_base = um
caaatttgttatttatcaggagt

SEQ ID NO: 960 - RNA, 23 nt, synthetic construct
  source 1..23: mol_type = other RNA
  modified_base 1: mod_base = gm
  misc_feature 1^2: note = Phosphorothioate bond
  modified_base 2: mod_base = OTHER; note = 2'-Fluoro-adenosine
  misc_feature 2^3: note = Phosphorothioate bond
  modified_base 3: mod_base = gm
  modified_base 4: mod_base = gm
  modified_base 5: mod_base = cm
  modified_base 6: mod_base = OTHER; note = 2'-Fluoro-cytidine
  modified_base 7: mod_base = um
  modified_base 8: mod_base = cm
  modified_base 9: mod_base = gm
  modified_base 10: mod_base = gm
  modified_base 11: mod_base = OTHER; note = 2'-O-methyl-adenosine
  modified_base 12: mod_base = OTHER; note = 2'-O-methyl-adenosine
  modified_base 13: mod_base = um
  modified_base 14: mod_base = OTHER; note = 2'-Fluoro-uridine
  modified_base 15: mod_base = cm
  modified_base 16: mod_base = OTHER; note = 2'-Fluoro-cytidine
  modified_base 17: mod_base = cm
  modified_base 18: mod_base = OTHER; note = 2'-Fluoro-uridine
  modified_base 19: mod_base = um
  modified_base 20: mod_base = um
  modified_base 21: mod_base = cm
  misc_feature 21^22: note = Phosphorothioate bond
  modified_base 22: mod_base = OTHER; note = 2'-O-methyl-adenosine
  misc_feature 22^23: note = Phosphorothioate bond
  modified_base 23: mod_base = gm
gaggcctcggaattccctttcag

SEQ ID NO: 961 - RNA, 23 nt, synthetic construct
  source 1..23: mol_type = other RNA
  modified_base 1: mod_base = OTHER; note = 2'-O-methyl-adenosine
  misc_feature 1^2: note = Phosphorothioate bond
  modified_base 2: mod_base = OTHER; note = 2'-Fluoro-guanosine
  misc_feature 2^3: note = Phosphorothioate bond
  modified_base 3: mod_base = OTHER; note = 2'-O-methyl-adenosine
  modified_base 4: mod_base = um
  modified_base 5: mod_base = OTHER; note = 2'-O-methyl-adenosine
  modified_base 6: mod_base = OTHER; note = 2'-Fluoro-uridine
  modified_base 7: mod_base = gm
  modified_base 8: mod_base = um
  modified_base 9: mod_base = um
  modified_base 10: mod_base = OTHER; note = 2'-O-methyl-adenosine
  modified_base 11: mod_base = um
  modified_base 12: mod_base = OTHER; note = 2'-O-methyl-adenosine
  modified_base 13: mod_base = um
  modified_base 14: mod_base = OTHER; note = 2'-Fluoro-adenosine
  modified_base 15: mod_base = OTHER; note = 2'-O-methyl-adenosine
  modified_base 16: mod_base = OTHER; note = 2'-Fluoro-uridine
  modified_base 17: mod_base = OTHER; note = 2'-O-methyl-adenosine
  modified_base 18: mod_base = OTHER; note = 2'-Fluoro-cytidine
  modified_base 19: mod_base = OTHER; note = 2'-O-methyl-adenosine
  modified_base 20: mod_base = OTHER; note = 2'-O-methyl-adenosine
  modified_base 21: mod_base = cm
  misc_feature 21^22: note = Phosphorothioate bond
  modified_base 22: mod_base = OTHER; note = 2'-O-methyl-adenosine
  misc_feature 22^23: note = Phosphorothioate bond
  modified_base 23: mod_base = um
agatatgttatataatacaacat

SEQ ID NO: 962 - RNA, 23 nt, synthetic construct
  source 1..23: mol_type = other RNA
  modified_base 1: mod_base = gm
  misc_feature 1^2: note = Phosphorothioate bond
  modified_base 2: mod_base = OTHER; note = 2'-Fluoro-cytidine
  misc_feature 2^3: note = Phosphorothioate bond
  modified_base 3: mod_base = OTHER; note = 2'-O-methyl-adenosine
  modified_base 4: mod_base = gm
  modified_base 5: mod_base = um
  modified_base 6: mod_base = OTHER; note = 2'-Fluoro-cytidine
  modified_base 7: mod_base = OTHER; note = 2'-O-methyl-adenosine
  modified_base 8: mod_base = cm
  modified_base 9: mod_base = cm
  modified_base 10: mod_base = gm
  modified_base 11: mod_base = OTHER; note = 2'-O-methyl-adenosine
  modified_base 12: mod_base = gm
  modified_base 13: mod_base = gm
  modified_base 14: mod_base = OTHER; note = 2'-Fluoro-cytidine
  modified_base 15: mod_base = cm
  modified_base 16: mod_base = OTHER; note = 2'-Fluoro-uridine
  modified_base 17: mod_base = cm
  modified_base 18: mod_base = OTHER; note = 2'-Fluoro-guanosine
  modified_base 19: mod_base = gm
  modified_base 20: mod_base = OTHER; note = 2'-O-methyl-adenosine
  modified_base 21: mod_base = OTHER; note = 2'-O-methyl-adenosine
  misc_feature 21^22: note = Phosphorothioate bond
  modified_base 22: mod_base = um
  misc_feature 22^23: note = Phosphorothioate bond
  modified_base 23: mod_base = um
gcagtcaccgaggcctcggaatt

SEQ ID NO: 963 - RNA, 23 nt, synthetic construct
  source 1..23: mol_type = other RNA
  modified_base 1: mod_base = cm
  misc_feature 1^2: note = Phosphorothioate bond
  modified_base 2: mod_base = OTHER; note = 2'-Fluoro-guanosine
  misc_feature 2^3: note = Phosphorothioate bond
  modified_base 3: mod_base = OTHER; note = 2'-O-methyl-adenosine
  modified_base 4: mod_base = gm
  modified_base 5: mod_base = gm
  modified_base 6: mod_base = OTHER; note = 2'-Fluoro-cytidine
  modified_base 7: mod_base = cm
  modified_base 8: mod_base = um
  modified_base 9: mod_base = cm
  modified_base 10: mod_base = gm
  modified_base 11: mod_base = gm
  modified_base 12: mod_base = OTHER; note = 2'-O-methyl-adenosine
  modified_base 13: mod_base = OTHER; note = 2'-O-methyl-adenosine
  modified_base 14: mod_base = OTHER; note = 2'-Fluoro-uridine
  modified_base 15: mod_base = um
  modified_base 16: mod_base = OTHER; note = 2'-Fluoro-cytidine
  modified_base 17: mod_base = cm
  modified_base 18: mod_base = OTHER; note = 2'-Fluoro-cytidine
  modified_base 19: mod_base = um
  modified_base 20: mod_base = um
  modified_base 21: mod_base = um
  misc_feature 21^22: note = Phosphorothioate bond
  modified_base 22: mod_base = cm
  misc_feature 22^23: note = Phosphorothioate bond
  modified_base 23: mod_base = OTHER; note = 2'-O-methyl-adenosine
cgaggcctcggaattccctttca

SEQ ID NO: 964 - RNA, 23 nt, synthetic construct
  source 1..23: mol_type = other RNA
  modified_base 1: mod_base = cm
  misc_feature 1^2: note = Phosphorothioate bond
  modified_base 2: mod_base = OTHER; note = 2'-Fluoro-adenosine
  misc_feature 2^3: note = Phosphorothioate bond
  modified_base 3: mod_base = OTHER; note = 2'-O-methyl-adenosine
  modified_base 4: mod_base = gm
  modified_base 5: mod_base = OTHER; note = 2'-O-methyl-adenosine
  modified_base 6: mod_base = OTHER; note = 2'-Fluoro-uridine
  modified_base 7: mod_base = OTHER; note = 2'-O-methyl-adenosine
  modified_base 8: mod_base = um
  modified_base 9: mod_base = gm
  modified_base 10: mod_base = um
  modified_base 11: mod_base = um
  modified_base 12: mod_base = OTHER; note = 2'-O-methyl-adenosine
  modified_base 13: mod_base = um
  modified_base 14: mod_base = OTHER; note = 2'-Fluoro-adenosine
  modified_base 15: mod_base = um
  modified_base 16: mod_base = OTHER; note = 2'-Fluoro-adenosine
  modified_base 17: mod_base = OTHER; note = 2'-O-methyl-adenosine
  modified_base 18: mod_base = OTHER; note = 2'-Fluoro-uridine
  modified_base 19: mod_base = OTHER; note = 2'-O-methyl-adenosine
  modified_base 20: mod_base = cm
  modified_base 21: mod_base = OTHER; note = 2'-O-methyl-adenosine
  misc_feature 21^22: note = Phosphorothioate bond
  modified_base 22: mod_base = OTHER; note = 2'-O-methyl-adenosine
  misc_feature 22^23: note = Phosphorothioate bond
  modified_base 23: mod_base = cm
caagatatgttatataatacaac

SEQ ID NO: 965 - RNA, 23 nt, synthetic construct
  source 1..23: mol_type = other RNA
  modified_base 1: mod_base = OTHER; note = 2'-O-methyl-adenosine
  misc_feature 1^2: note = Phosphorothioate bond
  modified_base 2: mod_base = OTHER; note = 2'-Fluoro-guanosine
  misc_feature 2^3: note = Phosphorothioate bond
  modified_base 3: mod_base = um
  modified_base 4: mod_base = cm
  modified_base 5: mod_base = OTHER; note = 2'-O-methyl-adenosine
  modified_base 6: mod_base = OTHER; note = 2'-Fluoro-cytidine
  modified_base 7: mod_base = cm
  modified_base 8: mod_base = gm
  modified_base 9: mod_base = OTHER; note = 2'-O-methyl-adenosine
  modified_base 10: mod_base = gm
  modified_base 11: mod_base = gm
  modified_base 12: mod_base = cm
  modified_base 13: mod_base = cm
  modified_base 14: mod_base = OTHER; note = 2'-Fluoro-uridine
  modified_base 15: mod_base = cm
  modified_base 16: mod_base = OTHER; note = 2'-Fluoro-guanosine
  modified_base 17: mod_base = gm
  modified_base 18: mod_base = OTHER; note = 2'-Fluoro-adenosine
  modified_base 19: mod_base = OTHER; note = 2'-O-methyl-adenosine
  modified_base 20: mod_base = um
  modified_base 21: mod_base = um
  misc_feature 21^22: note = Phosphorothioate bond
  modified_base 22: mod_base = cm
  misc_feature 22^23: note = Phosphorothioate bond
  modified_base 23: mod_base = cm
agtcaccgaggcctcggaattcc

SEQ ID NO: 966 - RNA, 23 nt, synthetic construct
  source 1..23: mol_type = other RNA
  modified_base 1: mod_base = cm
  misc_feature 1^2: note = Phosphorothioate bond
  modified_base 2: mod_base = OTHER; note = 2'-Fluoro-adenosine
  misc_feature 2^3: note = Phosphorothioate bond
  modified_base 3: mod_base = cm
  modified_base 4: mod_base = cm
  modified_base 5: mod_base = gm
  modified_base 6: mod_base = OTHER; note = 2'-Fluoro-adenosine
  modified_base 7: mod_base = gm
  modified_base 8: mod_base = gm
  modified_base 9: mod_base = cm
  modified_base 10: mod_base = cm
  modified_base 11: mod_base = um
  modified_base 12: mod_base = cm
  modified_base 13: mod_base = gm
  modified_base 14: mod_base = OTHER; note = 2'-Fluoro-guanosine
  modified_base 15: mod_base = OTHER; note = 2'-O-methyl-adenosine
  modified_base 16: mod_base = OTHER; note = 2'-Fluoro-adenosine
  modified_base 17: mod_base = um
  modified_base 18: mod_base = OTHER; note = 2'-Fluoro-uridine
  modified_base 19: mod_base = cm
  modified_base 20: mod_base = cm
  modified_base 21: mod_base = cm
  misc_feature 21^22: note = Phosphorothioate bond
  modified_base 22: mod_base = um
  misc_feature 22^23: note = Phosphorothioate bond
  modified_base 23: mod_base = um
caccgaggcctcggaattccctt

SEQ ID NO: 967 - RNA, 23 nt, synthetic construct
  source 1..23: mol_type = other RNA
  modified_base 1: mod_base = cm
  misc_feature 1^2: note = Phosphorothioate bond
  modified_base 2: mod_base = OTHER; note = 2'-Fluoro-cytidine
  misc_feature 2^3: note = Phosphorothioate bond
  modified_base 3: mod_base = um
  modified_base 4: mod_base = cm
  modified_base 5: mod_base = gm
  modified_base 6: mod_base = OTHER; note = 2'-Fluoro-guanosine
  modified_base 7: mod_base = OTHER; note = 2'-O-methyl-adenosine
  modified_base 8: mod_base = OTHER; note = 2'-O-methyl-adenosine
  modified_base 9: mod_base = um
  modified_base 10: mod_base = um
  modified_base 11: mod_base = cm
  modified_base 12: mod_base = cm
  modified_base 13: mod_base = cm
  modified_base 14: mod_base = OTHER; note = 2'-Fluoro-uridine
  modified_base 15: mod_base = um
  modified_base 16: mod_base = OTHER; note = 2'-Fluoro-uridine
  modified_base 17: mod_base = cm
  modified_base 18: mod_base = OTHER; note = 2'-Fluoro-adenosine
  modified_base 19: mod_base = gm
  modified_base 20: mod_base = cm
  modified_base 21: mod_base = um
  misc_feature 21^22: note = Phosphorothioate bond
  modified_base 22: mod_base = cm
  misc_feature 22^23: note = Phosphorothioate bond
  modified_base 23: mod_base = cm
cctcggaattccctttcagctcc

SEQ ID NO: 968 - RNA, 23 nt, synthetic construct
  source 1..23: mol_type = other RNA
  modified_base 1: mod_base = um
  misc_feature 1^2: note = Phosphorothioate bond
  modified_base 2: mod_base = OTHER; note = 2'-Fluoro-cytidine
  misc_feature 2^3: note = Phosphorothioate bond
  modified_base 3: mod_base = gm
  modified_base 4: mod_base = gm
  modified_base 5: mod_base = OTHER; note = 2'-O-methyl-adenosine
  modified_base 6: mod_base = OTHER; note = 2'-Fluoro-adenosine
  modified_base 7: mod_base = um
  modified_base 8: mod_base = um
  modified_base 9: mod_base = cm
  modified_base 10: mod_base = cm
  modified_base 11: mod_base = cm
  modified_base 12: mod_base = um
  modified_base 13: mod_base = um
  modified_base 14: mod_base = OTHER; note = 2'-Fluoro-uridine
  modified_base 15: mod_base = cm
  modified_base 16: mod_base = OTHER; note = 2'-Fluoro-adenosine
  modified_base 17: mod_base = gm
  modified_base 18: mod_base = OTHER; note = 2'-Fluoro-cytidine
  modified_base 19: mod_base = um
  modified_base 20: mod_base = cm
  modified_base 21: mod_base = cm
  misc_feature 21^22: note = Phosphorothioate bond
  modified_base 22: mod_base = OTHER; note = 2'-O-methyl-adenosine
  misc_feature 22^23: note = Phosphorothioate bond
  modified_base 23: mod_base = gm
tcggaattccctttcagctccag

SEQ ID NO: 969 - RNA, 23 nt, synthetic construct
  source 1..23: mol_type = other RNA
  modified_base 1: mod_base = gm
  misc_feature 1^2: note = Phosphorothioate bond
  modified_base 2: mod_base = OTHER; note = 2'-Fluoro-guanosine
  misc_feature 2^3: note = Phosphorothioate bond
  modified_base 3: mod_base = cm
  modified_base 4: mod_base = cm
  modified_base 5: mod_base = um
  modified_base 6: mod_base = OTHER; note = 2'-Fluoro-cytidine
  modified_base 7: mod_base = gm
  modified_base 8: mod_base = gm
  modified_base 9: mod_base = OTHER; note = 2'-O-methyl-adenosine
  modified_base 10: mod_base = OTHER; note = 2'-O-methyl-adenosine
  modified_base 11: mod_base = um
  modified_base 12: mod_base = um
  modified_base 13: mod_base = cm
  modified_base 14: mod_base = OTHER; note = 2'-Fluoro-cytidine
  modified_base 15: mod_base = cm
  modified_base 16: mod_base = OTHER; note = 2'-Fluoro-uridine
  modified_base 17: mod_base = um
  modified_base 18: mod_base = OTHER; note = 2'-Fluoro-uridine
  modified_base 19: mod_base = cm
  modified_base 20: mod_base = OTHER; note = 2'-O-methyl-adenosine
  modified_base 21: mod_base = gm
  misc_feature 21^22: note = Phosphorothioate bond
  modified_base 22: mod_base = cm
  misc_feature 22^23: note = Phosphorothioate bond
  modified_base 23: mod_base = um
ggcctcggaattccctttcagct

SEQ ID NO: 970 - RNA, 23 nt, synthetic construct
  source 1..23: mol_type = other RNA
  modified_base 1: mod_base = cm
  misc_feature 1^2: note = Phosphorothioate bond
  modified_base 2: mod_base = OTHER; note = 2'-Fluoro-uridine
  misc_feature 2^3: note = Phosphorothioate bond
  modified_base 3: mod_base = cm
  modified_base 4: mod_base = gm
  modified_base 5: mod_base = gm
  modified_base 6: mod_base = OTHER; note = 2'-Fluoro-adenosine
  modified_base 7: mod_base = OTHER; note = 2'-O-methyl-adenosine
  modified_base 8: mod_base = um
  modified_base 9: mod_base = um
  modified_base 10: mod_base = cm
  modified_base 11: mod_base = cm
  modified_base 12: mod_base = cm
  modified_base 13: mod_base = um
  modified_base 14: mod_base = OTHER; note = 2'-Fluoro-uridine
  modified_base 15: mod_base = um
  modified_base 16: mod_base = OTHER; note = 2'-Fluoro-cytidine
  modified_base 17: mod_base = OTHER; note = 2'-O-methyl-adenosine
  modified_base 18: mod_base = OTHER; note = 2'-Fluoro-guanosine
  modified_base 19: mod_base = cm
  modified_base 20: mod_base = um
  modified_base 21: mod_base = cm
  misc_feature 21^22: note = Phosphorothioate bond
  modified_base 22: mod_base = cm
  misc_feature 22^23: note = Phosphorothioate bond
  modified_base 23: mod_base = OTHER; note = 2'-O-methyl-adenosine
ctcggaattccctttcagctcca

SEQ ID NO: 971 - RNA, 23 nt, synthetic construct
  source 1..23: mol_type = other RNA
  modified_base 1: mod_base = gm
  misc_feature 1^2: note = Phosphorothioate bond
  modified_base 2: mod_base = OTHER; note = 2'-Fluoro-cytidine
  misc_feature 2^3: note = Phosphorothioate bond
  modified_base 3: mod_base = cm
  modified_base 4: mod_base = um
  modified_base 5: mod_base = cm
  modified_base 6: mod_base = OTHER; note = 2'-Fluoro-guanosine
  modified_base 7: mod_base = gm
  modified_base 8: mod_base = OTHER; note = 2'-O-methyl-adenosine
  modified_base 9: mod_base = OTHER; note = 2'-O-methyl-adenosine
  modified_base 10: mod_base = um
  modified_base 11: mod_base = um
  modified_base 12: mod_base = cm
  modified_base 13: mod_base = cm
  modified_base 14: mod_base = OTHER; note = 2'-Fluoro-cytidine
  modified_base 15: mod_base = um
  modified_base 16: mod_base = OTHER; note = 2'-Fluoro-uridine
  modified_base 17: mod_base = um
  modified_base 18: mod_base = OTHER; note = 2'-Fluoro-cytidine
  modified_base 19: mod_base = OTHER; note = 2'-O-methyl-adenosine
  modified_base 20: mod_base = gm
  modified_base 21: mod_base = cm
  misc_feature 21^22: note = Phosphorothioate bond
  modified_base 22: mod_base = um
  misc_feature 22^23: note = Phosphorothioate bond
  modified_base 23: mod_base = cm
gcctcggaattccctttcagctc

SEQ ID NO: 972 - RNA, 23 nt, synthetic construct
  source 1..23: mol_type = other RNA
  modified_base 1: mod_base = OTHER; note = 2'-O-methyl-adenosine
  misc_feature 1^2: note = Phosphorothioate bond
  modified_base 2: mod_base = OTHER; note = 2'-Fluoro-uridine
  misc_feature 2^3: note = Phosphorothioate bond
  modified_base 3: mod_base = gm
  modified_base 4: mod_base = um
  modified_base 5: mod_base = um
  modified_base 6: mod_base = OTHER; note = 2'-Fluoro-adenosine
  modified_base 7: mod_base = um
  modified_base 8: mod_base = OTHER; note = 2'-O-methyl-adenosine
  modified_base 9: mod_base = um
  modified_base 10: mod_base = OTHER; note = 2'-O-methyl-adenosine
  modified_base 11: mod_base = OTHER; note = 2'-O-methyl-adenosine
  modified_base 12: mod_base = um
  modified_base 13: mod_base = OTHER; note = 2'-O-methyl-adenosine
  modified_base 14: mod_base = OTHER; note = 2'-Fluoro-cytidine
  modified_base 15: mod_base = OTHER; note = 2'-O-methyl-adenosine
  modified_base 16: mod_base = OTHER; note = 2'-Fluoro-adenosine
  modified_base 17: mod_base = cm
  modified_base 18: mod_base = OTHER; note = 2'-Fluoro-adenosine
  modified_base 19: mod_base = um
  modified_base 20: mod_base = gm
  modified_base 21: mod_base = cm
  misc_feature 21^22: note = Phosphorothioate bond
  modified_base 22: mod_base = cm
  misc_feature 22^23: note = Phosphorothioate bond
  modified_base 23: mod_base = um
atgttatataatacaacatgcct

SEQ ID NO: 973 - RNA, 23 nt, synthetic construct
  source 1..23: mol_type = other RNA
  modified_base 1: mod_base = OTHER; note = 2'-O-methyl-adenosine
  misc_feature 1^2: note = Phosphorothioate bond
  modified_base 2: mod_base = OTHER; note = 2'-Fluoro-adenosine
  misc_feature 2^3: note = Phosphorothioate bond
  modified_base 3: mod_base = gm
  modified_base 4: mod_base = OTHER; note = 2'-O-methyl-adenosine
  modified_base 5: mod_base = um
  modified_base 6: mod_base = OTHER; note = 2'-Fluoro-adenosine
  modified_base 7: mod_base = um
  modified_base 8: mod_base = gm
  modified_base 9: mod_base = um
  modified_base 10: mod_base = um
  modified_base 11: mod_base = OTHER; note = 2'-O-methyl-adenosine
  modified_base 12: mod_base = um
  modified_base 13: mod_base = OTHER; note = 2'-O-methyl-adenosine
  modified_base 14: mod_base = OTHER; note = 2'-Fluoro-uridine
  modified_base 15: mod_base = OTHER; note = 2'-O-methyl-adenosine
  modified_base 16: mod_base = OTHER; note = 2'-Fluoro-adenosine
  modified_base 17: mod_base = um
  modified_base 18: mod_base = OTHER; note = 2'-Fluoro-adenosine
  modified_base 19: mod_base = cm
  modified_base 20: mod_base = OTHER; note = 2'-O-methyl-adenosine
  modified_base 21: mod_base = OTHER; note = 2'-O-methyl-adenosine
  misc_feature 21^22: note = Phosphorothioate bond
  modified_base 22: mod_base = cm
  misc_feature 22^23: note = Phosphorothioate bond
  modified_base 23: mod_base = OTHER; note = 2'-O-methyl-adenosine
aagatatgttatataatacaaca

SEQ ID NO: 974 - RNA, 23 nt, synthetic construct
  source 1..23: mol_type = other RNA
  modified_base 1: mod_base = um
  misc_feature 1^2: note = Phosphorothioate bond
  modified_base 2: mod_base = OTHER; note = 2'-Fluoro-cytidine
  misc_feature 2^3: note = Phosphorothioate bond
  modified_base 3: mod_base = OTHER; note = 2'-O-methyl-adenosine
  modified_base 4: mod_base = OTHER; note = 2'-O-methyl-adenosine
  modified_base 5: mod_base = gm
  modified_base 6: mod_base = OTHER; note = 2'-Fluoro-adenosine
  modified_base 7: mod_base = um
  modified_base 8: mod_base = OTHER; note = 2'-O-methyl-adenosine
  modified_base 9: mod_base = um
  modified_base 10: mod_base = gm
  modified_base 11: mod_base = um
  modified_base 12: mod_base = um
  modified_base 13: mod_base = OTHER; note = 2'-O-methyl-adenosine
  modified_base 14: mod_base = OTHER; note = 2'-Fluoro-uridine
  modified_base 15: mod_base = OTHER; note = 2'-O-methyl-adenosine
  modified_base 16: mod_base = OTHER; note = 2'-Fluoro-uridine
  modified_base 17: mod_base = OTHER; note = 2'-O-methyl-adenosine
  modified_base 18: mod_base = OTHER; note = 2'-Fluoro-adenosine
  modified_base 19: mod_base = um
  modified_base 20: mod_base = OTHER; note = 2'-O-methyl-adenosine
  modified_base 21: mod_base = cm
  misc_feature 21^22: note = Phosphorothioate bond
  modified_base 22: mod_base = OTHER; note = 2'-O-methyl-adenosine
  misc_feature 22^23: note = Phosphorothioate bond
  modified_base 23: mod_base = OTHER; note = 2'-O-methyl-adenosine
tcaagatatgttatataatacaa

SEQ ID NO: 975 - RNA, 23 nt, synthetic construct
  source 1..23: mol_type = other RNA
  modified_base 1: mod_base = um
  misc_feature 1^2: note = Phosphorothioate bond
  modified_base 2: mod_base = OTHER; note = 2'-Fluoro-guanosine
  misc_feature 2^3: note = Phosphorothioate bond
  modified_base 3: mod_base = um
  modified_base 4: mod_base = um
  modified_base 5: mod_base = OTHER; note = 2'-O-methyl-adenosine
  modified_base 6: mod_base = OTHER; note = 2'-Fluoro-uridine
  modified_base 7: mod_base = OTHER; note = 2'-O-methyl-adenosine
  modified_base 8: mod_base = um
  modified_base 9: mod_base = OTHER; note = 2'-O-methyl-adenosine
  modified_base 10: mod_base = OTHER; note = 2'-O-methyl-adenosine
  modified_base 11: mod_base = um
  modified_base 12: mod_base = OTHER; note = 2'-O-methyl-adenosine
  modified_base 13: mod_base = cm
  modified_base 14: mod_base = OTHER; note = 2'-Fluoro-adenosine
  modified_base 15: mod_base = OTHER; note = 2'-O-methyl-adenosine
  modified_base 16: mod_base = OTHER; note = 2'-Fluoro-cytidine
  modified_base 17: mod_base = OTHER; note = 2'-O-methyl-adenosine
  modified_base 18: mod_base = OTHER; note = 2'-Fluoro-uridine
  modified_base 19: mod_base = gm
  modified_base 20: mod_base = cm
  modified_base 21: mod_base = cm
  misc_feature 21^22: note = Phosphorothioate bond
  modified_base 22: mod_base = um
  misc_feature 22^23: note = Phosphorothioate bond
  modified_base 23: mod_base = gm
tgttatataatacaacatgcctg

SEQ ID NO: 976 - RNA, 23 nt, synthetic construct
  source 1..23: mol_type = other RNA
  modified_base 1: mod_base = cm
  misc_feature 1^2: note = Phosphorothioate bond
  modified_base 2: mod_base = OTHER; note = 2'-Fluoro-cytidine
  misc_feature 2^3: note = Phosphorothioate bond
  modified_base 3: mod_base = gm
  modified_base 4: mod_base = OTHER; note = 2'-O-methyl-adenosine
  modified_base 5: mod_base = gm
  modified_base 6: mod_base = OTHER; note = 2'-Fluoro-guanosine
  modified_base 7: mod_base = cm
  modified_base 8: mod_base = cm
  modified_base 9: mod_base = um
  modified_base 10: mod_base = cm
  modified_base 11: mod_base = gm
  modified_base 12: mod_base = gm
  modified_base 13: mod_base = OTHER; note = 2'-O-methyl-adenosine
  modified_base 14: mod_base = OTHER; note = 2'-Fluoro-adenosine
  modified_base 15: mod_base = um
  modified_base 16: mod_base = OTHER; note = 2'-Fluoro-uridine
  modified_base 17: mod_base = cm
  modified_base 18: mod_base = OTHER; note = 2'-Fluoro-cytidine
  modified_base 19: mod_base = cm
  modified_base 20: mod_base = um
  modified_base 21: mod_base = um
  misc_feature 21^22: note = Phosphorothioate bond
  modified_base 22: mod_base = um
  misc_feature 22^23: note = Phosphorothioate bond
  modified_base 23: mod_base = cm
ccgaggcctcggaattccctttc

SEQ ID NO: 977 - RNA, 23 nt, synthetic construct
  source 1..23: mol_type = other RNA
  modified_base 1: mod_base = gm
  misc_feature 1^2: note = Phosphorothioate bond
  modified_base 2: mod_base = OTHER; note = 2'-Fluoro-uridine
  misc_feature 2^3: note = Phosphorothioate bond
  modified_base 3: mod_base = cm
  modified_base 4: mod_base = OTHER; note = 2'-O-methyl-adenosine
  modified_base 5: mod_base = cm
  modified_base 6: mod_base = OTHER; note = 2'-Fluoro-cytidine
  modified_base 7: mod_base = gm
  modified_base 8: mod_base = OTHER; note = 2'-O-methyl-adenosine
  modified_base 9: mod_base = gm
  modified_base 10: mod_base = gm
  modified_base 11: mod_base = cm
  modified_base 12: mod_base = cm
  modified_base 13: mod_base = um
  modified_base 14: mod_base = OTHER; note = 2'-Fluoro-cytidine
  modified_base 15: mod_base = gm
  modified_base 16: mod_base = OTHER; note = 2'-Fluoro-guanosine
  modified_base 17: mod_base = OTHER; note = 2'-O-methyl-adenosine
  modified_base 18: mod_base = OTHER; note = 2'-Fluoro-adenosine
  modified_base 19: mod_base = um
  modified_base 20: mod_base = um
  modified_base 21: mod_base = cm
  misc_feature 21^22: note = Phosphorothioate bond
  modified_base 22: mod_base = cm
  misc_feature 22^23: note = Phosphorothioate bond
  modified_base 23: mod_base = cm
gtcaccgaggcctcggaattccc

SEQ ID NO: 978 - RNA, 23 nt, synthetic construct
  source 1..23: mol_type = other RNA
  modified_base 1: mod_base = OTHER; note = 2'-O-methyl-adenosine
  misc_feature 1^2: note = Phosphorothioate bond
  modified_base 2: mod_base = OTHER; note = 2'-Fluoro-cytidine
  misc_feature 2^3: note = Phosphorothioate bond
  modified_base 3: mod_base = cm
  modified_base 4: mod_base = gm
  modified_base 5: mod_base = OTHER; note = 2'-O-methyl-adenosine
  modified_base 6: mod_base = OTHER; note = 2'-Fluoro-guanosine
  modified_base 7: mod_base = gm
  modified_base 8: mod_base = cm
  modified_base 9: mod_base = cm
  modified_base 10: mod_base = um
  modified_base 11: mod_base = cm
  modified_base 12: mod_base = gm
  modified_base 13: mod_base = gm
  modified_base 14: mod_base = OTHER; note = 2'-Fluoro-adenosine
  modified_base 15: mod_base = OTHER; note = 2'-O-methyl-adenosine
  modified_base 16: mod_base = OTHER; note = 2'-Fluoro-uridine
  modified_base 17: mod_base = um
  modified_base 18: mod_base = OTHER; note = 2'-Fluoro-cytidine
  modified_base 19: mod_base = cm
  modified_base 20: mod_base = cm
  modified_base 21: mod_base = um
  misc_feature 21^22: note = Phosphorothioate bond
  modified_base 22: mod_base = um
  misc_feature 22^23: note = Phosphorothioate bond
  modified_base 23: mod_base = um
accgaggcctcggaattcccttt

SEQ ID NO: 979 - RNA, 23 nt, synthetic construct
  source 1..23: mol_type = other RNA
  modified_base 1: mod_base = um
  misc_feature 1^2: note = Phosphorothioate bond
  modified_base 2: mod_base = OTHER; note = 2'-Fluoro-cytidine
  misc_feature 2^3: note = Phosphorothioate bond
  modified_base 3: mod_base = OTHER; note = 2'-O-methyl-adenosine
  modified_base 4: mod_base = cm
  modified_base 5: mod_base = cm
  modified_base 6: mod_base = OTHER; note = 2'-Fluoro-guanosine
  modified_base 7: mod_base = OTHER; note = 2'-O-methyl-adenosine
  modified_base 8: mod_base = gm
  modified_base 9: mod_base = gm
  modified_base 10: mod_base = cm
  modified_base 11: mod_base = cm
  modified_base 12: mod_base = um
  modified_base 13: mod_base = cm
  modified_base 14: mod_base = OTHER; note = 2'-Fluoro-guanosine
  modified_base 15: mod_base = gm
  modified_base 16: mod_base = OTHER; note = 2'-Fluoro-adenosine
  modified_base 17: mod_base = OTHER; note = 2'-O-methyl-adenosine
  modified_base 18: mod_base = OTHER; note = 2'-Fluoro-uridine
  modified_base 19: mod_base = um
  modified_base 20: mod_base = cm
  modified_base 21: mod_base = cm
  misc_feature 21^22: note = Phosphorothioate bond
  modified_base 22: mod_base = cm
  misc_feature 22^23: note = Phosphorothioate bond
  modified_base 23: mod_base = um
tcaccgaggcctcggaattccct

SEQ ID NO: 980 - RNA, 23 nt, synthetic construct
  source 1..23: mol_type = other RNA
  modified_base 1: mod_base = OTHER; note = 2'-O-methyl-adenosine
  misc_feature 1^2: note = Phosphorothioate bond
  modified_base 2: mod_base = OTHER; note = 2'-Fluoro-uridine
  misc_feature 2^3: note = Phosphorothioate bond
  modified_base 3: mod_base = um
  modified_base 4: mod_base = um
  modified_base 5: mod_base = cm
  modified_base 6: mod_base = OTHER; note = 2'-Fluoro-adenosine
  modified_base 7: mod_base = um
  modified_base 8: mod_base = cm
  modified_base 9: mod_base = OTHER; note = 2'-O-methyl-adenosine
  modified_base 10: mod_base = um
  modified_base 11: mod_base = OTHER; note = 2'-O-methyl-adenosine
  modified_base 12: mod_base = cm
  modified_base 13: mod_base = OTHER; note = 2'-O-methyl-adenosine
  modified_base 14: mod_base = OTHER; note = 2'-Fluoro-adenosine
  modified_base 15: mod_base = gm
  modified_base 16: mod_base = OTHER; note = 2'-Fluoro-adenosine
  modified_base 17: mod_base = cm
  modified_base 18: mod_base = OTHER; note = 2'-Fluoro-adenosine
  modified_base 19: mod_base = OTHER; note = 2'-O-methyl-adenosine
  modified_base 20: mod_base = gm
  modified_base 21: mod_base = cm
  misc_feature 21^22: note = Phosphorothioate bond
  modified_base 22: mod_base = OTHER; note = 2'-O-methyl-adenosine
  misc_feature 22^23: note = Phosphorothioate bond
  modified_base 23: mod_base = cm
atttcatcatacaagacaagcac

SEQ ID NO: 981 - RNA, 23 nt, synthetic construct
  source 1..23: mol_type = other RNA
  modified_base 1: mod_base = um
  misc_feature 1^2: note = Phosphorothioate bond
  modified_base 2: mod_base = OTHER; note = 2'-Fluoro-guanosine
  misc_feature 2^3: note = Phosphorothioate bond
  modified_base 3: mod_base = um
  modified_base 4: mod_base = OTHER; note = 2'-O-methyl-adenosine
  modified_base 5: mod_base = um
  modified_base 6: mod_base = OTHER; note = 2'-Fluoro-uridine
  modified_base 7: mod_base = um
  modified_base 8: mod_base = OTHER; note = 2'-O-methyl-adenosine
  modified_base 9: mod_base = um
  modified_base 10: mod_base = cm
  modified_base 11: mod_base = um
  modified_base 12: mod_base = um
  modified_base 13: mod_base = um
  modified_base 14: mod_base = OTHER; note = 2'-Fluoro-guanosine
  modified_base 15: mod_base = OTHER; note = 2'-O-methyl-adenosine
  modified_base 16: mod_base = OTHER; note = 2'-Fluoro-adenosine
  modified_base 17: mod_base = gm
  modified_base 18: mod_base = OTHER; note = 2'-Fluoro-guanosine
  modified_base 19: mod_base = cm
  modified_base 20: mod_base = gm
  modified_base 21: mod_base = OTHER; note = 2'-O-methyl-adenosine
  misc_feature 21^22: note = Phosphorothioate bond
  modified_base 22: mod_base = OTHER; note = 2'-O-methyl-adenosine
  misc_feature 22^23: note = Phosphorothioate bond
  modified_base 23: mod_base = gm
tgtatttatctttgaaggcgaag

SEQ ID NO: 982 - RNA, 23 nt, synthetic construct
  source 1..23: mol_type = other RNA
  modified_base 1: mod_base = OTHER; note = 2'-O-methyl-adenosine
  misc_feature 1^2: note = Phosphorothioate bond
  modified_base 2: mod_base = OTHER; note = 2'-Fluoro-uridine
  misc_feature 2^3: note = Phosphorothioate bond
  modified_base 3: mod_base = um
  modified_base 4: mod_base = um
  modified_base 5: mod_base = gm
  modified_base 6: mod_base = OTHER; note = 2'-Fluoro-uridine
  modified_base 7: mod_base = OTHER; note = 2'-O-methyl-adenosine
  modified_base 8: mod_base = gm
  modified_base 9: mod_base = OTHER; note = 2'-O-methyl-adenosine
  modified_base 10: mod_base = um
  modified_base 11: mod_base = cm
  modified_base 12: mod_base = um
  modified_base 13: mod_base = um
  modified_base 14: mod_base = OTHER; note = 2'-Fluoro-adenosine
  modified_base 15: mod_base = OTHER; note = 2'-O-methyl-adenosine
  modified_base 16: mod_base = OTHER; note = 2'-Fluoro-cytidine
  modified_base 17: mod_base = cm
  modified_base 18: mod_base = OTHER; note = 2'-Fluoro-adenosine
  modified_base 19: mod_base = gm
  modified_base 20: mod_base = gm
  modified_base 21: mod_base = cm
  misc_feature 21^22: note = Phosphorothioate bond
  modified_base 22: mod_base = OTHER; note = 2'-O-methyl-adenosine
  misc_feature 22^23: note = Phosphorothioate bond
  modified_base 23: mod_base = gm
atttgtagatcttaaccaggcag

SEQ ID NO: 983 - RNA, 23 nt, synthetic construct
  source 1..23: mol_type = other RNA
  modified_base 1: mod_base = um
  misc_feature 1^2: note = Phosphorothioate bond
  modified_base 2: mod_base = OTHER; note = 2'-Fluoro-uridine
  misc_feature 2^3: note = Phosphorothioate bond
  modified_base 3: mod_base = cm
  modified_base 4: mod_base = cm
  modified_base 5: mod_base = cm
  modified_base 6: mod_base = OTHER; note = 2'-Fluoro-uridine
  modified_base 7: mod_base = um
  modified_base 8: mod_base = um
  modified_base 9: mod_base = gm
  modified_base 10: mod_base = cm
  modified_base 11: mod_base = OTHER; note = 2'-O-methyl-adenosine
  modified_base 12: mod_base = gm
  modified_base 13: mod_base = um
  modified_base 14: mod_base = OTHER; note = 2'-Fluoro-guanosine
  modified_base 15: mod_base = um
  modified_base 16: mod_base = OTHER; note = 2'-Fluoro-cytidine
  modified_base 17: mod_base = OTHER; note = 2'-O-methyl-adenosine
  modified_base 18: mod_base = OTHER; note = 2'-Fluoro-uridine
  modified_base 19: mod_base = OTHER; note = 2'-O-methyl-adenosine
  modified_base 20: mod_base = gm
  modified_base 21: mod_base = OTHER; note = 2'-O-methyl-adenosine
  misc_feature 21^22: note = Phosphorothioate bond
  modified_base 22: mod_base = um
  misc_feature 22^23: note = Phosphorothioate bond
  modified_base 23: mod_base = OTHER; note = 2'-O-methyl-adenosine
ttccctttgcagtgtcatagata

SEQ ID NO: 984 - RNA, 23 nt, synthetic construct
  source 1..23: mol_type = other RNA
  modified_base 1: mod_base = OTHER; note = 2'-O-methyl-adenosine
  misc_feature 1^2: note = Phosphorothioate bond
  modified_base 2: mod_base = OTHER; note = 2'-Fluoro-uridine
  misc_feature 2^3: note = Phosphorothioate bond
  modified_base 3: mod_base = cm
  modified_base 4: mod_base = OTHER; note = 2'-O-methyl-adenosine
  modified_base 5: mod_base = um
  modified_base 6: mod_base = OTHER; note = 2'-Fluoro-adenosine
  modified_base 7: mod_base = cm
  modified_base 8: mod_base = OTHER; note = 2'-O-methyl-adenosine
  modified_base 9: mod_base = OTHER; note = 2'-O-methyl-adenosine
  modified_base 10: mod_base = gm
  modified_base 11: mod_base = OTHER; note = 2'-O-methyl-adenosine
  modified_base 12: mod_base = cm
  modified_base 13: mod_base = OTHER; note = 2'-O-methyl-adenosine
  modified_base 14: mod_base = OTHER; note = 2'-Fluoro-adenosine
  modified_base 15: mod_base = gm
  modified_base 16: mod_base = OTHER; note = 2'-Fluoro-cytidine
  modified_base 17: mod_base = OTHER; note = 2'-O-methyl-adenosine
  modified_base 18: mod_base = OTHER; note = 2'-Fluoro-cytidine
  modified_base 19: mod_base = OTHER; note = 2'-O-methyl-adenosine
  modified_base 20: mod_base = OTHER; note = 2'-O-methyl-adenosine
  modified_base 21: mod_base = OTHER; note = 2'-O-methyl-adenosine
  misc_feature 21^22: note = Phosphorothioate bond
  modified_base 22: mod_base = OTHER; note = 2'-O-methyl-adenosine
  misc_feature 22^23: note = Phosphorothioate bond
  modified_base 23: mod_base = gm
atcatacaagacaagcacaaaag

SEQ ID NO: 985 - RNA, 23 nt, synthetic construct
  source 1..23: mol_type = other RNA
  modified_base 1: mod_base = um
  misc_feature 1^2: note = Phosphorothioate bond
  modified_base 2: mod_base = OTHER; note = 2'-Fluoro-adenosine
  misc_feature 2^3: note = Phosphorothioate bond
  modified_base 3: mod_base = gm
  modified_base 4: mod_base = OTHER; note = 2'-O-methyl-adenosine
  modified_base 5: mod_base = um
  modified_base 6: mod_base = OTHER; note = 2'-Fluoro-cytidine
  modified_base 7: mod_base = um
  modified_base 8: mod_base = um
  modified_base 9: mod_base = OTHER; note = 2'-O-methyl-adenosine
  modified_base 10: mod_base = OTHER; note = 2'-O-methyl-adenosine
  modified_base 11: mod_base = cm
  modified_base 12: mod_base = cm
  modified_base 13: mod_base = OTHER; note = 2'-O-methyl-adenosine
  modified_base 14: mod_base = OTHER; note = 2'-Fluoro-guanosine
  modified_base 15: mod_base = gm
  modified_base 16: mod_base = OTHER; note = 2'-Fluoro-cytidine
  modified_base 17: mod_base = OTHER; note = 2'-O-methyl-adenosine
  modified_base 18: mod_base = OTHER; note = 2'-Fluoro-guanosine
  modified_base 19: mod_base = um
  modified_base 20: mod_base = cm
  modified_base 21: mod_base = OTHER; note = 2'-O-methyl-adenosine
  misc_feature 21^22: note = Phosphorothioate bond
  modified_base 22: mod_base = cm
  misc_feature 22^23: note = Phosphorothioate bond
  modified_base 23: mod_base = cm
tagatcttaaccaggcagtcacc

SEQ ID NO: 986 - RNA, 23 nt, synthetic construct
  source 1..23: mol_type = other RNA
  modified_base 1: mod_base = OTHER; note = 2'-O-methyl-adenosine
  misc_feature 1^2: note = Phosphorothioate bond
  modified_base 2: mod_base = OTHER; note = 2'-Fluoro-adenosine
  misc_feature 2^3: note = Phosphorothioate bond
  modified_base 3: mod_base = gm
  modified_base 4: mod_base = cm
  modified_base 5: mod_base = OTHER; note = 2'-O-methyl-adenosine
  modified_base 6: mod_base = OTHER; note = 2'-Fluoro-uridine
  modified_base 7: mod_base = um
  modified_base 8: mod_base = cm
  modified_base 9: mod_base = cm
  modified_base 10: mod_base = cm
  modified_base 11: mod_base = um
  modified_base 12: mod_base = um
  modified_base 13: mod_base = um
  modified_base 14: mod_base = OTHER; note = 2'-Fluoro-guanosine
  modified_base 15: mod_base = cm
  modified_base 16: mod_base = OTHER; note = 2'-Fluoro-adenosine
  modified_base 17: mod_base = gm
  modified_base 18: mod_base = OTHER; note = 2'-Fluoro-uridine
  modified_base 19: mod_base = gm
  modified_base 20: mod_base = um
  modified_base 21: mod_base = cm
  misc_feature 21^22: note = Phosphorothioate bond
  modified_base 22: mod_base = OTHER; note = 2'-O-methyl-adenosine
  misc_feature 22^23: note = Phosphorothioate bond
  modified_base 23: mod_base = um
aagcattccctttgcagtgtcat

SEQ ID NO: 987 - RNA, 23 nt, synthetic construct
  source 1..23: mol_type = other RNA
  modified_base 1: mod_base = um
  misc_feature 1^2: note = Phosphorothioate bond
  modified_base 2: mod_base = OTHER; note = 2'-Fluoro-uridine
  misc_feature 2^3: note = Phosphorothioate bond
  modified_base 3: mod_base = um
  modified_base 4: mod_base = gm
  modified_base 5: mod_base = cm
  modified_base 6: mod_base = OTHER; note = 2'-Fluoro-adenosine
  modified_base 7: mod_base = gm
  modified_base 8: mod_base = um
  modified_base 9: mod_base = gm
  modified_base 10: mod_base = um
  modified_base 11: mod_base = cm
  modified_base 12: mod_base = OTHER; note = 2'-O-methyl-adenosine
  modified_base 13: mod_base = um
  modified_base 14: mod_base = OTHER; note = 2'-Fluoro-adenosine
  modified_base 15: mod_base = gm
  modified_base 16: mod_base = OTHER; note = 2'-Fluoro-adenosine
  modified_base 17: mod_base = um
  modified_base 18: mod_base = OTHER; note = 2'-Fluoro-adenosine
  modified_base 19: mod_base = cm
  modified_base 20: mod_base = cm
  modified_base 21: mod_base = gm
  misc_feature 21^22: note = Phosphorothioate bond
  modified_base 22: mod_base = OTHER; note = 2'-O-methyl-adenosine
  misc_feature 22^23: note = Phosphorothioate bond
  modified_base 23: mod_base = OTHER; note = 2'-O-methyl-adenosine
tttgcagtgtcatagataccgaa

SEQ ID NO: 988 - RNA, 23 nt, synthetic construct
  source 1..23: mol_type = other RNA
  modified_base 1: mod_base = OTHER; note = 2'-O-methyl-adenosine
  misc_feature 1^2: note = Phosphorothioate bond
  modified_base 2: mod_base = OTHER; note = 2'-Fluoro-guanosine
  misc_feature 2^3: note = Phosphorothioate bond
  modified_base 3: mod_base = OTHER; note = 2'-O-methyl-adenosine
  modified_base 4: mod_base = gm
  modified_base 5: mod_base = OTHER; note = 2'-O-methyl-adenosine
  modified_base 6: mod_base = OTHER; note = 2'-Fluoro-adenosine
  modified_base 7: mod_base = OTHER; note = 2'-O-methyl-adenosine
  modified_base 8: mod_base = OTHER; note = 2'-O-methyl-adenosine
  modified_base 9: mod_base = cm
  modified_base 10: mod_base = um
  modified_base 11: mod_base = gm
  modified_base 12: mod_base = gm
  modified_base 13: mod_base = um
  modified_base 14: mod_base = OTHER; note = 2'-Fluoro-cytidine
  modified_base 15: mod_base = OTHER; note = 2'-O-methyl-adenosine
  modified_base 16: mod_base = OTHER; note = 2'-Fluoro-guanosine
  modified_base 17: mod_base = OTHER; note = 2'-O-methyl-adenosine
  modified_base 18: mod_base = OTHER; note = 2'-Fluoro-uridine
  modified_base 19: mod_base = gm
  modified_base 20: mod_base = OTHER; note = 2'-O-methyl-adenosine
  modified_base 21: mod_base = OTHER; note = 2'-O-methyl-adenosine
  misc_feature 21^22: note = Phosphorothioate bond
  modified_base 22: mod_base = um
  misc_feature 22^23: note = Phosphorothioate bond
  modified_base 23: mod_base = OTHER; note = 2'-O-methyl-adenosine
agagaaaactggtcagatgaata

SEQ ID NO: 989 - RNA, 23 nt, synthetic construct
  source 1..23: mol_type = other RNA
  modified_base 1: mod_base = um
  misc_feature 1^2: note = Phosphorothioate bond
  modified_base 2: mod_base = OTHER; note = 2'-Fluoro-guanosine
  misc_feature 2^3: note = Phosphorothioate bond
  modified_base 3: mod_base = cm
  modified_base 4: mod_base = OTHER; note = 2'-O-methyl-adenosine
  modified_base 5: mod_base = gm
  modified_base 6: mod_base = OTHER; note = 2'-Fluoro-uridine
  modified_base 7: mod_base = gm
  modified_base 8: mod_base = um
  modified_base 9: mod_base = cm
  modified_base 10: mod_base = OTHER; note = 2'-O-methyl-adenosine
  modified_base 11: mod_base = um
  modified_base 12: mod_base = OTHER; note = 2'-O-methyl-adenosine
  modified_base 13: mod_base = gm
  modified_base 14: mod_base = OTHER; note = 2'-Fluoro-adenosine
  modified_base 15: mod_base = um
  modified_base 16: mod_base = OTHER; note = 2'-Fluoro-adenosine
  modified_base 17: mod_base = cm
  modified_base 18: mod_base = OTHER; note = 2'-Fluoro-cytidine
  modified_base 19: mod_base = gm
  modified_base 20: mod_base = OTHER; note = 2'-O-methyl-adenosine
  modified_base 21: mod_base = OTHER; note = 2'-O-methyl-adenosine
  misc_feature 21^22: note = Phosphorothioate bond
  modified_base 22: mod_base = gm
  misc_feature 22^23: note = Phosphorothioate bond
  modified_base 23: mod_base = um
tgcagtgtcatagataccgaagt

SEQ ID NO: 990 - RNA, 23 nt, synthetic construct
  source 1..23: mol_type = other RNA
  modified_base 1: mod_base = um
  misc_feature 1^2: note = Phosphorothioate bond
  modified_base 2: mod_base = OTHER; note = 2'-Fluoro-cytidine
  misc_feature 2^3: note = Phosphorothioate bond
  modified_base 3: mod_base = OTHER; note = 2'-O-methyl-adenosine
  modified_base 4: mod_base = gm
  modified_base 5: mod_base = OTHER; note = 2'-O-methyl-adenosine
  modified_base 6: mod_base = OTHER; note = 2'-Fluoro-uridine
  modified_base 7: mod_base = um
  modified_base 8: mod_base = um
  modified_base 9: mod_base = gm
  modified_base 10: mod_base = um
  modified_base 11: mod_base = OTHER; note = 2'-O-methyl-adenosine
  modified_base 12: mod_base = gm
  modified_base 13: mod_base = OTHER; note = 2'-O-methyl-adenosine
  modified_base 14: mod_base = OTHER; note = 2'-Fluoro-uridine
  modified_base 15: mod_base = cm
  modified_base 16: mod_base = OTHER; note = 2'-Fluoro-uridine
  modified_base 17: mod_base = um
  modified_base 18: mod_base = OTHER; note = 2'-Fluoro-adenosine
  modified_base 19: mod_base = OTHER; note = 2'-O-methyl-adenosine
  modified_base 20: mod_base = cm
  modified_base 21: mod_base = cm
  misc_feature 21^22: note = Phosphorothioate bond
  modified_base 22: mod_base = OTHER; note = 2'-O-methyl-adenosine
  misc_feature 22^23: note = Phosphorothioate bond
  modified_base 23: mod_base = gm
tcagatttgtagatcttaaccag

SEQ ID NO: 991 - RNA, 23 nt, synthetic construct
  source 1..23: mol_type = other RNA
  modified_base 1: mod_base = um
  misc_feature 1^2: note = Phosphorothioate bond
  modified_base 2: mod_base = OTHER; note = 2'-Fluoro-cytidine
  misc_feature 2^3: note = Phosphorothioate bond
  modified_base 3: mod_base = cm
  modified_base 4: mod_base = cm
  modified_base 5: mod_base = um
  modified_base 6: mod_base = OTHER; note = 2'-Fluoro-uridine
  modified_base 7: mod_base = um
  modified_base 8: mod_base = gm
  modified_base 9: mod_base = cm
  modified_base 10: mod_base = OTHER; note = 2'-O-methyl-adenosine
  modified_base 11: mod_base = gm
  modified_base 12: mod_base = um
  modified_base 13: mod_base = gm
  modified_base 14: mod_base = OTHER; note = 2'-Fluoro-uridine
  modified_base 15: mod_base = cm
  modified_base 16: mod_base = OTHER; note = 2'-Fluoro-adenosine
  modified_base 17: mod_base = um
  modified_base 18: mod_base = OTHER; note = 2'-Fluoro-adenosine
  modified_base 19: mod_base = gm
  modified_base 20: mod_base = OTHER; note = 2'-O-methyl-adenosine
  modified_base 21: mod_base = um
  misc_feature 21^22: note = Phosphorothioate bond
  modified_base 22: mod_base = OTHER; note = 2'-O-methyl-adenosine
  misc_feature 22^23: note = Phosphorothioate bond
  modified_base 23: mod_base = cm
tccctttgcagtgtcatagatac

SEQ ID NO: 992 - RNA, 23 nt, synthetic construct
  source 1..23: mol_type = other RNA
  modified_base 1: mod_base = gm
  misc_feature 1^2: note = Phosphorothioate bond
  modified_base 2: mod_base = OTHER; note = 2'-Fluoro-adenosine
  misc_feature 2^3: note = Phosphorothioate bond
  modified_base 3: mod_base = OTHER; note = 2'-O-methyl-adenosine
  modified_base 4: mod_base = cm
  modified_base 5: mod_base = OTHER; note = 2'-O-methyl-adenosine
  modified_base 6: mod_base = OTHER; note = 2'-Fluoro-uridine
  modified_base 7: mod_base = um
  modified_base 8: mod_base = gm
  modified_base 9: mod_base = gm
  modified_base 10: mod_base = OTHER; note = 2'-O-methyl-adenosine
  modified_base 11: mod_base = cm
  modified_base 12: mod_base = cm
  modified_base 13: mod_base = OTHER; note = 2'-O-methyl-adenosine
  modified_base 14: mod_base = OTHER; note = 2'-Fluoro-uridine
  modified_base 15: mod_base = gm
  modified_base 16: mod_base = OTHER; note = 2'-Fluoro-cytidine
  modified_base 17: mod_base = OTHER; note = 2'-O-methyl-adenosine
  modified_base 18: mod_base = OTHER; note = 2'-Fluoro-cytidine
  modified_base 19: mod_base = cm
  modified_base 20: mod_base = cm
  modified_base 21: mod_base = um
  misc_feature 21^22: note = Phosphorothioate bond
  modified_base 22: mod_base = um
  misc_feature 22^23: note = Phosphorothioate bond
  modified_base 23: mod_base = gm
gaacattggaccatgcacccttg

SEQ ID NO: 993 - RNA, 23 nt, synthetic construct
  source 1..23: mol_type = other RNA
  modified_base 1: mod_base = OTHER; note = 2'-O-methyl-adenosine
  misc_feature 1^2: note = Phosphorothioate bond
  modified_base 2: mod_base = OTHER; note = 2'-Fluoro-adenosine
  misc_feature 2^3: note = Phosphorothioate bond
  modified_base 3: mod_base = um
  modified_base 4: mod_base = cm
  modified_base 5: mod_base = cm
  modified_base 6: mod_base = OTHER; note = 2'-Fluoro-cytidine
  modified_base 7: mod_base = OTHER; note = 2'-O-methyl-adenosine
  modified_base 8: mod_base = um
  modified_base 9: mod_base = cm
  modified_base 10: mod_base = OTHER; note = 2'-O-methyl-adenosine
  modified_base 11: mod_base = gm
  modified_base 12: mod_base = OTHER; note = 2'-O-methyl-adenosine
  modified_base 13: mod_base = um
  modified_base 14: mod_base = OTHER; note = 2'-Fluoro-uridine
  modified_base 15: mod_base = um
  modified_base 16: mod_base = OTHER; note = 2'-Fluoro-guanosine
  modified_base 17: mod_base = um
  modified_base 18: mod_base = OTHER; note = 2'-Fluoro-adenosine
  modified_base 19: mod_base = gm
  modified_base 20: mod_base = OTHER; note = 2'-O-methyl-adenosine
  modified_base 21: mod_base = um
  misc_feature 21^22: note = Phosphorothioate bond
  modified_base 22: mod_base = cm
  misc_feature 22^23: note = Phosphorothioate bond
  modified_base 23: mod_base = um
aatcccatcagatttgtagatct

SEQ ID NO: 994 - RNA, 23 nt, synthetic construct
  source 1..23: mol_type = other RNA
  modified_base 1: mod_base = gm
  misc_feature 1^2: note = Phosphorothioate bond
  modified_base 2: mod_base = OTHER; note = 2'-Fluoro-cytidine
  misc_feature 2^3: note = Phosphorothioate bond
  modified_base 3: mod_base = OTHER; note = 2'-O-methyl-adenosine
  modified_base 4: mod_base = gm
  modified_base 5: mod_base = um
  modified_base 6: mod_base = OTHER; note = 2'-Fluoro-guanosine
  modified_base 7: mod_base = um
  modified_base 8: mod_base = cm
  modified_base 9: mod_base = OTHER; note = 2'-O-methyl-adenosine
  modified_base 10: mod_base = um
  modified_base 11: mod_base = OTHER; note = 2'-O-methyl-adenosine
  modified_base 12: mod_base = gm
  modified_base 13: mod_base = OTHER; note = 2'-O-methyl-adenosine
  modified_base 14: mod_base = OTHER; note = 2'-Fluoro-uridine
  modified_base 15: mod_base = OTHER; note = 2'-O-methyl-adenosine
  modified_base 16: mod_base = OTHER; note = 2'-Fluoro-cytidine
  modified_base 17: mod_base = cm
  modified_base 18: mod_base = OTHER; note = 2'-Fluoro-guanosine
  modified_base 19: mod_base = OTHER; note = 2'-O-methyl-adenosine
  modified_base 20: mod_base = OTHER; note = 2'-O-methyl-adenosine
  modified_base 21: mod_base = gm
  misc_feature 21^22: note = Phosphorothioate bond
  modified_base 22: mod_base = um
  misc_feature 22^23: note = Phosphorothioate bond
  modified_base 23: mod_base = OTHER; note = 2'-O-methyl-adenosine
gcagtgtcatagataccgaagta

SEQ ID NO: 995 - RNA, 23 nt, synthetic construct
  source 1..23: mol_type = other RNA
  modified_base 1: mod_base = cm
  misc_feature 1^2: note = Phosphorothioate bond
  modified_base 2: mod_base = OTHER; note = 2'-Fluoro-adenosine
  misc_feature 2^3: note = Phosphorothioate bond
  modified_base 3: mod_base = OTHER; note = 2'-O-methyl-adenosine
  modified_base 4: mod_base = gm
  modified_base 5: mod_base = cm
  modified_base 6: mod_base = OTHER; note = 2'-Fluoro-adenosine
  modified_base 7: mod_base = cm
  modified_base 8: mod_base = OTHER; note = 2'-O-methyl-adenosine
  modified_base 9: mod_base = OTHER; note = 2'-O-methyl-adenosine
  modified_base 10: mod_base = OTHER; note = 2'-O-methyl-adenosine
  modified_base 11: mod_base = OTHER; note = 2'-O-methyl-adenosine
  modified_base 12: mod_base = gm
  modified_base 13: mod_base = cm
  modified_base 14: mod_base = OTHER; note = 2'-Fluoro-adenosine
  modified_base 15: mod_base = cm
  modified_base 16: mod_base = OTHER; note = 2'-Fluoro-cytidine
  modified_base 17: mod_base = OTHER; note = 2'-O-methyl-adenosine
  modified_base 18: mod_base = OTHER; note = 2'-Fluoro-cytidine
  modified_base 19: mod_base = cm
  modified_base 20: mod_base = cm
  modified_base 21: mod_base = OTHER; note = 2'-O-methyl-adenosine
  misc_feature 21^22: note = Phosphorothioate bond
  modified_base 22: mod_base = um
  misc_feature 22^23: note = Phosphorothioate bond
  modified_base 23: mod_base = gm
caagcacaaaagcaccacccatg

SEQ ID NO: 996 - RNA, 23 nt, synthetic construct
  source 1..23: mol_type = other RNA
  modified_base 1: mod_base = gm
  misc_feature 1^2: note = Phosphorothioate bond
  modified_base 2: mod_base = OTHER; note = 2'-Fluoro-cytidine
  misc_feature 2^3: note = Phosphorothioate bond
  modified_base 3: mod_base = gm
  modified_base 4: mod_base = gm
  modified_base 5: mod_base = cm
  modified_base 6: mod_base = OTHER; note = 2'-Fluoro-uridine
  modified_base 7: mod_base = cm
  modified_base 8: mod_base = gm
  modified_base 9: mod_base = gm
  modified_base 10: mod_base = um
  modified_base 11: mod_base = OTHER; note = 2'-O-methyl-adenosine
  modified_base 12: mod_base = gm
  modified_base 13: mod_base = OTHER; note = 2'-O-methyl-adenosine
  modified_base 14: mod_base = OTHER; note = 2'-Fluoro-uridine
  modified_base 15: mod_base = gm
  modified_base 16: mod_base = OTHER; note = 2'-Fluoro-adenosine
  modified_base 17: mod_base = um
  modified_base 18: mod_base = OTHER; note = 2'-Fluoro-adenosine
  modified_base 19: mod_base = OTHER; note = 2'-O-methyl-adenosine
  modified_base 20: mod_base = um
  modified_base 21: mod_base = OTHER; note = 2'-O-methyl-adenosine
  misc_feature 21^22: note = Phosphorothioate bond
  modified_base 22: mod_base = cm
  misc_feature 22^23: note = Phosphorothioate bond
  modified_base 23: mod_base = cm
gcggctcggtagatgataatacc

SEQ ID NO: 997 - RNA, 23 nt, synthetic construct
  source 1..23: mol_type = other RNA
  modified_base 1: mod_base = cm
  misc_feature 1^2: note = Phosphorothioate bond
  modified_base 2: mod_base = OTHER; note = 2'-Fluoro-uridine
  misc_feature 2^3: note = Phosphorothioate bond
  modified_base 3: mod_base = cm
  modified_base 4: mod_base = cm
  modified_base 5: mod_base = um
  modified_base 6: mod_base = OTHER; note = 2'-Fluoro-uridine
  modified_base 7: mod_base = gm
  modified_base 8: mod_base = gm
  modified_base 9: mod_base = gm
  modified_base 10: mod_base = OTHER; note = 2'-O-methyl-adenosine
  modified_base 11: mod_base = OTHER; note = 2'-O-methyl-adenosine
  modified_base 12: mod_base = um
  modified_base 13: mod_base = OTHER; note = 2'-O-methyl-adenosine
  modified_base 14: mod_base = OTHER; note = 2'-Fluoro-cytidine
  modified_base 15: mod_base = gm
  modified_base 16: mod_base = OTHER; note = 2'-Fluoro-guanosine
  modified_base 17: mod_base = OTHER; note = 2'-O-methyl-adenosine
  modified_base 18: mod_base = OTHER; note = 2'-Fluoro-cytidine
  modified_base 19: mod_base = cm
  modified_base 20: mod_base = OTHER; note = 2'-O-methyl-adenosine
  modified_base 21: mod_base = cm
  misc_feature 21^22: note = Phosphorothioate bond
  modified_base 22: mod_base = gm
  misc_feature 22^23: note = Phosphorothioate bond
  modified_base 23: mod_base = cm
ctccttgggaatacggaccacgc

SEQ ID NO: 998 - RNA, 23 nt, synthetic construct
  source 1..23: mol_type = other RNA
  modified_base 1: mod_base = OTHER; note = 2'-O-methyl-adenosine
  misc_feature 1^2: note = Phosphorothioate bond
  modified_base 2: mod_base = OTHER; note = 2'-Fluoro-uridine
  misc_feature 2^3: note = Phosphorothioate bond
  modified_base 3: mod_base = um
  modified_base 4: mod_base = cm
  modified_base 5: mod_base = cm
  modified_base 6: mod_base = OTHER; note = 2'-Fluoro-cytidine
  modified_base 7: mod_base = um
  modified_base 8: mod_base = um
  modified_base 9: mod_base = um
  modified_base 10: mod_base = gm
  modified_base 11: mod_base = cm
  modified_base 12: mod_base = OTHER; note = 2'-O-methyl-adenosine
  modified_base 13: mod_base = gm
  modified_base 14: mod_base = OTHER; note = 2'-Fluoro-uridine
  modified_base 15: mod_base = gm
  modified_base 16: mod_base = OTHER; note = 2'-Fluoro-uridine
  modified_base 17: mod_base = cm
  modified_base 18: mod_base = OTHER; note = 2'-Fluoro-adenosine
  modified_base 19: mod_base = um
  modified_base 20: mod_base = OTHER; note = 2'-O-methyl-adenosine
  modified_base 21: mod_base = gm
  misc_feature 21^22: note = Phosphorothioate bond
  modified_base 22: mod_base = OTHER; note = 2'-O-methyl-adenosine
  misc_feature 22^23: note = Phosphorothioate bond
  modified_base 23: mod_base = um
attccctttgcagtgtcatagat

SEQ ID NO: 999 - RNA, 23 nt, synthetic construct
  source 1..23: mol_type = other RNA
  modified_base 1: mod_base = cm
  misc_feature 1^2: note = Phosphorothioate bond
  modified_base 2: mod_base = OTHER; note = 2'-Fluoro-adenosine
  misc_feature 2^3: note = Phosphorothioate bond
  modified_base 3: mod_base = um
  modified_base 4: mod_base = OTHER; note = 2'-O-methyl-adenosine
  modified_base 5: mod_base = cm
  modified_base 6: mod_base = OTHER; note = 2'-Fluoro-adenosine
  modified_base 7: mod_base = OTHER; note = 2'-O-methyl-adenosine
  modified_base 8: mod_base = gm
  modified_base 9: mod_base = OTHER; note = 2'-O-methyl-adenosine
  modified_base 10: mod_base = cm
  modified_base 11: mod_base = OTHER; note = 2'-O-methyl-adenosine
  modified_base 12: mod_base = OTHER; note = 2'-O-methyl-adenosine
  modified_base 13: mod_base = gm
  modified_base 14: mod_base = OTHER; note = 2'-Fluoro-cytidine
  modified_base 15: mod_base = OTHER; note = 2'-O-methyl-adenosine
  modified_base 16: mod_base = OTHER; note = 2'-Fluoro-cytidine
  modified_base 17: mod_base = OTHER; note = 2'-O-methyl-adenosine
  modified_base 18: mod_base = OTHER; note = 2'-Fluoro-adenosine
  modified_base 19: mod_base = OTHER; note = 2'-O-methyl-adenosine
  modified_base 20: mod_base = OTHER; note = 2'-O-methyl-adenosine
  modified_base 21: mod_base = gm
  misc_feature 21^22: note = Phosphorothioate bond
  modified_base 22: mod_base = cm
  misc_feature 22^23: note = Phosphorothioate bond
  modified_base 23: mod_base = OTHER; note = 2'-O-methyl-adenosine
catacaagacaagcacaaaagca

SEQ ID NO: 1000 - RNA, 23 nt, synthetic construct
  source 1..23: mol_type = other RNA
  modified_base 1: mod_base = OTHER; note = 2'-O-methyl-adenosine
  misc_feature 1^2: note = Phosphorothioate bond
  modified_base 2: mod_base = OTHER; note = 2'-Fluoro-guanosine
  misc_feature 2^3: note = Phosphorothioate bond
  modified_base 3: mod_base = OTHER; note = 2'-O-methyl-adenosine
  modified_base 4: mod_base = cm
  modified_base 5: mod_base = OTHER; note = 2'-O-methyl-adenosine
  modified_base 6: mod_base = OTHER; note = 2'-Fluoro-cytidine
  modified_base 7: mod_base = gm
  modified_base 8: mod_base = um
  modified_base 9: mod_base = um
  modified_base 10: mod_base = OTHER; note = 2'-O-methyl-adenosine
  modified_base 11: mod_base = OTHER; note = 2'-O-methyl-adenosine
  modified_base 12: mod_base = OTHER; note = 2'-O-methyl-adenosine
  modified_base 13: mod_base = gm
  modified_base 14: mod_base = OTHER; note = 2'-Fluoro-cytidine
  modified_base 15: mod_base = cm
  modified_base 16: mod_base = OTHER; note = 2'-Fluoro-uridine
  modified_base 17: mod_base = um
  modified_base 18: mod_base = OTHER; note = 2'-Fluoro-guanosine
  modified_base 19: mod_base = gm
  modified_base 20: mod_base = um
  modified_base 21: mod_base = OTHER; note = 2'-O-methyl-adenosine
  misc_feature 21^22: note = Phosphorothioate bond
  modified_base 22: mod_base = cm
  misc_feature 22^23: note = Phosphorothioate bond
  modified_base 23: mod_base = OTHER; note = 2'-O-methyl-adenosine
agacacgttaaagccttggtaca

SEQ ID NO: 1001 - RNA, 23 nt, synthetic construct
  source 1..23: mol_type = other RNA
  modified_base 1: mod_base = um
  misc_feature 1^2: note = Phosphorothioate bond
  modified_base 2: mod_base = OTHER; note = 2'-Fluoro-guanosine
  misc_feature 2^3: note = Phosphorothioate bond
  modified_base 3: mod_base = OTHER; note = 2'-O-methyl-adenosine
  modified_base 4: mod_base = gm
  modified_base 5: mod_base = OTHER; note = 2'-O-methyl-adenosine
  modified_base 6: mod_base = OTHER; note = 2'-Fluoro-adenosine
  modified_base 7: mod_base = cm
  modified_base 8: mod_base = OTHER; note = 2'-O-methyl-adenosine
  modified_base 9: mod_base = um
  modified_base 10: mod_base = um
  modified_base 11: mod_base = gm
  modified_base 12: mod_base = gm
  modified_base 13: mod_base = OTHER; note = 2'-O-methyl-adenosine
  modified_base 14: mod_base = OTHER; note = 2'-Fluoro-cytidine
  modified_base 15: mod_base = cm
  modified_base 16: mod_base = OTHER; note = 2'-Fluoro-adenosine
  modified_base 17: mod_base = um
  modified_base 18: mod_base = OTHER; note = 2'-Fluoro-guanosine
  modified_base 19: mod_base = cm
  modified_base 20: mod_base = OTHER; note = 2'-O-methyl-adenosine
  modified_base 21: mod_base = cm
  misc_feature 21^22: note = Phosphorothioate bond
  modified_base 22: mod_base = cm
  misc_feature 22^23: note = Phosphorothioate bond
  modified_base 23: mod_base = cm
tgagaacattggaccatgcaccc

SEQ ID NO: 1002 - RNA, 23 nt, synthetic construct
  source 1..23: mol_type = other RNA
  modified_base 1: mod_base = gm
  misc_feature 1^2: note = Phosphorothioate bond
  modified_base 2: mod_base = OTHER; note = 2'-Fluoro-cytidine
  misc_feature 2^3: note = Phosphorothioate bond
  modified_base 3: mod_base = um
  modified_base 4: mod_base = um
  modified_base 5: mod_base = gm
  modified_base 6: mod_base = OTHER; note = 2'-Fluoro-uridine
  modified_base 7: mod_base = OTHER; note = 2'-O-methyl-adenosine
  modified_base 8: mod_base = um
  modified_base 9: mod_base = um
  modified_base 10: mod_base = um
  modified_base 11: mod_base = OTHER; note = 2'-O-methyl-adenosine
  modified_base 12: mod_base = um
  modified_base 13: mod_base = cm
  modified_base 14: mod_base = OTHER; note = 2'-Fluoro-uridine
  modified_base 15: mod_base = um
  modified_base 16: mod_base = OTHER; note = 2'-Fluoro-uridine
  modified_base 17: mod_base = gm
  modified_base 18: mod_base = OTHER; note = 2'-Fluoro-adenosine
  modified_base 19: mod_base = OTHER; note = 2'-O-methyl-adenosine
  modified_base 20: mod_base = gm
  modified_base 21: mod_base = gm
  misc_feature 21^22: note = Phosphorothioate bond
  modified_base 22: mod_base = cm
  misc_feature 22^23: note = Phosphorothioate bond
  modified_base 23: mod_base = gm
gcttgtatttatctttgaaggcg

SEQ ID NO: 1003 - RNA, 23 nt, synthetic construct
  source 1..23: mol_type = other RNA
  modified_base 1: mod_base = gm
  misc_feature 1^2: note = Phosphorothioate bond
  modified_base 2: mod_base = OTHER; note = 2'-Fluoro-cytidine
  misc_feature 2^3: note = Phosphorothioate bond
  modified_base 3: mod_base = um
  modified_base 4: mod_base = cm
  modified_base 5: mod_base = gm
  modified_base 6: mod_base = OTHER; note = 2'-Fluoro-guanosine
  modified_base 7: mod_base = um
  modified_base 8: mod_base = OTHER; note = 2'-O-methyl-adenosine
  modified_base 9: mod_base = gm
  modified_base 10: mod_base = OTHER; note = 2'-O-methyl-adenosine
  modified_base 11: mod_base = um
  modified_base 12: mod_base = gm
  modified_base 13: mod_base = OTHER; note = 2'-O-methyl-adenosine
  modified_base 14: mod_base = OTHER; note = 2'-Fluoro-uridine
  modified_base 15: mod_base = OTHER; note = 2'-O-methyl-adenosine
  modified_base 16: mod_base = OTHER; note = 2'-Fluoro-adenosine
  modified_base 17: mod_base = um
  modified_base 18: mod_base = OTHER; note = 2'-Fluoro-adenosine
  modified_base 19: mod_base = cm
  modified_base 20: mod_base = cm
  modified_base 21: mod_base = cm
  misc_feature 21^22: note = Phosphorothioate bond
  modified_base 22: mod_base = um
  misc_feature 22^23: note = Phosphorothioate bond
  modified_base 23: mod_base = gm
gctcggtagatgataataccctg

SEQ ID NO: 1004 - RNA, 23 nt, synthetic construct
  source 1..23: mol_type = other RNA
  modified_base 1: mod_base = OTHER; note = 2'-O-methyl-adenosine
  misc_feature 1^2: note = Phosphorothioate bond
  modified_base 2: mod_base = OTHER; note = 2'-Fluoro-guanosine
  misc_feature 2^3: note = Phosphorothioate bond
  modified_base 3: mod_base = um
  modified_base 4: mod_base = gm
  modified_base 5: mod_base = um
  modified_base 6: mod_base = OTHER; note = 2'-Fluoro-cytidine
  modified_base 7: mod_base = OTHER; note = 2'-O-methyl-adenosine
  modified_base 8: mod_base = um
  modified_base 9: mod_base = OTHER; note = 2'-O-methyl-adenosine
  modified_base 10: mod_base = gm
  modified_base 11: mod_base = OTHER; note = 2'-O-methyl-adenosine
  modified_base 12: mod_base = um
  modified_base 13: mod_base = OTHER; note = 2'-O-methyl-adenosine
  modified_base 14: mod_base = OTHER; note = 2'-Fluoro-cytidine
  modified_base 15: mod_base = cm
  modified_base 16: mod_base = OTHER; note = 2'-Fluoro-guanosine
  modified_base 17: mod_base = OTHER; note = 2'-O-methyl-adenosine
  modified_base 18: mod_base = OTHER; note = 2'-Fluoro-adenosine
  modified_base 19: mod_base = gm
  modified_base 20: mod_base = um
  modified_base 21: mod_base = OTHER; note = 2'-O-methyl-adenosine
  misc_feature 21^22: note = Phosphorothioate bond
  modified_base 22: mod_base = gm
  misc_feature 22^23: note = Phosphorothioate bond
  modified_base 23: mod_base = gm
agtgtcatagataccgaagtagg

SEQ ID NO: 1005 - RNA, 23 nt, synthetic construct
  source 1..23: mol_type = other RNA
  modified_base 1: mod_base = OTHER; note = 2'-O-methyl-adenosine
  misc_feature 1^2: note = Phosphorothioate bond
  modified_base 2: mod_base = OTHER; note = 2'-Fluoro-uridine
  misc_feature 2^3: note = Phosphorothioate bond
  modified_base 3: mod_base = cm
  modified_base 4: mod_base = OTHER; note = 2'-O-methyl-adenosine
  modified_base 5: mod_base = gm
  modified_base 6: mod_base = OTHER; note = 2'-Fluoro-adenosine
  modified_base 7: mod_base = um
  modified_base 8: mod_base = um
  modified_base 9: mod_base = um
  modified_base 10: mod_base = gm
  modified_base 11: mod_base = um
  modified_base 12: mod_base = OTHER; note = 2'-O-methyl-adenosine
  modified_base 13: mod_base = gm
  modified_base 14: mod_base = OTHER; note = 2'-Fluoro-adenosine
  modified_base 15: mod_base = um
  modified_base 16: mod_base = OTHER; note = 2'-Fluoro-cytidine
  modified_base 17: mod_base = um
  modified_base 18: mod_base = OTHER; note = 2'-Fluoro-uridine
  modified_base 19: mod_base = OTHER; note = 2'-O-methyl-adenosine
  modified_base 20: mod_base = OTHER; note = 2'-O-methyl-adenosine
  modified_base 21: mod_base = cm
  misc_feature 21^22: note = Phosphorothioate bond
  modified_base 22: mod_base = cm
  misc_feature 22^23: note = Phosphorothioate bond
  modified_base 23: mod_base = OTHER; note = 2'-O-methyl-adenosine
atcagatttgtagatcttaacca

SEQ ID NO: 1006 - RNA, 23 nt, synthetic construct
  source 1..23: mol_type = other RNA
  modified_base 1: mod_base = gm
  misc_feature 1^2: note = Phosphorothioate bond
  modified_base 2: mod_base = OTHER; note = 2'-Fluoro-guanosine
  misc_feature 2^3: note = Phosphorothioate bond
  modified_base 3: mod_base = um
  modified_base 4: mod_base = OTHER; note = 2'-O-methyl-adenosine
  modified_base 5: mod_base = gm
  modified_base 6: mod_base = OTHER; note = 2'-Fluoro-adenosine
  modified_base 7: mod_base = um
  modified_base 8: mod_base = gm
  modified_base 9: mod_base = OTHER; note = 2'-O-methyl-adenosine
  modified_base 10: mod_base = um
  modified_base 11: mod_base = OTHER; note = 2'-O-methyl-adenosine
  modified_base 12: mod_base = OTHER; note = 2'-O-methyl-adenosine
  modified_base 13: mod_base = um
  modified_base 14: mod_base = OTHER; note = 2'-Fluoro-adenosine
  modified_base 15: mod_base = cm
  modified_base 16: mod_base = OTHER; note = 2'-Fluoro-cytidine
  modified_base 17: mod_base = cm
  modified_base 18: mod_base = OTHER; note = 2'-Fluoro-uridine
  modified_base 19: mod_base = gm
  modified_base 20: mod_base = cm
  modified_base 21: mod_base = OTHER; note = 2'-O-methyl-adenosine
  misc_feature 21^22: note = Phosphorothioate bond
  modified_base 22: mod_base = cm
  misc_feature 22^23: note = Phosphorothioate bond
  modified_base 23: mod_base = OTHER; note = 2'-O-methyl-adenosine
ggtagatgataataccctgcaca

SEQ ID NO: 1007 - RNA, 23 nt, synthetic construct
  source 1..23: mol_type = other RNA
  modified_base 1: mod_base = cm
  misc_feature 1^2: note = Phosphorothioate bond
  modified_base 2: mod_base = OTHER; note = 2'-Fluoro-adenosine
  misc_feature 2^3: note = Phosphorothioate bond
  modified_base 3: mod_base = gm
  modified_base 4: mod_base = gm
  modified_base 5: mod_base = cm
  modified_base 6: mod_base = OTHER; note = 2'-Fluoro-cytidine
  modified_base 7: mod_base = cm
  modified_base 8: mod_base = um
  modified_base 9: mod_base = um
  modified_base 10: mod_base = OTHER; note = 2'-O-methyl-adenosine
  modified_base 11: mod_base = OTHER; note = 2'-O-methyl-adenosine
  modified_base 12: mod_base = um
  modified_base 13: mod_base = cm
  modified_base 14: mod_base = OTHER; note = 2'-Fluoro-cytidine
  modified_base 15: mod_base = cm
  modified_base 16: mod_base = OTHER; note = 2'-Fluoro-adenosine
  modified_base 17: mod_base = um
  modified_base 18: mod_base = OTHER; note = 2'-Fluoro-cytidine
  modified_base 19: mod_base = OTHER; note = 2'-O-methyl-adenosine
  modified_base 20: mod_base = gm
  modified_base 21: mod_base = OTHER; note = 2'-O-methyl-adenosine
  misc_feature 21^22: note = Phosphorothioate bond
  modified_base 22: mod_base = um
  misc_feature 22^23: note = Phosphorothioate bond
  modified_base 23: mod_base = um
caggcccttaatcccatcagatt

SEQ ID NO: 1008 - RNA, 23 nt, synthetic construct
  source 1..23: mol_type = other RNA
  modified_base 1: mod_base = OTHER; note = 2'-O-methyl-adenosine
  misc_feature 1^2: note = Phosphorothioate bond
  modified_base 2: mod_base = OTHER; note = 2'-Fluoro-guanosine
  misc_feature 2^3: note = Phosphorothioate bond
  modified_base 3: mod_base = OTHER; note = 2'-O-methyl-adenosine
  modified_base 4: mod_base = um
  modified_base 5: mod_base = gm
  modified_base 6: mod_base = OTHER; note = 2'-Fluoro-adenosine
  modified_base 7: mod_base = um
  modified_base 8: mod_base = OTHER; note = 2'-O-methyl-adenosine
  modified_base 9: mod_base = OTHER; note = 2'-O-methyl-adenosine
  modified_base 10: mod_base = um
  modified_base 11: mod_base = OTHER; note = 2'-O-methyl-adenosine
  modified_base 12: mod_base = cm
  modified_base 13: mod_base = cm
  modified_base 14: mod_base = OTHER; note = 2'-Fluoro-cytidine
  modified_base 15: mod_base = um
  modified_base 16: mod_base = OTHER; note = 2'-Fluoro-guanosine
  modified_base 17: mod_base = cm
  modified_base 18: mod_base = OTHER; note = 2'-Fluoro-adenosine
  modified_base 19: mod_base = cm
  modified_base 20: mod_base = OTHER; note = 2'-O-methyl-adenosine
  modified_base 21: mod_base = gm
  misc_feature 21^22: note = Phosphorothioate bond
  modified_base 22: mod_base = OTHER; note = 2'-O-methyl-adenosine
  misc_feature 22^23: note = Phosphorothioate bond
  modified_base 23: mod_base = cm
agatgataataccctgcacagac

SEQ ID NO: 1009 - RNA, 23 nt, synthetic construct
  source 1..23: mol_type = other RNA
  modified_base 1: mod_base = um
  misc_feature 1^2: note = Phosphorothioate bond
  modified_base 2: mod_base = OTHER; note = 2'-Fluoro-adenosine
  misc_feature 2^3: note = Phosphorothioate bond
  modified_base 3: mod_base = cm
  modified_base 4: mod_base = OTHER; note = 2'-O-methyl-adenosine
  modified_base 5: mod_base = gm
  modified_base 6: mod_base = OTHER; note = 2'-Fluoro-guanosine
  modified_base 7: mod_base = cm
  modified_base 8: mod_base = cm
  modified_base 9: mod_base = cm
  modified_base 10: mod_base = um
  modified_base 11: mod_base = um
  modified_base 12: mod_base = OTHER; note = 2'-O-methyl-adenosine
  modified_base 13: mod_base = OTHER; note = 2'-O-methyl-adenosine
  modified_base 14: mod_base = OTHER; note = 2'-Fluoro-uridine
  modified_base 15: mod_base = cm
  modified_base 16: mod_base = OTHER; note = 2'-Fluoro-cytidine
  modified_base 17: mod_base = cm
  modified_base 18: mod_base = OTHER; note = 2'-Fluoro-adenosine
  modified_base 19: mod_base = um
  modified_base 20: mod_base = cm
  modified_base 21: mod_base = OTHER; note = 2'-O-methyl-adenosine
  misc_feature 21^22: note = Phosphorothioate bond
  modified_base 22: mod_base = gm
  misc_feature 22^23: note = Phosphorothioate bond
  modified_base 23: mod_base = OTHER; note = 2'-O-methyl-adenosine
tacaggcccttaatcccatcaga

SEQ ID NO: 1010 - RNA, 23 nt, synthetic construct
  source 1..23: mol_type = other RNA
  modified_base 1: mod_base = OTHER; note = 2'-O-methyl-adenosine
  misc_feature 1^2: note = Phosphorothioate bond
  modified_base 2: mod_base = OTHER; note = 2'-Fluoro-cytidine
  misc_feature 2^3: note = Phosphorothioate bond
  modified_base 3: mod_base = OTHER; note = 2'-O-methyl-adenosine
  modified_base 4: mod_base = gm
  modified_base 5: mod_base = OTHER; note = 2'-O-methyl-adenosine
  modified_base 6: mod_base = OTHER; note = 2'-Fluoro-cytidine
  modified_base 7: mod_base = OTHER; note = 2'-O-methyl-adenosine
  modified_base 8: mod_base = cm
  modified_base 9: mod_base = gm
  modified_base 10: mod_base = um
  modified_base 11: mod_base = um
  modified_base 12: mod_base = OTHER; note = 2'-O-methyl-adenosine
  modified_base 13: mod_base = OTHER; note = 2'-O-methyl-adenosine
  modified_base 14: mod_base = OTHER; note = 2'-Fluoro-adenosine
  modified_base 15: mod_base = gm
  modified_base 16: mod_base = OTHER; note = 2'-Fluoro-cytidine
  modified_base 17: mod_base = cm
  modified_base 18: mod_base = OTHER; note = 2'-Fluoro-uridine
  modified_base 19: mod_base = um
  modified_base 20: mod_base = gm
  modified_base 21: mod_base = gm
  misc_feature 21^22: note = Phosphorothioate bond
  modified_base 22: mod_base = um
  misc_feature 22^23: note = Phosphorothioate bond
  modified_base 23: mod_base = OTHER; note = 2'-O-methyl-adenosine
acagacacgttaaagccttggta

SEQ ID NO: 1011 - RNA, 23 nt, synthetic construct
  source 1..23: mol_type = other RNA
  modified_base 1: mod_base = OTHER; note = 2'-O-methyl-adenosine
  misc_feature 1^2: note = Phosphorothioate bond
  modified_base 2: mod_base = OTHER; note = 2'-Fluoro-guanosine
  misc_feature 2^3: note = Phosphorothioate bond
  modified_base 3: mod_base = OTHER; note = 2'-O-methyl-adenosine
  modified_base 4: mod_base = OTHER; note = 2'-O-methyl-adenosine
  modified_base 5: mod_base = OTHER; note = 2'-O-methyl-adenosine
  modified_base 6: mod_base = OTHER; note = 2'-Fluoro-adenosine
  modified_base 7: mod_base = cm
  modified_base 8: mod_base = um
  modified_base 9: mod_base = gm
  modified_base 10: mod_base = gm
  modified_base 11: mod_base = um
  modified_base 12: mod_base = cm
  modified_base 13: mod_base = OTHER; note = 2'-O-methyl-adenosine
  modified_base 14: mod_base = OTHER; note = 2'-Fluoro-guanosine
  modified_base 15: mod_base = OTHER; note = 2'-O-methyl-adenosine
  modified_base 16: mod_base = OTHER; note = 2'-Fluoro-uridine
  modified_base 17: mod_base = gm
  modified_base 18: mod_base = OTHER; note = 2'-Fluoro-adenosine
  modified_base 19: mod_base = OTHER; note = 2'-O-methyl-adenosine
  modified_base 20: mod_base = um
  modified_base 21: mod_base = OTHER; note = 2'-O-methyl-adenosine
  misc_feature 21^22: note = Phosphorothioate bond
  modified_base 22: mod_base = um
  misc_feature 22^23: note = Phosphorothioate bond
  modified_base 23: mod_base = um
agaaaactggtcagatgaatatt

SEQ ID NO: 1012 - RNA, 23 nt, synthetic construct
  source 1..23: mol_type = other RNA
  modified_base 1: mod_base = um
  misc_feature 1^2: note = Phosphorothioate bond
  modified_base 2: mod_base = OTHER; note = 2'-Fluoro-guanosine
  misc_feature 2^3: note = Phosphorothioate bond
  modified_base 3: mod_base = um
  modified_base 4: mod_base = OTHER; note = 2'-O-methyl-adenosine
  modified_base 5: mod_base = gm
  modified_base 6: mod_base = OTHER; note = 2'-Fluoro-adenosine
  modified_base 7: mod_base = um
  modified_base 8: mod_base = cm
  modified_base 9: mod_base = um
  modified_base 10: mod_base = um
  modified_base 11: mod_base = OTHER; note = 2'-O-methyl-adenosine
  modified_base 12: mod_base = OTHER; note = 2'-O-methyl-adenosine
  modified_base 13: mod_base = cm
  modified_base 14: mod_base = OTHER; note = 2'-Fluoro-cytidine
  modified_base 15: mod_base = OTHER; note = 2'-O-methyl-adenosine
  modified_base 16: mod_base = OTHER; note = 2'-Fluoro-guanosine
  modified_base 17: mod_base = gm
  modified_base 18: mod_base = OTHER; note = 2'-Fluoro-cytidine
  modified_base 19: mod_base = OTHER; note = 2'-O-methyl-adenosine
  modified_base 20: mod_base = gm
  modified_base 21: mod_base = um
  misc_feature 21^22: note = Phosphorothioate bond
  modified_base 22: mod_base = cm
  misc_feature 22^23: note = Phosphorothioate bond
  modified_base 23: mod_base = OTHER; note = 2'-O-methyl-adenosine
tgtagatcttaaccaggcagtca

SEQ ID NO: 1013 - RNA, 23 nt, synthetic construct
  source 1..23: mol_type = other RNA
  modified_base 1: mod_base = um
  misc_feature 1^2: note = Phosphorothioate bond
  modified_base 2: mod_base = OTHER; note = 2'-Fluoro-cytidine
  misc_feature 2^3: note = Phosphorothioate bond
  modified_base 3: mod_base = OTHER; note = 2'-O-methyl-adenosine
  modified_base 4: mod_base = OTHER; note = 2'-O-methyl-adenosine
  modified_base 5: mod_base = OTHER; note = 2'-O-methyl-adenosine
  modified_base 6: mod_base = OTHER; note = 2'-Fluoro-uridine
  modified_base 7: mod_base = gm
  modified_base 8: mod_base = gm
  modified_base 9: mod_base = OTHER; note = 2'-O-methyl-adenosine
  modified_base 10: mod_base = um
  modified_base 11: mod_base = OTHER; note = 2'-O-methyl-adenosine
  modified_base 12: mod_base = gm
  modified_base 13: mod_base = gm
  modified_base 14: mod_base = OTHER; note = 2'-Fluoro-adenosine
  modified_base 15: mod_base = OTHER; note = 2'-O-methyl-adenosine
  modified_base 16: mod_base = OTHER; note = 2'-Fluoro-guanosine
  modified_base 17: mod_base = um
  modified_base 18: mod_base = OTHER; note = 2'-Fluoro-cytidine
  modified_base 19: mod_base = OTHER; note = 2'-O-methyl-adenosine
  modified_base 20: mod_base = OTHER; note = 2'-O-methyl-adenosine
  modified_base 21: mod_base = cm
  misc_feature 21^22: note = Phosphorothioate bond
  modified_base 22: mod_base = cm
  misc_feature 22^23: note = Phosphorothioate bond
  modified_base 23: mod_base = cm
tcaaatggataggaagtcaaccc

SEQ ID NO: 1014 - RNA, 23 nt, synthetic construct
  source 1..23: mol_type = other RNA
  modified_base 1: mod_base = cm
  misc_feature 1^2: note = Phosphorothioate bond
  modified_base 2: mod_base = OTHER; note = 2'-Fluoro-adenosine
  misc_feature 2^3: note = Phosphorothioate bond
  modified_base 3: mod_base = um
  modified_base 4: mod_base = um
  modified_base 5: mod_base = cm
  modified_base 6: mod_base = OTHER; note = 2'-Fluoro-cytidine
  modified_base 7: mod_base = cm
  modified_base 8: mod_base = um
  modified_base 9: mod_base = um
  modified_base 10: mod_base = um
  modified_base 11: mod_base = gm
  modified_base 12: mod_base = cm
  modified_base 13: mod_base = OTHER; note = 2'-O-methyl-adenosine
  modified_base 14: mod_base = OTHER; note = 2'-Fluoro-guanosine
  modified_base 15: mod_base = um
  modified_base 16: mod_base = OTHER; note = 2'-Fluoro-guanosine
  modified_base 17: mod_base = um
  modified_base 18: mod_base = OTHER; note = 2'-Fluoro-cytidine
  modified_base 19: mod_base = OTHER; note = 2'-O-methyl-adenosine
  modified_base 20: mod_base = um
  modified_base 21: mod_base = OTHER; note = 2'-O-methyl-adenosine
  misc_feature 21^22: note = Phosphorothioate bond
  modified_base 22: mod_base = gm
  misc_feature 22^23: note = Phosphorothioate bond
  modified_base 23: mod_base = OTHER; note = 2'-O-methyl-adenosine
cattccctttgcagtgtcataga

SEQ ID NO: 1015 - RNA, 23 nt, synthetic construct
  source 1..23: mol_type = other RNA
  modified_base 1: mod_base = cm
  misc_feature 1^2: note = Phosphorothioate bond
  modified_base 2: mod_base = OTHER; note = 2'-Fluoro-adenosine
  misc_feature 2^3: note = Phosphorothioate bond
  modified_base 3: mod_base = um
  modified_base 4: mod_base = cm
  modified_base 5: mod_base = OTHER; note = 2'-O-methyl-adenosine
  modified_base 6: mod_base = OTHER; note = 2'-Fluoro-guanosine
  modified_base 7: mod_base = OTHER; note = 2'-O-methyl-adenosine
  modified_base 8: mod_base = um
  modified_base 9: mod_base = um
  modified_base 10: mod_base = um
  modified_base 11: mod_base = gm
  modified_base 12: mod_base = um
  modified_base 13: mod_base = OTHER; note = 2'-O-methyl-adenosine
  modified_base 14: mod_base = OTHER; note = 2'-Fluoro-guanosine
  modified_base 15: mod_base = OTHER; note = 2'-O-methyl-adenosine
  modified_base 16: mod_base = OTHER; note = 2'-Fluoro-uridine
  modified_base 17: mod_base = cm
  modified_base 18: mod_base = OTHER; note = 2'-Fluoro-uridine
  modified_base 19: mod_base = um
  modified_base 20: mod_base = OTHER; note = 2'-O-methyl-adenosine
  modified_base 21: mod_base = OTHER; note = 2'-O-methyl-adenosine
  misc_feature 21^22: note = Phosphorothioate bond
  modified_base 22: mod_base = cm
  misc_feature 22^23: note = Phosphorothioate bond
  modified_base 23: mod_base = cm
catcagatttgtagatcttaacc

SEQ ID NO: 1016 - RNA, 23 nt, synthetic construct
  source 1..23: mol_type = other RNA
  modified_base 1: mod_base = cm
  misc_feature 1^2: note = Phosphorothioate bond
  modified_base 2: mod_base = OTHER; note = 2'-Fluoro-uridine
  misc_feature 2^3: note = Phosphorothioate bond
  modified_base 3: mod_base = cm
  modified_base 4: mod_base = gm
  modified_base 5: mod_base = gm
  modified_base 6: mod_base = OTHER; note = 2'-Fluoro-uridine
  modified_base 7: mod_base = OTHER; note = 2'-O-methyl-adenosine
  modified_base 8: mod_base = gm
  modified_base 9: mod_base = OTHER; note = 2'-O-methyl-adenosine
  modified_base 10: mod_base = um
  modified_base 11: mod_base = gm
  modified_base 12: mod_base = OTHER; note = 2'-O-methyl-adenosine
  modified_base 13: mod_base = um
  modified_base 14: mod_base = OTHER; note = 2'-Fluoro-adenosine
  modified_base 15: mod_base = OTHER; note = 2'-O-methyl-adenosine
  modified_base 16: mod_base = OTHER; note = 2'-Fluoro-uridine
  modified_base 17: mod_base = OTHER; note = 2'-O-methyl-adenosine
  modified_base 18: mod_base = OTHER; note = 2'-Fluoro-cytidine
  modified_base 19: mod_base = cm
  modified_base 20: mod_base = cm
  modified_base 21: mod_base = um
  misc_feature 21^22: note = Phosphorothioate bond
  modified_base 22: mod_base = gm
  misc_feature 22^23: note = Phosphorothioate bond
  modified_base 23: mod_base = cm
ctcggtagatgataataccctgc

SEQ ID NO: 1017 - RNA, 23 nt, synthetic construct
  source 1..23: mol_type = other RNA
  modified_base 1: mod_base = um
  misc_feature 1^2: note = Phosphorothioate bond
  modified_base 2: mod_base = OTHER; note = 2'-Fluoro-uridine
  misc_feature 2^3: note = Phosphorothioate bond
  modified_base 3: mod_base = um
  modified_base 4: mod_base = gm
  modified_base 5: mod_base = um
  modified_base 6: mod_base = OTHER; note = 2'-Fluoro-adenosine
  modified_base 7: mod_base = gm
  modified_base 8: mod_base = OTHER; note = 2'-O-methyl-adenosine
  modified_base 9: mod_base = um
  modified_base 10: mod_base = cm
  modified_base 11: mod_base = um
  modified_base 12: mod_base = um
  modified_base 13: mod_base = OTHER; note = 2'-O-methyl-adenosine
  modified_base 14: mod_base = OTHER; note = 2'-Fluoro-adenosine
  modified_base 15: mod_base = cm
  modified_base 16: mod_base = OTHER; note = 2'-Fluoro-cytidine
  modified_base 17: mod_base = OTHER; note = 2'-O-methyl-adenosine
  modified_base 18: mod_base = OTHER; note = 2'-Fluoro-guanosine
  modified_base 19: mod_base = gm
  modified_base 20: mod_base = cm
  modified_base 21: mod_base = OTHER; note = 2'-O-methyl-adenosine
  misc_feature 21^22: note = Phosphorothioate bond
  modified_base 22: mod_base = gm
  misc_feature 22^23: note = Phosphorothioate bond
  modified_base 23: mod_base = um
tttgtagatcttaaccaggcagt

SEQ ID NO: 1018 - RNA, 23 nt, synthetic construct
  source 1..23: mol_type = other RNA
  modified_base 1: mod_base = OTHER; note = 2'-O-methyl-adenosine
  misc_feature 1^2: note = Phosphorothioate bond
  modified_base 2: mod_base = OTHER; note = 2'-Fluoro-cytidine
  misc_feature 2^3: note = Phosphorothioate bond
  modified_base 3: mod_base = OTHER; note = 2'-O-methyl-adenosine
  modified_base 4: mod_base = gm
  modified_base 5: mod_base = gm
  modified_base 6: mod_base = OTHER; note = 2'-Fluoro-cytidine
  modified_base 7: mod_base = cm
  modified_base 8: mod_base = cm
  modified_base 9: mod_base = um
  modified_base 10: mod_base = um
  modified_base 11: mod_base = OTHER; note = 2'-O-methyl-adenosine
  modified_base 12: mod_base = OTHER; note = 2'-O-methyl-adenosine
  modified_base 13: mod_base = um
  modified_base 14: mod_base = OTHER; note = 2'-Fluoro-cytidine
  modified_base 15: mod_base = cm
  modified_base 16: mod_base = OTHER; note = 2'-Fluoro-cytidine
  modified_base 17: mod_base = OTHER; note = 2'-O-methyl-adenosine
  modified_base 18: mod_base = OTHER; note = 2'-Fluoro-uridine
  modified_base 19: mod_base = cm
  modified_base 20: mod_base = OTHER; note = 2'-O-methyl-adenosine
  modified_base 21: mod_base = gm
  misc_feature 21^22: note = Phosphorothioate bond
  modified_base 22: mod_base = OTHER; note = 2'-O-methyl-adenosine
  misc_feature 22^23: note = Phosphorothioate bond
  modified_base 23: mod_base = um
acaggcccttaatcccatcagat

SEQ ID NO: 1019 - RNA, 23 nt, synthetic construct
  source 1..23: mol_type = other RNA
  modified_base 1: mod_base = cm
  misc_feature 1^2: note = Phosphorothioate bond
  modified_base 2: mod_base = OTHER; note = 2'-Fluoro-uridine
  misc_feature 2^3: note = Phosphorothioate bond
  modified_base 3: mod_base = um
  modified_base 4: mod_base = um
  modified_base 5: mod_base = gm
  modified_base 6: mod_base = OTHER; note = 2'-Fluoro-cytidine
  modified_base 7: mod_base = OTHER; note = 2'-O-methyl-adenosine
  modified_base 8: mod_base = gm
  modified_base 9: mod_base = um
  modified_base 10: mod_base = gm
  modified_base 11: mod_base = um
  modified_base 12: mod_base = cm
  modified_base 13: mod_base = OTHER; note = 2'-O-methyl-adenosine
  modified_base 14: mod_base = OTHER; note = 2'-Fluoro-uridine
  modified_base 15: mod_base = OTHER; note = 2'-O-methyl-adenosine
  modified_base 16: mod_base = OTHER; note = 2'-Fluoro-guanosine
  modified_base 17: mod_base = OTHER; note = 2'-O-methyl-adenosine
  modified_base 18: mod_base = OTHER; note = 2'-Fluoro-uridine
  modified_base 19: mod_base = OTHER; note = 2'-O-methyl-adenosine
  modified_base 20: mod_base = cm
  modified_base 21: mod_base = cm
  misc_feature 21^22: note = Phosphorothioate bond
  modified_base 22: mod_base = gm
  misc_feature 22^23: note = Phosphorothioate bond
  modified_base 23: mod_base = OTHER; note = 2'-O-methyl-adenosine
ctttgcagtgtcatagataccga

SEQ ID NO: 1020 - RNA, 23 nt, synthetic construct
  source 1..23: mol_type = other RNA
  modified_base 1: mod_base = cm
  misc_feature 1^2: note = Phosphorothioate bond
  modified_base 2: mod_base = OTHER; note = 2'-Fluoro-adenosine
  misc_feature 2^3: note = Phosphorothioate bond
  modified_base 3: mod_base = cm
  modified_base 4: mod_base = OTHER; note = 2'-O-methyl-adenosine
  modified_base 5: mod_base = um
  modified_base 6: mod_base = OTHER; note = 2'-Fluoro-cytidine
  modified_base 7: mod_base = OTHER; note = 2'-O-methyl-adenosine
  modified_base 8: mod_base = gm
  modified_base 9: mod_base = cm
  modified_base 10: mod_base = um
  modified_base 11: mod_base = gm
  modified_base 12: mod_base = cm
  modified_base 13: mod_base = um
  modified_base 14: mod_base = OTHER; note = 2'-Fluoro-adenosine
  modified_base 15: mod_base = gm
  modified_base 16: mod_base = OTHER; note = 2'-Fluoro-adenosine
  modified_base 17: mod_base = cm
  modified_base 18: mod_base = OTHER; note = 2'-Fluoro-guanosine
  modified_base 19: mod_base = gm
  modified_base 20: mod_base = gm
  modified_base 21: mod_base = um
  misc_feature 21^22: note = Phosphorothioate bond
  modified_base 22: mod_base = OTHER; note = 2'-O-methyl-adenosine
  misc_feature 22^23: note = Phosphorothioate bond
  modified_base 23: mod_base = cm
cacatcagctgctagacgggtac

SEQ ID NO: 1021 - RNA, 23 nt, synthetic construct
  source 1..23: mol_type = other RNA
  modified_base 1: mod_base = cm
  misc_feature 1^2: note = Phosphorothioate bond
  modified_base 2: mod_base = OTHER; note = 2'-Fluoro-cytidine
  misc_feature 2^3: note = Phosphorothioate bond
  modified_base 3: mod_base = cm
  modified_base 4: mod_base = um
  modified_base 5: mod_base = um
  modified_base 6: mod_base = OTHER; note = 2'-Fluoro-uridine
  modified_base 7: mod_base = gm
  modified_base 8: mod_base = cm
  modified_base 9: mod_base = OTHER; note = 2'-O-methyl-adenosine
  modified_base 10: mod_base = gm
  modified_base 11: mod_base = um
  modified_base 12: mod_base = gm
  modified_base 13: mod_base = um
  modified_base 14: mod_base = OTHER; note = 2'-Fluoro-cytidine
  modified_base 15: mod_base = OTHER; note = 2'-O-methyl-adenosine
  modified_base 16: mod_base = OTHER; note = 2'-Fluoro-uridine
  modified_base 17: mod_base = OTHER; note = 2'-O-methyl-adenosine
  modified_base 18: mod_base = OTHER; note = 2'-Fluoro-guanosine
  modified_base 19: mod_base = OTHER; note = 2'-O-methyl-adenosine
  modified_base 20: mod_base = um
  modified_base 21: mod_base = OTHER; note = 2'-O-methyl-adenosine
  misc_feature 21^22: note = Phosphorothioate bond
  modified_base 22: mod_base = cm
  misc_feature 22^23: note = Phosphorothioate bond
  modified_base 23: mod_base = cm
ccctttgcagtgtcatagatacc

SEQ ID NO: 1022 - RNA, 23 nt, synthetic construct
  source 1..23: mol_type = other RNA
  modified_base 1: mod_base = cm
  misc_feature 1^2: note = Phosphorothioate bond
  modified_base 2: mod_base = OTHER; note = 2'-Fluoro-uridine
  misc_feature 2^3: note = Phosphorothioate bond
  modified_base 3: mod_base = cm
  modified_base 4: mod_base = cm
  modified_base 5: mod_base = OTHER; note = 2'-O-methyl-adenosine
  modified_base 6: mod_base = OTHER; note = 2'-Fluoro-guanosine
  modified_base 7: mod_base = cm
  modified_base 8: mod_base = um
  modified_base 9: mod_base = um
  modified_base 10: mod_base = um
  modified_base 11: mod_base = OTHER; note = 2'-O-methyl-adenosine
  modified_base 12: mod_base = cm
  modified_base 13: mod_base = cm
  modified_base 14: mod_base = OTHER; note = 2'-Fluoro-cytidine
  modified_base 15: mod_base = OTHER; note = 2'-O-methyl-adenosine
  modified_base 16: mod_base = OTHER; note = 2'-Fluoro-cytidine
  modified_base 17: mod_base = OTHER; note = 2'-O-methyl-adenosine
  modified_base 18: mod_base = OTHER; note = 2'-Fluoro-uridine
  modified_base 19: mod_base = cm
  modified_base 20: mod_base = OTHER; note = 2'-O-methyl-adenosine
  modified_base 21: mod_base = gm
  misc_feature 21^22: note = Phosphorothioate bond
  modified_base 22: mod_base = cm
  misc_feature 22^23: note = Phosphorothioate bond
  modified_base 23: mod_base = um
ctccagctttacccacatcagct

SEQ ID NO: 1023 - RNA, 23 nt, synthetic construct
  source 1..23: mol_type = other RNA
  modified_base 1: mod_base = um
  misc_feature 1^2: note = Phosphorothioate bond
  modified_base 2: mod_base = OTHER; note = 2'-Fluoro-uridine
  misc_feature 2^3: note = Phosphorothioate bond
  modified_base 3: mod_base = OTHER; note = 2'-O-methyl-adenosine
  modified_base 4: mod_base = cm
  modified_base 5: mod_base = cm
  modified_base 6: mod_base = OTHER; note = 2'-Fluoro-cytidine
  modified_base 7: mod_base = OTHER; note = 2'-O-methyl-adenosine
  modified_base 8: mod_base = cm
  modified_base 9: mod_base = OTHER; note = 2'-O-methyl-adenosine
  modified_base 10: mod_base = um
  modified_base 11: mod_base = cm
  modified_base 12: mod_base = OTHER; note = 2'-O-methyl-adenosine
  modified_base 13: mod_base = gm
  modified_base 14: mod_base = OTHER; note = 2'-Fluoro-cytidine
  modified_base 15: mod_base = um
  modified_base 16: mod_base = OTHER; note = 2'-Fluoro-guanosine
  modified_base 17: mod_base = cm
  modified_base 18: mod_base = OTHER; note = 2'-Fluoro-uridine
  modified_base 19: mod_base = OTHER; note = 2'-O-methyl-adenosine
  modified_base 20: mod_base = gm
  modified_base 21: mod_base = OTHER; note = 2'-O-methyl-adenosine
  misc_feature 21^22: note = Phosphorothioate bond
  modified_base 22: mod_base = cm
  misc_feature 22^23: note = Phosphorothioate bond
  modified_base 23: mod_base = gm
ttacccacatcagctgctagacg

SEQ ID NO: 1024 - RNA, 23 nt, synthetic construct
  source 1..23: mol_type = other RNA
  modified_base 1: mod_base = um
  misc_feature 1^2: note = Phosphorothioate bond
  modified_base 2: mod_base = OTHER; note = 2'-Fluoro-uridine
  misc_feature 2^3: note = Phosphorothioate bond
  modified_base 3: mod_base = OTHER; note = 2'-O-methyl-adenosine
  modified_base 4: mod_base = OTHER; note = 2'-O-methyl-adenosine
  modified_base 5: mod_base = OTHER; note = 2'-O-methyl-adenosine
  modified_base 6: mod_base = OTHER; note = 2'-Fluoro-guanosine
  modified_base 7: mod_base = cm
  modified_base 8: mod_base = cm
  modified_base 9: mod_base = um
  modified_base 10: mod_base = um
  modified_base 11: mod_base = gm
  modified_base 12: mod_base = gm
  modified_base 13: mod_base = um
  modified_base 14: mod_base = OTHER; note = 2'-Fluoro-adenosine
  modified_base 15: mod_base = cm
  modified_base 16: mod_base = OTHER; note = 2'-Fluoro-adenosine
  modified_base 17: mod_base = gm
  modified_base 18: mod_base = OTHER; note = 2'-Fluoro-guanosine
  modified_base 19: mod_base = cm
  modified_base 20: mod_base = cm
  modified_base 21: mod_base = cm
  misc_feature 21^22: note = Phosphorothioate bond
  modified_base 22: mod_base = um
  misc_feature 22^23: note = Phosphorothioate bond
  modified_base 23: mod_base = um
ttaaagccttggtacaggccctt

SEQ ID NO: 1025 - RNA, 23 nt, synthetic construct
  source 1..23: mol_type = other RNA
  modified_base 1: mod_base = cm
  misc_feature 1^2: note = Phosphorothioate bond
  modified_base 2: mod_base = OTHER; note = 2'-Fluoro-adenosine
  misc_feature 2^3: note = Phosphorothioate bond
  modified_base 3: mod_base = gm
  modified_base 4: mod_base = cm
  modified_base 5: mod_base = um
  modified_base 6: mod_base = OTHER; note = 2'-Fluoro-guanosine
  modified_base 7: mod_base = cm
  modified_base 8: mod_base = um
  modified_base 9: mod_base = OTHER; note = 2'-O-methyl-adenosine
  modified_base 10: mod_base = gm
  modified_base 11: mod_base = OTHER; note = 2'-O-methyl-adenosine
  modified_base 12: mod_base = cm
  modified_base 13: mod_base = gm
  modified_base 14: mod_base = OTHER; note = 2'-Fluoro-guanosine
  modified_base 15: mod_base = gm
  modified_base 16: mod_base = OTHER; note = 2'-Fluoro-uridine
  modified_base 17: mod_base = OTHER; note = 2'-O-methyl-adenosine
  modified_base 18: mod_base = OTHER; note = 2'-Fluoro-cytidine
  modified_base 19: mod_base = gm
  modified_base 20: mod_base = gm
  modified_base 21: mod_base = gm
  misc_feature 21^22: note = Phosphorothioate bond
  modified_base 22: mod_base = cm
  misc_feature 22^23: note = Phosphorothioate bond
  modified_base 23: mod_base = OTHER; note = 2'-O-methyl-adenosine
cagctgctagacgggtacgggca

SEQ ID NO: 1026 - RNA, 23 nt, synthetic construct
  source 1..23: mol_type = other RNA
  modified_base 1: mod_base = cm
  misc_feature 1^2: note = Phosphorothioate bond
  modified_base 2: mod_base = OTHER; note = 2'-Fluoro-adenosine
  misc_feature 2^3: note = Phosphorothioate bond
  modified_base 3: mod_base = gm
  modified_base 4: mod_base = cm
  modified_base 5: mod_base = um
  modified_base 6: mod_base = OTHER; note = 2'-Fluoro-uridine
  modified_base 7: mod_base = um
  modified_base 8: mod_base = OTHER; note = 2'-O-methyl-adenosine
  modified_base 9: mod_base = cm
  modified_base 10: mod_base = cm
  modified_base 11: mod_base = cm
  modified_base 12: mod_base = OTHER; note = 2'-O-methyl-adenosine
  modified_base 13: mod_base = cm
  modified_base 14: mod_base = OTHER; note = 2'-Fluoro-adenosine
  modified_base 15: mod_base = um
  modified_base 16: mod_base = OTHER; note = 2'-Fluoro-cytidine
  modified_base 17: mod_base = OTHER; note = 2'-O-methyl-adenosine
  modified_base 18: mod_base = OTHER; note = 2'-Fluoro-guanosine
  modified_base 19: mod_base = cm
  modified_base 20: mod_base = um
  modified_base 21: mod_base = gm
  misc_feature 21^22: note = Phosphorothioate bond
  modified_base 22: mod_base = cm
  misc_feature 22^23: note = Phosphorothioate bond
  modified_base 23: mod_base = um
cagctttacccacatcagctgct

SEQ ID NO: 1027 - RNA, 23 nt, synthetic construct
  source 1..23: mol_type = other RNA
  modified_base 1: mod_base = um
  misc_feature 1^2: note = Phosphorothioate bond
  modified_base 2: mod_base = OTHER; note = 2'-Fluoro-cytidine
  misc_feature 2^3: note = Phosphorothioate bond
  modified_base 3: mod_base = OTHER; note = 2'-O-methyl-adenosine
  modified_base 4: mod_base = gm
  modified_base 5: mod_base = cm
  modified_base 6: mod_base = OTHER; note = 2'-Fluoro-uridine
  modified_base 7: mod_base = gm
  modified_base 8: mod_base = cm
  modified_base 9: mod_base = um
  modified_base 10: mod_base = OTHER; note = 2'-O-methyl-adenosine
  modified_base 11: mod_base = gm
  modified_base 12: mod_base = OTHER; note = 2'-O-methyl-adenosine
  modified_base 13: mod_base = cm
  modified_base 14: mod_base = OTHER; note = 2'-Fluoro-guanosine
  modified_base 15: mod_base = gm
  modified_base 16: mod_base = OTHER; note = 2'-Fluoro-guanosine
  modified_base 17: mod_base = um
  modified_base 18: mod_base = OTHER; note = 2'-Fluoro-adenosine
  modified_base 19: mod_base = cm
  modified_base 20: mod_base = gm
  modified_base 21: mod_base = gm
  misc_feature 21^22: note = Phosphorothioate bond
  modified_base 22: mod_base = gm
  misc_feature 22^23: note = Phosphorothioate bond
  modified_base 23: mod_base = cm
tcagctgctagacgggtacgggc

SEQ ID NO: 1028 - RNA, 23 nt, synthetic construct
  source 1..23: mol_type = other RNA
  modified_base 1: mod_base = um
  misc_feature 1^2: note = Phosphorothioate bond
  modified_base 2: mod_base = OTHER; note = 2'-Fluoro-cytidine
  misc_feature 2^3: note = Phosphorothioate bond
  modified_base 3: mod_base = cm
  modified_base 4: mod_base = OTHER; note = 2'-O-methyl-adenosine
  modified_base 5: mod_base = gm
  modified_base 6: mod_base = OTHER; note = 2'-Fluoro-cytidine
  modified_base 7: mod_base = um
  modified_base 8: mod_base = um
  modified_base 9: mod_base = um
  modified_base 10: mod_base = OTHER; note = 2'-O-methyl-adenosine
  modified_base 11: mod_base = cm
  modified_base 12: mod_base = cm
  modified_base 13: mod_base = cm
  modified_base 14: mod_base = OTHER; note = 2'-Fluoro-adenosine
  modified_base 15: mod_base = cm
  modified_base 16: mod_base = OTHER; note = 2'-Fluoro-adenosine
  modified_base 17: mod_base = um
  modified_base 18: mod_base = OTHER; note = 2'-Fluoro-cytidine
  modified_base 19: mod_base = OTHER; note = 2'-O-methyl-adenosine
  modified_base 20: mod_base = gm
  modified_base 21: mod_base = cm
  misc_feature 21^22: note = Phosphorothioate bond
  modified_base 22: mod_base = um
  misc_feature 22^23: note = Phosphorothioate bond
  modified_base 23: mod_base = gm
tccagctttacccacatcagctg

SEQ ID NO: 1029 - RNA, 23 nt, synthetic construct
  source 1..23: mol_type = other RNA
  modified_base 1: mod_base = gm
  misc_feature 1^2: note = Phosphorothioate bond
  modified_base 2: mod_base = OTHER; note = 2'-Fluoro-guanosine
  misc_feature 2^3: note = Phosphorothioate bond
  modified_base 3: mod_base = cm
  modified_base 4: mod_base = um
  modified_base 5: mod_base = cm
  modified_base 6: mod_base = OTHER; note = 2'-Fluoro-guanosine
  modified_base 7: mod_base = gm
  modified_base 8: mod_base = um
  modified_base 9: mod_base = OTHER; note = 2'-O-methyl-adenosine
  modified_base 10: mod_base = gm
  modified_base 11: mod_base = OTHER; note = 2'-O-methyl-adenosine
  modified_base 12: mod_base = um
  modified_base 13: mod_base = gm
  modified_base 14: mod_base = OTHER; note = 2'-Fluoro-adenosine
  modified_base 15: mod_base = um
  modified_base 16: mod_base = OTHER; note = 2'-Fluoro-adenosine
  modified_base 17: mod_base = OTHER; note = 2'-O-methyl-adenosine
  modified_base 18: mod_base = OTHER; note = 2'-Fluoro-uridine
  modified_base 19: mod_base = OTHER; note = 2'-O-methyl-adenosine
  modified_base 20: mod_base = cm
  modified_base 21: mod_base = cm
  misc_feature 21^22: note = Phosphorothioate bond
  modified_base 22: mod_base = cm
  misc_feature 22^23: note = Phosphorothioate bond
  modified_base 23: mod_base = um
ggctcggtagatgataataccct

SEQ ID NO: 1030 - RNA, 23 nt, synthetic construct
  source 1..23: mol_type = other RNA
  modified_base 1: mod_base = OTHER; note = 2'-O-methyl-adenosine
  misc_feature 1^2: note = Phosphorothioate bond
  modified_base 2: mod_base = OTHER; note = 2'-Fluoro-guanosine
  misc_feature 2^3: note = Phosphorothioate bond
  modified_base 3: mod_base = gm
  modified_base 4: mod_base = cm
  modified_base 5: mod_base = gm
  modified_base 6: mod_base = OTHER; note = 2'-Fluoro-guanosine
  modified_base 7: mod_base = cm
  modified_base 8: mod_base = um
  modified_base 9: mod_base = cm
  modified_base 10: mod_base = gm
  modified_base 11: mod_base = gm
  modified_base 12: mod_base = um
  modified_base 13: mod_base = OTHER; note = 2'-O-methyl-adenosine
  modified_base 14: mod_base = OTHER; note = 2'-Fluoro-guanosine
  modified_base 15: mod_base = OTHER; note = 2'-O-methyl-adenosine
  modified_base 16: mod_base = OTHER; note = 2'-Fluoro-uridine
  modified_base 17: mod_base = gm
  modified_base 18: mod_base = OTHER; note = 2'-Fluoro-adenosine
  modified_base 19: mod_base = um
  modified_base 20: mod_base = OTHER; note = 2'-O-methyl-adenosine
  modified_base 21: mod_base = OTHER; note = 2'-O-methyl-adenosine
  misc_feature 21^22: note = Phosphorothioate bond
  modified_base 22: mod_base = um
  misc_feature 22^23: note = Phosphorothioate bond
  modified_base 23: mod_base = OTHER; note = 2'-O-methyl-adenosine
aggcggctcggtagatgataata

SEQ ID NO: 1031 - RNA, 23 nt, synthetic construct
  source 1..23: mol_type = other RNA
  modified_base 1: mod_base = cm
  misc_feature 1^2: note = Phosphorothioate bond
  modified_base 2: mod_base = OTHER; note = 2'-Fluoro-adenosine
  misc_feature 2^3: note = Phosphorothioate bond
  modified_base 3: mod_base = um
  modified_base 4: mod_base = cm
  modified_base 5: mod_base = OTHER; note = 2'-O-methyl-adenosine
  modified_base 6: mod_base = OTHER; note = 2'-Fluoro-guanosine
  modified_base 7: mod_base = cm
  modified_base 8: mod_base = um
  modified_base 9: mod_base = gm
  modified_base 10: mod_base = cm
  modified_base 11: mod_base = um
  modified_base 12: mod_base = OTHER; note = 2'-O-methyl-adenosine
  modified_base 13: mod_base = gm
  modified_base 14: mod_base = OTHER; note = 2'-Fluoro-adenosine
  modified_base 15: mod_base = cm
  modified_base 16: mod_base = OTHER; note = 2'-Fluoro-guanosine
  modified_base 17: mod_base = gm
  modified_base 18: mod_base = OTHER; note = 2'-Fluoro-guanosine
  modified_base 19: mod_base = um
  modified_base 20: mod_base = OTHER; note = 2'-O-methyl-adenosine
  modified_base 21: mod_base = cm
  misc_feature 21^22: note = Phosphorothioate bond
  modified_base 22: mod_base = gm
  misc_feature 22^23: note = Phosphorothioate bond
  modified_base 23: mod_base = gm
catcagctgctagacgggtacgg

SEQ ID NO: 1032 - RNA, 23 nt, synthetic construct
  source 1..23: mol_type = other RNA
  modified_base 1: mod_base = gm
  misc_feature 1^2: note = Phosphorothioate bond
  modified_base 2: mod_base = OTHER; note = 2'-Fluoro-uridine
  misc_feature 2^3: note = Phosphorothioate bond
  modified_base 3: mod_base = OTHER; note = 2'-O-methyl-adenosine
  modified_base 4: mod_base = cm
  modified_base 5: mod_base = OTHER; note = 2'-O-methyl-adenosine
  modified_base 6: mod_base = OTHER; note = 2'-Fluoro-guanosine
  modified_base 7: mod_base = gm
  modified_base 8: mod_base = cm
  modified_base 9: mod_base = cm
  modified_base 10: mod_base = cm
  modified_base 11: mod_base = um
  modified_base 12: mod_base = um
  modified_base 13: mod_base = OTHER; note = 2'-O-methyl-adenosine
  modified_base 14: mod_base = OTHER; note = 2'-Fluoro-adenosine
  modified_base 15: mod_base = um
  modified_base 16: mod_base = OTHER; note = 2'-Fluoro-cytidine
  modified_base 17: mod_base = cm
  modified_base 18: mod_base = OTHER; note = 2'-Fluoro-cytidine
  modified_base 19: mod_base = OTHER; note = 2'-O-methyl-adenosine
  modified_base 20: mod_base = um
  modified_base 21: mod_base = cm
  misc_feature 21^22: note = Phosphorothioate bond
  modified_base 22: mod_base = OTHER; note = 2'-O-methyl-adenosine
  misc_feature 22^23: note = Phosphorothioate bond
  modified_base 23: mod_base = gm
gtacaggcccttaatcccatcag

SEQ ID NO: 1033 - RNA, 23 nt, synthetic construct
  source 1..23: mol_type = other RNA
  modified_base 1: mod_base = OTHER; note = 2'-O-methyl-adenosine
  misc_feature 1^2: note = Phosphorothioate bond
  modified_base 2: mod_base = OTHER; note = 2'-Fluoro-uridine
  misc_feature 2^3: note = Phosphorothioate bond
  modified_base 3: mod_base = gm
  modified_base 4: mod_base = OTHER; note = 2'-O-methyl-adenosine
  modified_base 5: mod_base = um
  modified_base 6: mod_base = OTHER; note = 2'-Fluoro-adenosine
  modified_base 7: mod_base = OTHER; note = 2'-O-methyl-adenosine
  modified_base 8: mod_base = um
  modified_base 9: mod_base = OTHER; note = 2'-O-methyl-adenosine
  modified_base 10: mod_base = cm
  modified_base 11: mod_base = cm
  modified_base 12: mod_base = cm
  modified_base 13: mod_base = um
  modified_base 14: mod_base = OTHER; note = 2'-Fluoro-guanosine
  modified_base 15: mod_base = cm
  modified_base 16: mod_base = OTHER; note = 2'-Fluoro-adenosine
  modified_base 17: mod_base = cm
  modified_base 18: mod_base = OTHER; note = 2'-Fluoro-adenosine
  modified_base 19: mod_base = gm
  modified_base 20: mod_base = OTHER; note = 2'-O-methyl-adenosine
  modified_base 21: mod_base = cm
  misc_feature 21^22: note = Phosphorothioate bond
  modified_base 22: mod_base = OTHER; note = 2'-O-methyl-adenosine
  misc_feature 22^23: note = Phosphorothioate bond
  modified_base 23: mod_base = cm
atgataataccctgcacagacac

SEQ ID NO: 1034 - RNA, 23 nt, synthetic construct
  source 1..23: mol_type = other RNA
  modified_base 1: mod_base = cm
  misc_feature 1^2: note = Phosphorothioate bond
  modified_base 2: mod_base = OTHER; note = 2'-Fluoro-cytidine
  misc_feature 2^3: note = Phosphorothioate bond
  modified_base 3: mod_base = um
  modified_base 4: mod_base = um
  modified_base 5: mod_base = gm
  modified_base 6: mod_base = OTHER; note = 2'-Fluoro-guanosine
  modified_base 7: mod_base = gm
  modified_base 8: mod_base = OTHER; note = 2'-O-methyl-adenosine
  modified_base 9: mod_base = OTHER; note = 2'-O-methyl-adenosine
  modified_base 10: mod_base = um
  modified_base 11: mod_base = OTHER; note = 2'-O-methyl-adenosine
  modified_base 12: mod_base = cm
  modified_base 13: mod_base = gm
  modified_base 14: mod_base = OTHER; note = 2'-Fluoro-guanosine
  modified_base 15: mod_base = OTHER; note = 2'-O-methyl-adenosine
  modified_base 16: mod_base = OTHER; note = 2'-Fluoro-cytidine
  modified_base 17: mod_base = cm
  modified_base 18: mod_base = OTHER; note = 2'-Fluoro-adenosine
  modified_base 19: mod_base = cm
  modified_base 20: mod_base = gm
  modified_base 21: mod_base = cm
  misc_feature 21^22: note = Phosphorothioate bond
  modified_base 22: mod_base = OTHER; note = 2'-O-methyl-adenosine
  misc_feature 22^23: note = Phosphorothioate bond
  modified_base 23: mod_base = gm
ccttgggaatacggaccacgcag

SEQ ID NO: 1035 - RNA, 23 nt, synthetic construct
  source 1..23: mol_type = other RNA
  modified_base 1: mod_base = um
  misc_feature 1^2: note = Phosphorothioate bond
  modified_base 2: mod_base = OTHER; note = 2'-Fluoro-cytidine
  misc_feature 2^3: note = Phosphorothioate bond
  modified_base 3: mod_base = cm
  modified_base 4: mod_base = um
  modified_base 5: mod_base = um
  modified_base 6: mod_base = OTHER; note = 2'-Fluoro-guanosine
  modified_base 7: mod_base = gm
  modified_base 8: mod_base = gm
  modified_base 9: mod_base = OTHER; note = 2'-O-methyl-adenosine
  modified_base 10: mod_base = OTHER; note = 2'-O-methyl-adenosine
  modified_base 11: mod_base = um
  modified_base 12: mod_base = OTHER; note = 2'-O-methyl-adenosine
  modified_base 13: mod_base = cm
  modified_base 14: mod_base = OTHER; note = 2'-Fluoro-guanosine
  modified_base 15: mod_base = gm
  modified_base 16: mod_base = OTHER; note = 2'-Fluoro-adenosine
  modified_base 17: mod_base = cm
  modified_base 18: mod_base = OTHER; note = 2'-Fluoro-cytidine
  modified_base 19: mod_base = OTHER; note = 2'-O-methyl-adenosine
  modified_base 20: mod_base = cm
  modified_base 21: mod_base = gm
  misc_feature 21^22: note = Phosphorothioate bond
  modified_base 22: mod_base = cm
  misc_feature 22^23: note = Phosphorothioate bond
  modified_base 23: mod_base = OTHER; note = 2'-O-methyl-adenosine
tccttgggaatacggaccacgca

SEQ ID NO: 1036 - RNA, 23 nt, synthetic construct
  source 1..23: mol_type = other RNA
  modified_base 1: mod_base = cm
  misc_feature 1^2: note = Phosphorothioate bond
  modified_base 2: mod_base = OTHER; note = 2'-Fluoro-adenosine
  misc_feature 2^3: note = Phosphorothioate bond
  modified_base 3: mod_base = gm
  modified_base 4: mod_base = OTHER; note = 2'-O-methyl-adenosine
  modified_base 5: mod_base = um
  modified_base 6: mod_base = OTHER; note = 2'-Fluoro-uridine
  modified_base 7: mod_base = um
  modified_base 8: mod_base = gm
  modified_base 9: mod_base = um
  modified_base 10: mod_base = OTHER; note = 2'-O-methyl-adenosine
  modified_base 11: mod_base = gm
  modified_base 12: mod_base = OTHER; note = 2'-O-methyl-adenosine
  modified_base 13: mod_base = um
  modified_base 14: mod_base = OTHER; note = 2'-Fluoro-cytidine
  modified_base 15: mod_base = um
  modified_base 16: mod_base = OTHER; note = 2'-Fluoro-uridine
  modified_base 17: mod_base = OTHER; note = 2'-O-methyl-adenosine
  modified_base 18: mod_base = OTHER; note = 2'-Fluoro-adenosine
  modified_base 19: mod_base = cm
  modified_base 20: mod_base = cm
  modified_base 21: mod_base = OTHER; note = 2'-O-methyl-adenosine
  misc_feature 21^22: note = Phosphorothioate bond
  modified_base 22: mod_base = gm
  misc_feature 22^23: note = Phosphorothioate bond
  modified_base 23: mod_base = gm
cagatttgtagatcttaaccagg

SEQ ID NO: 1037 - RNA, 23 nt, synthetic construct
  source 1..23: mol_type = other RNA
  modified_base 1: mod_base = um
  misc_feature 1^2: note = Phosphorothioate bond
  modified_base 2: mod_base = OTHER; note = 2'-Fluoro-guanosine
  misc_feature 2^3: note = Phosphorothioate bond
  modified_base 3: mod_base = um
  modified_base 4: mod_base = OTHER; note = 2'-O-methyl-adenosine
  modified_base 5: mod_base = cm
  modified_base 6: mod_base = OTHER; note = 2'-Fluoro-uridine
  modified_base 7: mod_base = um
  modified_base 8: mod_base = cm
  modified_base 9: mod_base = um
  modified_base 10: mod_base = um
  modified_base 11: mod_base = gm
  modified_base 12: mod_base = OTHER; note = 2'-O-methyl-adenosine
  modified_base 13: mod_base = um
  modified_base 14: mod_base = OTHER; note = 2'-Fluoro-uridine
  modified_base 15: mod_base = um
  modified_base 16: mod_base = OTHER; note = 2'-Fluoro-cytidine
  modified_base 17: mod_base = OTHER; note = 2'-O-methyl-adenosine
  modified_base 18: mod_base = OTHER; note = 2'-Fluoro-uridine
  modified_base 19: mod_base = cm
  modified_base 20: mod_base = OTHER; note = 2'-O-methyl-adenosine
  modified_base 21: mod_base = um
  misc_feature 21^22: note = Phosphorothioate bond
  modified_base 22: mod_base = OTHER; note = 2'-O-methyl-adenosine
  misc_feature 22^23: note = Phosphorothioate bond
  modified_base 23: mod_base = cm
tgtacttcttgatttcatcatac

SEQ ID NO: 1038 - RNA, 23 nt, synthetic construct
  source 1..23: mol_type = other RNA
  modified_base 1: mod_base = OTHER; note = 2'-O-methyl-adenosine
  misc_feature 1^2: note = Phosphorothioate bond
  modified_base 2: mod_base = OTHER; note = 2'-Fluoro-uridine
  misc_feature 2^3: note = Phosphorothioate bond
  modified_base 3: mod_base = cm
  modified_base 4: mod_base = cm
  modified_base 5: mod_base = cm
  modified_base 6: mod_base = OTHER; note = 2'-Fluoro-adenosine
  modified_base 7: mod_base = um
  modified_base 8: mod_base = cm
  modified_base 9: mod_base = OTHER; note = 2'-O-methyl-adenosine
  modified_base 10: mod_base = gm
  modified_base 11: mod_base = OTHER; note = 2'-O-methyl-adenosine
  modified_base 12: mod_base = um
  modified_base 13: mod_base = um
  modified_base 14: mod_base = OTHER; note = 2'-Fluoro-uridine
  modified_base 15: mod_base = gm
  modified_base 16: mod_base = OTHER; note = 2'-Fluoro-uridine
  modified_base 17: mod_base = OTHER; note = 2'-O-methyl-adenosine
  modified_base 18: mod_base = OTHER; note = 2'-Fluoro-guanosine
  modified_base 19: mod_base = OTHER; note = 2'-O-methyl-adenosine
  modified_base 20: mod_base = um
  modified_base 21: mod_base = cm
  misc_feature 21^22: note = Phosphorothioate bond
  modified_base 22: mod_base = um
  misc_feature 22^23: note = Phosphorothioate bond
  modified_base 23: mod_base = um
atcccatcagatttgtagatctt

SEQ ID NO: 1039 - RNA, 23 nt, synthetic construct
  source 1..23: mol_type = other RNA
  modified_base 1: mod_base = gm
  misc_feature 1^2: note = Phosphorothioate bond
  modified_base 2: mod_base = OTHER; note = 2'-Fluoro-uridine
  misc_feature 2^3: note = Phosphorothioate bond
  modified_base 3: mod_base = OTHER; note = 2'-O-methyl-adenosine
  modified_base 4: mod_base = gm
  modified_base 5: mod_base = OTHER; note = 2'-O-methyl-adenosine
  modified_base 6: mod_base = OTHER; note = 2'-Fluoro-uridine
  modified_base 7: mod_base = gm
  modified_base 8: mod_base = OTHER; note = 2'-O-methyl-adenosine
  modified_base 9: mod_base = um
  modified_base 10: mod_base = OTHER; note = 2'-O-methyl-adenosine
  modified_base 11: mod_base = OTHER; note = 2'-O-methyl-adenosine
  modified_base 12: mod_base = um
  modified_base 13: mod_base = OTHER; note = 2'-O-methyl-adenosine
  modified_base 14: mod_base = OTHER; note = 2'-Fluoro-cytidine
  modified_base 15: mod_base = cm
  modified_base 16: mod_base = OTHER; note = 2'-Fluoro-cytidine
  modified_base 17: mod_base = um
  modified_base 18: mod_base = OTHER; note = 2'-Fluoro-guanosine
  modified_base 19: mod_base = cm
  modified_base 20: mod_base = OTHER; note = 2'-O-methyl-adenosine
  modified_base 21: mod_base = cm
  misc_feature 21^22: note = Phosphorothioate bond
  modified_base 22: mod_base = OTHER; note = 2'-O-methyl-adenosine
  misc_feature 22^23: note = Phosphorothioate bond
  modified_base 23: mod_base = gm
gtagatgataataccctgcacag

SEQ ID NO: 1040 - RNA, 23 nt, synthetic construct
  source 1..23: mol_type = other RNA
  modified_base 1: mod_base = gm
  misc_feature 1^2: note = Phosphorothioate bond
  modified_base 2: mod_base = OTHER; note = 2'-Fluoro-adenosine
  misc_feature 2^3: note = Phosphorothioate bond
  modified_base 3: mod_base = cm
  modified_base 4: mod_base = OTHER; note = 2'-O-methyl-adenosine
  modified_base 5: mod_base = cm
  modified_base 6: mod_base = OTHER; note = 2'-Fluoro-guanosine
  modified_base 7: mod_base = um
  modified_base 8: mod_base = um
  modified_base 9: mod_base = OTHER; note = 2'-O-methyl-adenosine
  modified_base 10: mod_base = OTHER; note = 2'-O-methyl-adenosine
  modified_base 11: mod_base = OTHER; note = 2'-O-methyl-adenosine
  modified_base 12: mod_base = gm
  modified_base 13: mod_base = cm
  modified_base 14: mod_base = OTHER; note = 2'-Fluoro-cytidine
  modified_base 15: mod_base = um
  modified_base 16: mod_base = OTHER; note = 2'-Fluoro-uridine
  modified_base 17: mod_base = gm
  modified_base 18: mod_base = OTHER; note = 2'-Fluoro-guanosine
  modified_base 19: mod_base = um
  modified_base 20: mod_base = OTHER; note = 2'-O-methyl-adenosine
  modified_base 21: mod_base = cm
  misc_feature 21^22: note = Phosphorothioate bond
  modified_base 22: mod_base = OTHER; note = 2'-O-methyl-adenosine
  misc_feature 22^23: note = Phosphorothioate bond
  modified_base 23: mod_base = gm
gacacgttaaagccttggtacag

SEQ ID NO: 1041 - RNA, 23 nt, synthetic construct
  source 1..23: mol_type = other RNA
  modified_base 1: mod_base = OTHER; note = 2'-O-methyl-adenosine
  misc_feature 1^2: note = Phosphorothioate bond
  modified_base 2: mod_base = OTHER; note = 2'-Fluoro-guanosine
  misc_feature 2^3: note = Phosphorothioate bond
  modified_base 3: mod_base = cm
  modified_base 4: mod_base = um
  modified_base 5: mod_base = um
  modified_base 6: mod_base = OTHER; note = 2'-Fluoro-uridine
  modified_base 7: mod_base = OTHER; note = 2'-O-methyl-adenosine
  modified_base 8: mod_base = cm
  modified_base 9: mod_base = cm
  modified_base 10: mod_base = cm
  modified_base 11: mod_base = OTHER; note = 2'-O-methyl-adenosine
  modified_base 12: mod_base = cm
  modified_base 13: mod_base = OTHER; note = 2'-O-methyl-adenosine
  modified_base 14: mod_base = OTHER; note = 2'-Fluoro-uridine
  modified_base 15: mod_base = cm
  modified_base 16: mod_base = OTHER; note = 2'-Fluoro-adenosine
  modified_base 17: mod_base = gm
  modified_base 18: mod_base = OTHER; note = 2'-Fluoro-cytidine
  modified_base 19: mod_base = um
  modified_base 20: mod_base = gm
  modified_base 21: mod_base = cm
  misc_feature 21^22: note = Phosphorothioate bond
  modified_base 22: mod_base = um
  misc_feature 22^23: note = Phosphorothioate bond
  modified_base 23: mod_base = OTHER; note = 2'-O-methyl-adenosine
agctttacccacatcagctgcta

SEQ ID NO: 1042 - RNA, 23 nt, synthetic construct
  source 1..23: mol_type = other RNA
  modified_base 1: mod_base = OTHER; note = 2'-O-methyl-adenosine
  misc_feature 1^2: note = Phosphorothioate bond
  modified_base 2: mod_base = OTHER; note = 2'-Fluoro-adenosine
  misc_feature 2^3: note = Phosphorothioate bond
  modified_base 3: mod_base = gm
  modified_base 4: mod_base = cm
  modified_base 5: mod_base = OTHER; note = 2'-O-methyl-adenosine
  modified_base 6: mod_base = OTHER; note = 2'-Fluoro-cytidine
  modified_base 7: mod_base = OTHER; note = 2'-O-methyl-adenosine
  modified_base 8: mod_base = OTHER; note = 2'-O-methyl-adenosine
  modified_base 9: mod_base = OTHER; note = 2'-O-methyl-adenosine
  modified_base 10: mod_base = OTHER; note = 2'-O-methyl-adenosine
  modified_base 11: mod_base = gm
  modified_base 12: mod_base = cm
  modified_base 13: mod_base = OTHER; note = 2'-O-methyl-adenosine
  modified_base 14: mod_base = OTHER; note = 2'-Fluoro-cytidine
  modified_base 15: mod_base = cm
  modified_base 16: mod_base = OTHER; note = 2'-Fluoro-adenosine
  modified_base 17: mod_base = cm
  modified_base 18: mod_base = OTHER; note = 2'-Fluoro-cytidine
  modified_base 19: mod_base = cm
  modified_base 20: mod_base = OTHER; note = 2'-O-methyl-adenosine
  modified_base 21: mod_base = um
  misc_feature 21^22: note = Phosphorothioate bond
  modified_base 22: mod_base = gm
  misc_feature 22^23: note = Phosphorothioate bond
  modified_base 23: mod_base = cm
aagcacaaaagcaccacccatgc

SEQ ID NO: 1043 - RNA, 23 nt, synthetic construct
  source 1..23: mol_type = other RNA
  modified_base 1: mod_base = OTHER; note = 2'-O-methyl-adenosine
  misc_feature 1^2: note = Phosphorothioate bond
  modified_base 2: mod_base = OTHER; note = 2'-Fluoro-uridine
  misc_feature 2^3: note = Phosphorothioate bond
  modified_base 3: mod_base = cm
  modified_base 4: mod_base = um
  modified_base 5: mod_base = um
  modified_base 6: mod_base = OTHER; note = 2'-Fluoro-adenosine
  modified_base 7: mod_base = OTHER; note = 2'-O-methyl-adenosine
  modified_base 8: mod_base = cm
  modified_base 9: mod_base = cm
  modified_base 10: mod_base = OTHER; note = 2'-O-methyl-adenosine
  modified_base 11: mod_base = gm
  modified_base 12: mod_base = gm
  modified_base 13: mod_base = cm
  modified_base 14: mod_base = OTHER; note = 2'-Fluoro-adenosine
  modified_base 15: mod_base = gm
  modified_base 16: mod_base = OTHER; note = 2'-Fluoro-uridine
  modified_base 17: mod_base = cm
  modified_base 18: mod_base = OTHER; note = 2'-Fluoro-adenosine
  modified_base 19: mod_base = cm
  modified_base 20: mod_base = cm
  modified_base 21: mod_base = gm
  misc_feature 21^22: note = Phosphorothioate bond
  modified_base 22: mod_base = OTHER; note = 2'-O-methyl-adenosine
  misc_feature 22^23: note = Phosphorothioate bond
  modified_base 23: mod_base = gm
atcttaaccaggcagtcaccgag

SEQ ID NO: 1044 - RNA, 23 nt, synthetic construct
  source 1..23: mol_type = other RNA
  modified_base 1: mod_base = um
  misc_feature 1^2: note = Phosphorothioate bond
  modified_base 2: mod_base = OTHER; note = 2'-Fluoro-uridine
  misc_feature 2^3: note = Phosphorothioate bond
  modified_base 3: mod_base = um
  modified_base 4: mod_base = OTHER; note = 2'-O-methyl-adenosine
  modified_base 5: mod_base = cm
  modified_base 6: mod_base = OTHER; note = 2'-Fluoro-cytidine
  modified_base 7: mod_base = cm
  modified_base 8: mod_base = OTHER; note = 2'-O-methyl-adenosine
  modified_base 9: mod_base = cm
  modified_base 10: mod_base = OTHER; note = 2'-O-methyl-adenosine
  modified_base 11: mod_base = um
  modified_base 12: mod_base = cm
  modified_base 13: mod_base = OTHER; note = 2'-O-methyl-adenosine
  modified_base 14: mod_base = OTHER; note = 2'-Fluoro-guanosine
  modified_base 15: mod_base = cm
  modified_base 16: mod_base = OTHER; note = 2'-Fluoro-uridine
  modified_base 17: mod_base = gm
  modified_base 18: mod_base = OTHER; note = 2'-Fluoro-cytidine
  modified_base 19: mod_base = um
  modified_base 20: mod_base = OTHER; note = 2'-O-methyl-adenosine
  modified_base 21: mod_base = gm
  misc_feature 21^22: note = Phosphorothioate bond
  modified_base 22: mod_base = OTHER; note = 2'-O-methyl-adenosine
  misc_feature 22^23: note = Phosphorothioate bond
  modified_base 23: mod_base = cm
tttacccacatcagctgctagac

SEQ ID NO: 1045 - RNA, 23 nt, synthetic construct
  source 1..23: mol_type = other RNA
  modified_base 1: mod_base = cm
  misc_feature 1^2: note = Phosphorothioate bond
  modified_base 2: mod_base = OTHER; note = 2'-Fluoro-uridine
  misc_feature 2^3: note = Phosphorothioate bond
  modified_base 3: mod_base = um
  modified_base 4: mod_base = OTHER; note = 2'-O-methyl-adenosine
  modified_base 5: mod_base = OTHER; note = 2'-O-methyl-adenosine
  modified_base 6: mod_base = OTHER; note = 2'-Fluoro-uridine
  modified_base 7: mod_base = cm
  modified_base 8: mod_base = cm
  modified_base 9: mod_base = cm
  modified_base 10: mod_base = OTHER; note = 2'-O-methyl-adenosine
  modified_base 11: mod_base = um
  modified_base 12: mod_base = cm
  modified_base 13: mod_base = OTHER; note = 2'-O-methyl-adenosine
  modified_base 14: mod_base = OTHER; note = 2'-Fluoro-guanosine
  modified_base 15: mod_base = OTHER; note = 2'-O-methyl-adenosine
  modified_base 16: mod_base = OTHER; note = 2'-Fluoro-uridine
  modified_base 17: mod_base = um
  modified_base 18: mod_base = OTHER; note = 2'-Fluoro-uridine
  modified_base 19: mod_base = gm
  modified_base 20: mod_base = um
  modified_base 21: mod_base = OTHER; note = 2'-O-methyl-adenosine
  misc_feature 21^22: note = Phosphorothioate bond
  modified_base 22: mod_base = gm
  misc_feature 22^23: note = Phosphorothioate bond
  modified_base 23: mod_base = OTHER; note = 2'-O-methyl-adenosine
cttaatcccatcagatttgtaga

SEQ ID NO: 1046 - RNA, 23 nt, synthetic construct
  source 1..23: mol_type = other RNA
  modified_base 1: mod_base = cm
  misc_feature 1^2: note = Phosphorothioate bond
  modified_base 2: mod_base = OTHER; note = 2'-Fluoro-adenosine
  misc_feature 2^3: note = Phosphorothioate bond
  modified_base 3: mod_base = gm
  modified_base 4: mod_base = um
  modified_base 5: mod_base = gm
  modified_base 6: mod_base = OTHER; note = 2'-Fluoro-uridine
  modified_base 7: mod_base = cm
  modified_base 8: mod_base = OTHER; note = 2'-O-methyl-adenosine
  modified_base 9: mod_base = um
  modified_base 10: mod_base = OTHER; note = 2'-O-methyl-adenosine
  modified_base 11: mod_base = gm
  modified_base 12: mod_base = OTHER; note = 2'-O-methyl-adenosine
  modified_base 13: mod_base = um
  modified_base 14: mod_base = OTHER; note = 2'-Fluoro-adenosine
  modified_base 15: mod_base = cm
  modified_base 16: mod_base = OTHER; note = 2'-Fluoro-cytidine
  modified_base 17: mod_base = gm
  modified_base 18: mod_base = OTHER; note = 2'-Fluoro-adenosine
  modified_base 19: mod_base = OTHER; note = 2'-O-methyl-adenosine
  modified_base 20: mod_base = gm
  modified_base 21: mod_base = um
  misc_feature 21^22: note = Phosphorothioate bond
  modified_base 22: mod_base = OTHER; note = 2'-O-methyl-adenosine
  misc_feature 22^23: note = Phosphorothioate bond
  modified_base 23: mod_base = gm
cagtgtcatagataccgaagtag

SEQ ID NO: 1047 - RNA, 23 nt, synthetic construct
  source 1..23: mol_type = other RNA
  modified_base 1: mod_base = cm
  misc_feature 1^2: note = Phosphorothioate bond
  modified_base 2: mod_base = OTHER; note = 2'-Fluoro-cytidine
  misc_feature 2^3: note = Phosphorothioate bond
  modified_base 3: mod_base = OTHER; note = 2'-O-methyl-adenosine
  modified_base 4: mod_base = gm
  modified_base 5: mod_base = cm
  modified_base 6: mod_base = OTHER; note = 2'-Fluoro-uridine
  modified_base 7: mod_base = um
  modified_base 8: mod_base = um
  modified_base 9: mod_base = OTHER; note = 2'-O-methyl-adenosine
  modified_base 10: mod_base = cm
  modified_base 11: mod_base = cm
  modified_base 12: mod_base = cm
  modified_base 13: mod_base = OTHER; note = 2'-O-methyl-adenosine
  modified_base 14: mod_base = OTHER; note = 2'-Fluoro-cytidine
  modified_base 15: mod_base = OTHER; note = 2'-O-methyl-adenosine
  modified_base 16: mod_base = OTHER; note = 2'-Fluoro-uridine
  modified_base 17: mod_base = cm
  modified_base 18: mod_base = OTHER; note = 2'-Fluoro-adenosine
  modified_base 19: mod_base = gm
  modified_base 20: mod_base = cm
  modified_base 21: mod_base = um
  misc_feature 21^22: note = Phosphorothioate bond
  modified_base 22: mod_base = gm
  misc_feature 22^23: note = Phosphorothioate bond
  modified_base 23: mod_base = cm
ccagctttacccacatcagctgc

SEQ ID NO: 1048 - RNA, 23 nt, synthetic construct
  source 1..23: mol_type = other RNA
  modified_base 1: mod_base = OTHER; note = 2'-O-methyl-adenosine
  misc_feature 1^2: note = Phosphorothioate bond
  modified_base 2: mod_base = OTHER; note = 2'-Fluoro-uridine
  misc_feature 2^3: note = Phosphorothioate bond
  modified_base 3: mod_base = cm
  modified_base 4: mod_base = OTHER; note = 2'-O-methyl-adenosine
  modified_base 5: mod_base = gm
  modified_base 6: mod_base = OTHER; note = 2'-Fluoro-cytidine
  modified_base 7: mod_base = um
  modified_base 8: mod_base = gm
  modified_base 9: mod_base = cm
  modified_base 10: mod_base = um
  modified_base 11: mod_base = OTHER; note = 2'-O-methyl-adenosine
  modified_base 12: mod_base = gm
  modified_base 13: mod_base = OTHER; note = 2'-O-methyl-adenosine
  modified_base 14: mod_base = OTHER; note = 2'-Fluoro-cytidine
  modified_base 15: mod_base = gm
  modified_base 16: mod_base = OTHER; note = 2'-Fluoro-guanosine
  modified_base 17: mod_base = gm
  modified_base 18: mod_base = OTHER; note = 2'-Fluoro-uridine
  modified_base 19: mod_base = OTHER; note = 2'-O-methyl-adenosine
  modified_base 20: mod_base = cm
  modified_base 21: mod_base = gm
  misc_feature 21^22: note = Phosphorothioate bond
  modified_base 22: mod_base = gm
  misc_feature 22^23: note = Phosphorothioate bond
  modified_base 23: mod_base = gm
atcagctgctagacgggtacggg

SEQ ID NO: 1049 - RNA, 23 nt, synthetic construct
  source 1..23: mol_type = other RNA
  modified_base 1: mod_base = gm
  misc_feature 1^2: note = Phosphorothioate bond
  modified_base 2: mod_base = OTHER; note = 2'-Fluoro-adenosine
  misc_feature 2^3: note = Phosphorothioate bond
  modified_base 3: mod_base = um
  modified_base 4: mod_base = gm
  modified_base 5: mod_base = OTHER; note = 2'-O-methyl-adenosine
  modified_base 6: mod_base = OTHER; note = 2'-Fluoro-uridine
  modified_base 7: mod_base = OTHER; note = 2'-O-methyl-adenosine
  modified_base 8: mod_base = OTHER; note = 2'-O-methyl-adenosine
  modified_base 9: mod_base = um
  modified_base 10: mod_base = OTHER; note = 2'-O-methyl-adenosine
  modified_base 11: mod_base = cm
  modified_base 12: mod_base = cm
  modified_base 13: mod_base = cm
  modified_base 14: mod_base = OTHER; note = 2'-Fluoro-uridine
  modified_base 15: mod_base = gm
  modified_base 16: mod_base = OTHER; note = 2'-Fluoro-cytidine
  modified_base 17: mod_base = OTHER; note = 2'-O-methyl-adenosine
  modified_base 18: mod_base = OTHER; note = 2'-Fluoro-cytidine
  modified_base 19: mod_base = OTHER; note = 2'-O-methyl-adenosine
  modified_base 20: mod_base = gm
  modified_base 21: mod_base = OTHER; note = 2'-O-methyl-adenosine
  misc_feature 21^22: note = Phosphorothioate bond
  modified_base 22: mod_base = cm
  misc_feature 22^23: note = Phosphorothioate bond
  modified_base 23: mod_base = OTHER; note = 2'-O-methyl-adenosine
gatgataataccctgcacagaca

SEQ ID NO: 1050 - RNA, 23 nt, synthetic construct
  source 1..23: mol_type = other RNA
  modified_base 1: mod_base = um
  misc_feature 1^2: note = Phosphorothioate bond
  modified_base 2: mod_base = OTHER; note = 2'-Fluoro-uridine
  misc_feature 2^3: note = Phosphorothioate bond
  modified_base 3: mod_base = um
  modified_base 4: mod_base = cm
  modified_base 5: mod_base = OTHER; note = 2'-O-methyl-adenosine
  modified_base 6: mod_base = OTHER; note = 2'-Fluoro-uridine
  modified_base 7: mod_base = cm
  modified_base 8: mod_base = OTHER; note = 2'-O-methyl-adenosine
  modified_base 9: mod_base = um
  modified_base 10: mod_base = OTHER; note = 2'-O-methyl-adenosine
  modified_base 11: mod_base = cm
  modified_base 12: mod_base = OTHER; note = 2'-O-methyl-adenosine
  modified_base 13: mod_base = OTHER; note = 2'-O-methyl-adenosine
  modified_base 14: mod_base = OTHER; note = 2'-Fluoro-guanosine
  modified_base 15: mod_base = OTHER; note = 2'-O-methyl-adenosine
  modified_base 16: mod_base = OTHER; note = 2'-Fluoro-cytidine
  modified_base 17: mod_base = OTHER; note = 2'-O-methyl-adenosine
  modified_base 18: mod_base = OTHER; note = 2'-Fluoro-adenosine
  modified_base 19: mod_base = gm
  modified_base 20: mod_base = cm
  modified_base 21: mod_base = OTHER; note = 2'-O-methyl-adenosine
  misc_feature 21^22: note = Phosphorothioate bond
  modified_base 22: mod_base = cm
  misc_feature 22^23: note = Phosphorothioate bond
  modified_base 23: mod_base = OTHER; note = 2'-O-methyl-adenosine
tttcatcatacaagacaagcaca

SEQ ID NO: 1051 - RNA, 23 nt, synthetic construct
  source 1..23: mol_type = other RNA
  modified_base 1: mod_base = cm
  misc_feature 1^2: note = Phosphorothioate bond
  modified_base 2: mod_base = OTHER; note = 2'-Fluoro-adenosine
  misc_feature 2^3: note = Phosphorothioate bond
  modified_base 3: mod_base = gm
  modified_base 4: mod_base = OTHER; note = 2'-O-methyl-adenosine
  modified_base 5: mod_base = cm
  modified_base 6: mod_base = OTHER; note = 2'-Fluoro-adenosine
  modified_base 7: mod_base = cm
  modified_base 8: mod_base = gm
  modified_base 9: mod_base = um
  modified_base 10: mod_base = um
  modified_base 11: mod_base = OTHER; note = 2'-O-methyl-adenosine
  modified_base 12: mod_base = OTHER; note = 2'-O-methyl-adenosine
  modified_base 13: mod_base = OTHER; note = 2'-O-methyl-adenosine
  modified_base 14: mod_base = OTHER; note = 2'-Fluoro-guanosine
  modified_base 15: mod_base = cm
  modified_base 16: mod_base = OTHER; note = 2'-Fluoro-cytidine
  modified_base 17: mod_base = um
  modified_base 18: mod_base = OTHER; note = 2'-Fluoro-uridine
  modified_base 19: mod_base = gm
  modified_base 20: mod_base = gm
  modified_base 21: mod_base = um
  misc_feature 21^22: note = Phosphorothioate bond
  modified_base 22: mod_base = OTHER; note = 2'-O-methyl-adenosine
  misc_feature 22^23: note = Phosphorothioate bond
  modified_base 23: mod_base = cm
cagacacgttaaagccttggtac

SEQ ID NO: 1052 - RNA, 23 nt, synthetic construct
  source 1..23: mol_type = other RNA
  modified_base 1: mod_base = OTHER; note = 2'-O-methyl-adenosine
  misc_feature 1^2: note = Phosphorothioate bond
  modified_base 2: mod_base = OTHER; note = 2'-Fluoro-guanosine
  misc_feature 2^3: note = Phosphorothioate bond
  modified_base 3: mod_base = OTHER; note = 2'-O-methyl-adenosine
  modified_base 4: mod_base = OTHER; note = 2'-O-methyl-adenosine
  modified_base 5: mod_base = cm
  modified_base 6: mod_base = OTHER; note = 2'-Fluoro-adenosine
  modified_base 7: mod_base = um
  modified_base 8: mod_base = um
  modified_base 9: mod_base = gm
  modified_base 10: mod_base = gm
  modified_base 11: mod_base = OTHER; note = 2'-O-methyl-adenosine
  modified_base 12: mod_base = cm
  modified_base 13: mod_base = cm
  modified_base 14: mod_base = OTHER; note = 2'-Fluoro-adenosine
  modified_base 15: mod_base = um
  modified_base 16: mod_base = OTHER; note = 2'-Fluoro-guanosine
  modified_base 17: mod_base = cm
  modified_base 18: mod_base = OTHER; note = 2'-Fluoro-adenosine
  modified_base 19: mod_base = cm
  modified_base 20: mod_base = cm
  modified_base 21: mod_base = cm
  misc_feature 21^22: note = Phosphorothioate bond
  modified_base 22: mod_base = um
  misc_feature 22^23: note = Phosphorothioate bond
  modified_base 23: mod_base = um
agaacattggaccatgcaccctt

SEQ ID NO: 1053 - RNA, 23 nt, synthetic construct
  source 1..23: mol_type = other RNA
  modified_base 1: mod_base = gm
  misc_feature 1^2: note = Phosphorothioate bond
  modified_base 2: mod_base = OTHER; note = 2'-Fluoro-uridine
  misc_feature 2^3: note = Phosphorothioate bond
  modified_base 3: mod_base = OTHER; note = 2'-O-methyl-adenosine
  modified_base 4: mod_base = gm
  modified_base 5: mod_base = OTHER; note = 2'-O-methyl-adenosine
  modified_base 6: mod_base = OTHER; note = 2'-Fluoro-uridine
  modified_base 7: mod_base = cm
  modified_base 8: mod_base = um
  modified_base 9: mod_base = um
  modified_base 10: mod_base = OTHER; note = 2'-O-methyl-adenosine
  modified_base 11: mod_base = OTHER; note = 2'-O-methyl-adenosine
  modified_base 12: mod_base = cm
  modified_base 13: mod_base = cm
  modified_base 14: mod_base = OTHER; note = 2'-Fluoro-adenosine
  modified_base 15: mod_base = gm
  modified_base 16: mod_base = OTHER; note = 2'-Fluoro-guanosine
  modified_base 17: mod_base = cm
  modified_base 18: mod_base = OTHER; note = 2'-Fluoro-adenosine
  modified_base 19: mod_base = gm
  modified_base 20: mod_base = um
  modified_base 21: mod_base = cm
  misc_feature 21^22: note = Phosphorothioate bond
  modified_base 22: mod_base = OTHER; note = 2'-O-methyl-adenosine
  misc_feature 22^23: note = Phosphorothioate bond
  modified_base 23: mod_base = cm
gtagatcttaaccaggcagtcac

SEQ ID NO: 1054 - RNA, 23 nt, synthetic construct
  source 1..23: mol_type = other RNA
  modified_base 1: mod_base = OTHER; note = 2'-O-methyl-adenosine
  misc_feature 1^2: note = Phosphorothioate bond
  modified_base 2: mod_base = OTHER; note = 2'-Fluoro-guanosine
  misc_feature 2^3: note = Phosphorothioate bond
  modified_base 3: mod_base = cm
  modified_base 4: mod_base = um
  modified_base 5: mod_base = cm
  modified_base 6: mod_base = OTHER; note = 2'-Fluoro-cytidine
  modified_base 7: mod_base = OTHER; note = 2'-O-methyl-adenosine
  modified_base 8: mod_base = gm
  modified_base 9: mod_base = cm
  modified_base 10: mod_base = um
  modified_base 11: mod_base = um
  modified_base 12: mod_base = um
  modified_base 13: mod_base = OTHER; note = 2'-O-methyl-adenosine
  modified_base 14: mod_base = OTHER; note = 2'-Fluoro-cytidine
  modified_base 15: mod_base = cm
  modified_base 16: mod_base = OTHER; note = 2'-Fluoro-cytidine
  modified_base 17: mod_base = OTHER; note = 2'-O-methyl-adenosine
  modified_base 18: mod_base = OTHER; note = 2'-Fluoro-cytidine
  modified_base 19: mod_base = OTHER; note = 2'-O-methyl-adenosine
  modified_base 20: mod_base = um
  modified_base 21: mod_base = cm
  misc_feature 21^22: note = Phosphorothioate bond
  modified_base 22: mod_base = OTHER; note = 2'-O-methyl-adenosine
  misc_feature 22^23: note = Phosphorothioate bond
  modified_base 23: mod_base = gm
agctccagctttacccacatcag

SEQ ID NO: 1055 - RNA, 23 nt, synthetic construct
  source 1..23: mol_type = other RNA
  modified_base 1: mod_base = gm
  misc_feature 1^2: note = Phosphorothioate bond
  modified_base 2: mod_base = OTHER; note = 2'-Fluoro-cytidine
  misc_feature 2^3: note = Phosphorothioate bond
  modified_base 3: mod_base = um
  modified_base 4: mod_base = cm
  modified_base 5: mod_base = cm
  modified_base 6: mod_base = OTHER; note = 2'-Fluoro-uridine
  modified_base 7: mod_base = um
  modified_base 8: mod_base = gm
  modified_base 9: mod_base = gm
  modified_base 10: mod_base = gm
  modified_base 11: mod_base = OTHER; note = 2'-O-methyl-adenosine
  modified_base 12: mod_base = OTHER; note = 2'-O-methyl-adenosine
  modified_base 13: mod_base = um
  modified_base 14: mod_base = OTHER; note = 2'-Fluoro-adenosine
  modified_base 15: mod_base = cm
  modified_base 16: mod_base = OTHER; note = 2'-Fluoro-guanosine
  modified_base 17: mod_base = gm
  modified_base 18: mod_base = OTHER; note = 2'-Fluoro-adenosine
  modified_base 19: mod_base = cm
  modified_base 20: mod_base = cm
  modified_base 21: mod_base = OTHER; note = 2'-O-methyl-adenosine
  misc_feature 21^22: note = Phosphorothioate bond
  modified_base 22: mod_base = cm
  misc_feature 22^23: note = Phosphorothioate bond
  modified_base 23: mod_base = gm
gctccttgggaatacggaccacg

SEQ ID NO: 1056 - RNA, 23 nt, synthetic construct
  source 1..23: mol_type = other RNA
  modified_base 1: mod_base = gm
  misc_feature 1^2: note = Phosphorothioate bond
  modified_base 2: mod_base = OTHER; note = 2'-Fluoro-adenosine
  misc_feature 2^3: note = Phosphorothioate bond
  modified_base 3: mod_base = OTHER; note = 2'-O-methyl-adenosine
  modified_base 4: mod_base = gm
  modified_base 5: mod_base = cm
  modified_base 6: mod_base = OTHER; note = 2'-Fluoro-adenosine
  modified_base 7: mod_base = um
  modified_base 8: mod_base = um
  modified_base 9: mod_base = cm
  modified_base 10: mod_base = cm
  modified_base 11: mod_base = cm
  modified_base 12: mod_base = um
  modified_base 13: mod_base = um
  modified_base 14: mod_base = OTHER; note = 2'-Fluoro-uridine
  modified_base 15: mod_base = gm
  modified_base 16: mod_base = OTHER; note = 2'-Fluoro-cytidine
  modified_base 17: mod_base = OTHER; note = 2'-O-methyl-adenosine
  modified_base 18: mod_base = OTHER; note = 2'-Fluoro-guanosine
  modified_base 19: mod_base = um
  modified_base 20: mod_base = gm
  modified_base 21: mod_base = um
  misc_feature 21^22: note = Phosphorothioate bond
  modified_base 22: mod_base = cm
  misc_feature 22^23: note = Phosphorothioate bond
  modified_base 23: mod_base = OTHER; note = 2'-O-methyl-adenosine
gaagcattccctttgcagtgtca

SEQ ID NO: 1057 - RNA, 23 nt, synthetic construct
  source 1..23: mol_type = other RNA
  modified_base 1: mod_base = cm
  misc_feature 1^2: note = Phosphorothioate bond
  modified_base 2: mod_base = OTHER; note = 2'-Fluoro-cytidine
  misc_feature 2^3: note = Phosphorothioate bond
  modified_base 3: mod_base = um
  modified_base 4: mod_base = um
  modified_base 5: mod_base = gm
  modified_base 6: mod_base = OTHER; note = 2'-Fluoro-guanosine
  modified_base 7: mod_base = um
  modified_base 8: mod_base = OTHER; note = 2'-O-methyl-adenosine
  modified_base 9: mod_base = cm
  modified_base 10: mod_base = OTHER; note = 2'-O-methyl-adenosine
  modified_base 11: mod_base = gm
  modified_base 12: mod_base = gm
  modified_base 13: mod_base = cm
  modified_base 14: mod_base = OTHER; note = 2'-Fluoro-cytidine
  modified_base 15: mod_base = cm
  modified_base 16: mod_base = OTHER; note = 2'-Fluoro-uridine
  modified_base 17: mod_base = um
  modified_base 18: mod_base = OTHER; note = 2'-Fluoro-adenosine
  modified_base 19: mod_base = OTHER; note = 2'-O-methyl-adenosine
  modified_base 20: mod_base = um
  modified_base 21: mod_base = cm
  misc_feature 21^22: note = Phosphorothioate bond
  modified_base 22: mod_base = cm
  misc_feature 22^23: note = Phosphorothioate bond
  modified_base 23: mod_base = cm
ccttggtacaggcccttaatccc

SEQ ID NO: 1058 - RNA, 23 nt, synthetic construct
  source 1..23: mol_type = other RNA
  modified_base 1: mod_base = um
  misc_feature 1^2: note = Phosphorothioate bond
  modified_base 2: mod_base = OTHER; note = 2'-Fluoro-adenosine
  misc_feature 2^3: note = Phosphorothioate bond
  modified_base 3: mod_base = gm
  modified_base 4: mod_base = OTHER; note = 2'-O-methyl-adenosine
  modified_base 5: mod_base = um
  modified_base 6: mod_base = OTHER; note = 2'-Fluoro-guanosine
  modified_base 7: mod_base = OTHER; note = 2'-O-methyl-adenosine
  modified_base 8: mod_base = um
  modified_base 9: mod_base = OTHER; note = 2'-O-methyl-adenosine
  modified_base 10: mod_base = OTHER; note = 2'-O-methyl-adenosine
  modified_base 11: mod_base = um
  modified_base 12: mod_base = OTHER; note = 2'-O-methyl-adenosine
  modified_base 13: mod_base = cm
  modified_base 14: mod_base = OTHER; note = 2'-Fluoro-cytidine
  modified_base 15: mod_base = cm
  modified_base 16: mod_base = OTHER; note = 2'-Fluoro-uridine
  modified_base 17: mod_base = gm
  modified_base 18: mod_base = OTHER; note = 2'-Fluoro-cytidine
  modified_base 19: mod_base = OTHER; note = 2'-O-methyl-adenosine
  modified_base 20: mod_base = cm
  modified_base 21: mod_base = OTHER; note = 2'-O-methyl-adenosine
  misc_feature 21^22: note = Phosphorothioate bond
  modified_base 22: mod_base = gm
  misc_feature 22^23: note = Phosphorothioate bond
  modified_base 23: mod_base = OTHER; note = 2'-O-methyl-adenosine
tagatgataataccctgcacaga

SEQ ID NO: 1059 - RNA, 23 nt, synthetic construct
  source 1..23: mol_type = other RNA
  modified_base 1: mod_base = OTHER; note = 2'-O-methyl-adenosine
  misc_feature 1^2: note = Phosphorothioate bond
  modified_base 2: mod_base = OTHER; note = 2'-Fluoro-adenosine
  misc_feature 2^3: note = Phosphorothioate bond
  modified_base 3: mod_base = um
  modified_base 4: mod_base = OTHER; note = 2'-O-methyl-adenosine
  modified_base 5: mod_base = cm
  modified_base 6: mod_base = OTHER; note = 2'-Fluoro-cytidine
  modified_base 7: mod_base = cm
  modified_base 8: mod_base = um
  modified_base 9: mod_base = gm
  modified_base 10: mod_base = cm
  modified_base 11: mod_base = OTHER; note = 2'-O-methyl-adenosine
  modified_base 12: mod_base = cm
  modified_base 13: mod_base = OTHER; note = 2'-O-methyl-adenosine
  modified_base 14: mod_base = OTHER; note = 2'-Fluoro-guanosine
  modified_base 15: mod_base = OTHER; note = 2'-O-methyl-adenosine
  modified_base 16: mod_base = OTHER; note = 2'-Fluoro-cytidine
  modified_base 17: mod_base = OTHER; note = 2'-O-methyl-adenosine
  modified_base 18: mod_base = OTHER; note = 2'-Fluoro-cytidine
  modified_base 19: mod_base = gm
  modified_base 20: mod_base = um
  modified_base 21: mod_base = um
  misc_feature 21^22: note = Phosphorothioate bond
  modified_base 22: mod_base = OTHER; note = 2'-O-methyl-adenosine
  misc_feature 22^23: note = Phosphorothioate bond
  modified_base 23: mod_base = OTHER; note = 2'-O-methyl-adenosine
aataccctgcacagacacgttaa

SEQ ID NO: 1060 - RNA, 23 nt, synthetic construct
  source 1..23: mol_type = other RNA
  modified_base 1: mod_base = gm
  misc_feature 1^2: note = Phosphorothioate bond
  modified_base 2: mod_base = OTHER; note = 2'-Fluoro-uridine
  misc_feature 2^3: note = Phosphorothioate bond
  modified_base 3: mod_base = um
  modified_base 4: mod_base = OTHER; note = 2'-O-methyl-adenosine
  modified_base 5: mod_base = OTHER; note = 2'-O-methyl-adenosine
  modified_base 6: mod_base = OTHER; note = 2'-Fluoro-adenosine
  modified_base 7: mod_base = gm
  modified_base 8: mod_base = cm
  modified_base 9: mod_base = cm
  modified_base 10: mod_base = um
  modified_base 11: mod_base = um
  modified_base 12: mod_base = gm
  modified_base 13: mod_base = gm
  modified_base 14: mod_base = OTHER; note = 2'-Fluoro-uridine
  modified_base 15: mod_base = OTHER; note = 2'-O-methyl-adenosine
  modified_base 16: mod_base = OTHER; note = 2'-Fluoro-cytidine
  modified_base 17: mod_base = OTHER; note = 2'-O-methyl-adenosine
  modified_base 18: mod_base = OTHER; note = 2'-Fluoro-guanosine
  modified_base 19: mod_base = gm
  modified_base 20: mod_base = cm
  modified_base 21: mod_base = cm
  misc_feature 21^22: note = Phosphorothioate bond
  modified_base 22: mod_base = cm
  misc_feature 22^23: note = Phosphorothioate bond
  modified_base 23: mod_base = um
gttaaagccttggtacaggccct

SEQ ID NO: 1061 - RNA, 23 nt, synthetic construct
  source 1..23: mol_type = other RNA
  modified_base 1: mod_base = OTHER; note = 2'-O-methyl-adenosine
  misc_feature 1^2: note = Phosphorothioate bond
  modified_base 2: mod_base = OTHER; note = 2'-Fluoro-guanosine
  misc_feature 2^3: note = Phosphorothioate bond
  modified_base 3: mod_base = cm
  modified_base 4: mod_base = OTHER; note = 2'-O-methyl-adenosine
  modified_base 5: mod_base = um
  modified_base 6: mod_base = OTHER; note = 2'-Fluoro-uridine
  modified_base 7: mod_base = cm
  modified_base 8: mod_base = cm
  modified_base 9: mod_base = cm
  modified_base 10: mod_base = um
  modified_base 11: mod_base = um
  modified_base 12: mod_base = um
  modified_base 13: mod_base = gm
  modified_base 14: mod_base = OTHER; note = 2'-Fluoro-cytidine
  modified_base 15: mod_base = OTHER; note = 2'-O-methyl-adenosine
  modified_base 16: mod_base = OTHER; note = 2'-Fluoro-guanosine
  modified_base 17: mod_base = um
  modified_base 18: mod_base = OTHER; note = 2'-Fluoro-guanosine
  modified_base 19: mod_base = um
  modified_base 20: mod_base = cm
  modified_base 21: mod_base = OTHER; note = 2'-O-methyl-adenosine
  misc_feature 21^22: note = Phosphorothioate bond
  modified_base 22: mod_base = um
  misc_feature 22^23: note = Phosphorothioate bond
  modified_base 23: mod_base = OTHER; note = 2'-O-methyl-adenosine
agcattccctttgcagtgtcata

SEQ ID NO: 1062 - RNA, 23 nt, synthetic construct
  source 1..23: mol_type = other RNA
  modified_base 1: mod_base = um
  misc_feature 1^2: note = Phosphorothioate bond
  modified_base 2: mod_base = OTHER; note = 2'-Fluoro-cytidine
  misc_feature 2^3: note = Phosphorothioate bond
  modified_base 3: mod_base = um
  modified_base 4: mod_base = um
  modified_base 5: mod_base = OTHER; note = 2'-O-methyl-adenosine
  modified_base 6: mod_base = OTHER; note = 2'-Fluoro-adenosine
  modified_base 7: mod_base = cm
  modified_base 8: mod_base = cm
  modified_base 9: mod_base = OTHER; note = 2'-O-methyl-adenosine
  modified_base 10: mod_base = gm
  modified_base 11: mod_base = gm
  modified_base 12: mod_base = cm
  modified_base 13: mod_base = OTHER; note = 2'-O-methyl-adenosine
  modified_base 14: mod_base = OTHER; note = 2'-Fluoro-guanosine
  modified_base 15: mod_base = um
  modified_base 16: mod_base = OTHER; note = 2'-Fluoro-cytidine
  modified_base 17: mod_base = OTHER; note = 2'-O-methyl-adenosine
  modified_base 18: mod_base = OTHER; note = 2'-Fluoro-cytidine
  modified_base 19: mod_base = cm
  modified_base 20: mod_base = gm
  modified_base 21: mod_base = OTHER; note = 2'-O-methyl-adenosine
  misc_feature 21^22: note = Phosphorothioate bond
  modified_base 22: mod_base = gm
  misc_feature 22^23: note = Phosphorothioate bond
  modified_base 23: mod_base = gm
tcttaaccaggcagtcaccgagg

SEQ ID NO: 1063 - RNA, 23 nt, synthetic construct
  source 1..23: mol_type = other RNA
  modified_base 1: mod_base = OTHER; note = 2'-O-methyl-adenosine
  misc_feature 1^2: note = Phosphorothioate bond
  modified_base 2: mod_base = OTHER; note = 2'-Fluoro-uridine
  misc_feature 2^3: note = Phosphorothioate bond
  modified_base 3: mod_base = OTHER; note = 2'-O-methyl-adenosine
  modified_base 4: mod_base = cm
  modified_base 5: mod_base = OTHER; note = 2'-O-methyl-adenosine
  modified_base 6: mod_base = OTHER; note = 2'-Fluoro-adenosine
  modified_base 7: mod_base = gm
  modified_base 8: mod_base = OTHER; note = 2'-O-methyl-adenosine
  modified_base 9: mod_base = cm
  modified_base 10: mod_base = OTHER; note = 2'-O-methyl-adenosine
  modified_base 11: mod_base = OTHER; note = 2'-O-methyl-adenosine
  modified_base 12: mod_base = gm
  modified_base 13: mod_base = cm
  modified_base 14: mod_base = OTHER; note = 2'-Fluoro-adenosine
  modified_base 15: mod_base = cm
  modified_base 16: mod_base = OTHER; note = 2'-Fluoro-adenosine
  modified_base 17: mod_base = OTHER; note = 2'-O-methyl-adenosine
  modified_base 18: mod_base = OTHER; note = 2'-Fluoro-adenosine
  modified_base 19: mod_base = OTHER; note = 2'-O-methyl-adenosine
  modified_base 20: mod_base = gm
  modified_base 21: mod_base = cm
  misc_feature 21^22: note = Phosphorothioate bond
  modified_base 22: mod_base = OTHER; note = 2'-O-methyl-adenosine
  misc_feature 22^23: note = Phosphorothioate bond
  modified_base 23: mod_base = cm
atacaagacaagcacaaaagcac

SEQ ID NO: 1064 - RNA, 23 nt, synthetic construct
  source 1..23: mol_type = other RNA
  modified_base 1: mod_base = gm
  misc_feature 1^2: note = Phosphorothioate bond
  modified_base 2: mod_base = OTHER; note = 2'-Fluoro-adenosine
  misc_feature 2^3: note = Phosphorothioate bond
  modified_base 3: mod_base = cm
  modified_base 4: mod_base = OTHER; note = 2'-O-methyl-adenosine
  modified_base 5: mod_base = OTHER; note = 2'-O-methyl-adenosine
  modified_base 6: mod_base = OTHER; note = 2'-Fluoro-guanosine
  modified_base 7: mod_base = cm
  modified_base 8: mod_base = OTHER; note = 2'-O-methyl-adenosine
  modified_base 9: mod_base = cm
  modified_base 10: mod_base = OTHER; note = 2'-O-methyl-adenosine
  modified_base 11: mod_base = OTHER; note = 2'-O-methyl-adenosine
  modified_base 12: mod_base = OTHER; note = 2'-O-methyl-adenosine
  modified_base 13: mod_base = OTHER; note = 2'-O-methyl-adenosine
  modified_base 14: mod_base = OTHER; note = 2'-Fluoro-guanosine
  modified_base 15: mod_base = cm
  modified_base 16: mod_base = OTHER; note = 2'-Fluoro-adenosine
  modified_base 17: mod_base = cm
  modified_base 18: mod_base = OTHER; note = 2'-Fluoro-cytidine
  modified_base 19: mod_base = OTHER; note = 2'-O-methyl-adenosine
  modified_base 20: mod_base = cm
  modified_base 21: mod_base = cm
  misc_feature 21^22: note = Phosphorothioate bond
  modified_base 22: mod_base = cm
  misc_feature 22^23: note = Phosphorothioate bond
  modified_base 23: mod_base = OTHER; note = 2'-O-methyl-adenosine
gacaagcacaaaagcaccaccca

SEQ ID NO: 1065 - RNA, 23 nt, synthetic construct
  source 1..23: mol_type = other RNA
  modified_base 1: mod_base = OTHER; note = 2'-O-methyl-adenosine
  misc_feature 1^2: note = Phosphorothioate bond
  modified_base 2: mod_base = OTHER; note = 2'-Fluoro-cytidine
  misc_feature 2^3: note = Phosphorothioate bond
  modified_base 3: mod_base = cm
  modified_base 4: mod_base = cm
  modified_base 5: mod_base = OTHER; note = 2'-O-methyl-adenosine
  modified_base 6: mod_base = OTHER; note = 2'-Fluoro-cytidine
  modified_base 7: mod_base = OTHER; note = 2'-O-methyl-adenosine
  modified_base 8: mod_base = um
  modified_base 9: mod_base = cm
  modified_base 10: mod_base = OTHER; note = 2'-O-methyl-adenosine
  modified_base 11: mod_base = gm
  modified_base 12: mod_base = cm
  modified_base 13: mod_base = um
  modified_base 14: mod_base = OTHER; note = 2'-Fluoro-guanosine
  modified_base 15: mod_base = cm
  modified_base 16: mod_base = OTHER; note = 2'-Fluoro-uridine
  modified_base 17: mod_base = OTHER; note = 2'-O-methyl-adenosine
  modified_base 18: mod_base = OTHER; note = 2'-Fluoro-guanosine
  modified_base 19: mod_base = OTHER; note = 2'-O-methyl-adenosine
  modified_base 20: mod_base = cm
  modified_base 21: mod_base = gm
  misc_feature 21^22: note = Phosphorothioate bond
  modified_base 22: mod_base = gm
  misc_feature 22^23: note = Phosphorothioate bond
  modified_base 23: mod_base = gm
acccacatcagctgctagacggg

SEQ ID NO: 1066 - RNA, 23 nt, synthetic construct
  source 1..23: mol_type = other RNA
  modified_base 1: mod_base = um
  misc_feature 1^2: note = Phosphorothioate bond
  modified_base 2: mod_base = OTHER; note = 2'-Fluoro-adenosine
  misc_feature 2^3: note = Phosphorothioate bond
  modified_base 3: mod_base = OTHER; note = 2'-O-methyl-adenosine
  modified_base 4: mod_base = OTHER; note = 2'-O-methyl-adenosine
  modified_base 5: mod_base = gm
  modified_base 6: mod_base = OTHER; note = 2'-Fluoro-cytidine
  modified_base 7: mod_base = cm
  modified_base 8: mod_base = um
  modified_base 9: mod_base = um
  modified_base 10: mod_base = gm
  modified_base 11: mod_base = gm
  modified_base 12: mod_base = um
  modified_base 13: mod_base = OTHER; note = 2'-O-methyl-adenosine
  modified_base 14: mod_base = OTHER; note = 2'-Fluoro-cytidine
  modified_base 15: mod_base = OTHER; note = 2'-O-methyl-adenosine
  modified_base 16: mod_base = OTHER; note = 2'-Fluoro-guanosine
  modified_base 17: mod_base = gm
  modified_base 18: mod_base = OTHER; note = 2'-Fluoro-cytidine
  modified_base 19: mod_base = cm
  modified_base 20: mod_base = cm
  modified_base 21: mod_base = um
  misc_feature 21^22: note = Phosphorothioate bond
  modified_base 22: mod_base = um
  misc_feature 22^23: note = Phosphorothioate bond
  modified_base 23: mod_base = OTHER; note = 2'-O-methyl-adenosine
taaagccttggtacaggccctta

SEQ ID NO: 1067 - RNA, 23 nt, synthetic construct
  source 1..23: mol_type = other RNA
  modified_base 1: mod_base = um
  misc_feature 1^2: note = Phosphorothioate bond
  modified_base 2: mod_base = OTHER; note = 2'-Fluoro-uridine
  misc_feature 2^3: note = Phosphorothioate bond
  modified_base 3: mod_base = cm
  modified_base 4: mod_base = OTHER; note = 2'-O-methyl-adenosine
  modified_base 5: mod_base = um
  modified_base 6: mod_base = OTHER; note = 2'-Fluoro-cytidine
  modified_base 7: mod_base = OTHER; note = 2'-O-methyl-adenosine
  modified_base 8: mod_base = um
  modified_base 9: mod_base = OTHER; note = 2'-O-methyl-adenosine
  modified_base 10: mod_base = cm
  modified_base 11: mod_base = OTHER; note = 2'-O-methyl-adenosine
  modified_base 12: mod_base = OTHER; note = 2'-O-methyl-adenosine
  modified_base 13: mod_base = gm
  modified_base 14: mod_base = OTHER; note = 2'-Fluoro-adenosine
  modified_base 15: mod_base = cm
  modified_base 16: mod_base = OTHER; note = 2'-Fluoro-adenosine
  modified_base 17: mod_base = OTHER; note = 2'-O-methyl-adenosine
  modified_base 18: mod_base = OTHER; note = 2'-Fluoro-guanosine
  modified_base 19: mod_base = cm
  modified_base 20: mod_base = OTHER; note = 2'-O-methyl-adenosine
  modified_base 21: mod_base = cm
  misc_feature 21^22: note = Phosphorothioate bond
  modified_base 22: mod_base = OTHER; note = 2'-O-methyl-adenosine
  misc_feature 22^23: note = Phosphorothioate bond
  modified_base 23: mod_base = OTHER; note = 2'-O-methyl-adenosine
ttcatcatacaagacaagcacaa

SEQ ID NO: 1068 - RNA, 23 nt, synthetic construct
  source 1..23: mol_type = other RNA
  modified_base 1: mod_base = gm
  misc_feature 1^2: note = Phosphorothioate bond
  modified_base 2: mod_base = OTHER; note = 2'-Fluoro-cytidine
  misc_feature 2^3: note = Phosphorothioate bond
  modified_base 3: mod_base = cm
  modified_base 4: mod_base = cm
  modified_base 5: mod_base = um
  modified_base 6: mod_base = OTHER; note = 2'-Fluoro-uridine
  modified_base 7: mod_base = OTHER; note = 2'-O-methyl-adenosine
  modified_base 8: mod_base = OTHER; note = 2'-O-methyl-adenosine
  modified_base 9: mod_base = um
  modified_base 10: mod_base = cm
  modified_base 11: mod_base = cm
  modified_base 12: mod_base = cm
  modified_base 13: mod_base = OTHER; note = 2'-O-methyl-adenosine
  modified_base 14: mod_base = OTHER; note = 2'-Fluoro-uridine
  modified_base 15: mod_base = cm
  modified_base 16: mod_base = OTHER; note = 2'-Fluoro-adenosine
  modified_base 17: mod_base = gm
  modified_base 18: mod_base = OTHER; note = 2'-Fluoro-adenosine
  modified_base 19: mod_base = um
  modified_base 20: mod_base = um
  modified_base 21: mod_base = um
  misc_feature 21^22: note = Phosphorothioate bond
  modified_base 22: mod_base = gm
  misc_feature 22^23: note = Phosphorothioate bond
  modified_base 23: mod_base = um
gcccttaatcccatcagatttgt

SEQ ID NO: 1069 - RNA, 23 nt, synthetic construct
  source 1..23: mol_type = other RNA
  modified_base 1: mod_base = um
  misc_feature 1^2: note = Phosphorothioate bond
  modified_base 2: mod_base = OTHER; note = 2'-Fluoro-uridine
  misc_feature 2^3: note = Phosphorothioate bond
  modified_base 3: mod_base = OTHER; note = 2'-O-methyl-adenosine
  modified_base 4: mod_base = OTHER; note = 2'-O-methyl-adenosine
  modified_base 5: mod_base = um
  modified_base 6: mod_base = OTHER; note = 2'-Fluoro-cytidine
  modified_base 7: mod_base = cm
  modified_base 8: mod_base = cm
  modified_base 9: mod_base = OTHER; note = 2'-O-methyl-adenosine
  modified_base 10: mod_base = um
  modified_base 11: mod_base = cm
  modified_base 12: mod_base = OTHER; note = 2'-O-methyl-adenosine
  modified_base 13: mod_base = gm
  modified_base 14: mod_base = OTHER; note = 2'-Fluoro-adenosine
  modified_base 15: mod_base = um
  modified_base 16: mod_base = OTHER; note = 2'-Fluoro-uridine
  modified_base 17: mod_base = um
  modified_base 18: mod_base = OTHER; note = 2'-Fluoro-guanosine
  modified_base 19: mod_base = um
  modified_base 20: mod_base = OTHER; note = 2'-O-methyl-adenosine
  modified_base 21: mod_base = gm
  misc_feature 21^22: note = Phosphorothioate bond
  modified_base 22: mod_base = OTHER; note = 2'-O-methyl-adenosine
  misc_feature 22^23: note = Phosphorothioate bond
  modified_base 23: mod_base = um
ttaatcccatcagatttgtagat

SEQ ID NO: 1070 - RNA, 23 nt, synthetic construct
  source 1..23: mol_type = other RNA
  modified_base 1: mod_base = um
  misc_feature 1^2: note = Phosphorothioate bond
  modified_base 2: mod_base = OTHER; note = 2'-Fluoro-cytidine
  misc_feature 2^3: note = Phosphorothioate bond
  modified_base 3: mod_base = gm
  modified_base 4: mod_base = gm
  modified_base 5: mod_base = um
  modified_base 6: mod_base = OTHER; note = 2'-Fluoro-adenosine
  modified_base 7: mod_base = gm
  modified_base 8: mod_base = OTHER; note = 2'-O-methyl-adenosine
  modified_base 9: mod_base = um
  modified_base 10: mod_base = gm
  modified_base 11: mod_base = OTHER; note = 2'-O-methyl-adenosine
  modified_base 12: mod_base = um
  modified_base 13: mod_base = OTHER; note = 2'-O-methyl-adenosine
  modified_base 14: mod_base = OTHER; note = 2'-Fluoro-adenosine
  modified_base 15: mod_base = um
  modified_base 16: mod_base = OTHER; note = 2'-Fluoro-adenosine
  modified_base 17: mod_base = cm
  modified_base 18: mod_base = OTHER; note = 2'-Fluoro-cytidine
  modified_base 19: mod_base = cm
  modified_base 20: mod_base = um
  modified_base 21: mod_base = gm
  misc_feature 21^22: note = Phosphorothioate bond
  modified_base 22: mod_base = cm
  misc_feature 22^23: note = Phosphorothioate bond
  modified_base 23: mod_base = OTHER; note = 2'-O-methyl-adenosine
tcggtagatgataataccctgca

SEQ ID NO: 1071 - RNA, 23 nt, synthetic construct
  source 1..23: mol_type = other RNA
  modified_base 1: mod_base = cm
  misc_feature 1^2: note = Phosphorothioate bond
  modified_base 2: mod_base = OTHER; note = 2'-Fluoro-adenosine
  misc_feature 2^3: note = Phosphorothioate bond
  modified_base 3: mod_base = cm
  modified_base 4: mod_base = gm
  modified_base 5: mod_base = um
  modified_base 6: mod_base = OTHER; note = 2'-Fluoro-uridine
  modified_base 7: mod_base = OTHER; note = 2'-O-methyl-adenosine
  modified_base 8: mod_base = OTHER; note = 2'-O-methyl-adenosine
  modified_base 9: mod_base = OTHER; note = 2'-O-methyl-adenosine
  modified_base 10: mod_base = gm
  modified_base 11: mod_base = cm
  modified_base 12: mod_base = cm
  modified_base 13: mod_base = um
  modified_base 14: mod_base = OTHER; note = 2'-Fluoro-uridine
  modified_base 15: mod_base = gm
  modified_base 16: mod_base = OTHER; note = 2'-Fluoro-guanosine
  modified_base 17: mod_base = um
  modified_base 18: mod_base = OTHER; note = 2'-Fluoro-adenosine
  modified_base 19: mod_base = cm
  modified_base 20: mod_base = OTHER; note = 2'-O-methyl-adenosine
  modified_base 21: mod_base = gm
  misc_feature 21^22: note = Phosphorothioate bond
  modified_base 22: mod_base = gm
  misc_feature 22^23: note = Phosphorothioate bond
  modified_base 23: mod_base = cm
cacgttaaagccttggtacaggc

SEQ ID NO: 1072 - RNA, 23 nt, synthetic construct
  source 1..23: mol_type = other RNA
  modified_base 1: mod_base = um
  misc_feature 1^2: note = Phosphorothioate bond
  modified_base 2: mod_base = OTHER; note = 2'-Fluoro-cytidine
  misc_feature 2^3: note = Phosphorothioate bond
  modified_base 3: mod_base = cm
  modified_base 4: mod_base = cm
  modified_base 5: mod_base = OTHER; note = 2'-O-methyl-adenosine
  modified_base 6: mod_base = OTHER; note = 2'-Fluoro-uridine
  modified_base 7: mod_base = cm
  modified_base 8: mod_base = OTHER; note = 2'-O-methyl-adenosine
  modified_base 9: mod_base = gm
  modified_base 10: mod_base = OTHER; note = 2'-O-methyl-adenosine
  modified_base 11: mod_base = um
  modified_base 12: mod_base = um
  modified_base 13: mod_base = um
  modified_base 14: mod_base = OTHER; note = 2'-Fluoro-guanosine
  modified_base 15: mod_base = um
  modified_base 16: mod_base = OTHER; note = 2'-Fluoro-adenosine
  modified_base 17: mod_base = gm
  modified_base 18: mod_base = OTHER; note = 2'-Fluoro-adenosine
  modified_base 19: mod_base = um
  modified_base 20: mod_base = cm
  modified_base 21: mod_base = um
  misc_feature 21^22: note = Phosphorothioate bond
  modified_base 22: mod_base = um
  misc_feature 22^23: note = Phosphorothioate bond
  modified_base 23: mod_base = OTHER; note = 2'-O-methyl-adenosine
tcccatcagatttgtagatctta

SEQ ID NO: 1073 - RNA, 23 nt, synthetic construct
  source 1..23: mol_type = other RNA
  modified_base 1: mod_base = um
  misc_feature 1^2: note = Phosphorothioate bond
  modified_base 2: mod_base = OTHER; note = 2'-Fluoro-cytidine
  misc_feature 2^3: note = Phosphorothioate bond
  modified_base 3: mod_base = OTHER; note = 2'-O-methyl-adenosine
  modified_base 4: mod_base = um
  modified_base 5: mod_base = OTHER; note = 2'-O-methyl-adenosine
  modified_base 6: mod_base = OTHER; note = 2'-Fluoro-cytidine
  modified_base 7: mod_base = OTHER; note = 2'-O-methyl-adenosine
  modified_base 8: mod_base = OTHER; note = 2'-O-methyl-adenosine
  modified_base 9: mod_base = gm
  modified_base 10: mod_base = OTHER; note = 2'-O-methyl-adenosine
  modified_base 11: mod_base = cm
  modified_base 12: mod_base = OTHER; note = 2'-O-methyl-adenosine
  modified_base 13: mod_base = OTHER; note = 2'-O-methyl-adenosine
  modified_base 14: mod_base = OTHER; note = 2'-Fluoro-guanosine
  modified_base 15: mod_base = cm
  modified_base 16: mod_base = OTHER; note = 2'-Fluoro-adenosine
  modified_base 17: mod_base = cm
  modified_base 18: mod_base = OTHER; note = 2'-Fluoro-adenosine
  modified_base 19: mod_base = OTHER; note = 2'-O-methyl-adenosine
  modified_base 20: mod_base = OTHER; note = 2'-O-methyl-adenosine
  modified_base 21: mod_base = OTHER; note = 2'-O-methyl-adenosine
  misc_feature 21^22: note = Phosphorothioate bond
  modified_base 22: mod_base = gm
  misc_feature 22^23: note = Phosphorothioate bond
  modified_base 23: mod_base = cm
tcatacaagacaagcacaaaagc

SEQ ID NO: 1074 - RNA, 23 nt, synthetic construct
  source 1..23: mol_type = other RNA
  modified_base 1: mod_base = cm
  misc_feature 1^2: note = Phosphorothioate bond
  modified_base 2: mod_base = OTHER; note = 2'-Fluoro-cytidine
  misc_feature 2^3: note = Phosphorothioate bond
  modified_base 3: mod_base = um
  modified_base 4: mod_base = um
  modified_base 5: mod_base = OTHER; note = 2'-O-methyl-adenosine
  modified_base 6: mod_base = OTHER; note = 2'-Fluoro-adenosine
  modified_base 7: mod_base = um
  modified_base 8: mod_base = cm
  modified_base 9: mod_base = cm
  modified_base 10: mod_base = cm
  modified_base 11: mod_base = OTHER; note = 2'-O-methyl-adenosine
  modified_base 12: mod_base = um
  modified_base 13: mod_base = cm
  modified_base 14: mod_base = OTHER; note = 2'-Fluoro-adenosine
  modified_base 15: mod_base = gm
  modified_base 16: mod_base = OTHER; note = 2'-Fluoro-adenosine
  modified_base 17: mod_base = um
  modified_base 18: mod_base = OTHER; note = 2'-Fluoro-uridine
  modified_base 19: mod_base = um
  modified_base 20: mod_base = gm
  modified_base 21: mod_base = um
  misc_feature 21^22: note = Phosphorothioate bond
  modified_base 22: mod_base = OTHER; note = 2'-O-methyl-adenosine
  misc_feature 22^23: note = Phosphorothioate bond
  modified_base 23: mod_base = gm
ccttaatcccatcagatttgtag

SEQ ID NO: 1075 - RNA, 23 nt, synthetic construct
  source 1..23: mol_type = other RNA
  modified_base 1: mod_base = OTHER; note = 2'-O-methyl-adenosine
  misc_feature 1^2: note = Phosphorothioate bond
  modified_base 2: mod_base = OTHER; note = 2'-Fluoro-cytidine
  misc_feature 2^3: note = Phosphorothioate bond
  modified_base 3: mod_base = OTHER; note = 2'-O-methyl-adenosine
  modified_base 4: mod_base = um
  modified_base 5: mod_base = um
  modified_base 6: mod_base = OTHER; note = 2'-Fluoro-guanosine
  modified_base 7: mod_base = gm
  modified_base 8: mod_base = OTHER; note = 2'-O-methyl-adenosine
  modified_base 9: mod_base = cm
  modified_base 10: mod_base = cm
  modified_base 11: mod_base = OTHER; note = 2'-O-methyl-adenosine
  modified_base 12: mod_base = um
  modified_base 13: mod_base = gm
  modified_base 14: mod_base = OTHER; note = 2'-Fluoro-cytidine
  modified_base 15: mod_base = OTHER; note = 2'-O-methyl-adenosine
  modified_base 16: mod_base = OTHER; note = 2'-Fluoro-cytidine
  modified_base 17: mod_base = cm
  modified_base 18: mod_base = OTHER; note = 2'-Fluoro-cytidine
  modified_base 19: mod_base = um
  modified_base 20: mod_base = um
  modified_base 21: mod_base = gm
  misc_feature 21^22: note = Phosphorothioate bond
  modified_base 22: mod_base = OTHER; note = 2'-O-methyl-adenosine
  misc_feature 22^23: note = Phosphorothioate bond
  modified_base 23: mod_base = OTHER; note = 2'-O-methyl-adenosine
acattggaccatgcacccttgaa

SEQ ID NO: 1076 - RNA, 23 nt, synthetic construct
  source 1..23: mol_type = other RNA
  modified_base 1: mod_base = cm
  misc_feature 1^2: note = Phosphorothioate bond
  modified_base 2: mod_base = OTHER; note = 2'-Fluoro-uridine
  misc_feature 2^3: note = Phosphorothioate bond
  modified_base 3: mod_base = um
  modified_base 4: mod_base = gm
  modified_base 5: mod_base = gm
  modified_base 6: mod_base = OTHER; note = 2'-Fluoro-uridine
  modified_base 7: mod_base = OTHER; note = 2'-O-methyl-adenosine
  modified_base 8: mod_base = cm
  modified_base 9: mod_base = OTHER; note = 2'-O-methyl-adenosine
  modified_base 10: mod_base = gm
  modified_base 11: mod_base = gm
  modified_base 12: mod_base = cm
  modified_base 13: mod_base = cm
  modified_base 14: mod_base = OTHER; note = 2'-Fluoro-cytidine
  modified_base 15: mod_base = um
  modified_base 16: mod_base = OTHER; note = 2'-Fluoro-uridine
  modified_base 17: mod_base = OTHER; note = 2'-O-methyl-adenosine
  modified_base 18: mod_base = OTHER; note = 2'-Fluoro-adenosine
  modified_base 19: mod_base = um
  modified_base 20: mod_base = cm
  modified_base 21: mod_base = cm
  misc_feature 21^22: note = Phosphorothioate bond
  modified_base 22: mod_base = cm
  misc_feature 22^23: note = Phosphorothioate bond
  modified_base 23: mod_base = OTHER; note = 2'-O-methyl-adenosine
cttggtacaggcccttaatccca

SEQ ID NO: 1077 - RNA, 23 nt, synthetic construct
  source 1..23: mol_type = other RNA
  modified_base 1: mod_base = um
  misc_feature 1^2: note = Phosphorothioate bond
  modified_base 2: mod_base = OTHER; note = 2'-Fluoro-uridine
  misc_feature 2^3: note = Phosphorothioate bond
  modified_base 3: mod_base = gm
  modified_base 4: mod_base = cm
  modified_base 5: mod_base = OTHER; note = 2'-O-methyl-adenosine
  modified_base 6: mod_base = OTHER; note = 2'-Fluoro-guanosine
  modified_base 7: mod_base = um
  modified_base 8: mod_base = gm
  modified_base 9: mod_base = um
  modified_base 10: mod_base = cm
  modified_base 11: mod_base = OTHER; note = 2'-O-methyl-adenosine
  modified_base 12: mod_base = um
  modified_base 13: mod_base = OTHER; note = 2'-O-methyl-adenosine
  modified_base 14: mod_base = OTHER; note = 2'-Fluoro-guanosine
  modified_base 15: mod_base = OTHER; note = 2'-O-methyl-adenosine
  modified_base 16: mod_base = OTHER; note = 2'-Fluoro-uridine
  modified_base 17: mod_base = OTHER; note = 2'-O-methyl-adenosine
  modified_base 18: mod_base = OTHER; note = 2'-Fluoro-cytidine
  modified_base 19: mod_base = cm
  modified_base 20: mod_base = gm
  modified_base 21: mod_base = OTHER; note = 2'-O-methyl-adenosine
  misc_feature 21^22: note = Phosphorothioate bond
  modified_base 22: mod_base = OTHER; note = 2'-O-methyl-adenosine
  misc_feature 22^23: note = Phosphorothioate bond
  modified_base 23: mod_base = gm
ttgcagtgtcatagataccgaag

SEQ ID NO: 1078 - RNA, 23 nt, synthetic construct
  source 1..23: mol_type = other RNA
  modified_base 1: mod_base = cm
  misc_feature 1^2: note = Phosphorothioate bond
  modified_base 2: mod_base = OTHER; note = 2'-Fluoro-adenosine
  misc_feature 2^3: note = Phosphorothioate bond
  modified_base 3: mod_base = cm
  modified_base 4: mod_base = OTHER; note = 2'-O-methyl-adenosine
  modified_base 5: mod_base = gm
  modified_base 6: mod_base = OTHER; note = 2'-Fluoro-adenosine
  modified_base 7: mod_base = cm
  modified_base 8: mod_base = OTHER; note = 2'-O-methyl-adenosine
  modified_base 9: mod_base = cm
  modified_base 10: mod_base = gm
  modified_base 11: mod_base = um
  modified_base 12: mod_base = um
  modified_base 13: mod_base = OTHER; note = 2'-O-methyl-adenosine
  modified_base 14: mod_base = OTHER; note = 2'-Fluoro-adenosine
  modified_base 15: mod_base = OTHER; note = 2'-O-methyl-adenosine
  modified_base 16: mod_base = OTHER; note = 2'-Fluoro-guanosine
  modified_base 17: mod_base = cm
  modified_base 18: mod_base = OTHER; note = 2'-Fluoro-cytidine
  modified_base 19: mod_base = um
  modified_base 20: mod_base = um
  modified_base 21: mod_base = gm
  misc_feature 21^22: note = Phosphorothioate bond
  modified_base 22: mod_base = gm
  misc_feature 22^23: note = Phosphorothioate bond
  modified_base 23: mod_base = um
cacagacacgttaaagccttggt

SEQ ID NO: 1079 - RNA, 23 nt, synthetic construct
  source 1..23: mol_type = other RNA
  modified_base 1: mod_base = OTHER; note = 2'-O-methyl-adenosine
  misc_feature 1^2: note = Phosphorothioate bond
  modified_base 2: mod_base = OTHER; note = 2'-Fluoro-guanosine
  misc_feature 2^3: note = Phosphorothioate bond
  modified_base 3: mod_base = cm
  modified_base 4: mod_base = OTHER; note = 2'-O-methyl-adenosine
  modified_base 5: mod_base = cm
  modified_base 6: mod_base = OTHER; note = 2'-Fluoro-adenosine
  modified_base 7: mod_base = OTHER; note = 2'-O-methyl-adenosine
  modified_base 8: mod_base = OTHER; note = 2'-O-methyl-adenosine
  modified_base 9: mod_base = OTHER; note = 2'-O-methyl-adenosine
  modified_base 10: mod_base = gm
  modified_base 11: mod_base = cm
  modified_base 12: mod_base = OTHER; note = 2'-O-methyl-adenosine
  modified_base 13: mod_base = cm
  modified_base 14: mod_base = OTHER; note = 2'-Fluoro-cytidine
  modified_base 15: mod_base = OTHER; note = 2'-O-methyl-adenosine
  modified_base 16: mod_base = OTHER; note = 2'-Fluoro-cytidine
  modified_base 17: mod_base = cm
  modified_base 18: mod_base = OTHER; note = 2'-Fluoro-cytidine
  modified_base 19: mod_base = OTHER; note = 2'-O-methyl-adenosine
  modified_base 20: mod_base = um
  modified_base 21: mod_base = gm
  misc_feature 21^22: note = Phosphorothioate bond
  modified_base 22: mod_base = cm
  misc_feature 22^23: note = Phosphorothioate bond
  modified_base 23: mod_base = cm
agcacaaaagcaccacccatgcc

SEQ ID NO: 1080 - RNA, 23 nt, synthetic construct
  source 1..23: mol_type = other RNA
  modified_base 1: mod_base = cm
  misc_feature 1^2: note = Phosphorothioate bond
  modified_base 2: mod_base = OTHER; note = 2'-Fluoro-cytidine
  misc_feature 2^3: note = Phosphorothioate bond
  modified_base 3: mod_base = OTHER; note = 2'-O-methyl-adenosine
  modified_base 4: mod_base = um
  modified_base 5: mod_base = cm
  modified_base 6: mod_base = OTHER; note = 2'-Fluoro-adenosine
  modified_base 7: mod_base = gm
  modified_base 8: mod_base = OTHER; note = 2'-O-methyl-adenosine
  modified_base 9: mod_base = um
  modified_base 10: mod_base = um
  modified_base 11: mod_base = um
  modified_base 12: mod_base = gm
  modified_base 13: mod_base = um
  modified_base 14: mod_base = OTHER; note = 2'-Fluoro-adenosine
  modified_base 15: mod_base = gm
  modified_base 16: mod_base = OTHER; note = 2'-Fluoro-adenosine
  modified_base 17: mod_base = um
  modified_base 18: mod_base = OTHER; note = 2'-Fluoro-cytidine
  modified_base 19: mod_base = um
  modified_base 20: mod_base = um
  modified_base 21: mod_base = OTHER; note = 2'-O-methyl-adenosine
  misc_feature 21^22: note = Phosphorothioate bond
  modified_base 22: mod_base = OTHER; note = 2'-O-methyl-adenosine
  misc_feature 22^23: note = Phosphorothioate bond
  modified_base 23: mod_base = cm
ccatcagatttgtagatcttaac

SEQ ID NO: 1081 - RNA, 23 nt, synthetic construct
  source 1..23: mol_type = other RNA
  modified_base 1: mod_base = cm
  misc_feature 1^2: note = Phosphorothioate bond
  modified_base 2: mod_base = OTHER; note = 2'-Fluoro-cytidine
  misc_feature 2^3: note = Phosphorothioate bond
  modified_base 3: mod_base = OTHER; note = 2'-O-methyl-adenosine
  modified_base 4: mod_base = cm
  modified_base 5: mod_base = OTHER; note = 2'-O-methyl-adenosine
  modified_base 6: mod_base = OTHER; note = 2'-Fluoro-uridine
  modified_base 7: mod_base = cm
  modified_base 8: mod_base = OTHER; note = 2'-O-methyl-adenosine
  modified_base 9: mod_base = gm
  modified_base 10: mod_base = cm
  modified_base 11: mod_base = um
  modified_base 12: mod_base = gm
  modified_base 13: mod_base = cm
  modified_base 14: mod_base = OTHER; note = 2'-Fluoro-uridine
  modified_base 15: mod_base = OTHER; note = 2'-O-methyl-adenosine
  modified_base 16: mod_base = OTHER; note = 2'-Fluoro-guanosine
  modified_base 17: mod_base = OTHER; note = 2'-O-methyl-adenosine
  modified_base 18: mod_base = OTHER; note = 2'-Fluoro-cytidine
  modified_base 19: mod_base = gm
  modified_base 20: mod_base = gm
  modified_base 21: mod_base = gm
  misc_feature 21^22: note = Phosphorothioate bond
  modified_base 22: mod_base = um
  misc_feature 22^23: note = Phosphorothioate bond
  modified_base 23: mod_base = OTHER; note = 2'-O-methyl-adenosine
ccacatcagctgctagacgggta

SEQ ID NO: 1082 - RNA, 23 nt, synthetic construct
  source 1..23: mol_type = other RNA
  modified_base 1: mod_base = gm
  misc_feature 1^2: note = Phosphorothioate bond
  modified_base 2: mod_base = OTHER; note = 2'-Fluoro-cytidine
  misc_feature 2^3: note = Phosphorothioate bond
  modified_base 3: mod_base = OTHER; note = 2'-O-methyl-adenosine
  modified_base 4: mod_base = um
  modified_base 5: mod_base = um
  modified_base 6: mod_base = OTHER; note = 2'-Fluoro-cytidine
  modified_base 7: mod_base = cm
  modified_base 8: mod_base = cm
  modified_base 9: mod_base = um
  modified_base 10: mod_base = um
  modified_base 11: mod_base = um
  modified_base 12: mod_base = gm
  modified_base 13: mod_base = cm
  modified_base 14: mod_base = OTHER; note = 2'-Fluoro-adenosine
  modified_base 15: mod_base = gm
  modified_base 16: mod_base = OTHER; note = 2'-Fluoro-uridine
  modified_base 17: mod_base = gm
  modified_base 18: mod_base = OTHER; note = 2'-Fluoro-uridine
  modified_base 19: mod_base = cm
  modified_base 20: mod_base = OTHER; note = 2'-O-methyl-adenosine
  modified_base 21: mod_base = um
  misc_feature 21^22: note = Phosphorothioate bond
  modified_base 22: mod_base = OTHER; note = 2'-O-methyl-adenosine
  misc_feature 22^23: note = Phosphorothioate bond
  modified_base 23: mod_base = gm
gcattccctttgcagtgtcatag

SEQ ID NO: 1083 - RNA, 23 nt, synthetic construct
  source 1..23: mol_type = other RNA
  modified_base 1: mod_base = cm
  misc_feature 1^2: note = Phosphorothioate bond
  modified_base 2: mod_base = OTHER; note = 2'-Fluoro-uridine
  misc_feature 2^3: note = Phosphorothioate bond
  modified_base 3: mod_base = um
  modified_base 4: mod_base = um
  modified_base 5: mod_base = OTHER; note = 2'-O-methyl-adenosine
  modified_base 6: mod_base = OTHER; note = 2'-Fluoro-cytidine
  modified_base 7: mod_base = cm
  modified_base 8: mod_base = cm
  modified_base 9: mod_base = OTHER; note = 2'-O-methyl-adenosine
  modified_base 10: mod_base = cm
  modified_base 11: mod_base = OTHER; note = 2'-O-methyl-adenosine
  modified_base 12: mod_base = um
  modified_base 13: mod_base = cm
  modified_base 14: mod_base = OTHER; note = 2'-Fluoro-adenosine
  modified_base 15: mod_base = gm
  modified_base 16: mod_base = OTHER; note = 2'-Fluoro-cytidine
  modified_base 17: mod_base = um
  modified_base 18: mod_base = OTHER; note = 2'-Fluoro-guanosine
  modified_base 19: mod_base = cm
  modified_base 20: mod_base = um
  modified_base 21: mod_base = OTHER; note = 2'-O-methyl-adenosine
  misc_feature 21^22: note = Phosphorothioate bond
  modified_base 22: mod_base = gm
  misc_feature 22^23: note = Phosphorothioate bond
  modified_base 23: mod_base = OTHER; note = 2'-O-methyl-adenosine
ctttacccacatcagctgctaga

SEQ ID NO: 1084 - RNA, 23 nt, synthetic construct
  source 1..23: mol_type = other RNA
  modified_base 1: mod_base = OTHER; note = 2'-O-methyl-adenosine
  misc_feature 1^2: note = Phosphorothioate bond
  modified_base 2: mod_base = OTHER; note = 2'-Fluoro-uridine
  misc_feature 2^3: note = Phosphorothioate bond
  modified_base 3: mod_base = cm
  modified_base 4: mod_base = cm
  modified_base 5: mod_base = gm
  modified_base 6: mod_base = OTHER; note = 2'-Fluoro-guanosine
  modified_base 7: mod_base = OTHER; note = 2'-O-methyl-adenosine
  modified_base 8: mod_base = OTHER; note = 2'-O-methyl-adenosine
  modified_base 9: mod_base = gm
  modified_base 10: mod_base = cm
  modified_base 11: mod_base = OTHER; note = 2'-O-methyl-adenosine
  modified_base 12: mod_base = um
  modified_base 13: mod_base = um
  modified_base 14: mod_base = OTHER; note = 2'-Fluoro-cytidine
  modified_base 15: mod_base = cm
  modified_base 16: mod_base = OTHER; note = 2'-Fluoro-cytidine
  modified_base 17: mod_base = um
  modified_base 18: mod_base = OTHER; note = 2'-Fluoro-uridine
  modified_base 19: mod_base = um
  modified_base 20: mod_base = gm
  modified_base 21: mod_base = cm
  misc_feature 21^22: note = Phosphorothioate bond
  modified_base 22: mod_base = OTHER; note = 2'-O-methyl-adenosine
  misc_feature 22^23: note = Phosphorothioate bond
  modified_base 23: mod_base = gm
atccggaagcattccctttgcag

SEQ ID NO: 1085 - RNA, 23 nt, synthetic construct
  source 1..23: mol_type = other RNA
  modified_base 1: mod_base = OTHER; note = 2'-O-methyl-adenosine
  misc_feature 1^2: note = Phosphorothioate bond
  modified_base 2: mod_base = OTHER; note = 2'-Fluoro-guanosine
  misc_feature 2^3: note = Phosphorothioate bond
  modified_base 3: mod_base = cm
  modified_base 4: mod_base = um
  modified_base 5: mod_base = gm
  modified_base 6: mod_base = OTHER; note = 2'-Fluoro-cytidine
  modified_base 7: mod_base = um
  modified_base 8: mod_base = OTHER; note = 2'-O-methyl-adenosine
  modified_base 9: mod_base = gm
  modified_base 10: mod_base = OTHER; note = 2'-O-methyl-adenosine
  modified_base 11: mod_base = cm
  modified_base 12: mod_base = gm
  modified_base 13: mod_base = gm
  modified_base 14: mod_base = OTHER; note = 2'-Fluoro-guanosine
  modified_base 15: mod_base = um
  modified_base 16: mod_base = OTHER; note = 2'-Fluoro-adenosine
  modified_base 17: mod_base = cm
  modified_base 18: mod_base = OTHER; note = 2'-Fluoro-guanosine
  modified_base 19: mod_base = gm
  modified_base 20: mod_base = gm
  modified_base 21: mod_base = cm
  misc_feature 21^22: note = Phosphorothioate bond
  modified_base 22: mod_base = OTHER; note = 2'-O-methyl-adenosine
  misc_feature 22^23: note = Phosphorothioate bond
  modified_base 23: mod_base = OTHER; note = 2'-O-methyl-adenosine
agctgctagacgggtacgggcaa

SEQ ID NO: 1086 - RNA, 23 nt, synthetic construct
  source 1..23: mol_type = other RNA
  modified_base 1: mod_base = cm
  misc_feature 1^2: note = Phosphorothioate bond
  modified_base 2: mod_base = OTHER; note = 2'-Fluoro-guanosine
  misc_feature 2^3: note = Phosphorothioate bond
  modified_base 3: mod_base = gm
  modified_base 4: mod_base = cm
  modified_base 5: mod_base = um
  modified_base 6: mod_base = OTHER; note = 2'-Fluoro-cytidine
  modified_base 7: mod_base = gm
  modified_base 8: mod_base = gm
  modified_base 9: mod_base = um
  modified_base 10: mod_base = OTHER; note = 2'-O-methyl-adenosine
  modified_base 11: mod_base = gm
  modified_base 12: mod_base = OTHER; note = 2'-O-methyl-adenosine
  modified_base 13: mod_base = um
  modified_base 14: mod_base = OTHER; note = 2'-Fluoro-guanosine
  modified_base 15: mod_base = OTHER; note = 2'-O-methyl-adenosine
  modified_base 16: mod_base = OTHER; note = 2'-Fluoro-uridine
  modified_base 17: mod_base = OTHER; note = 2'-O-methyl-adenosine
  modified_base 18: mod_base = OTHER; note = 2'-Fluoro-adenosine
  modified_base 19: mod_base = um
  modified_base 20: mod_base = OTHER; note = 2'-O-methyl-adenosine
  modified_base 21: mod_base = cm
  misc_feature 21^22: note = Phosphorothioate bond
  modified_base 22: mod_base = cm
  misc_feature 22^23: note = Phosphorothioate bond
  modified_base 23: mod_base = cm
cggctcggtagatgataataccc

SEQ ID NO: 1087 - RNA, 23 nt, synthetic construct
  source 1..23: mol_type = other RNA
  modified_base 1: mod_base = gm
  misc_feature 1^2: note = Phosphorothioate bond
  modified_base 2: mod_base = OTHER; note = 2'-Fluoro-guanosine
  misc_feature 2^3: note = Phosphorothioate bond
  modified_base 3: mod_base = gm
  modified_base 4: mod_base = um
  modified_base 5: mod_base = OTHER; note = 2'-O-methyl-adenosine
  modified_base 6: mod_base = OTHER; note = 2'-Fluoro-cytidine
  modified_base 7: mod_base = gm
  modified_base 8: mod_base = gm
  modified_base 9: mod_base = gm
  modified_base 10: mod_base = cm
  modified_base 11: mod_base = OTHER; note = 2'-O-methyl-adenosine
  modified_base 12: mod_base = OTHER; note = 2'-O-methyl-adenosine
  modified_base 13: mod_base = OTHER; note = 2'-O-methyl-adenosine
  modified_base 14: mod_base = OTHER; note = 2'-Fluoro-adenosine
  modified_base 15: mod_base = um
  modified_base 16: mod_base = OTHER; note = 2'-Fluoro-cytidine
  modified_base 17: mod_base = OTHER; note = 2'-O-methyl-adenosine
  modified_base 18: mod_base = OTHER; note = 2'-Fluoro-adenosine
  modified_base 19: mod_base = gm
  modified_base 20: mod_base = OTHER; note = 2'-O-methyl-adenosine
  modified_base 21: mod_base = gm
  misc_feature 21^22: note = Phosphorothioate bond
  modified_base 22: mod_base = gm
  misc_feature 22^23: note = Phosphorothioate bond
  modified_base 23: mod_base = gm
gggtacgggcaaaatcaagaggg

SEQ ID NO: 1088 - RNA, 23 nt, synthetic construct
  source 1..23: mol_type = other RNA
  modified_base 1: mod_base = OTHER; note = 2'-O-methyl-adenosine
  misc_feature 1^2: note = Phosphorothioate bond
  modified_base 2: mod_base = OTHER; note = 2'-Fluoro-cytidine
  misc_feature 2^3: note = Phosphorothioate bond
  modified_base 3: mod_base = OTHER; note = 2'-O-methyl-adenosine
  modified_base 4: mod_base = um
  modified_base 5: mod_base = cm
  modified_base 6: mod_base = OTHER; note = 2'-Fluoro-adenosine
  modified_base 7: mod_base = gm
  modified_base 8: mod_base = cm
  modified_base 9: mod_base = um
  modified_base 10: mod_base = gm
  modified_base 11: mod_base = cm
  modified_base 12: mod_base = um
  modified_base 13: mod_base = OTHER; note = 2'-O-methyl-adenosine
  modified_base 14: mod_base = OTHER; note = 2'-Fluoro-guanosine
  modified_base 15: mod_base = OTHER; note = 2'-O-methyl-adenosine
  modified_base 16: mod_base = OTHER; note = 2'-Fluoro-cytidine
  modified_base 17: mod_base = gm
  modified_base 18: mod_base = OTHER; note = 2'-Fluoro-guanosine
  modified_base 19: mod_base = gm
  modified_base 20: mod_base = um
  modified_base 21: mod_base = OTHER; note = 2'-O-methyl-adenosine
  misc_feature 21^22: note = Phosphorothioate bond
  modified_base 22: mod_base = cm
  misc_feature 22^23: note = Phosphorothioate bond
  modified_base 23: mod_base = gm
acatcagctgctagacgggtacg

SEQ ID NO: 1089 - RNA, 23 nt, synthetic construct
  source 1..23: mol_type = other RNA
  modified_base 1: mod_base = cm
  misc_feature 1^2: note = Phosphorothioate bond
  modified_base 2: mod_base = OTHER; note = 2'-Fluoro-cytidine
  misc_feature 2^3: note = Phosphorothioate bond
  modified_base 3: mod_base = cm
  modified_base 4: mod_base = um
  modified_base 5: mod_base = um
  modified_base 6: mod_base = OTHER; note = 2'-Fluoro-adenosine
  modified_base 7: mod_base = OTHER; note = 2'-O-methyl-adenosine
  modified_base 8: mod_base = um
  modified_base 9: mod_base = cm
  modified_base 10: mod_base = cm
  modified_base 11: mod_base = cm
  modified_base 12: mod_base = OTHER; note = 2'-O-methyl-adenosine
  modified_base 13: mod_base = um
  modified_base 14: mod_base = OTHER; note = 2'-Fluoro-cytidine
  modified_base 15: mod_base = OTHER; note = 2'-O-methyl-adenosine
  modified_base 16: mod_base = OTHER; note = 2'-Fluoro-guanosine
  modified_base 17: mod_base = OTHER; note = 2'-O-methyl-adenosine
  modified_base 18: mod_base = OTHER; note = 2'-Fluoro-uridine
  modified_base 19: mod_base = um
  modified_base 20: mod_base = um
  modified_base 21: mod_base = gm
  misc_feature 21^22: note = Phosphorothioate bond
  modified_base 22: mod_base = um
  misc_feature 22^23: note = Phosphorothioate bond
  modified_base 23: mod_base = OTHER; note = 2'-O-methyl-adenosine
cccttaatcccatcagatttgta

SEQ ID NO: 1090 - RNA, 23 nt, synthetic construct
  source 1..23: mol_type = other RNA
  modified_base 1: mod_base = cm
  misc_feature 1^2: note = Phosphorothioate bond
  modified_base 2: mod_base = OTHER; note = 2'-Fluoro-guanosine
  misc_feature 2^3: note = Phosphorothioate bond
  modified_base 3: mod_base = gm
  modified_base 4: mod_base = gm
  modified_base 5: mod_base = cm
  modified_base 6: mod_base = OTHER; note = 2'-Fluoro-adenosine
  modified_base 7: mod_base = OTHER; note = 2'-O-methyl-adenosine
  modified_base 8: mod_base = OTHER; note = 2'-O-methyl-adenosine
  modified_base 9: mod_base = OTHER; note = 2'-O-methyl-adenosine
  modified_base 10: mod_base = um
  modified_base 11: mod_base = cm
  modified_base 12: mod_base = OTHER; note = 2'-O-methyl-adenosine
  modified_base 13: mod_base = OTHER; note = 2'-O-methyl-adenosine
  modified_base 14: mod_base = OTHER; note = 2'-Fluoro-guanosine
  modified_base 15: mod_base = OTHER; note = 2'-O-methyl-adenosine
  modified_base 16: mod_base = OTHER; note = 2'-Fluoro-guanosine
  modified_base 17: mod_base = gm
  modified_base 18: mod_base = OTHER; note = 2'-Fluoro-guanosine
  modified_base 19: mod_base = um
  modified_base 20: mod_base = OTHER; note = 2'-O-methyl-adenosine
  modified_base 21: mod_base = cm
  misc_feature 21^22: note = Phosphorothioate bond
  modified_base 22: mod_base = OTHER; note = 2'-O-methyl-adenosine
  misc_feature 22^23: note = Phosphorothioate bond
  modified_base 23: mod_base = cm
cgggcaaaatcaagagggtacac

SEQ ID NO: 1091 - RNA, 23 nt, synthetic construct
  source 1..23: mol_type = other RNA
  modified_base 1: mod_base = OTHER; note = 2'-O-methyl-adenosine
  misc_feature 1^2: note = Phosphorothioate bond
  modified_base 2: mod_base = OTHER; note = 2'-Fluoro-cytidine
  misc_feature 2^3: note = Phosphorothioate bond
  modified_base 3: mod_base = gm
  modified_base 4: mod_base = um
  modified_base 5: mod_base = um
  modified_base 6: mod_base = OTHER; note = 2'-Fluoro-adenosine
  modified_base 7: mod_base = OTHER; note = 2'-O-methyl-adenosine
  modified_base 8: mod_base = OTHER; note = 2'-O-methyl-adenosine
  modified_base 9: mod_base = gm
  modified_base 10: mod_base = cm
  modified_base 11: mod_base = cm
  modified_base 12: mod_base = um
  modified_base 13: mod_base = um
  modified_base 14: mod_base = OTHER; note = 2'-Fluoro-guanosine
  modified_base 15: mod_base = gm
  modified_base 16: mod_base = OTHER; note = 2'-Fluoro-uridine
  modified_base 17: mod_base = OTHER; note = 2'-O-methyl-adenosine
  modified_base 18: mod_base = OTHER; note = 2'-Fluoro-cytidine
  modified_base 19: mod_base = OTHER; note = 2'-O-methyl-adenosine
  modified_base 20: mod_base = gm
  modified_base 21: mod_base = gm
  misc_feature 21^22: note = Phosphorothioate bond
  modified_base 22: mod_base = cm
  misc_feature 22^23: note = Phosphorothioate bond
  modified_base 23: mod_base = cm
acgttaaagccttggtacaggcc

SEQ ID NO: 1092 - RNA, 23 nt, synthetic construct
  source 1..23: mol_type = other RNA
  modified_base 1: mod_base = um
  misc_feature 1^2: note = Phosphorothioate bond
  modified_base 2: mod_base = OTHER; note = 2'-Fluoro-guanosine
  misc_feature 2^3: note = Phosphorothioate bond
  modified_base 3: mod_base = gm
  modified_base 4: mod_base = um
  modified_base 5: mod_base = OTHER; note = 2'-O-methyl-adenosine
  modified_base 6: mod_base = OTHER; note = 2'-Fluoro-cytidine
  modified_base 7: mod_base = OTHER; note = 2'-O-methyl-adenosine
  modified_base 8: mod_base = gm
  modified_base 9: mod_base = gm
  modified_base 10: mod_base = cm
  modified_base 11: mod_base = cm
  modified_base 12: mod_base = cm
  modified_base 13: mod_base = um
  modified_base 14: mod_base = OTHER; note = 2'-Fluoro-uridine
  modified_base 15: mod_base = OTHER; note = 2'-O-methyl-adenosine
  modified_base 16: mod_base = OTHER; note = 2'-Fluoro-adenosine
  modified_base 17: mod_base = um
  modified_base 18: mod_base = OTHER; note = 2'-Fluoro-cytidine
  modified_base 19: mod_base = cm
  modified_base 20: mod_base = cm
  modified_base 21: mod_base = OTHER; note = 2'-O-methyl-adenosine
  misc_feature 21^22: note = Phosphorothioate bond
  modified_base 22: mod_base = um
  misc_feature 22^23: note = Phosphorothioate bond
  modified_base 23: mod_base = cm
tggtacaggcccttaatcccatc

SEQ ID NO: 1093 - RNA, 23 nt, synthetic construct
  source 1..23: mol_type = other RNA
  modified_base 1: mod_base = gm
  misc_feature 1^2: note = Phosphorothioate bond
  modified_base 2: mod_base = OTHER; note = 2'-Fluoro-guanosine
  misc_feature 2^3: note = Phosphorothioate bond
  modified_base 3: mod_base = cm
  modified_base 4: mod_base = gm
  modified_base 5: mod_base = gm
  modified_base 6: mod_base = OTHER; note = 2'-Fluoro-cytidine
  modified_base 7: mod_base = um
  modified_base 8: mod_base = cm
  modified_base 9: mod_base = gm
  modified_base 10: mod_base = gm
  modified_base 11: mod_base = um
  modified_base 12: mod_base = OTHER; note = 2'-O-methyl-adenosine
  modified_base 13: mod_base = gm
  modified_base 14: mod_base = OTHER; note = 2'-Fluoro-adenosine
  modified_base 15: mod_base = um
  modified_base 16: mod_base = OTHER; note = 2'-Fluoro-guanosine
  modified_base 17: mod_base = OTHER; note = 2'-O-methyl-adenosine
  modified_base 18: mod_base = OTHER; note = 2'-Fluoro-uridine
  modified_base 19: mod_base = OTHER; note = 2'-O-methyl-adenosine
  modified_base 20: mod_base = OTHER; note = 2'-O-methyl-adenosine
  modified_base 21: mod_base = um
  misc_feature 21^22: note = Phosphorothioate bond
  modified_base 22: mod_base = OTHER; note = 2'-O-methyl-adenosine
  misc_feature 22^23: note = Phosphorothioate bond
  modified_base 23: mod_base = cm
ggcggctcggtagatgataatac

SEQ ID NO: 1094 - RNA, 23 nt, synthetic construct
  source 1..23: mol_type = other RNA
  modified_base 1: mod_base = cm
  misc_feature 1^2: note = Phosphorothioate bond
  modified_base 2: mod_base = OTHER; note = 2'-Fluoro-guanosine
  misc_feature 2^3: note = Phosphorothioate bond
  modified_base 3: mod_base = um
  modified_base 4: mod_base = um
  modified_base 5: mod_base = OTHER; note = 2'-O-methyl-adenosine
  modified_base 6: mod_base = OTHER; note = 2'-Fluoro-adenosine
  modified_base 7: mod_base = OTHER; note = 2'-O-methyl-adenosine
  modified_base 8: mod_base = gm
  modified_base 9: mod_base = cm
  modified_base 10: mod_base = cm
  modified_base 11: mod_base = um
  modified_base 12: mod_base = um
  modified_base 13: mod_base = gm
  modified_base 14: mod_base = OTHER; note = 2'-Fluoro-guanosine
  modified_base 15: mod_base = um
  modified_base 16: mod_base = OTHER; note = 2'-Fluoro-adenosine
  modified_base 17: mod_base = cm
  modified_base 18: mod_base = OTHER; note = 2'-Fluoro-adenosine
  modified_base 19: mod_base = gm
  modified_base 20: mod_base = gm
  modified_base 21: mod_base = cm
  misc_feature 21^22: note = Phosphorothioate bond
  modified_base 22: mod_base = cm
  misc_feature 22^23: note = Phosphorothioate bond
  modified_base 23: mod_base = cm
cgttaaagccttggtacaggccc

SEQ ID NO: 1095 - RNA, 23 nt, synthetic construct
  source 1..23: mol_type = other RNA
  modified_base 1: mod_base = gm
  misc_feature 1^2: note = Phosphorothioate bond
  modified_base 2: mod_base = OTHER; note = 2'-Fluoro-guanosine
  misc_feature 2^3: note = Phosphorothioate bond
  modified_base 3: mod_base = um
  modified_base 4: mod_base = OTHER; note = 2'-O-methyl-adenosine
  modified_base 5: mod_base = cm
  modified_base 6: mod_base = OTHER; note = 2'-Fluoro-adenosine
  modified_base 7: mod_base = gm
  modified_base 8: mod_base = gm
  modified_base 9: mod_base = cm
  modified_base 10: mod_base = cm
  modified_base 11: mod_base = cm
  modified_base 12: mod_base = um
  modified_base 13: mod_base = um
  modified_base 14: mod_base = OTHER; note = 2'-Fluoro-adenosine
  modified_base 15: mod_base = OTHER; note = 2'-O-methyl-adenosine
  modified_base 16: mod_base = OTHER; note = 2'-Fluoro-uridine
  modified_base 17: mod_base = cm
  modified_base 18: mod_base = OTHER; note = 2'-Fluoro-cytidine
  modified_base 19: mod_base = cm
  modified_base 20: mod_base = OTHER; note = 2'-O-methyl-adenosine
  modified_base 21: mod_base = um
  misc_feature 21^22: note = Phosphorothioate bond
  modified_base 22: mod_base = cm
  misc_feature 22^23: note = Phosphorothioate bond
  modified_base 23: mod_base = OTHER; note = 2'-O-methyl-adenosine
ggtacaggcccttaatcccatca

SEQ ID NO: 1096 - RNA, 23 nt, synthetic construct
  source 1..23: mol_type = other RNA
  modified_base 1: mod_base = um
  misc_feature 1^2: note = Phosphorothioate bond
  modified_base 2: mod_base = OTHER; note = 2'-Fluoro-adenosine
  misc_feature 2^3: note = Phosphorothioate bond
  modified_base 3: mod_base = OTHER; note = 2'-O-methyl-adenosine
  modified_base 4: mod_base = um
  modified_base 5: mod_base = OTHER; note = 2'-O-methyl-adenosine
  modified_base 6: mod_base = OTHER; note = 2'-Fluoro-cytidine
  modified_base 7: mod_base = cm
  modified_base 8: mod_base = cm
  modified_base 9: mod_base = um
  modified_base 10: mod_base = gm
  modified_base 11: mod_base = cm
  modified_base 12: mod_base = OTHER; note = 2'-O-methyl-adenosine
  modified_base 13: mod_base = cm
  modified_base 14: mod_base = OTHER; note = 2'-Fluoro-adenosine
  modified_base 15: mod_base = gm
  modified_base 16: mod_base = OTHER; note = 2'-Fluoro-adenosine
  modified_base 17: mod_base = cm
  modified_base 18: mod_base = OTHER; note = 2'-Fluoro-adenosine
  modified_base 19: mod_base = cm
  modified_base 20: mod_base = gm
  modified_base 21: mod_base = um
  misc_feature 21^22: note = Phosphorothioate bond
  modified_base 22: mod_base = um
  misc_feature 22^23: note = Phosphorothioate bond
  modified_base 23: mod_base = OTHER; note = 2'-O-methyl-adenosine
taataccctgcacagacacgtta

SEQ ID NO: 1097 - RNA, 23 nt, synthetic construct
  source 1..23: mol_type = other RNA
  modified_base 1: mod_base = gm
  misc_feature 1^2: note = Phosphorothioate bond
  modified_base 2: mod_base = OTHER; note = 2'-Fluoro-adenosine
  misc_feature 2^3: note = Phosphorothioate bond
  modified_base 3: mod_base = cm
  modified_base 4: mod_base = cm
  modified_base 5: mod_base = OTHER; note = 2'-O-methyl-adenosine
  modified_base 6: mod_base = OTHER; note = 2'-Fluoro-cytidine
  modified_base 7: mod_base = gm
  modified_base 8: mod_base = cm
  modified_base 9: mod_base = OTHER; note = 2'-O-methyl-adenosine
  modified_base 10: mod_base = gm
  modified_base 11: mod_base = um
  modified_base 12: mod_base = cm
  modified_base 13: mod_base = um
  modified_base 14: mod_base = OTHER; note = 2'-Fluoro-adenosine
  modified_base 15: mod_base = um
  modified_base 16: mod_base = OTHER; note = 2'-Fluoro-adenosine
  modified_base 17: mod_base = OTHER; note = 2'-O-methyl-adenosine
  modified_base 18: mod_base = OTHER; note = 2'-Fluoro-uridine
  modified_base 19: mod_base = gm
  modified_base 20: mod_base = cm
  modified_base 21: mod_base = cm
  misc_feature 21^22: note = Phosphorothioate bond
  modified_base 22: mod_base = um
  misc_feature 22^23: note = Phosphorothioate bond
  modified_base 23: mod_base = um
gaccacgcagtctataatgcctt

SEQ ID NO: 1098 - RNA, 23 nt, synthetic construct
  source 1..23: mol_type = other RNA
  modified_base 1: mod_base = gm
  misc_feature 1^2: note = Phosphorothioate bond
  modified_base 2: mod_base = OTHER; note = 2'-Fluoro-uridine
  misc_feature 2^3: note = Phosphorothioate bond
  modified_base 3: mod_base = um
  modified_base 4: mod_base = OTHER; note = 2'-O-methyl-adenosine
  modified_base 5: mod_base = OTHER; note = 2'-O-methyl-adenosine
  modified_base 6: mod_base = OTHER; note = 2'-Fluoro-guanosine
  modified_base 7: mod_base = OTHER; note = 2'-O-methyl-adenosine
  modified_base 8: mod_base = gm
  modified_base 9: mod_base = cm
  modified_base 10: mod_base = cm
  modified_base 11: mod_base = um
  modified_base 12: mod_base = gm
  modified_base 13: mod_base = gm
  modified_base 14: mod_base = OTHER; note = 2'-Fluoro-guanosine
  modified_base 15: mod_base = um
  modified_base 16: mod_base = OTHER; note = 2'-Fluoro-guanosine
  modified_base 17: mod_base = gm
  modified_base 18: mod_base = OTHER; note = 2'-Fluoro-guanosine
  modified_base 19: mod_base = gm
  modified_base 20: mod_base = OTHER; note = 2'-O-methyl-adenosine
  modified_base 21: mod_base = OTHER; note = 2'-O-methyl-adenosine
  misc_feature 21^22: note = Phosphorothioate bond
  modified_base 22: mod_base = gm
  misc_feature 22^23: note = Phosphorothioate bond
  modified_base 23: mod_base = um
gttaagagcctgggtggggaagt

SEQ ID NO: 1099 - RNA, 23 nt, synthetic construct
  source 1..23: mol_type = other RNA
  modified_base 1: mod_base = um
  misc_feature 1^2: note = Phosphorothioate bond
  modified_base 2: mod_base = OTHER; note = 2'-Fluoro-guanosine
  misc_feature 2^3: note = Phosphorothioate bond
  modified_base 3: mod_base = gm
  modified_base 4: mod_base = gm
  modified_base 5: mod_base = gm
  modified_base 6: mod_base = OTHER; note = 2'-Fluoro-adenosine
  modified_base 7: mod_base = OTHER; note = 2'-O-methyl-adenosine
  modified_base 8: mod_base = gm
  modified_base 9: mod_base = um
  modified_base 10: mod_base = OTHER; note = 2'-O-methyl-adenosine
  modified_base 11: mod_base = um
  modified_base 12: mod_base = cm
  modified_base 13: mod_base = um
  modified_base 14: mod_base = OTHER; note = 2'-Fluoro-guanosine
  modified_base 15: mod_base = OTHER; note = 2'-O-methyl-adenosine
  modified_base 16: mod_base = OTHER; note = 2'-Fluoro-uridine
  modified_base 17: mod_base = gm
  modified_base 18: mod_base = OTHER; note = 2'-Fluoro-adenosine
  modified_base 19: mod_base = cm
  modified_base 20: mod_base = OTHER; note = 2'-O-methyl-adenosine
  modified_base 21: mod_base = um
  misc_feature 21^22: note = Phosphorothioate bond
  modified_base 22: mod_base = um
  misc_feature 22^23: note = Phosphorothioate bond
  modified_base 23: mod_base = gm
tggggaagtatctgatgacattg

SEQ ID NO: 1100 - RNA, 23 nt, synthetic construct
  source 1..23: mol_type = other RNA
  modified_base 1: mod_base = gm
  misc_feature 1^2: note = Phosphorothioate bond
  modified_base 2: mod_base = OTHER; note = 2'-Fluoro-guanosine
  misc_feature 2^3: note = Phosphorothioate bond
  modified_base 3: mod_base = um
  modified_base 4: mod_base = gm
  modified_base 5: mod_base = gm
  modified_base 6: mod_base = OTHER; note = 2'-Fluoro-guanosine
  modified_base 7: mod_base = gm
  modified_base 8: mod_base = OTHER; note = 2'-O-methyl-adenosine
  modified_base 9: mod_base = OTHER; note = 2'-O-methyl-adenosine
  modified_base 10: mod_base = gm
  modified_base 11: mod_base = um
  modified_base 12: mod_base = OTHER; note = 2'-O-methyl-adenosine
  modified_base 13: mod_base = um
  modified_base 14: mod_base = OTHER; note = 2'-Fluoro-cytidine
  modified_base 15: mod_base = um
  modified_base 16: mod_base = OTHER; note = 2'-Fluoro-guanosine
  modified_base 17: mod_base = OTHER; note = 2'-O-methyl-adenosine
  modified_base 18: mod_base = OTHER; note = 2'-Fluoro-uridine
  modified_base 19: mod_base = gm
  modified_base 20: mod_base = OTHER; note = 2'-O-methyl-adenosine
  modified_base 21: mod_base = cm
  misc_feature 21^22: note = Phosphorothioate bond
  modified_base 22: mod_base = OTHER; note = 2'-O-methyl-adenosine
  misc_feature 22^23: note = Phosphorothioate bond
  modified_base 23: mod_base = um
ggtggggaagtatctgatgacat

SEQ ID NO: 1101 - RNA, 23 nt, synthetic construct
  source 1..23: mol_type = other RNA
  modified_base 1: mod_base = gm
  misc_feature 1^2: note = Phosphorothioate bond
  modified_base 2: mod_base = OTHER; note = 2'-Fluoro-uridine
  misc_feature 2^3: note = Phosphorothioate bond
  modified_base 3: mod_base = gm
  modified_base 4: mod_base = gm
  modified_base 5: mod_base = gm
  modified_base 6: mod_base = OTHER; note = 2'-Fluoro-guanosine
  modified_base 7: mod_base = OTHER; note = 2'-O-methyl-adenosine
  modified_base 8: mod_base = OTHER; note = 2'-O-methyl-adenosine
  modified_base 9: mod_base = gm
  modified_base 10: mod_base = um
  modified_base 11: mod_base = OTHER; note = 2'-O-methyl-adenosine
  modified_base 12: mod_base = um
  modified_base 13: mod_base = cm
  modified_base 14: mod_base = OTHER; note = 2'-Fluoro-uridine
  modified_base 15: mod_base = gm
  modified_base 16: mod_base = OTHER; note = 2'-Fluoro-adenosine
  modified_base 17: mod_base = um
  modified_base 18: mod_base = OTHER; note = 2'-Fluoro-guanosine
  modified_base 19: mod_base = OTHER; note = 2'-O-methyl-adenosine
  modified_base 20: mod_base = cm
  modified_base 21: mod_base = OTHER; note = 2'-O-methyl-adenosine
  misc_feature 21^22: note = Phosphorothioate bond
  modified_base 22: mod_base = um
  misc_feature 22^23: note = Phosphorothioate bond
  modified_base 23: mod_base = um
gtggggaagtatctgatgacatt

SEQ ID NO: 1102 - RNA, 23 nt, synthetic construct
  source 1..23: mol_type = other RNA
  modified_base 1: mod_base = gm
  misc_feature 1^2: note = Phosphorothioate bond
  modified_base 2: mod_base = OTHER; note = 2'-Fluoro-guanosine
  misc_feature 2^3: note = Phosphorothioate bond
  modified_base 3: mod_base = gm
  modified_base 4: mod_base = gm
  modified_base 5: mod_base = OTHER; note = 2'-O-methyl-adenosine
  modified_base 6: mod_base = OTHER; note = 2'-Fluoro-adenosine
  modified_base 7: mod_base = gm
  modified_base 8: mod_base = um
  modified_base 9: mod_base = OTHER; note = 2'-O-methyl-adenosine
  modified_base 10: mod_base = um
  modified_base 11: mod_base = cm
  modified_base 12: mod_base = um
  modified_base 13: mod_base = gm
  modified_base 14: mod_base = OTHER; note = 2'-Fluoro-adenosine
  modified_base 15: mod_base = um
  modified_base 16: mod_base = OTHER; note = 2'-Fluoro-guanosine
  modified_base 17: mod_base = OTHER; note = 2'-O-methyl-adenosine
  modified_base 18: mod_base = OTHER; note = 2'-Fluoro-cytidine
  modified_base 19: mod_base = OTHER; note = 2'-O-methyl-adenosine
  modified_base 20: mod_base = um
  modified_base 21: mod_base = um
  misc_feature 21^22: note = Phosphorothioate bond
  modified_base 22: mod_base = gm
  misc_feature 22^23: note = Phosphorothioate bond
  modified_base 23: mod_base = gm
ggggaagtatctgatgacattgg

SEQ ID NO: 1103 - RNA, 23 nt, synthetic construct
  source 1..23: mol_type = other RNA
  modified_base 1: mod_base = um
  misc_feature 1^2: note = Phosphorothioate bond
  modified_base 2: mod_base = OTHER; note = 2'-Fluoro-uridine
  misc_feature 2^3: note = Phosphorothioate bond
  modified_base 3: mod_base = OTHER; note = 2'-O-methyl-adenosine
  modified_base 4: mod_base = OTHER; note = 2'-O-methyl-adenosine
  modified_base 5: mod_base = gm
  modified_base 6: mod_base = OTHER; note = 2'-Fluoro-adenosine
  modified_base 7: mod_base = gm
  modified_base 8: mod_base = cm
  modified_base 9: mod_base = cm
  modified_base 10: mod_base = um
  modified_base 11: mod_base = gm
  modified_base 12: mod_base = gm
  modified_base 13: mod_base = gm
  modified_base 14: mod_base = OTHER; note = 2'-Fluoro-uridine
  modified_base 15: mod_base = gm
  modified_base 16: mod_base = OTHER; note = 2'-Fluoro-guanosine
  modified_base 17: mod_base = gm
  modified_base 18: mod_base = OTHER; note = 2'-Fluoro-guanosine
  modified_base 19: mod_base = OTHER; note = 2'-O-methyl-adenosine
  modified_base 20: mod_base = OTHER; note = 2'-O-methyl-adenosine
  modified_base 21: mod_base = gm
  misc_feature 21^22: note = Phosphorothioate bond
  modified_base 22: mod_base = um
  misc_feature 22^23: note = Phosphorothioate bond
  modified_base 23: mod_base = OTHER; note = 2'-O-methyl-adenosine
ttaagagcctgggtggggaagta

SEQ ID NO: 1104 - RNA, 23 nt, synthetic construct
  source 1..23: mol_type = other RNA
  modified_base 1: mod_base = cm
  misc_feature 1^2: note = Phosphorothioate bond
  modified_base 2: mod_base = OTHER; note = 2'-Fluoro-cytidine
  misc_feature 2^3: note = Phosphorothioate bond
  modified_base 3: mod_base = gm
  modified_base 4: mod_base = OTHER; note = 2'-O-methyl-adenosine
  modified_base 5: mod_base = OTHER; note = 2'-O-methyl-adenosine
  modified_base 6: mod_base = OTHER; note = 2'-Fluoro-guanosine
  modified_base 7: mod_base = um
  modified_base 8: mod_base = OTHER; note = 2'-O-methyl-adenosine
  modified_base 9: mod_base = gm
  modified_base 10: mod_base = gm
  modified_base 11: mod_base = cm
  modified_base 12: mod_base = gm
  modified_base 13: mod_base = gm
  modified_base 14: mod_base = OTHER; note = 2'-Fluoro-cytidine
  modified_base 15: mod_base = um
  modified_base 16: mod_base = OTHER; note = 2'-Fluoro-cytidine
  modified_base 17: mod_base = gm
  modified_base 18: mod_base = OTHER; note = 2'-Fluoro-guanosine
  modified_base 19: mod_base = um
  modified_base 20: mod_base = OTHER; note = 2'-O-methyl-adenosine
  modified_base 21: mod_base = gm
  misc_feature 21^22: note = Phosphorothioate bond
  modified_base 22: mod_base = OTHER; note = 2'-O-methyl-adenosine
  misc_feature 22^23: note = Phosphorothioate bond
  modified_base 23: mod_base = um
ccgaagtaggcggctcggtagat

SEQ ID NO: 1105 - RNA, 21 nt, synthetic construct
  source 1..21: mol_type = other RNA
  modified_base <1: mod_base = OTHER; note = two inverted abasic nucleosides
  modified_base 1: mod_base = um
  misc_feature 1^2: note = Phosphorothioate bond
  modified_base 2: mod_base = OTHER; note = 2'-O-methyl-adenosine
  misc_feature 2^3: note = Phosphorothioate bond
  modified_base 3: mod_base = um
  modified_base 4: mod_base = um
  modified_base 5: mod_base = um
  modified_base 6: mod_base = OTHER; note = 2'-O-methyl-adenosine
  modified_base 7: mod_base = cm
  modified_base 8: mod_base = um
  modified_base 9: mod_base = OTHER; note = 2'-Fluoro-guanosine
  modified_base 10: mod_base = OTHER; note = 2'-Fluoro-guanosine
  modified_base 11: mod_base = OTHER; note = 2'-Fluoro-uridine
  modified_base 12: mod_base = um
  modified_base 13: mod_base = gm
  modified_base 14: mod_base = OTHER; note = 2'-O-methyl-adenosine
  modified_base 15: mod_base = OTHER; note = 2'-O-methyl-adenosine
  modified_base 16: mod_base = OTHER; note = 2'-O-methyl-adenosine
  modified_base 17: mod_base = OTHER; note = 2'-O-methyl-adenosine
  modified_base 18: mod_base = um
  modified_base 19: mod_base = gm
  modified_base 20: mod_base = gm
  modified_base 21: mod_base = gm
tatttactggttgaaaatggg

SEQ ID NO: 1106 - RNA, 21 nt, synthetic construct
  source 1..21: mol_type = other RNA
  modified_base <1: mod_base = OTHER; note = two inverted abasic nucleosides
  modified_base 1: mod_base = cm
  misc_feature 1^2: note = Phosphorothioate bond
  modified_base 2: mod_base = OTHER; note = 2'-O-methyl-adenosine
  misc_feature 2^3: note = Phosphorothioate bond
  modified_base 3: mod_base = OTHER; note = 2'-O-methyl-adenosine
  modified_base 4: mod_base = OTHER; note = 2'-O-methyl-adenosine
  modified_base 5: mod_base = gm
  modified_base 6: mod_base = gm
  modified_base 7: mod_base = cm
  modified_base 8: mod_base = OTHER; note = 2'-O-methyl-adenosine
  modified_base 9: mod_base = OTHER; note = 2'-Fluoro-uridine
  modified_base 10: mod_base = OTHER; note = 2'-Fluoro-uridine
  modified_base 11: mod_base = OTHER; note = 2'-Fluoro-adenosine
  modified_base 12: mod_base = um
  modified_base 13: mod_base = OTHER; note = 2'-O-methyl-adenosine
  modified_base 14: mod_base = gm
  modified_base 15: mod_base = OTHER; note = 2'-O-methyl-adenosine
  modified_base 16: mod_base = cm
  modified_base 17: mod_base = um
  modified_base 18: mod_base = gm
  modified_base 19: mod_base = cm
  modified_base 20: mod_base = gm
  modified_base 21: mod_base = um
caaaggcattatagactgcgt

SEQ ID NO: 1107 - RNA, 21 nt, synthetic construct
  source 1..21: mol_type = other RNA
  modified_base <1: mod_base = OTHER; note = two inverted abasic nucleosides
  modified_base 1: mod_base = um
  misc_feature 1^2: note = Phosphorothioate bond
  modified_base 2: mod_base = gm
  misc_feature 2^3: note = Phosphorothioate bond
  modified_base 3: mod_base = OTHER; note = 2'-O-methyl-adenosine
  modified_base 4: mod_base = um
  modified_base 5: mod_base = gm
  modified_base 6: mod_base = OTHER; note = 2'-O-methyl-adenosine
  modified_base 7: mod_base = OTHER; note = 2'-O-methyl-adenosine
  modified_base 8: mod_base = OTHER; note = 2'-O-methyl-adenosine
  modified_base 9: mod_base = OTHER; note = 2'-Fluoro-uridine
  modified_base 10: mod_base = OTHER; note = 2'-Fluoro-cytidine
  modified_base 11: mod_base = OTHER; note = 2'-Fluoro-adenosine
  modified_base 12: mod_base = OTHER; note = 2'-O-methyl-adenosine
  modified_base 13: mod_base = gm
  modified_base 14: mod_base = OTHER; note = 2'-O-methyl-adenosine
  modified_base 15: mod_base = OTHER; note = 2'-O-methyl-adenosine
  modified_base 16: mod_base = gm
  modified_base 17: mod_base = um
  modified_base 18: mod_base = OTHER; note = 2'-O-methyl-adenosine
  modified_base 19: mod_base = cm
  modified_base 20: mod_base = OTHER; note = 2'-O-methyl-adenosine
  modified_base 21: mod_base = cm
tgatgaaatcaagaagtacac

SEQ ID NO: 1108 - RNA, 21 nt, synthetic construct
  source 1..21: mol_type = other RNA
  modified_base <1: mod_base = OTHER; note = two inverted abasic nucleosides
  modified_base 1: mod_base = gm
  misc_feature 1^2: note = Phosphorothioate bond
  modified_base 2: mod_base = OTHER; note = 2'-O-methyl-adenosine
  misc_feature 2^3: note = Phosphorothioate bond
  modified_base 3: mod_base = um
  modified_base 4: mod_base = gm
  modified_base 5: mod_base = OTHER; note = 2'-O-methyl-adenosine
  modified_base 6: mod_base = um
  modified_base 7: mod_base = gm
  modified_base 8: mod_base = gm
  modified_base 9: mod_base = OTHER; note = 2'-Fluoro-guanosine
  modified_base 10: mod_base = OTHER; note = 2'-Fluoro-adenosine
  modified_base 11: mod_base = OTHER; note = 2'-Fluoro-cytidine
  modified_base 12: mod_base = um
  modified_base 13: mod_base = cm
  modified_base 14: mod_base = OTHER; note = 2'-O-methyl-adenosine
  modified_base 15: mod_base = OTHER; note = 2'-O-methyl-adenosine
  modified_base 16: mod_base = um
  modified_base 17: mod_base = um
  modified_base 18: mod_base = gm
  modified_base 19: mod_base = um
  modified_base 20: mod_base = OTHER; note = 2'-O-methyl-adenosine
  modified_base 21: mod_base = um
gatgatgggactcaattgtat

SEQ ID NO: 1109 - RNA, 21 nt, synthetic construct
  source 1..21: mol_type = other RNA
  modified_base <1: mod_base = OTHER; note = two inverted abasic nucleosides
  modified_base 1: mod_base = gm
  misc_feature 1^2: note = Phosphorothioate bond
  modified_base 2: mod_base = cm
  misc_feature 2^3: note = Phosphorothioate bond
  modified_base 3: mod_base = OTHER; note = 2'-O-methyl-adenosine
  modified_base 4: mod_base = um
  modified_base 5: mod_base = um
  modified_base 6: mod_base = OTHER; note = 2'-O-methyl-adenosine
  modified_base 7: mod_base = um
  modified_base 8: mod_base = OTHER; note = 2'-O-methyl-adenosine
  modified_base 9: mod_base = OTHER; note = 2'-Fluoro-guanosine
  modified_base 10: mod_base = OTHER; note = 2'-Fluoro-adenosine
  modified_base 11: mod_base = OTHER; note = 2'-Fluoro-cytidine
  modified_base 12: mod_base = um
  modified_base 13: mod_base = gm
  modified_base 14: mod_base = cm
  modified_base 15: mod_base = gm
  modified_base 16: mod_base = um
  modified_base 17: mod_base = gm
  modified_base 18: mod_base = gm
  modified_base 19: mod_base = um
  modified_base 20: mod_base = cm
  modified_base 21: mod_base = cm
gcattatagactgcgtggtcc

SEQ ID NO: 1110 - RNA, 21 nt, synthetic construct
  source 1..21: mol_type = other RNA
  modified_base <1: mod_base = OTHER; note = two inverted abasic nucleosides
  modified_base 1: mod_base = gm
  misc_feature 1^2: note = Phosphorothioate bond
  modified_base 2: mod_base = um
  misc_feature 2^3: note = Phosphorothioate bond
  modified_base 3: mod_base = cm
  modified_base 4: mod_base = OTHER; note = 2'-O-methyl-adenosine
  modified_base 5: mod_base = cm
  modified_base 6: mod_base = um
  modified_base 7: mod_base = cm
  modified_base 8: mod_base = cm
  modified_base 9: mod_base = OTHER; note = 2'-Fluoro-uridine
  modified_base 10: mod_base = OTHER; note = 2'-Fluoro-guanosine
  modified_base 11: mod_base = OTHER; note = 2'-Fluoro-adenosine
  modified_base 12: mod_base = um
  modified_base 13: mod_base = OTHER; note = 2'-O-methyl-adenosine
  modified_base 14: mod_base = OTHER; note = 2'-O-methyl-adenosine
  modified_base 15: mod_base = OTHER; note = 2'-O-methyl-adenosine
  modified_base 16: mod_base = um
  modified_base 17: mod_base = OTHER; note = 2'-O-methyl-adenosine
  modified_base 18: mod_base = OTHER; note = 2'-O-methyl-adenosine
  modified_base 19: mod_base = cm
  modified_base 20: mod_base = OTHER; note = 2'-O-methyl-adenosine
  modified_base 21: mod_base = OTHER; note = 2'-O-methyl-adenosine
gtcactcctgataaataacaa

SEQ ID NO: 1111 - RNA, 21 nt, synthetic construct
  source 1..21: mol_type = other RNA
  modified_base <1: mod_base = OTHER; note = two inverted abasic nucleosides
  modified_base 1: mod_base = OTHER; note = 2'-O-methyl-adenosine
  misc_feature 1^2: note = Phosphorothioate bond
  modified_base 2: mod_base = um
  misc_feature 2^3: note = Phosphorothioate bond
  modified_base 3: mod_base = OTHER; note = 2'-O-methyl-adenosine
  modified_base 4: mod_base = cm
  modified_base 5: mod_base = OTHER; note = 2'-O-methyl-adenosine
  modified_base 6: mod_base = OTHER; note = 2'-O-methyl-adenosine
  modified_base 7: mod_base = OTHER; note = 2'-O-methyl-adenosine
  modified_base 8: mod_base = gm
  modified_base 9: mod_base = OTHER; note = 2'-Fluoro-guanosine
  modified_base 10: mod_base = OTHER; note = 2'-Fluoro-cytidine
  modified_base 11: mod_base = OTHER; note = 2'-Fluoro-adenosine
  modified_base 12: mod_base = um
  modified_base 13: mod_base = um
  modified_base 14: mod_base = OTHER; note = 2'-O-methyl-adenosine
  modified_base 15: mod_base = um
  modified_base 16: mod_base = OTHER; note = 2'-O-methyl-adenosine
  modified_base 17: mod_base = gm
  modified_base 18: mod_base = OTHER; note = 2'-O-methyl-adenosine
  modified_base 19: mod_base = cm
  modified_base 20: mod_base = um
  modified_base 21: mod_base = gm
atacaaaggcattatagactg

SEQ ID NO: 1112 - RNA, 21 nt, synthetic construct
  source 1..21: mol_type = other RNA
  modified_base <1: mod_base = OTHER; note = two inverted abasic nucleosides
  modified_base 1: mod_base = gm
  misc_feature 1^2: note = Phosphorothioate bond
  modified_base 2: mod_base = cm
  misc_feature 2^3: note = Phosphorothioate bond
  modified_base 3: mod_base = cm
  modified_base 4: mod_base = gm
  modified_base 5: mod_base = cm
  modified_base 6: mod_base = cm
  modified_base 7: mod_base = um
  modified_base 8: mod_base = OTHER; note = 2'-O-methyl-adenosine
  modified_base 9: mod_base = OTHER; note = 2'-Fluoro-cytidine
  modified_base 10: mod_base = OTHER; note = 2'-Fluoro-uridine
  modified_base 11: mod_base = OTHER; note = 2'-Fluoro-uridine
  modified_base 12: mod_base = cm
  modified_base 13: mod_base = gm
  modified_base 14: mod_base = gm
  modified_base 15: mod_base = um
  modified_base 16: mod_base = OTHER; note = 2'-O-methyl-adenosine
  modified_base 17: mod_base = um
  modified_base 18: mod_base = cm
  modified_base 19: mod_base = um
  modified_base 20: mod_base = OTHER; note = 2'-O-methyl-adenosine
  modified_base 21: mod_base = um
gccgcctacttcggtatctat

SEQ ID NO: 1113 - RNA, 21 nt, synthetic construct
  source 1..21: mol_type = other RNA
  modified_base <1: mod_base = OTHER; note = two inverted abasic nucleosides
  modified_base 1: mod_base = OTHER; note = 2'-O-methyl-adenosine
  misc_feature 1^2: note = Phosphorothioate bond
  modified_base 2: mod_base = gm
  misc_feature 2^3: note = Phosphorothioate bond
  modified_base 3: mod_base = cm
  modified_base 4: mod_base = cm
  modified_base 5: mod_base = gm
  modified_base 6: mod_base = cm
  modified_base 7: mod_base = cm
  modified_base 8: mod_base = um
  modified_base 9: mod_base = OTHER; note = 2'-Fluoro-adenosine
  modified_base 10: mod_base = OTHER; note = 2'-Fluoro-cytidine
  modified_base 11: mod_base = OTHER; note = 2'-Fluoro-uridine
  modified_base 12: mod_base = um
  modified_base 13: mod_base = cm
  modified_base 14: mod_base = gm
  modified_base 15: mod_base = gm
  modified_base 16: mod_base = um
  modified_base 17: mod_base = OTHER; note = 2'-O-methyl-adenosine
  modified_base 18: mod_base = um
  modified_base 19: mod_base = cm
  modified_base 20: mod_base = um
  modified_base 21: mod_base = OTHER; note = 2'-O-methyl-adenosine
agccgcctacttcggtatcta

SEQ ID NO: 1114 - RNA, 21 nt, synthetic construct
  source 1..21: mol_type = other RNA
  modified_base <1: mod_base = OTHER; note = two inverted abasic nucleosides
  modified_base 1: mod_base = OTHER; note = 2'-O-methyl-adenosine
  misc_feature 1^2: note = Phosphorothioate bond
  modified_base 2: mod_base = gm
  misc_feature 2^3: note = Phosphorothioate bond
  modified_base 3: mod_base = OTHER; note = 2'-O-methyl-adenosine
  modified_base 4: mod_base = cm
  modified_base 5: mod_base = um
  modified_base 6: mod_base = gm
  modified_base 7: mod_base = cm
  modified_base 8: mod_base = gm
  modified_base 9: mod_base = OTHER; note = 2'-Fluoro-uridine
  modified_base 10: mod_base = OTHER; note = 2'-Fluoro-guanosine
  modified_base 11: mod_base = OTHER; note = 2'-Fluoro-guanosine
  modified_base 12: mod_base = um
  modified_base 13: mod_base = cm
  modified_base 14: mod_base = cm
  modified_base 15: mod_base = gm
  modified_base 16: mod_base = um
  modified_base 17: mod_base = OTHER; note = 2'-O-methyl-adenosine
  modified_base 18: mod_base = um
  modified_base 19: mod_base = um
  modified_base 20: mod_base = cm
  modified_base 21: mod_base = cm
agactgcgtggtccgtattcc

SEQ ID NO: 1115 - RNA, 21 nt, synthetic construct
  source 1..21: mol_type = other RNA
  modified_base <1: mod_base = OTHER; note = two inverted abasic nucleosides
  modified_base 1: mod_base = cm
  misc_feature 1^2: note = Phosphorothioate bond
  modified_base 2: mod_base = OTHER; note = 2'-O-methyl-adenosine
  misc_feature 2^3: note = Phosphorothioate bond
  modified_base 3: mod_base = cm
  modified_base 4: mod_base = um
  modified_base 5: mod_base = cm
  modified_base 6: mod_base = OTHER; note = 2'-O-methyl-adenosine
  modified_base 7: mod_base = cm
  modified_base 8: mod_base = OTHER; note = 2'-O-methyl-adenosine
  modified_base 9: mod_base = OTHER; note = 2'-Fluoro-uridine
  modified_base 10: mod_base = OTHER; note = 2'-Fluoro-cytidine
  modified_base 11: mod_base = OTHER; note = 2'-Fluoro-guanosine
  modified_base 12: mod_base = um
  modified_base 13: mod_base = cm
  modified_base 14: mod_base = OTHER; note = 2'-O-methyl-adenosine
  modified_base 15: mod_base = um
  modified_base 16: mod_base = cm
  modified_base 17: mod_base = OTHER; note = 2'-O-methyl-adenosine
  modified_base 18: mod_base = gm
  modified_base 19: mod_base = cm
  modified_base 20: mod_base = um
  modified_base 21: mod_base = gm
cactcacatcgtcatcagctg

SEQ ID NO: 1116 - RNA, 21 nt, synthetic construct
  source 1..21: mol_type = other RNA
  modified_base <1: mod_base = OTHER; note = two inverted abasic nucleosides
  modified_base 1: mod_base = OTHER; note = 2'-O-methyl-adenosine
  misc_feature 1^2: note = Phosphorothioate bond
  modified_base 2: mod_base = cm
  misc_feature 2^3: note = Phosphorothioate bond
  modified_base 3: mod_base = um
  modified_base 4: mod_base = um
  modified_base 5: mod_base = cm
  modified_base 6: mod_base = gm
  modified_base 7: mod_base = cm
  modified_base 8: mod_base = cm
  modified_base 9: mod_base = OTHER; note = 2'-Fluoro-uridine
  modified_base 10: mod_base = OTHER; note = 2'-Fluoro-uridine
  modified_base 11: mod_base = OTHER; note = 2'-Fluoro-cytidine
  modified_base 12: mod_base = OTHER; note = 2'-O-methyl-adenosine
  modified_base 13: mod_base = OTHER; note = 2'-O-methyl-adenosine
  modified_base 14: mod_base = OTHER; note = 2'-O-methyl-adenosine
  modified_base 15: mod_base = gm
  modified_base 16: mod_base = OTHER; note = 2'-O-methyl-adenosine
  modified_base 17: mod_base = um
  modified_base 18: mod_base = OTHER; note = 2'-O-methyl-adenosine
  modified_base 19: mod_base = OTHER; note = 2'-O-methyl-adenosine
  modified_base 20: mod_base = OTHER; note = 2'-O-methyl-adenosine
  modified_base 21: mod_base = um
acttcgccttcaaagataaat

SEQ ID NO: 1117 - RNA, 21 nt, synthetic construct
  source 1..21: mol_type = other RNA
  modified_base <1: mod_base = OTHER; note = two inverted abasic nucleosides
  modified_base 1: mod_base = cm
  misc_feature 1^2: note = Phosphorothioate bond
  modified_base 2: mod_base = um
  misc_feature 2^3: note = Phosphorothioate bond
  modified_base 3: mod_base = OTHER; note = 2'-O-methyl-adenosine
  modified_base 4: mod_base = cm
  modified_base 5: mod_base = um
  modified_base 6: mod_base = um
  modified_base 7: mod_base = cm
  modified_base 8: mod_base = gm
  modified_base 9: mod_base = OTHER; note = 2'-Fluoro-guanosine
  modified_base 10: mod_base = OTHER; note = 2'-Fluoro-uridine
  modified_base 11: mod_base = OTHER; note = 2'-Fluoro-adenosine
  modified_base 12: mod_base = um
  modified_base 13: mod_base = cm
  modified_base 14: mod_base = um
  modified_base 15: mod_base = OTHER; note = 2'-O-methyl-adenosine
  modified_base 16: mod_base = um
  modified_base 17: mod_base = gm
  modified_base 18: mod_base = OTHER; note = 2'-O-methyl-adenosine
  modified_base 19: mod_base = cm
  modified_base 20: mod_base = OTHER; note = 2'-O-methyl-adenosine
  modified_base 21: mod_base = cm
ctacttcggtatctatgacac

SEQ ID NO: 1118 - RNA, 21 nt, synthetic construct
  source 1..21: mol_type = other RNA
  modified_base <1: mod_base = OTHER; note = two inverted abasic nucleosides
  modified_base 1: mod_base = um
  misc_feature 1^2: note = Phosphorothioate bond
  modified_base 2: mod_base = um
  misc_feature 2^3: note = Phosphorothioate bond
  modified_base 3: mod_base = um
  modified_base 4: mod_base = OTHER; note = 2'-O-methyl-adenosine
  modified_base 5: mod_base = cm
  modified_base 6: mod_base = um
  modified_base 7: mod_base = gm
  modified_base 8: mod_base = gm
  modified_base 9: mod_base = OTHER; note = 2'-Fluoro-uridine
  modified_base 10: mod_base = OTHER; note = 2'-Fluoro-uridine
  modified_base 11: mod_base = OTHER; note = 2'-Fluoro-guanosine
  modified_base 12: mod_base = OTHER; note = 2'-O-methyl-adenosine
  modified_base 13: mod_base = OTHER; note = 2'-O-methyl-adenosine
  modified_base 14: mod_base = OTHER; note = 2'-O-methyl-adenosine
  modified_base 15: mod_base = OTHER; note = 2'-O-methyl-adenosine
  modified_base 16: mod_base = um
  modified_base 17: mod_base = gm
  modified_base 18: mod_base = gm
  modified_base 19: mod_base = gm
  modified_base 20: mod_base = OTHER; note = 2'-O-methyl-adenosine
  modified_base 21: mod_base = OTHER; note = 2'-O-methyl-adenosine
tttactggttgaaaatgggaa

SEQ ID NO: 1119 - RNA, 21 nt, synthetic construct
  source 1..21: mol_type = other RNA
  modified_base <1: mod_base = OTHER; note = two inverted abasic nucleosides
  modified_base 1: mod_base = um
  misc_feature 1^2: note = Phosphorothioate bond
  modified_base 2: mod_base = gm
  misc_feature 2^3: note = Phosphorothioate bond
  modified_base 3: mod_base = cm
  modified_base 4: mod_base = cm
  modified_base 5: mod_base = cm
  modified_base 6: mod_base = gm
  modified_base 7: mod_base = um
  modified_base 8: mod_base = OTHER; note = 2'-O-methyl-adenosine
  modified_base 9: mod_base = OTHER; note = 2'-Fluoro-cytidine
  modified_base 10: mod_base = OTHER; note = 2'-Fluoro-cytidine
  modified_base 11: mod_base = OTHER; note = 2'-Fluoro-cytidine
  modified_base 12: mod_base = gm
  modified_base 13: mod_base = um
  modified_base 14: mod_base = cm
  modified_base 15: mod_base = um
  modified_base 16: mod_base = OTHER; note = 2'-O-methyl-adenosine
  modified_base 17: mod_base = gm
  modified_base 18: mod_base = cm
  modified_base 19: mod_base = OTHER; note = 2'-O-methyl-adenosine
  modified_base 20: mod_base = gm
  modified_base 21: mod_base = cm
tgcccgtacccgtctagcagc

SEQ ID NO: 1120 - RNA, 21 nt, synthetic construct
  source 1..21: mol_type = other RNA
  modified_base <1: mod_base = OTHER; note = two inverted abasic nucleosides
  modified_base 1: mod_base = OTHER; note = 2'-O-methyl-adenosine
  misc_feature 1^2: note = Phosphorothioate bond
  modified_base 2: mod_base = gm
  misc_feature 2^3: note = Phosphorothioate bond
  modified_base 3: mod_base = um
  modified_base 4: mod_base = cm
  modified_base 5: mod_base = OTHER; note = 2'-O-methyl-adenosine
  modified_base 6: mod_base = gm
  modified_base 7: mod_base = gm
  modified_base 8: mod_base = gm
  modified_base 9: mod_base = OTHER; note = 2'-Fluoro-cytidine
  modified_base 10: mod_base = OTHER; note = 2'-Fluoro-guanosine
  modified_base 11: mod_base = OTHER; note = 2'-Fluoro-cytidine
  modified_base 12: mod_base = OTHER; note = 2'-O-methyl-adenosine
  modified_base 13: mod_base = OTHER; note = 2'-O-methyl-adenosine
  modified_base 14: mod_base = OTHER; note = 2'-O-methyl-adenosine
  modified_base 15: mod_base = gm
  modified_base 16: mod_base = gm
  modified_base 17: mod_base = OTHER; note = 2'-O-methyl-adenosine
  modified_base 18: mod_base = OTHER; note = 2'-O-methyl-adenosine
  modified_base 19: mod_base = cm
  modified_base 20: mod_base = um
  modified_base 21: mod_base = gm
agtcagggcgcaaaggaactg

SEQ ID NO: 1121 - RNA, 21 nt, synthetic construct
  source 1..21: mol_type = other RNA
  modified_base <1: mod_base = OTHER; note = two inverted abasic nucleosides
  modified_base 1: mod_base = um
  misc_feature 1^2: note = Phosphorothioate bond
  modified_base 2: mod_base = um
  misc_feature 2^3: note = Phosphorothioate bond
  modified_base 3: mod_base = OTHER; note = 2'-O-methyl-adenosine
  modified_base 4: mod_base = cm
  modified_base 5: mod_base = um
  modified_base 6: mod_base = gm
  modified_base 7: mod_base = gm
  modified_base 8: mod_base = um
  modified_base 9: mod_base = OTHER; note = 2'-Fluoro-uridine
  modified_base 10: mod_base = OTHER; note = 2'-Fluoro-guanosine
  modified_base 11: mod_base = OTHER; note = 2'-Fluoro-adenosine
  modified_base 12: mod_base = OTHER; note = 2'-O-methyl-adenosine
  modified_base 13: mod_base = OTHER; note = 2'-O-methyl-adenosine
  modified_base 14: mod_base = OTHER; note = 2'-O-methyl-adenosine
  modified_base 15: mod_base = um
  modified_base 16: mod_base = gm
  modified_base 17: mod_base = gm
  modified_base 18: mod_base = gm
  modified_base 19: mod_base = OTHER; note = 2'-O-methyl-adenosine
  modified_base 20: mod_base = OTHER; note = 2'-O-methyl-adenosine
  modified_base 21: mod_base = gm
ttactggttgaaaatgggaag

SEQ ID NO: 1122 - RNA, 21 nt, synthetic construct
  source 1..21: mol_type = other RNA
  modified_base <1: mod_base = OTHER; note = two inverted abasic nucleosides
  modified_base 1: mod_base = gm
  misc_feature 1^2: note = Phosphorothioate bond
  modified_base 2: mod_base = OTHER; note = 2'-O-methyl-adenosine
  misc_feature 2^3: note = Phosphorothioate bond
  modified_base 3: mod_base = gm
  modified_base 4: mod_base = cm
  modified_base 5: mod_base = cm
  modified_base 6: mod_base = gm
  modified_base 7: mod_base = cm
  modified_base 8: mod_base = cm
  modified_base 9: mod_base = OTHER; note = 2'-Fluoro-uridine
  modified_base 10: mod_base = OTHER; note = 2'-Fluoro-adenosine
  modified_base 11: mod_base = OTHER; note = 2'-Fluoro-cytidine
  modified_base 12: mod_base = um
  modified_base 13: mod_base = um
  modified_base 14: mod_base = cm
  modified_base 15: mod_base = gm
  modified_base 16: mod_base = gm
  modified_base 17: mod_base = um
  modified_base 18: mod_base = OTHER; note = 2'-O-methyl-adenosine
  modified_base 19: mod_base = um
  modified_base 20: mod_base = cm
  modified_base 21: mod_base = um
gagccgcctacttcggtatct

SEQ ID NO: 1123 - RNA, 21 nt, synthetic construct
  source 1..21: mol_type = other RNA
  modified_base <1: mod_base = OTHER; note = two inverted abasic nucleosides
  modified_base 1: mod_base = cm
  misc_feature 1^2: note = Phosphorothioate bond
  modified_base 2: mod_base = cm
  misc_feature 2^3: note = Phosphorothioate bond
  modified_base 3: mod_base = um
  modified_base 4: mod_base = cm
  modified_base 5: mod_base = gm
  modified_base 6: mod_base = gm
  modified_base 7: mod_base = um
  modified_base 8: mod_base = gm
  modified_base 9: mod_base = OTHER; note = 2'-Fluoro-adenosine
  modified_base 10: mod_base = OTHER; note = 2'-Fluoro-cytidine
  modified_base 11: mod_base = OTHER; note = 2'-Fluoro-uridine
  modified_base 12: mod_base = gm
  modified_base 13: mod_base = cm
  modified_base 14: mod_base = cm
  modified_base 15: mod_base = um
  modified_base 16: mod_base = gm
  modified_base 17: mod_base = gm
  modified_base 18: mod_base = um
  modified_base 19: mod_base = um
  modified_base 20: mod_base = OTHER; note = 2'-O-methyl-adenosine
  modified_base 21: mod_base = OTHER; note = 2'-O-methyl-adenosine
cctcggtgactgcctggttaa

SEQ ID NO: 1124 - RNA, 21 nt, synthetic construct
  source 1..21: mol_type = other RNA
  modified_base <1: mod_base = OTHER; note = two inverted abasic nucleosides
  modified_base 1: mod_base = cm
  misc_feature 1^2: note = Phosphorothioate bond
  modified_base 2: mod_base = OTHER; note = 2'-O-methyl-adenosine
  misc_feature 2^3: note = Phosphorothioate bond
  modified_base 3: mod_base = um
  modified_base 4: mod_base = cm
  modified_base 5: mod_base = gm
  modified_base 6: mod_base = um
  modified_base 7: mod_base = cm
  modified_base 8: mod_base = OTHER; note = 2'-O-methyl-adenosine
  modified_base 9: mod_base = OTHER; note = 2'-Fluoro-uridine
  modified_base 10: mod_base = OTHER; note = 2'-Fluoro-cytidine
  modified_base 11: mod_base = OTHER; note = 2'-Fluoro-adenosine
  modified_base 12: mod_base = gm
  modified_base 13: mod_base = cm
  modified_base 14: mod_base = um
  modified_base 15: mod_base = gm
  modified_base 16: mod_base = gm
  modified_base 17: mod_base = OTHER; note = 2'-O-methyl-adenosine
  modified_base 18: mod_base = um
  modified_base 19: mod_base = gm
  modified_base 20: mod_base = OTHER; note = 2'-O-methyl-adenosine
  modified_base 21: mod_base = um
catcgtcatcagctggatgat

SEQ ID NO: 1125 - RNA, 21 nt, synthetic construct
  source 1..21: mol_type = other RNA
  modified_base <1: mod_base = OTHER; note = two inverted abasic nucleosides
  modified_base 1: mod_base = um
  misc_feature 1^2: note = Phosphorothioate bond
  modified_base 2: mod_base = um
  misc_feature 2^3: note = Phosphorothioate bond
  modified_base 3: mod_base = um
  modified_base 4: mod_base = cm
  modified_base 5: mod_base = OTHER; note = 2'-O-methyl-adenosine
  modified_base 6: mod_base = gm
  modified_base 7: mod_base = um
  modified_base 8: mod_base = cm
  modified_base 9: mod_base = OTHER; note = 2'-Fluoro-adenosine
  modified_base 10: mod_base = OTHER; note = 2'-Fluoro-cytidine
  modified_base 11: mod_base = OTHER; note = 2'-Fluoro-uridine
  modified_base 12: mod_base = cm
  modified_base 13: mod_base = cm
  modified_base 14: mod_base = um
  modified_base 15: mod_base = gm
  modified_base 16: mod_base = OTHER; note = 2'-O-methyl-adenosine
  modified_base 17: mod_base = um
  modified_base 18: mod_base = OTHER; note = 2'-O-methyl-adenosine
  modified_base 19: mod_base = OTHER; note = 2'-O-methyl-adenosine
  modified_base 20: mod_base = OTHER; note = 2'-O-methyl-adenosine
  modified_base 21: mod_base = um
tttcagtcactcctgataaat

SEQ ID NO: 1126 - RNA, 21 nt, synthetic construct
  source 1..21: mol_type = other RNA
  modified_base <1: mod_base = OTHER; note = two inverted abasic nucleosides
  modified_base 1: mod_base = um
  misc_feature 1^2: note = Phosphorothioate bond
  modified_base 2: mod_base = gm
  misc_feature 2^3: note = Phosphorothioate bond
  modified_base 3: mod_base = gm
  modified_base 4: mod_base = OTHER; note = 2'-O-methyl-adenosine
  modified_base 5: mod_base = um
  modified_base 6: mod_base = gm
  modified_base 7: mod_base = OTHER; note = 2'-O-methyl-adenosine
  modified_base 8: mod_base = um
  modified_base 9: mod_base = OTHER; note = 2'-Fluoro-cytidine
  modified_base 10: mod_base = OTHER; note = 2'-Fluoro-guanosine
  modified_base 11: mod_base = OTHER; note = 2'-Fluoro-cytidine
  modified_base 12: mod_base = OTHER; note = 2'-O-methyl-adenosine
  modified_base 13: mod_base = cm
  modified_base 14: mod_base = OTHER; note = 2'-O-methyl-adenosine
  modified_base 15: mod_base = gm
  modified_base 16: mod_base = OTHER; note = 2'-O-methyl-adenosine
  modified_base 17: mod_base = cm
  modified_base 18: mod_base = um
  modified_base 19: mod_base = gm
  modified_base 20: mod_base = um
  modified_base 21: mod_base = cm
tggatgatcgcacagactgtc

SEQ ID NO: 1127 - RNA, 21 nt, synthetic construct
  source 1..21: mol_type = other RNA
  modified_base <1: mod_base = OTHER; note = two inverted abasic nucleosides
  modified_base 1: mod_base = gm
  misc_feature 1^2: note = Phosphorothioate bond
  modified_base 2: mod_base = cm
  misc_feature 2^3: note = Phosphorothioate bond
  modified_base 3: mod_base = OTHER; note = 2'-O-methyl-adenosine
  modified_base 4: mod_base = OTHER; note = 2'-O-methyl-adenosine
  modified_base 5: mod_base = um
  modified_base 6: mod_base = OTHER; note = 2'-O-methyl-adenosine
  modified_base 7: mod_base = cm
  modified_base 8: mod_base = OTHER; note = 2'-O-methyl-adenosine
  modified_base 9: mod_base = OTHER; note = 2'-Fluoro-adenosine
  modified_base 10: mod_base = OTHER; note = 2'-Fluoro-adenosine
  modified_base 11: mod_base = OTHER; note = 2'-Fluoro-guanosine
  modified_base 12: mod_base = gm
  modified_base 13: mod_base = cm
  modified_base 14: mod_base = OTHER; note = 2'-O-methyl-adenosine
  modified_base 15: mod_base = um
  modified_base 16: mod_base = um
  modified_base 17: mod_base = OTHER; note = 2'-O-methyl-adenosine
  modified_base 18: mod_base = um
  modified_base 19: mod_base = OTHER; note = 2'-O-methyl-adenosine
  modified_base 20: mod_base = gm
  modified_base 21: mod_base = OTHER; note = 2'-O-methyl-adenosine
gcaatacaaaggcattataga

SEQ ID NO: 1128 - RNA, 21 nt, synthetic construct
  source 1..21: mol_type = other RNA
  modified_base <1: mod_base = OTHER; note = two inverted abasic nucleosides
  modified_base 1: mod_base = gm
  misc_feature 1^2: note = Phosphorothioate bond
  modified_base 2: mod_base = cm
  misc_feature 2^3: note = Phosphorothioate bond
  modified_base 3: mod_base = cm
  modified_base 4: mod_base = um
  modified_base 5: mod_base = cm
  modified_base 6: mod_base = gm
  modified_base 7: mod_base = gm
  modified_base 8: mod_base = um
  modified_base 9: mod_base = OTHER; note = 2'-Fluoro-guanosine
  modified_base 10: mod_base = OTHER; note = 2'-Fluoro-adenosine
  modified_base 11: mod_base = OTHER; note = 2'-Fluoro-cytidine
  modified_base 12: mod_base = um
  modified_base 13: mod_base = gm
  modified_base 14: mod_base = cm
  modified_base 15: mod_base = cm
  modified_base 16: mod_base = um
  modified_base 17: mod_base = gm
  modified_base 18: mod_base = gm
  modified_base 19: mod_base = um
  modified_base 20: mod_base = um
  modified_base 21: mod_base = OTHER; note = 2'-O-methyl-adenosine
gcctcggtgactgcctggtta

SEQ ID NO: 1129 - RNA, 21 nt, synthetic construct
  source 1..21: mol_type = other RNA
  modified_base <1: mod_base = OTHER; note = two inverted abasic nucleosides
  modified_base 1: mod_base = cm
  misc_feature 1^2: note = Phosphorothioate bond
  modified_base 2: mod_base = um
  misc_feature 2^3: note = Phosphorothioate bond
  modified_base 3: mod_base = um
  modified_base 4: mod_base = um
  modified_base 5: mod_base = OTHER; note = 2'-O-methyl-adenosine
  modified_base 6: mod_base = OTHER; note = 2'-O-methyl-adenosine
  modified_base 7: mod_base = cm
  modified_base 8: mod_base = gm
  modified_base 9: mod_base = OTHER; note = 2'-Fluoro-uridine
  modified_base 10: mod_base = OTHER; note = 2'-Fluoro-guanosine
  modified_base 11: mod_base = OTHER; note = 2'-Fluoro-uridine
  modified_base 12: mod_base = cm
  modified_base 13: mod_base = um
  modified_base 14: mod_base = gm
  modified_base 15: mod_base = um
  modified_base 16: mod_base = gm
  modified_base 17: mod_base = cm
  modified_base 18: mod_base = OTHER; note = 2'-O-methyl-adenosine
  modified_base 19: mod_base = gm
  modified_base 20: mod_base = gm
  modified_base 21: mod_base = gm
ctttaacgtgtctgtgcaggg

SEQ ID NO: 1130 - RNA, 21 nt, synthetic construct
  source 1..21: mol_type = other RNA
  modified_base <1: mod_base = OTHER; note = two inverted abasic nucleosides
  modified_base 1: mod_base = OTHER; note = 2'-O-methyl-adenosine
  misc_feature 1^2: note = Phosphorothioate bond
  modified_base 2: mod_base = OTHER; note = 2'-O-methyl-adenosine
  misc_feature 2^3: note = Phosphorothioate bond
  modified_base 3: mod_base = OTHER; note = 2'-O-methyl-adenosine
  modified_base 4: mod_base = gm
  modified_base 5: mod_base = gm
  modified_base 6: mod_base = cm
  modified_base 7: mod_base = OTHER; note = 2'-O-methyl-adenosine
  modified_base 8: mod_base = um
  modified_base 9: mod_base = OTHER; note = 2'-Fluoro-uridine
  modified_base 10: mod_base = OTHER; note = 2'-Fluoro-adenosine
  modified_base 11: mod_base = OTHER; note = 2'-Fluoro-uridine
  modified_base 12: mod_base = OTHER; note = 2'-O-methyl-adenosine
  modified_base 13: mod_base = gm
  modified_base 14: mod_base = OTHER; note = 2'-O-methyl-adenosine
  modified_base 15: mod_base = cm
  modified_base 16: mod_base = um
  modified_base 17: mod_base = gm
  modified_base 18: mod_base = cm
  modified_base 19: mod_base = gm
  modified_base 20: mod_base = um
  modified_base 21: mod_base = gm
aaaggcattatagactgcgtg

SEQ ID NO: 1131 - RNA, 21 nt, synthetic construct
  source 1..21: mol_type = other RNA
  modified_base <1: mod_base = OTHER; note = two inverted abasic nucleosides
  modified_base 1: mod_base = gm
  misc_feature 1^2: note = Phosphorothioate bond
  modified_base 2: mod_base = um
  misc_feature 2^3: note = Phosphorothioate bond
  modified_base 3: mod_base = gm
  modified_base 4: mod_base = OTHER; note = 2'-O-methyl-adenosine
  modified_base 5: mod_base = OTHER; note = 2'-O-methyl-adenosine
  modified_base 6: mod_base = cm
  modified_base 7: mod_base = OTHER; note = 2'-O-methyl-adenosine
  modified_base 8: mod_base = gm
  modified_base 9: mod_base = OTHER; note = 2'-Fluoro-guanosine
  modified_base 10: mod_base = OTHER; note = 2'-Fluoro-cytidine
  modified_base 11: mod_base = OTHER; note = 2'-Fluoro-adenosine
  modified_base 12: mod_base = um
  modified_base 13: mod_base = gm
  modified_base 14: mod_base = um
  modified_base 15: mod_base = um
  modified_base 16: mod_base = gm
  modified_base 17: mod_base = um
  modified_base 18: mod_base = OTHER; note = 2'-O-methyl-adenosine
  modified_base 19: mod_base = um
  modified_base 20: mod_base = um
  modified_base 21: mod_base = OTHER; note = 2'-O-methyl-adenosine
gtgaacaggcatgttgtatta

SEQ ID NO: 1132 - RNA, 21 nt, synthetic construct
  source 1..21: mol_type = other RNA
  modified_base <1: mod_base = OTHER; note = two inverted abasic nucleosides
  modified_base 1: mod_base = OTHER; note = 2'-O-methyl-adenosine
  misc_feature 1^2: note = Phosphorothioate bond
  modified_base 2: mod_base = um
  misc_feature 2^3: note = Phosphorothioate bond
  modified_base 3: mod_base = cm
  modified_base 4: mod_base = um
  modified_base 5: mod_base = gm
  modified_base 6: mod_base = OTHER; note = 2'-O-methyl-adenosine
  modified_base 7: mod_base = cm
  modified_base 8: mod_base = cm
  modified_base 9: mod_base = OTHER; note = 2'-Fluoro-adenosine
  modified_base 10: mod_base = OTHER; note = 2'-Fluoro-guanosine
  modified_base 11: mod_base = OTHER; note = 2'-Fluoro-uridine
  modified_base 12: mod_base = um
  modified_base 13: mod_base = um
  modified_base 14: mod_base = um
  modified_base 15: mod_base = cm
  modified_base 16: mod_base = um
  modified_base 17: mod_base = cm
  modified_base 18: mod_base = um
  modified_base 19: mod_base = um
  modified_base 20: mod_base = OTHER; note = 2'-O-methyl-adenosine
  modified_base 21: mod_base = OTHER; note = 2'-O-methyl-adenosine
atctgaccagttttctcttaa

SEQ ID NO: 1133 - RNA, 21 nt, synthetic construct
  source 1..21: mol_type = other RNA
  modified_base <1: mod_base = OTHER; note = two inverted abasic nucleosides
  modified_base 1: mod_base = OTHER; note = 2'-O-methyl-adenosine
  misc_feature 1^2: note = Phosphorothioate bond
  modified_base 2: mod_base = gm
  misc_feature 2^3: note = Phosphorothioate bond
  modified_base 3: mod_base = gm
  modified_base 4: mod_base = cm
  modified_base 5: mod_base = um
  modified_base 6: mod_base = um
  modified_base 7: mod_base = um
  modified_base 8: mod_base = OTHER; note = 2'-O-methyl-adenosine
  modified_base 9: mod_base = OTHER; note = 2'-Fluoro-adenosine
  modified_base 10: mod_base = OTHER; note = 2'-Fluoro-cytidine
  modified_base 11: mod_base = OTHER; note = 2'-Fluoro-guanosine
  modified_base 12: mod_base = um
  modified_base 13: mod_base = gm
  modified_base 14: mod_base = um
  modified_base 15: mod_base = cm
  modified_base 16: mod_base = um
  modified_base 17: mod_base = gm
  modified_base 18: mod_base = um
  modified_base 19: mod_base = gm
  modified_base 20: mod_base = cm
  modified_base 21: mod_base = OTHER; note = 2'-O-methyl-adenosine
aggctttaacgtgtctgtgca

SEQ ID NO: 1134 - RNA, 21 nt, synthetic construct
  source 1..21: mol_type = other RNA
  modified_base <1: mod_base = OTHER; note = two inverted abasic nucleosides
  modified_base 1: mod_base = gm
  misc_feature 1^2: note = Phosphorothioate bond
  modified_base 2: mod_base = cm
  misc_feature 2^3: note = Phosphorothioate bond
  modified_base 3: mod_base = OTHER; note = 2'-O-methyl-adenosine
  modified_base 4: mod_base = gm
  modified_base 5: mod_base = um
  modified_base 6: mod_base = cm
  modified_base 7: mod_base = OTHER; note = 2'-O-methyl-adenosine
  modified_base 8: mod_base = gm
  modified_base 9: mod_base = OTHER; note = 2'-Fluoro-guanosine
  modified_base 10: mod_base = OTHER; note = 2'-Fluoro-guanosine
  modified_base 11: mod_base = OTHER; note = 2'-Fluoro-cytidine
  modified_base 12: mod_base = gm
  modified_base 13: mod_base = cm
  modified_base 14: mod_base = OTHER; note = 2'-O-methyl-adenosine
  modified_base 15: mod_base = OTHER; note = 2'-O-methyl-adenosine
  modified_base 16: mod_base = OTHER; note = 2'-O-methyl-adenosine
  modified_base 17: mod_base = gm
  modified_base 18: mod_base = gm
  modified_base 19: mod_base = OTHER; note = 2'-O-methyl-adenosine
  modified_base 20: mod_base = OTHER; note = 2'-O-methyl-adenosine
  modified_base 21: mod_base = cm
gcagtcagggcgcaaaggaac

SEQ ID NO: 1135 - RNA, 21 nt, synthetic construct
  source 1..21: mol_type = other RNA
  modified_base <1: mod_base = OTHER; note = two inverted abasic nucleosides
  modified_base 1: mod_base = gm
  misc_feature 1^2: note = Phosphorothioate bond
  modified_base 2: mod_base = OTHER; note = 2'-O-methyl-adenosine
  misc_feature 2^3: note = Phosphorothioate bond
  modified_base 3: mod_base = um
  modified_base 4: mod_base = gm
  modified_base 5: mod_base = OTHER; note = 2'-O-methyl-adenosine
  modified_base 6: mod_base = um
  modified_base 7: mod_base = cm
  modified_base 8: mod_base = gm
  modified_base 9: mod_base = OTHER; note = 2'-Fluoro-cytidine
  modified_base 10: mod_base = OTHER; note = 2'-Fluoro-adenosine
  modified_base 11: mod_base = OTHER; note = 2'-Fluoro-cytidine
  modified_base 12: mod_base = OTHER; note = 2'-O-methyl-adenosine
  modified_base 13: mod_base = gm
  modified_base 14: mod_base = OTHER; note = 2'-O-methyl-adenosine
  modified_base 15: mod_base = cm
  modified_base 16: mod_base = um
  modified_base 17: mod_base = gm
  modified_base 18: mod_base = um
  modified_base 19: mod_base = cm
  modified_base 20: mod_base = OTHER; note = 2'-O-methyl-adenosine
  modified_base 21: mod_base = cm
gatgatcgcacagactgtcac

SEQ ID NO: 1136 - RNA, 21 nt, synthetic construct
  source 1..21: mol_type = other RNA
  modified_base <1: mod_base = OTHER; note = two inverted abasic nucleosides
  modified_base 1: mod_base = OTHER; note = 2'-O-methyl-adenosine
  misc_feature 1^2: note = Phosphorothioate bond
  modified_base 2: mod_base = gm
  misc_feature 2^3: note = Phosphorothioate bond
  modified_base 3: mod_base = gm
  modified_base 4: mod_base = cm
  modified_base 5: mod_base = OTHER; note = 2'-O-methyl-adenosine
  modified_base 6: mod_base = um
  modified_base 7: mod_base = um
  modified_base 8: mod_base = OTHER; note = 2'-O-methyl-adenosine
  modified_base 9: mod_base = OTHER; note = 2'-Fluoro-uridine
  modified_base 10: mod_base = OTHER; note = 2'-Fluoro-adenosine
  modified_base 11: mod_base = OTHER; note = 2'-Fluoro-guanosine
  modified_base 12: mod_base = OTHER; note = 2'-O-methyl-adenosine
  modified_base 13: mod_base = cm
  modified_base 14: mod_base = um
  modified_base 15: mod_base = gm
  modified_base 16: mod_base = cm
  modified_base 17: mod_base = gm
  modified_base 18: mod_base = um
  modified_base 19: mod_base = gm
  modified_base 20: mod_base = gm
  modified_base 21: mod_base = um
aggcattatagactgcgtggt

SEQ ID NO: 1137 - RNA, 21 nt, synthetic construct
  source 1..21: mol_type = other RNA
  modified_base <1: mod_base = OTHER; note = two inverted abasic nucleosides
  modified_base 1: mod_base = um
  misc_feature 1^2: note = Phosphorothioate bond
  modified_base 2: mod_base = gm
  misc_feature 2^3: note = Phosphorothioate bond
  modified_base 3: mod_base = OTHER; note = 2'-O-methyl-adenosine
  modified_base 4: mod_base = um
  modified_base 5: mod_base = cm
  modified_base 6: mod_base = gm
  modified_base 7: mod_base = cm
  modified_base 8: mod_base = OTHER; note = 2'-O-methyl-adenosine
  modified_base 9: mod_base = OTHER; note = 2'-Fluoro-cytidine
  modified_base 10: mod_base = OTHER; note = 2'-Fluoro-adenosine
  modified_base 11: mod_base = OTHER; note = 2'-Fluoro-guanosine
  modified_base 12: mod_base = OTHER; note = 2'-O-methyl-adenosine
  modified_base 13: mod_base = cm
  modified_base 14: mod_base = um
  modified_base 15: mod_base = gm
  modified_base 16: mod_base = um
  modified_base 17: mod_base = cm
  modified_base 18: mod_base = OTHER; note = 2'-O-methyl-adenosine
  modified_base 19: mod_base = cm
  modified_base 20: mod_base = um
  modified_base 21: mod_base = gm
tgatcgcacagactgtcactg

SEQ ID NO: 1138 - RNA, 21 nt, synthetic construct
  source 1..21: mol_type = other RNA
  modified_base <1: mod_base = OTHER; note = two inverted abasic nucleosides
  modified_base 1: mod_base = cm
  misc_feature 1^2: note = Phosphorothioate bond
  modified_base 2: mod_base = um
  misc_feature 2^3: note = Phosphorothioate bond
  modified_base 3: mod_base = gm
  modified_base 4: mod_base = cm
  modified_base 5: mod_base = gm
  modified_base 6: mod_base = um
  modified_base 7: mod_base = gm
  modified_base 8: mod_base = gm
  modified_base 9: mod_base = OTHER; note = 2'-Fluoro-uridine
  modified_base 10: mod_base = OTHER; note = 2'-Fluoro-cytidine
  modified_base 11: mod_base = OTHER; note = 2'-Fluoro-cytidine
  modified_base 12: mod_base = gm
  modified_base 13: mod_base = um
  modified_base 14: mod_base = OTHER; note = 2'-O-methyl-adenosine
  modified_base 15: mod_base = um
  modified_base 16: mod_base = um
  modified_base 17: mod_base = cm
  modified_base 18: mod_base = cm
  modified_base 19: mod_base = cm
  modified_base 20: mod_base = OTHER; note = 2'-O-methyl-adenosine
  modified_base 21: mod_base = OTHER; note = 2'-O-methyl-adenosine
ctgcgtggtccgtattcccaa

SEQ ID NO: 1139 - RNA, 21 nt, synthetic construct
  source 1..21: mol_type = other RNA
  modified_base <1: mod_base = OTHER; note = two inverted abasic nucleosides
  modified_base 1: mod_base = cm
  misc_feature 1^2: note = Phosphorothioate bond
  modified_base 2: mod_base = OTHER; note = 2'-O-methyl-adenosine
  misc_feature 2^3: note = Phosphorothioate bond
  modified_base 3: mod_base = OTHER; note = 2'-O-methyl-adenosine
  modified_base 4: mod_base = um
  modified_base 5: mod_base = OTHER; note = 2'-O-methyl-adenosine
  modified_base 6: mod_base = cm
  modified_base 7: mod_base = OTHER; note = 2'-O-methyl-adenosine
  modified_base 8: mod_base = OTHER; note = 2'-O-methyl-adenosine
  modified_base 9: mod_base = OTHER; note = 2'-Fluoro-adenosine
  modified_base 10: mod_base = OTHER; note = 2'-Fluoro-guanosine
  modified_base 11: mod_base = OTHER; note = 2'-Fluoro-guanosine
  modified_base 12: mod_base = cm
  modified_base 13: mod_base = OTHER; note = 2'-O-methyl-adenosine
  modified_base 14: mod_base = um
  modified_base 15: mod_base = um
  modified_base 16: mod_base = OTHER; note = 2'-O-methyl-adenosine
  modified_base 17: mod_base = um
  modified_base 18: mod_base = OTHER; note = 2'-O-methyl-adenosine
  modified_base 19: mod_base = gm
  modified_base 20: mod_base = OTHER; note = 2'-O-methyl-adenosine
  modified_base 21: mod_base = cm
caatacaaaggcattatagac

SEQ ID NO: 1140 - RNA, 21 nt, synthetic construct
  source 1..21: mol_type = other RNA
  modified_base <1: mod_base = OTHER; note = two inverted abasic nucleosides
  modified_base 1: mod_base = cm
  misc_feature 1^2: note = Phosphorothioate bond
  modified_base 2: mod_base = OTHER; note = 2'-O-methyl-adenosine
  misc_feature 2^3: note = Phosphorothioate bond
  modified_base 3: mod_base = um
  modified_base 4: mod_base = cm
  modified_base 5: mod_base = OTHER; note = 2'-O-methyl-adenosine
  modified_base 6: mod_base = gm
  modified_base 7: mod_base = cm
  modified_base 8: mod_base = um
  modified_base 9: mod_base = OTHER; note = 2'-Fluoro-guanosine
  modified_base 10: mod_base = OTHER; note = 2'-Fluoro-guanosine
  modified_base 11: mod_base = OTHER; note = 2'-Fluoro-adenosine
  modified_base 12: mod_base = um
  modified_base 13: mod_base = gm
  modified_base 14: mod_base = OTHER; note = 2'-O-methyl-adenosine
  modified_base 15: mod_base = um
  modified_base 16: mod_base = cm
  modified_base 17: mod_base = gm
  modified_base 18: mod_base = cm
  modified_base 19: mod_base = OTHER; note = 2'-O-methyl-adenosine
  modified_base 20: mod_base = cm
  modified_base 21: mod_base = OTHER; note = 2'-O-methyl-adenosine
catcagctggatgatcgcaca

SEQ ID NO: 1141 - RNA, 21 nt, synthetic construct
  source 1..21: mol_type = other RNA
  modified_base <1: mod_base = OTHER; note = two inverted abasic nucleosides
  modified_base 1: mod_base = OTHER; note = 2'-O-methyl-adenosine
  misc_feature 1^2: note = Phosphorothioate bond
  modified_base 2: mod_base = um
  misc_feature 2^3: note = Phosphorothioate bond
  modified_base 3: mod_base = um
  modified_base 4: mod_base = OTHER; note = 2'-O-methyl-adenosine
  modified_base 5: mod_base = um
  modified_base 6: mod_base = OTHER; note = 2'-O-methyl-adenosine
  modified_base 7: mod_base = gm
  modified_base 8: mod_base = OTHER; note = 2'-O-methyl-adenosine
  modified_base 9: mod_base = OTHER; note = 2'-Fluoro-cytidine
  modified_base 10: mod_base = OTHER; note = 2'-Fluoro-uridine
  modified_base 11: mod_base = OTHER; note = 2'-Fluoro-guanosine
  modified_base 12: mod_base = cm
  modified_base 13: mod_base = gm
  modified_base 14: mod_base = um
  modified_base 15: mod_base = gm
  modified_base 16: mod_base = gm
  modified_base 17: mod_base = um
  modified_base 18: mod_base = cm
  modified_base 19: mod_base = cm
  modified_base 20: mod_base = gm
  modified_base 21: mod_base = um
attatagactgcgtggtccgt

SEQ ID NO: 1142 - RNA, 21 nt, synthetic construct
  source 1..21: mol_type = other RNA
  modified_base <1: mod_base = OTHER; note = two inverted abasic nucleosides
  modified_base 1: mod_base = um
  misc_feature 1^2: note = Phosphorothioate bond
  modified_base 2: mod_base = um
  misc_feature 2^3: note = Phosphorothioate bond
  modified_base 3: mod_base = um
  modified_base 4: mod_base = gm
  modified_base 5: mod_base = cm
  modified_base 6: mod_base = cm
  modified_base 7: mod_base = cm
  modified_base 8: mod_base = gm
  modified_base 9: mod_base = OTHER; note = 2'-Fluoro-uridine
  modified_base 10: mod_base = OTHER; note = 2'-Fluoro-adenosine
  modified_base 11: mod_base = OTHER; note = 2'-Fluoro-cytidine
  modified_base 12: mod_base = cm
  modified_base 13: mod_base = cm
  modified_base 14: mod_base = gm
  modified_base 15: mod_base = um
  modified_base 16: mod_base = cm
  modified_base 17: mod_base = um
  modified_base 18: mod_base = OTHER; note = 2'-O-methyl-adenosine
  modified_base 19: mod_base = gm
  modified_base 20: mod_base = cm
  modified_base 21: mod_base = OTHER; note = 2'-O-methyl-adenosine
tttgcccgtacccgtctagca

SEQ ID NO: 1143 - RNA, 21 nt, synthetic construct
  source 1..21: mol_type = other RNA
  modified_base <1: mod_base = OTHER; note = two inverted abasic nucleosides
  modified_base 1: mod_base = OTHER; note = 2'-O-methyl-adenosine
  misc_feature 1^2: note = Phosphorothioate bond
  modified_base 2: mod_base = cm
  misc_feature 2^3: note = Phosphorothioate bond
  modified_base 3: mod_base = OTHER; note = 2'-O-methyl-adenosine
  modified_base 4: mod_base = um
  modified_base 5: mod_base = cm
  modified_base 6: mod_base = gm
  modified_base 7: mod_base = um
  modified_base 8: mod_base = cm
  modified_base 9: mod_base = OTHER; note = 2'-Fluoro-adenosine
  modified_base 10: mod_base = OTHER; note = 2'-Fluoro-uridine
  modified_base 11: mod_base = OTHER; note = 2'-Fluoro-cytidine
  modified_base 12: mod_base = OTHER; note = 2'-O-methyl-adenosine
  modified_base 13: mod_base = gm
  modified_base 14: mod_base = cm
  modified_base 15: mod_base = um
  modified_base 16: mod_base = gm
  modified_base 17: mod_base = gm
  modified_base 18: mod_base = OTHER; note = 2'-O-methyl-adenosine
  modified_base 19: mod_base = um
  modified_base 20: mod_base = gm
  modified_base 21: mod_base = OTHER; note = 2'-O-methyl-adenosine
acatcgtcatcagctggatga

SEQ ID NO: 1144 - RNA, 21 nt, synthetic construct
  source 1..21: mol_type = other RNA
  modified_base <1: mod_base = OTHER; note = two inverted abasic nucleosides
  modified_base 1: mod_base = um
  misc_feature 1^2: note = Phosphorothioate bond
  modified_base 2: mod_base = cm
  misc_feature 2^3: note = Phosphorothioate bond
  modified_base 3: mod_base = um
  modified_base 4: mod_base = um
  modified_base 5: mod_base = gm
  modified_base 6: mod_base = OTHER; note = 2'-O-methyl-adenosine
  modified_base 7: mod_base = um
  modified_base 8: mod_base = um
  modified_base 9: mod_base = OTHER; note = 2'-Fluoro-uridine
  modified_base 10: mod_base = OTHER; note = 2'-Fluoro-uridine
  modified_base 11: mod_base = OTHER; note = 2'-Fluoro-guanosine
  modified_base 12: mod_base = cm
  modified_base 13: mod_base = cm
  modified_base 14: mod_base = cm
  modified_base 15: mod_base = gm
  modified_base 16: mod_base = um
  modified_base 17: mod_base = OTHER; note = 2'-O-methyl-adenosine
  modified_base 18: mod_base = cm
  modified_base 19: mod_base = cm
  modified_base 20: mod_base = cm
  modified_base 21: mod_base = gm
tcttgattttgcccgtacccg

SEQ ID NO: 1145 - RNA, 21 nt, synthetic construct
  source 1..21: mol_type = other RNA
  modified_base <1: mod_base = OTHER; note = two inverted abasic nucleosides
  modified_base 1: mod_base = OTHER; note = 2'-O-methyl-adenosine
  misc_feature 1^2: note = Phosphorothioate bond
  modified_base 2: mod_base = um
  misc_feature 2^3: note = Phosphorothioate bond
  modified_base 3: mod_base = OTHER; note = 2'-O-methyl-adenosine
  modified_base 4: mod_base = gm
  modified_base 5: mod_base = OTHER; note = 2'-O-methyl-adenosine
  modified_base 6: mod_base = cm
  modified_base 7: mod_base = um
  modified_base 8: mod_base = gm
  modified_base 9: mod_base = OTHER; note = 2'-Fluoro-cytidine
  modified_base 10: mod_base = OTHER; note = 2'-Fluoro-guanosine
  modified_base 11: mod_base = OTHER; note = 2'-Fluoro-uridine
  modified_base 12: mod_base = gm
  modified_base 13: mod_base = gm
  modified_base 14: mod_base = um
  modified_base 15: mod_base = cm
  modified_base 16: mod_base = cm
  modified_base 17: mod_base = gm
  modified_base 18: mod_base = um
  modified_base 19: mod_base = OTHER; note = 2'-O-methyl-adenosine
  modified_base 20: mod_base = um
  modified_base 21: mod_base = um
atagactgcgtggtccgtatt

SEQ ID NO: 1146 - RNA, 21 nt, synthetic construct
  source 1..21: mol_type = other RNA
  modified_base <1: mod_base = OTHER; note = two inverted abasic nucleosides
  modified_base 1: mod_base = cm
  misc_feature 1^2: note = Phosphorothioate bond
  modified_base 2: mod_base = gm
  misc_feature 2^3: note = Phosphorothioate bond
  modified_base 3: mod_base = cm
  modified_base 4: mod_base = cm
  modified_base 5: mod_base = um
  modified_base 6: mod_base = OTHER; note = 2'-O-methyl-adenosine
  modified_base 7: mod_base = cm
  modified_base 8: mod_base = um
  modified_base 9: mod_base = OTHER; note = 2'-Fluoro-uridine
  modified_base 10: mod_base = OTHER; note = 2'-Fluoro-cytidine
  modified_base 11: mod_base = OTHER; note = 2'-Fluoro-guanosine
  modified_base 12: mod_base = gm
  modified_base 13: mod_base = um
  modified_base 14: mod_base = OTHER; note = 2'-O-methyl-adenosine
  modified_base 15: mod_base = um
  modified_base 16: mod_base = cm
  modified_base 17: mod_base = um
  modified_base 18: mod_base = OTHER; note = 2'-O-methyl-adenosine
  modified_base 19: mod_base = um
  modified_base 20: mod_base = gm
  modified_base 21: mod_base = OTHER; note = 2'-O-methyl-adenosine
cgcctacttcggtatctatga

SEQ ID NO: 1147 - RNA, 21 nt, synthetic construct
  source 1..21: mol_type = other RNA
  modified_base <1: mod_base = OTHER; note = two inverted abasic nucleosides
  modified_base 1: mod_base = gm
  misc_feature 1^2: note = Phosphorothioate bond
  modified_base 2: mod_base = OTHER; note = 2'-O-methyl-adenosine
  misc_feature 2^3: note = Phosphorothioate bond
  modified_base 3: mod_base = cm
  modified_base 4: mod_base = um
  modified_base 5: mod_base = gm
  modified_base 6: mod_base = cm
  modified_base 7: mod_base = gm
  modified_base 8: mod_base = um
  modified_base 9: mod_base = OTHER; note = 2'-Fluoro-guanosine
  modified_base 10: mod_base = OTHER; note = 2'-Fluoro-guanosine
  modified_base 11: mod_base = OTHER; note = 2'-Fluoro-uridine
  modified_base 12: mod_base = cm
  modified_base 13: mod_base = cm
  modified_base 14: mod_base = gm
  modified_base 15: mod_base = um
  modified_base 16: mod_base = OTHER; note = 2'-O-methyl-adenosine
  modified_base 17: mod_base = um
  modified_base 18: mod_base = um
  modified_base 19: mod_base = cm
  modified_base 20: mod_base = cm
  modified_base 21: mod_base = cm
gactgcgtggtccgtattccc

SEQ ID NO: 1148 - RNA, 21 nt, synthetic construct
  source 1..21: mol_type = other RNA
  modified_base <1: mod_base = OTHER; note = two inverted abasic nucleosides
  modified_base 1: mod_base = um
  misc_feature 1^2: note = Phosphorothioate bond
  modified_base 2: mod_base = cm
  misc_feature 2^3: note = Phosphorothioate bond
  modified_base 3: mod_base = OTHER; note = 2'-O-methyl-adenosine
  modified_base 4: mod_base = um
  modified_base 5: mod_base = cm
  modified_base 6: mod_base = OTHER; note = 2'-O-methyl-adenosine
  modified_base 7: mod_base = gm
  modified_base 8: mod_base = cm
  modified_base 9: mod_base = OTHER; note = 2'-Fluoro-uridine
  modified_base 10: mod_base = OTHER; note = 2'-Fluoro-guanosine
  modified_base 11: mod_base = OTHER; note = 2'-Fluoro-guanosine
  modified_base 12: mod_base = OTHER; note = 2'-O-methyl-adenosine
  modified_base 13: mod_base = um
  modified_base 14: mod_base = gm
  modified_base 15: mod_base = OTHER; note = 2'-O-methyl-adenosine
  modified_base 16: mod_base = um
  modified_base 17: mod_base = cm
  modified_base 18: mod_base = gm
  modified_base 19: mod_base = cm
  modified_base 20: mod_base = OTHER; note = 2'-O-methyl-adenosine
  modified_base 21: mod_base = cm
tcatcagctggatgatcgcac

SEQ ID NO: 1149 - RNA, 21 nt, synthetic construct
  source 1..21: mol_type = other RNA
  modified_base <1: mod_base = OTHER; note = two inverted abasic nucleosides
  modified_base 1: mod_base = um
  misc_feature 1^2: note = Phosphorothioate bond
  modified_base 2: mod_base = um
  misc_feature 2^3: note = Phosphorothioate bond
  modified_base 3: mod_base = OTHER; note = 2'-O-methyl-adenosine
  modified_base 4: mod_base = um
  modified_base 5: mod_base = OTHER; note = 2'-O-methyl-adenosine
  modified_base 6: mod_base = gm
  modified_base 7: mod_base = OTHER; note = 2'-O-methyl-adenosine
  modified_base 8: mod_base = cm
  modified_base 9: mod_base = OTHER; note = 2'-Fluoro-uridine
  modified_base 10: mod_base = OTHER; note = 2'-Fluoro-guanosine
  modified_base 11: mod_base = OTHER; note = 2'-Fluoro-cytidine
  modified_base 12: mod_base = gm
  modified_base 13: mod_base = um
  modified_base 14: mod_base = gm
  modified_base 15: mod_base = gm
  modified_base 16: mod_base = um
  modified_base 17: mod_base = cm
  modified_base 18: mod_base = cm
  modified_base 19: mod_base = gm
  modified_base 20: mod_base = um
  modified_base 21: mod_base = OTHER; note = 2'-O-methyl-adenosine
ttatagactgcgtggtccgta

SEQ ID NO: 1150 - RNA, 21 nt, synthetic construct
  source 1..21: mol_type = other RNA
  modified_base <1: mod_base = OTHER; note = two inverted abasic nucleosides
  modified_base 1: mod_base = cm
  misc_feature 1^2: note = Phosphorothioate bond
  modified_base 2: mod_base = cm
  misc_feature 2^3: note = Phosphorothioate bond
  modified_base 3: mod_base = um
  modified_base 4: mod_base = OTHER; note = 2'-O-methyl-adenosine
  modified_base 5: mod_base = cm
  modified_base 6: mod_base = um
  modified_base 7: mod_base = um
  modified_base 8: mod_base = cm
  modified_base 9: mod_base = OTHER; note = 2'-Fluoro-guanosine
  modified_base 10: mod_base = OTHER; note = 2'-Fluoro-guanosine
  modified_base 11: mod_base = OTHER; note = 2'-Fluoro-uridine
  modified_base 12: mod_base = OTHER; note = 2'-O-methyl-adenosine
  modified_base 13: mod_base = um
  modified_base 14: mod_base = cm
  modified_base 15: mod_base = um
  modified_base 16: mod_base = OTHER; note = 2'-O-methyl-adenosine
  modified_base 17: mod_base = um
  modified_base 18: mod_base = gm
  modified_base 19: mod_base = OTHER; note = 2'-O-methyl-adenosine
  modified_base 20: mod_base = cm
  modified_base 21: mod_base = OTHER; note = 2'-O-methyl-adenosine
cctacttcggtatctatgaca

SEQ ID NO: 1151 - RNA, 21 nt, synthetic construct
  source 1..21: mol_type = other RNA
  modified_base <1: mod_base = OTHER; note = two inverted abasic nucleosides
  modified_base 1: mod_base = um
  misc_feature 1^2: note = Phosphorothioate bond
  modified_base 2: mod_base = um
  misc_feature 2^3: note = Phosphorothioate bond
  modified_base 3: mod_base = OTHER; note = 2'-O-methyl-adenosine
  modified_base 4: mod_base = um
  modified_base 5: mod_base = um
  modified_base 6: mod_base = um
  modified_base 7: mod_base = cm
  modified_base 8: mod_base = OTHER; note = 2'-O-methyl-adenosine
  modified_base 9: mod_base = OTHER; note = 2'-Fluoro-guanosine
  modified_base 10: mod_base = OTHER; note = 2'-Fluoro-uridine
  modified_base 11: mod_base = OTHER; note = 2'-Fluoro-cytidine
  modified_base 12: mod_base = OTHER; note = 2'-O-methyl-adenosine
  modified_base 13: mod_base = cm
  modified_base 14: mod_base = um
  modified_base 15: mod_base = cm
  modified_base 16: mod_base = cm
  modified_base 17: mod_base = um
  modified_base 18: mod_base = gm
  modified_base 19: mod_base = OTHER; note = 2'-O-methyl-adenosine
  modified_base 20: mod_base = um
  modified_base 21: mod_base = OTHER; note = 2'-O-methyl-adenosine
ttatttcagtcactcctgata

SEQ ID NO: 1152 - RNA, 21 nt, synthetic construct
  source 1..21: mol_type = other RNA
  modified_base <1: mod_base = OTHER; note = two inverted abasic nucleosides
  modified_base 1: mod_base = gm
  misc_feature 1^2: note = Phosphorothioate bond
  modified_base 2: mod_base = um
  misc_feature 2^3: note = Phosphorothioate bond
  modified_base 3: mod_base = cm
  modified_base 4: mod_base = OTHER; note = 2'-O-methyl-adenosine
  modified_base 5: mod_base = um
  modified_base 6: mod_base = cm
  modified_base 7: mod_base = OTHER; note = 2'-O-methyl-adenosine
  modified_base 8: mod_base = gm
  modified_base 9: mod_base = OTHER; note = 2'-Fluoro-cytidine
  modified_base 10: mod_base = OTHER; note = 2'-Fluoro-uridine
  modified_base 11: mod_base = OTHER; note = 2'-Fluoro-guanosine
  modified_base 12: mod_base = gm
  modified_base 13: mod_base = OTHER; note = 2'-O-methyl-adenosine
  modified_base 14: mod_base = um
  modified_base 15: mod_base = gm
  modified_base 16: mod_base = OTHER; note = 2'-O-methyl-adenosine
  modified_base 17: mod_base = um
  modified_base 18: mod_base = cm
  modified_base 19: mod_base = gm
  modified_base 20: mod_base = cm
  modified_base 21: mod_base = OTHER; note = 2'-O-methyl-adenosine
gtcatcagctggatgatcgca

SEQ ID NO: 1153 - RNA, 21 nt, synthetic construct
  source 1..21: mol_type = other RNA
  modified_base <1: mod_base = OTHER; note = two inverted abasic nucleosides
  modified_base 1: mod_base = OTHER; note = 2'-O-methyl-adenosine
  misc_feature 1^2: note = Phosphorothioate bond
  modified_base 2: mod_base = um
  misc_feature 2^3: note = Phosphorothioate bond
  modified_base 3: mod_base = um
  modified_base 4: mod_base = um
  modified_base 5: mod_base = um
  modified_base 6: mod_base = gm
  modified_base 7: mod_base = cm
  modified_base 8: mod_base = cm
  modified_base 9: mod_base = OTHER; note = 2'-Fluoro-cytidine
  modified_base 10: mod_base = OTHER; note = 2'-Fluoro-guanosine
  modified_base 11: mod_base = OTHER; note = 2'-Fluoro-uridine
  modified_base 12: mod_base = OTHER; note = 2'-O-methyl-adenosine
  modified_base 13: mod_base = cm
  modified_base 14: mod_base = cm
  modified_base 15: mod_base = cm
  modified_base 16: mod_base = gm
  modified_base 17: mod_base = um
  modified_base 18: mod_base = cm
  modified_base 19: mod_base = um
  modified_base 20: mod_base = OTHER; note = 2'-O-methyl-adenosine
  modified_base 21: mod_base = gm
attttgcccgtacccgtctag

SEQ ID NO: 1154 - RNA, 21 nt, synthetic construct
  source 1..21: mol_type = other RNA
  modified_base <1: mod_base = OTHER; note = two inverted abasic nucleosides
  modified_base 1: mod_base = cm
  misc_feature 1^2: note = Phosphorothioate bond
  modified_base 2: mod_base = OTHER; note = 2'-O-methyl-adenosine
  misc_feature 2^3: note = Phosphorothioate bond
  modified_base 3: mod_base = OTHER; note = 2'-O-methyl-adenosine
  modified_base 4: mod_base = OTHER; note = 2'-O-methyl-adenosine
  modified_base 5: mod_base = gm
  modified_base 6: mod_base = gm
  modified_base 7: mod_base = gm
  modified_base 8: mod_base = OTHER; note = 2'-O-methyl-adenosine
  modified_base 9: mod_base = OTHER; note = 2'-Fluoro-adenosine
  modified_base 10: mod_base = OTHER; note = 2'-Fluoro-uridine
  modified_base 11: mod_base = OTHER; note = 2'-Fluoro-guanosine
  modified_base 12: mod_base = cm
  modified_base 13: mod_base = um
  modified_base 14: mod_base = um
  modified_base 15: mod_base = cm
  modified_base 16: mod_base = cm
  modified_base 17: mod_base = gm
  modified_base 18: mod_base = gm
  modified_base 19: mod_base = OTHER; note = 2'-O-methyl-adenosine
  modified_base 20: mod_base = um
  modified_base 21: mod_base = cm
caaagggaatgcttccggatc

SEQ ID NO: 1155 - RNA, 21 nt, synthetic construct
  source 1..21: mol_type = other RNA
  modified_base <1: mod_base = OTHER; note = two inverted abasic nucleosides
  modified_base 1: mod_base = OTHER; note = 2'-O-methyl-adenosine
  misc_feature 1^2: note = Phosphorothioate bond
  modified_base 2: mod_base = OTHER; note = 2'-O-methyl-adenosine
  misc_feature 2^3: note = Phosphorothioate bond
  modified_base 3: mod_base = gm
  modified_base 4: mod_base = gm
  modified_base 5: mod_base = cm
  modified_base 6: mod_base = um
  modified_base 7: mod_base = um
  modified_base 8: mod_base = um
  modified_base 9: mod_base = OTHER; note = 2'-Fluoro-adenosine
  modified_base 10: mod_base = OTHER; note = 2'-Fluoro-adenosine
  modified_base 11: mod_base = OTHER; note = 2'-Fluoro-cytidine
  modified_base 12: mod_base = gm
  modified_base 13: mod_base = um
  modified_base 14: mod_base = gm
  modified_base 15: mod_base = um
  modified_base 16: mod_base = cm
  modified_base 17: mod_base = um
  modified_base 18: mod_base = gm
  modified_base 19: mod_base = um
  modified_base 20: mod_base = gm
  modified_base 21: mod_base = cm
aaggctttaacgtgtctgtgc

SEQ ID NO: 1156 - RNA, 21 nt, synthetic construct
  source 1..21: mol_type = other RNA
  modified_base <1: mod_base = OTHER; note = two inverted abasic nucleosides
  modified_base 1: mod_base = OTHER; note = 2'-O-methyl-adenosine
  misc_feature 1^2: note = Phosphorothioate bond
  modified_base 2: mod_base = OTHER; note = 2'-O-methyl-adenosine
  misc_feature 2^3: note = Phosphorothioate bond
  modified_base 3: mod_base = gm
  modified_base 4: mod_base = gm
  modified_base 5: mod_base = cm
  modified_base 6: mod_base = OTHER; note = 2'-O-methyl-adenosine
  modified_base 7: mod_base = um
  modified_base 8: mod_base = um
  modified_base 9: mod_base = OTHER; note = 2'-Fluoro-adenosine
  modified_base 10: mod_base = OTHER; note = 2'-Fluoro-uridine
  modified_base 11: mod_base = OTHER; note = 2'-Fluoro-adenosine
  modified_base 12: mod_base = gm
  modified_base 13: mod_base = OTHER; note = 2'-O-methyl-adenosine
  modified_base 14: mod_base = cm
  modified_base 15: mod_base = um
  modified_base 16: mod_base = gm
  modified_base 17: mod_base = cm
  modified_base 18: mod_base = gm
  modified_base 19: mod_base = um
  modified_base 20: mod_base = gm
  modified_base 21: mod_base = gm
aaggcattatagactgcgtgg

SEQ ID NO: 1157 - RNA, 21 nt, synthetic construct
  source 1..21: mol_type = other RNA
  modified_base <1: mod_base = OTHER; note = two inverted abasic nucleosides
  modified_base 1: mod_base = um
  misc_feature 1^2: note = Phosphorothioate bond
  modified_base 2: mod_base = um
  misc_feature 2^3: note = Phosphorothioate bond
  modified_base 3: mod_base = gm
  modified_base 4: mod_base = OTHER; note = 2'-O-methyl-adenosine
  modified_base 5: mod_base = um
  modified_base 6: mod_base = um
  modified_base 7: mod_base = um
  modified_base 8: mod_base = um
  modified_base 9: mod_base = OTHER; note = 2'-Fluoro-guanosine
  modified_base 10: mod_base = OTHER; note = 2'-Fluoro-cytidine
  modified_base 11: mod_base = OTHER; note = 2'-Fluoro-cytidine
  modified_base 12: mod_base = cm
  modified_base 13: mod_base = gm
  modified_base 14: mod_base = um
  modified_base 15: mod_base = OTHER; note = 2'-O-methyl-adenosine
  modified_base 16: mod_base = cm
  modified_base 17: mod_base = cm
  modified_base 18: mod_base = cm
  modified_base 19: mod_base = gm
  modified_base 20: mod_base = um
  modified_base 21: mod_base = cm
ttgattttgcccgtacccgtc

SEQ ID NO: 1158 - RNA, 21 nt, synthetic construct
  source 1..21: mol_type = other RNA
  modified_base <1: mod_base = OTHER; note = two inverted abasic nucleosides
  modified_base 1: mod_base = cm
  misc_feature 1^2: note = Phosphorothioate bond
  modified_base 2: mod_base = gm
  misc_feature 2^3: note = Phosphorothioate bond
  modified_base 3: mod_base = OTHER; note = 2'-O-methyl-adenosine
  modified_base 4: mod_base = gm
  modified_base 5: mod_base = cm
  modified_base 6: mod_base = cm
  modified_base 7: mod_base = gm
  modified_base 8: mod_base = cm
  modified_base 9: mod_base = OTHER; note = 2'-Fluoro-cytidine
  modified_base 10: mod_base = OTHER; note = 2'-Fluoro-uridine
  modified_base 11: mod_base = OTHER; note = 2'-Fluoro-adenosine
  modified_base 12: mod_base = cm
  modified_base 13: mod_base = um
  modified_base 14: mod_base = um
  modified_base 15: mod_base = cm
  modified_base 16: mod_base = gm
  modified_base 17: mod_base = gm
  modified_base 18: mod_base = um
  modified_base 19: mod_base = OTHER; note = 2'-O-methyl-adenosine
  modified_base 20: mod_base = um
  modified_base 21: mod_base = cm
cgagccgcctacttcggtatc

SEQ ID NO: 1159 - RNA, 21 nt, synthetic construct
  source 1..21: mol_type = other RNA
  modified_base <1: mod_base = OTHER; note = two inverted abasic nucleosides
  modified_base 1: mod_base = OTHER; note = 2'-O-methyl-adenosine
  misc_feature 1^2: note = Phosphorothioate bond
  modified_base 2: mod_base = um
  misc_feature 2^3: note = Phosphorothioate bond
  modified_base 3: mod_base = cm
  modified_base 4: mod_base = OTHER; note = 2'-O-methyl-adenosine
  modified_base 5: mod_base = um
  modified_base 6: mod_base = cm
  modified_base 7: mod_base = um
  modified_base 8: mod_base = OTHER; note = 2'-O-methyl-adenosine
  modified_base 9: mod_base = OTHER; note = 2'-Fluoro-cytidine
  modified_base 10: mod_base = OTHER; note = 2'-Fluoro-cytidine
  modified_base 11: mod_base = OTHER; note = 2'-Fluoro-guanosine
  modified_base 12: mod_base = OTHER; note = 2'-O-methyl-adenosine
  modified_base 13: mod_base = gm
  modified_base 14: mod_base = cm
  modified_base 15: mod_base = cm
  modified_base 16: mod_base = gm
  modified_base 17: mod_base = cm
  modified_base 18: mod_base = cm
  modified_base 19: mod_base = um
  modified_base 20: mod_base = OTHER; note = 2'-O-methyl-adenosine
  modified_base 21: mod_base = cm
atcatctaccgagccgcctac

SEQ ID NO: 1160 - RNA, 21 nt, synthetic construct
  source 1..21: mol_type = other RNA
  modified_base <1: mod_base = OTHER; note = two inverted abasic nucleosides
  modified_base 1: mod_base = um
  misc_feature 1^2: note = Phosphorothioate bond
  modified_base 2: mod_base = gm
  misc_feature 2^3: note = Phosphorothioate bond
  modified_base 3: mod_base = OTHER; note = 2'-O-methyl-adenosine
  modified_base 4: mod_base = um
  modified_base 5: mod_base = um
  modified_base 6: mod_base = um
  modified_base 7: mod_base = um
  modified_base 8: mod_base = gm
  modified_base 9: mod_base = OTHER; note = 2'-Fluoro-cytidine
  modified_base 10: mod_base = OTHER; note = 2'-Fluoro-cytidine
  modified_base 11: mod_base = OTHER; note = 2'-Fluoro-cytidine
  modified_base 12: mod_base = gm
  modified_base 13: mod_base = um
  modified_base 14: mod_base = OTHER; note = 2'-O-methyl-adenosine
  modified_base 15: mod_base = cm
  modified_base 16: mod_base = cm
  modified_base 17: mod_base = cm
  modified_base 18: mod_base = gm
  modified_base 19: mod_base = um
  modified_base 20: mod_base = cm
  modified_base 21: mod_base = um
tgattttgcccgtacccgtct

SEQ ID NO: 1161 - RNA, 21 nt, synthetic construct
  source 1..21: mol_type = other RNA
  modified_base <1: mod_base = OTHER; note = two inverted abasic nucleosides
  modified_base 1: mod_base = um
  misc_feature 1^2: note = Phosphorothioate bond
  modified_base 2: mod_base = OTHER; note = 2'-O-methyl-adenosine
  misc_feature 2^3: note = Phosphorothioate bond
  modified_base 3: mod_base = um
  modified_base 4: mod_base = cm
  modified_base 5: mod_base = OTHER; note = 2'-O-methyl-adenosine
  modified_base 6: mod_base = um
  modified_base 7: mod_base = cm
  modified_base 8: mod_base = um
  modified_base 9: mod_base = OTHER; note = 2'-Fluoro-adenosine
  modified_base 10: mod_base = OTHER; note = 2'-Fluoro-cytidine
  modified_base 11: mod_base = OTHER; note = 2'-Fluoro-cytidine
  modified_base 12: mod_base = gm
  modified_base 13: mod_base = OTHER; note = 2'-O-methyl-adenosine
  modified_base 14: mod_base = gm
  modified_base 15: mod_base = cm
  modified_base 16: mod_base = cm
  modified_base 17: mod_base = gm
  modified_base 18: mod_base = cm
  modified_base 19: mod_base = cm
  modified_base 20: mod_base = um
  modified_base 21: mod_base = OTHER; note = 2'-O-methyl-adenosine
tatcatctaccgagccgccta

SEQ ID NO: 1162 - RNA, 21 nt, synthetic construct
  source 1..21: mol_type = other RNA
  modified_base <1: mod_base = OTHER; note = two inverted abasic nucleosides
  modified_base 1: mod_base = cm
  misc_feature 1^2: note = Phosphorothioate bond
  modified_base 2: mod_base = OTHER; note = 2'-O-methyl-adenosine
  misc_feature 2^3: note = Phosphorothioate bond
  modified_base 3: mod_base = um
  modified_base 4: mod_base = cm
  modified_base 5: mod_base = um
  modified_base 6: mod_base = OTHER; note = 2'-O-methyl-adenosine
  modified_base 7: mod_base = cm
  modified_base 8: mod_base = cm
  modified_base 9: mod_base = OTHER; note = 2'-Fluoro-guanosine
  modified_base 10: mod_base = OTHER; note = 2'-Fluoro-adenosine
  modified_base 11: mod_base = OTHER; note = 2'-Fluoro-guanosine
  modified_base 12: mod_base = cm
  modified_base 13: mod_base = cm
  modified_base 14: mod_base = gm
  modified_base 15: mod_base = cm
  modified_base 16: mod_base = cm
  modified_base 17: mod_base = um
  modified_base 18: mod_base = OTHER; note = 2'-O-methyl-adenosine
  modified_base 19: mod_base = cm
  modified_base 20: mod_base = um
  modified_base 21: mod_base = um
catctaccgagccgcctactt

SEQ ID NO: 1163 - RNA, 21 nt, synthetic construct
  source 1..21: mol_type = other RNA
  modified_base <1: mod_base = OTHER; note = two inverted abasic nucleosides
  modified_base 1: mod_base = cm
  misc_feature 1^2: note = Phosphorothioate bond
  modified_base 2: mod_base = um
  misc_feature 2^3: note = Phosphorothioate bond
  modified_base 3: mod_base = cm
  modified_base 4: mod_base = um
  modified_base 5: mod_base = um
  modified_base 6: mod_base = OTHER; note = 2'-O-methyl-adenosine
  modified_base 7: mod_base = OTHER; note = 2'-O-methyl-adenosine
  modified_base 8: mod_base = cm
  modified_base 9: mod_base = OTHER; note = 2'-Fluoro-uridine
  modified_base 10: mod_base = OTHER; note = 2'-Fluoro-uridine
  modified_base 11: mod_base = OTHER; note = 2'-Fluoro-cytidine
  modified_base 12: mod_base = gm
  modified_base 13: mod_base = cm
  modified_base 14: mod_base = cm
  modified_base 15: mod_base = um
  modified_base 16: mod_base = um
  modified_base 17: mod_base = cm
  modified_base 18: mod_base = OTHER; note = 2'-O-methyl-adenosine
  modified_base 19: mod_base = OTHER; note = 2'-O-methyl-adenosine
  modified_base 20: mod_base = OTHER; note = 2'-O-methyl-adenosine
  modified_base 21: mod_base = gm
ctcttaacttcgccttcaaag

SEQ ID NO: 1164 - RNA, 21 nt, synthetic construct
  source 1..21: mol_type = other RNA
  modified_base <1: mod_base = OTHER; note = two inverted abasic nucleosides
  modified_base 1: mod_base = cm
  misc_feature 1^2: note = Phosphorothioate bond
  modified_base 2: mod_base = cm
  misc_feature 2^3: note = Phosphorothioate bond
  modified_base 3: mod_base = OTHER; note = 2'-O-methyl-adenosine
  modified_base 4: mod_base = cm
  modified_base 5: mod_base = cm
  modified_base 6: mod_base = cm
  modified_base 7: mod_base = OTHER; note = 2'-O-methyl-adenosine
  modified_base 8: mod_base = gm
  modified_base 9: mod_base = OTHER; note = 2'-Fluoro-guanosine
  modified_base 10: mod_base = OTHER; note = 2'-Fluoro-cytidine
  modified_base 11: mod_base = OTHER; note = 2'-Fluoro-uridine
  modified_base 12: mod_base = cm
  modified_base 13: mod_base = um
  modified_base 14: mod_base = um
  modified_base 15: mod_base = OTHER; note = 2'-O-methyl-adenosine
  modified_base 16: mod_base = OTHER; note = 2'-O-methyl-adenosine
  modified_base 17: mod_base = cm
  modified_base 18: mod_base = um
  modified_base 19: mod_base = um
  modified_base 20: mod_base = cm
  modified_base 21: mod_base = gm
ccacccaggctcttaacttcg

SEQ ID NO: 1165 - RNA, 21 nt, synthetic construct
  source 1..21: mol_type = other RNA
  modified_base <1: mod_base = OTHER; note = two inverted abasic nucleosides
  modified_base 1: mod_base = cm
  misc_feature 1^2: note = Phosphorothioate bond
  modified_base 2: mod_base = cm
  misc_feature 2^3: note = Phosphorothioate bond
  modified_base 3: mod_base = gm
  modified_base 4: mod_base = um
  modified_base 5: mod_base = OTHER; note = 2'-O-methyl-adenosine
  modified_base 6: mod_base = um
  modified_base 7: mod_base = um
  modified_base 8: mod_base = cm
  modified_base 9: mod_base = OTHER; note = 2'-Fluoro-cytidine
  modified_base 10: mod_base = OTHER; note = 2'-Fluoro-cytidine
  modified_base 11: mod_base = OTHER; note = 2'-Fluoro-adenosine
  modified_base 12: mod_base = OTHER; note = 2'-O-methyl-adenosine
  modified_base 13: mod_base = gm
  modified_base 14: mod_base = gm
  modified_base 15: mod_base = OTHER; note = 2'-O-methyl-adenosine
  modified_base 16: mod_base = gm
  modified_base 17: mod_base = cm
  modified_base 18: mod_base = OTHER; note = 2'-O-methyl-adenosine
  modified_base 19: mod_base = gm
  modified_base 20: mod_base = gm
  modified_base 21: mod_base = gm
ccgtattcccaaggagcaggg

SEQ ID NO: 1166 - RNA, 21 nt, synthetic construct
  source 1..21: mol_type = other RNA
  modified_base <1: mod_base = OTHER; note = two inverted abasic nucleosides
  modified_base 1: mod_base = gm
  misc_feature 1^2: note = Phosphorothioate bond
  modified_base 2: mod_base = OTHER; note = 2'-O-methyl-adenosine
  misc_feature 2^3: note = Phosphorothioate bond
  modified_base 3: mod_base = gm
  modified_base 4: mod_base = cm
  modified_base 5: mod_base = OTHER; note = 2'-O-methyl-adenosine
  modified_base 6: mod_base = gm
  modified_base 7: mod_base = gm
  modified_base 8: mod_base = gm
  modified_base 9: mod_base = OTHER; note = 2'-Fluoro-adenosine
  modified_base 10: mod_base = OTHER; note = 2'-Fluoro-guanosine
  modified_base 11: mod_base = OTHER; note = 2'-Fluoro-uridine
  modified_base 12: mod_base = um
  modified_base 13: mod_base = cm
  modified_base 14: mod_base = um
  modified_base 15: mod_base = gm
  modified_base 16: mod_base = um
  modified_base 17: mod_base = cm
  modified_base 18: mod_base = cm
  modified_base 19: mod_base = um
  modified_base 20: mod_base = um
  modified_base 21: mod_base = cm
gagcagggagttctgtccttc

SEQ ID NO: 1167 - RNA, 21 nt, synthetic construct
  source 1..21: mol_type = other RNA
  modified_base <1: mod_base = OTHER; note = two inverted abasic nucleosides
  modified_base 1: mod_base = um
  misc_feature 1^2: note = Phosphorothioate bond
  modified_base 2: mod_base = cm
  misc_feature 2^3: note = Phosphorothioate bond
  modified_base 3: mod_base = cm
  modified_base 4: mod_base = cm
  modified_base 5: mod_base = OTHER; note = 2'-O-methyl-adenosine
  modified_base 6: mod_base = OTHER; note = 2'-O-methyl-adenosine
  modified_base 7: mod_base = gm
  modified_base 8: mod_base = gm
  modified_base 9: mod_base = OTHER; note = 2'-Fluoro-adenosine
  modified_base 10: mod_base = OTHER; note = 2'-Fluoro-guanosine
  modified_base 11: mod_base = OTHER; note = 2'-Fluoro-cytidine
  modified_base 12: mod_base = OTHER; note = 2'-O-methyl-adenosine
  modified_base 13: mod_base = gm
  modified_base 14: mod_base = gm
  modified_base 15: mod_base = gm
  modified_base 16: mod_base = OTHER; note = 2'-O-methyl-adenosine
  modified_base 17: mod_base = gm
  modified_base 18: mod_base = um
  modified_base 19: mod_base = um
  modified_base 20: mod_base = cm
  modified_base 21: mod_base = um
tcccaaggagcagggagttct

SEQ ID NO: 1168 - RNA, 21 nt, synthetic construct
  source 1..21: mol_type = other RNA
  modified_base <1: mod_base = OTHER; note = two inverted abasic nucleosides
  modified_base 1: mod_base = um
  misc_feature 1^2: note = Phosphorothioate bond
  modified_base 2: mod_base = cm
  misc_feature 2^3: note = Phosphorothioate bond
  modified_base 3: mod_base = cm
  modified_base 4: mod_base = gm
  modified_base 5: mod_base = um
  modified_base 6: mod_base = OTHER; note = 2'-O-methyl-adenosine
  modified_base 7: mod_base = um
  modified_base 8: mod_base = um
  modified_base 9: mod_base = OTHER; note = 2'-Fluoro-cytidine
  modified_base 10: mod_base = OTHER; note = 2'-Fluoro-cytidine
  modified_base 11: mod_base = OTHER; note = 2'-Fluoro-cytidine
  modified_base 12: mod_base = OTHER; note = 2'-O-methyl-adenosine
  modified_base 13: mod_base = OTHER; note = 2'-O-methyl-adenosine
  modified_base 14: mod_base = gm
  modified_base 15: mod_base = gm
  modified_base 16: mod_base = OTHER; note = 2'-O-methyl-adenosine
  modified_base 17: mod_base = gm
  modified_base 18: mod_base = cm
  modified_base 19: mod_base = OTHER; note = 2'-O-methyl-adenosine
  modified_base 20: mod_base = gm
  modified_base 21: mod_base = gm
tccgtattcccaaggagcagg

SEQ ID NO: 1169 - RNA, 21 nt, synthetic construct
  source 1..21: mol_type = other RNA
  modified_base <1: mod_base = OTHER; note = two inverted abasic nucleosides
  modified_base 1: mod_base = gm
  misc_feature 1^2: note = Phosphorothioate bond
  modified_base 2: mod_base = cm
  misc_feature 2^3: note = Phosphorothioate bond
  modified_base 3: mod_base = OTHER; note = 2'-O-methyl-adenosine
  modified_base 4: mod_base = gm
  modified_base 5: mod_base = gm
  modified_base 6: mod_base = gm
  modified_base 7: mod_base = OTHER; note = 2'-O-methyl-adenosine
  modified_base 8: mod_base = gm
  modified_base 9: mod_base = OTHER; note = 2'-Fluoro-uridine
  modified_base 10: mod_base = OTHER; note = 2'-Fluoro-uridine
  modified_base 11: mod_base = OTHER; note = 2'-Fluoro-cytidine
  modified_base 12: mod_base = um
  modified_base 13: mod_base = gm
  modified_base 14: mod_base = um
  modified_base 15: mod_base = cm
  modified_base 16: mod_base = cm
  modified_base 17: mod_base = um
  modified_base 18: mod_base = um
  modified_base 19: mod_base = cm
  modified_base 20: mod_base = um
  modified_base 21: mod_base = gm
gcagggagttctgtccttctg

SEQ ID NO: 1170 - RNA, 21 nt, synthetic construct
  source 1..21: mol_type = other RNA
  modified_base <1: mod_base = OTHER; note = two inverted abasic nucleosides
  modified_base 1: mod_base = gm
  misc_feature 1^2: note = Phosphorothioate bond
  modified_base 2: mod_base = um
  misc_feature 2^3: note = Phosphorothioate bond
  modified_base 3: mod_base = cm
  modified_base 4: mod_base = cm
  modified_base 5: mod_base = gm
  modified_base 6: mod_base = um
  modified_base 7: mod_base = OTHER; note = 2'-O-methyl-adenosine
  modified_base 8: mod_base = um
  modified_base 9: mod_base = OTHER; note = 2'-Fluoro-uridine
  modified_base 10: mod_base = OTHER; note = 2'-Fluoro-cytidine
  modified_base 11: mod_base = OTHER; note = 2'-Fluoro-cytidine
  modified_base 12: mod_base = cm
  modified_base 13: mod_base = OTHER; note = 2'-O-methyl-adenosine
  modified_base 14: mod_base = OTHER; note = 2'-O-methyl-adenosine
  modified_base 15: mod_base = gm
  modified_base 16: mod_base = gm
  modified_base 17: mod_base = OTHER; note = 2'-O-methyl-adenosine
  modified_base 18: mod_base = gm
  modified_base 19: mod_base = cm
  modified_base 20: mod_base = OTHER; note = 2'-O-methyl-adenosine
  modified_base 21: mod_base = gm
gtccgtattcccaaggagcag

SEQ ID NO: 1171 - RNA, 21 nt, synthetic construct
  source 1..21: mol_type = other RNA
  modified_base <1: mod_base = OTHER; note = two inverted abasic nucleosides
  modified_base 1: mod_base = OTHER; note = 2'-O-methyl-adenosine
  misc_feature 1^2: note = Phosphorothioate bond
  modified_base 2: mod_base = gm
  misc_feature 2^3: note = Phosphorothioate bond
  modified_base 3: mod_base = cm
  modified_base 4: mod_base = OTHER; note = 2'-O-methyl-adenosine
  modified_base 5: mod_base = gm
  modified_base 6: mod_base = gm
  modified_base 7: mod_base = gm
  modified_base 8: mod_base = OTHER; note = 2'-O-methyl-adenosine
  modified_base 9: mod_base = OTHER; note = 2'-Fluoro-guanosine
  modified_base 10: mod_base = OTHER; note = 2'-Fluoro-uridine
  modified_base 11: mod_base = OTHER; note = 2'-Fluoro-uridine
  modified_base 12: mod_base = cm
  modified_base 13: mod_base = um
  modified_base 14: mod_base = gm
  modified_base 15: mod_base = um
  modified_base 16: mod_base = cm
  modified_base 17: mod_base = cm
  modified_base 18: mod_base = um
  modified_base 19: mod_base = um
  modified_base 20: mod_base = cm
  modified_base 21: mod_base = um
agcagggagttctgtccttct

SEQ ID NO: 1172 - RNA, 21 nt, synthetic construct
  source 1..21: mol_type = other RNA
  modified_base <1: mod_base = OTHER; note = two inverted abasic nucleosides
  modified_base 1: mod_base = gm
  misc_feature 1^2: note = Phosphorothioate bond
  modified_base 2: mod_base = gm
  misc_feature 2^3: note = Phosphorothioate bond
  modified_base 3: mod_base = OTHER; note = 2'-O-methyl-adenosine
  modified_base 4: mod_base = gm
  modified_base 5: mod_base = cm
  modified_base 6: mod_base = OTHER; note = 2'-O-methyl-adenosine
  modified_base 7: mod_base = gm
  modified_base 8: mod_base = gm
  modified_base 9: mod_base = OTHER; note = 2'-Fluoro-guanosine
  modified_base 10: mod_base = OTHER; note = 2'-Fluoro-adenosine
  modified_base 11: mod_base = OTHER; note = 2'-Fluoro-guanosine
  modified_base 12: mod_base = um
  modified_base 13: mod_base = um
  modified_base 14: mod_base = cm
  modified_base 15: mod_base = um
  modified_base 16: mod_base = gm
  modified_base 17: mod_base = um
  modified_base 18: mod_base = cm
  modified_base 19: mod_base = cm
  modified_base 20: mod_base = um
  modified_base 21: mod_base = um
ggagcagggagttctgtcctt

SEQ ID NO: 1173 - RNA, 21 nt, synthetic construct
  source 1..21: mol_type = other RNA
  modified_base <1: mod_base = OTHER; note = two inverted abasic nucleosides
  modified_base 1: mod_base = um
  misc_feature 1^2: note = Phosphorothioate bond
  modified_base 2: mod_base = um
  misc_feature 2^3: note = Phosphorothioate bond
  modified_base 3: mod_base = cm
  modified_base 4: mod_base = cm
  modified_base 5: mod_base = cm
  modified_base 6: mod_base = OTHER; note = 2'-O-methyl-adenosine
  modified_base 7: mod_base = OTHER; note = 2'-O-methyl-adenosine
  modified_base 8: mod_base = gm
  modified_base 9: mod_base = OTHER; note = 2'-Fluoro-guanosine
  modified_base 10: mod_base = OTHER; note = 2'-Fluoro-adenosine
  modified_base 11: mod_base = OTHER; note = 2'-Fluoro-guanosine
  modified_base 12: mod_base = cm
  modified_base 13: mod_base = OTHER; note = 2'-O-methyl-adenosine
  modified_base 14: mod_base = gm
  modified_base 15: mod_base = gm
  modified_base 16: mod_base = gm
  modified_base 17: mod_base = OTHER; note = 2'-O-methyl-adenosine
  modified_base 18: mod_base = gm
  modified_base 19: mod_base = um
  modified_base 20: mod_base = um
  modified_base 21: mod_base = cm
ttcccaaggagcagggagttc

SEQ ID NO: 1174 - RNA, 21 nt, synthetic construct
  source 1..21: mol_type = other RNA
  modified_base <1: mod_base = OTHER; note = two inverted abasic nucleosides
  modified_base 1: mod_base = OTHER; note = 2'-O-methyl-adenosine
  misc_feature 1^2: note = Phosphorothioate bond
  modified_base 2: mod_base = gm
  misc_feature 2^3: note = Phosphorothioate bond
  modified_base 3: mod_base = gm
  modified_base 4: mod_base = OTHER; note = 2'-O-methyl-adenosine
  modified_base 5: mod_base = gm
  modified_base 6: mod_base = cm
  modified_base 7: mod_base = OTHER; note = 2'-O-methyl-adenosine
  modified_base 8: mod_base = gm
  modified_base 9: mod_base = OTHER; note = 2'-Fluoro-guanosine
  modified_base 10: mod_base = OTHER; note = 2'-Fluoro-guanosine
  modified_base 11: mod_base = OTHER; note = 2'-Fluoro-adenosine
  modified_base 12: mod_base = gm
  modified_base 13: mod_base = um
  modified_base 14: mod_base = um
  modified_base 15: mod_base = cm
  modified_base 16: mod_base = um
  modified_base 17: mod_base = gm
  modified_base 18: mod_base = um
  modified_base 19: mod_base = cm
  modified_base 20: mod_base = cm
  modified_base 21: mod_base = um
aggagcagggagttctgtcct

SEQ ID NO: 1175 - RNA, 21 nt, synthetic construct
  source 1..21: mol_type = other RNA
  modified_base <1: mod_base = OTHER; note = two inverted abasic nucleosides
  modified_base 1: mod_base = cm
  misc_feature 1^2: note = Phosphorothioate bond
  modified_base 2: mod_base = cm
  misc_feature 2^3: note = Phosphorothioate bond
  modified_base 3: mod_base = cm
  modified_base 4: mod_base = OTHER; note = 2'-O-methyl-adenosine
  modified_base 5: mod_base = cm
  modified_base 6: mod_base = cm
  modified_base 7: mod_base = cm
  modified_base 8: mod_base = OTHER; note = 2'-O-methyl-adenosine
  modified_base 9: mod_base = OTHER; note = 2'-Fluoro-guanosine
  modified_base 10: mod_base = OTHER; note = 2'-Fluoro-guanosine
  modified_base 11: mod_base = OTHER; note = 2'-Fluoro-cytidine
  modified_base 12: mod_base = um
  modified_base 13: mod_base = cm
  modified_base 14: mod_base = um
  modified_base 15: mod_base = um
  modified_base 16: mod_base = OTHER; note = 2'-O-methyl-adenosine
  modified_base 17: mod_base = OTHER; note = 2'-O-methyl-adenosine
  modified_base 18: mod_base = cm
  modified_base 19: mod_base = um
  modified_base 20: mod_base = um
  modified_base 21: mod_base = cm
cccacccaggctcttaacttc

SEQ ID NO: 1176 - RNA, 21 nt, synthetic construct
  source 1..21: mol_type = other RNA
  modified_base <1: mod_base = OTHER; note = two inverted abasic nucleosides
  modified_base 1: mod_base = um
  misc_feature 1^2: note = Phosphorothioate bond
  modified_base 2: mod_base = cm
  misc_feature 2^3: note = Phosphorothioate bond
  modified_base 3: mod_base = um
  modified_base 4: mod_base = um
  modified_base 5: mod_base = OTHER; note = 2'-O-methyl-adenosine
  modified_base 6: mod_base = OTHER; note = 2'-O-methyl-adenosine
  modified_base 7: mod_base = cm
  modified_base 8: mod_base = um
  modified_base 9: mod_base = OTHER; note = 2'-Fluoro-uridine
  modified_base 10: mod_base = OTHER; note = 2'-Fluoro-cytidine
  modified_base 11: mod_base = OTHER; note = 2'-Fluoro-guanosine
  modified_base 12: mod_base = cm
  modified_base 13: mod_base = cm
  modified_base 14: mod_base = um
  modified_base 15: mod_base = um
  modified_base 16: mod_base = cm
  modified_base 17: mod_base = OTHER; note = 2'-O-methyl-adenosine
  modified_base 18: mod_base = OTHER; note = 2'-O-methyl-adenosine
  modified_base 19: mod_base = OTHER; note = 2'-O-methyl-adenosine
  modified_base 20: mod_base = gm
  modified_base 21: mod_base = OTHER; note = 2'-O-methyl-adenosine
tcttaacttcgccttcaaaga

SEQ ID NO: 1177 - RNA, 21 nt, synthetic construct
  source 1..21: mol_type = other RNA
  modified_base <1: mod_base = OTHER; note = two inverted abasic nucleosides
  modified_base 1: mod_base = um
  misc_feature 1^2: note = Phosphorothioate bond
  modified_base 2: mod_base = um
  misc_feature 2^3: note = Phosphorothioate bond
  modified_base 3: mod_base = cm
  modified_base 4: mod_base = OTHER; note = 2'-O-methyl-adenosine
  modified_base 5: mod_base = gm
  modified_base 6: mod_base = um
  modified_base 7: mod_base = cm
  modified_base 8: mod_base = OTHER; note = 2'-O-methyl-adenosine
  modified_base 9: mod_base = OTHER; note = 2'-Fluoro-cytidine
  modified_base 10: mod_base = OTHER; note = 2'-Fluoro-uridine
  modified_base 11: mod_base = OTHER; note = 2'-Fluoro-cytidine
  modified_base 12: mod_base = cm
  modified_base 13: mod_base = um
  modified_base 14: mod_base = gm
  modified_base 15: mod_base = OTHER; note = 2'-O-methyl-adenosine
  modified_base 16: mod_base = um
  modified_base 17: mod_base = OTHER; note = 2'-O-methyl-adenosine
  modified_base 18: mod_base = OTHER; note = 2'-O-methyl-adenosine
  modified_base 19: mod_base = OTHER; note = 2'-O-methyl-adenosine
  modified_base 20: mod_base = um
  modified_base 21: mod_base = OTHER; note = 2'-O-methyl-adenosine
ttcagtcactcctgataaata

SEQ ID NO: 1178 - RNA, 21 nt, synthetic construct
  source 1..21: mol_type = other RNA
  modified_base <1: mod_base = OTHER; note = two inverted abasic nucleosides
  modified_base 1: mod_base = cm
  misc_feature 1^2: note = Phosphorothioate bond
  modified_base 2: mod_base = OTHER; note = 2'-O-methyl-adenosine
  misc_feature 2^3: note = Phosphorothioate bond
  modified_base 3: mod_base = gm
  modified_base 4: mod_base = um
  modified_base 5: mod_base = cm
  modified_base 6: mod_base = OTHER; note = 2'-O-methyl-adenosine
  modified_base 7: mod_base = cm
  modified_base 8: mod_base = um
  modified_base 9: mod_base = OTHER; note = 2'-Fluoro-cytidine
  modified_base 10: mod_base = OTHER; note = 2'-Fluoro-cytidine
  modified_base 11: mod_base = OTHER; note = 2'-Fluoro-uridine
  modified_base 12: mod_base = gm
  modified_base 13: mod_base = OTHER; note = 2'-O-methyl-adenosine
  modified_base 14: mod_base = um
  modified_base 15: mod_base = OTHER; note = 2'-O-methyl-adenosine
  modified_base 16: mod_base = OTHER; note = 2'-O-methyl-adenosine
  modified_base 17: mod_base = OTHER; note = 2'-O-methyl-adenosine
  modified_base 18: mod_base = um
  modified_base 19: mod_base = OTHER; note = 2'-O-methyl-adenosine
  modified_base 20: mod_base = OTHER; note = 2'-O-methyl-adenosine
  modified_base 21: mod_base = cm
cagtcactcctgataaataac

SEQ ID NO: 1179 - RNA, 21 nt, synthetic construct
  source 1..21: mol_type = other RNA
  modified_base <1: mod_base = OTHER; note = two inverted abasic nucleosides
  modified_base 1: mod_base = um
  misc_feature 1^2: note = Phosphorothioate bond
  modified_base 2: mod_base = cm
  misc_feature 2^3: note = Phosphorothioate bond
  modified_base 3: mod_base = OTHER; note = 2'-O-methyl-adenosine
  modified_base 4: mod_base = gm
  modified_base 5: mod_base = um
  modified_base 6: mod_base = cm
  modified_base 7: mod_base = OTHER; note = 2'-O-methyl-adenosine
  modified_base 8: mod_base = cm
  modified_base 9: mod_base = OTHER; note = 2'-Fluoro-uridine
  modified_base 10: mod_base = OTHER; note = 2'-Fluoro-cytidine
  modified_base 11: mod_base = OTHER; note = 2'-Fluoro-cytidine
  modified_base 12: mod_base = um
  modified_base 13: mod_base = gm
  modified_base 14: mod_base = OTHER; note = 2'-O-methyl-adenosine
  modified_base 15: mod_base = um
  modified_base 16: mod_base = OTHER; note = 2'-O-methyl-adenosine
  modified_base 17: mod_base = OTHER; note = 2'-O-methyl-adenosine
  modified_base 18: mod_base = OTHER; note = 2'-O-methyl-adenosine
  modified_base 19: mod_base = um
  modified_base 20: mod_base = OTHER; note = 2'-O-methyl-adenosine
  modified_base 21: mod_base = OTHER; note = 2'-O-methyl-adenosine
tcagtcactcctgataaataa

SEQ ID NO: 1180 - RNA, 21 nt, synthetic construct
  source 1..21: mol_type = other RNA
  modified_base <1: mod_base = OTHER; note = two inverted abasic nucleosides
  modified_base 1: mod_base = um
  misc_feature 1^2: note = Phosphorothioate bond
  modified_base 2: mod_base = gm
  misc_feature 2^3: note = Phosphorothioate bond
  modified_base 3: mod_base = OTHER; note = 2'-O-methyl-adenosine
  modified_base 4: mod_base = um
  modified_base 5: mod_base = gm
  modified_base 6: mod_base = gm
  modified_base 7: mod_base = gm
  modified_base 8: mod_base = OTHER; note = 2'-O-methyl-adenosine
  modified_base 9: mod_base = OTHER; note = 2'-Fluoro-cytidine
  modified_base 10: mod_base = OTHER; note = 2'-Fluoro-uridine
  modified_base 11: mod_base = OTHER; note = 2'-Fluoro-cytidine
  modified_base 12: mod_base = OTHER; note = 2'-O-methyl-adenosine
  modified_base 13: mod_base = OTHER; note = 2'-O-methyl-adenosine
  modified_base 14: mod_base = um
  modified_base 15: mod_base = um
  modified_base 16: mod_base = gm
  modified_base 17: mod_base = um
  modified_base 18: mod_base = OTHER; note = 2'-O-methyl-adenosine
  modified_base 19: mod_base = um
  modified_base 20: mod_base = um
  modified_base 21: mod_base = um
tgatgggactcaattgtattt

SEQ ID NO: 1181 - RNA, 21 nt, synthetic construct
  source 1..21: mol_type = other RNA
  modified_base <1: mod_base = OTHER; note = two inverted abasic nucleosides
  modified_base 1: mod_base = gm
  misc_feature 1^2: note = Phosphorothioate bond
  modified_base 2: mod_base = OTHER; note = 2'-O-methyl-adenosine
  misc_feature 2^3: note = Phosphorothioate bond
  modified_base 3: mod_base = um
  modified_base 4: mod_base = gm
  modified_base 5: mod_base = gm
  modified_base 6: mod_base = gm
  modified_base 7: mod_base = OTHER; note = 2'-O-methyl-adenosine
  modified_base 8: mod_base = cm
  modified_base 9: mod_base = OTHER; note = 2'-Fluoro-uridine
  modified_base 10: mod_base = OTHER; note = 2'-Fluoro-cytidine
  modified_base 11: mod_base = OTHER; note = 2'-Fluoro-adenosine
  modified_base 12: mod_base = OTHER; note = 2'-O-methyl-adenosine
  modified_base 13: mod_base = um
  modified_base 14: mod_base = um
  modified_base 15: mod_base = gm
  modified_base 16: mod_base = um
  modified_base 17: mod_base = OTHER; note = 2'-O-methyl-adenosine
  modified_base 18: mod_base = um
  modified_base 19: mod_base = um
  modified_base 20: mod_base = um
  modified_base 21: mod_base = um
gatgggactcaattgtatttt

SEQ ID NO: 1182 - RNA, 21 nt, synthetic construct
  source 1..21: mol_type = other RNA
  modified_base <1: mod_base = OTHER; note = two inverted abasic nucleosides
  modified_base 1: mod_base = cm
  misc_feature 1^2: note = Phosphorothioate bond
  modified_base 2: mod_base = OTHER; note = 2'-O-methyl-adenosine
  misc_feature 2^3: note = Phosphorothioate bond
  modified_base 3: mod_base = cm
  modified_base 4: mod_base = um
  modified_base 5: mod_base = cm
  modified_base 6: mod_base = cm
  modified_base 7: mod_base = um
  modified_base 8: mod_base = gm
  modified_base 9: mod_base = OTHER; note = 2'-Fluoro-adenosine
  modified_base 10: mod_base = OTHER; note = 2'-Fluoro-uridine
  modified_base 11: mod_base = OTHER; note = 2'-Fluoro-adenosine
  modified_base 12: mod_base = OTHER; note = 2'-O-methyl-adenosine
  modified_base 13: mod_base = OTHER; note = 2'-O-methyl-adenosine
  modified_base 14: mod_base = um
  modified_base 15: mod_base = OTHER; note = 2'-O-methyl-adenosine
  modified_base 16: mod_base = OTHER; note = 2'-O-methyl-adenosine
  modified_base 17: mod_base = cm
  modified_base 18: mod_base = OTHER; note = 2'-O-methyl-adenosine
  modified_base 19: mod_base = OTHER; note = 2'-O-methyl-adenosine
  modified_base 20: mod_base = OTHER; note = 2'-O-methyl-adenosine
  modified_base 21: mod_base = um
cactcctgataaataacaaat

SEQ ID NO: 1183 - RNA, 21 nt, synthetic construct
  source 1..21: mol_type = other RNA
  modified_base <1: mod_base = OTHER; note = two inverted abasic nucleosides
  modified_base 1: mod_base = OTHER; note = 2'-O-methyl-adenosine
  misc_feature 1^2: note = Phosphorothioate bond
  modified_base 2: mod_base = um
  misc_feature 2^3: note = Phosphorothioate bond
  modified_base 3: mod_base = um
  modified_base 4: mod_base = cm
  modified_base 5: mod_base = OTHER; note = 2'-O-methyl-adenosine
  modified_base 6: mod_base = um
  modified_base 7: mod_base = cm
  modified_base 8: mod_base = um
  modified_base 9: mod_base = OTHER; note = 2'-Fluoro-guanosine
  modified_base 10: mod_base = OTHER; note = 2'-Fluoro-adenosine
  modified_base 11: mod_base = OTHER; note = 2'-Fluoro-cytidine
  modified_base 12: mod_base = cm
  modified_base 13: mod_base = OTHER; note = 2'-O-methyl-adenosine
  modified_base 14: mod_base = gm
  modified_base 15: mod_base = um
  modified_base 16: mod_base = um
  modified_base 17: mod_base = um
  modified_base 18: mod_base = um
  modified_base 19: mod_base = cm
  modified_base 20: mod_base = um
  modified_base 21: mod_base = cm
attcatctgaccagttttctc

SEQ ID NO: 1184 - RNA, 21 nt, synthetic construct
  source 1..21: mol_type = other RNA
  modified_base <1: mod_base = OTHER; note = two inverted abasic nucleosides
  modified_base 1: mod_base = OTHER; note = 2'-O-methyl-adenosine
  misc_feature 1^2: note = Phosphorothioate bond
  modified_base 2: mod_base = OTHER; note = 2'-O-methyl-adenosine
  misc_feature 2^3: note = Phosphorothioate bond
  modified_base 3: mod_base = cm
  modified_base 4: mod_base = OTHER; note = 2'-O-methyl-adenosine
  modified_base 5: mod_base = gm
  modified_base 6: mod_base = gm
  modified_base 7: mod_base = cm
  modified_base 8: mod_base = OTHER; note = 2'-O-methyl-adenosine
  modified_base 9: mod_base = OTHER; note = 2'-Fluoro-uridine
  modified_base 10: mod_base = OTHER; note = 2'-Fluoro-guanosine
  modified_base 11: mod_base = OTHER; note = 2'-Fluoro-uridine
  modified_base 12: mod_base = um
  modified_base 13: mod_base = gm
  modified_base 14: mod_base = um
  modified_base 15: mod_base = OTHER; note = 2'-O-methyl-adenosine
  modified_base 16: mod_base = um
  modified_base 17: mod_base = um
  modified_base 18: mod_base = OTHER; note = 2'-O-methyl-adenosine
  modified_base 19: mod_base = um
  modified_base 20: mod_base = OTHER; note = 2'-O-methyl-adenosine
  modified_base 21: mod_base = um
aacaggcatgttgtattatat

SEQ ID NO: 1185 - RNA, 21 nt, synthetic construct
  source 1..21: mol_type = other RNA
  modified_base <1: mod_base = OTHER; note = two inverted abasic nucleosides
  modified_base 1: mod_base = OTHER; note = 2'-O-methyl-adenosine
  misc_feature 1^2: note = Phosphorothioate bond
  modified_base 2: mod_base = gm
  misc_feature 2^3: note = Phosphorothioate bond
  modified_base 3: mod_base = gm
  modified_base 4: mod_base = gm
  modified_base 5: mod_base = OTHER; note = 2'-O-methyl-adenosine
  modified_base 6: mod_base = OTHER; note = 2'-O-methyl-adenosine
  modified_base 7: mod_base = um
  modified_base 8: mod_base = gm
  modified_base 9: mod_base = OTHER; note = 2'-Fluoro-cytidine
  modified_base 10: mod_base = OTHER; note = 2'-Fluoro-uridine
  modified_base 11: mod_base = OTHER; note = 2'-Fluoro-uridine
  modified_base 12: mod_base = cm
  modified_base 13: mod_base = cm
  modified_base 14: mod_base = gm
  modified_base 15: mod_base = gm
  modified_base 16: mod_base = OTHER; note = 2'-O-methyl-adenosine
  modified_base 17: mod_base = um
  modified_base 18: mod_base = cm
  modified_base 19: mod_base = cm
  modified_base 20: mod_base = cm
  modified_base 21: mod_base = OTHER; note = 2'-O-methyl-adenosine
agggaatgcttccggatccca

SEQ ID NO: 1186 - RNA, 21 nt, synthetic construct
  source 1..21: mol_type = other RNA
  modified_base <1: mod_base = OTHER; note = two inverted abasic nucleosides
  modified_base 1: mod_base = gm
  misc_feature 1^2: note = Phosphorothioate bond
  modified_base 2: mod_base = gm
  misc_feature 2^3: note = Phosphorothioate bond
  modified_base 3: mod_base = gm
  modified_base 4: mod_base = OTHER; note = 2'-O-methyl-adenosine
  modified_base 5: mod_base = OTHER; note = 2'-O-methyl-adenosine
  modified_base 6: mod_base = um
  modified_base 7: mod_base = gm
  modified_base 8: mod_base = cm
  modified_base 9: mod_base = OTHER; note = 2'-Fluoro-uridine
  modified_base 10: mod_base = OTHER; note = 2'-Fluoro-uridine
  modified_base 11: mod_base = OTHER; note = 2'-Fluoro-cytidine
  modified_base 12: mod_base = cm
  modified_base 13: mod_base = gm
  modified_base 14: mod_base = gm
  modified_base 15: mod_base = OTHER; note = 2'-O-methyl-adenosine
  modified_base 16: mod_base = um
  modified_base 17: mod_base = cm
  modified_base 18: mod_base = cm
  modified_base 19: mod_base = cm
  modified_base 20: mod_base = OTHER; note = 2'-O-methyl-adenosine
  modified_base 21: mod_base = OTHER; note = 2'-O-methyl-adenosine
gggaatgcttccggatcccaa

SEQ ID NO: 1187 - RNA, 21 nt, synthetic construct
  source 1..21: mol_type = other RNA
  modified_base <1: mod_base = OTHER; note = two inverted abasic nucleosides
  modified_base 1: mod_base = cm
  misc_feature 1^2: note = Phosphorothioate bond
  modified_base 2: mod_base = gm
  misc_feature 2^3: note = Phosphorothioate bond
  modified_base 3: mod_base = OTHER; note = 2'-O-methyl-adenosine
  modified_base 4: mod_base = gm
  modified_base 5: mod_base = gm
  modified_base 6: mod_base = cm
  modified_base 7: mod_base = cm
  modified_base 8: mod_base = um
  modified_base 9: mod_base = OTHER; note = 2'-Fluoro-cytidine
  modified_base 10: mod_base = OTHER; note = 2'-Fluoro-guanosine
  modified_base 11: mod_base = OTHER; note = 2'-Fluoro-guanosine
  modified_base 12: mod_base = um
  modified_base 13: mod_base = gm
  modified_base 14: mod_base = OTHER; note = 2'-O-methyl-adenosine
  modified_base 15: mod_base = cm
  modified_base 16: mod_base = um
  modified_base 17: mod_base = gm
  modified_base 18: mod_base = cm
  modified_base 19: mod_base = cm
  modified_base 20: mod_base = um
  modified_base 21: mod_base = gm
cgaggcctcggtgactgcctg

SEQ ID NO: 1188 - RNA, 21 nt, synthetic construct
  source 1..21: mol_type = other RNA
  modified_base <1: mod_base = OTHER; note = two inverted abasic nucleosides
  modified_base 1: mod_base = OTHER; note = 2'-O-methyl-adenosine
  misc_feature 1^2: note = Phosphorothioate bond
  modified_base 2: mod_base = cm
  misc_feature 2^3: note = Phosphorothioate bond
  modified_base 3: mod_base = OTHER; note = 2'-O-methyl-adenosine
  modified_base 4: mod_base = gm
  modified_base 5: mod_base = gm
  modified_base 6: mod_base = cm
  modified_base 7: mod_base = OTHER; note = 2'-O-methyl-adenosine
  modified_base 8: mod_base = um
  modified_base 9: mod_base = OTHER; note = 2'-Fluoro-guanosine
  modified_base 10: mod_base = OTHER; note = 2'-Fluoro-uridine
  modified_base 11: mod_base = OTHER; note = 2'-Fluoro-uridine
  modified_base 12: mod_base = gm
  modified_base 13: mod_base = um
  modified_base 14: mod_base = OTHER; note = 2'-O-methyl-adenosine
  modified_base 15: mod_base = um
  modified_base 16: mod_base = um
  modified_base 17: mod_base = OTHER; note = 2'-O-methyl-adenosine
  modified_base 18: mod_base = um
  modified_base 19: mod_base = OTHER; note = 2'-O-methyl-adenosine
  modified_base 20: mod_base = um
  modified_base 21: mod_base = OTHER; note = 2'-O-methyl-adenosine
acaggcatgttgtattatata

SEQ ID NO: 1189 - RNA, 21 nt, synthetic construct
  source 1..21: mol_type = other RNA
  modified_base <1: mod_base = OTHER; note = two inverted abasic nucleosides
  modified_base 1: mod_base = OTHER; note = 2'-O-methyl-adenosine
  misc_feature 1^2: note = Phosphorothioate bond
  modified_base 2: mod_base = OTHER; note = 2'-O-methyl-adenosine
  misc_feature 2^3: note = Phosphorothioate bond
  modified_base 3: mod_base = um
  modified_base 4: mod_base = OTHER; note = 2'-O-methyl-adenosine
  modified_base 5: mod_base = cm
  modified_base 6: mod_base = OTHER; note = 2'-O-methyl-adenosine
  modified_base 7: mod_base = OTHER; note = 2'-O-methyl-adenosine
  modified_base 8: mod_base = OTHER; note = 2'-O-methyl-adenosine
  modified_base 9: mod_base = OTHER; note = 2'-Fluoro-guanosine
  modified_base 10: mod_base = OTHER; note = 2'-Fluoro-guanosine
  modified_base 11: mod_base = OTHER; note = 2'-Fluoro-cytidine
  modified_base 12: mod_base = OTHER; note = 2'-O-methyl-adenosine
  modified_base 13: mod_base = um
  modified_base 14: mod_base = um
  modified_base 15: mod_base = OTHER; note = 2'-O-methyl-adenosine
  modified_base 16: mod_base = um
  modified_base 17: mod_base = OTHER; note = 2'-O-methyl-adenosine
  modified_base 18: mod_base = gm
  modified_base 19: mod_base = OTHER; note = 2'-O-methyl-adenosine
  modified_base 20: mod_base = cm
  modified_base 21: mod_base = um
aatacaaaggcattatagact

SEQ ID NO: 1190 - RNA, 21 nt, synthetic construct
  source 1..21: mol_type = other RNA
  modified_base <1: mod_base = OTHER; note = two inverted abasic nucleosides
  modified_base 1: mod_base = OTHER; note = 2'-O-methyl-adenosine
  misc_feature 1^2: note = Phosphorothioate bond
  modified_base 2: mod_base = um
  misc_feature 2^3: note = Phosphorothioate bond
  modified_base 3: mod_base = um
  modified_base 4: mod_base = um
  modified_base 5: mod_base = cm
  modified_base 6: mod_base = OTHER; note = 2'-O-methyl-adenosine
  modified_base 7: mod_base = gm
  modified_base 8: mod_base = um
  modified_base 9: mod_base = OTHER; note = 2'-Fluoro-cytidine
  modified_base 10: mod_base = OTHER; note = 2'-Fluoro-adenosine
  modified_base 11: mod_base = OTHER; note = 2'-Fluoro-cytidine
  modified_base 12: mod_base = um
  modified_base 13: mod_base = cm
  modified_base 14: mod_base = cm
  modified_base 15: mod_base = um
  modified_base 16: mod_base = gm
  modified_base 17: mod_base = OTHER; note = 2'-O-methyl-adenosine
  modified_base 18: mod_base = um
  modified_base 19: mod_base = OTHER; note = 2'-O-methyl-adenosine
  modified_base 20: mod_base = OTHER; note = 2'-O-methyl-adenosine
  modified_base 21: mod_base = OTHER; note = 2'-O-methyl-adenosine
atttcagtcactcctgataaa

SEQ ID NO: 1191 - RNA, 21 nt, synthetic construct
  source 1..21: mol_type = other RNA
  modified_base <1: mod_base = OTHER; note = two inverted abasic nucleosides
  modified_base 1: mod_base = OTHER; note = 2'-O-methyl-adenosine
  misc_feature 1^2: note = Phosphorothioate bond
  modified_base 2: mod_base = um
  misc_feature 2^3: note = Phosphorothioate bond
  modified_base 3: mod_base = gm
  modified_base 4: mod_base = OTHER; note = 2'-O-methyl-adenosine
  modified_base 5: mod_base = um
  modified_base 6: mod_base = gm
  modified_base 7: mod_base = gm
  modified_base 8: mod_base = gm
  modified_base 9: mod_base = OTHER; note = 2'-Fluoro-adenosine
  modified_base 10: mod_base = OTHER; note = 2'-Fluoro-cytidine
  modified_base 11: mod_base = OTHER; note = 2'-Fluoro-uridine
  modified_base 12: mod_base = cm
  modified_base 13: mod_base = OTHER; note = 2'-O-methyl-adenosine
  modified_base 14: mod_base = OTHER; note = 2'-O-methyl-adenosine
  modified_base 15: mod_base = um
  modified_base 16: mod_base = um
  modified_base 17: mod_base = gm
  modified_base 18: mod_base = um
  modified_base 19: mod_base = OTHER; note = 2'-O-methyl-adenosine
  modified_base 20: mod_base = um
  modified_base 21: mod_base = um
atgatgggactcaattgtatt

SEQ ID NO: 1192 - RNA, 21 nt, synthetic construct
  source 1..21: mol_type = other RNA
  modified_base <1: mod_base = OTHER; note = two inverted abasic nucleosides
  modified_base 1: mod_base = cm
  misc_feature 1^2: note = Phosphorothioate bond
  modified_base 2: mod_base = um
  misc_feature 2^3: note = Phosphorothioate bond
  modified_base 3: mod_base = gm
  modified_base 4: mod_base = OTHER; note = 2'-O-methyl-adenosine
  modified_base 5: mod_base = cm
  modified_base 6: mod_base = cm
  modified_base 7: mod_base = OTHER; note = 2'-O-methyl-adenosine
  modified_base 8: mod_base = gm
  modified_base 9: mod_base = OTHER; note = 2'-Fluoro-uridine
  modified_base 10: mod_base = OTHER; note = 2'-Fluoro-uridine
  modified_base 11: mod_base = OTHER; note = 2'-Fluoro-uridine
  modified_base 12: mod_base = um
  modified_base 13: mod_base = cm
  modified_base 14: mod_base = um
  modified_base 15: mod_base = cm
  modified_base 16: mod_base = um
  modified_base 17: mod_base = um
  modified_base 18: mod_base = OTHER; note = 2'-O-methyl-adenosine
  modified_base 19: mod_base = OTHER; note = 2'-O-methyl-adenosine
  modified_base 20: mod_base = OTHER; note = 2'-O-methyl-adenosine
  modified_base 21: mod_base = gm
ctgaccagttttctcttaaag

SEQ ID NO: 1193 - RNA, 21 nt, synthetic construct
  source 1..21: mol_type = other RNA
  modified_base <1: mod_base = OTHER; note = two inverted abasic nucleosides
  modified_base 1: mod_base = um
  misc_feature 1^2: note = Phosphorothioate bond
  modified_base 2: mod_base = gm
  misc_feature 2^3: note = Phosphorothioate bond
  modified_base 3: mod_base = OTHER; note = 2'-O-methyl-adenosine
  modified_base 4: mod_base = cm
  modified_base 5: mod_base = cm
  modified_base 6: mod_base = OTHER; note = 2'-O-methyl-adenosine
  modified_base 7: mod_base = gm
  modified_base 8: mod_base = um
  modified_base 9: mod_base = OTHER; note = 2'-Fluoro-uridine
  modified_base 10: mod_base = OTHER; note = 2'-Fluoro-uridine
  modified_base 11: mod_base = OTHER; note = 2'-Fluoro-uridine
  modified_base 12: mod_base = cm
  modified_base 13: mod_base = um
  modified_base 14: mod_base = cm
  modified_base 15: mod_base = um
  modified_base 16: mod_base = um
  modified_base 17: mod_base = OTHER; note = 2'-O-methyl-adenosine
  modified_base 18: mod_base = OTHER; note = 2'-O-methyl-adenosine
  modified_base 19: mod_base = OTHER; note = 2'-O-methyl-adenosine
  modified_base 20: mod_base = gm
  modified_base 21: mod_base = cm
tgaccagttttctcttaaagc

SEQ ID NO: 1194 - RNA, 21 nt, synthetic construct
  source 1..21: mol_type = other RNA
  modified_base <1: mod_base = OTHER; note = two inverted abasic nucleosides
  modified_base 1: mod_base = gm
  misc_feature 1^2: note = Phosphorothioate bond
  modified_base 2: mod_base = OTHER; note = 2'-O-methyl-adenosine
  misc_feature 2^3: note = Phosphorothioate bond
  modified_base 3: mod_base = um
  modified_base 4: mod_base = OTHER; note = 2'-O-methyl-adenosine
  modified_base 5: mod_base = OTHER; note = 2'-O-methyl-adenosine
  modified_base 6: mod_base = gm
  modified_base 7: mod_base = cm
  modified_base 8: mod_base = OTHER; note = 2'-O-methyl-adenosine
  modified_base 9: mod_base = OTHER; note = 2'-Fluoro-adenosine
  modified_base 10: mod_base = OTHER; note = 2'-Fluoro-uridine
  modified_base 11: mod_base = OTHER; note = 2'-Fluoro-adenosine
  modified_base 12: mod_base = cm
  modified_base 13: mod_base = OTHER; note = 2'-O-methyl-adenosine
  modified_base 14: mod_base = OTHER; note = 2'-O-methyl-adenosine
  modified_base 15: mod_base = OTHER; note = 2'-O-methyl-adenosine
  modified_base 16: mod_base = gm
  modified_base 17: mod_base = gm
  modified_base 18: mod_base = cm
  modified_base 19: mod_base = OTHER; note = 2'-O-methyl-adenosine
  modified_base 20: mod_base = um
  modified_base 21: mod_base = um
gataagcaatacaaaggcatt

SEQ ID NO: 1195 - RNA, 21 nt, synthetic construct
  source 1..21: mol_type = other RNA
  modified_base <1: mod_base = OTHER; note = two inverted abasic nucleosides
  modified_base 1: mod_base = OTHER; note = 2'-O-methyl-adenosine
  misc_feature 1^2: note = Phosphorothioate bond
  modified_base 2: mod_base = um
  misc_feature 2^3: note = Phosphorothioate bond
  modified_base 3: mod_base = OTHER; note = 2'-O-methyl-adenosine
  modified_base 4: mod_base = OTHER; note = 2'-O-methyl-adenosine
  modified_base 5: mod_base = gm
  modified_base 6: mod_base = cm
  modified_base 7: mod_base = OTHER; note = 2'-O-methyl-adenosine
  modified_base 8: mod_base = OTHER; note = 2'-O-methyl-adenosine
  modified_base 9: mod_base = OTHER; note = 2'-Fluoro-uridine
  modified_base 10: mod_base = OTHER; note = 2'-Fluoro-adenosine
  modified_base 11: mod_base = OTHER; note = 2'-Fluoro-cytidine
  modified_base 12: mod_base = OTHER; note = 2'-O-methyl-adenosine
  modified_base 13: mod_base = OTHER; note = 2'-O-methyl-adenosine
  modified_base 14: mod_base = OTHER; note = 2'-O-methyl-adenosine
  modified_base 15: mod_base = gm
  modified_base 16: mod_base = gm
  modified_base 17: mod_base = cm
  modified_base 18: mod_base = OTHER; note = 2'-O-methyl-adenosine
  modified_base 19: mod_base = um
  modified_base 20: mod_base = um
  modified_base 21: mod_base = OTHER; note = 2'-O-methyl-adenosine
ataagcaatacaaaggcatta

SEQ ID NO: 1196 - RNA, 21 nt, synthetic construct
  source 1..21: mol_type = other RNA
  modified_base <1: mod_base = OTHER; note = two inverted abasic nucleosides
  modified_base 1: mod_base = um
  misc_feature 1^2: note = Phosphorothioate bond
  modified_base 2: mod_base = um
  misc_feature 2^3: note = Phosphorothioate bond
  modified_base 3: mod_base = OTHER; note = 2'-O-methyl-adenosine
  modified_base 4: mod_base = OTHER; note = 2'-O-methyl-adenosine
  modified_base 5: mod_base = cm
  modified_base 6: mod_base = gm
  modified_base 7: mod_base = um
  modified_base 8: mod_base = gm
  modified_base 9: mod_base = OTHER; note = 2'-Fluoro-uridine
  modified_base 10: mod_base = OTHER; note = 2'-Fluoro-cytidine
  modified_base 11: mod_base = OTHER; note = 2'-Fluoro-uridine
  modified_base 12: mod_base = gm
  modified_base 13: mod_base = um
  modified_base 14: mod_base = gm
  modified_base 15: mod_base = cm
  modified_base 16: mod_base = OTHER; note = 2'-O-methyl-adenosine
  modified_base 17: mod_base = gm
  modified_base 18: mod_base = gm
  modified_base 19: mod_base = gm
  modified_base 20: mod_base = um
  modified_base 21: mod_base = OTHER; note = 2'-O-methyl-adenosine
ttaacgtgtctgtgcagggta

SEQ ID NO: 1197 - RNA, 21 nt, synthetic construct
  source 1..21: mol_type = other RNA
  modified_base <1: mod_base = OTHER; note = two inverted abasic nucleosides
  modified_base 1: mod_base = um
  misc_feature 1^2: note = Phosphorothioate bond
  modified_base 2: mod_base = OTHER; note = 2'-O-methyl-adenosine
  misc_feature 2^3: note = Phosphorothioate bond
  modified_base 3: mod_base = OTHER; note = 2'-O-methyl-adenosine
  modified_base 4: mod_base = cm
  modified_base 5: mod_base = gm
  modified_base 6: mod_base = um
  modified_base 7: mod_base = gm
  modified_base 8: mod_base = um
  modified_base 9: mod_base = OTHER; note = 2'-Fluoro-cytidine
  modified_base 10: mod_base = OTHER; note = 2'-Fluoro-uridine
  modified_base 11: mod_base = OTHER; note = 2'-Fluoro-guanosine
  modified_base 12: mod_base = um
  modified_base 13: mod_base = gm
  modified_base 14: mod_base = cm
  modified_base 15: mod_base = OTHER; note = 2'-O-methyl-adenosine
  modified_base 16: mod_base = gm
  modified_base 17: mod_base = gm
  modified_base 18: mod_base = gm
  modified_base 19: mod_base = um
  modified_base 20: mod_base = OTHER; note = 2'-O-methyl-adenosine
  modified_base 21: mod_base = um
taacgtgtctgtgcagggtat

SEQ ID NO: 1198 - RNA, 21 nt, synthetic construct
  source 1..21: mol_type = other RNA
  modified_base <1: mod_base = OTHER; note = two inverted abasic nucleosides
  modified_base 1: mod_base = um
  misc_feature 1^2: note = Phosphorothioate bond
  modified_base 2: mod_base = cm
  misc_feature 2^3: note = Phosphorothioate bond
  modified_base 3: mod_base = OTHER; note = 2'-O-methyl-adenosine
  modified_base 4: mod_base = cm
  modified_base 5: mod_base = OTHER; note = 2'-O-methyl-adenosine
  modified_base 6: mod_base = um
  modified_base 7: mod_base = cm
  modified_base 8: mod_base = gm
  modified_base 9: mod_base = OTHER; note = 2'-Fluoro-uridine
  modified_base 10: mod_base = OTHER; note = 2'-Fluoro-cytidine
  modified_base 11: mod_base = OTHER; note = 2'-Fluoro-adenosine
  modified_base 12: mod_base = um
  modified_base 13: mod_base = cm
  modified_base 14: mod_base = OTHER; note = 2'-O-methyl-adenosine
  modified_base 15: mod_base = gm
  modified_base 16: mod_base = cm
  modified_base 17: mod_base = um
  modified_base 18: mod_base = gm
  modified_base 19: mod_base = gm
  modified_base 20: mod_base = OTHER; note = 2'-O-methyl-adenosine
  modified_base 21: mod_base = um
tcacatcgtcatcagctggat

SEQ ID NO: 1199 - RNA, 21 nt, synthetic construct
  source 1..21: mol_type = other RNA
  modified_base <1: mod_base = OTHER; note = two inverted abasic nucleosides
  modified_base 1: mod_base = um
  misc_feature 1^2: note = Phosphorothioate bond
  modified_base 2: mod_base = gm
  misc_feature 2^3: note = Phosphorothioate bond
  modified_base 3: mod_base = OTHER; note = 2'-O-methyl-adenosine
  modified_base 4: mod_base = um
  modified_base 5: mod_base = gm
  modified_base 6: mod_base = OTHER; note = 2'-O-methyl-adenosine
  modified_base 7: mod_base = um
  modified_base 8: mod_base = gm
  modified_base 9: mod_base = OTHER; note = 2'-Fluoro-guanosine
  modified_base 10: mod_base = OTHER; note = 2'-Fluoro-guanosine
  modified_base 11: mod_base = OTHER; note = 2'-Fluoro-adenosine
  modified_base 12: mod_base = cm
  modified_base 13: mod_base = um
  modified_base 14: mod_base = cm
  modified_base 15: mod_base = OTHER; note = 2'-O-methyl-adenosine
  modified_base 16: mod_base = OTHER; note = 2'-O-methyl-adenosine
  modified_base 17: mod_base = um
  modified_base 18: mod_base = um
  modified_base 19: mod_base = gm
  modified_base 20: mod_base = um
  modified_base 21: mod_base = OTHER; note = 2'-O-methyl-adenosine
tgatgatgggactcaattgta

SEQ ID NO: 1200 - RNA, 21 nt, synthetic construct
  source 1..21: mol_type = other RNA
  modified_base <1: mod_base = OTHER; note = two inverted abasic nucleosides
  modified_base 1: mod_base = OTHER; note = 2'-O-methyl-adenosine
  misc_feature 1^2: note = Phosphorothioate bond
  modified_base 2: mod_base = cm
  misc_feature 2^3: note = Phosphorothioate bond
  modified_base 3: mod_base = um
  modified_base 4: mod_base = gm
  modified_base 5: mod_base = cm
  modified_base 6: mod_base = gm
  modified_base 7: mod_base = um
  modified_base 8: mod_base = gm
  modified_base 9: mod_base = OTHER; note = 2'-Fluoro-guanosine
  modified_base 10: mod_base = OTHER; note = 2'-Fluoro-uridine
  modified_base 11: mod_base = OTHER; note = 2'-Fluoro-cytidine
  modified_base 12: mod_base = cm
  modified_base 13: mod_base = gm
  modified_base 14: mod_base = um
  modified_base 15: mod_base = OTHER; note = 2'-O-methyl-adenosine
  modified_base 16: mod_base = um
  modified_base 17: mod_base = um
  modified_base 18: mod_base = cm
  modified_base 19: mod_base = cm
  modified_base 20: mod_base = cm
  modified_base 21: mod_base = OTHER; note = 2'-O-methyl-adenosine
actgcgtggtccgtattccca

SEQ ID NO: 1201 - RNA, 21 nt, synthetic construct
  source 1..21: mol_type = other RNA
  modified_base <1: mod_base = OTHER; note = two inverted abasic nucleosides
  modified_base 1: mod_base = gm
  misc_feature 1^2: note = Phosphorothioate bond
  modified_base 2: mod_base = OTHER; note = 2'-O-methyl-adenosine
  misc_feature 2^3: note = Phosphorothioate bond
  modified_base 3: mod_base = OTHER; note = 2'-O-methyl-adenosine
  modified_base 4: mod_base = cm
  modified_base 5: mod_base = OTHER; note = 2'-O-methyl-adenosine
  modified_base 6: mod_base = gm
  modified_base 7: mod_base = gm
  modified_base 8: mod_base = cm
  modified_base 9: mod_base = OTHER; note = 2'-Fluoro-adenosine
  modified_base 10: mod_base = OTHER; note = 2'-Fluoro-uridine
  modified_base 11: mod_base = OTHER; note = 2'-Fluoro-guanosine
  modified_base 12: mod_base = um
  modified_base 13: mod_base = um
  modified_base 14: mod_base = gm
  modified_base 15: mod_base = um
  modified_base 16: mod_base = OTHER; note = 2'-O-methyl-adenosine
  modified_base 17: mod_base = um
  modified_base 18: mod_base = um
  modified_base 19: mod_base = OTHER; note = 2'-O-methyl-adenosine
  modified_base 20: mod_base = um
  modified_base 21: mod_base = OTHER; note = 2'-O-methyl-adenosine
gaacaggcatgttgtattata

SEQ ID NO: 1202 - RNA, 21 nt, synthetic construct
  source 1..21: mol_type = other RNA
  modified_base <1: mod_base = OTHER; note = two inverted abasic nucleosides
  modified_base 1: mod_base = um
  misc_feature 1^2: note = Phosphorothioate bond
  modified_base 2: mod_base = OTHER; note = 2'-O-methyl-adenosine
  misc_feature 2^3: note = Phosphorothioate bond
  modified_base 3: mod_base = um
  modified_base 4: mod_base = um
  modified_base 5: mod_base = um
  modified_base 6: mod_base = cm
  modified_base 7: mod_base = OTHER; note = 2'-O-methyl-adenosine
  modified_base 8: mod_base = gm
  modified_base 9: mod_base = OTHER; note = 2'-Fluoro-uridine
  modified_base 10: mod_base = OTHER; note = 2'-Fluoro-cytidine
  modified_base 11: mod_base = OTHER; note = 2'-Fluoro-adenosine
  modified_base 12: mod_base = cm
  modified_base 13: mod_base = um
  modified_base 14: mod_base = cm
  modified_base 15: mod_base = cm
  modified_base 16: mod_base = um
  modified_base 17: mod_base = gm
  modified_base 18: mod_base = OTHER; note = 2'-O-methyl-adenosine
  modified_base 19: mod_base = um
  modified_base 20: mod_base = OTHER; note = 2'-O-methyl-adenosine
  modified_base 21: mod_base = OTHER; note = 2'-O-methyl-adenosine
tatttcagtcactcctgataa

SEQ ID NO: 1203 - RNA, 21 nt, synthetic construct
  source 1..21: mol_type = other RNA
  modified_base <1: mod_base = OTHER; note = two inverted abasic nucleosides
  modified_base 1: mod_base = um
  misc_feature 1^2: note = Phosphorothioate bond
  modified_base 2: mod_base = OTHER; note = 2'-O-methyl-adenosine
  misc_feature 2^3: note = Phosphorothioate bond
  modified_base 3: mod_base = OTHER; note = 2'-O-methyl-adenosine
  modified_base 4: mod_base = gm
  modified_base 5: mod_base = cm
  modified_base 6: mod_base = OTHER; note = 2'-O-methyl-adenosine
  modified_base 7: mod_base = OTHER; note = 2'-O-methyl-adenosine
  modified_base 8: mod_base = um
  modified_base 9: mod_base = OTHER; note = 2'-Fluoro-adenosine
  modified_base 10: mod_base = OTHER; note = 2'-Fluoro-cytidine
  modified_base 11: mod_base = OTHER; note = 2'-Fluoro-adenosine
  modified_base 12: mod_base = OTHER; note = 2'-O-methyl-adenosine
  modified_base 13: mod_base = OTHER; note = 2'-O-methyl-adenosine
  modified_base 14: mod_base = gm
  modified_base 15: mod_base = gm
  modified_base 16: mod_base = cm
  modified_base 17: mod_base = OTHER; note = 2'-O-methyl-adenosine
  modified_base 18: mod_base = um
  modified_base 19: mod_base = um
  modified_base 20: mod_base = OTHER; note = 2'-O-methyl-adenosine
  modified_base 21: mod_base = um
taagcaatacaaaggcattat

SEQ ID NO: 1204 - RNA, 21 nt, synthetic construct
  source 1..21: mol_type = other RNA
  modified_base <1: mod_base = OTHER; note = two inverted abasic nucleosides
  modified_base 1: mod_base = OTHER; note = 2'-O-methyl-adenosine
  misc_feature 1^2: note = Phosphorothioate bond
  modified_base 2: mod_base = cm
  misc_feature 2^3: note = Phosphorothioate bond
  modified_base 3: mod_base = um
  modified_base 4: mod_base = cm
  modified_base 5: mod_base = OTHER; note = 2'-O-methyl-adenosine
  modified_base 6: mod_base = cm
  modified_base 7: mod_base = OTHER; note = 2'-O-methyl-adenosine
  modified_base 8: mod_base = um
  modified_base 9: mod_base = OTHER; note = 2'-Fluoro-cytidine
  modified_base 10: mod_base = OTHER; note = 2'-Fluoro-guanosine
  modified_base 11: mod_base = OTHER; note = 2'-Fluoro-uridine
  modified_base 12: mod_base = cm
  modified_base 13: mod_base = OTHER; note = 2'-O-methyl-adenosine
  modified_base 14: mod_base = um
  modified_base 15: mod_base = cm
  modified_base 16: mod_base = OTHER; note = 2'-O-methyl-adenosine
  modified_base 17: mod_base = gm
  modified_base 18: mod_base = cm
  modified_base 19: mod_base = um
  modified_base 20: mod_base = gm
  modified_base 21: mod_base = gm
actcacatcgtcatcagctgg

SEQ ID NO: 1205 - RNA, 21 nt, synthetic construct
  source 1..21: mol_type = other RNA
  modified_base <1: mod_base = OTHER; note = two inverted abasic nucleosides
  modified_base 1: mod_base = cm
  misc_feature 1^2: note = Phosphorothioate bond
  modified_base 2: mod_base = cm
  misc_feature 2^3: note = Phosphorothioate bond
  modified_base 3: mod_base = gm
  modified_base 4: mod_base = cm
  modified_base 5: mod_base = cm
  modified_base 6: mod_base = um
  modified_base 7: mod_base = OTHER; note = 2'-O-methyl-adenosine
  modified_base 8: mod_base = cm
  modified_base 9: mod_base = OTHER; note = 2'-Fluoro-uridine
  modified_base 10: mod_base = OTHER; note = 2'-Fluoro-uridine
  modified_base 11: mod_base = OTHER; note = 2'-Fluoro-cytidine
  modified_base 12: mod_base = gm
  modified_base 13: mod_base = gm
  modified_base 14: mod_base = um
  modified_base 15: mod_base = OTHER; note = 2'-O-methyl-adenosine
  modified_base 16: mod_base = um
  modified_base 17: mod_base = cm
  modified_base 18: mod_base = um
  modified_base 19: mod_base = OTHER; note = 2'-O-methyl-adenosine
  modified_base 20: mod_base = um
  modified_base 21: mod_base = gm
ccgcctacttcggtatctatg

SEQ ID NO: 1206 - RNA, 21 nt, synthetic construct
  source 1..21: mol_type = other RNA
  modified_base <1: mod_base = OTHER; note = two inverted abasic nucleosides
  modified_base 1: mod_base = cm
  misc_feature 1^2: note = Phosphorothioate bond
  modified_base 2: mod_base = OTHER; note = 2'-O-methyl-adenosine
  misc_feature 2^3: note = Phosphorothioate bond
  modified_base 3: mod_base = cm
  modified_base 4: mod_base = OTHER; note = 2'-O-methyl-adenosine
  modified_base 5: mod_base = um
  modified_base 6: mod_base = cm
  modified_base 7: mod_base = gm
  modified_base 8: mod_base = um
  modified_base 9: mod_base = OTHER; note = 2'-Fluoro-cytidine
  modified_base 10: mod_base = OTHER; note = 2'-Fluoro-adenosine
  modified_base 11: mod_base = OTHER; note = 2'-Fluoro-uridine
  modified_base 12: mod_base = cm
  modified_base 13: mod_base = OTHER; note = 2'-O-methyl-adenosine
  modified_base 14: mod_base = gm
  modified_base 15: mod_base = cm
  modified_base 16: mod_base = um
  modified_base 17: mod_base = gm
  modified_base 18: mod_base = gm
  modified_base 19: mod_base = OTHER; note = 2'-O-methyl-adenosine
  modified_base 20: mod_base = um
  modified_base 21: mod_base = gm
cacatcgtcatcagctggatg

SEQ ID NO: 1207 - RNA, 21 nt, synthetic construct
  source 1..21: mol_type = other RNA
  modified_base <1: mod_base = OTHER; note = two inverted abasic nucleosides
  modified_base 1: mod_base = gm
  misc_feature 1^2: note = Phosphorothioate bond
  modified_base 2: mod_base = cm
  misc_feature 2^3: note = Phosphorothioate bond
  modified_base 3: mod_base = cm
  modified_base 4: mod_base = um
  modified_base 5: mod_base = OTHER; note = 2'-O-methyl-adenosine
  modified_base 6: mod_base = cm
  modified_base 7: mod_base = um
  modified_base 8: mod_base = um
  modified_base 9: mod_base = OTHER; note = 2'-Fluoro-cytidine
  modified_base 10: mod_base = OTHER; note = 2'-Fluoro-guanosine
  modified_base 11: mod_base = OTHER; note = 2'-Fluoro-guanosine
  modified_base 12: mod_base = um
  modified_base 13: mod_base = OTHER; note = 2'-O-methyl-adenosine
  modified_base 14: mod_base = um
  modified_base 15: mod_base = cm
  modified_base 16: mod_base = um
  modified_base 17: mod_base = OTHER; note = 2'-O-methyl-adenosine
  modified_base 18: mod_base = um
  modified_base 19: mod_base = gm
  modified_base 20: mod_base = OTHER; note = 2'-O-methyl-adenosine
  modified_base 21: mod_base = cm
gcctacttcggtatctatgac

SEQ ID NO: 1208 - RNA, 21 nt, synthetic construct
  source 1..21: mol_type = other RNA
  modified_base <1: mod_base = OTHER; note = two inverted abasic nucleosides
  modified_base 1: mod_base = um
  misc_feature 1^2: note = Phosphorothioate bond
  modified_base 2: mod_base = um
  misc_feature 2^3: note = Phosphorothioate bond
  modified_base 3: mod_base = um
  modified_base 4: mod_base = OTHER; note = 2'-O-methyl-adenosine
  modified_base 5: mod_base = OTHER; note = 2'-O-methyl-adenosine
  modified_base 6: mod_base = cm
  modified_base 7: mod_base = gm
  modified_base 8: mod_base = um
  modified_base 9: mod_base = OTHER; note = 2'-Fluoro-guanosine
  modified_base 10: mod_base = OTHER; note = 2'-Fluoro-uridine
  modified_base 11: mod_base = OTHER; note = 2'-Fluoro-cytidine
  modified_base 12: mod_base = um
  modified_base 13: mod_base = gm
  modified_base 14: mod_base = um
  modified_base 15: mod_base = gm
  modified_base 16: mod_base = cm
  modified_base 17: mod_base = OTHER; note = 2'-O-methyl-adenosine
  modified_base 18: mod_base = gm
  modified_base 19: mod_base = gm
  modified_base 20: mod_base = gm
  modified_base 21: mod_base = um
tttaacgtgtctgtgcagggt

SEQ ID NO: 1209 - RNA, 21 nt, synthetic construct
  source 1..21: mol_type = other RNA
  modified_base <1: mod_base = OTHER; note = two inverted abasic nucleosides
  modified_base 1: mod_base = um
  misc_feature 1^2: note = Phosphorothioate bond
  modified_base 2: mod_base = cm
  misc_feature 2^3: note = Phosphorothioate bond
  modified_base 3: mod_base = gm
  modified_base 4: mod_base = cm
  modified_base 5: mod_base = cm
  modified_base 6: mod_base = gm
  modified_base 7: mod_base = cm
  modified_base 8: mod_base = cm
  modified_base 9: mod_base = OTHER; note = 2'-Fluoro-guanosine
  modified_base 10: mod_base = OTHER; note = 2'-Fluoro-cytidine
  modified_base 11: mod_base = OTHER; note = 2'-Fluoro-adenosine
  modified_base 12: mod_base = um
  modified_base 13: mod_base = gm
  modified_base 14: mod_base = OTHER; note = 2'-O-methyl-adenosine
  modified_base 15: mod_base = um
  modified_base 16: mod_base = gm
  modified_base 17: mod_base = OTHER; note = 2'-O-methyl-adenosine
  modified_base 18: mod_base = um
  modified_base 19: mod_base = gm
  modified_base 20: mod_base = cm
  modified_base 21: mod_base = OTHER; note = 2'-O-methyl-adenosine
tcgccgccgcatgatgatgca

SEQ ID NO: 1210 - RNA, 21 nt, synthetic construct
  source 1..21: mol_type = other RNA
  modified_base <1: mod_base = OTHER; note = two inverted abasic nucleosides
  modified_base 1: mod_base = cm
  misc_feature 1^2: note = Phosphorothioate bond
  modified_base 2: mod_base = OTHER; note = 2'-O-methyl-adenosine
  misc_feature 2^3: note = Phosphorothioate bond
  modified_base 3: mod_base = um
  modified_base 4: mod_base = um
  modified_base 5: mod_base = OTHER; note = 2'-O-methyl-adenosine
  modified_base 6: mod_base = um
  modified_base 7: mod_base = OTHER; note = 2'-O-methyl-adenosine
  modified_base 8: mod_base = gm
  modified_base 9: mod_base = OTHER; note = 2'-Fluoro-adenosine
  modified_base 10: mod_base = OTHER; note = 2'-Fluoro-cytidine
  modified_base 11: mod_base = OTHER; note = 2'-Fluoro-uridine
  modified_base 12: mod_base = gm
  modified_base 13: mod_base = cm
  modified_base 14: mod_base = gm
  modified_base 15: mod_base = um
  modified_base 16: mod_base = gm
  modified_base 17: mod_base = gm
  modified_base 18: mod_base = um
  modified_base 19: mod_base = cm
  modified_base 20: mod_base = cm
  modified_base 21: mod_base = gm
cattatagactgcgtggtccg

SEQ ID NO: 1211 - RNA, 21 nt, synthetic construct
  source 1..21: mol_type = other RNA
  modified_base <1: mod_base = OTHER; note = two inverted abasic nucleosides
  modified_base 1: mod_base = um
  misc_feature 1^2: note = Phosphorothioate bond
  modified_base 2: mod_base = gm
  misc_feature 2^3: note = Phosphorothioate bond
  modified_base 3: mod_base = cm
  modified_base 4: mod_base = gm
  modified_base 5: mod_base = um
  modified_base 6: mod_base = gm
  modified_base 7: mod_base = gm
  modified_base 8: mod_base = um
  modified_base 9: mod_base = OTHER; note = 2'-Fluoro-cytidine
  modified_base 10: mod_base = OTHER; note = 2'-Fluoro-cytidine
  modified_base 11: mod_base = OTHER; note = 2'-Fluoro-guanosine
  modified_base 12: mod_base = um
  modified_base 13: mod_base = OTHER; note = 2'-O-methyl-adenosine
  modified_base 14: mod_base = um
  modified_base 15: mod_base = um
  modified_base 16: mod_base = cm
  modified_base 17: mod_base = cm
  modified_base 18: mod_base = cm
  modified_base 19: mod_base = OTHER; note = 2'-O-methyl-adenosine
  modified_base 20: mod_base = OTHER; note = 2'-O-methyl-adenosine
  modified_base 21: mod_base = gm
tgcgtggtccgtattcccaag

SEQ ID NO: 1212 - RNA, 21 nt, synthetic construct
  source 1..21: mol_type = other RNA
  modified_base <1: mod_base = OTHER; note = two inverted abasic nucleosides
  modified_base 1: mod_base = OTHER; note = 2'-O-methyl-adenosine
  misc_feature 1^2: note = Phosphorothioate bond
  modified_base 2: mod_base = um
  misc_feature 2^3: note = Phosphorothioate bond
  modified_base 3: mod_base = cm
  modified_base 4: mod_base = um
  modified_base 5: mod_base = OTHER; note = 2'-O-methyl-adenosine
  modified_base 6: mod_base = cm
  modified_base 7: mod_base = cm
  modified_base 8: mod_base = gm
  modified_base 9: mod_base = OTHER; note = 2'-Fluoro-adenosine
  modified_base 10: mod_base = OTHER; note = 2'-Fluoro-guanosine
  modified_base 11: mod_base = OTHER; note = 2'-Fluoro-cytidine
  modified_base 12: mod_base = cm
  modified_base 13: mod_base = gm
  modified_base 14: mod_base = cm
  modified_base 15: mod_base = cm
  modified_base 16: mod_base = um
  modified_base 17: mod_base = OTHER; note = 2'-O-methyl-adenosine
  modified_base 18: mod_base = cm
  modified_base 19: mod_base = um
  modified_base 20: mod_base = um
  modified_base 21: mod_base = cm
atctaccgagccgcctacttc

SEQ ID NO: 1213 - RNA, 21 nt, synthetic construct
  source 1..21: mol_type = other RNA
  modified_base <1: mod_base = OTHER; note = two inverted abasic nucleosides
  modified_base 1: mod_base = um
  misc_feature 1^2: note = Phosphorothioate bond
  modified_base 2: mod_base = um
  misc_feature 2^3: note = Phosphorothioate bond
  modified_base 3: mod_base = gm
  modified_base 4: mod_base = cm
  modified_base 5: mod_base = cm
  modified_base 6: mod_base = cm
  modified_base 7: mod_base = gm
  modified_base 8: mod_base = um
  modified_base 9: mod_base = OTHER; note = 2'-Fluoro-adenosine
  modified_base 10: mod_base = OTHER; note = 2'-Fluoro-cytidine
  modified_base 11: mod_base = OTHER; note = 2'-Fluoro-cytidine
  modified_base 12: mod_base = cm
  modified_base 13: mod_base = gm
  modified_base 14: mod_base = um
  modified_base 15: mod_base = cm
  modified_base 16: mod_base = um
  modified_base 17: mod_base = OTHER; note = 2'-O-methyl-adenosine
  modified_base 18: mod_base = gm
  modified_base 19: mod_base = cm
  modified_base 20: mod_base = OTHER; note = 2'-O-methyl-adenosine
  modified_base 21: mod_base = gm
ttgcccgtacccgtctagcag

SEQ ID NO: 1214 - RNA, 21 nt, synthetic construct
  source 1..21: mol_type = other RNA
  modified_base <1: mod_base = OTHER; note = two inverted abasic nucleosides
  modified_base 1: mod_base = cm
  misc_feature 1^2: note = Phosphorothioate bond
  modified_base 2: mod_base = um
  misc_feature 2^3: note = Phosphorothioate bond
  modified_base 3: mod_base = cm
  modified_base 4: mod_base = OTHER; note = 2'-O-methyl-adenosine
  modified_base 5: mod_base = cm
  modified_base 6: mod_base = OTHER; note = 2'-O-methyl-adenosine
  modified_base 7: mod_base = um
  modified_base 8: mod_base = cm
  modified_base 9: mod_base = OTHER; note = 2'-Fluoro-guanosine
  modified_base 10: mod_base = OTHER; note = 2'-Fluoro-uridine
  modified_base 11: mod_base = OTHER; note = 2'-Fluoro-cytidine
  modified_base 12: mod_base = OTHER; note = 2'-O-methyl-adenosine
  modified_base 13: mod_base = um
  modified_base 14: mod_base = cm
  modified_base 15: mod_base = OTHER; note = 2'-O-methyl-adenosine
  modified_base 16: mod_base = gm
  modified_base 17: mod_base = cm
  modified_base 18: mod_base = um
  modified_base 19: mod_base = gm
  modified_base 20: mod_base = gm
  modified_base 21: mod_base = OTHER; note = 2'-O-methyl-adenosine
ctcacatcgtcatcagctgga

SEQ ID NO: 1215 - RNA, 21 nt, synthetic construct
  source 1..21: mol_type = other RNA
  modified_base <1: mod_base = OTHER; note = two inverted abasic nucleosides
  modified_base 1: mod_base = um
  misc_feature 1^2: note = Phosphorothioate bond
  modified_base 2: mod_base = OTHER; note = 2'-O-methyl-adenosine
  misc_feature 2^3: note = Phosphorothioate bond
  modified_base 3: mod_base = um
  modified_base 4: mod_base = OTHER; note = 2'-O-methyl-adenosine
  modified_base 5: mod_base = gm
  modified_base 6: mod_base = OTHER; note = 2'-O-methyl-adenosine
  modified_base 7: mod_base = cm
  modified_base 8: mod_base = um
  modified_base 9: mod_base = OTHER; note = 2'-Fluoro-guanosine
  modified_base 10: mod_base = OTHER; note = 2'-Fluoro-cytidine
  modified_base 11: mod_base = OTHER; note = 2'-Fluoro-guanosine
  modified_base 12: mod_base = um
  modified_base 13: mod_base = gm
  modified_base 14: mod_base = gm
  modified_base 15: mod_base = um
  modified_base 16: mod_base = cm
  modified_base 17: mod_base = cm
  modified_base 18: mod_base = gm
  modified_base 19: mod_base = um
  modified_base 20: mod_base = OTHER; note = 2'-O-methyl-adenosine
  modified_base 21: mod_base = um
tatagactgcgtggtccgtat

SEQ ID NO: 1216 - RNA, 21 nt, synthetic construct
  source 1..21: mol_type = other RNA
  modified_base <1: mod_base = OTHER; note = two inverted abasic nucleosides
  modified_base 1: mod_base = gm
  misc_feature 1^2: note = Phosphorothioate bond
  modified_base 2: mod_base = gm
  misc_feature 2^3: note = Phosphorothioate bond
  modified_base 3: mod_base = cm
  modified_base 4: mod_base = cm
  modified_base 5: mod_base = um
  modified_base 6: mod_base = cm
  modified_base 7: mod_base = gm
  modified_base 8: mod_base = gm
  modified_base 9: mod_base = OTHER; note = 2'-Fluoro-uridine
  modified_base 10: mod_base = OTHER; note = 2'-Fluoro-guanosine
  modified_base 11: mod_base = OTHER; note = 2'-Fluoro-adenosine
  modified_base 12: mod_base = cm
  modified_base 13: mod_base = um
  modified_base 14: mod_base = gm
  modified_base 15: mod_base = cm
  modified_base 16: mod_base = cm
  modified_base 17: mod_base = um
  modified_base 18: mod_base = gm
  modified_base 19: mod_base = gm
  modified_base 20: mod_base = um
  modified_base 21: mod_base = um
ggcctcggtgactgcctggtt

SEQ ID NO: 1217 - RNA, 21 nt, synthetic construct
  source 1..21: mol_type = other RNA
  modified_base <1: mod_base = OTHER; note = two inverted abasic nucleosides
  modified_base 1: mod_base = gm
  misc_feature 1^2: note = Phosphorothioate bond
  modified_base 2: mod_base = gm
  misc_feature 2^3: note = Phosphorothioate bond
  modified_base 3: mod_base = OTHER; note = 2'-O-methyl-adenosine
  modified_base 4: mod_base = um
  modified_base 5: mod_base = gm
  modified_base 6: mod_base = OTHER; note = 2'-O-methyl-adenosine
  modified_base 7: mod_base = um
  modified_base 8: mod_base = cm
  modified_base 9: mod_base = OTHER; note = 2'-Fluoro-guanosine
  modified_base 10: mod_base = OTHER; note = 2'-Fluoro-cytidine
  modified_base 11: mod_base = OTHER; note = 2'-Fluoro-adenosine
  modified_base 12: mod_base = cm
  modified_base 13: mod_base = OTHER; note = 2'-O-methyl-adenosine
  modified_base 14: mod_base = gm
  modified_base 15: mod_base = OTHER; note = 2'-O-methyl-adenosine
  modified_base 16: mod_base = cm
  modified_base 17: mod_base = um
  modified_base 18: mod_base = gm
  modified_base 19: mod_base = um
  modified_base 20: mod_base = cm
  modified_base 21: mod_base = OTHER; note = 2'-O-methyl-adenosine
ggatgatcgcacagactgtca

SEQ ID NO: 1218 - RNA, 21 nt, synthetic construct
  source 1..21: mol_type = other RNA
  modified_base <1: mod_base = OTHER; note = two inverted abasic nucleosides
  modified_base 1: mod_base = gm
  misc_feature 1^2: note = Phosphorothioate bond
  modified_base 2: mod_base = OTHER; note = 2'-O-methyl-adenosine
  misc_feature 2^3: note = Phosphorothioate bond
  modified_base 3: mod_base = um
  modified_base 4: mod_base = um
  modified_base 5: mod_base = um
  modified_base 6: mod_base = um
  modified_base 7: mod_base = gm
  modified_base 8: mod_base = cm
  modified_base 9: mod_base = OTHER; note = 2'-Fluoro-cytidine
  modified_base 10: mod_base = OTHER; note = 2'-Fluoro-cytidine
  modified_base 11: mod_base = OTHER; note = 2'-Fluoro-guanosine
  modified_base 12: mod_base = um
  modified_base 13: mod_base = OTHER; note = 2'-O-methyl-adenosine
  modified_base 14: mod_base = cm
  modified_base 15: mod_base = cm
  modified_base 16: mod_base = cm
  modified_base 17: mod_base = gm
  modified_base 18: mod_base = um
  modified_base 19: mod_base = cm
  modified_base 20: mod_base = um
  modified_base 21: mod_base = OTHER; note = 2'-O-methyl-adenosine
gattttgcccgtacccgtcta

SEQ ID NO: 1219 - RNA, 21 nt, synthetic construct
  source 1..21: mol_type = other RNA
  modified_base <1: mod_base = OTHER; note = two inverted abasic nucleosides
  modified_base 1: mod_base = gm
  misc_feature 1^2: note = Phosphorothioate bond
  modified_base 2: mod_base = OTHER; note = 2'-O-methyl-adenosine
  misc_feature 2^3: note = Phosphorothioate bond
  modified_base 3: mod_base = um
  modified_base 4: mod_base = cm
  modified_base 5: mod_base = gm
  modified_base 6: mod_base = cm
  modified_base 7: mod_base = OTHER; note = 2'-O-methyl-adenosine
  modified_base 8: mod_base = cm
  modified_base 9: mod_base = OTHER; note = 2'-Fluoro-adenosine
  modified_base 10: mod_base = OTHER; note = 2'-Fluoro-guanosine
  modified_base 11: mod_base = OTHER; note = 2'-Fluoro-adenosine
  modified_base 12: mod_base = cm
  modified_base 13: mod_base = um
  modified_base 14: mod_base = gm
  modified_base 15: mod_base = um
  modified_base 16: mod_base = cm
  modified_base 17: mod_base = OTHER; note = 2'-O-methyl-adenosine
  modified_base 18: mod_base = cm
  modified_base 19: mod_base = um
  modified_base 20: mod_base = gm
  modified_base 21: mod_base = cm
gatcgcacagactgtcactgc

SEQ ID NO: 1220 - RNA, 21 nt, synthetic construct
  source 1..21: mol_type = other RNA
  modified_base <1: mod_base = OTHER; note = two inverted abasic nucleosides
  modified_base 1: mod_base = OTHER; note = 2'-O-methyl-adenosine
  misc_feature 1^2: note = Phosphorothioate bond
  modified_base 2: mod_base = um
  misc_feature 2^3: note = Phosphorothioate bond
  modified_base 3: mod_base = gm
  modified_base 4: mod_base = OTHER; note = 2'-O-methyl-adenosine
  modified_base 5: mod_base = um
  modified_base 6: mod_base = cm
  modified_base 7: mod_base = gm
  modified_base 8: mod_base = cm
  modified_base 9: mod_base = OTHER; note = 2'-Fluoro-adenosine
  modified_base 10: mod_base = OTHER; note = 2'-Fluoro-cytidine
  modified_base 11: mod_base = OTHER; note = 2'-Fluoro-adenosine
  modified_base 12: mod_base = gm
  modified_base 13: mod_base = OTHER; note = 2'-O-methyl-adenosine
  modified_base 14: mod_base = cm
  modified_base 15: mod_base = um
  modified_base 16: mod_base = gm
  modified_base 17: mod_base = um
  modified_base 18: mod_base = cm
  modified_base 19: mod_base = OTHER; note = 2'-O-methyl-adenosine
  modified_base 20: mod_base = cm
  modified_base 21: mod_base = um
atgatcgcacagactgtcact

SEQ ID NO: 1221 - RNA, 21 nt, synthetic construct
  source 1..21: mol_type = other RNA
  modified_base <1: mod_base = OTHER; note = two inverted abasic nucleosides
  modified_base 1: mod_base = um
  misc_feature 1^2: note = Phosphorothioate bond
  modified_base 2: mod_base = um
  misc_feature 2^3: note = Phosphorothioate bond
  modified_base 3: mod_base = um
  modified_base 4: mod_base = um
  modified_base 5: mod_base = gm
  modified_base 6: mod_base = cm
  modified_base 7: mod_base = cm
  modified_base 8: mod_base = cm
  modified_base 9: mod_base = OTHER; note = 2'-Fluoro-guanosine
  modified_base 10: mod_base = OTHER; note = 2'-Fluoro-uridine
  modified_base 11: mod_base = OTHER; note = 2'-Fluoro-adenosine
  modified_base 12: mod_base = cm
  modified_base 13: mod_base = cm
  modified_base 14: mod_base = cm
  modified_base 15: mod_base = gm
  modified_base 16: mod_base = um
  modified_base 17: mod_base = cm
  modified_base 18: mod_base = um
  modified_base 19: mod_base = OTHER; note = 2'-O-methyl-adenosine
  modified_base 20: mod_base = gm
  modified_base 21: mod_base = cm
ttttgcccgtacccgtctagc

SEQ ID NO: 1222 - RNA, 21 nt, synthetic construct
  source 1..21: mol_type = other RNA
  modified_base <1: mod_base = OTHER; note = two inverted abasic nucleosides
  modified_base 1: mod_base = um
  misc_feature 1^2: note = Phosphorothioate bond
  modified_base 2: mod_base = cm
  misc_feature 2^3: note = Phosphorothioate bond
  modified_base 3: mod_base = OTHER; note = 2'-O-methyl-adenosine
  modified_base 4: mod_base = um
  modified_base 5: mod_base = cm
  modified_base 6: mod_base = um
  modified_base 7: mod_base = OTHER; note = 2'-O-methyl-adenosine
  modified_base 8: mod_base = cm
  modified_base 9: mod_base = OTHER; note = 2'-Fluoro-cytidine
  modified_base 10: mod_base = OTHER; note = 2'-Fluoro-guanosine
  modified_base 11: mod_base = OTHER; note = 2'-Fluoro-adenosine
  modified_base 12: mod_base = gm
  modified_base 13: mod_base = cm
  modified_base 14: mod_base = cm
  modified_base 15: mod_base = gm
  modified_base 16: mod_base = cm
  modified_base 17: mod_base = cm
  modified_base 18: mod_base = um
  modified_base 19: mod_base = OTHER; note = 2'-O-methyl-adenosine
  modified_base 20: mod_base = cm
  modified_base 21: mod_base = um
tcatctaccgagccgcctact

SEQ ID NO: 1223 - RNA, 21 nt, synthetic construct
  source 1..21: mol_type = other RNA
  modified_base <1: mod_base = OTHER; note = two inverted abasic nucleosides
  modified_base 1: mod_base = um
  misc_feature 1^2: note = Phosphorothioate bond
  modified_base 2: mod_base = OTHER; note = 2'-O-methyl-adenosine
  misc_feature 2^3: note = Phosphorothioate bond
  modified_base 3: mod_base = gm
  modified_base 4: mod_base = OTHER; note = 2'-O-methyl-adenosine
  modified_base 5: mod_base = cm
  modified_base 6: mod_base = um
  modified_base 7: mod_base = gm
  modified_base 8: mod_base = cm
  modified_base 9: mod_base = OTHER; note = 2'-Fluoro-guanosine
  modified_base 10: mod_base = OTHER; note = 2'-Fluoro-uridine
  modified_base 11: mod_base = OTHER; note = 2'-Fluoro-guanosine
  modified_base 12: mod_base = gm
  modified_base 13: mod_base = um
  modified_base 14: mod_base = cm
  modified_base 15: mod_base = cm
  modified_base 16: mod_base = gm
  modified_base 17: mod_base = um
  modified_base 18: mod_base = OTHER; note = 2'-O-methyl-adenosine
  modified_base 19: mod_base = um
  modified_base 20: mod_base = um
  modified_base 21: mod_base = cm
tagactgcgtggtccgtattc

SEQ ID NO: 1224 - RNA, 21 nt, synthetic construct
  source 1..21: mol_type = other RNA
  modified_base <1: mod_base = OTHER; note = two inverted abasic nucleosides
  modified_base 1: mod_base = cm
  misc_feature 1^2: note = Phosphorothioate bond
  modified_base 2: mod_base = um
  misc_feature 2^3: note = Phosphorothioate bond
  modified_base 3: mod_base = gm
  modified_base 4: mod_base = cm
  modified_base 5: mod_base = OTHER; note = 2'-O-methyl-adenosine
  modified_base 6: mod_base = gm
  modified_base 7: mod_base = OTHER; note = 2'-O-methyl-adenosine
  modified_base 8: mod_base = um
  modified_base 9: mod_base = OTHER; note = 2'-Fluoro-adenosine
  modified_base 10: mod_base = OTHER; note = 2'-Fluoro-adenosine
  modified_base 11: mod_base = OTHER; note = 2'-Fluoro-guanosine
  modified_base 12: mod_base = cm
  modified_base 13: mod_base = OTHER; note = 2'-O-methyl-adenosine
  modified_base 14: mod_base = OTHER; note = 2'-O-methyl-adenosine
  modified_base 15: mod_base = um
  modified_base 16: mod_base = OTHER; note = 2'-O-methyl-adenosine
  modified_base 17: mod_base = cm
  modified_base 18: mod_base = OTHER; note = 2'-O-methyl-adenosine
  modified_base 19: mod_base = OTHER; note = 2'-O-methyl-adenosine
  modified_base 20: mod_base = OTHER; note = 2'-O-methyl-adenosine
  modified_base 21: mod_base = gm
ctgcagataagcaatacaaag

SEQ ID NO: 1225 - RNA, 21 nt, synthetic construct
  source 1..21: mol_type = other RNA
  modified_base <1: mod_base = OTHER; note = two inverted abasic nucleosides
  modified_base 1: mod_base = OTHER; note = 2'-O-methyl-adenosine
  misc_feature 1^2: note = Phosphorothioate bond
  modified_base 2: mod_base = cm
  misc_feature 2^3: note = Phosphorothioate bond
  modified_base 3: mod_base = um
  modified_base 4: mod_base = gm
  modified_base 5: mod_base = cm
  modified_base 6: mod_base = OTHER; note = 2'-O-methyl-adenosine
  modified_base 7: mod_base = gm
  modified_base 8: mod_base = OTHER; note = 2'-O-methyl-adenosine
  modified_base 9: mod_base = OTHER; note = 2'-Fluoro-uridine
  modified_base 10: mod_base = OTHER; note = 2'-Fluoro-adenosine
  modified_base 11: mod_base = OTHER; note = 2'-Fluoro-adenosine
  modified_base 12: mod_base = gm
  modified_base 13: mod_base = cm
  modified_base 14: mod_base = OTHER; note = 2'-O-methyl-adenosine
  modified_base 15: mod_base = OTHER; note = 2'-O-methyl-adenosine
  modified_base 16: mod_base = um
  modified_base 17: mod_base = OTHER; note = 2'-O-methyl-adenosine
  modified_base 18: mod_base = cm
  modified_base 19: mod_base = OTHER; note = 2'-O-methyl-adenosine
  modified_base 20: mod_base = OTHER; note = 2'-O-methyl-adenosine
  modified_base 21: mod_base = OTHER; note = 2'-O-methyl-adenosine
actgcagataagcaatacaaa

SEQ ID NO: 1226 - RNA, 21 nt, synthetic construct
  source 1..21: mol_type = other RNA
  modified_base <1: mod_base = OTHER; note = two inverted abasic nucleosides
  modified_base 1: mod_base = cm
  misc_feature 1^2: note = Phosphorothioate bond
  modified_base 2: mod_base = OTHER; note = 2'-O-methyl-adenosine
  misc_feature 2^3: note = Phosphorothioate bond
  modified_base 3: mod_base = cm
  modified_base 4: mod_base = um
  modified_base 5: mod_base = gm
  modified_base 6: mod_base = cm
  modified_base 7: mod_base = OTHER; note = 2'-O-methyl-adenosine
  modified_base 8: mod_base = gm
  modified_base 9: mod_base = OTHER; note = 2'-Fluoro-adenosine
  modified_base 10: mod_base = OTHER; note = 2'-Fluoro-uridine
  modified_base 11: mod_base = OTHER; note = 2'-Fluoro-adenosine
  modified_base 12: mod_base = OTHER; note = 2'-O-methyl-adenosine
  modified_base 13: mod_base = gm
  modified_base 14: mod_base = cm
  modified_base 15: mod_base = OTHER; note = 2'-O-methyl-adenosine
  modified_base 16: mod_base = OTHER; note = 2'-O-methyl-adenosine
  modified_base 17: mod_base = um
  modified_base 18: mod_base = OTHER; note = 2'-O-methyl-adenosine
  modified_base 19: mod_base = cm
  modified_base 20: mod_base = OTHER; note = 2'-O-methyl-adenosine
  modified_base 21: mod_base = OTHER; note = 2'-O-methyl-adenosine
cactgcagataagcaatacaa

SEQ ID NO: 1227 - RNA, 21 nt, synthetic construct
  source 1..21: mol_type = other RNA
  modified_base <1: mod_base = OTHER; note = two inverted abasic nucleosides
  modified_base 1: mod_base = gm
  misc_feature 1^2: note = Phosphorothioate bond
  modified_base 2: mod_base = cm
  misc_feature 2^3: note = Phosphorothioate bond
  modified_base 3: mod_base = OTHER; note = 2'-O-methyl-adenosine
  modified_base 4: mod_base = OTHER; note = 2'-O-methyl-adenosine
  modified_base 5: mod_base = gm
  modified_base 6: mod_base = cm
  modified_base 7: mod_base = OTHER; note = 2'-O-methyl-adenosine
  modified_base 8: mod_base = gm
  modified_base 9: mod_base = OTHER; note = 2'-Fluoro-adenosine
  modified_base 10: mod_base = OTHER; note = 2'-Fluoro-uridine
  modified_base 11: mod_base = OTHER; note = 2'-Fluoro-cytidine
  modified_base 12: mod_base = OTHER; note = 2'-O-methyl-adenosine
  modified_base 13: mod_base = cm
  modified_base 14: mod_base = um
  modified_base 15: mod_base = gm
  modified_base 16: mod_base = cm
  modified_base 17: mod_base = OTHER; note = 2'-O-methyl-adenosine
  modified_base 18: mod_base = gm
  modified_base 19: mod_base = OTHER; note = 2'-O-methyl-adenosine
  modified_base 20: mod_base = um
  modified_base 21: mod_base = OTHER; note = 2'-O-methyl-adenosine
gcaagcagatcactgcagata

SEQ ID NO: 1228 - RNA, 21 nt, synthetic construct
  source 1..21: mol_type = other RNA
  modified_base <1: mod_base = OTHER; note = two inverted abasic nucleosides
  modified_base 1: mod_base = OTHER; note = 2'-O-methyl-adenosine
  misc_feature 1^2: note = Phosphorothioate bond
  modified_base 2: mod_base = um
  misc_feature 2^3: note = Phosphorothioate bond
  modified_base 3: mod_base = cm
  modified_base 4: mod_base = OTHER; note = 2'-O-methyl-adenosine
  modified_base 5: mod_base = cm
  modified_base 6: mod_base = um
  modified_base 7: mod_base = gm
  modified_base 8: mod_base = cm
  modified_base 9: mod_base = OTHER; note = 2'-Fluoro-adenosine
  modified_base 10: mod_base = OTHER; note = 2'-Fluoro-guanosine
  modified_base 11: mod_base = OTHER; note = 2'-Fluoro-adenosine
  modified_base 12: mod_base = um
  modified_base 13: mod_base = OTHER; note = 2'-O-methyl-adenosine
  modified_base 14: mod_base = OTHER; note = 2'-O-methyl-adenosine
  modified_base 15: mod_base = gm
  modified_base 16: mod_base = cm
  modified_base 17: mod_base = OTHER; note = 2'-O-methyl-adenosine
  modified_base 18: mod_base = OTHER; note = 2'-O-methyl-adenosine
  modified_base 19: mod_base = um
  modified_base 20: mod_base = OTHER; note = 2'-O-methyl-adenosine
  modified_base 21: mod_base = cm
atcactgcagataagcaatac

SEQ ID NO: 1229 - RNA, 21 nt, synthetic construct
  source 1..21: mol_type = other RNA
  modified_base <1: mod_base = OTHER; note = two inverted abasic nucleosides
  modified_base 1: mod_base = um
  misc_feature 1^2: note = Phosphorothioate bond
  modified_base 2: mod_base = cm
  misc_feature 2^3: note = Phosphorothioate bond
  modified_base 3: mod_base = OTHER; note = 2'-O-methyl-adenosine
  modified_base 4: mod_base = cm
  modified_base 5: mod_base = um
  modified_base 6: mod_base = gm
  modified_base 7: mod_base = cm
  modified_base 8: mod_base = OTHER; note = 2'-O-methyl-adenosine
  modified_base 9: mod_base = OTHER; note = 2'-Fluoro-guanosine
  modified_base 10: mod_base = OTHER; note = 2'-Fluoro-adenosine
  modified_base 11: mod_base = OTHER; note = 2'-Fluoro-uridine
  modified_base 12: mod_base = OTHER; note = 2'-O-methyl-adenosine
  modified_base 13: mod_base = OTHER; note = 2'-O-methyl-adenosine
  modified_base 14: mod_base = gm
  modified_base 15: mod_base = cm
  modified_base 16: mod_base = OTHER; note = 2'-O-methyl-adenosine
  modified_base 17: mod_base = OTHER; note = 2'-O-methyl-adenosine
  modified_base 18: mod_base = um
  modified_base 19: mod_base = OTHER; note = 2'-O-methyl-adenosine
  modified_base 20: mod_base = cm
  modified_base 21: mod_base = OTHER; note = 2'-O-methyl-adenosine
tcactgcagataagcaataca

SEQ ID NO: 1230 - RNA, 21 nt, synthetic construct
  source 1..21: mol_type = other RNA
  modified_base <1: mod_base = OTHER; note = two inverted abasic nucleosides
  modified_base 1: mod_base = gm
  misc_feature 1^2: note = Phosphorothioate bond
  modified_base 2: mod_base = cm
  misc_feature 2^3: note = Phosphorothioate bond
  modified_base 3: mod_base = OTHER; note = 2'-O-methyl-adenosine
  modified_base 4: mod_base = gm
  modified_base 5: mod_base = OTHER; note = 2'-O-methyl-adenosine
  modified_base 6: mod_base = um
  modified_base 7: mod_base = cm
  modified_base 8: mod_base = OTHER; note = 2'-O-methyl-adenosine
  modified_base 9: mod_base = OTHER; note = 2'-Fluoro-cytidine
  modified_base 10: mod_base = OTHER; note = 2'-Fluoro-uridine
  modified_base 11: mod_base = OTHER; note = 2'-Fluoro-guanosine
  modified_base 12: mod_base = cm
  modified_base 13: mod_base = OTHER; note = 2'-O-methyl-adenosine
  modified_base 14: mod_base = gm
  modified_base 15: mod_base = OTHER; note = 2'-O-methyl-adenosine
  modified_base 16: mod_base = um
  modified_base 17: mod_base = OTHER; note = 2'-O-methyl-adenosine
  modified_base 18: mod_base = OTHER; note = 2'-O-methyl-adenosine
  modified_base 19: mod_base = gm
  modified_base 20: mod_base = cm
  modified_base 21: mod_base = OTHER; note = 2'-O-methyl-adenosine
gcagatcactgcagataagca

SEQ ID NO: 1231 - RNA, 21 nt, synthetic construct
  source 1..21: mol_type = other RNA
  modified_base <1: mod_base = OTHER; note = two inverted abasic nucleosides
  modified_base 1: mod_base = cm
  misc_feature 1^2: note = Phosphorothioate bond
  modified_base 2: mod_base = OTHER; note = 2'-O-methyl-adenosine
  misc_feature 2^3: note = Phosphorothioate bond
  modified_base 3: mod_base = gm
  modified_base 4: mod_base = OTHER; note = 2'-O-methyl-adenosine
  modified_base 5: mod_base = um
  modified_base 6: mod_base = cm
  modified_base 7: mod_base = OTHER; note = 2'-O-methyl-adenosine
  modified_base 8: mod_base = cm
  modified_base 9: mod_base = OTHER; note = 2'-Fluoro-uridine
  modified_base 10: mod_base = OTHER; note = 2'-Fluoro-guanosine
  modified_base 11: mod_base = OTHER; note = 2'-Fluoro-cytidine
  modified_base 12: mod_base = OTHER; note = 2'-O-methyl-adenosine
  modified_base 13: mod_base = gm
  modified_base 14: mod_base = OTHER; note = 2'-O-methyl-adenosine
  modified_base 15: mod_base = um
  modified_base 16: mod_base = OTHER; note = 2'-O-methyl-adenosine
  modified_base 17: mod_base = OTHER; note = 2'-O-methyl-adenosine
  modified_base 18: mod_base = gm
  modified_base 19: mod_base = cm
  modified_base 20: mod_base = OTHER; note = 2'-O-methyl-adenosine
  modified_base 21: mod_base = OTHER; note = 2'-O-methyl-adenosine
cagatcactgcagataagcaa

SEQ ID NO: 1232 - RNA, 21 nt, synthetic construct
  source 1..21: mol_type = other RNA
  modified_base <1: mod_base = OTHER; note = two inverted abasic nucleosides
  modified_base 1: mod_base = OTHER; note = 2'-O-methyl-adenosine
  misc_feature 1^2: note = Phosphorothioate bond
  modified_base 2: mod_base = gm
  misc_feature 2^3: note = Phosphorothioate bond
  modified_base 3: mod_base = cm
  modified_base 4: mod_base = OTHER; note = 2'-O-methyl-adenosine
  modified_base 5: mod_base = OTHER; note = 2'-O-methyl-adenosine
  modified_base 6: mod_base = gm
  modified_base 7: mod_base = cm
  modified_base 8: mod_base = OTHER; note = 2'-O-methyl-adenosine
  modified_base 9: mod_base = OTHER; note = 2'-Fluoro-guanosine
  modified_base 10: mod_base = OTHER; note = 2'-Fluoro-adenosine
  modified_base 11: mod_base = OTHER; note = 2'-Fluoro-uridine
  modified_base 12: mod_base = cm
  modified_base 13: mod_base = OTHER; note = 2'-O-methyl-adenosine
  modified_base 14: mod_base = cm
  modified_base 15: mod_base = um
  modified_base 16: mod_base = gm
  modified_base 17: mod_base = cm
  modified_base 18: mod_base = OTHER; note = 2'-O-methyl-adenosine
  modified_base 19: mod_base = gm
  modified_base 20: mod_base = OTHER; note = 2'-O-methyl-adenosine
  modified_base 21: mod_base = um
agcaagcagatcactgcagat

SEQ ID NO: 1233 - RNA, 21 nt, synthetic construct
  source 1..21: mol_type = other RNA
  modified_base <1: mod_base = OTHER; note = two inverted abasic nucleosides
  modified_base 1: mod_base = gm
  misc_feature 1^2: note = Phosphorothioate bond
  modified_base 2: mod_base = OTHER; note = 2'-O-methyl-adenosine
  misc_feature 2^3: note = Phosphorothioate bond
  modified_base 3: mod_base = um
  modified_base 4: mod_base = cm
  modified_base 5: mod_base = OTHER; note = 2'-O-methyl-adenosine
  modified_base 6: mod_base = cm
  modified_base 7: mod_base = um
  modified_base 8: mod_base = gm
  modified_base 9: mod_base = OTHER; note = 2'-Fluoro-cytidine
  modified_base 10: mod_base = OTHER; note = 2'-Fluoro-adenosine
  modified_base 11: mod_base = OTHER; note = 2'-Fluoro-guanosine
  modified_base 12: mod_base = OTHER; note = 2'-O-methyl-adenosine
  modified_base 13: mod_base = um
  modified_base 14: mod_base = OTHER; note = 2'-O-methyl-adenosine
  modified_base 15: mod_base = OTHER; note = 2'-O-methyl-adenosine
  modified_base 16: mod_base = gm
  modified_base 17: mod_base = cm
  modified_base 18: mod_base = OTHER; note = 2'-O-methyl-adenosine
  modified_base 19: mod_base = OTHER; note = 2'-O-methyl-adenosine
  modified_base 20: mod_base = um
  modified_base 21: mod_base = OTHER; note = 2'-O-methyl-adenosine
gatcactgcagataagcaata

SEQ ID NO: 1234 - RNA, 21 nt, synthetic construct
  source 1..21: mol_type = other RNA
  modified_base <1: mod_base = OTHER; note = two inverted abasic nucleosides
  modified_base 1: mod_base = OTHER; note = 2'-O-methyl-adenosine
  misc_feature 1^2: note = Phosphorothioate bond
  modified_base 2: mod_base = um
  misc_feature 2^3: note = Phosphorothioate bond
  modified_base 3: mod_base = OTHER; note = 2'-O-methyl-adenosine
  modified_base 4: mod_base = OTHER; note = 2'-O-methyl-adenosine
  modified_base 5: mod_base = OTHER; note = 2'-O-methyl-adenosine
  modified_base 6: mod_base = um
  modified_base 7: mod_base = OTHER; note = 2'-O-methyl-adenosine
  modified_base 8: mod_base = OTHER; note = 2'-O-methyl-adenosine
  modified_base 9: mod_base = OTHER; note = 2'-Fluoro-cytidine
  modified_base 10: mod_base = OTHER; note = 2'-Fluoro-adenosine
  modified_base 11: mod_base = OTHER; note = 2'-Fluoro-adenosine
  modified_base 12: mod_base = OTHER; note = 2'-O-methyl-adenosine
  modified_base 13: mod_base = um
  modified_base 14: mod_base = um
  modified_base 15: mod_base = um
  modified_base 16: mod_base = gm
  modified_base 17: mod_base = gm
  modified_base 18: mod_base = OTHER; note = 2'-O-methyl-adenosine
  modified_base 19: mod_base = gm
  modified_base 20: mod_base = OTHER; note = 2'-O-methyl-adenosine
  modified_base 21: mod_base = OTHER; note = 2'-O-methyl-adenosine
ataaataacaaatttggagaa

SEQ ID NO: 1235 - RNA, 21 nt, synthetic construct
  source 1..21: mol_type = other RNA
  modified_base <1: mod_base = OTHER; note = two inverted abasic nucleosides
  modified_base 1: mod_base = um
  misc_feature 1^2: note = Phosphorothioate bond
  modified_base 2: mod_base = cm
  misc_feature 2^3: note = Phosphorothioate bond
  modified_base 3: mod_base = cm
  modified_base 4: mod_base = um
  modified_base 5: mod_base = gm
  modified_base 6: mod_base = OTHER; note = 2'-O-methyl-adenosine
  modified_base 7: mod_base = um
  modified_base 8: mod_base = OTHER; note = 2'-O-methyl-adenosine
  modified_base 9: mod_base = OTHER; note = 2'-Fluoro-adenosine
  modified_base 10: mod_base = OTHER; note = 2'-Fluoro-adenosine
  modified_base 11: mod_base = OTHER; note = 2'-Fluoro-uridine
  modified_base 12: mod_base = OTHER; note = 2'-O-methyl-adenosine
  modified_base 13: mod_base = OTHER; note = 2'-O-methyl-adenosine
  modified_base 14: mod_base = cm
  modified_base 15: mod_base = OTHER; note = 2'-O-methyl-adenosine
  modified_base 16: mod_base = OTHER; note = 2'-O-methyl-adenosine
  modified_base 17: mod_base = OTHER; note = 2'-O-methyl-adenosine
  modified_base 18: mod_base = um
  modified_base 19: mod_base = um
  modified_base 20: mod_base = um
  modified_base 21: mod_base = gm
tcctgataaataacaaatttg

SEQ ID NO: 1236 - RNA, 21 nt, synthetic construct
  source 1..21: mol_type = other RNA
  modified_base <1: mod_base = OTHER; note = two inverted abasic nucleosides
  modified_base 1: mod_base = gm
  misc_feature 1^2: note = Phosphorothioate bond
  modified_base 2: mod_base = OTHER; note = 2'-O-methyl-adenosine
  misc_feature 2^3: note = Phosphorothioate bond
  modified_base 3: mod_base = OTHER; note = 2'-O-methyl-adenosine
  modified_base 4: mod_base = OTHER; note = 2'-O-methyl-adenosine
  modified_base 5: mod_base = gm
  modified_base 6: mod_base = gm
  modified_base 7: mod_base = gm
  modified_base 8: mod_base = OTHER; note = 2'-O-methyl-adenosine
  modified_base 9: mod_base = OTHER; note = 2'-Fluoro-adenosine
  modified_base 10: mod_base = OTHER; note = 2'-Fluoro-uridine
  modified_base 11: mod_base = OTHER; note = 2'-Fluoro-uridine
  modified_base 12: mod_base = cm
  modified_base 13: mod_base = cm
  modified_base 14: mod_base = gm
  modified_base 15: mod_base = OTHER; note = 2'-O-methyl-adenosine
  modified_base 16: mod_base = gm
  modified_base 17: mod_base = gm
  modified_base 18: mod_base = cm
  modified_base 19: mod_base = cm
  modified_base 20: mod_base = um
  modified_base 21: mod_base = cm
gaaagggaattccgaggcctc

SEQ ID NO: 1237 - RNA, 21 nt, synthetic construct
  source 1..21: mol_type = other RNA
  modified_base <1: mod_base = OTHER; note = two inverted abasic nucleosides
  modified_base 1: mod_base = gm
  misc_feature 1^2: note = Phosphorothioate bond
  modified_base 2: mod_base = um
  misc_feature 2^3: note = Phosphorothioate bond
  modified_base 3: mod_base = um
  modified_base 4: mod_base = gm
  modified_base 5: mod_base = um
  modified_base 6: mod_base = OTHER; note = 2'-O-methyl-adenosine
  modified_base 7: mod_base = um
  modified_base 8: mod_base = um
  modified_base 9: mod_base = OTHER; note = 2'-Fluoro-adenosine
  modified_base 10: mod_base = OTHER; note = 2'-Fluoro-uridine
  modified_base 11: mod_base = OTHER; note = 2'-Fluoro-adenosine
  modified_base 12: mod_base = um
  modified_base 13: mod_base = OTHER; note = 2'-O-methyl-adenosine
  modified_base 14: mod_base = OTHER; note = 2'-O-methyl-adenosine
  modified_base 15: mod_base = cm
  modified_base 16: mod_base = OTHER; note = 2'-O-methyl-adenosine
  modified_base 17: mod_base = um
  modified_base 18: mod_base = OTHER; note = 2'-O-methyl-adenosine
  modified_base 19: mod_base = um
  modified_base 20: mod_base = cm
  modified_base 21: mod_base = um
gttgtattatataacatatct

SEQ ID NO: 1238 - RNA, 21 nt, synthetic construct
  source 1..21: mol_type = other RNA
  modified_base <1: mod_base = OTHER; note = two inverted abasic nucleosides
  modified_base 1: mod_base = um
  misc_feature 1^2: note = Phosphorothioate bond
  modified_base 2: mod_base = um
  misc_feature 2^3: note = Phosphorothioate bond
  modified_base 3: mod_base = cm
  modified_base 4: mod_base = cm
  modified_base 5: mod_base = gm
  modified_base 6: mod_base = OTHER; note = 2'-O-methyl-adenosine
  modified_base 7: mod_base = gm
  modified_base 8: mod_base = gm
  modified_base 9: mod_base = OTHER; note = 2'-Fluoro-cytidine
  modified_base 10: mod_base = OTHER; note = 2'-Fluoro-cytidine
  modified_base 11: mod_base = OTHER; note = 2'-Fluoro-uridine
  modified_base 12: mod_base = cm
  modified_base 13: mod_base = gm
  modified_base 14: mod_base = gm
  modified_base 15: mod_base = um
  modified_base 16: mod_base = gm
  modified_base 17: mod_base = OTHER; note = 2'-O-methyl-adenosine
  modified_base 18: mod_base = cm
  modified_base 19: mod_base = um
  modified_base 20: mod_base = gm
  modified_base 21: mod_base = cm
ttccgaggcctcggtgactgc

SEQ ID NO: 1239 - RNA, 21 nt, synthetic construct
  source 1..21: mol_type = other RNA
  modified_base <1: mod_base = OTHER; note = two inverted abasic nucleosides
  modified_base 1: mod_base = OTHER; note = 2'-O-methyl-adenosine
  misc_feature 1^2: note = Phosphorothioate bond
  modified_base 2: mod_base = OTHER; note = 2'-O-methyl-adenosine
  misc_feature 2^3: note = Phosphorothioate bond
  modified_base 3: mod_base = OTHER; note = 2'-O-methyl-adenosine
  modified_base 4: mod_base = gm
  modified_base 5: mod_base = gm
  modified_base 6: mod_base = gm
  modified_base 7: mod_base = OTHER; note = 2'-O-methyl-adenosine
  modified_base 8: mod_base = OTHER; note = 2'-O-methyl-adenosine
  modified_base 9: mod_base = OTHER; note = 2'-Fluoro-uridine
  modified_base 10: mod_base = OTHER; note = 2'-Fluoro-uridine
  modified_base 11: mod_base = OTHER; note = 2'-Fluoro-cytidine
  modified_base 12: mod_base = cm
  modified_base 13: mod_base = gm
  modified_base 14: mod_base = OTHER; note = 2'-O-methyl-adenosine
  modified_base 15: mod_base = gm
  modified_base 16: mod_base = gm
  modified_base 17: mod_base = cm
  modified_base 18: mod_base = cm
  modified_base 19: mod_base = um
  modified_base 20: mod_base = cm
  modified_base 21: mod_base = gm
aaagggaattccgaggcctcg

SEQ ID NO: 1240 - RNA, 21 nt, synthetic construct
  source 1..21: mol_type = other RNA
  modified_base <1: mod_base = OTHER; note = two inverted abasic nucleosides
  modified_base 1: mod_base = um
  misc_feature 1^2: note = Phosphorothioate bond
  modified_base 2: mod_base = gm
  misc_feature 2^3: note = Phosphorothioate bond
  modified_base 3: mod_base = um
  modified_base 4: mod_base = OTHER; note = 2'-O-methyl-adenosine
  modified_base 5: mod_base = um
  modified_base 6: mod_base = um
  modified_base 7: mod_base = OTHER; note = 2'-O-methyl-adenosine
  modified_base 8: mod_base = um
  modified_base 9: mod_base = OTHER; note = 2'-Fluoro-adenosine
  modified_base 10: mod_base = OTHER; note = 2'-Fluoro-uridine
  modified_base 11: mod_base = OTHER; note = 2'-Fluoro-adenosine
  modified_base 12: mod_base = OTHER; note = 2'-O-methyl-adenosine
  modified_base 13: mod_base = cm
  modified_base 14: mod_base = OTHER; note = 2'-O-methyl-adenosine
  modified_base 15: mod_base = um
  modified_base 16: mod_base = OTHER; note = 2'-O-methyl-adenosine
  modified_base 17: mod_base = um
  modified_base 18: mod_base = cm
  modified_base 19: mod_base = um
  modified_base 20: mod_base = um
  modified_base 21: mod_base = gm
tgtattatataacatatcttg

SEQ ID NO: 1241 - RNA, 21 nt, synthetic construct
  source 1..21: mol_type = other RNA
  modified_base <1: mod_base = OTHER; note = two inverted abasic nucleosides
  modified_base 1: mod_base = OTHER; note = 2'-O-methyl-adenosine
  misc_feature 1^2: note = Phosphorothioate bond
  modified_base 2: mod_base = OTHER; note = 2'-O-methyl-adenosine
  misc_feature 2^3: note = Phosphorothioate bond
  modified_base 3: mod_base = um
  modified_base 4: mod_base = um
  modified_base 5: mod_base = cm
  modified_base 6: mod_base = cm
  modified_base 7: mod_base = gm
  modified_base 8: mod_base = OTHER; note = 2'-O-methyl-adenosine
  modified_base 9: mod_base = OTHER; note = 2'-Fluoro-guanosine
  modified_base 10: mod_base = OTHER; note = 2'-Fluoro-guanosine
  modified_base 11: mod_base = OTHER; note = 2'-Fluoro-cytidine
  modified_base 12: mod_base = cm
  modified_base 13: mod_base = um
  modified_base 14: mod_base = cm
  modified_base 15: mod_base = gm
  modified_base 16: mod_base = gm
  modified_base 17: mod_base = um
  modified_base 18: mod_base = gm
  modified_base 19: mod_base = OTHER; note = 2'-O-methyl-adenosine
  modified_base 20: mod_base = cm
  modified_base 21: mod_base = um
aattccgaggcctcggtgact

SEQ ID NO: 1242 - RNA, 21 nt, synthetic construct
  source 1..21: mol_type = other RNA
  modified_base <1: mod_base = OTHER; note = two inverted abasic nucleosides
  modified_base 1: mod_base = gm
  misc_feature 1^2: note = Phosphorothioate bond
  modified_base 2: mod_base = gm
  misc_feature 2^3: note = Phosphorothioate bond
  modified_base 3: mod_base = gm
  modified_base 4: mod_base = OTHER; note = 2'-O-methyl-adenosine
  modified_base 5: mod_base = OTHER; note = 2'-O-methyl-adenosine
  modified_base 6: mod_base = um
  modified_base 7: mod_base = um
  modified_base 8: mod_base = cm
  modified_base 9: mod_base = OTHER; note = 2'-Fluoro-cytidine
  modified_base 10: mod_base = OTHER; note = 2'-Fluoro-guanosine
  modified_base 11: mod_base = OTHER; note = 2'-Fluoro-adenosine
  modified_base 12: mod_base = gm
  modified_base 13: mod_base = gm
  modified_base 14: mod_base = cm
  modified_base 15: mod_base = cm
  modified_base 16: mod_base = um
  modified_base 17: mod_base = cm
  modified_base 18: mod_base = gm
  modified_base 19: mod_base = gm
  modified_base 20: mod_base = um
  modified_base 21: mod_base = gm
gggaattccgaggcctcggtg

SEQ ID NO: 1243 - RNA, 21 nt, synthetic construct
  source 1..21: mol_type = other RNA
  modified_base <1: mod_base = OTHER; note = two inverted abasic nucleosides
  modified_base 1: mod_base = OTHER; note = 2'-O-methyl-adenosine
  misc_feature 1^2: note = Phosphorothioate bond
  modified_base 2: mod_base = gm
  misc_feature 2^3: note = Phosphorothioate bond
  modified_base 3: mod_base = cm
  modified_base 4: mod_base = um
  modified_base 5: mod_base = gm
  modified_base 6: mod_base = OTHER; note = 2'-O-methyl-adenosine
  modified_base 7: mod_base = OTHER; note = 2'-O-methyl-adenosine
  modified_base 8: mod_base = OTHER; note = 2'-O-methyl-adenosine
  modified_base 9: mod_base = OTHER; note = 2'-Fluoro-guanosine
  modified_base 10: mod_base = OTHER; note = 2'-Fluoro-guanosine
  modified_base 11: mod_base = OTHER; note = 2'-Fluoro-guanosine
  modified_base 12: mod_base = OTHER; note = 2'-O-methyl-adenosine
  modified_base 13: mod_base = OTHER; note = 2'-O-methyl-adenosine
  modified_base 14: mod_base = um
  modified_base 15: mod_base = um
  modified_base 16: mod_base = cm
  modified_base 17: mod_base = cm
  modified_base 18: mod_base = gm
  modified_base 19: mod_base = OTHER; note = 2'-O-methyl-adenosine
  modified_base 20: mod_base = gm
  modified_base 21: mod_base = gm
agctgaaagggaattccgagg

SEQ ID NO: 1244 - RNA, 21 nt, synthetic construct
  source 1..21: mol_type = other RNA
  modified_base <1: mod_base = OTHER; note = two inverted abasic nucleosides
  modified_base 1: mod_base = gm
  misc_feature 1^2: note = Phosphorothioate bond
  modified_base 2: mod_base = gm
  misc_feature 2^3: note = Phosphorothioate bond
  modified_base 3: mod_base = OTHER; note = 2'-O-methyl-adenosine
  modified_base 4: mod_base = gm
  modified_base 5: mod_base = cm
  modified_base 6: mod_base = um
  modified_base 7: mod_base = gm
  modified_base 8: mod_base = OTHER; note = 2'-O-methyl-adenosine
  modified_base 9: mod_base = OTHER; note = 2'-Fluoro-adenosine
  modified_base 10: mod_base = OTHER; note = 2'-Fluoro-adenosine
  modified_base 11: mod_base = OTHER; note = 2'-Fluoro-guanosine
  modified_base 12: mod_base = gm
  modified_base 13: mod_base = gm
  modified_base 14: mod_base = OTHER; note = 2'-O-methyl-adenosine
  modified_base 15: mod_base = OTHER; note = 2'-O-methyl-adenosine
  modified_base 16: mod_base = um
  modified_base 17: mod_base = um
  modified_base 18: mod_base = cm
  modified_base 19: mod_base = cm
  modified_base 20: mod_base = gm
  modified_base 21: mod_base = OTHER; note = 2'-O-methyl-adenosine
ggagctgaaagggaattccga

SEQ ID NO: 1245 - RNA, 21 nt, synthetic construct
  source 1..21: mol_type = other RNA
  modified_base <1: mod_base = OTHER; note = two inverted abasic nucleosides
  modified_base 1: mod_base = cm
  misc_feature 1^2: note = Phosphorothioate bond
  modified_base 2: mod_base = um
  misc_feature 2^3: note = Phosphorothioate bond
  modified_base 3: mod_base = gm
  modified_base 4: mod_base = OTHER; note = 2'-O-methyl-adenosine
  modified_base 5: mod_base = OTHER; note = 2'-O-methyl-adenosine
  modified_base 6: mod_base = OTHER; note = 2'-O-methyl-adenosine
  modified_base 7: mod_base = gm
  modified_base 8: mod_base = gm
  modified_base 9: mod_base = OTHER; note = 2'-Fluoro-guanosine
  modified_base 10: mod_base = OTHER; note = 2'-Fluoro-adenosine
  modified_base 11: mod_base = OTHER; note = 2'-Fluoro-adenosine
  modified_base 12: mod_base = um
  modified_base 13: mod_base = um
  modified_base 14: mod_base = cm
  modified_base 15: mod_base = cm
  modified_base 16: mod_base = gm
  modified_base 17: mod_base = OTHER; note = 2'-O-methyl-adenosine
  modified_base 18: mod_base = gm
  modified_base 19: mod_base = gm
  modified_base 20: mod_base = cm
  modified_base 21: mod_base = cm
ctgaaagggaattccgaggcc

SEQ ID NO: 1246 - RNA, 21 nt, synthetic construct
  source 1..21: mol_type = other RNA
  modified_base <1: mod_base = OTHER; note = two inverted abasic nucleosides
  modified_base 1: mod_base = gm
  misc_feature 1^2: note = Phosphorothioate bond
  modified_base 2: mod_base = OTHER; note = 2'-O-methyl-adenosine
  misc_feature 2^3: note = Phosphorothioate bond
  modified_base 3: mod_base = gm
  modified_base 4: mod_base = cm
  modified_base 5: mod_base = um
  modified_base 6: mod_base = gm
  modified_base 7: mod_base = OTHER; note = 2'-O-methyl-adenosine
  modified_base 8: mod_base = OTHER; note = 2'-O-methyl-adenosine
  modified_base 9: mod_base = OTHER; note = 2'-Fluoro-adenosine
  modified_base 10: mod_base = OTHER; note = 2'-Fluoro-guanosine
  modified_base 11: mod_base = OTHER; note = 2'-Fluoro-guanosine
  modified_base 12: mod_base = gm
  modified_base 13: mod_base = OTHER; note = 2'-O-methyl-adenosine
  modified_base 14: mod_base = OTHER; note = 2'-O-methyl-adenosine
  modified_base 15: mod_base = um
  modified_base 16: mod_base = um
  modified_base 17: mod_base = cm
  modified_base 18: mod_base = cm
  modified_base 19: mod_base = gm
  modified_base 20: mod_base = OTHER; note = 2'-O-methyl-adenosine
  modified_base 21: mod_base = gm
gagctgaaagggaattccgag

SEQ ID NO: 1247 - RNA, 21 nt, synthetic construct
  source 1..21: mol_type = other RNA
  modified_base <1: mod_base = OTHER; note = two inverted abasic nucleosides
  modified_base 1: mod_base = gm
  misc_feature 1^2: note = Phosphorothioate bond
  modified_base 2: mod_base = cm
  misc_feature 2^3: note = Phosphorothioate bond
  modified_base 3: mod_base = um
  modified_base 4: mod_base = gm
  modified_base 5: mod_base = OTHER; note = 2'-O-methyl-adenosine
  modified_base 6: mod_base = OTHER; note = 2'-O-methyl-adenosine
  modified_base 7: mod_base = OTHER; note = 2'-O-methyl-adenosine
  modified_base 8: mod_base = gm
  modified_base 9: mod_base = OTHER; note = 2'-Fluoro-guanosine
  modified_base 10: mod_base = OTHER; note = 2'-Fluoro-guanosine
  modified_base 11: mod_base = OTHER; note = 2'-Fluoro-adenosine
  modified_base 12: mod_base = OTHER; note = 2'-O-methyl-adenosine
  modified_base 13: mod_base = um
  modified_base 14: mod_base = um
  modified_base 15: mod_base = cm
  modified_base 16: mod_base = cm
  modified_base 17: mod_base = gm
  modified_base 18: mod_base = OTHER; note = 2'-O-methyl-adenosine
  modified_base 19: mod_base = gm
  modified_base 20: mod_base = gm
  modified_base 21: mod_base = cm
gctgaaagggaattccgaggc

SEQ ID NO: 1248 - RNA, 21 nt, synthetic construct
  source 1..21: mol_type = other RNA
  modified_base <1: mod_base = OTHER; note = two inverted abasic nucleosides
  modified_base 1: mod_base = gm
  misc_feature 1^2: note = Phosphorothioate bond
  modified_base 2: mod_base = cm
  misc_feature 2^3: note = Phosphorothioate bond
  modified_base 3: mod_base = OTHER; note = 2'-O-methyl-adenosine
  modified_base 4: mod_base = um
  modified_base 5: mod_base = gm
  modified_base 6: mod_base = um
  modified_base 7: mod_base = um
  modified_base 8: mod_base = gm
  modified_base 9: mod_base = OTHER; note = 2'-Fluoro-uridine
  modified_base 10: mod_base = OTHER; note = 2'-Fluoro-adenosine
  modified_base 11: mod_base = OTHER; note = 2'-Fluoro-uridine
  modified_base 12: mod_base = um
  modified_base 13: mod_base = OTHER; note = 2'-O-methyl-adenosine
  modified_base 14: mod_base = um
  modified_base 15: mod_base = OTHER; note = 2'-O-methyl-adenosine
  modified_base 16: mod_base = um
  modified_base 17: mod_base = OTHER; note = 2'-O-methyl-adenosine
  modified_base 18: mod_base = OTHER; note = 2'-O-methyl-adenosine
  modified_base 19: mod_base = cm
  modified_base 20: mod_base = OTHER; note = 2'-O-methyl-adenosine
  modified_base 21: mod_base = um
gcatgttgtattatataacat

SEQ ID NO: 1249 - RNA, 21 nt, synthetic construct
  source 1..21: mol_type = other RNA
  modified_base <1: mod_base = OTHER; note = two inverted abasic nucleosides
  modified_base 1: mod_base = um
  misc_feature 1^2: note = Phosphorothioate bond
  modified_base 2: mod_base = um
  misc_feature 2^3: note = Phosphorothioate bond
  modified_base 3: mod_base = gm
  modified_base 4: mod_base = um
  modified_base 5: mod_base = OTHER; note = 2'-O-methyl-adenosine
  modified_base 6: mod_base = um
  modified_base 7: mod_base = um
  modified_base 8: mod_base = OTHER; note = 2'-O-methyl-adenosine
  modified_base 9: mod_base = OTHER; note = 2'-Fluoro-uridine
  modified_base 10: mod_base = OTHER; note = 2'-Fluoro-adenosine
  modified_base 11: mod_base = OTHER; note = 2'-Fluoro-uridine
  modified_base 12: mod_base = OTHER; note = 2'-O-methyl-adenosine
  modified_base 13: mod_base = OTHER; note = 2'-O-methyl-adenosine
  modified_base 14: mod_base = cm
  modified_base 15: mod_base = OTHER; note = 2'-O-methyl-adenosine
  modified_base 16: mod_base = um
  modified_base 17: mod_base = OTHER; note = 2'-O-methyl-adenosine
  modified_base 18: mod_base = um
  modified_base 19: mod_base = cm
  modified_base 20: mod_base = um
  modified_base 21: mod_base = um
ttgtattatataacatatctt

SEQ ID NO: 1250 - RNA, 21 nt, synthetic construct
  source 1..21: mol_type = other RNA
  modified_base <1: mod_base = OTHER; note = two inverted abasic nucleosides
  modified_base 1: mod_base = gm
  misc_feature 1^2: note = Phosphorothioate bond
  modified_base 2: mod_base = um
  misc_feature 2^3: note = Phosphorothioate bond
  modified_base 3: mod_base = OTHER; note = 2'-O-methyl-adenosine
  modified_base 4: mod_base = um
  modified_base 5: mod_base = um
  modified_base 6: mod_base = OTHER; note = 2'-O-methyl-adenosine
  modified_base 7: mod_base = um
  modified_base 8: mod_base = OTHER; note = 2'-O-methyl-adenosine
  modified_base 9: mod_base = OTHER; note = 2'-Fluoro-uridine
  modified_base 10: mod_base = OTHER; note = 2'-Fluoro-adenosine
  modified_base 11: mod_base = OTHER; note = 2'-Fluoro-adenosine
  modified_base 12: mod_base = cm
  modified_base 13: mod_base = OTHER; note = 2'-O-methyl-adenosine
  modified_base 14: mod_base = um
  modified_base 15: mod_base = OTHER; note = 2'-O-methyl-adenosine
  modified_base 16: mod_base = um
  modified_base 17: mod_base = cm
  modified_base 18: mod_base = um
  modified_base 19: mod_base = um
  modified_base 20: mod_base = gm
  modified_base 21: mod_base = OTHER; note = 2'-O-methyl-adenosine
gtattatataacatatcttga

SEQ ID NO: 1251 - RNA, 21 nt, synthetic construct
  source 1..21: mol_type = other RNA
  modified_base <1: mod_base = OTHER; note = two inverted abasic nucleosides
  modified_base 1: mod_base = gm
  misc_feature 1^2: note = Phosphorothioate bond
  modified_base 2: mod_base = gm
  misc_feature 2^3: note = Phosphorothioate bond
  modified_base 3: mod_base = cm
  modified_base 4: mod_base = OTHER; note = 2'-O-methyl-adenosine
  modified_base 5: mod_base = um
  modified_base 6: mod_base = gm
  modified_base 7: mod_base = um
  modified_base 8: mod_base = um
  modified_base 9: mod_base = OTHER; note = 2'-Fluoro-guanosine
  modified_base 10: mod_base = OTHER; note = 2'-Fluoro-uridine
  modified_base 11: mod_base = OTHER; note = 2'-Fluoro-adenosine
  modified_base 12: mod_base = um
  modified_base 13: mod_base = um
  modified_base 14: mod_base = OTHER; note = 2'-O-methyl-adenosine
  modified_base 15: mod_base = um
  modified_base 16: mod_base = OTHER; note = 2'-O-methyl-adenosine
  modified_base 17: mod_base = um
  modified_base 18: mod_base = OTHER; note = 2'-O-methyl-adenosine
  modified_base 19: mod_base = OTHER; note = 2'-O-methyl-adenosine
  modified_base 20: mod_base = cm
  modified_base 21: mod_base = OTHER; note = 2'-O-methyl-adenosine
ggcatgttgtattatataaca

SEQ ID NO: 1252 - RNA, 21 nt, synthetic construct
  source 1..21: mol_type = other RNA
  modified_base <1: mod_base = OTHER; note = two inverted abasic nucleosides
  modified_base 1: mod_base = OTHER; note = 2'-O-methyl-adenosine
  misc_feature 1^2: note = Phosphorothioate bond
  modified_base 2: mod_base = OTHER; note = 2'-O-methyl-adenosine
  misc_feature 2^3: note = Phosphorothioate bond
  modified_base 3: mod_base = gm
  modified_base 4: mod_base = gm
  modified_base 5: mod_base = gm
  modified_base 6: mod_base = OTHER; note = 2'-O-methyl-adenosine
  modified_base 7: mod_base = OTHER; note = 2'-O-methyl-adenosine
  modified_base 8: mod_base = um
  modified_base 9: mod_base = OTHER; note = 2'-Fluoro-uridine
  modified_base 10: mod_base = OTHER; note = 2'-Fluoro-cytidine
  modified_base 11: mod_base = OTHER; note = 2'-Fluoro-cytidine
  modified_base 12: mod_base = gm
  modified_base 13: mod_base = OTHER; note = 2'-O-methyl-adenosine
  modified_base 14: mod_base = gm
  modified_base 15: mod_base = gm
  modified_base 16: mod_base = cm
  modified_base 17: mod_base = cm
  modified_base 18: mod_base = um
  modified_base 19: mod_base = cm
  modified_base 20: mod_base = gm
  modified_base 21: mod_base = gm
aagggaattccgaggcctcgg

SEQ ID NO: 1253 - RNA, 21 nt, synthetic construct
  source 1..21: mol_type = other RNA
  modified_base <1: mod_base = OTHER; note = two inverted abasic nucleosides
  modified_base 1: mod_base = gm
  misc_feature 1^2: note = Phosphorothioate bond
  modified_base 2: mod_base = OTHER; note = 2'-O-methyl-adenosine
  misc_feature 2^3: note = Phosphorothioate bond
  modified_base 3: mod_base = OTHER; note = 2'-O-methyl-adenosine
  modified_base 4: mod_base = um
  modified_base 5: mod_base = um
  modified_base 6: mod_base = cm
  modified_base 7: mod_base = cm
  modified_base 8: mod_base = gm
  modified_base 9: mod_base = OTHER; note = 2'-Fluoro-adenosine
  modified_base 10: mod_base = OTHER; note = 2'-Fluoro-guanosine
  modified_base 11: mod_base = OTHER; note = 2'-Fluoro-guanosine
  modified_base 12: mod_base = cm
  modified_base 13: mod_base = cm
  modified_base 14: mod_base = um
  modified_base 15: mod_base = cm
  modified_base 16: mod_base = gm
  modified_base 17: mod_base = gm
  modified_base 18: mod_base = um
  modified_base 19: mod_base = gm
  modified_base 20: mod_base = OTHER; note = 2'-O-methyl-adenosine
  modified_base 21: mod_base = cm
gaattccgaggcctcggtgac

SEQ ID NO: 1254 - RNA, 21 nt, synthetic construct
  source 1..21: mol_type = other RNA
  modified_base <1: mod_base = OTHER; note = two inverted abasic nucleosides
  modified_base 1: mod_base = OTHER; note = 2'-O-methyl-adenosine
  misc_feature 1^2: note = Phosphorothioate bond
  modified_base 2: mod_base = gm
  misc_feature 2^3: note = Phosphorothioate bond
  modified_base 3: mod_base = gm
  modified_base 4: mod_base = gm
  modified_base 5: mod_base = OTHER; note = 2'-O-methyl-adenosine
  modified_base 6: mod_base = OTHER; note = 2'-O-methyl-adenosine
  modified_base 7: mod_base = um
  modified_base 8: mod_base = um
  modified_base 9: mod_base = OTHER; note = 2'-Fluoro-cytidine
  modified_base 10: mod_base = OTHER; note = 2'-Fluoro-cytidine
  modified_base 11: mod_base = OTHER; note = 2'-Fluoro-guanosine
  modified_base 12: mod_base = OTHER; note = 2'-O-methyl-adenosine
  modified_base 13: mod_base = gm
  modified_base 14: mod_base = gm
  modified_base 15: mod_base = cm
  modified_base 16: mod_base = cm
  modified_base 17: mod_base = um
  modified_base 18: mod_base = cm
  modified_base 19: mod_base = gm
  modified_base 20: mod_base = gm
  modified_base 21: mod_base = um
agggaattccgaggcctcggt

SEQ ID NO: 1255 - RNA, 21 nt, synthetic construct
  source 1..21: mol_type = other RNA
  modified_base <1: mod_base = OTHER; note = two inverted abasic nucleosides
  modified_base 1: mod_base = gm
  misc_feature 1^2: note = Phosphorothioate bond
  modified_base 2: mod_base = gm
  misc_feature 2^3: note = Phosphorothioate bond
  modified_base 3: mod_base = OTHER; note = 2'-O-methyl-adenosine
  modified_base 4: mod_base = OTHER; note = 2'-O-methyl-adenosine
  modified_base 5: mod_base = um
  modified_base 6: mod_base = um
  modified_base 7: mod_base = cm
  modified_base 8: mod_base = cm
  modified_base 9: mod_base = OTHER; note = 2'-Fluoro-guanosine
  modified_base 10: mod_base = OTHER; note = 2'-Fluoro-adenosine
  modified_base 11: mod_base = OTHER; note = 2'-Fluoro-guanosine
  modified_base 12: mod_base = gm
  modified_base 13: mod_base = cm
  modified_base 14: mod_base = cm
  modified_base 15: mod_base = um
  modified_base 16: mod_base = cm
  modified_base 17: mod_base = gm
  modified_base 18: mod_base = gm
  modified_base 19: mod_base = um
  modified_base 20: mod_base = gm
  modified_base 21: mod_base = OTHER; note = 2'-O-methyl-adenosine
ggaattccgaggcctcggtga

SEQ ID NO: 1256 - RNA, 21 nt, synthetic construct
  source 1..21: mol_type = other RNA
  modified_base <1: mod_base = OTHER; note = two inverted abasic nucleosides
  modified_base 1: mod_base = gm
  misc_feature 1^2: note = Phosphorothioate bond
  modified_base 2: mod_base = cm
  misc_feature 2^3: note = Phosphorothioate bond
  modified_base 3: mod_base = um
  modified_base 4: mod_base = um
  modified_base 5: mod_base = gm
  modified_base 6: mod_base = um
  modified_base 7: mod_base = cm
  modified_base 8: mod_base = um
  modified_base 9: mod_base = OTHER; note = 2'-Fluoro-uridine
  modified_base 10: mod_base = OTHER; note = 2'-Fluoro-guanosine
  modified_base 11: mod_base = OTHER; note = 2'-Fluoro-uridine
  modified_base 12: mod_base = OTHER; note = 2'-O-methyl-adenosine
  modified_base 13: mod_base = um
  modified_base 14: mod_base = gm
  modified_base 15: mod_base = OTHER; note = 2'-O-methyl-adenosine
  modified_base 16: mod_base = um
  modified_base 17: mod_base = gm
  modified_base 18: mod_base = OTHER; note = 2'-O-methyl-adenosine
  modified_base 19: mod_base = OTHER; note = 2'-O-methyl-adenosine
  modified_base 20: mod_base = OTHER; note = 2'-O-methyl-adenosine
  modified_base 21: mod_base = um
gcttgtcttgtatgatgaaat

SEQ ID NO: 1257 - RNA, 21 nt, synthetic construct
  source 1..21: mol_type = other RNA
  modified_base <1: mod_base = OTHER; note = two inverted abasic nucleosides
  modified_base 1: mod_base = um
  misc_feature 1^2: note = Phosphorothioate bond
  modified_base 2: mod_base = cm
  misc_feature 2^3: note = Phosphorothioate bond
  modified_base 3: mod_base = gm
  modified_base 4: mod_base = cm
  modified_base 5: mod_base = cm
  modified_base 6: mod_base = um
  modified_base 7: mod_base = um
  modified_base 8: mod_base = cm
  modified_base 9: mod_base = OTHER; note = 2'-Fluoro-adenosine
  modified_base 10: mod_base = OTHER; note = 2'-Fluoro-adenosine
  modified_base 11: mod_base = OTHER; note = 2'-Fluoro-adenosine
  modified_base 12: mod_base = gm
  modified_base 13: mod_base = OTHER; note = 2'-O-methyl-adenosine
  modified_base 14: mod_base = um
  modified_base 15: mod_base = OTHER; note = 2'-O-methyl-adenosine
  modified_base 16: mod_base = OTHER; note = 2'-O-methyl-adenosine
  modified_base 17: mod_base = OTHER; note = 2'-O-methyl-adenosine
  modified_base 18: mod_base = um
  modified_base 19: mod_base = OTHER; note = 2'-O-methyl-adenosine
  modified_base 20: mod_base = cm
  modified_base 21: mod_base = OTHER; note = 2'-O-methyl-adenosine
tcgccttcaaagataaataca

SEQ ID NO: 1258 - RNA, 21 nt, synthetic construct
  source 1..21: mol_type = other RNA
  modified_base <1: mod_base = OTHER; note = two inverted abasic nucleosides
  modified_base 1: mod_base = gm
  misc_feature 1^2: note = Phosphorothioate bond
  modified_base 2: mod_base = cm
  misc_feature 2^3: note = Phosphorothioate bond
  modified_base 3: mod_base = cm
  modified_base 4: mod_base = um
  modified_base 5: mod_base = gm
  modified_base 6: mod_base = gm
  modified_base 7: mod_base = um
  modified_base 8: mod_base = um
  modified_base 9: mod_base = OTHER; note = 2'-Fluoro-adenosine
  modified_base 10: mod_base = OTHER; note = 2'-Fluoro-adenosine
  modified_base 11: mod_base = OTHER; note = 2'-Fluoro-guanosine
  modified_base 12: mod_base = OTHER; note = 2'-O-methyl-adenosine
  modified_base 13: mod_base = um
  modified_base 14: mod_base = cm
  modified_base 15: mod_base = um
  modified_base 16: mod_base = OTHER; note = 2'-O-methyl-adenosine
  modified_base 17: mod_base = cm
  modified_base 18: mod_base = OTHER; note = 2'-O-methyl-adenosine
  modified_base 19: mod_base = OTHER; note = 2'-O-methyl-adenosine
  modified_base 20: mod_base = OTHER; note = 2'-O-methyl-adenosine
  modified_base 21: mod_base = um
gcctggttaagatctacaaat

SEQ ID NO: 1259 - RNA, 21 nt, synthetic construct
  source 1..21: mol_type = other RNA
  modified_base <1: mod_base = OTHER; note = two inverted abasic nucleosides
  modified_base 1: mod_base = um
  misc_feature 1^2: note = Phosphorothioate bond
  modified_base 2: mod_base = cm
  misc_feature 2^3: note = Phosphorothioate bond
  modified_base 3: mod_base = um
  modified_base 4: mod_base = OTHER; note = 2'-O-methyl-adenosine
  modified_base 5: mod_base = um
  modified_base 6: mod_base = gm
  modified_base 7: mod_base = OTHER; note = 2'-O-methyl-adenosine
  modified_base 8: mod_base = cm
  modified_base 9: mod_base = OTHER; note = 2'-Fluoro-adenosine
  modified_base 10: mod_base = OTHER; note = 2'-Fluoro-cytidine
  modified_base 11: mod_base = OTHER; note = 2'-Fluoro-uridine
  modified_base 12: mod_base = gm
  modified_base 13: mod_base = cm
  modified_base 14: mod_base = OTHER; note = 2'-O-methyl-adenosine
  modified_base 15: mod_base = OTHER; note = 2'-O-methyl-adenosine
  modified_base 16: mod_base = OTHER; note = 2'-O-methyl-adenosine
  modified_base 17: mod_base = gm
  modified_base 18: mod_base = gm
  modified_base 19: mod_base = gm
  modified_base 20: mod_base = OTHER; note = 2'-O-methyl-adenosine
  modified_base 21: mod_base = OTHER; note = 2'-O-methyl-adenosine
tctatgacactgcaaagggaa

SEQ ID NO: 1260 - RNA, 21 nt, synthetic construct
  source 1..21: mol_type = other RNA
  modified_base <1: mod_base = OTHER; note = two inverted abasic nucleosides
  modified_base 1: mod_base = um
  misc_feature 1^2: note = Phosphorothioate bond
  modified_base 2: mod_base = um
  misc_feature 2^3: note = Phosphorothioate bond
  modified_base 3: mod_base = um
  modified_base 4: mod_base = gm
  modified_base 5: mod_base = um
  modified_base 6: mod_base = gm
  modified_base 7: mod_base = cm
  modified_base 8: mod_base = um
  modified_base 9: mod_base = OTHER; note = 2'-Fluoro-uridine
  modified_base 10: mod_base = OTHER; note = 2'-Fluoro-guanosine
  modified_base 11: mod_base = OTHER; note = 2'-Fluoro-uridine
  modified_base 12: mod_base = cm
  modified_base 13: mod_base = um
  modified_base 14: mod_base = um
  modified_base 15: mod_base = gm
  modified_base 16: mod_base = um
  modified_base 17: mod_base = OTHER; note = 2'-O-methyl-adenosine
  modified_base 18: mod_base = um
  modified_base 19: mod_base = gm
  modified_base 20: mod_base = OTHER; note = 2'-O-methyl-adenosine
  modified_base 21: mod_base = um
tttgtgcttgtcttgtatgat

SEQ ID NO: 1261 - RNA, 21 nt, synthetic construct
  source 1..21: mol_type = other RNA
  modified_base <1: mod_base = OTHER; note = two inverted abasic nucleosides
  modified_base 1: mod_base = um
  misc_feature 1^2: note = Phosphorothioate bond
  modified_base 2: mod_base = gm
  misc_feature 2^3: note = Phosphorothioate bond
  modified_base 3: mod_base = OTHER; note = 2'-O-methyl-adenosine
  modified_base 4: mod_base = cm
  modified_base 5: mod_base = um
  modified_base 6: mod_base = gm
  modified_base 7: mod_base = cm
  modified_base 8: mod_base = cm
  modified_base 9: mod_base = OTHER; note = 2'-Fluoro-uridine
  modified_base 10: mod_base = OTHER; note = 2'-Fluoro-guanosine
  modified_base 11: mod_base = OTHER; note = 2'-Fluoro-guanosine
  modified_base 12: mod_base = um
  modified_base 13: mod_base = um
  modified_base 14: mod_base = OTHER; note = 2'-O-methyl-adenosine
  modified_base 15: mod_base = OTHER; note = 2'-O-methyl-adenosine
  modified_base 16: mod_base = gm
  modified_base 17: mod_base = OTHER; note = 2'-O-methyl-adenosine
  modified_base 18: mod_base = um
  modified_base 19: mod_base = cm
  modified_base 20: mod_base = um
  modified_base 21: mod_base = OTHER; note = 2'-O-methyl-adenosine
tgactgcctggttaagatcta

SEQ ID NO: 1262 - RNA, 21 nt, synthetic construct
  source 1..21: mol_type = other RNA
  modified_base <1: mod_base = OTHER; note = two inverted abasic nucleosides
  modified_base 1: mod_base = gm
  misc_feature 1^2: note = Phosphorothioate bond
  modified_base 2: mod_base = OTHER; note = 2'-O-methyl-adenosine
  misc_feature 2^3: note = Phosphorothioate bond
  modified_base 3: mod_base = cm
  modified_base 4: mod_base = OTHER; note = 2'-O-methyl-adenosine
  modified_base 5: mod_base = cm
  modified_base 6: mod_base = um
  modified_base 7: mod_base = gm
  modified_base 8: mod_base = cm
  modified_base 9: mod_base = OTHER; note = 2'-Fluoro-adenosine
  modified_base 10: mod_base = OTHER; note = 2'-Fluoro-adenosine
  modified_base 11: mod_base = OTHER; note = 2'-Fluoro-adenosine
  modified_base 12: mod_base = gm
  modified_base 13: mod_base = gm
  modified_base 14: mod_base = gm
  modified_base 15: mod_base = OTHER; note = 2'-O-methyl-adenosine
  modified_base 16: mod_base = OTHER; note = 2'-O-methyl-adenosine
  modified_base 17: mod_base = um
  modified_base 18: mod_base = gm
  modified_base 19: mod_base = cm
  modified_base 20: mod_base = um
  modified_base 21: mod_base = um
gacactgcaaagggaatgctt

SEQ ID NO: 1263 - RNA, 21 nt, synthetic construct
  source 1..21: mol_type = other RNA
  modified_base <1: mod_base = OTHER; note = two inverted abasic nucleosides
  modified_base 1: mod_base = cm
  misc_feature 1^2: note = Phosphorothioate bond
  modified_base 2: mod_base = gm
  misc_feature 2^3: note = Phosphorothioate bond
  modified_base 3: mod_base = gm
  modified_base 4: mod_base = um
  modified_base 5: mod_base = OTHER; note = 2'-O-methyl-adenosine
  modified_base 6: mod_base = um
  modified_base 7: mod_base = cm
  modified_base 8: mod_base = um
  modified_base 9: mod_base = OTHER; note = 2'-Fluoro-adenosine
  modified_base 10: mod_base = OTHER; note = 2'-Fluoro-uridine
  modified_base 11: mod_base = OTHER; note = 2'-Fluoro-guanosine
  modified_base 12: mod_base = OTHER; note = 2'-O-methyl-adenosine
  modified_base 13: mod_base = cm
  modified_base 14: mod_base = OTHER; note = 2'-O-methyl-adenosine
  modified_base 15: mod_base = cm
  modified_base 16: mod_base = um
  modified_base 17: mod_base = gm
  modified_base 18: mod_base = cm
  modified_base 19: mod_base = OTHER; note = 2'-O-methyl-adenosine
  modified_base 20: mod_base = OTHER; note = 2'-O-methyl-adenosine
  modified_base 21: mod_base = OTHER; note = 2'-O-methyl-adenosine
cggtatctatgacactgcaaa

SEQ ID NO: 1264 - RNA, 21 nt, synthetic construct
  source 1..21: mol_type = other RNA
  modified_base <1: mod_base = OTHER; note = two inverted abasic nucleosides
  modified_base 1: mod_base = um
  misc_feature 1^2: note = Phosphorothioate bond
  modified_base 2: mod_base = um
  misc_feature 2^3: note = Phosphorothioate bond
  modified_base 3: mod_base = cm
  modified_base 4: mod_base = OTHER; note = 2'-O-methyl-adenosine
  modified_base 5: mod_base = um
  modified_base 6: mod_base = cm
  modified_base 7: mod_base = um
  modified_base 8: mod_base = gm
  modified_base 9: mod_base = OTHER; note = 2'-Fluoro-adenosine
  modified_base 10: mod_base = OTHER; note = 2'-Fluoro-cytidine
  modified_base 11: mod_base = OTHER; note = 2'-Fluoro-cytidine
  modified_base 12: mod_base = OTHER; note = 2'-O-methyl-adenosine
  modified_base 13: mod_base = gm
  modified_base 14: mod_base = um
  modified_base 15: mod_base = um
  modified_base 16: mod_base = um
  modified_base 17: mod_base = um
  modified_base 18: mod_base = cm
  modified_base 19: mod_base = um
  modified_base 20: mod_base = cm
  modified_base 21: mod_base = um
ttcatctgaccagttttctct

SEQ ID NO: 1265 - RNA, 21 nt, synthetic construct
  source 1..21: mol_type = other RNA
  modified_base <1: mod_base = OTHER; note = two inverted abasic nucleosides
  modified_base 1: mod_base = um
  misc_feature 1^2: note = Phosphorothioate bond
  modified_base 2: mod_base = um
  misc_feature 2^3: note = Phosphorothioate bond
  modified_base 3: mod_base = cm
  modified_base 4: mod_base = gm
  modified_base 5: mod_base = gm
  modified_base 6: mod_base = um
  modified_base 7: mod_base = OTHER; note = 2'-O-methyl-adenosine
  modified_base 8: mod_base = um
  modified_base 9: mod_base = OTHER; note = 2'-Fluoro-cytidine
  modified_base 10: mod_base = OTHER; note = 2'-Fluoro-uridine
  modified_base 11: mod_base = OTHER; note = 2'-Fluoro-adenosine
  modified_base 12: mod_base = um
  modified_base 13: mod_base = gm
  modified_base 14: mod_base = OTHER; note = 2'-O-methyl-adenosine
  modified_base 15: mod_base = cm
  modified_base 16: mod_base = OTHER; note = 2'-O-methyl-adenosine
  modified_base 17: mod_base = cm
  modified_base 18: mod_base = um
  modified_base 19: mod_base = gm
  modified_base 20: mod_base = cm
  modified_base 21: mod_base = OTHER; note = 2'-O-methyl-adenosine
ttcggtatctatgacactgca

SEQ ID NO: 1266 - RNA, 21 nt, synthetic construct
  source 1..21: mol_type = other RNA
  modified_base <1: mod_base = OTHER; note = two inverted abasic nucleosides
  modified_base 1: mod_base = gm
  misc_feature 1^2: note = Phosphorothioate bond
  modified_base 2: mod_base = gm
  misc_feature 2^3: note = Phosphorothioate bond
  modified_base 3: mod_base = um
  modified_base 4: mod_base = um
  modified_base 5: mod_base = OTHER; note = 2'-O-methyl-adenosine
  modified_base 6: mod_base = OTHER; note = 2'-O-methyl-adenosine
  modified_base 7: mod_base = gm
  modified_base 8: mod_base = OTHER; note = 2'-O-methyl-adenosine
  modified_base 9: mod_base = OTHER; note = 2'-Fluoro-uridine
  modified_base 10: mod_base = OTHER; note = 2'-Fluoro-cytidine
  modified_base 11: mod_base = OTHER; note = 2'-Fluoro-uridine
  modified_base 12: mod_base = OTHER; note = 2'-O-methyl-adenosine
  modified_base 13: mod_base = cm
  modified_base 14: mod_base = OTHER; note = 2'-O-methyl-adenosine
  modified_base 15: mod_base = OTHER; note = 2'-O-methyl-adenosine
  modified_base 16: mod_base = OTHER; note = 2'-O-methyl-adenosine
  modified_base 17: mod_base = um
  modified_base 18: mod_base = cm
  modified_base 19: mod_base = um
  modified_base 20: mod_base = gm
  modified_base 21: mod_base = OTHER; note = 2'-O-methyl-adenosine
ggttaagatctacaaatctga

SEQ ID NO: 1267 - RNA, 21 nt, synthetic construct
  source 1..21: mol_type = other RNA
  modified_base <1: mod_base = OTHER; note = two inverted abasic nucleosides
  modified_base 1: mod_base = OTHER; note = 2'-O-methyl-adenosine
  misc_feature 1^2: note = Phosphorothioate bond
  modified_base 2: mod_base = um
  misc_feature 2^3: note = Phosphorothioate bond
  modified_base 3: mod_base = cm
  modified_base 4: mod_base = um
  modified_base 5: mod_base = OTHER; note = 2'-O-methyl-adenosine
  modified_base 6: mod_base = um
  modified_base 7: mod_base = gm
  modified_base 8: mod_base = OTHER; note = 2'-O-methyl-adenosine
  modified_base 9: mod_base = OTHER; note = 2'-Fluoro-cytidine
  modified_base 10: mod_base = OTHER; note = 2'-Fluoro-adenosine
  modified_base 11: mod_base = OTHER; note = 2'-Fluoro-cytidine
  modified_base 12: mod_base = um
  modified_base 13: mod_base = gm
  modified_base 14: mod_base = cm
  modified_base 15: mod_base = OTHER; note = 2'-O-methyl-adenosine
  modified_base 16: mod_base = OTHER; note = 2'-O-methyl-adenosine
  modified_base 17: mod_base = OTHER; note = 2'-O-methyl-adenosine
  modified_base 18: mod_base = gm
  modified_base 19: mod_base = gm
  modified_base 20: mod_base = gm
  modified_base 21: mod_base = OTHER; note = 2'-O-methyl-adenosine
atctatgacactgcaaaggga

SEQ ID NO: 1268 - RNA, 21 nt, synthetic construct
  source 1..21: mol_type = other RNA
  modified_base <1: mod_base = OTHER; note = two inverted abasic nucleosides
  modified_base 1: mod_base = OTHER; note = 2'-O-methyl-adenosine
  misc_feature 1^2: note = Phosphorothioate bond
  modified_base 2: mod_base = gm
  misc_feature 2^3: note = Phosphorothioate bond
  modified_base 3: mod_base = gm
  modified_base 4: mod_base = gm
  modified_base 5: mod_base = um
  modified_base 6: mod_base = gm
  modified_base 7: mod_base = cm
  modified_base 8: mod_base = OTHER; note = 2'-O-methyl-adenosine
  modified_base 9: mod_base = OTHER; note = 2'-Fluoro-uridine
  modified_base 10: mod_base = OTHER; note = 2'-Fluoro-guanosine
  modified_base 11: mod_base = OTHER; note = 2'-Fluoro-guanosine
  modified_base 12: mod_base = um
  modified_base 13: mod_base = cm
  modified_base 14: mod_base = cm
  modified_base 15: mod_base = OTHER; note = 2'-O-methyl-adenosine
  modified_base 16: mod_base = OTHER; note = 2'-O-methyl-adenosine
  modified_base 17: mod_base = um
  modified_base 18: mod_base = gm
  modified_base 19: mod_base = um
  modified_base 20: mod_base = um
  modified_base 21: mod_base = cm
agggtgcatggtccaatgttc

SEQ ID NO: 1269 - RNA, 21 nt, synthetic construct
  source 1..21: mol_type = other RNA
  modified_base <1: mod_base = OTHER; note = two inverted abasic nucleosides
  modified_base 1: mod_base = OTHER; note = 2'-O-methyl-adenosine
  misc_feature 1^2: note = Phosphorothioate bond
  modified_base 2: mod_base = um
  misc_feature 2^3: note = Phosphorothioate bond
  modified_base 3: mod_base = cm
  modified_base 4: mod_base = um
  modified_base 5: mod_base = OTHER; note = 2'-O-methyl-adenosine
  modified_base 6: mod_base = cm
  modified_base 7: mod_base = OTHER; note = 2'-O-methyl-adenosine
  modified_base 8: mod_base = OTHER; note = 2'-O-methyl-adenosine
  modified_base 9: mod_base = OTHER; note = 2'-Fluoro-adenosine
  modified_base 10: mod_base = OTHER; note = 2'-Fluoro-uridine
  modified_base 11: mod_base = OTHER; note = 2'-Fluoro-cytidine
  modified_base 12: mod_base = um
  modified_base 13: mod_base = gm
  modified_base 14: mod_base = OTHER; note = 2'-O-methyl-adenosine
  modified_base 15: mod_base = um
  modified_base 16: mod_base = gm
  modified_base 17: mod_base = gm
  modified_base 18: mod_base = gm
  modified_base 19: mod_base = OTHER; note = 2'-O-methyl-adenosine
  modified_base 20: mod_base = um
  modified_base 21: mod_base = um
atctacaaatctgatgggatt

SEQ ID NO: 1270 - RNA, 21 nt, synthetic construct
  source 1..21: mol_type = other RNA
  modified_base <1: mod_base = OTHER; note = two inverted abasic nucleosides
  modified_base 1: mod_base = cm
  misc_feature 1^2: note = Phosphorothioate bond
  modified_base 2: mod_base = um
  misc_feature 2^3: note = Phosphorothioate bond
  modified_base 3: mod_base = um
  modified_base 4: mod_base = cm
  modified_base 5: mod_base = gm
  modified_base 6: mod_base = gm
  modified_base 7: mod_base = um
  modified_base 8: mod_base = OTHER; note = 2'-O-methyl-adenosine
  modified_base 9: mod_base = OTHER; note = 2'-Fluoro-uridine
  modified_base 10: mod_base = OTHER; note = 2'-Fluoro-cytidine
  modified_base 11: mod_base = OTHER; note = 2'-Fluoro-uridine
  modified_base 12: mod_base = OTHER; note = 2'-O-methyl-adenosine
  modified_base 13: mod_base = um
  modified_base 14: mod_base = gm
  modified_base 15: mod_base = OTHER; note = 2'-O-methyl-adenosine
  modified_base 16: mod_base = cm
  modified_base 17: mod_base = OTHER; note = 2'-O-methyl-adenosine
  modified_base 18: mod_base = cm
  modified_base 19: mod_base = um
  modified_base 20: mod_base = gm
  modified_base 21: mod_base = cm
cttcggtatctatgacactgc

SEQ ID NO: 1271 - RNA, 21 nt, synthetic construct
  source 1..21: mol_type = other RNA
  modified_base <1: mod_base = OTHER; note = two inverted abasic nucleosides
  modified_base 1: mod_base = um
  misc_feature 1^2: note = Phosphorothioate bond
  modified_base 2: mod_base = gm
  misc_feature 2^3: note = Phosphorothioate bond
  modified_base 3: mod_base = gm
  modified_base 4: mod_base = gm
  modified_base 5: mod_base = um
  modified_base 6: mod_base = gm
  modified_base 7: mod_base = gm
  modified_base 8: mod_base = um
  modified_base 9: mod_base = OTHER; note = 2'-Fluoro-guanosine
  modified_base 10: mod_base = OTHER; note = 2'-Fluoro-cytidine
  modified_base 11: mod_base = OTHER; note = 2'-Fluoro-uridine
  modified_base 12: mod_base = um
  modified_base 13: mod_base = um
  modified_base 14: mod_base = um
  modified_base 15: mod_base = gm
  modified_base 16: mod_base = um
  modified_base 17: mod_base = gm
  modified_base 18: mod_base = cm
  modified_base 19: mod_base = um
  modified_base 20: mod_base = um
  modified_base 21: mod_base = gm
tgggtggtgcttttgtgcttg

SEQ ID NO: 1272 - RNA, 21 nt, synthetic construct
  source 1..21: mol_type = other RNA
  modified_base <1: mod_base = OTHER; note = two inverted abasic nucleosides
  modified_base 1: mod_base = um
  misc_feature 1^2: note = Phosphorothioate bond
  modified_base 2: mod_base = OTHER; note = 2'-O-methyl-adenosine
  misc_feature 2^3: note = Phosphorothioate bond
  modified_base 3: mod_base = um
  modified_base 4: mod_base = um
  modified_base 5: mod_base = OTHER; note = 2'-O-methyl-adenosine
  modified_base 6: mod_base = um
  modified_base 7: mod_base = cm
  modified_base 8: mod_base = OTHER; note = 2'-O-methyl-adenosine
  modified_base 9: mod_base = OTHER; note = 2'-Fluoro-uridine
  modified_base 10: mod_base = OTHER; note = 2'-Fluoro-cytidine
  modified_base 11: mod_base = OTHER; note = 2'-Fluoro-uridine
  modified_base 12: mod_base = OTHER; note = 2'-O-methyl-adenosine
  modified_base 13: mod_base = cm
  modified_base 14: mod_base = cm
  modified_base 15: mod_base = gm
  modified_base 16: mod_base = OTHER; note = 2'-O-methyl-adenosine
  modified_base 17: mod_base = gm
  modified_base 18: mod_base = cm
  modified_base 19: mod_base = cm
  modified_base 20: mod_base = gm
  modified_base 21: mod_base = cm
tattatcatctaccgagccgc

SEQ ID NO: 1273 - RNA, 21 nt, synthetic construct
  source 1..21: mol_type = other RNA
  modified_base <1: mod_base = OTHER; note = two inverted abasic nucleosides
  modified_base 1: mod_base = gm
  misc_feature 1^2: note = Phosphorothioate bond
  modified_base 2: mod_base = um
  misc_feature 2^3: note = Phosphorothioate bond
  modified_base 3: mod_base = gm
  modified_base 4: mod_base = gm
  modified_base 5: mod_base = um
  modified_base 6: mod_base = cm
  modified_base 7: mod_base = cm
  modified_base 8: mod_base = gm
  modified_base 9: mod_base = OTHER; note = 2'-Fluoro-uridine
  modified_base 10: mod_base = OTHER; note = 2'-Fluoro-adenosine
  modified_base 11: mod_base = OTHER; note = 2'-Fluoro-uridine
  modified_base 12: mod_base = um
  modified_base 13: mod_base = cm
  modified_base 14: mod_base = cm
  modified_base 15: mod_base = cm
  modified_base 16: mod_base = OTHER; note = 2'-O-methyl-adenosine
  modified_base 17: mod_base = OTHER; note = 2'-O-methyl-adenosine
  modified_base 18: mod_base = gm
  modified_base 19: mod_base = gm
  modified_base 20: mod_base = OTHER; note = 2'-O-methyl-adenosine
  modified_base 21: mod_base = gm
gtggtccgtattcccaaggag

SEQ ID NO: 1274 - RNA, 21 nt, synthetic construct
  source 1..21: mol_type = other RNA
  modified_base <1: mod_base = OTHER; note = two inverted abasic nucleosides
  modified_base 1: mod_base = cm
  misc_feature 1^2: note = Phosphorothioate bond
  modified_base 2: mod_base = um
  misc_feature 2^3: note = Phosphorothioate bond
  modified_base 3: mod_base = OTHER; note = 2'-O-methyl-adenosine
  modified_base 4: mod_base = um
  modified_base 5: mod_base = gm
  modified_base 6: mod_base = OTHER; note = 2'-O-methyl-adenosine
  modified_base 7: mod_base = cm
  modified_base 8: mod_base = OTHER; note = 2'-O-methyl-adenosine
  modified_base 9: mod_base = OTHER; note = 2'-Fluoro-cytidine
  modified_base 10: mod_base = OTHER; note = 2'-Fluoro-uridine
  modified_base 11: mod_base = OTHER; note = 2'-Fluoro-guanosine
  modified_base 12: mod_base = cm
  modified_base 13: mod_base = OTHER; note = 2'-O-methyl-adenosine
  modified_base 14: mod_base = OTHER; note = 2'-O-methyl-adenosine
  modified_base 15: mod_base = OTHER; note = 2'-O-methyl-adenosine
  modified_base 16: mod_base = gm
  modified_base 17: mod_base = gm
  modified_base 18: mod_base = gm
  modified_base 19: mod_base = OTHER; note = 2'-O-methyl-adenosine
  modified_base 20: mod_base = OTHER; note = 2'-O-methyl-adenosine
  modified_base 21: mod_base = um
ctatgacactgcaaagggaat

SEQ ID NO: 1275 - RNA, 21 nt, synthetic construct
  source 1..21: mol_type = other RNA
  modified_base <1: mod_base = OTHER; note = two inverted abasic nucleosides
  modified_base 1: mod_base = cm
  misc_feature 1^2: note = Phosphorothioate bond
  modified_base 2: mod_base = um
  misc_feature 2^3: note = Phosphorothioate bond
  modified_base 3: mod_base = um
  modified_base 4: mod_base = um
  modified_base 5: mod_base = um
  modified_base 6: mod_base = gm
  modified_base 7: mod_base = um
  modified_base 8: mod_base = gm
  modified_base 9: mod_base = OTHER; note = 2'-Fluoro-cytidine
  modified_base 10: mod_base = OTHER; note = 2'-Fluoro-uridine
  modified_base 11: mod_base = OTHER; note = 2'-Fluoro-uridine
  modified_base 12: mod_base = gm
  modified_base 13: mod_base = um
  modified_base 14: mod_base = cm
  modified_base 15: mod_base = um
  modified_base 16: mod_base = um
  modified_base 17: mod_base = gm
  modified_base 18: mod_base = um
  modified_base 19: mod_base = OTHER; note = 2'-O-methyl-adenosine
  modified_base 20: mod_base = um
  modified_base 21: mod_base = gm
cttttgtgcttgtcttgtatg

SEQ ID NO: 1276 - RNA, 21 nt, synthetic construct
  source 1..21: mol_type = other RNA
  modified_base <1: mod_base = OTHER; note = two inverted abasic nucleosides
  modified_base 1: mod_base = um
  misc_feature 1^2: note = Phosphorothioate bond
  modified_base 2: mod_base = OTHER; note = 2'-O-methyl-adenosine
  misc_feature 2^3: note = Phosphorothioate bond
  modified_base 3: mod_base = cm
  modified_base 4: mod_base = cm
  modified_base 5: mod_base = OTHER; note = 2'-O-methyl-adenosine
  modified_base 6: mod_base = OTHER; note = 2'-O-methyl-adenosine
  modified_base 7: mod_base = gm
  modified_base 8: mod_base = gm
  modified_base 9: mod_base = OTHER; note = 2'-Fluoro-cytidine
  modified_base 10: mod_base = OTHER; note = 2'-Fluoro-uridine
  modified_base 11: mod_base = OTHER; note = 2'-Fluoro-uridine
  modified_base 12: mod_base = um
  modified_base 13: mod_base = OTHER; note = 2'-O-methyl-adenosine
  modified_base 14: mod_base = OTHER; note = 2'-O-methyl-adenosine
  modified_base 15: mod_base = cm
  modified_base 16: mod_base = gm
  modified_base 17: mod_base = um
  modified_base 18: mod_base = gm
  modified_base 19: mod_base = um
  modified_base 20: mod_base = cm
  modified_base 21: mod_base = um
taccaaggctttaacgtgtct

SEQ ID NO: 1277 - RNA, 21 nt, synthetic construct
  source 1..21: mol_type = other RNA
  modified_base <1: mod_base = OTHER; note = two inverted abasic nucleosides
  modified_base 1: mod_base = gm
  misc_feature 1^2: note = Phosphorothioate bond
  modified_base 2: mod_base = um
  misc_feature 2^3: note = Phosphorothioate bond
  modified_base 3: mod_base = gm
  modified_base 4: mod_base = cm
  modified_base 5: mod_base = OTHER; note = 2'-O-methyl-adenosine
  modified_base 6: mod_base = um
  modified_base 7: mod_base = gm
  modified_base 8: mod_base = gm
  modified_base 9: mod_base = OTHER; note = 2'-Fluoro-uridine
  modified_base 10: mod_base = OTHER; note = 2'-Fluoro-cytidine
  modified_base 11: mod_base = OTHER; note = 2'-Fluoro-cytidine
  modified_base 12: mod_base = OTHER; note = 2'-O-methyl-adenosine
  modified_base 13: mod_base = OTHER; note = 2'-O-methyl-adenosine
  modified_base 14: mod_base = um
  modified_base 15: mod_base = gm
  modified_base 16: mod_base = um
  modified_base 17: mod_base = um
  modified_base 18: mod_base = cm
  modified_base 19: mod_base = um
  modified_base 20: mod_base = cm
  modified_base 21: mod_base = OTHER; note = 2'-O-methyl-adenosine
gtgcatggtccaatgttctca

SEQ ID NO: 1278 - RNA, 21 nt, synthetic construct
  source 1..21: mol_type = other RNA
  modified_base <1: mod_base = OTHER; note = two inverted abasic nucleosides
  modified_base 1: mod_base = cm
  misc_feature 1^2: note = Phosphorothioate bond
  modified_base 2: mod_base = cm
  misc_feature 2^3: note = Phosphorothioate bond
  modified_base 3: mod_base = um
  modified_base 4: mod_base = um
  modified_base 5: mod_base = cm
  modified_base 6: mod_base = OTHER; note = 2'-O-methyl-adenosine
  modified_base 7: mod_base = OTHER; note = 2'-O-methyl-adenosine
  modified_base 8: mod_base = OTHER; note = 2'-O-methyl-adenosine
  modified_base 9: mod_base = OTHER; note = 2'-Fluoro-guanosine
  modified_base 10: mod_base = OTHER; note = 2'-Fluoro-adenosine
  modified_base 11: mod_base = OTHER; note = 2'-Fluoro-uridine
  modified_base 12: mod_base = OTHER; note = 2'-O-methyl-adenosine
  modified_base 13: mod_base = OTHER; note = 2'-O-methyl-adenosine
  modified_base 14: mod_base = OTHER; note = 2'-O-methyl-adenosine
  modified_base 15: mod_base = um
  modified_base 16: mod_base = OTHER; note = 2'-O-methyl-adenosine
  modified_base 17: mod_base = cm
  modified_base 18: mod_base = OTHER; note = 2'-O-methyl-adenosine
  modified_base 19: mod_base = OTHER; note = 2'-O-methyl-adenosine
  modified_base 20: mod_base = gm
  modified_base 21: mod_base = cm
ccttcaaagataaatacaagc

SEQ ID NO: 1279 - RNA, 21 nt, synthetic construct
  source 1..21: mol_type = other RNA
  modified_base <1: mod_base = OTHER; note = two inverted abasic nucleosides
  modified_base 1: mod_base = gm
  misc_feature 1^2: note = Phosphorothioate bond
  modified_base 2: mod_base = gm
  misc_feature 2^3: note = Phosphorothioate bond
  modified_base 3: mod_base = gm
  modified_base 4: mod_base = um
  modified_base 5: mod_base = OTHER; note = 2'-O-methyl-adenosine
  modified_base 6: mod_base = um
  modified_base 7: mod_base = um
  modified_base 8: mod_base = OTHER; note = 2'-O-methyl-adenosine
  modified_base 9: mod_base = OTHER; note = 2'-Fluoro-uridine
  modified_base 10: mod_base = OTHER; note = 2'-Fluoro-cytidine
  modified_base 11: mod_base = OTHER; note = 2'-Fluoro-adenosine
  modified_base 12: mod_base = um
  modified_base 13: mod_base = cm
  modified_base 14: mod_base = um
  modified_base 15: mod_base = OTHER; note = 2'-O-methyl-adenosine
  modified_base 16: mod_base = cm
  modified_base 17: mod_base = cm
  modified_base 18: mod_base = gm
  modified_base 19: mod_base = OTHER; note = 2'-O-methyl-adenosine
  modified_base 20: mod_base = gm
  modified_base 21: mod_base = cm
gggtattatcatctaccgagc

SEQ ID NO: 1280 - RNA, 21 nt, synthetic construct
  source 1..21: mol_type = other RNA
  modified_base <1: mod_base = OTHER; note = two inverted abasic nucleosides
  modified_base 1: mod_base = um
  misc_feature 1^2: note = Phosphorothioate bond
  modified_base 2: mod_base = OTHER; note = 2'-O-methyl-adenosine
  misc_feature 2^3: note = Phosphorothioate bond
  modified_base 3: mod_base = cm
  modified_base 4: mod_base = um
  modified_base 5: mod_base = um
  modified_base 6: mod_base = cm
  modified_base 7: mod_base = gm
  modified_base 8: mod_base = gm
  modified_base 9: mod_base = OTHER; note = 2'-Fluoro-uridine
  modified_base 10: mod_base = OTHER; note = 2'-Fluoro-adenosine
  modified_base 11: mod_base = OTHER; note = 2'-Fluoro-uridine
  modified_base 12: mod_base = cm
  modified_base 13: mod_base = um
  modified_base 14: mod_base = OTHER; note = 2'-O-methyl-adenosine
  modified_base 15: mod_base = um
  modified_base 16: mod_base = gm
  modified_base 17: mod_base = OTHER; note = 2'-O-methyl-adenosine
  modified_base 18: mod_base = cm
  modified_base 19: mod_base = OTHER; note = 2'-O-methyl-adenosine
  modified_base 20: mod_base = cm
  modified_base 21: mod_base = um
tacttcggtatctatgacact

SEQ ID NO: 1281 - RNA, 21 nt, synthetic construct
  source 1..21: mol_type = other RNA
  modified_base <1: mod_base = OTHER; note = two inverted abasic nucleosides
  modified_base 1: mod_base = gm
  misc_feature 1^2: note = Phosphorothioate bond
  modified_base 2: mod_base = um
  misc_feature 2^3: note = Phosphorothioate bond
  modified_base 3: mod_base = um
  modified_base 4: mod_base = OTHER; note = 2'-O-methyl-adenosine
  modified_base 5: mod_base = OTHER; note = 2'-O-methyl-adenosine
  modified_base 6: mod_base = gm
  modified_base 7: mod_base = OTHER; note = 2'-O-methyl-adenosine
  modified_base 8: mod_base = um
  modified_base 9: mod_base = OTHER; note = 2'-Fluoro-cytidine
  modified_base 10: mod_base = OTHER; note = 2'-Fluoro-uridine
  modified_base 11: mod_base = OTHER; note = 2'-Fluoro-adenosine
  modified_base 12: mod_base = cm
  modified_base 13: mod_base = OTHER; note = 2'-O-methyl-adenosine
  modified_base 14: mod_base = OTHER; note = 2'-O-methyl-adenosine
  modified_base 15: mod_base = OTHER; note = 2'-O-methyl-adenosine
  modified_base 16: mod_base = um
  modified_base 17: mod_base = cm
  modified_base 18: mod_base = um
  modified_base 19: mod_base = gm
  modified_base 20: mod_base = OTHER; note = 2'-O-methyl-adenosine
  modified_base 21: mod_base = um
gttaagatctacaaatctgat

SEQ ID NO: 1282 - RNA, 21 nt, synthetic construct
  source 1..21: mol_type = other RNA
  modified_base <1: mod_base = OTHER; note = two inverted abasic nucleosides
  modified_base 1: mod_base = um
  misc_feature 1^2: note = Phosphorothioate bond
  modified_base 2: mod_base = gm
  misc_feature 2^3: note = Phosphorothioate bond
  modified_base 3: mod_base = cm
  modified_base 4: mod_base = OTHER; note = 2'-O-methyl-adenosine
  modified_base 5: mod_base = gm
  modified_base 6: mod_base = gm
  modified_base 7: mod_base = gm
  modified_base 8: mod_base = um
  modified_base 9: mod_base = OTHER; note = 2'-Fluoro-adenosine
  modified_base 10: mod_base = OTHER; note = 2'-Fluoro-uridine
  modified_base 11: mod_base = OTHER; note = 2'-Fluoro-uridine
  modified_base 12: mod_base = OTHER; note = 2'-O-methyl-adenosine
  modified_base 13: mod_base = um
  modified_base 14: mod_base = cm
  modified_base 15: mod_base = OTHER; note = 2'-O-methyl-adenosine
  modified_base 16: mod_base = um
  modified_base 17: mod_base = cm
  modified_base 18: mod_base = um
  modified_base 19: mod_base = OTHER; note = 2'-O-methyl-adenosine
  modified_base 20: mod_base = cm
  modified_base 21: mod_base = cm
tgcagggtattatcatctacc

SEQ ID NO: 1283 - RNA, 21 nt, synthetic construct
  source 1..21: mol_type = other RNA
  modified_base <1: mod_base = OTHER; note = two inverted abasic nucleosides
  modified_base 1: mod_base = um
  misc_feature 1^2: note = Phosphorothioate bond
  modified_base 2: mod_base = cm
  misc_feature 2^3: note = Phosphorothioate bond
  modified_base 3: mod_base = um
  modified_base 4: mod_base = gm
  modified_base 5: mod_base = OTHER; note = 2'-O-methyl-adenosine
  modified_base 6: mod_base = um
  modified_base 7: mod_base = gm
  modified_base 8: mod_base = gm
  modified_base 9: mod_base = OTHER; note = 2'-Fluoro-guanosine
  modified_base 10: mod_base = OTHER; note = 2'-Fluoro-adenosine
  modified_base 11: mod_base = OTHER; note = 2'-Fluoro-uridine
  modified_base 12: mod_base = um
  modified_base 13: mod_base = OTHER; note = 2'-O-methyl-adenosine
  modified_base 14: mod_base = OTHER; note = 2'-O-methyl-adenosine
  modified_base 15: mod_base = gm
  modified_base 16: mod_base = gm
  modified_base 17: mod_base = gm
  modified_base 18: mod_base = cm
  modified_base 19: mod_base = cm
  modified_base 20: mod_base = um
  modified_base 21: mod_base = gm
tctgatgggattaagggcctg

SEQ ID NO: 1284 - RNA, 21 nt, synthetic construct
  source 1..21: mol_type = other RNA
  modified_base <1: mod_base = OTHER; note = two inverted abasic nucleosides
  modified_base 1: mod_base = cm
  misc_feature 1^2: note = Phosphorothioate bond
  modified_base 2: mod_base = um
  misc_feature 2^3: note = Phosphorothioate bond
  modified_base 3: mod_base = gm
  modified_base 4: mod_base = um
  modified_base 5: mod_base = gm
  modified_base 6: mod_base = cm
  modified_base 7: mod_base = OTHER; note = 2'-O-methyl-adenosine
  modified_base 8: mod_base = gm
  modified_base 9: mod_base = OTHER; note = 2'-Fluoro-guanosine
  modified_base 10: mod_base = OTHER; note = 2'-Fluoro-guanosine
  modified_base 11: mod_base = OTHER; note = 2'-Fluoro-uridine
  modified_base 12: mod_base = OTHER; note = 2'-O-methyl-adenosine
  modified_base 13: mod_base = um
  modified_base 14: mod_base = um
  modified_base 15: mod_base = OTHER; note = 2'-O-methyl-adenosine
  modified_base 16: mod_base = um
  modified_base 17: mod_base = cm
  modified_base 18: mod_base = OTHER; note = 2'-O-methyl-adenosine
  modified_base 19: mod_base = um
  modified_base 20: mod_base = cm
  modified_base 21: mod_base = um
ctgtgcagggtattatcatct

SEQ ID NO: 1285 - RNA, 21 nt, synthetic construct
  source 1..21: mol_type = other RNA
  modified_base <1: mod_base = OTHER; note = two inverted abasic nucleosides
  modified_base 1: mod_base = um
  misc_feature 1^2: note = Phosphorothioate bond
  modified_base 2: mod_base = gm
  misc_feature 2^3: note = Phosphorothioate bond
  modified_base 3: mod_base = OTHER; note = 2'-O-methyl-adenosine
  modified_base 4: mod_base = um
  modified_base 5: mod_base = gm
  modified_base 6: mod_base = gm
  modified_base 7: mod_base = gm
  modified_base 8: mod_base = OTHER; note = 2'-O-methyl-adenosine
  modified_base 9: mod_base = OTHER; note = 2'-Fluoro-uridine
  modified_base 10: mod_base = OTHER; note = 2'-Fluoro-uridine
  modified_base 11: mod_base = OTHER; note = 2'-Fluoro-adenosine
  modified_base 12: mod_base = OTHER; note = 2'-O-methyl-adenosine
  modified_base 13: mod_base = gm
  modified_base 14: mod_base = gm
  modified_base 15: mod_base = gm
  modified_base 16: mod_base = cm
  modified_base 17: mod_base = cm
  modified_base 18: mod_base = um
  modified_base 19: mod_base = gm
  modified_base 20: mod_base = um
  modified_base 21: mod_base = OTHER; note = 2'-O-methyl-adenosine
tgatgggattaagggcctgta

SEQ ID NO: 1286 - RNA, 21 nt, synthetic construct
  source 1..21: mol_type = other RNA
  modified_base <1: mod_base = OTHER; note = two inverted abasic nucleosides
  modified_base 1: mod_base = cm
  misc_feature 1^2: note = Phosphorothioate bond
  modified_base 2: mod_base = cm
  misc_feature 2^3: note = Phosphorothioate bond
  modified_base 3: mod_base = OTHER; note = 2'-O-methyl-adenosine
  modified_base 4: mod_base = OTHER; note = 2'-O-methyl-adenosine
  modified_base 5: mod_base = gm
  modified_base 6: mod_base = gm
  modified_base 7: mod_base = cm
  modified_base 8: mod_base = um
  modified_base 9: mod_base = OTHER; note = 2'-Fluoro-uridine
  modified_base 10: mod_base = OTHER; note = 2'-Fluoro-uridine
  modified_base 11: mod_base = OTHER; note = 2'-Fluoro-adenosine
  modified_base 12: mod_base = OTHER; note = 2'-O-methyl-adenosine
  modified_base 13: mod_base = cm
  modified_base 14: mod_base = gm
  modified_base 15: mod_base = um
  modified_base 16: mod_base = gm
  modified_base 17: mod_base = um
  modified_base 18: mod_base = cm
  modified_base 19: mod_base = um
  modified_base 20: mod_base = gm
  modified_base 21: mod_base = um
ccaaggctttaacgtgtctgt

SEQ ID NO: 1287 - RNA, 21 nt, synthetic construct
  source 1..21: mol_type = other RNA
  modified_base <1: mod_base = OTHER; note = two inverted abasic nucleosides
  modified_base 1: mod_base = um
  misc_feature 1^2: note = Phosphorothioate bond
  modified_base 2: mod_base = OTHER; note = 2'-O-methyl-adenosine
  misc_feature 2^3: note = Phosphorothioate bond
  modified_base 3: mod_base = um
  modified_base 4: mod_base = um
  modified_base 5: mod_base = cm
  modified_base 6: mod_base = OTHER; note = 2'-O-methyl-adenosine
  modified_base 7: mod_base = um
  modified_base 8: mod_base = cm
  modified_base 9: mod_base = OTHER; note = 2'-Fluoro-uridine
  modified_base 10: mod_base = OTHER; note = 2'-Fluoro-guanosine
  modified_base 11: mod_base = OTHER; note = 2'-Fluoro-adenosine
  modified_base 12: mod_base = cm
  modified_base 13: mod_base = cm
  modified_base 14: mod_base = OTHER; note = 2'-O-methyl-adenosine
  modified_base 15: mod_base = gm
  modified_base 16: mod_base = um
  modified_base 17: mod_base = um
  modified_base 18: mod_base = um
  modified_base 19: mod_base = um
  modified_base 20: mod_base = cm
  modified_base 21: mod_base = um
tattcatctgaccagttttct

SEQ ID NO: 1288 - RNA, 21 nt, synthetic construct
  source 1..21: mol_type = other RNA
  modified_base <1: mod_base = OTHER; note = two inverted abasic nucleosides
  modified_base 1: mod_base = OTHER; note = 2'-O-methyl-adenosine
  misc_feature 1^2: note = Phosphorothioate bond
  modified_base 2: mod_base = cm
  misc_feature 2^3: note = Phosphorothioate bond
  modified_base 3: mod_base = um
  modified_base 4: mod_base = gm
  modified_base 5: mod_base = cm
  modified_base 6: mod_base = cm
  modified_base 7: mod_base = um
  modified_base 8: mod_base = gm
  modified_base 9: mod_base = OTHER; note = 2'-Fluoro-guanosine
  modified_base 10: mod_base = OTHER; note = 2'-Fluoro-uridine
  modified_base 11: mod_base = OTHER; note = 2'-Fluoro-uridine
  modified_base 12: mod_base = OTHER; note = 2'-O-methyl-adenosine
  modified_base 13: mod_base = OTHER; note = 2'-O-methyl-adenosine
  modified_base 14: mod_base = gm
  modified_base 15: mod_base = OTHER; note = 2'-O-methyl-adenosine
  modified_base 16: mod_base = um
  modified_base 17: mod_base = cm
  modified_base 18: mod_base = um
  modified_base 19: mod_base = OTHER; note = 2'-O-methyl-adenosine
  modified_base 20: mod_base = cm
  modified_base 21: mod_base = OTHER; note = 2'-O-methyl-adenosine
actgcctggttaagatctaca

SEQ ID NO: 1289 - RNA, 21 nt, synthetic construct
  source 1..21: mol_type = other RNA
  modified_base <1: mod_base = OTHER; note = two inverted abasic nucleosides
  modified_base 1: mod_base = gm
  misc_feature 1^2: note = Phosphorothioate bond
  modified_base 2: mod_base = um
  misc_feature 2^3: note = Phosphorothioate bond
  modified_base 3: mod_base = um
  modified_base 4: mod_base = gm
  modified_base 5: mod_base = OTHER; note = 2'-O-methyl-adenosine
  modified_base 6: mod_base = cm
  modified_base 7: mod_base = um
  modified_base 8: mod_base = um
  modified_base 9: mod_base = OTHER; note = 2'-Fluoro-cytidine
  modified_base 10: mod_base = OTHER; note = 2'-Fluoro-cytidine
  modified_base 11: mod_base = OTHER; note = 2'-Fluoro-uridine
  modified_base 12: mod_base = OTHER; note = 2'-O-methyl-adenosine
  modified_base 13: mod_base = um
  modified_base 14: mod_base = cm
  modified_base 15: mod_base = cm
  modified_base 16: mod_base = OTHER; note = 2'-O-methyl-adenosine
  modified_base 17: mod_base = um
  modified_base 18: mod_base = um
  modified_base 19: mod_base = um
  modified_base 20: mod_base = gm
  modified_base 21: mod_base = OTHER; note = 2'-O-methyl-adenosine
gttgacttcctatccatttga

SEQ ID NO: 1290 - RNA, 21 nt, synthetic construct
  source 1..21: mol_type = other RNA
  modified_base <1: mod_base = OTHER; note = two inverted abasic nucleosides
  modified_base 1: mod_base = um
  misc_feature 1^2: note = Phosphorothioate bond
  modified_base 2: mod_base = OTHER; note = 2'-O-methyl-adenosine
  misc_feature 2^3: note = Phosphorothioate bond
  modified_base 3: mod_base = um
  modified_base 4: mod_base = gm
  modified_base 5: mod_base = OTHER; note = 2'-O-methyl-adenosine
  modified_base 6: mod_base = cm
  modified_base 7: mod_base = OTHER; note = 2'-O-methyl-adenosine
  modified_base 8: mod_base = cm
  modified_base 9: mod_base = OTHER; note = 2'-Fluoro-uridine
  modified_base 10: mod_base = OTHER; note = 2'-Fluoro-guanosine
  modified_base 11: mod_base = OTHER; note = 2'-Fluoro-cytidine
  modified_base 12: mod_base = OTHER; note = 2'-O-methyl-adenosine
  modified_base 13: mod_base = OTHER; note = 2'-O-methyl-adenosine
  modified_base 14: mod_base = OTHER; note = 2'-O-methyl-adenosine
  modified_base 15: mod_base = gm
  modified_base 16: mod_base = gm
  modified_base 17: mod_base = gm
  modified_base 18: mod_base = OTHER; note = 2'-O-methyl-adenosine
  modified_base 19: mod_base = OTHER; note = 2'-O-methyl-adenosine
  modified_base 20: mod_base = um
  modified_base 21: mod_base = gm
tatgacactgcaaagggaatg

SEQ ID NO: 1291 - RNA, 21 nt, synthetic construct
  source 1..21: mol_type = other RNA
  modified_base <1: mod_base = OTHER; note = two inverted abasic nucleosides
  modified_base 1: mod_base = um
  misc_feature 1^2: note = Phosphorothioate bond
  modified_base 2: mod_base = um
  misc_feature 2^3: note = Phosphorothioate bond
  modified_base 3: mod_base = OTHER; note = 2'-O-methyl-adenosine
  modified_base 4: mod_base = OTHER; note = 2'-O-methyl-adenosine
  modified_base 5: mod_base = gm
  modified_base 6: mod_base = OTHER; note = 2'-O-methyl-adenosine
  modified_base 7: mod_base = um
  modified_base 8: mod_base = cm
  modified_base 9: mod_base = OTHER; note = 2'-Fluoro-uridine
  modified_base 10: mod_base = OTHER; note = 2'-Fluoro-adenosine
  modified_base 11: mod_base = OTHER; note = 2'-Fluoro-cytidine
  modified_base 12: mod_base = OTHER; note = 2'-O-methyl-adenosine
  modified_base 13: mod_base = OTHER; note = 2'-O-methyl-adenosine
  modified_base 14: mod_base = OTHER; note = 2'-O-methyl-adenosine
  modified_base 15: mod_base = um
  modified_base 16: mod_base = cm
  modified_base 17: mod_base = um
  modified_base 18: mod_base = gm
  modified_base 19: mod_base = OTHER; note = 2'-O-methyl-adenosine
  modified_base 20: mod_base = um
  modified_base 21: mod_base = gm
ttaagatctacaaatctgatg

SEQ ID NO: 1292 - RNA, 21 nt, synthetic construct
  source 1..21: mol_type = other RNA
  modified_base <1: mod_base = OTHER; note = two inverted abasic nucleosides
  modified_base 1: mod_base = OTHER; note = 2'-O-methyl-adenosine
  misc_feature 1^2: note = Phosphorothioate bond
  modified_base 2: mod_base = gm
  misc_feature 2^3: note = Phosphorothioate bond
  modified_base 3: mod_base = gm
  modified_base 4: mod_base = gm
  modified_base 5: mod_base = um
  modified_base 6: mod_base = OTHER; note = 2'-O-methyl-adenosine
  modified_base 7: mod_base = um
  modified_base 8: mod_base = um
  modified_base 9: mod_base = OTHER; note = 2'-Fluoro-adenosine
  modified_base 10: mod_base = OTHER; note = 2'-Fluoro-uridine
  modified_base 11: mod_base = OTHER; note = 2'-Fluoro-cytidine
  modified_base 12: mod_base = OTHER; note = 2'-O-methyl-adenosine
  modified_base 13: mod_base = um
  modified_base 14: mod_base = cm
  modified_base 15: mod_base = um
  modified_base 16: mod_base = OTHER; note = 2'-O-methyl-adenosine
  modified_base 17: mod_base = cm
  modified_base 18: mod_base = cm
  modified_base 19: mod_base = gm
  modified_base 20: mod_base = OTHER; note = 2'-O-methyl-adenosine
  modified_base 21: mod_base = gm
agggtattatcatctaccgag

SEQ ID NO: 1293 - RNA, 21 nt, synthetic construct
  source 1..21: mol_type = other RNA
  modified_base <1: mod_base = OTHER; note = two inverted abasic nucleosides
  modified_base 1: mod_base = um
  misc_feature 1^2: note = Phosphorothioate bond
  modified_base 2: mod_base = gm
  misc_feature 2^3: note = Phosphorothioate bond
  modified_base 3: mod_base = cm
  modified_base 4: mod_base = cm
  modified_base 5: mod_base = um
  modified_base 6: mod_base = gm
  modified_base 7: mod_base = gm
  modified_base 8: mod_base = um
  modified_base 9: mod_base = OTHER; note = 2'-Fluoro-uridine
  modified_base 10: mod_base = OTHER; note = 2'-Fluoro-adenosine
  modified_base 11: mod_base = OTHER; note = 2'-Fluoro-adenosine
  modified_base 12: mod_base = gm
  modified_base 13: mod_base = OTHER; note = 2'-O-methyl-adenosine
  modified_base 14: mod_base = um
  modified_base 15: mod_base = cm
  modified_base 16: mod_base = um
  modified_base 17: mod_base = OTHER; note = 2'-O-methyl-adenosine
  modified_base 18: mod_base = cm
  modified_base 19: mod_base = OTHER; note = 2'-O-methyl-adenosine
  modified_base 20: mod_base = OTHER; note = 2'-O-methyl-adenosine
  modified_base 21: mod_base = OTHER; note = 2'-O-methyl-adenosine
tgcctggttaagatctacaaa

SEQ ID NO: 1294 - RNA, 21 nt, synthetic construct
  source 1..21: mol_type = other RNA
  modified_base <1: mod_base = OTHER; note = two inverted abasic nucleosides
  modified_base 1: mod_base = cm
  misc_feature 1^2: note = Phosphorothioate bond
  modified_base 2: mod_base = um
  misc_feature 2^3: note = Phosphorothioate bond
  modified_base 3: mod_base = gm
  modified_base 4: mod_base = OTHER; note = 2'-O-methyl-adenosine
  modified_base 5: mod_base = um
  modified_base 6: mod_base = gm
  modified_base 7: mod_base = gm
  modified_base 8: mod_base = gm
  modified_base 9: mod_base = OTHER; note = 2'-Fluoro-adenosine
  modified_base 10: mod_base = OTHER; note = 2'-Fluoro-uridine
  modified_base 11: mod_base = OTHER; note = 2'-Fluoro-uridine
  modified_base 12: mod_base = OTHER; note = 2'-O-methyl-adenosine
  modified_base 13: mod_base = OTHER; note = 2'-O-methyl-adenosine
  modified_base 14: mod_base = gm
  modified_base 15: mod_base = gm
  modified_base 16: mod_base = gm
  modified_base 17: mod_base = cm
  modified_base 18: mod_base = cm
  modified_base 19: mod_base = um
  modified_base 20: mod_base = gm
  modified_base 21: mod_base = um
ctgatgggattaagggcctgt

SEQ ID NO: 1295 - RNA, 21 nt, synthetic construct
  source 1..21: mol_type = other RNA
  modified_base <1: mod_base = OTHER; note = two inverted abasic nucleosides
  modified_base 1: mod_base = gm
  misc_feature 1^2: note = Phosphorothioate bond
  modified_base 2: mod_base = gm
  misc_feature 2^3: note = Phosphorothioate bond
  modified_base 3: mod_base = um
  modified_base 4: mod_base = OTHER; note = 2'-O-methyl-adenosine
  modified_base 5: mod_base = um
  modified_base 6: mod_base = cm
  modified_base 7: mod_base = um
  modified_base 8: mod_base = OTHER; note = 2'-O-methyl-adenosine
  modified_base 9: mod_base = OTHER; note = 2'-Fluoro-uridine
  modified_base 10: mod_base = OTHER; note = 2'-Fluoro-guanosine
  modified_base 11: mod_base = OTHER; note = 2'-Fluoro-adenosine
  modified_base 12: mod_base = cm
  modified_base 13: mod_base = OTHER; note = 2'-O-methyl-adenosine
  modified_base 14: mod_base = cm
  modified_base 15: mod_base = um
  modified_base 16: mod_base = gm
  modified_base 17: mod_base = cm
  modified_base 18: mod_base = OTHER; note = 2'-O-methyl-adenosine
  modified_base 19: mod_base = OTHER; note = 2'-O-methyl-adenosine
  modified_base 20: mod_base = OTHER; note = 2'-O-methyl-adenosine
  modified_base 21: mod_base = gm
ggtatctatgacactgcaaag

SEQ ID NO: 1296 - RNA, 21 nt, synthetic construct
  source 1..21: mol_type = other RNA
  modified_base <1: mod_base = OTHER; note = two inverted abasic nucleosides
  modified_base 1: mod_base = OTHER; note = 2'-O-methyl-adenosine
  misc_feature 1^2: note = Phosphorothioate bond
  modified_base 2: mod_base = cm
  misc_feature 2^3: note = Phosphorothioate bond
  modified_base 3: mod_base = cm
  modified_base 4: mod_base = cm
  modified_base 5: mod_base = gm
  modified_base 6: mod_base = um
  modified_base 7: mod_base = cm
  modified_base 8: mod_base = um
  modified_base 9: mod_base = OTHER; note = 2'-Fluoro-adenosine
  modified_base 10: mod_base = OTHER; note = 2'-Fluoro-guanosine
  modified_base 11: mod_base = OTHER; note = 2'-Fluoro-cytidine
  modified_base 12: mod_base = OTHER; note = 2'-O-methyl-adenosine
  modified_base 13: mod_base = gm
  modified_base 14: mod_base = cm
  modified_base 15: mod_base = um
  modified_base 16: mod_base = gm
  modified_base 17: mod_base = OTHER; note = 2'-O-methyl-adenosine
  modified_base 18: mod_base = um
  modified_base 19: mod_base = gm
  modified_base 20: mod_base = um
  modified_base 21: mod_base = gm
acccgtctagcagctgatgtg

SEQ ID NO: 1297 - RNA, 21 nt, synthetic construct
  source 1..21: mol_type = other RNA
  modified_base <1: mod_base = OTHER; note = two inverted abasic nucleosides
  modified_base 1: mod_base = um
  misc_feature 1^2: note = Phosphorothioate bond
  modified_base 2: mod_base = OTHER; note = 2'-O-methyl-adenosine
  misc_feature 2^3: note = Phosphorothioate bond
  modified_base 3: mod_base = um
  modified_base 4: mod_base = cm
  modified_base 5: mod_base = um
  modified_base 6: mod_base = OTHER; note = 2'-O-methyl-adenosine
  modified_base 7: mod_base = um
  modified_base 8: mod_base = gm
  modified_base 9: mod_base = OTHER; note = 2'-Fluoro-adenosine
  modified_base 10: mod_base = OTHER; note = 2'-Fluoro-cytidine
  modified_base 11: mod_base = OTHER; note = 2'-Fluoro-adenosine
  modified_base 12: mod_base = cm
  modified_base 13: mod_base = um
  modified_base 14: mod_base = gm
  modified_base 15: mod_base = cm
  modified_base 16: mod_base = OTHER; note = 2'-O-methyl-adenosine
  modified_base 17: mod_base = OTHER; note = 2'-O-methyl-adenosine
  modified_base 18: mod_base = OTHER; note = 2'-O-methyl-adenosine
  modified_base 19: mod_base = gm
  modified_base 20: mod_base = gm
  modified_base 21: mod_base = gm
tatctatgacactgcaaaggg

SEQ ID NO: 1298 - RNA, 21 nt, synthetic construct
  source 1..21: mol_type = other RNA
  modified_base <1: mod_base = OTHER; note = two inverted abasic nucleosides
  modified_base 1: mod_base = cm
  misc_feature 1^2: note = Phosphorothioate bond
  modified_base 2: mod_base = um
  misc_feature 2^3: note = Phosphorothioate bond
  modified_base 3: mod_base = gm
  modified_base 4: mod_base = OTHER; note = 2'-O-methyl-adenosine
  modified_base 5: mod_base = um
  modified_base 6: mod_base = gm
  modified_base 7: mod_base = um
  modified_base 8: mod_base = gm
  modified_base 9: mod_base = OTHER; note = 2'-Fluoro-guanosine
  modified_base 10: mod_base = OTHER; note = 2'-Fluoro-guanosine
  modified_base 11: mod_base = OTHER; note = 2'-Fluoro-uridine
  modified_base 12: mod_base = OTHER; note = 2'-O-methyl-adenosine
  modified_base 13: mod_base = OTHER; note = 2'-O-methyl-adenosine
  modified_base 14: mod_base = OTHER; note = 2'-O-methyl-adenosine
  modified_base 15: mod_base = gm
  modified_base 16: mod_base = cm
  modified_base 17: mod_base = um
  modified_base 18: mod_base = gm
  modified_base 19: mod_base = gm
  modified_base 20: mod_base = OTHER; note = 2'-O-methyl-adenosine
  modified_base 21: mod_base = gm
ctgatgtgggtaaagctggag

SEQ ID NO: 1299 - RNA, 21 nt, synthetic construct
  source 1..21: mol_type = other RNA
  modified_base <1: mod_base = OTHER; note = two inverted abasic nucleosides
  modified_base 1: mod_base = um
  misc_feature 1^2: note = Phosphorothioate bond
  modified_base 2: mod_base = cm
  misc_feature 2^3: note = Phosphorothioate bond
  modified_base 3: mod_base = um
  modified_base 4: mod_base = OTHER; note = 2'-O-methyl-adenosine
  modified_base 5: mod_base = gm
  modified_base 6: mod_base = cm
  modified_base 7: mod_base = OTHER; note = 2'-O-methyl-adenosine
  modified_base 8: mod_base = gm
  modified_base 9: mod_base = OTHER; note = 2'-Fluoro-cytidine
  modified_base 10: mod_base = OTHER; note = 2'-Fluoro-uridine
  modified_base 11: mod_base = OTHER; note = 2'-Fluoro-guanosine
  modified_base 12: mod_base = OTHER; note = 2'-O-methyl-adenosine
  modified_base 13: mod_base = um
  modified_base 14: mod_base = gm
  modified_base 15: mod_base = um
  modified_base 16: mod_base = gm
  modified_base 17: mod_base = gm
  modified_base 18: mod_base = gm
  modified_base 19: mod_base = um
  modified_base 20: mod_base = OTHER; note = 2'-O-methyl-adenosine
  modified_base 21: mod_base = OTHER; note = 2'-O-methyl-adenosine
tctagcagctgatgtgggtaa

SEQ ID NO: 1300 - RNA, 21 nt, synthetic construct
  source 1..21: mol_type = other RNA
  modified_base <1: mod_base = OTHER; note = two inverted abasic nucleosides
  modified_base 1: mod_base = gm
  misc_feature 1^2: note = Phosphorothioate bond
  modified_base 2: mod_base = gm
  misc_feature 2^3: note = Phosphorothioate bond
  modified_base 3: mod_base = gm
  modified_base 4: mod_base = cm
  modified_base 5: mod_base = cm
  modified_base 6: mod_base = um
  modified_base 7: mod_base = gm
  modified_base 8: mod_base = um
  modified_base 9: mod_base = OTHER; note = 2'-Fluoro-adenosine
  modified_base 10: mod_base = OTHER; note = 2'-Fluoro-cytidine
  modified_base 11: mod_base = OTHER; note = 2'-Fluoro-cytidine
  modified_base 12: mod_base = OTHER; note = 2'-O-methyl-adenosine
  modified_base 13: mod_base = OTHER; note = 2'-O-methyl-adenosine
  modified_base 14: mod_base = gm
  modified_base 15: mod_base = gm
  modified_base 16: mod_base = cm
  modified_base 17: mod_base = um
  modified_base 18: mod_base = um
  modified_base 19: mod_base = um
  modified_base 20: mod_base = OTHER; note = 2'-O-methyl-adenosine
  modified_base 21: mod_base = OTHER; note = 2'-O-methyl-adenosine
gggcctgtaccaaggctttaa

SEQ ID NO: 1301 - RNA, 21 nt, synthetic construct
  source 1..21: mol_type = other RNA
  modified_base <1: mod_base = OTHER; note = two inverted abasic nucleosides
  modified_base 1: mod_base = cm
  misc_feature 1^2: note = Phosphorothioate bond
  modified_base 2: mod_base = cm
  misc_feature 2^3: note = Phosphorothioate bond
  modified_base 3: mod_base = cm
  modified_base 4: mod_base = gm
  modified_base 5: mod_base = um
  modified_base 6: mod_base = OTHER; note = 2'-O-methyl-adenosine
  modified_base 7: mod_base = cm
  modified_base 8: mod_base = cm
  modified_base 9: mod_base = OTHER; note = 2'-Fluoro-cytidine
  modified_base 10: mod_base = OTHER; note = 2'-Fluoro-guanosine
  modified_base 11: mod_base = OTHER; note = 2'-Fluoro-uridine
  modified_base 12: mod_base = cm
  modified_base 13: mod_base = um
  modified_base 14: mod_base = OTHER; note = 2'-O-methyl-adenosine
  modified_base 15: mod_base = gm
  modified_base 16: mod_base = cm
  modified_base 17: mod_base = OTHER; note = 2'-O-methyl-adenosine
  modified_base 18: mod_base = gm
  modified_base 19: mod_base = cm
  modified_base 20: mod_base = um
  modified_base 21: mod_base = gm
cccgtacccgtctagcagctg

SEQ ID NO: 1302 - RNA, 21 nt, synthetic construct
  source 1..21: mol_type = other RNA
  modified_base <1: mod_base = OTHER; note = two inverted abasic nucleosides
  modified_base 1: mod_base = cm
  misc_feature 1^2: note = Phosphorothioate bond
  modified_base 2: mod_base = OTHER; note = 2'-O-methyl-adenosine
  misc_feature 2^3: note = Phosphorothioate bond
  modified_base 3: mod_base = gm
  modified_base 4: mod_base = cm
  modified_base 5: mod_base = um
  modified_base 6: mod_base = gm
  modified_base 7: mod_base = OTHER; note = 2'-O-methyl-adenosine
  modified_base 8: mod_base = um
  modified_base 9: mod_base = OTHER; note = 2'-Fluoro-guanosine
  modified_base 10: mod_base = OTHER; note = 2'-Fluoro-uridine
  modified_base 11: mod_base = OTHER; note = 2'-Fluoro-guanosine
  modified_base 12: mod_base = gm
  modified_base 13: mod_base = gm
  modified_base 14: mod_base = um
  modified_base 15: mod_base = OTHER; note = 2'-O-methyl-adenosine
  modified_base 16: mod_base = OTHER; note = 2'-O-methyl-adenosine
  modified_base 17: mod_base = OTHER; note = 2'-O-methyl-adenosine
  modified_base 18: mod_base = gm
  modified_base 19: mod_base = cm
  modified_base 20: mod_base = um
  modified_base 21: mod_base = gm
cagctgatgtgggtaaagctg

SEQ ID NO: 1303 - RNA, 21 nt, synthetic construct
  source 1..21: mol_type = other RNA
  modified_base <1: mod_base = OTHER; note = two inverted abasic nucleosides
  modified_base 1: mod_base = cm
  misc_feature 1^2: note = Phosphorothioate bond
  modified_base 2: mod_base = cm
  misc_feature 2^3: note = Phosphorothioate bond
  modified_base 3: mod_base = gm
  modified_base 4: mod_base = um
  modified_base 5: mod_base = OTHER; note = 2'-O-methyl-adenosine
  modified_base 6: mod_base = cm
  modified_base 7: mod_base = cm
  modified_base 8: mod_base = cm
  modified_base 9: mod_base = OTHER; note = 2'-Fluoro-guanosine
  modified_base 10: mod_base = OTHER; note = 2'-Fluoro-uridine
  modified_base 11: mod_base = OTHER; note = 2'-Fluoro-cytidine
  modified_base 12: mod_base = um
  modified_base 13: mod_base = OTHER; note = 2'-O-methyl-adenosine
  modified_base 14: mod_base = gm
  modified_base 15: mod_base = cm
  modified_base 16: mod_base = OTHER; note = 2'-O-methyl-adenosine
  modified_base 17: mod_base = gm
  modified_base 18: mod_base = cm
  modified_base 19: mod_base = um
  modified_base 20: mod_base = gm
  modified_base 21: mod_base = OTHER; note = 2'-O-methyl-adenosine
ccgtacccgtctagcagctga

SEQ ID NO: 1304 - RNA, 21 nt, synthetic construct
  source 1..21: mol_type = other RNA
  modified_base <1: mod_base = OTHER; note = two inverted abasic nucleosides
  modified_base 1: mod_base = gm
  misc_feature 1^2: note = Phosphorothioate bond
  modified_base 2: mod_base = cm
  misc_feature 2^3: note = Phosphorothioate bond
  modified_base 3: mod_base = um
  modified_base 4: mod_base = gm
  modified_base 5: mod_base = OTHER; note = 2'-O-methyl-adenosine
  modified_base 6: mod_base = um
  modified_base 7: mod_base = gm
  modified_base 8: mod_base = um
  modified_base 9: mod_base = OTHER; note = 2'-Fluoro-guanosine
  modified_base 10: mod_base = OTHER; note = 2'-Fluoro-guanosine
  modified_base 11: mod_base = OTHER; note = 2'-Fluoro-guanosine
  modified_base 12: mod_base = um
  modified_base 13: mod_base = OTHER; note = 2'-O-methyl-adenosine
  modified_base 14: mod_base = OTHER; note = 2'-O-methyl-adenosine
  modified_base 15: mod_base = OTHER; note = 2'-O-methyl-adenosine
  modified_base 16: mod_base = gm
  modified_base 17: mod_base = cm
  modified_base 18: mod_base = um
  modified_base 19: mod_base = gm
  modified_base 20: mod_base = gm
  modified_base 21: mod_base = OTHER; note = 2'-O-methyl-adenosine
gctgatgtgggtaaagctgga

SEQ ID NO: 1305 - RNA, 21 nt, synthetic construct
  source 1..21: mol_type = other RNA
  modified_base <1: mod_base = OTHER; note = two inverted abasic nucleosides
  modified_base 1: mod_base = gm
  misc_feature 1^2: note = Phosphorothioate bond
  modified_base 2: mod_base = gm
  misc_feature 2^3: note = Phosphorothioate bond
  modified_base 3: mod_base = um
  modified_base 4: mod_base = OTHER; note = 2'-O-methyl-adenosine
  modified_base 5: mod_base = um
  modified_base 6: mod_base = um
  modified_base 7: mod_base = OTHER; note = 2'-O-methyl-adenosine
  modified_base 8: mod_base = um
  modified_base 9: mod_base = OTHER; note = 2'-Fluoro-cytidine
  modified_base 10: mod_base = OTHER; note = 2'-Fluoro-adenosine
  modified_base 11: mod_base = OTHER; note = 2'-Fluoro-uridine
  modified_base 12: mod_base = cm
  modified_base 13: mod_base = um
  modified_base 14: mod_base = OTHER; note = 2'-O-methyl-adenosine
  modified_base 15: mod_base = cm
  modified_base 16: mod_base = cm
  modified_base 17: mod_base = gm
  modified_base 18: mod_base = OTHER; note = 2'-O-methyl-adenosine
  modified_base 19: mod_base = gm
  modified_base 20: mod_base = cm
  modified_base 21: mod_base = cm
ggtattatcatctaccgagcc

SEQ ID NO: 1306 - RNA, 21 nt, synthetic construct
  source 1..21: mol_type = other RNA
  modified_base <1: mod_base = OTHER; note = two inverted abasic nucleosides
  modified_base 1: mod_base = um
  misc_feature 1^2: note = Phosphorothioate bond
  modified_base 2: mod_base = um
  misc_feature 2^3: note = Phosphorothioate bond
  modified_base 3: mod_base = OTHER; note = 2'-O-methyl-adenosine
  modified_base 4: mod_base = um
  modified_base 5: mod_base = cm
  modified_base 6: mod_base = OTHER; note = 2'-O-methyl-adenosine
  modified_base 7: mod_base = um
  modified_base 8: mod_base = cm
  modified_base 9: mod_base = OTHER; note = 2'-Fluoro-uridine
  modified_base 10: mod_base = OTHER; note = 2'-Fluoro-adenosine
  modified_base 11: mod_base = OTHER; note = 2'-Fluoro-cytidine
  modified_base 12: mod_base = cm
  modified_base 13: mod_base = gm
  modified_base 14: mod_base = OTHER; note = 2'-O-methyl-adenosine
  modified_base 15: mod_base = gm
  modified_base 16: mod_base = cm
  modified_base 17: mod_base = cm
  modified_base 18: mod_base = gm
  modified_base 19: mod_base = cm
  modified_base 20: mod_base = cm
  modified_base 21: mod_base = um
ttatcatctaccgagccgcct

SEQ ID NO: 1307 - RNA, 21 nt, synthetic construct
  source 1..21: mol_type = other RNA
  modified_base <1: mod_base = OTHER; note = two inverted abasic nucleosides
  modified_base 1: mod_base = gm
  misc_feature 1^2: note = Phosphorothioate bond
  modified_base 2: mod_base = um
  misc_feature 2^3: note = Phosphorothioate bond
  modified_base 3: mod_base = OTHER; note = 2'-O-methyl-adenosine
  modified_base 4: mod_base = cm
  modified_base 5: mod_base = cm
  modified_base 6: mod_base = cm
  modified_base 7: mod_base = gm
  modified_base 8: mod_base = um
  modified_base 9: mod_base = OTHER; note = 2'-Fluoro-cytidine
  modified_base 10: mod_base = OTHER; note = 2'-Fluoro-uridine
  modified_base 11: mod_base = OTHER; note = 2'-Fluoro-adenosine
  modified_base 12: mod_base = gm
  modified_base 13: mod_base = cm
  modified_base 14: mod_base = OTHER; note = 2'-O-methyl-adenosine
  modified_base 15: mod_base = gm
  modified_base 16: mod_base = cm
  modified_base 17: mod_base = um
  modified_base 18: mod_base = gm
  modified_base 19: mod_base = OTHER; note = 2'-O-methyl-adenosine
  modified_base 20: mod_base = um
  modified_base 21: mod_base = gm
gtacccgtctagcagctgatg

SEQ ID NO: 1308 - RNA, 21 nt, synthetic construct
  source 1..21: mol_type = other RNA
  modified_base <1: mod_base = OTHER; note = two inverted abasic nucleosides
  modified_base 1: mod_base = gm
  misc_feature 1^2: note = Phosphorothioate bond
  modified_base 2: mod_base = OTHER; note = 2'-O-methyl-adenosine
  misc_feature 2^3: note = Phosphorothioate bond
  modified_base 3: mod_base = um
  modified_base 4: mod_base = gm
  modified_base 5: mod_base = gm
  modified_base 6: mod_base = gm
  modified_base 7: mod_base = OTHER; note = 2'-O-methyl-adenosine
  modified_base 8: mod_base = um
  modified_base 9: mod_base = OTHER; note = 2'-Fluoro-uridine
  modified_base 10: mod_base = OTHER; note = 2'-Fluoro-adenosine
  modified_base 11: mod_base = OTHER; note = 2'-Fluoro-adenosine
  modified_base 12: mod_base = gm
  modified_base 13: mod_base = gm
  modified_base 14: mod_base = gm
  modified_base 15: mod_base = cm
  modified_base 16: mod_base = cm
  modified_base 17: mod_base = um
  modified_base 18: mod_base = gm
  modified_base 19: mod_base = um
  modified_base 20: mod_base = OTHER; note = 2'-O-methyl-adenosine
  modified_base 21: mod_base = cm
gatgggattaagggcctgtac

SEQ ID NO: 1309 - RNA, 21 nt, synthetic construct
  source 1..21: mol_type = other RNA
  modified_base <1: mod_base = OTHER; note = two inverted abasic nucleosides
  modified_base 1: mod_base = gm
  misc_feature 1^2: note = Phosphorothioate bond
  modified_base 2: mod_base = um
  misc_feature 2^3: note = Phosphorothioate bond
  modified_base 3: mod_base = cm
  modified_base 4: mod_base = um
  modified_base 5: mod_base = gm
  modified_base 6: mod_base = um
  modified_base 7: mod_base = gm
  modified_base 8: mod_base = cm
  modified_base 9: mod_base = OTHER; note = 2'-Fluoro-adenosine
  modified_base 10: mod_base = OTHER; note = 2'-Fluoro-guanosine
  modified_base 11: mod_base = OTHER; note = 2'-Fluoro-guanosine
  modified_base 12: mod_base = gm
  modified_base 13: mod_base = um
  modified_base 14: mod_base = OTHER; note = 2'-O-methyl-adenosine
  modified_base 15: mod_base = um
  modified_base 16: mod_base = um
  modified_base 17: mod_base = OTHER; note = 2'-O-methyl-adenosine
  modified_base 18: mod_base = um
  modified_base 19: mod_base = cm
  modified_base 20: mod_base = OTHER; note = 2'-O-methyl-adenosine
  modified_base 21: mod_base = um
gtctgtgcagggtattatcat

SEQ ID NO: 1310 - RNA, 21 nt, synthetic construct
  source 1..21: mol_type = other RNA
  modified_base <1: mod_base = OTHER; note = two inverted abasic nucleosides
  modified_base 1: mod_base = gm
  misc_feature 1^2: note = Phosphorothioate bond
  modified_base 2: mod_base = cm
  misc_feature 2^3: note = Phosphorothioate bond
  modified_base 3: mod_base = gm
  modified_base 4: mod_base = um
  modified_base 5: mod_base = gm
  modified_base 6: mod_base = gm
  modified_base 7: mod_base = um
  modified_base 8: mod_base = cm
  modified_base 9: mod_base = OTHER; note = 2'-Fluoro-cytidine
  modified_base 10: mod_base = OTHER; note = 2'-Fluoro-guanosine
  modified_base 11: mod_base = OTHER; note = 2'-Fluoro-uridine
  modified_base 12: mod_base = OTHER; note = 2'-O-methyl-adenosine
  modified_base 13: mod_base = um
  modified_base 14: mod_base = um
  modified_base 15: mod_base = cm
  modified_base 16: mod_base = cm
  modified_base 17: mod_base = cm
  modified_base 18: mod_base = OTHER; note = 2'-O-methyl-adenosine
  modified_base 19: mod_base = OTHER; note = 2'-O-methyl-adenosine
  modified_base 20: mod_base = gm
  modified_base 21: mod_base = gm
gcgtggtccgtattcccaagg

SEQ ID NO: 1311 - RNA, 21 nt, synthetic construct
  source 1..21: mol_type = other RNA
  modified_base <1: mod_base = OTHER; note = two inverted abasic nucleosides
  modified_base 1: mod_base = cm
  misc_feature 1^2: note = Phosphorothioate bond
  modified_base 2: mod_base = gm
  misc_feature 2^3: note = Phosphorothioate bond
  modified_base 3: mod_base = um
  modified_base 4: mod_base = gm
  modified_base 5: mod_base = gm
  modified_base 6: mod_base = um
  modified_base 7: mod_base = cm
  modified_base 8: mod_base = cm
  modified_base 9: mod_base = OTHER; note = 2'-Fluoro-guanosine
  modified_base 10: mod_base = OTHER; note = 2'-Fluoro-uridine
  modified_base 11: mod_base = OTHER; note = 2'-Fluoro-adenosine
  modified_base 12: mod_base = um
  modified_base 13: mod_base = um
  modified_base 14: mod_base = cm
  modified_base 15: mod_base = cm
  modified_base 16: mod_base = cm
  modified_base 17: mod_base = OTHER; note = 2'-O-methyl-adenosine
  modified_base 18: mod_base = OTHER; note = 2'-O-methyl-adenosine
  modified_base 19: mod_base = gm
  modified_base 20: mod_base = gm
  modified_base 21: mod_base = OTHER; note = 2'-O-methyl-adenosine
cgtggtccgtattcccaagga

SEQ ID NO: 1312 - RNA, 21 nt, synthetic construct
  source 1..21: mol_type = other RNA
  modified_base <1: mod_base = OTHER; note = two inverted abasic nucleosides
  modified_base 1: mod_base = um
  misc_feature 1^2: note = Phosphorothioate bond
  modified_base 2: mod_base = gm
  misc_feature 2^3: note = Phosphorothioate bond
  modified_base 3: mod_base = gm
  modified_base 4: mod_base = um
  modified_base 5: mod_base = um
  modified_base 6: mod_base = OTHER; note = 2'-O-methyl-adenosine
  modified_base 7: mod_base = OTHER; note = 2'-O-methyl-adenosine
  modified_base 8: mod_base = gm
  modified_base 9: mod_base = OTHER; note = 2'-Fluoro-adenosine
  modified_base 10: mod_base = OTHER; note = 2'-Fluoro-uridine
  modified_base 11: mod_base = OTHER; note = 2'-Fluoro-cytidine
  modified_base 12: mod_base = um
  modified_base 13: mod_base = OTHER; note = 2'-O-methyl-adenosine
  modified_base 14: mod_base = cm
  modified_base 15: mod_base = OTHER; note = 2'-O-methyl-adenosine
  modified_base 16: mod_base = OTHER; note = 2'-O-methyl-adenosine
  modified_base 17: mod_base = OTHER; note = 2'-O-methyl-adenosine
  modified_base 18: mod_base = um
  modified_base 19: mod_base = cm
  modified_base 20: mod_base = um
  modified_base 21: mod_base = gm
tggttaagatctacaaatctg

SEQ ID NO: 1313 - RNA, 21 nt, synthetic construct
  source 1..21: mol_type = other RNA
  modified_base <1: mod_base = OTHER; note = two inverted abasic nucleosides
  modified_base 1: mod_base = OTHER; note = 2'-O-methyl-adenosine
  misc_feature 1^2: note = Phosphorothioate bond
  modified_base 2: mod_base = um
  misc_feature 2^3: note = Phosphorothioate bond
  modified_base 3: mod_base = gm
  modified_base 4: mod_base = OTHER; note = 2'-O-methyl-adenosine
  modified_base 5: mod_base = um
  modified_base 6: mod_base = gm
  modified_base 7: mod_base = OTHER; note = 2'-O-methyl-adenosine
  modified_base 8: mod_base = OTHER; note = 2'-O-methyl-adenosine
  modified_base 9: mod_base = OTHER; note = 2'-Fluoro-adenosine
  modified_base 10: mod_base = OTHER; note = 2'-Fluoro-uridine
  modified_base 11: mod_base = OTHER; note = 2'-Fluoro-cytidine
  modified_base 12: mod_base = OTHER; note = 2'-O-methyl-adenosine
  modified_base 13: mod_base = OTHER; note = 2'-O-methyl-adenosine
  modified_base 14: mod_base = gm
  modified_base 15: mod_base = OTHER; note = 2'-O-methyl-adenosine
  modified_base 16: mod_base = OTHER; note = 2'-O-methyl-adenosine
  modified_base 17: mod_base = gm
  modified_base 18: mod_base = um
  modified_base 19: mod_base = OTHER; note = 2'-O-methyl-adenosine
  modified_base 20: mod_base = cm
  modified_base 21: mod_base = OTHER; note = 2'-O-methyl-adenosine
atgatgaaatcaagaagtaca

SEQ ID NO: 1314 - RNA, 21 nt, synthetic construct
  source 1..21: mol_type = other RNA
  modified_base <1: mod_base = OTHER; note = two inverted abasic nucleosides
  modified_base 1: mod_base = gm
  misc_feature 1^2: note = Phosphorothioate bond
  modified_base 2: mod_base = OTHER; note = 2'-O-methyl-adenosine
  misc_feature 2^3: note = Phosphorothioate bond
  modified_base 3: mod_base = um
  modified_base 4: mod_base = cm
  modified_base 5: mod_base = um
  modified_base 6: mod_base = OTHER; note = 2'-O-methyl-adenosine
  modified_base 7: mod_base = cm
  modified_base 8: mod_base = OTHER; note = 2'-O-methyl-adenosine
  modified_base 9: mod_base = OTHER; note = 2'-Fluoro-adenosine
  modified_base 10: mod_base = OTHER; note = 2'-Fluoro-adenosine
  modified_base 11: mod_base = OTHER; note = 2'-Fluoro-uridine
  modified_base 12: mod_base = cm
  modified_base 13: mod_base = um
  modified_base 14: mod_base = gm
  modified_base 15: mod_base = OTHER; note = 2'-O-methyl-adenosine
  modified_base 16: mod_base = um
  modified_base 17: mod_base = gm
  modified_base 18: mod_base = gm
  modified_base 19: mod_base = gm
  modified_base 20: mod_base = OTHER; note = 2'-O-methyl-adenosine
  modified_base 21: mod_base = um
gatctacaaatctgatgggat

SEQ ID NO: 1315 - RNA, 21 nt, synthetic construct
  source 1..21: mol_type = other RNA
  modified_base <1: mod_base = OTHER; note = two inverted abasic nucleosides
  modified_base 1: mod_base = gm
  misc_feature 1^2: note = Phosphorothioate bond
  modified_base 2: mod_base = um
  misc_feature 2^3: note = Phosphorothioate bond
  modified_base 3: mod_base = gm
  modified_base 4: mod_base = cm
  modified_base 5: mod_base = OTHER; note = 2'-O-methyl-adenosine
  modified_base 6: mod_base = gm
  modified_base 7: mod_base = gm
  modified_base 8: mod_base = gm
  modified_base 9: mod_base = OTHER; note = 2'-Fluoro-uridine
  modified_base 10: mod_base = OTHER; note = 2'-Fluoro-adenosine
  modified_base 11: mod_base = OTHER; note = 2'-Fluoro-uridine
  modified_base 12: mod_base = um
  modified_base 13: mod_base = OTHER; note = 2'-O-methyl-adenosine
  modified_base 14: mod_base = um
  modified_base 15: mod_base = cm
  modified_base 16: mod_base = OTHER; note = 2'-O-methyl-adenosine
  modified_base 17: mod_base = um
  modified_base 18: mod_base = cm
  modified_base 19: mod_base = um
  modified_base 20: mod_base = OTHER; note = 2'-O-methyl-adenosine
  modified_base 21: mod_base = cm
gtgcagggtattatcatctac

SEQ ID NO: 1316 - RNA, 21 nt, synthetic construct
  source 1..21: mol_type = other RNA
  modified_base <1: mod_base = OTHER; note = two inverted abasic nucleosides
  modified_base 1: mod_base = gm
  misc_feature 1^2: note = Phosphorothioate bond
  modified_base 2: mod_base = um
  misc_feature 2^3: note = Phosphorothioate bond
  modified_base 3: mod_base = OTHER; note = 2'-O-methyl-adenosine
  modified_base 4: mod_base = cm
  modified_base 5: mod_base = cm
  modified_base 6: mod_base = OTHER; note = 2'-O-methyl-adenosine
  modified_base 7: mod_base = OTHER; note = 2'-O-methyl-adenosine
  modified_base 8: mod_base = gm
  modified_base 9: mod_base = OTHER; note = 2'-Fluoro-guanosine
  modified_base 10: mod_base = OTHER; note = 2'-Fluoro-cytidine
  modified_base 11: mod_base = OTHER; note = 2'-Fluoro-uridine
  modified_base 12: mod_base = um
  modified_base 13: mod_base = um
  modified_base 14: mod_base = OTHER; note = 2'-O-methyl-adenosine
  modified_base 15: mod_base = OTHER; note = 2'-O-methyl-adenosine
  modified_base 16: mod_base = cm
  modified_base 17: mod_base = gm
  modified_base 18: mod_base = um
  modified_base 19: mod_base = gm
  modified_base 20: mod_base = um
  modified_base 21: mod_base = cm
gtaccaaggctttaacgtgtc

SEQ ID NO: 1317 - RNA, 21 nt, synthetic construct
  source 1..21: mol_type = other RNA
  modified_base <1: mod_base = OTHER; note = two inverted abasic nucleosides
  modified_base 1: mod_base = gm
  misc_feature 1^2: note = Phosphorothioate bond
  modified_base 2: mod_base = cm
  misc_feature 2^3: note = Phosphorothioate bond
  modified_base 3: mod_base = OTHER; note = 2'-O-methyl-adenosine
  modified_base 4: mod_base = gm
  modified_base 5: mod_base = cm
  modified_base 6: mod_base = um
  modified_base 7: mod_base = gm
  modified_base 8: mod_base = OTHER; note = 2'-O-methyl-adenosine
  modified_base 9: mod_base = OTHER; note = 2'-Fluoro-uridine
  modified_base 10: mod_base = OTHER; note = 2'-Fluoro-guanosine
  modified_base 11: mod_base = OTHER; note = 2'-Fluoro-uridine
  modified_base 12: mod_base = gm
  modified_base 13: mod_base = gm
  modified_base 14: mod_base = gm
  modified_base 15: mod_base = um
  modified_base 16: mod_base = OTHER; note = 2'-O-methyl-adenosine
  modified_base 17: mod_base = OTHER; note = 2'-O-methyl-adenosine
  modified_base 18: mod_base = OTHER; note = 2'-O-methyl-adenosine
  modified_base 19: mod_base = gm
  modified_base 20: mod_base = cm
  modified_base 21: mod_base = um
gcagctgatgtgggtaaagct

SEQ ID NO: 1318 - RNA, 21 nt, synthetic construct
  source 1..21: mol_type = other RNA
  modified_base <1: mod_base = OTHER; note = two inverted abasic nucleosides
  modified_base 1: mod_base = OTHER; note = 2'-O-methyl-adenosine
  misc_feature 1^2: note = Phosphorothioate bond
  modified_base 2: mod_base = um
  misc_feature 2^3: note = Phosphorothioate bond
  modified_base 3: mod_base = gm
  modified_base 4: mod_base = gm
  modified_base 5: mod_base = gm
  modified_base 6: mod_base = um
  modified_base 7: mod_base = gm
  modified_base 8: mod_base = gm
  modified_base 9: mod_base = OTHER; note = 2'-Fluoro-uridine
  modified_base 10: mod_base = OTHER; note = 2'-Fluoro-guanosine
  modified_base 11: mod_base = OTHER; note = 2'-Fluoro-cytidine
  modified_base 12: mod_base = um
  modified_base 13: mod_base = um
  modified_base 14: mod_base = um
  modified_base 15: mod_base = um
  modified_base 16: mod_base = gm
  modified_base 17: mod_base = um
  modified_base 18: mod_base = gm
  modified_base 19: mod_base = cm
  modified_base 20: mod_base = um
  modified_base 21: mod_base = um
atgggtggtgcttttgtgctt

SEQ ID NO: 1319 - RNA, 21 nt, synthetic construct
  source 1..21: mol_type = other RNA
  modified_base <1: mod_base = OTHER; note = two inverted abasic nucleosides
  modified_base 1: mod_base = cm
  misc_feature 1^2: note = Phosphorothioate bond
  modified_base 2: mod_base = gm
  misc_feature 2^3: note = Phosphorothioate bond
  modified_base 3: mod_base = gm
  modified_base 4: mod_base = um
  modified_base 5: mod_base = gm
  modified_base 6: mod_base = OTHER; note = 2'-O-methyl-adenosine
  modified_base 7: mod_base = cm
  modified_base 8: mod_base = um
  modified_base 9: mod_base = OTHER; note = 2'-Fluoro-guanosine
  modified_base 10: mod_base = OTHER; note = 2'-Fluoro-cytidine
  modified_base 11: mod_base = OTHER; note = 2'-Fluoro-cytidine
  modified_base 12: mod_base = um
  modified_base 13: mod_base = gm
  modified_base 14: mod_base = gm
  modified_base 15: mod_base = um
  modified_base 16: mod_base = um
  modified_base 17: mod_base = OTHER; note = 2'-O-methyl-adenosine
  modified_base 18: mod_base = OTHER; note = 2'-O-methyl-adenosine
  modified_base 19: mod_base = gm
  modified_base 20: mod_base = OTHER; note = 2'-O-methyl-adenosine
  modified_base 21: mod_base = um
cggtgactgcctggttaagat

SEQ ID NO: 1320 - RNA, 21 nt, synthetic construct
  source 1..21: mol_type = other RNA
  modified_base <1: mod_base = OTHER; note = two inverted abasic nucleosides
  modified_base 1: mod_base = cm
  misc_feature 1^2: note = Phosphorothioate bond
  modified_base 2: mod_base = um
  misc_feature 2^3: note = Phosphorothioate bond
  modified_base 3: mod_base = OTHER; note = 2'-O-methyl-adenosine
  modified_base 4: mod_base = gm
  modified_base 5: mod_base = cm
  modified_base 6: mod_base = OTHER; note = 2'-O-methyl-adenosine
  modified_base 7: mod_base = gm
  modified_base 8: mod_base = cm
  modified_base 9: mod_base = OTHER; note = 2'-Fluoro-uridine
  modified_base 10: mod_base = OTHER; note = 2'-Fluoro-guanosine
  modified_base 11: mod_base = OTHER; note = 2'-Fluoro-adenosine
  modified_base 12: mod_base = um
  modified_base 13: mod_base = gm
  modified_base 14: mod_base = um
  modified_base 15: mod_base = gm
  modified_base 16: mod_base = gm
  modified_base 17: mod_base = gm
  modified_base 18: mod_base = um
  modified_base 19: mod_base = OTHER; note = 2'-O-methyl-adenosine
  modified_base 20: mod_base = OTHER; note = 2'-O-methyl-adenosine
  modified_base 21: mod_base = OTHER; note = 2'-O-methyl-adenosine
ctagcagctgatgtgggtaaa

SEQ ID NO: 1321 - RNA, 21 nt, synthetic construct
  source 1..21: mol_type = other RNA
  modified_base <1: mod_base = OTHER; note = two inverted abasic nucleosides
  modified_base 1: mod_base = um
  misc_feature 1^2: note = Phosphorothioate bond
  modified_base 2: mod_base = OTHER; note = 2'-O-methyl-adenosine
  misc_feature 2^3: note = Phosphorothioate bond
  modified_base 3: mod_base = cm
  modified_base 4: mod_base = OTHER; note = 2'-O-methyl-adenosine
  modified_base 5: mod_base = OTHER; note = 2'-O-methyl-adenosine
  modified_base 6: mod_base = OTHER; note = 2'-O-methyl-adenosine
  modified_base 7: mod_base = um
  modified_base 8: mod_base = cm
  modified_base 9: mod_base = OTHER; note = 2'-Fluoro-uridine
  modified_base 10: mod_base = OTHER; note = 2'-Fluoro-guanosine
  modified_base 11: mod_base = OTHER; note = 2'-Fluoro-adenosine
  modified_base 12: mod_base = um
  modified_base 13: mod_base = gm
  modified_base 14: mod_base = gm
  modified_base 15: mod_base = gm
  modified_base 16: mod_base = OTHER; note = 2'-O-methyl-adenosine
  modified_base 17: mod_base = um
  modified_base 18: mod_base = um
  modified_base 19: mod_base = OTHER; note = 2'-O-methyl-adenosine
  modified_base 20: mod_base = OTHER; note = 2'-O-methyl-adenosine
  modified_base 21: mod_base = gm
tacaaatctgatgggattaag

SEQ ID NO: 1322 - RNA, 21 nt, synthetic construct
  source 1..21: mol_type = other RNA
  modified_base <1: mod_base = OTHER; note = two inverted abasic nucleosides
  modified_base 1: mod_base = OTHER; note = 2'-O-methyl-adenosine
  misc_feature 1^2: note = Phosphorothioate bond
  modified_base 2: mod_base = cm
  misc_feature 2^3: note = Phosphorothioate bond
  modified_base 3: mod_base = um
  modified_base 4: mod_base = um
  modified_base 5: mod_base = cm
  modified_base 6: mod_base = gm
  modified_base 7: mod_base = gm
  modified_base 8: mod_base = um
  modified_base 9: mod_base = OTHER; note = 2'-Fluoro-adenosine
  modified_base 10: mod_base = OTHER; note = 2'-Fluoro-uridine
  modified_base 11: mod_base = OTHER; note = 2'-Fluoro-cytidine
  modified_base 12: mod_base = um
  modified_base 13: mod_base = OTHER; note = 2'-O-methyl-adenosine
  modified_base 14: mod_base = um
  modified_base 15: mod_base = gm
  modified_base 16: mod_base = OTHER; note = 2'-O-methyl-adenosine
  modified_base 17: mod_base = cm
  modified_base 18: mod_base = OTHER; note = 2'-O-methyl-adenosine
  modified_base 19: mod_base = cm
  modified_base 20: mod_base = um
  modified_base 21: mod_base = gm
acttcggtatctatgacactg

SEQ ID NO: 1323 - RNA, 21 nt, synthetic construct
  source 1..21: mol_type = other RNA
  modified_base <1: mod_base = OTHER; note = two inverted abasic nucleosides
  modified_base 1: mod_base = OTHER; note = 2'-O-methyl-adenosine
  misc_feature 1^2: note = Phosphorothioate bond
  modified_base 2: mod_base = gm
  misc_feature 2^3: note = Phosphorothioate bond
  modified_base 3: mod_base = cm
  modified_base 4: mod_base = um
  modified_base 5: mod_base = gm
  modified_base 6: mod_base = OTHER; note = 2'-O-methyl-adenosine
  modified_base 7: mod_base = um
  modified_base 8: mod_base = gm
  modified_base 9: mod_base = OTHER; note = 2'-Fluoro-uridine
  modified_base 10: mod_base = OTHER; note = 2'-Fluoro-guanosine
  modified_base 11: mod_base = OTHER; note = 2'-Fluoro-guanosine
  modified_base 12: mod_base = gm
  modified_base 13: mod_base = um
  modified_base 14: mod_base = OTHER; note = 2'-O-methyl-adenosine
  modified_base 15: mod_base = OTHER; note = 2'-O-methyl-adenosine
  modified_base 16: mod_base = OTHER; note = 2'-O-methyl-adenosine
  modified_base 17: mod_base = gm
  modified_base 18: mod_base = cm
  modified_base 19: mod_base = um
  modified_base 20: mod_base = gm
  modified_base 21: mod_base = gm
agctgatgtgggtaaagctgg

SEQ ID NO: 1324 - RNA, 21 nt, synthetic construct
  source 1..21: mol_type = other RNA
  modified_base <1: mod_base = OTHER; note = two inverted abasic nucleosides
  modified_base 1: mod_base = cm
  misc_feature 1^2: note = Phosphorothioate bond
  modified_base 2: mod_base = gm
  misc_feature 2^3: note = Phosphorothioate bond
  modified_base 3: mod_base = um
  modified_base 4: mod_base = OTHER; note = 2'-O-methyl-adenosine
  modified_base 5: mod_base = cm
  modified_base 6: mod_base = cm
  modified_base 7: mod_base = cm
  modified_base 8: mod_base = gm
  modified_base 9: mod_base = OTHER; note = 2'-Fluoro-uridine
  modified_base 10: mod_base = OTHER; note = 2'-Fluoro-cytidine
  modified_base 11: mod_base = OTHER; note = 2'-Fluoro-uridine
  modified_base 12: mod_base = OTHER; note = 2'-O-methyl-adenosine
  modified_base 13: mod_base = gm
  modified_base 14: mod_base = cm
  modified_base 15: mod_base = OTHER; note = 2'-O-methyl-adenosine
  modified_base 16: mod_base = gm
  modified_base 17: mod_base = cm
  modified_base 18: mod_base = um
  modified_base 19: mod_base = gm
  modified_base 20: mod_base = OTHER; note = 2'-O-methyl-adenosine
  modified_base 21: mod_base = um
cgtacccgtctagcagctgat

SEQ ID NO: 1325 - RNA, 21 nt, synthetic construct
  source 1..21: mol_type = other RNA
  modified_base <1: mod_base = OTHER; note = two inverted abasic nucleosides
  modified_base 1: mod_base = um
  misc_feature 1^2: note = Phosphorothioate bond
  modified_base 2: mod_base = cm
  misc_feature 2^3: note = Phosphorothioate bond
  modified_base 3: mod_base = um
  modified_base 4: mod_base = gm
  modified_base 5: mod_base = um
  modified_base 6: mod_base = gm
  modified_base 7: mod_base = cm
  modified_base 8: mod_base = OTHER; note = 2'-O-methyl-adenosine
  modified_base 9: mod_base = OTHER; note = 2'-Fluoro-guanosine
  modified_base 10: mod_base = OTHER; note = 2'-Fluoro-guanosine
  modified_base 11: mod_base = OTHER; note = 2'-Fluoro-guanosine
  modified_base 12: mod_base = um
  modified_base 13: mod_base = OTHER; note = 2'-O-methyl-adenosine
  modified_base 14: mod_base = um
  modified_base 15: mod_base = um
  modified_base 16: mod_base = OTHER; note = 2'-O-methyl-adenosine
  modified_base 17: mod_base = um
  modified_base 18: mod_base = cm
  modified_base 19: mod_base = OTHER; note = 2'-O-methyl-adenosine
  modified_base 20: mod_base = um
  modified_base 21: mod_base = cm
tctgtgcagggtattatcatc

SEQ ID NO: 1326 - RNA, 21 nt, synthetic construct
  source 1..21: mol_type = other RNA
  modified_base <1: mod_base = OTHER; note = two inverted abasic nucleosides
  modified_base 1: mod_base = um
  misc_feature 1^2: note = Phosphorothioate bond
  modified_base 2: mod_base = gm
  misc_feature 2^3: note = Phosphorothioate bond
  modified_base 3: mod_base = cm
  modified_base 4: mod_base = um
  modified_base 5: mod_base = um
  modified_base 6: mod_base = gm
  modified_base 7: mod_base = um
  modified_base 8: mod_base = cm
  modified_base 9: mod_base = OTHER; note = 2'-Fluoro-uridine
  modified_base 10: mod_base = OTHER; note = 2'-Fluoro-uridine
  modified_base 11: mod_base = OTHER; note = 2'-Fluoro-guanosine
  modified_base 12: mod_base = um
  modified_base 13: mod_base = OTHER; note = 2'-O-methyl-adenosine
  modified_base 14: mod_base = um
  modified_base 15: mod_base = gm
  modified_base 16: mod_base = OTHER; note = 2'-O-methyl-adenosine
  modified_base 17: mod_base = um
  modified_base 18: mod_base = gm
  modified_base 19: mod_base = OTHER; note = 2'-O-methyl-adenosine
  modified_base 20: mod_base = OTHER; note = 2'-O-methyl-adenosine
  modified_base 21: mod_base = OTHER; note = 2'-O-methyl-adenosine
tgcttgtcttgtatgatgaaa

SEQ ID NO: 1327 - RNA, 21 nt, synthetic construct
  source 1..21: mol_type = other RNA
  modified_base <1: mod_base = OTHER; note = two inverted abasic nucleosides
  modified_base 1: mod_base = OTHER; note = 2'-O-methyl-adenosine
  misc_feature 1^2: note = Phosphorothioate bond
  modified_base 2: mod_base = cm
  misc_feature 2^3: note = Phosphorothioate bond
  modified_base 3: mod_base = cm
  modified_base 4: mod_base = OTHER; note = 2'-O-methyl-adenosine
  modified_base 5: mod_base = OTHER; note = 2'-O-methyl-adenosine
  modified_base 6: mod_base = gm
  modified_base 7: mod_base = gm
  modified_base 8: mod_base = cm
  modified_base 9: mod_base = OTHER; note = 2'-Fluoro-uridine
  modified_base 10: mod_base = OTHER; note = 2'-Fluoro-uridine
  modified_base 11: mod_base = OTHER; note = 2'-Fluoro-uridine
  modified_base 12: mod_base = OTHER; note = 2'-O-methyl-adenosine
  modified_base 13: mod_base = OTHER; note = 2'-O-methyl-adenosine
  modified_base 14: mod_base = cm
  modified_base 15: mod_base = gm
  modified_base 16: mod_base = um
  modified_base 17: mod_base = gm
  modified_base 18: mod_base = um
  modified_base 19: mod_base = cm
  modified_base 20: mod_base = um
  modified_base 21: mod_base = gm
accaaggctttaacgtgtctg

SEQ ID NO: 1328 - RNA, 21 nt, synthetic construct
  source 1..21: mol_type = other RNA
  modified_base <1: mod_base = OTHER; note = two inverted abasic nucleosides
  modified_base 1: mod_base = gm
  misc_feature 1^2: note = Phosphorothioate bond
  modified_base 2: mod_base = gm
  misc_feature 2^3: note = Phosphorothioate bond
  modified_base 3: mod_base = gm
  modified_base 4: mod_base = um
  modified_base 5: mod_base = gm
  modified_base 6: mod_base = cm
  modified_base 7: mod_base = OTHER; note = 2'-O-methyl-adenosine
  modified_base 8: mod_base = um
  modified_base 9: mod_base = OTHER; note = 2'-Fluoro-guanosine
  modified_base 10: mod_base = OTHER; note = 2'-Fluoro-guanosine
  modified_base 11: mod_base = OTHER; note = 2'-Fluoro-uridine
  modified_base 12: mod_base = cm
  modified_base 13: mod_base = cm
  modified_base 14: mod_base = OTHER; note = 2'-O-methyl-adenosine
  modified_base 15: mod_base = OTHER; note = 2'-O-methyl-adenosine
  modified_base 16: mod_base = um
  modified_base 17: mod_base = gm
  modified_base 18: mod_base = um
  modified_base 19: mod_base = um
  modified_base 20: mod_base = cm
  modified_base 21: mod_base = um
gggtgcatggtccaatgttct

SEQ ID NO: 1329 - RNA, 21 nt, synthetic construct
  source 1..21: mol_type = other RNA
  modified_base <1: mod_base = OTHER; note = two inverted abasic nucleosides
  modified_base 1: mod_base = gm
  misc_feature 1^2: note = Phosphorothioate bond
  modified_base 2: mod_base = OTHER; note = 2'-O-methyl-adenosine
  misc_feature 2^3: note = Phosphorothioate bond
  modified_base 3: mod_base = cm
  modified_base 4: mod_base = um
  modified_base 5: mod_base = gm
  modified_base 6: mod_base = cm
  modified_base 7: mod_base = cm
  modified_base 8: mod_base = um
  modified_base 9: mod_base = OTHER; note = 2'-Fluoro-guanosine
  modified_base 10: mod_base = OTHER; note = 2'-Fluoro-guanosine
  modified_base 11: mod_base = OTHER; note = 2'-Fluoro-uridine
  modified_base 12: mod_base = um
  modified_base 13: mod_base = OTHER; note = 2'-O-methyl-adenosine
  modified_base 14: mod_base = OTHER; note = 2'-O-methyl-adenosine
  modified_base 15: mod_base = gm
  modified_base 16: mod_base = OTHER; note = 2'-O-methyl-adenosine
  modified_base 17: mod_base = um
  modified_base 18: mod_base = cm
  modified_base 19: mod_base = um
  modified_base 20: mod_base = OTHER; note = 2'-O-methyl-adenosine
  modified_base 21: mod_base = cm
gactgcctggttaagatctac

SEQ ID NO: 1330 - RNA, 21 nt, synthetic construct
  source 1..21: mol_type = other RNA
  modified_base <1: mod_base = OTHER; note = two inverted abasic nucleosides
  modified_base 1: mod_base = gm
  misc_feature 1^2: note = Phosphorothioate bond
  modified_base 2: mod_base = OTHER; note = 2'-O-methyl-adenosine
  misc_feature 2^3: note = Phosphorothioate bond
  modified_base 3: mod_base = um
  modified_base 4: mod_base = gm
  modified_base 5: mod_base = um
  modified_base 6: mod_base = gm
  modified_base 7: mod_base = gm
  modified_base 8: mod_base = gm
  modified_base 9: mod_base = OTHER; note = 2'-Fluoro-uridine
  modified_base 10: mod_base = OTHER; note = 2'-Fluoro-adenosine
  modified_base 11: mod_base = OTHER; note = 2'-Fluoro-adenosine
  modified_base 12: mod_base = OTHER; note = 2'-O-methyl-adenosine
  modified_base 13: mod_base = gm
  modified_base 14: mod_base = cm
  modified_base 15: mod_base = um
  modified_base 16: mod_base = gm
  modified_base 17: mod_base = gm
  modified_base 18: mod_base = OTHER; note = 2'-O-methyl-adenosine
  modified_base 19: mod_base = gm
  modified_base 20: mod_base = cm
  modified_base 21: mod_base = um
gatgtgggtaaagctggagct

SEQ ID NO: 1331 - RNA, 21 nt, synthetic construct
  source 1..21: mol_type = other RNA
  modified_base <1: mod_base = OTHER; note = two inverted abasic nucleosides
  modified_base 1: mod_base = um
  misc_feature 1^2: note = Phosphorothioate bond
  modified_base 2: mod_base = gm
  misc_feature 2^3: note = Phosphorothioate bond
  modified_base 3: mod_base = gm
  modified_base 4: mod_base = um
  modified_base 5: mod_base = cm
  modified_base 6: mod_base = cm
  modified_base 7: mod_base = gm
  modified_base 8: mod_base = um
  modified_base 9: mod_base = OTHER; note = 2'-Fluoro-adenosine
  modified_base 10: mod_base = OTHER; note = 2'-Fluoro-uridine
  modified_base 11: mod_base = OTHER; note = 2'-Fluoro-uridine
  modified_base 12: mod_base = cm
  modified_base 13: mod_base = cm
  modified_base 14: mod_base = cm
  modified_base 15: mod_base = OTHER; note = 2'-O-methyl-adenosine
  modified_base 16: mod_base = OTHER; note = 2'-O-methyl-adenosine
  modified_base 17: mod_base = gm
  modified_base 18: mod_base = gm
  modified_base 19: mod_base = OTHER; note = 2'-O-methyl-adenosine
  modified_base 20: mod_base = gm
  modified_base 21: mod_base = cm
tggtccgtattcccaaggagc

SEQ ID NO: 1332 - RNA, 21 nt, synthetic construct
  source 1..21: mol_type = other RNA
  modified_base <1: mod_base = OTHER; note = two inverted abasic nucleosides
  modified_base 1: mod_base = OTHER; note = 2'-O-methyl-adenosine
  misc_feature 1^2: note = Phosphorothioate bond
  modified_base 2: mod_base = cm
  misc_feature 2^3: note = Phosphorothioate bond
  modified_base 3: mod_base = OTHER; note = 2'-O-methyl-adenosine
  modified_base 4: mod_base = cm
  modified_base 5: mod_base = um
  modified_base 6: mod_base = gm
  modified_base 7: mod_base = cm
  modified_base 8: mod_base = OTHER; note = 2'-O-methyl-adenosine
  modified_base 9: mod_base = OTHER; note = 2'-Fluoro-adenosine
  modified_base 10: mod_base = OTHER; note = 2'-Fluoro-adenosine
  modified_base 11: mod_base = OTHER; note = 2'-Fluoro-guanosine
  modified_base 12: mod_base = gm
  modified_base 13: mod_base = gm
  modified_base 14: mod_base = OTHER; note = 2'-O-methyl-adenosine
  modified_base 15: mod_base = OTHER; note = 2'-O-methyl-adenosine
  modified_base 16: mod_base = um
  modified_base 17: mod_base = gm
  modified_base 18: mod_base = cm
  modified_base 19: mod_base = um
  modified_base 20: mod_base = um
  modified_base 21: mod_base = cm
acactgcaaagggaatgcttc

SEQ ID NO: 1333 - RNA, 21 nt, synthetic construct
  source 1..21: mol_type = other RNA
  modified_base <1: mod_base = OTHER; note = two inverted abasic nucleosides
  modified_base 1: mod_base = gm
  misc_feature 1^2: note = Phosphorothioate bond
  modified_base 2: mod_base = OTHER; note = 2'-O-methyl-adenosine
  misc_feature 2^3: note = Phosphorothioate bond
  modified_base 3: mod_base = um
  modified_base 4: mod_base = um
  modified_base 5: mod_base = OTHER; note = 2'-O-methyl-adenosine
  modified_base 6: mod_base = OTHER; note = 2'-O-methyl-adenosine
  modified_base 7: mod_base = gm
  modified_base 8: mod_base = gm
  modified_base 9: mod_base = OTHER; note = 2'-Fluoro-guanosine
  modified_base 10: mod_base = OTHER; note = 2'-Fluoro-cytidine
  modified_base 11: mod_base = OTHER; note = 2'-Fluoro-cytidine
  modified_base 12: mod_base = um
  modified_base 13: mod_base = gm
  modified_base 14: mod_base = um
  modified_base 15: mod_base = OTHER; note = 2'-O-methyl-adenosine
  modified_base 16: mod_base = cm
  modified_base 17: mod_base = cm
  modified_base 18: mod_base = OTHER; note = 2'-O-methyl-adenosine
  modified_base 19: mod_base = OTHER; note = 2'-O-methyl-adenosine
  modified_base 20: mod_base = gm
  modified_base 21: mod_base = gm
gattaagggcctgtaccaagg

SEQ ID NO: 1334 - RNA, 21 nt, synthetic construct
  source 1..21: mol_type = other RNA
  modified_base <1: mod_base = OTHER; note = two inverted abasic nucleosides
  modified_base 1: mod_base = um
  misc_feature 1^2: note = Phosphorothioate bond
  modified_base 2: mod_base = gm
  misc_feature 2^3: note = Phosphorothioate bond
  modified_base 3: mod_base = um
  modified_base 4: mod_base = gm
  modified_base 5: mod_base = cm
  modified_base 6: mod_base = OTHER; note = 2'-O-methyl-adenosine
  modified_base 7: mod_base = gm
  modified_base 8: mod_base = gm
  modified_base 9: mod_base = OTHER; note = 2'-Fluoro-guanosine
  modified_base 10: mod_base = OTHER; note = 2'-Fluoro-uridine
  modified_base 11: mod_base = OTHER; note = 2'-Fluoro-adenosine
  modified_base 12: mod_base = um
  modified_base 13: mod_base = um
  modified_base 14: mod_base = OTHER; note = 2'-O-methyl-adenosine
  modified_base 15: mod_base = um
  modified_base 16: mod_base = cm
  modified_base 17: mod_base = OTHER; note = 2'-O-methyl-adenosine
  modified_base 18: mod_base = um
  modified_base 19: mod_base = cm
  modified_base 20: mod_base = um
  modified_base 21: mod_base = OTHER; note = 2'-O-methyl-adenosine
tgtgcagggtattatcatcta

SEQ ID NO: 1335 - RNA, 21 nt, synthetic construct
  source 1..21: mol_type = other RNA
  modified_base <1: mod_base = OTHER; note = two inverted abasic nucleosides
  modified_base 1: mod_base = OTHER; note = 2'-O-methyl-adenosine
  misc_feature 1^2: note = Phosphorothioate bond
  modified_base 2: mod_base = OTHER; note = 2'-O-methyl-adenosine
  misc_feature 2^3: note = Phosphorothioate bond
  modified_base 3: mod_base = cm
  modified_base 4: mod_base = gm
  modified_base 5: mod_base = um
  modified_base 6: mod_base = gm
  modified_base 7: mod_base = um
  modified_base 8: mod_base = cm
  modified_base 9: mod_base = OTHER; note = 2'-Fluoro-uridine
  modified_base 10: mod_base = OTHER; note = 2'-Fluoro-guanosine
  modified_base 11: mod_base = OTHER; note = 2'-Fluoro-uridine
  modified_base 12: mod_base = gm
  modified_base 13: mod_base = cm
  modified_base 14: mod_base = OTHER; note = 2'-O-methyl-adenosine
  modified_base 15: mod_base = gm
  modified_base 16: mod_base = gm
  modified_base 17: mod_base = gm
  modified_base 18: mod_base = um
  modified_base 19: mod_base = OTHER; note = 2'-O-methyl-adenosine
  modified_base 20: mod_base = um
  modified_base 21: mod_base = um
aacgtgtctgtgcagggtatt

SEQ ID NO: 1336 - RNA, 21 nt, synthetic construct
  source 1..21: mol_type = other RNA
  modified_base <1: mod_base = OTHER; note = two inverted abasic nucleosides
  modified_base 1: mod_base = gm
  misc_feature 1^2: note = Phosphorothioate bond
  modified_base 2: mod_base = gm
  misc_feature 2^3: note = Phosphorothioate bond
  modified_base 3: mod_base = cm
  modified_base 4: mod_base = cm
  modified_base 5: mod_base = um
  modified_base 6: mod_base = gm
  modified_base 7: mod_base = um
  modified_base 8: mod_base = OTHER; note = 2'-O-methyl-adenosine
  modified_base 9: mod_base = OTHER; note = 2'-Fluoro-cytidine
  modified_base 10: mod_base = OTHER; note = 2'-Fluoro-cytidine
  modified_base 11: mod_base = OTHER; note = 2'-Fluoro-adenosine
  modified_base 12: mod_base = OTHER; note = 2'-O-methyl-adenosine
  modified_base 13: mod_base = gm
  modified_base 14: mod_base = gm
  modified_base 15: mod_base = cm
  modified_base 16: mod_base = um
  modified_base 17: mod_base = um
  modified_base 18: mod_base = um
  modified_base 19: mod_base = OTHER; note = 2'-O-methyl-adenosine
  modified_base 20: mod_base = OTHER; note = 2'-O-methyl-adenosine
  modified_base 21: mod_base = cm
ggcctgtaccaaggctttaac

SEQ ID NO: 1337 - RNA, 21 nt, synthetic construct
  source 1..21: mol_type = other RNA
  modified_base <1: mod_base = OTHER; note = two inverted abasic nucleosides
  modified_base 1: mod_base = um
  misc_feature 1^2: note = Phosphorothioate bond
  modified_base 2: mod_base = gm
  misc_feature 2^3: note = Phosphorothioate bond
  modified_base 3: mod_base = OTHER; note = 2'-O-methyl-adenosine
  modified_base 4: mod_base = cm
  modified_base 5: mod_base = OTHER; note = 2'-O-methyl-adenosine
  modified_base 6: mod_base = cm
  modified_base 7: mod_base = um
  modified_base 8: mod_base = gm
  modified_base 9: mod_base = OTHER; note = 2'-Fluoro-cytidine
  modified_base 10: mod_base = OTHER; note = 2'-Fluoro-adenosine
  modified_base 11: mod_base = OTHER; note = 2'-Fluoro-adenosine
  modified_base 12: mod_base = OTHER; note = 2'-O-methyl-adenosine
  modified_base 13: mod_base = gm
  modified_base 14: mod_base = gm
  modified_base 15: mod_base = gm
  modified_base 16: mod_base = OTHER; note = 2'-O-methyl-adenosine
  modified_base 17: mod_base = OTHER; note = 2'-O-methyl-adenosine
  modified_base 18: mod_base = um
  modified_base 19: mod_base = gm
  modified_base 20: mod_base = cm
  modified_base 21: mod_base = um
tgacactgcaaagggaatgct

SEQ ID NO: 1338 - RNA, 21 nt, synthetic construct
  source 1..21: mol_type = other RNA
  modified_base <1: mod_base = OTHER; note = two inverted abasic nucleosides
  modified_base 1: mod_base = um
  misc_feature 1^2: note = Phosphorothioate bond
  modified_base 2: mod_base = cm
  misc_feature 2^3: note = Phosphorothioate bond
  modified_base 3: mod_base = gm
  modified_base 4: mod_base = gm
  modified_base 5: mod_base = um
  modified_base 6: mod_base = gm
  modified_base 7: mod_base = OTHER; note = 2'-O-methyl-adenosine
  modified_base 8: mod_base = cm
  modified_base 9: mod_base = OTHER; note = 2'-Fluoro-uridine
  modified_base 10: mod_base = OTHER; note = 2'-Fluoro-guanosine
  modified_base 11: mod_base = OTHER; note = 2'-Fluoro-cytidine
  modified_base 12: mod_base = cm
  modified_base 13: mod_base = um
  modified_base 14: mod_base = gm
  modified_base 15: mod_base = gm
  modified_base 16: mod_base = um
  modified_base 17: mod_base = um
  modified_base 18: mod_base = OTHER; note = 2'-O-methyl-adenosine
  modified_base 19: mod_base = OTHER; note = 2'-O-methyl-adenosine
  modified_base 20: mod_base = gm
  modified_base 21: mod_base = OTHER; note = 2'-O-methyl-adenosine
tcggtgactgcctggttaaga

SEQ ID NO: 1339 - RNA, 21 nt, synthetic construct
  source 1..21: mol_type = other RNA
  modified_base <1: mod_base = OTHER; note = two inverted abasic nucleosides
  modified_base 1: mod_base = gm
  misc_feature 1^2: note = Phosphorothioate bond
  modified_base 2: mod_base = cm
  misc_feature 2^3: note = Phosphorothioate bond
  modified_base 3: mod_base = um
  modified_base 4: mod_base = um
  modified_base 5: mod_base = um
  modified_base 6: mod_base = um
  modified_base 7: mod_base = gm
  modified_base 8: mod_base = um
  modified_base 9: mod_base = OTHER; note = 2'-Fluoro-guanosine
  modified_base 10: mod_base = OTHER; note = 2'-Fluoro-cytidine
  modified_base 11: mod_base = OTHER; note = 2'-Fluoro-uridine
  modified_base 12: mod_base = um
  modified_base 13: mod_base = gm
  modified_base 14: mod_base = um
  modified_base 15: mod_base = cm
  modified_base 16: mod_base = um
  modified_base 17: mod_base = um
  modified_base 18: mod_base = gm
  modified_base 19: mod_base = um
  modified_base 20: mod_base = OTHER; note = 2'-O-methyl-adenosine
  modified_base 21: mod_base = um
gcttttgtgcttgtcttgtat

SEQ ID NO: 1340 - RNA, 21 nt, synthetic construct
  source 1..21: mol_type = other RNA
  modified_base <1: mod_base = OTHER; note = two inverted abasic nucleosides
  modified_base 1: mod_base = gm
  misc_feature 1^2: note = Phosphorothioate bond
  modified_base 2: mod_base = gm
  misc_feature 2^3: note = Phosphorothioate bond
  modified_base 3: mod_base = um
  modified_base 4: mod_base = gm
  modified_base 5: mod_base = gm
  modified_base 6: mod_base = um
  modified_base 7: mod_base = gm
  modified_base 8: mod_base = cm
  modified_base 9: mod_base = OTHER; note = 2'-Fluoro-uridine
  modified_base 10: mod_base = OTHER; note = 2'-Fluoro-uridine
  modified_base 11: mod_base = OTHER; note = 2'-Fluoro-uridine
  modified_base 12: mod_base = um
  modified_base 13: mod_base = gm
  modified_base 14: mod_base = um
  modified_base 15: mod_base = gm
  modified_base 16: mod_base = cm
  modified_base 17: mod_base = um
  modified_base 18: mod_base = um
  modified_base 19: mod_base = gm
  modified_base 20: mod_base = um
  modified_base 21: mod_base = cm
ggtggtgcttttgtgcttgtc

SEQ ID NO: 1341 - RNA, 21 nt, synthetic construct
  source 1..21: mol_type = other RNA
  modified_base <1: mod_base = OTHER; note = two inverted abasic nucleosides
  modified_base 1: mod_base = cm
  misc_feature 1^2: note = Phosphorothioate bond
  modified_base 2: mod_base = gm
  misc_feature 2^3: note = Phosphorothioate bond
  modified_base 3: mod_base = um
  modified_base 4: mod_base = cm
  modified_base 5: mod_base = um
  modified_base 6: mod_base = OTHER; note = 2'-O-methyl-adenosine
  modified_base 7: mod_base = gm
  modified_base 8: mod_base = cm
  modified_base 9: mod_base = OTHER; note = 2'-Fluoro-adenosine
  modified_base 10: mod_base = OTHER; note = 2'-Fluoro-guanosine
  modified_base 11: mod_base = OTHER; note = 2'-Fluoro-cytidine
  modified_base 12: mod_base = um
  modified_base 13: mod_base = gm
  modified_base 14: mod_base = OTHER; note = 2'-O-methyl-adenosine
  modified_base 15: mod_base = um
  modified_base 16: mod_base = gm
  modified_base 17: mod_base = um
  modified_base 18: mod_base = gm
  modified_base 19: mod_base = gm
  modified_base 20: mod_base = gm
  modified_base 21: mod_base = um
cgtctagcagctgatgtgggt

SEQ ID NO: 1342 - RNA, 21 nt, synthetic construct
  source 1..21: mol_type = other RNA
  modified_base <1: mod_base = OTHER; note = two inverted abasic nucleosides
  modified_base 1: mod_base = OTHER; note = 2'-O-methyl-adenosine
  misc_feature 1^2: note = Phosphorothioate bond
  modified_base 2: mod_base = gm
  misc_feature 2^3: note = Phosphorothioate bond
  modified_base 3: mod_base = gm
  modified_base 4: mod_base = gm
  modified_base 5: mod_base = cm
  modified_base 6: mod_base = cm
  modified_base 7: mod_base = um
  modified_base 8: mod_base = gm
  modified_base 9: mod_base = OTHER; note = 2'-Fluoro-uridine
  modified_base 10: mod_base = OTHER; note = 2'-Fluoro-adenosine
  modified_base 11: mod_base = OTHER; note = 2'-Fluoro-cytidine
  modified_base 12: mod_base = cm
  modified_base 13: mod_base = OTHER; note = 2'-O-methyl-adenosine
  modified_base 14: mod_base = OTHER; note = 2'-O-methyl-adenosine
  modified_base 15: mod_base = gm
  modified_base 16: mod_base = gm
  modified_base 17: mod_base = cm
  modified_base 18: mod_base = um
  modified_base 19: mod_base = um
  modified_base 20: mod_base = um
  modified_base 21: mod_base = OTHER; note = 2'-O-methyl-adenosine
agggcctgtaccaaggcttta

SEQ ID NO: 1343 - RNA, 21 nt, synthetic construct
  source 1..21: mol_type = other RNA
  modified_base <1: mod_base = OTHER; note = two inverted abasic nucleosides
  modified_base 1: mod_base = gm
  misc_feature 1^2: note = Phosphorothioate bond
  modified_base 2: mod_base = um
  misc_feature 2^3: note = Phosphorothioate bond
  modified_base 3: mod_base = gm
  modified_base 4: mod_base = cm
  modified_base 5: mod_base = um
  modified_base 6: mod_base = um
  modified_base 7: mod_base = gm
  modified_base 8: mod_base = um
  modified_base 9: mod_base = OTHER; note = 2'-Fluoro-cytidine
  modified_base 10: mod_base = OTHER; note = 2'-Fluoro-uridine
  modified_base 11: mod_base = OTHER; note = 2'-Fluoro-uridine
  modified_base 12: mod_base = gm
  modified_base 13: mod_base = um
  modified_base 14: mod_base = OTHER; note = 2'-O-methyl-adenosine
  modified_base 15: mod_base = um
  modified_base 16: mod_base = gm
  modified_base 17: mod_base = OTHER; note = 2'-O-methyl-adenosine
  modified_base 18: mod_base = um
  modified_base 19: mod_base = gm
  modified_base 20: mod_base = OTHER; note = 2'-O-methyl-adenosine
  modified_base 21: mod_base = OTHER; note = 2'-O-methyl-adenosine
gtgcttgtcttgtatgatgaa

SEQ ID NO: 1344 - RNA, 21 nt, synthetic construct
  source 1..21: mol_type = other RNA
  modified_base <1: mod_base = OTHER; note = two inverted abasic nucleosides
  modified_base 1: mod_base = OTHER; note = 2'-O-methyl-adenosine
  misc_feature 1^2: note = Phosphorothioate bond
  modified_base 2: mod_base = OTHER; note = 2'-O-methyl-adenosine
  misc_feature 2^3: note = Phosphorothioate bond
  modified_base 3: mod_base = OTHER; note = 2'-O-methyl-adenosine
  modified_base 4: mod_base = um
  modified_base 5: mod_base = cm
  modified_base 6: mod_base = um
  modified_base 7: mod_base = gm
  modified_base 8: mod_base = OTHER; note = 2'-O-methyl-adenosine
  modified_base 9: mod_base = OTHER; note = 2'-Fluoro-uridine
  modified_base 10: mod_base = OTHER; note = 2'-Fluoro-guanosine
  modified_base 11: mod_base = OTHER; note = 2'-Fluoro-guanosine
  modified_base 12: mod_base = gm
  modified_base 13: mod_base = OTHER; note = 2'-O-methyl-adenosine
  modified_base 14: mod_base = um
  modified_base 15: mod_base = um
  modified_base 16: mod_base = OTHER; note = 2'-O-methyl-adenosine
  modified_base 17: mod_base = OTHER; note = 2'-O-methyl-adenosine
  modified_base 18: mod_base = gm
  modified_base 19: mod_base = gm
  modified_base 20: mod_base = gm
  modified_base 21: mod_base = cm
aaatctgatgggattaagggc

SEQ ID NO: 1345 - RNA, 21 nt, synthetic construct
  source 1..21: mol_type = other RNA
  modified_base <1: mod_base = OTHER; note = two inverted abasic nucleosides
  modified_base 1: mod_base = cm
  misc_feature 1^2: note = Phosphorothioate bond
  modified_base 2: mod_base = um
  misc_feature 2^3: note = Phosphorothioate bond
  modified_base 3: mod_base = OTHER; note = 2'-O-methyl-adenosine
  modified_base 4: mod_base = cm
  modified_base 5: mod_base = OTHER; note = 2'-O-methyl-adenosine
  modified_base 6: mod_base = OTHER; note = 2'-O-methyl-adenosine
  modified_base 7: mod_base = OTHER; note = 2'-O-methyl-adenosine
  modified_base 8: mod_base = um
  modified_base 9: mod_base = OTHER; note = 2'-Fluoro-cytidine
  modified_base 10: mod_base = OTHER; note = 2'-Fluoro-uridine
  modified_base 11: mod_base = OTHER; note = 2'-Fluoro-guanosine
  modified_base 12: mod_base = OTHER; note = 2'-O-methyl-adenosine
  modified_base 13: mod_base = um
  modified_base 14: mod_base = gm
  modified_base 15: mod_base = gm
  modified_base 16: mod_base = gm
  modified_base 17: mod_base = OTHER; note = 2'-O-methyl-adenosine
  modified_base 18: mod_base = um
  modified_base 19: mod_base = um
  modified_base 20: mod_base = OTHER; note = 2'-O-methyl-adenosine
  modified_base 21: mod_base = OTHER; note = 2'-O-methyl-adenosine
ctacaaatctgatgggattaa

SEQ ID NO: 1346 - RNA, 21 nt, synthetic construct
  source 1..21: mol_type = other RNA
  modified_base <1: mod_base = OTHER; note = two inverted abasic nucleosides
  modified_base 1: mod_base = cm
  misc_feature 1^2: note = Phosphorothioate bond
  modified_base 2: mod_base = OTHER; note = 2'-O-methyl-adenosine
  misc_feature 2^3: note = Phosphorothioate bond
  modified_base 3: mod_base = gm
  modified_base 4: mod_base = gm
  modified_base 5: mod_base = gm
  modified_base 6: mod_base = um
  modified_base 7: mod_base = OTHER; note = 2'-O-methyl-adenosine
  modified_base 8: mod_base = um
  modified_base 9: mod_base = OTHER; note = 2'-Fluoro-uridine
  modified_base 10: mod_base = OTHER; note = 2'-Fluoro-adenosine
  modified_base 11: mod_base = OTHER; note = 2'-Fluoro-uridine
  modified_base 12: mod_base = cm
  modified_base 13: mod_base = OTHER; note = 2'-O-methyl-adenosine
  modified_base 14: mod_base = um
  modified_base 15: mod_base = cm
  modified_base 16: mod_base = um
  modified_base 17: mod_base = OTHER; note = 2'-O-methyl-adenosine
  modified_base 18: mod_base = cm
  modified_base 19: mod_base = cm
  modified_base 20: mod_base = gm
  modified_base 21: mod_base = OTHER; note = 2'-O-methyl-adenosine
cagggtattatcatctaccga

SEQ ID NO: 1347 - RNA, 21 nt, synthetic construct
  source 1..21: mol_type = other RNA
  modified_base <1: mod_base = OTHER; note = two inverted abasic nucleosides
  modified_base 1: mod_base = cm
  misc_feature 1^2: note = Phosphorothioate bond
  modified_base 2: mod_base = um
  misc_feature 2^3: note = Phosphorothioate bond
  modified_base 3: mod_base = gm
  modified_base 4: mod_base = um
  modified_base 5: mod_base = OTHER; note = 2'-O-methyl-adenosine
  modified_base 6: mod_base = cm
  modified_base 7: mod_base = cm
  modified_base 8: mod_base = OTHER; note = 2'-O-methyl-adenosine
  modified_base 9: mod_base = OTHER; note = 2'-Fluoro-adenosine
  modified_base 10: mod_base = OTHER; note = 2'-Fluoro-guanosine
  modified_base 11: mod_base = OTHER; note = 2'-Fluoro-guanosine
  modified_base 12: mod_base = cm
  modified_base 13: mod_base = um
  modified_base 14: mod_base = um
  modified_base 15: mod_base = um
  modified_base 16: mod_base = OTHER; note = 2'-O-methyl-adenosine
  modified_base 17: mod_base = OTHER; note = 2'-O-methyl-adenosine
  modified_base 18: mod_base = cm
  modified_base 19: mod_base = gm
  modified_base 20: mod_base = um
  modified_base 21: mod_base = gm
ctgtaccaaggctttaacgtg

SEQ ID NO: 1348 - RNA, 21 nt, synthetic construct
  source 1..21: mol_type = other RNA
  modified_base <1: mod_base = OTHER; note = two inverted abasic nucleosides
  modified_base 1: mod_base = OTHER; note = 2'-O-methyl-adenosine
  misc_feature 1^2: note = Phosphorothioate bond
  modified_base 2: mod_base = gm
  misc_feature 2^3: note = Phosphorothioate bond
  modified_base 3: mod_base = OTHER; note = 2'-O-methyl-adenosine
  modified_base 4: mod_base = um
  modified_base 5: mod_base = cm
  modified_base 6: mod_base = um
  modified_base 7: mod_base = OTHER; note = 2'-O-methyl-adenosine
  modified_base 8: mod_base = cm
  modified_base 9: mod_base = OTHER; note = 2'-Fluoro-adenosine
  modified_base 10: mod_base = OTHER; note = 2'-Fluoro-adenosine
  modified_base 11: mod_base = OTHER; note = 2'-Fluoro-adenosine
  modified_base 12: mod_base = um
  modified_base 13: mod_base = cm
  modified_base 14: mod_base = um
  modified_base 15: mod_base = gm
  modified_base 16: mod_base = OTHER; note = 2'-O-methyl-adenosine
  modified_base 17: mod_base = um
  modified_base 18: mod_base = gm
  modified_base 19: mod_base = gm
  modified_base 20: mod_base = gm
  modified_base 21: mod_base = OTHER; note = 2'-O-methyl-adenosine
agatctacaaatctgatggga

SEQ ID NO: 1349 - RNA, 21 nt, synthetic construct
  source 1..21: mol_type = other RNA
  modified_base <1: mod_base = OTHER; note = two inverted abasic nucleosides
  modified_base 1: mod_base = um
  misc_feature 1^2: note = Phosphorothioate bond
  modified_base 2: mod_base = um
  misc_feature 2^3: note = Phosphorothioate bond
  modified_base 3: mod_base = um
  modified_base 4: mod_base = um
  modified_base 5: mod_base = gm
  modified_base 6: mod_base = um
  modified_base 7: mod_base = gm
  modified_base 8: mod_base = cm
  modified_base 9: mod_base = OTHER; note = 2'-Fluoro-uridine
  modified_base 10: mod_base = OTHER; note = 2'-Fluoro-uridine
  modified_base 11: mod_base = OTHER; note = 2'-Fluoro-guanosine
  modified_base 12: mod_base = um
  modified_base 13: mod_base = cm
  modified_base 14: mod_base = um
  modified_base 15: mod_base = um
  modified_base 16: mod_base = gm
  modified_base 17: mod_base = um
  modified_base 18: mod_base = OTHER; note = 2'-O-methyl-adenosine
  modified_base 19: mod_base = um
  modified_base 20: mod_base = gm
  modified_base 21: mod_base = OTHER; note = 2'-O-methyl-adenosine
ttttgtgcttgtcttgtatga

SEQ ID NO: 1350 - RNA, 21 nt, synthetic construct
  source 1..21: mol_type = other RNA
  modified_base <1: mod_base = OTHER; note = two inverted abasic nucleosides
  modified_base 1: mod_base = OTHER; note = 2'-O-methyl-adenosine
  misc_feature 1^2: note = Phosphorothioate bond
  modified_base 2: mod_base = cm
  misc_feature 2^3: note = Phosphorothioate bond
  modified_base 3: mod_base = OTHER; note = 2'-O-methyl-adenosine
  modified_base 4: mod_base = OTHER; note = 2'-O-methyl-adenosine
  modified_base 5: mod_base = OTHER; note = 2'-O-methyl-adenosine
  modified_base 6: mod_base = um
  modified_base 7: mod_base = cm
  modified_base 8: mod_base = um
  modified_base 9: mod_base = OTHER; note = 2'-Fluoro-guanosine
  modified_base 10: mod_base = OTHER; note = 2'-Fluoro-adenosine
  modified_base 11: mod_base = OTHER; note = 2'-Fluoro-uridine
  modified_base 12: mod_base = gm
  modified_base 13: mod_base = gm
  modified_base 14: mod_base = gm
  modified_base 15: mod_base = OTHER; note = 2'-O-methyl-adenosine
  modified_base 16: mod_base = um
  modified_base 17: mod_base = um
  modified_base 18: mod_base = OTHER; note = 2'-O-methyl-adenosine
  modified_base 19: mod_base = OTHER; note = 2'-O-methyl-adenosine
  modified_base 20: mod_base = gm
  modified_base 21: mod_base = gm
acaaatctgatgggattaagg

SEQ ID NO: 1351 - RNA, 21 nt, synthetic construct
  source 1..21: mol_type = other RNA
  modified_base <1: mod_base = OTHER; note = two inverted abasic nucleosides
  modified_base 1: mod_base = cm
  misc_feature 1^2: note = Phosphorothioate bond
  modified_base 2: mod_base = OTHER; note = 2'-O-methyl-adenosine
  misc_feature 2^3: note = Phosphorothioate bond
  modified_base 3: mod_base = OTHER; note = 2'-O-methyl-adenosine
  modified_base 4: mod_base = gm
  modified_base 5: mod_base = gm
  modified_base 6: mod_base = gm
  modified_base 7: mod_base = um
  modified_base 8: mod_base = gm
  modified_base 9: mod_base = OTHER; note = 2'-Fluoro-cytidine
  modified_base 10: mod_base = OTHER; note = 2'-Fluoro-adenosine
  modified_base 11: mod_base = OTHER; note = 2'-Fluoro-uridine
  modified_base 12: mod_base = gm
  modified_base 13: mod_base = gm
  modified_base 14: mod_base = um
  modified_base 15: mod_base = cm
  modified_base 16: mod_base = cm
  modified_base 17: mod_base = OTHER; note = 2'-O-methyl-adenosine
  modified_base 18: mod_base = OTHER; note = 2'-O-methyl-adenosine
  modified_base 19: mod_base = um
  modified_base 20: mod_base = gm
  modified_base 21: mod_base = um
caagggtgcatggtccaatgt

SEQ ID NO: 1352 - RNA, 21 nt, synthetic construct
  source 1..21: mol_type = other RNA
  modified_base <1: mod_base = OTHER; note = two inverted abasic nucleosides
  modified_base 1: mod_base = gm
  misc_feature 1^2: note = Phosphorothioate bond
  modified_base 2: mod_base = gm
  misc_feature 2^3: note = Phosphorothioate bond
  modified_base 3: mod_base = OTHER; note = 2'-O-methyl-adenosine
  modified_base 4: mod_base = um
  modified_base 5: mod_base = um
  modified_base 6: mod_base = OTHER; note = 2'-O-methyl-adenosine
  modified_base 7: mod_base = OTHER; note = 2'-O-methyl-adenosine
  modified_base 8: mod_base = gm
  modified_base 9: mod_base = OTHER; note = 2'-Fluoro-guanosine
  modified_base 10: mod_base = OTHER; note = 2'-Fluoro-guanosine
  modified_base 11: mod_base = OTHER; note = 2'-Fluoro-cytidine
  modified_base 12: mod_base = cm
  modified_base 13: mod_base = um
  modified_base 14: mod_base = gm
  modified_base 15: mod_base = um
  modified_base 16: mod_base = OTHER; note = 2'-O-methyl-adenosine
  modified_base 17: mod_base = cm
  modified_base 18: mod_base = cm
  modified_base 19: mod_base = OTHER; note = 2'-O-methyl-adenosine
  modified_base 20: mod_base = OTHER; note = 2'-O-methyl-adenosine
  modified_base 21: mod_base = gm
ggattaagggcctgtaccaag

SEQ ID NO: 1353 - RNA, 21 nt, synthetic construct
  source 1..21: mol_type = other RNA
  modified_base <1: mod_base = OTHER; note = two inverted abasic nucleosides
  modified_base 1: mod_base = um
  misc_feature 1^2: note = Phosphorothioate bond
  modified_base 2: mod_base = cm
  misc_feature 2^3: note = Phosphorothioate bond
  modified_base 3: mod_base = gm
  modified_base 4: mod_base = gm
  modified_base 5: mod_base = um
  modified_base 6: mod_base = OTHER; note = 2'-O-methyl-adenosine
  modified_base 7: mod_base = um
  modified_base 8: mod_base = cm
  modified_base 9: mod_base = OTHER; note = 2'-Fluoro-uridine
  modified_base 10: mod_base = OTHER; note = 2'-Fluoro-adenosine
  modified_base 11: mod_base = OTHER; note = 2'-Fluoro-uridine
  modified_base 12: mod_base = gm
  modified_base 13: mod_base = OTHER; note = 2'-O-methyl-adenosine
  modified_base 14: mod_base = cm
  modified_base 15: mod_base = OTHER; note = 2'-O-methyl-adenosine
  modified_base 16: mod_base = cm
  modified_base 17: mod_base = um
  modified_base 18: mod_base = gm
  modified_base 19: mod_base = cm
  modified_base 20: mod_base = OTHER; note = 2'-O-methyl-adenosine
  modified_base 21: mod_base = OTHER; note = 2'-O-methyl-adenosine
tcggtatctatgacactgcaa

SEQ ID NO: 1354 - RNA, 21 nt, synthetic construct
  source 1..21: mol_type = other RNA
  modified_base <1: mod_base = OTHER; note = two inverted abasic nucleosides
  modified_base 1: mod_base = cm
  misc_feature 1^2: note = Phosphorothioate bond
  modified_base 2: mod_base = OTHER; note = 2'-O-methyl-adenosine
  misc_feature 2^3: note = Phosphorothioate bond
  modified_base 3: mod_base = OTHER; note = 2'-O-methyl-adenosine
  modified_base 4: mod_base = gm
  modified_base 5: mod_base = gm
  modified_base 6: mod_base = cm
  modified_base 7: mod_base = um
  modified_base 8: mod_base = um
  modified_base 9: mod_base = OTHER; note = 2'-Fluoro-uridine
  modified_base 10: mod_base = OTHER; note = 2'-Fluoro-adenosine
  modified_base 11: mod_base = OTHER; note = 2'-Fluoro-adenosine
  modified_base 12: mod_base = cm
  modified_base 13: mod_base = gm
  modified_base 14: mod_base = um
  modified_base 15: mod_base = gm
  modified_base 16: mod_base = um
  modified_base 17: mod_base = cm
  modified_base 18: mod_base = um
  modified_base 19: mod_base = gm
  modified_base 20: mod_base = um
  modified_base 21: mod_base = gm
caaggctttaacgtgtctgtg

SEQ ID NO: 1355 - RNA, 21 nt, synthetic construct
  source 1..21: mol_type = other RNA
  modified_base <1: mod_base = OTHER; note = two inverted abasic nucleosides
  modified_base 1: mod_base = cm
  misc_feature 1^2: note = Phosphorothioate bond
  modified_base 2: mod_base = OTHER; note = 2'-O-methyl-adenosine
  misc_feature 2^3: note = Phosphorothioate bond
  modified_base 3: mod_base = um
  modified_base 4: mod_base = gm
  modified_base 5: mod_base = gm
  modified_base 6: mod_base = gm
  modified_base 7: mod_base = um
  modified_base 8: mod_base = gm
  modified_base 9: mod_base = OTHER; note = 2'-Fluoro-guanosine
  modified_base 10: mod_base = OTHER; note = 2'-Fluoro-uridine
  modified_base 11: mod_base = OTHER; note = 2'-Fluoro-guanosine
  modified_base 12: mod_base = cm
  modified_base 13: mod_base = um
  modified_base 14: mod_base = um
  modified_base 15: mod_base = um
  modified_base 16: mod_base = um
  modified_base 17: mod_base = gm
  modified_base 18: mod_base = um
  modified_base 19: mod_base = gm
  modified_base 20: mod_base = cm
  modified_base 21: mod_base = um
catgggtggtgcttttgtgct

SEQ ID NO: 1356 - RNA, 21 nt, synthetic construct
  source 1..21: mol_type = other RNA
  modified_base <1: mod_base = OTHER; note = two inverted abasic nucleosides
  modified_base 1: mod_base = um
  misc_feature 1^2: note = Phosphorothioate bond
  modified_base 2: mod_base = OTHER; note = 2'-O-methyl-adenosine
  misc_feature 2^3: note = Phosphorothioate bond
  modified_base 3: mod_base = OTHER; note = 2'-O-methyl-adenosine
  modified_base 4: mod_base = gm
  modified_base 5: mod_base = OTHER; note = 2'-O-methyl-adenosine
  modified_base 6: mod_base = um
  modified_base 7: mod_base = cm
  modified_base 8: mod_base = um
  modified_base 9: mod_base = OTHER; note = 2'-Fluoro-adenosine
  modified_base 10: mod_base = OTHER; note = 2'-Fluoro-cytidine
  modified_base 11: mod_base = OTHER; note = 2'-Fluoro-adenosine
  modified_base 12: mod_base = OTHER; note = 2'-O-methyl-adenosine
  modified_base 13: mod_base = OTHER; note = 2'-O-methyl-adenosine
  modified_base 14: mod_base = um
  modified_base 15: mod_base = cm
  modified_base 16: mod_base = um
  modified_base 17: mod_base = gm
  modified_base 18: mod_base = OTHER; note = 2'-O-methyl-adenosine
  modified_base 19: mod_base = um
  modified_base 20: mod_base = gm
  modified_base 21: mod_base = gm
taagatctacaaatctgatgg

SEQ ID NO: 1357 - RNA, 21 nt, synthetic construct
  source 1..21: mol_type = other RNA
  modified_base <1: mod_base = OTHER; note = two inverted abasic nucleosides
  modified_base 1: mod_base = cm
  misc_feature 1^2: note = Phosphorothioate bond
  modified_base 2: mod_base = cm
  misc_feature 2^3: note = Phosphorothioate bond
  modified_base 3: mod_base = cm
  modified_base 4: mod_base = gm
  modified_base 5: mod_base = um
  modified_base 6: mod_base = cm
  modified_base 7: mod_base = um
  modified_base 8: mod_base = OTHER; note = 2'-O-methyl-adenosine
  modified_base 9: mod_base = OTHER; note = 2'-Fluoro-guanosine
  modified_base 10: mod_base = OTHER; note = 2'-Fluoro-cytidine
  modified_base 11: mod_base = OTHER; note = 2'-Fluoro-adenosine
  modified_base 12: mod_base = gm
  modified_base 13: mod_base = cm
  modified_base 14: mod_base = um
  modified_base 15: mod_base = gm
  modified_base 16: mod_base = OTHER; note = 2'-O-methyl-adenosine
  modified_base 17: mod_base = um
  modified_base 18: mod_base = gm
  modified_base 19: mod_base = um
  modified_base 20: mod_base = gm
  modified_base 21: mod_base = gm
cccgtctagcagctgatgtgg

SEQ ID NO: 1358 - RNA, 21 nt, synthetic construct
  source 1..21: mol_type = other RNA
  modified_base <1: mod_base = OTHER; note = two inverted abasic nucleosides
  modified_base 1: mod_base = OTHER; note = 2'-O-methyl-adenosine
  misc_feature 1^2: note = Phosphorothioate bond
  modified_base 2: mod_base = um
  misc_feature 2^3: note = Phosphorothioate bond
  modified_base 3: mod_base = gm
  modified_base 4: mod_base = OTHER; note = 2'-O-methyl-adenosine
  modified_base 5: mod_base = cm
  modified_base 6: mod_base = OTHER; note = 2'-O-methyl-adenosine
  modified_base 7: mod_base = cm
  modified_base 8: mod_base = um
  modified_base 9: mod_base = OTHER; note = 2'-Fluoro-guanosine
  modified_base 10: mod_base = OTHER; note = 2'-Fluoro-cytidine
  modified_base 11: mod_base = OTHER; note = 2'-Fluoro-adenosine
  modified_base 12: mod_base = OTHER; note = 2'-O-methyl-adenosine
  modified_base 13: mod_base = OTHER; note = 2'-O-methyl-adenosine
  modified_base 14: mod_base = gm
  modified_base 15: mod_base = gm
  modified_base 16: mod_base = gm
  modified_base 17: mod_base = OTHER; note = 2'-O-methyl-adenosine
  modified_base 18: mod_base = OTHER; note = 2'-O-methyl-adenosine
  modified_base 19: mod_base = um
  modified_base 20: mod_base = gm
  modified_base 21: mod_base = cm
atgacactgcaaagggaatgc

SEQ ID NO: 1359 - RNA, 21 nt, synthetic construct
  source 1..21: mol_type = other RNA
  modified_base <1: mod_base = OTHER; note = two inverted abasic nucleosides
  modified_base 1: mod_base = um
  misc_feature 1^2: note = Phosphorothioate bond
  modified_base 2: mod_base = OTHER; note = 2'-O-methyl-adenosine
  misc_feature 2^3: note = Phosphorothioate bond
  modified_base 3: mod_base = gm
  modified_base 4: mod_base = cm
  modified_base 5: mod_base = OTHER; note = 2'-O-methyl-adenosine
  modified_base 6: mod_base = gm
  modified_base 7: mod_base = cm
  modified_base 8: mod_base = um
  modified_base 9: mod_base = OTHER; note = 2'-Fluoro-guanosine
  modified_base 10: mod_base = OTHER; note = 2'-Fluoro-adenosine
  modified_base 11: mod_base = OTHER; note = 2'-Fluoro-uridine
  modified_base 12: mod_base = gm
  modified_base 13: mod_base = um
  modified_base 14: mod_base = gm
  modified_base 15: mod_base = gm
  modified_base 16: mod_base = gm
  modified_base 17: mod_base = um
  modified_base 18: mod_base = OTHER; note = 2'-O-methyl-adenosine
  modified_base 19: mod_base = OTHER; note = 2'-O-methyl-adenosine
  modified_base 20: mod_base = OTHER; note = 2'-O-methyl-adenosine
  modified_base 21: mod_base = gm
tagcagctgatgtgggtaaag

SEQ ID NO: 1360 - RNA, 21 nt, synthetic construct
  source 1..21: mol_type = other RNA
  modified_base <1: mod_base = OTHER; note = two inverted abasic nucleosides
  modified_base 1: mod_base = gm
  misc_feature 1^2: note = Phosphorothioate bond
  modified_base 2: mod_base = cm
  misc_feature 2^3: note = Phosphorothioate bond
  modified_base 3: mod_base = OTHER; note = 2'-O-methyl-adenosine
  modified_base 4: mod_base = OTHER; note = 2'-O-methyl-adenosine
  modified_base 5: mod_base = OTHER; note = 2'-O-methyl-adenosine
  modified_base 6: mod_base = gm
  modified_base 7: mod_base = gm
  modified_base 8: mod_base = gm
  modified_base 9: mod_base = OTHER; note = 2'-Fluoro-adenosine
  modified_base 10: mod_base = OTHER; note = 2'-Fluoro-adenosine
  modified_base 11: mod_base = OTHER; note = 2'-Fluoro-uridine
  modified_base 12: mod_base = gm
  modified_base 13: mod_base = cm
  modified_base 14: mod_base = um
  modified_base 15: mod_base = um
  modified_base 16: mod_base = cm
  modified_base 17: mod_base = cm
  modified_base 18: mod_base = gm
  modified_base 19: mod_base = gm
  modified_base 20: mod_base = OTHER; note = 2'-O-methyl-adenosine
  modified_base 21: mod_base = um
gcaaagggaatgcttccggat

SEQ ID NO: 1361 - RNA, 21 nt, synthetic construct
  source 1..21: mol_type = other RNA
  modified_base <1: mod_base = OTHER; note = two inverted abasic nucleosides
  modified_base 1: mod_base = gm
  misc_feature 1^2: note = Phosphorothioate bond
  modified_base 2: mod_base = cm
  misc_feature 2^3: note = Phosphorothioate bond
  modified_base 3: mod_base = cm
  modified_base 4: mod_base = cm
  modified_base 5: mod_base = gm
  modified_base 6: mod_base = um
  modified_base 7: mod_base = OTHER; note = 2'-O-methyl-adenosine
  modified_base 8: mod_base = cm
  modified_base 9: mod_base = OTHER; note = 2'-Fluoro-cytidine
  modified_base 10: mod_base = OTHER; note = 2'-Fluoro-cytidine
  modified_base 11: mod_base = OTHER; note = 2'-Fluoro-guanosine
  modified_base 12: mod_base = um
  modified_base 13: mod_base = cm
  modified_base 14: mod_base = um
  modified_base 15: mod_base = OTHER; note = 2'-O-methyl-adenosine
  modified_base 16: mod_base = gm
  modified_base 17: mod_base = cm
  modified_base 18: mod_base = OTHER; note = 2'-O-methyl-adenosine
  modified_base 19: mod_base = gm
  modified_base 20: mod_base = cm
  modified_base 21: mod_base = um
gcccgtacccgtctagcagct

SEQ ID NO: 1362 - RNA, 21 nt, synthetic construct
  source 1..21: mol_type = other RNA
  modified_base <1: mod_base = OTHER; note = two inverted abasic nucleosides
  modified_base 1: mod_base = gm
  misc_feature 1^2: note = Phosphorothioate bond
  modified_base 2: mod_base = um
  misc_feature 2^3: note = Phosphorothioate bond
  modified_base 3: mod_base = OTHER; note = 2'-O-methyl-adenosine
  modified_base 4: mod_base = um
  modified_base 5: mod_base = um
  modified_base 6: mod_base = OTHER; note = 2'-O-methyl-adenosine
  modified_base 7: mod_base = um
  modified_base 8: mod_base = cm
  modified_base 9: mod_base = OTHER; note = 2'-Fluoro-adenosine
  modified_base 10: mod_base = OTHER; note = 2'-Fluoro-uridine
  modified_base 11: mod_base = OTHER; note = 2'-Fluoro-cytidine
  modified_base 12: mod_base = um
  modified_base 13: mod_base = OTHER; note = 2'-O-methyl-adenosine
  modified_base 14: mod_base = cm
  modified_base 15: mod_base = cm
  modified_base 16: mod_base = gm
  modified_base 17: mod_base = OTHER; note = 2'-O-methyl-adenosine
  modified_base 18: mod_base = gm
  modified_base 19: mod_base = cm
  modified_base 20: mod_base = cm
  modified_base 21: mod_base = gm
gtattatcatctaccgagccg

SEQ ID NO: 1363 - RNA, 21 nt, synthetic construct
  source 1..21: mol_type = other RNA
  modified_base <1: mod_base = OTHER; note = two inverted abasic nucleosides
  modified_base 1: mod_base = cm
  misc_feature 1^2: note = Phosphorothioate bond
  modified_base 2: mod_base = um
  misc_feature 2^3: note = Phosphorothioate bond
  modified_base 3: mod_base = cm
  modified_base 4: mod_base = um
  modified_base 5: mod_base = um
  modified_base 6: mod_base = gm
  modified_base 7: mod_base = OTHER; note = 2'-O-methyl-adenosine
  modified_base 8: mod_base = um
  modified_base 9: mod_base = OTHER; note = 2'-Fluoro-uridine
  modified_base 10: mod_base = OTHER; note = 2'-Fluoro-uridine
  modified_base 11: mod_base = OTHER; note = 2'-Fluoro-uridine
  modified_base 12: mod_base = gm
  modified_base 13: mod_base = cm
  modified_base 14: mod_base = cm
  modified_base 15: mod_base = cm
  modified_base 16: mod_base = gm
  modified_base 17: mod_base = um
  modified_base 18: mod_base = OTHER; note = 2'-O-methyl-adenosine
  modified_base 19: mod_base = cm
  modified_base 20: mod_base = cm
  modified_base 21: mod_base = cm
ctcttgattttgcccgtaccc

SEQ ID NO: 1364 - RNA, 21 nt, synthetic construct
  source 1..21: mol_type = other RNA
  modified_base <1: mod_base = OTHER; note = two inverted abasic nucleosides
  modified_base 1: mod_base = um
  misc_feature 1^2: note = Phosphorothioate bond
  modified_base 2: mod_base = OTHER; note = 2'-O-methyl-adenosine
  misc_feature 2^3: note = Phosphorothioate bond
  modified_base 3: mod_base = cm
  modified_base 4: mod_base = cm
  modified_base 5: mod_base = cm
  modified_base 6: mod_base = gm
  modified_base 7: mod_base = um
  modified_base 8: mod_base = cm
  modified_base 9: mod_base = OTHER; note = 2'-Fluoro-uridine
  modified_base 10: mod_base = OTHER; note = 2'-Fluoro-adenosine
  modified_base 11: mod_base = OTHER; note = 2'-Fluoro-guanosine
  modified_base 12: mod_base = cm
  modified_base 13: mod_base = OTHER; note = 2'-O-methyl-adenosine
  modified_base 14: mod_base = gm
  modified_base 15: mod_base = cm
  modified_base 16: mod_base = um
  modified_base 17: mod_base = gm
  modified_base 18: mod_base = OTHER; note = 2'-O-methyl-adenosine
  modified_base 19: mod_base = um
  modified_base 20: mod_base = gm
  modified_base 21: mod_base = um
tacccgtctagcagctgatgt

SEQ ID NO: 1365 - RNA, 21 nt, synthetic construct
  source 1..21: mol_type = other RNA
  modified_base <1: mod_base = OTHER; note = two inverted abasic nucleosides
  modified_base 1: mod_base = cm
  misc_feature 1^2: note = Phosphorothioate bond
  modified_base 2: mod_base = OTHER; note = 2'-O-methyl-adenosine
  misc_feature 2^3: note = Phosphorothioate bond
  modified_base 3: mod_base = OTHER; note = 2'-O-methyl-adenosine
  modified_base 4: mod_base = OTHER; note = 2'-O-methyl-adenosine
  modified_base 5: mod_base = um
  modified_base 6: mod_base = cm
  modified_base 7: mod_base = um
  modified_base 8: mod_base = gm
  modified_base 9: mod_base = OTHER; note = 2'-Fluoro-adenosine
  modified_base 10: mod_base = OTHER; note = 2'-Fluoro-uridine
  modified_base 11: mod_base = OTHER; note = 2'-Fluoro-guanosine
  modified_base 12: mod_base = gm
  modified_base 13: mod_base = gm
  modified_base 14: mod_base = OTHER; note = 2'-O-methyl-adenosine
  modified_base 15: mod_base = um
  modified_base 16: mod_base = um
  modified_base 17: mod_base = OTHER; note = 2'-O-methyl-adenosine
  modified_base 18: mod_base = OTHER; note = 2'-O-methyl-adenosine
  modified_base 19: mod_base = gm
  modified_base 20: mod_base = gm
  modified_base 21: mod_base = gm
caaatctgatgggattaaggg

SEQ ID NO: 1366 - RNA, 21 nt, synthetic construct
  source 1..21: mol_type = other RNA
  modified_base <1: mod_base = OTHER; note = two inverted abasic nucleosides
  modified_base 1: mod_base = gm
  misc_feature 1^2: note = Phosphorothioate bond
  modified_base 2: mod_base = um
  misc_feature 2^3: note = Phosphorothioate bond
  modified_base 3: mod_base = OTHER; note = 2'-O-methyl-adenosine
  modified_base 4: mod_base = cm
  modified_base 5: mod_base = cm
  modified_base 6: mod_base = cm
  modified_base 7: mod_base = um
  modified_base 8: mod_base = cm
  modified_base 9: mod_base = OTHER; note = 2'-Fluoro-uridine
  modified_base 10: mod_base = OTHER; note = 2'-Fluoro-uridine
  modified_base 11: mod_base = OTHER; note = 2'-Fluoro-guanosine
  modified_base 12: mod_base = OTHER; note = 2'-O-methyl-adenosine
  modified_base 13: mod_base = um
  modified_base 14: mod_base = um
  modified_base 15: mod_base = um
  modified_base 16: mod_base = um
  modified_base 17: mod_base = gm
  modified_base 18: mod_base = cm
  modified_base 19: mod_base = cm
  modified_base 20: mod_base = cm
  modified_base 21: mod_base = gm
gtaccctcttgattttgcccg

SEQ ID NO: 1367 - RNA, 21 nt, synthetic construct
  source 1..21: mol_type = other RNA
  modified_base <1: mod_base = OTHER; note = two inverted abasic nucleosides
  modified_base 1: mod_base = cm
  misc_feature 1^2: note = Phosphorothioate bond
  modified_base 2: mod_base = cm
  misc_feature 2^3: note = Phosphorothioate bond
  modified_base 3: mod_base = um
  modified_base 4: mod_base = gm
  modified_base 5: mod_base = um
  modified_base 6: mod_base = OTHER; note = 2'-O-methyl-adenosine
  modified_base 7: mod_base = cm
  modified_base 8: mod_base = cm
  modified_base 9: mod_base = OTHER; note = 2'-Fluoro-adenosine
  modified_base 10: mod_base = OTHER; note = 2'-Fluoro-adenosine
  modified_base 11: mod_base = OTHER; note = 2'-Fluoro-guanosine
  modified_base 12: mod_base = gm
  modified_base 13: mod_base = cm
  modified_base 14: mod_base = um
  modified_base 15: mod_base = um
  modified_base 16: mod_base = um
  modified_base 17: mod_base = OTHER; note = 2'-O-methyl-adenosine
  modified_base 18: mod_base = OTHER; note = 2'-O-methyl-adenosine
  modified_base 19: mod_base = cm
  modified_base 20: mod_base = gm
  modified_base 21: mod_base = um
cctgtaccaaggctttaacgt

SEQ ID NO: 1368 - RNA, 21 nt, synthetic construct
  source 1..21: mol_type = other RNA
  modified_base <1: mod_base = OTHER; note = two inverted abasic nucleosides
  modified_base 1: mod_base = um
  misc_feature 1^2: note = Phosphorothioate bond
  modified_base 2: mod_base = gm
  misc_feature 2^3: note = Phosphorothioate bond
  modified_base 3: mod_base = gm
  modified_base 4: mod_base = gm
  modified_base 5: mod_base = OTHER; note = 2'-O-methyl-adenosine
  modified_base 6: mod_base = um
  modified_base 7: mod_base = um
  modified_base 8: mod_base = OTHER; note = 2'-O-methyl-adenosine
  modified_base 9: mod_base = OTHER; note = 2'-Fluoro-adenosine
  modified_base 10: mod_base = OTHER; note = 2'-Fluoro-guanosine
  modified_base 11: mod_base = OTHER; note = 2'-Fluoro-guanosine
  modified_base 12: mod_base = gm
  modified_base 13: mod_base = cm
  modified_base 14: mod_base = cm
  modified_base 15: mod_base = um
  modified_base 16: mod_base = gm
  modified_base 17: mod_base = um
  modified_base 18: mod_base = OTHER; note = 2'-O-methyl-adenosine
  modified_base 19: mod_base = cm
  modified_base 20: mod_base = cm
  modified_base 21: mod_base = OTHER; note = 2'-O-methyl-adenosine
tgggattaagggcctgtacca

SEQ ID NO: 1369 - RNA, 21 nt, synthetic construct
  source 1..21: mol_type = other RNA
  modified_base <1: mod_base = OTHER; note = two inverted abasic nucleosides
  modified_base 1: mod_base = OTHER; note = 2'-O-methyl-adenosine
  misc_feature 1^2: note = Phosphorothioate bond
  modified_base 2: mod_base = um
  misc_feature 2^3: note = Phosphorothioate bond
  modified_base 3: mod_base = um
  modified_base 4: mod_base = OTHER; note = 2'-O-methyl-adenosine
  modified_base 5: mod_base = um
  modified_base 6: mod_base = cm
  modified_base 7: mod_base = OTHER; note = 2'-O-methyl-adenosine
  modified_base 8: mod_base = um
  modified_base 9: mod_base = OTHER; note = 2'-Fluoro-cytidine
  modified_base 10: mod_base = OTHER; note = 2'-Fluoro-uridine
  modified_base 11: mod_base = OTHER; note = 2'-Fluoro-adenosine
  modified_base 12: mod_base = cm
  modified_base 13: mod_base = cm
  modified_base 14: mod_base = gm
  modified_base 15: mod_base = OTHER; note = 2'-O-methyl-adenosine
  modified_base 16: mod_base = gm
  modified_base 17: mod_base = cm
  modified_base 18: mod_base = cm
  modified_base 19: mod_base = gm
  modified_base 20: mod_base = cm
  modified_base 21: mod_base = cm
attatcatctaccgagccgcc

SEQ ID NO: 1370 - RNA, 21 nt, synthetic construct
  source 1..21: mol_type = other RNA
  modified_base <1: mod_base = OTHER; note = two inverted abasic nucleosides
  modified_base 1: mod_base = gm
  misc_feature 1^2: note = Phosphorothioate bond
  modified_base 2: mod_base = cm
  misc_feature 2^3: note = Phosphorothioate bond
  modified_base 3: mod_base = cm
  modified_base 4: mod_base = um
  modified_base 5: mod_base = gm
  modified_base 6: mod_base = um
  modified_base 7: mod_base = OTHER; note = 2'-O-methyl-adenosine
  modified_base 8: mod_base = cm
  modified_base 9: mod_base = OTHER; note = 2'-Fluoro-cytidine
  modified_base 10: mod_base = OTHER; note = 2'-Fluoro-adenosine
  modified_base 11: mod_base = OTHER; note = 2'-Fluoro-adenosine
  modified_base 12: mod_base = gm
  modified_base 13: mod_base = gm
  modified_base 14: mod_base = cm
  modified_base 15: mod_base = um
  modified_base 16: mod_base = um
  modified_base 17: mod_base = um
  modified_base 18: mod_base = OTHER; note = 2'-O-methyl-adenosine
  modified_base 19: mod_base = OTHER; note = 2'-O-methyl-adenosine
  modified_base 20: mod_base = cm
  modified_base 21: mod_base = gm
gcctgtaccaaggctttaacg

SEQ ID NO: 1371 - RNA, 21 nt, synthetic construct
  source 1..21: mol_type = other RNA
  modified_base <1: mod_base = OTHER; note = two inverted abasic nucleosides
  modified_base 1: mod_base = OTHER; note = 2'-O-methyl-adenosine
  misc_feature 1^2: note = Phosphorothioate bond
  modified_base 2: mod_base = um
  misc_feature 2^3: note = Phosphorothioate bond
  modified_base 3: mod_base = gm
  modified_base 4: mod_base = gm
  modified_base 5: mod_base = gm
  modified_base 6: mod_base = OTHER; note = 2'-O-methyl-adenosine
  modified_base 7: mod_base = um
  modified_base 8: mod_base = um
  modified_base 9: mod_base = OTHER; note = 2'-Fluoro-adenosine
  modified_base 10: mod_base = OTHER; note = 2'-Fluoro-adenosine
  modified_base 11: mod_base = OTHER; note = 2'-Fluoro-guanosine
  modified_base 12: mod_base = gm
  modified_base 13: mod_base = gm
  modified_base 14: mod_base = cm
  modified_base 15: mod_base = cm
  modified_base 16: mod_base = um
  modified_base 17: mod_base = gm
  modified_base 18: mod_base = um
  modified_base 19: mod_base = OTHER; note = 2'-O-methyl-adenosine
  modified_base 20: mod_base = cm
  modified_base 21: mod_base = cm
atgggattaagggcctgtacc

SEQ ID NO: 1372 - RNA, 21 nt, synthetic construct
  source 1..21: mol_type = other RNA
  modified_base <1: mod_base = OTHER; note = two inverted abasic nucleosides
  modified_base 1: mod_base = OTHER; note = 2'-O-methyl-adenosine
  misc_feature 1^2: note = Phosphorothioate bond
  modified_base 2: mod_base = cm
  misc_feature 2^3: note = Phosphorothioate bond
  modified_base 3: mod_base = gm
  modified_base 4: mod_base = um
  modified_base 5: mod_base = gm
  modified_base 6: mod_base = um
  modified_base 7: mod_base = cm
  modified_base 8: mod_base = um
  modified_base 9: mod_base = OTHER; note = 2'-Fluoro-guanosine
  modified_base 10: mod_base = OTHER; note = 2'-Fluoro-uridine
  modified_base 11: mod_base = OTHER; note = 2'-Fluoro-guanosine
  modified_base 12: mod_base = cm
  modified_base 13: mod_base = OTHER; note = 2'-O-methyl-adenosine
  modified_base 14: mod_base = gm
  modified_base 15: mod_base = gm
  modified_base 16: mod_base = gm
  modified_base 17: mod_base = um
  modified_base 18: mod_base = OTHER; note = 2'-O-methyl-adenosine
  modified_base 19: mod_base = um
  modified_base 20: mod_base = um
  modified_base 21: mod_base = OTHER; note = 2'-O-methyl-adenosine
acgtgtctgtgcagggtatta

SEQ ID NO: 1373 - RNA, 21 nt, synthetic construct
  source 1..21: mol_type = other RNA
  modified_base <1: mod_base = OTHER; note = two inverted abasic nucleosides
  modified_base 1: mod_base = gm
  misc_feature 1^2: note = Phosphorothioate bond
  modified_base 2: mod_base = gm
  misc_feature 2^3: note = Phosphorothioate bond
  modified_base 3: mod_base = cm
  modified_base 4: mod_base = OTHER; note = 2'-O-methyl-adenosine
  modified_base 5: mod_base = um
  modified_base 6: mod_base = um
  modified_base 7: mod_base = OTHER; note = 2'-O-methyl-adenosine
  modified_base 8: mod_base = um
  modified_base 9: mod_base = OTHER; note = 2'-Fluoro-adenosine
  modified_base 10: mod_base = OTHER; note = 2'-Fluoro-guanosine
  modified_base 11: mod_base = OTHER; note = 2'-Fluoro-adenosine
  modified_base 12: mod_base = cm
  modified_base 13: mod_base = um
  modified_base 14: mod_base = gm
  modified_base 15: mod_base = cm
  modified_base 16: mod_base = gm
  modified_base 17: mod_base = um
  modified_base 18: mod_base = gm
  modified_base 19: mod_base = gm
  modified_base 20: mod_base = um
  modified_base 21: mod_base = cm
ggcattatagactgcgtggtc

SEQ ID NO: 1374 - RNA, 21 nt, synthetic construct
  source 1..21: mol_type = other RNA
  modified_base <1: mod_base = OTHER; note = two inverted abasic nucleosides
  modified_base 1: mod_base = um
  misc_feature 1^2: note = Phosphorothioate bond
  modified_base 2: mod_base = um
  misc_feature 2^3: note = Phosphorothioate bond
  modified_base 3: mod_base = cm
  modified_base 4: mod_base = cm
  modified_base 5: mod_base = cm
  modified_base 6: mod_base = cm
  modified_base 7: mod_base = OTHER; note = 2'-O-methyl-adenosine
  modified_base 8: mod_base = cm
  modified_base 9: mod_base = OTHER; note = 2'-Fluoro-cytidine
  modified_base 10: mod_base = OTHER; note = 2'-Fluoro-cytidine
  modified_base 11: mod_base = OTHER; note = 2'-Fluoro-adenosine
  modified_base 12: mod_base = gm
  modified_base 13: mod_base = gm
  modified_base 14: mod_base = cm
  modified_base 15: mod_base = um
  modified_base 16: mod_base = cm
  modified_base 17: mod_base = um
  modified_base 18: mod_base = um
  modified_base 19: mod_base = OTHER; note = 2'-O-methyl-adenosine
  modified_base 20: mod_base = OTHER; note = 2'-O-methyl-adenosine
  modified_base 21: mod_base = cm
ttccccacccaggctcttaac

SEQ ID NO: 1375 - RNA, 21 nt, synthetic construct
  source 1..21: mol_type = other RNA
  modified_base <1: mod_base = OTHER; note = two inverted abasic nucleosides
  modified_base 1: mod_base = OTHER; note = 2'-O-methyl-adenosine
  misc_feature 1^2: note = Phosphorothioate bond
  modified_base 2: mod_base = um
  misc_feature 2^3: note = Phosphorothioate bond
  modified_base 3: mod_base = gm
  modified_base 4: mod_base = um
  modified_base 5: mod_base = cm
  modified_base 6: mod_base = OTHER; note = 2'-O-methyl-adenosine
  modified_base 7: mod_base = um
  modified_base 8: mod_base = cm
  modified_base 9: mod_base = OTHER; note = 2'-Fluoro-adenosine
  modified_base 10: mod_base = OTHER; note = 2'-Fluoro-guanosine
  modified_base 11: mod_base = OTHER; note = 2'-Fluoro-adenosine
  modified_base 12: mod_base = um
  modified_base 13: mod_base = OTHER; note = 2'-O-methyl-adenosine
  modified_base 14: mod_base = cm
  modified_base 15: mod_base = um
  modified_base 16: mod_base = um
  modified_base 17: mod_base = cm
  modified_base 18: mod_base = cm
  modified_base 19: mod_base = cm
  modified_base 20: mod_base = cm
  modified_base 21: mod_base = OTHER; note = 2'-O-methyl-adenosine
atgtcatcagatacttcccca

SEQ ID NO: 1376 - RNA, 21 nt, synthetic construct
  source 1..21: mol_type = other RNA
  modified_base <1: mod_base = OTHER; note = two inverted abasic nucleosides
  modified_base 1: mod_base = gm
  misc_feature 1^2: note = Phosphorothioate bond
  modified_base 2: mod_base = um
  misc_feature 2^3: note = Phosphorothioate bond
  modified_base 3: mod_base = cm
  modified_base 4: mod_base = OTHER; note = 2'-O-methyl-adenosine
  modified_base 5: mod_base = um
  modified_base 6: mod_base = cm
  modified_base 7: mod_base = OTHER; note = 2'-O-methyl-adenosine
  modified_base 8: mod_base = gm
  modified_base 9: mod_base = OTHER; note = 2'-Fluoro-adenosine
  modified_base 10: mod_base = OTHER; note = 2'-Fluoro-uridine
  modified_base 11: mod_base = OTHER; note = 2'-Fluoro-adenosine
  modified_base 12: mod_base = cm
  modified_base 13: mod_base = um
  modified_base 14: mod_base = um
  modified_base 15: mod_base = cm
  modified_base 16: mod_base = cm
  modified_base 17: mod_base = cm
  modified_base 18: mod_base = cm
  modified_base 19: mod_base = OTHER; note = 2'-O-methyl-adenosine
  modified_base 20: mod_base = cm
  modified_base 21: mod_base = cm
gtcatcagatacttccccacc

SEQ ID NO: 1377 - RNA, 21 nt, synthetic construct
  source 1..21: mol_type = other RNA
  modified_base <1: mod_base = OTHER; note = two inverted abasic nucleosides
  modified_base 1: mod_base = um
  misc_feature 1^2: note = Phosphorothioate bond
  modified_base 2: mod_base = gm
  misc_feature 2^3: note = Phosphorothioate bond
  modified_base 3: mod_base = um
  modified_base 4: mod_base = cm
  modified_base 5: mod_base = OTHER; note = 2'-O-methyl-adenosine
  modified_base 6: mod_base = um
  modified_base 7: mod_base = cm
  modified_base 8: mod_base = OTHER; note = 2'-O-methyl-adenosine
  modified_base 9: mod_base = OTHER; note = 2'-Fluoro-guanosine
  modified_base 10: mod_base = OTHER; note = 2'-Fluoro-adenosine
  modified_base 11: mod_base = OTHER; note = 2'-Fluoro-uridine
  modified_base 12: mod_base = OTHER; note = 2'-O-methyl-adenosine
  modified_base 13: mod_base = cm
  modified_base 14: mod_base = um
  modified_base 15: mod_base = um
  modified_base 16: mod_base = cm
  modified_base 17: mod_base = cm
  modified_base 18: mod_base = cm
  modified_base 19: mod_base = cm
  modified_base 20: mod_base = OTHER; note = 2'-O-methyl-adenosine
  modified_base 21: mod_base = cm
tgtcatcagatacttccccac

SEQ ID NO: 1378 - RNA, 21 nt, synthetic construct
  source 1..21: mol_type = other RNA
  modified_base <1: mod_base = OTHER; note = two inverted abasic nucleosides
  modified_base 1: mod_base = OTHER; note = 2'-O-methyl-adenosine
  misc_feature 1^2: note = Phosphorothioate bond
  modified_base 2: mod_base = OTHER; note = 2'-O-methyl-adenosine
  misc_feature 2^3: note = Phosphorothioate bond
  modified_base 3: mod_base = um
  modified_base 4: mod_base = gm
  modified_base 5: mod_base = um
  modified_base 6: mod_base = cm
  modified_base 7: mod_base = OTHER; note = 2'-O-methyl-adenosine
  modified_base 8: mod_base = um
  modified_base 9: mod_base = OTHER; note = 2'-Fluoro-cytidine
  modified_base 10: mod_base = OTHER; note = 2'-Fluoro-adenosine
  modified_base 11: mod_base = OTHER; note = 2'-Fluoro-guanosine
  modified_base 12: mod_base = OTHER; note = 2'-O-methyl-adenosine
  modified_base 13: mod_base = um
  modified_base 14: mod_base = OTHER; note = 2'-O-methyl-adenosine
  modified_base 15: mod_base = cm
  modified_base 16: mod_base = um
  modified_base 17: mod_base = um
  modified_base 18: mod_base = cm
  modified_base 19: mod_base = cm
  modified_base 20: mod_base = cm
  modified_base 21: mod_base = cm
aatgtcatcagatacttcccc

SEQ ID NO: 1379 - RNA, 21 nt, synthetic construct
  source 1..21: mol_type = other RNA
  modified_base <1: mod_base = OTHER; note = two inverted abasic nucleosides
  modified_base 1: mod_base = cm
  misc_feature 1^2: note = Phosphorothioate bond
  modified_base 2: mod_base = um
  misc_feature 2^3: note = Phosphorothioate bond
  modified_base 3: mod_base = um
  modified_base 4: mod_base = cm
  modified_base 5: mod_base = cm
  modified_base 6: mod_base = cm
  modified_base 7: mod_base = cm
  modified_base 8: mod_base = OTHER; note = 2'-O-methyl-adenosine
  modified_base 9: mod_base = OTHER; note = 2'-Fluoro-cytidine
  modified_base 10: mod_base = OTHER; note = 2'-Fluoro-cytidine
  modified_base 11: mod_base = OTHER; note = 2'-Fluoro-cytidine
  modified_base 12: mod_base = OTHER; note = 2'-O-methyl-adenosine
  modified_base 13: mod_base = gm
  modified_base 14: mod_base = gm
  modified_base 15: mod_base = cm
  modified_base 16: mod_base = um
  modified_base 17: mod_base = cm
  modified_base 18: mod_base = um
  modified_base 19: mod_base = um
  modified_base 20: mod_base = OTHER; note = 2'-O-methyl-adenosine
  modified_base 21: mod_base = OTHER; note = 2'-O-methyl-adenosine
cttccccacccaggctcttaa

SEQ ID NO: 1380 - RNA, 21 nt, synthetic construct
  source 1..21: mol_type = other RNA
  modified_base <1: mod_base = OTHER; note = two inverted abasic nucleosides
  modified_base 1: mod_base = cm
  misc_feature 1^2: note = Phosphorothioate bond
  modified_base 2: mod_base = um
  misc_feature 2^3: note = Phosphorothioate bond
  modified_base 3: mod_base = OTHER; note = 2'-O-methyl-adenosine
  modified_base 4: mod_base = cm
  modified_base 5: mod_base = cm
  modified_base 6: mod_base = gm
  modified_base 7: mod_base = OTHER; note = 2'-O-methyl-adenosine
  modified_base 8: mod_base = gm
  modified_base 9: mod_base = OTHER; note = 2'-Fluoro-cytidine
  modified_base 10: mod_base = OTHER; note = 2'-Fluoro-cytidine
  modified_base 11: mod_base = OTHER; note = 2'-Fluoro-guanosine
  modified_base 12: mod_base = cm
  modified_base 13: mod_base = cm
  modified_base 14: mod_base = um
  modified_base 15: mod_base = OTHER; note = 2'-O-methyl-adenosine
  modified_base 16: mod_base = cm
  modified_base 17: mod_base = um
  modified_base 18: mod_base = um
  modified_base 19: mod_base = cm
  modified_base 20: mod_base = gm
  modified_base 21: mod_base = gm
ctaccgagccgcctacttcgg

SEQ ID NO: 1381 - DNA, 2975 bp, Homo sapiens
  source 1..2975: mol_type = genomic DNA
atcggccatttgcttcgctccgccccgcagcgccggagtcaaagccggttcccggcccagtcccgtcctgcagcagtctgcctcctctttcaacatgacagatgccgctgtgtccttcgccaaggacttcctggcaggtggagtggccgcagccatctccaagacggcggtagcgcccatcgagcgggtcaagctgctgctgcaggtacgtcctgggatccaggagcccaaccaggaagtggggggaagggtcgcacagaaggcgggcgcccgaggggtggcggggagcgaactctaaagacatggccagggaagcggcttaggagaggccagagcggggcgcagaggcagaacagaagtcaaactggtgggaggcgcctttagtgacctgaagtagtgagtctaggaaggggccgggggcagagggcaggaccaggctctcggcatctccgaggcggcggactcggatggagcagtttctgagtgacggcctccccgggcctgggcgtcaagggcgaaggccgaaagccggcgttagaaagaggaacgccagttcttaccgaagacctcaaggtcgcggcaaggagataactgcccgggggaggccatgcgcccgggtccagcggcctcccagcccgcggacgcgctcaaacctcgccgggccggaagccggcgccgggaagcgcgtgtgccttttacgtccgcccccgcgcagccgcggccgctgccgccgcgtctccgcctgcctccctgcgccgcgcgctctccagtgccggctctagagggcgctcctgggctagcgtgtagggctggcggcggcggcgctcgggtcacctctgggagcggagtgggggcggagcgagacggaagcagctcaggagacttgaggcgtaggctgcggtccccaaggtgaccgcgccctatgtgggactcgccctaatgcctctgaacctgggtttgaggtaatgacctttctcctaggtctgaaggtcacgggtccgctggaggatgccccctctccactcagaggggtggaggcttaatgctactggtgcagatcacctcttcccctgtgacagcctcagagggttgggagggtccagccagtatgatatacgaagactagatttgagagaggggagcctaccttaaagggcattgatcgagatggcataagctcttctctttcccttccccatggttataactgtccctgttggcttccttcctgtctgttaggtgcagcatgccagcaagcagatcactgcagataagcaatacaaaggcattatagactgcgtggtccgtattcccaaggagcagggagttctgtccttctggcgcggtaacctggccaatgtcatcagatacttccccacccaggctcttaacttcgccttcaaagataaatacaagcagatcttcctgggtggtgtggacaagagaacccagttttggctctactttgcagggaatctggcatcgggtggtgccgcaggggccacatccctgtgttttgtgtaccctcttgattttgcccgtacccgtctagcagctgatgtgggtaaagctggagctgaaagggaattccgaggcctcggtgactgcctggttaagatctacaaatctgatgggattaagggcctgtaccaaggctttaacgtgtctgtgcagggtattatcatctaccgagccgcctacttcggtatctatgacactgcaaagggtaagtttgctgtgggctttaacgttgtgttcttaggagacagtttaaaagagcattgtaccaacctaacagtccaagagctaaagagttgtttttttaattgctaaaggaagccaagatcatccaatgcaacccttgtgtacagatgacgtgtttaggggatgtggggaaaggaagtcagtaaaactctgctttttggtaaaagcatctctttcctattcccaggaatgcttccggatcccaagaacactcacatcgtcatcagctggatgatcgcacagactgtcactgctgttgccgggttgacttcctatccatttgacactgttcgccgccgcatgatgatgcagtcagggcgcaaaggaagtaagttccacttgagcagaagataaagttgtagtcgtggggcaatctgctgccacaaactggtgatacatacctttaaaatggctgtctgtccaagtcaagggatggggttgatagcatctgtgtctgttccacaactgcctttgagctggcccttcagatgcctatgaatgagggtgcttaaatggtgttagaggttaagaccaatgggtagtctgtattcctgtggtcatagcattaatatttcagtgttgcccatgctaatgtgtgaatgttggatttaaagctgacgttcttagaggtggggctctgctttatttagcctagtgaatcttaggatttttcatcggccttcagtcactaactccatgtctttattctttgcagctgacatcatgtacacaggcacgcttgactgctggcggaagattgctcgtgatgaaggaggcaaagcttttttcaagggtgcatggtccaatgttctcagaggcatgggtggtgcttttgtgcttgtcttgtatgatgaaatcaagaagtacacataagttatttcctaggatttttccccctgtgaacaggcatgttgtattatataacatatcttgagcattcttgacagactcctggctgtcagtttctcagtggcaactatttactggttgaaaatgggaagcaataatattcatctgaccagttttctcttaaagccatttccatgatgatgatgatgggactcaattgtattttttatttcagtcactcctgataaataacaaatttggagaaataaaaatatctaaaataaattttgtctgcagtatattttcatataaaaatgcatatttgagtgctacattcgaataaatactacctttttagtgaa

SEQ ID NO: 1382 - RNA, 19 nt, synthetic construct
  source 1..19: mol_type = other RNA
ttaaagccttggtacaggc

SEQ ID NO: 1383 - RNA, 19 nt, synthetic construct
  source 1..19: mol_type = other RNA
gcctgtaccaaggctttaa

SEQ ID NO: 1384 - DNA, 23 bp, synthetic construct
  source 1..23: mol_type = other DNA
actgacatcatgtacacaggcac

SEQ ID NO: 1385 - DNA, 21 bp, synthetic construct
  source 1..21: mol_type = other DNA
acccatgcctctgagaacatt

SEQ ID NO: 1386 - DNA, 19 bp, synthetic construct
  source 1..19: mol_type = other DNA
gaaggtgaaggtcggagtc

SEQ ID NO: 1387 - DNA, 20 bp, synthetic construct
  source 1..20: mol_type = other DNA
gaagatggtgatgggatttc

SEQ ID NO: 1388 - protein, 31 aa, Homo sapiens
HAEGTFTSDVSSYLEGQAAKEFIAWLVKGRG

SEQ ID NO: 1389 - protein, 38 aa, synthetic construct
  SITE 2: note = Aib
  SITE 13: note = Aib
  SITE 20: note = K at position 20 is chemically modified through conjugation to the epsilon-amino group of the K side-chain with (2-[2-(2-Amino-ethoxy)-ethoxy]-acetyl)2-(gammaGlu)1-CO-(CH2)18-CO2H
  SITE 38: note = the C-terminal amino acid is amidated as a C-terminal primary amide
YXEGTFTSDYSIXLDKIAQKAFVQWLMGGPSSGAPPPS

SEQ ID NO: 1390 - protein, 9 aa, Mus musculus
QIFLGGVDK

SEQ ID NO: 1391 - protein, 9 aa, Mus musculus
EQGVLSFWR